European Patent Application EP 4 520 821 A1 - sequence listing, part 15

SEQ ID NO: 19186 - RNA, 4853 nt, Homo sapiens
  source 1..4853: mol_type = other RNA
tgtcttctctcctcccaaacaggcatttgatttgaaaacagaaaccagaacagagcatacaccacaaggaaacatggtacttacaaatattgtcaaataattcagcagaactctttaagaaaaaaaaaaggttcttagaaattgagaaagcagtagaaccacccagcctggcagatcaatctaccagatgttctgcatgcgagagggctcccaaccacctgtaacttcagaaaggccgccaggcactattacgaaggaaacaggtgcagatcctaactggagatgactttatcacaaagccttaagacaaagggaccatcctcttccaagacaacaggtgtgaacagaggcaaggagcgagaggagagggctccctcagcagatgggtggaaagcaagcctgcccttgcacggcccttggcacactcaatctaccccctttcccttctctgcccctggcaaagaaaggctgggcaagtgcaagagcccagaatggctcctccaggcacatggttaaagtaagagtaagaggaaaacaagccccttctgggtgaaatatggcaacttttctgagacatggcaacgaggcagagttaatctctttggccctcatcaggtaaagcagcaactaaggagcctactcagggccttacgtgggccccttctatgtccacaagaaagtgcatccttagctcagttcaacatttaaaaagagctaacgctacttgcaaaaggcccaccatggattcaaacacttaataccaaagaggtccagcaactcgcgagtctgtctgtgttctgtgatctgaagcagagctaaggggggcctggctcacagggtcacgctcttctgccaaggcgcctcagggagggaaaaaaaggcatgatgatgtctgtgagccagaacctgcaggaggaccaccggtagagattctagaagacaaagaagccctcaggaggctctgagaggtgtccaatgtctaagagacggccaccccctccatctctagcttcgagtcaacgctgttacagtcactctccggaaaccagctcttcctttatccacctgcacggcccctgccacagtgagggaaagatctggtccctctgacagtaaggaaattgtatagaaattatcctgaggaaaaaaaaaaccactgtgacgctacctaaaagaaagagtatttcaatttgcttacacagatttagtcagtacactccagactgtaagaaatgtatgaagagactgcttacggaactcaaagactaaacagtgaatactactgtggcccagacacggatcgaaaacacttctcccagtggcttctggtgctatgtctgctctcccgagagcgtccagcaaggtcttccatgcagacagggtgaggagccacagagctcaagattgttgaagctgatttagtgagctctgtaaagcaatactcaaacagctccgtacgaaaaggtgtcatttacattattatttatatatagtatctcgaagtaaggaaaaaagcaccattttactgaaaataaaaaggctcacgcaggctttggtcctcctgaaatgacaccagcctgagtgagaagcagttggcccttggggagcggggagatgatggaacgctgtcaccggcaagaagggaggccaagtggcccggcaagccacaagaatggggcaataaggggagcaggtggaggggcctcggagagcagccaggctagtctggggatggagccacctgctctgagagatcaaaagtaggtgtgcggcactgtcaggacaagtctctaggactggggcattggcaaacaaaaggggcaatgtctgacccgagatgatgttctacttaatgcatctcatttcccccaaaacctgtcacctgcagacagaggcttggacaagtagctcagatgtactcttttccccaggaactgcaggccgacaaggacagaaaagctgcaatgactgctcctttctcaagggatgaaaaaacaggctgtttcttggatgctgcacttcacaaatgtactaattgcccccaaaaaagcaaagagtagattttcctgcctagatgcatcacttggcattgactacaccatggaaagcaagagtctgtctatgtgggctggattcctgaactacagcttagaagggaagggcgtagaatatcatcattaactggctcacaaggaatagtcatcttgggcgaacacatgctaatacgtttcacagaatgaggggtgacagcctagaatccaaaatgtgatgtttggaacatttctcgccaaaccttactatgaaagcctgcaaccagtgagaggagaactgcaaagacggcagcagagaaacagcaaacagcacaaaagagataatttaccaagagactttccctcctttcagaggcaaccaagccagaaggagatgacagaagttcacgtgtacagagaacagaagggctaaaaccagaagaaggtgagctaatcatgaaagcaatttatcccatttttgttgttcaataacactggccaacctgctagggtcagatgtcttcttcagaaaggcagcatctctgaacctgggataaaggacacttgaactgaatgcatgagcagaaggacccaatggagaagcataattgaaatcatccttggactgcttaagaatttcttgaaaacttccaaagaaagaaggttatctggatctgcagctatatggctgtataactatcttctacctggctcctcctggaagaggtctttgtctgcttgggagctggggctgttgagcggcacagcccaggcacaaccatgccaggctgggcctctaggccaagctcagtgaggggtgcagacaatcatccaaccagcaatggaactccttggagatgggggcccaaagggcaagacatttaaacaggagtcactgggagatactctgctgctcaacgaacaccacagcaagtgtgagagctccttgcccaagactgagcagctcttcctctcccaccgtgcgttcacaggcagcagcagcacggcgggagggagcccaggaaaggaagcgttgatgaggtaccaaaagaagaactgacatctttgggttcttaaaacaaaaactcaaattgaggaagcgagagaatgaaaaagggaaagaattaaatctgaatcaatggacagaaatatgtggcttactaacccacccccattttgcatacaattttatacaaaaaaggaaaaaaaaaacaccccaactcattgcaatgcagtccaaatgtttgcaaccaaagatgtatgaaaatatttcaattgaaactgctttttttttttttaaaaaaaacaaagcttttgatcattcccttgtcaacataattggcagatctactctcaaacacacttaagagtattccacacaacatgttcggaattcagatttattgatttccatcgtattgactttaaaaatggtatgaagctgactgcaagaaagggaactggtaattttaagttaaaattaagctaatggtgaaagtacatcacctctggcttcagtcaccacatcacctcagattgaatatagattttttatgaacaaagttccagaactctgaaatccagggatgctgcaggcctctcccggcaatgtccttcactttgggtcagtctcctgggccagaggtgaaagtgctttcaaaaatactgccatttccccagcacagtgtctttgattgcatccacatattgagttggaacccagtacacccagtagtaagaggcttccgtggggcccaactgaaacgccatcatgtggtagtcttcatgtccttcgataggttcactgaccacattttttatggagcccatgggcaatttctcagtccgctagtgctggtcagaaacaggtgatttaggcatgttcggttccctccaggaatctttagtgccaatccacagctggtcttgttctagtttaaaggtgagtctcacttttcctccagatttattgtacatgccggacagcggtaccgttggcaggcgctcctgggcccccttaacagatggcatcacatcttcaggttttcctttatccaacactttcctgtgttgtttctgcctgcagagaggctccttcttgttctcttcggcctttgcatcctgctgcgcagcatctttgggtgtgtttactgctaaaacatcattgatggtggagccaaccaccatgatcttggccccactggtcacttttatttctctcaatgttttatcctcggggacgagtcccttatacatgactttctgcatggcaggcgggagacctgtaatcgagtggatcttctgtttcagctcggagcctgtgctgtccagggggaacttcacgtcatgcttggtcttattccagatgatcttcaagtccaccagctccctgcccgcgccgccgcccgcgtcttcgccgttgctgaccgaggcctgggctgcggggtccccagggggctgggccggggccggctgcaggctgcctcgtgcggcgccggagtcctcggccgccgcccccgccgcggcttcagcctccaggcagttgacgggccgcgcgggagcctcagtagccacagtctcggcctccgtgtccatgccaggttcctccatgccatccggggccccggccgccgccatgatgattgtgtacaacacccaccgctcccgcagaggccgctgggaagaggcgagctggctgagattggcccccgcagcagcccctaatctctcacagcccggccggaaacaggtggaggtttctatggagacccgcctcctccgctcccaggtccggcccctgccacgctttcgctttcccaagct

SEQ ID NO: 19187 - RNA, 4873 nt, Homo sapiens
  source 1..4873: mol_type = other RNA
tgtcttctctcctcccaaacaggcatttgatttgaaaacagaaaccagaacagagcatacaccacaaggaaacatggtacttacaaatattgtcaaataattcagcagaactctttaagaaaaaaaaaaggttcttagaaattgagaaagcagtagaaccacccagcctggcagatcaatctaccagatgttctgcatgcgagagggctcccaaccacctgtaacttcagaaaggccgccaggcactattacgaaggaaacaggtgcagatcctaactggagatgactttatcacaaagccttaagacaaagggaccatcctcttccaagacaacaggtgtgaacagaggcaaggagcgagaggagagggctccctcagcagatgggtggaaagcaagcctgcccttgcacggcccttggcacactcaatctaccccctttcccttctctgcccctggcaaagaaaggctgggcaagtgcaagagcccagaatggctcctccaggcacatggttaaagtaagagtaagaggaaaacaagccccttctgggtgaaatatggcaacttttctgagacatggcaacgaggcagagttaatctctttggccctcatcaggtaaagcagcaactaaggagcctactcagggccttacgtgggccccttctatgtccacaagaaagtgcatccttagctcagttcaacatttaaaaagagctaacgctacttgcaaaaggcccaccatggattcaaacacttaataccaaagaggtccagcaactcgcgagtctgtctgtgttctgtgatctgaagcagagctaaggggggcctggctcacagggtcacgctcttctgccaaggcgcctcagggagggaaaaaaaggcatgatgatgtctgtgagccagaacctgcaggaggaccaccggtagagattctagaagacaaagaagccctcaggaggctctgagaggtgtccaatgtctaagagacggccaccccctccatctctagcttcgagtcaacgctgttacagtcactctccggaaaccagctcttcctttatccacctgcacggcccctgccacagtgagggaaagatctggtccctctgacagtaaggaaattgtatagaaattatcctgaggaaaaaaaaaaccactgtgacgctacctaaaagaaagagtatttcaatttgcttacacagatttagtcagtacactccagactgtaagaaatgtatgaagagactgcttacggaactcaaagactaaacagtgaatactactgtggcccagacacggatcgaaaacacttctcccagtggcttctggtgctatgtctgctctcccgagagcgtccagcaaggtcttccatgcagacagggtgaggagccacagagctcaagattgttgaagctgatttagtgagctctgtaaagcaatactcaaacagctccgtacgaaaaggtgtcatttacattattatttatatatagtatctcgaagtaaggaaaaaagcaccattttactgaaaataaaaaggctcacgcaggctttggtcctcctgaaatgacaccagcctgagtgagaagcagttggcccttggggagcggggagatgatggaacgctgtcaccggcaagaagggaggccaagtggcccggcaagccacaagaatggggcaataaggggagcaggtggaggggcctcggagagcagccaggctagtctggggatggagccacctgctctgagagatcaaaagtaggtgtgcggcactgtcaggacaagtctctaggactggggcattggcaaacaaaaggggcaatgtctgacccgagatgatgttctacttaatgcatctcatttcccccaaaacctgtcacctgcagacagaggcttggacaagtagctcagatgtactcttttccccaggaactgcaggccgacaaggacagaaaagctgcaatgactgctcctttctcaagggatgaaaaaacaggctgtttcttggatgctgcacttcacaaatgtactaattgcccccaaaaaagcaaagagtagattttcctgcctagatgcatcacttggcattgactacaccatggaaagcaagagtctgtctatgtgggctggattcctgaactacagcttagaagggaagggcgtagaatatcatcattaactggctcacaaggaatagtcatcttgggcgaacacatgctaatacgtttcacagaatgaggggtgacagcctagaatccaaaatgtgatgtttggaacatttctcgccaaaccttactatgaaagcctgcaaccagtgagaggagaactgcaaagacggcagcagagaaacagcaaacagcacaaaagagataatttaccaagagactttccctcctttcagaggcaaccaagccagaaggagatgacagaagttcacgtgtacagagaacagaagggctaaaaccagaagaaggtgagctaatcatgaaagcaatttatcccatttttgttgttcaataacactggccaacctgctagggtcagatgtcttcttcagaaaggcagcatctctgaacctgggataaaggacacttgaactgaatgcatgagcagaaggacccaatggagaagcataattgaaatcatccttggactgcttaagaatttcttgaaaacttccaaagaaagaaggttatctggatctgcagctatatggctgtataactatcttctacctggctcctcctggaagaggtctttgtctgcttgggagctggggctgttgagcggcacagcccaggcacaaccatgccaggctgggcctctaggccaagctcagtgaggggtgcagacaatcatccaaccagcaatggaactccttggagatgggggcccaaagggcaagacatttaaacaggagtcactgggagatactctgctgctcaacgaacaccacagcaagtgtgagagctccttgcccaagactgagcagctcttcctctcccaccgtgcgttcacaggcagcagcagcacggcgggagggagcccaggaaaggaagcgttgatgaggtaccaaaagaagaactgacatctttgggttcttaaaacaaaaactcaaattgaggaagcgagagaatgaaaaagggaaagaattaaatctgaatcaatggacagaaatatgtggcttactaacccacccccattttgcatacaattttatacaaaaaaggaaaaaaaaaacaccccaactcattgcaatgcagtccaaatgtttgcaaccaaagatgtatgaaaatatttcaattgaaactgctttttttttttttaaaaaaaacaaagcttttgatcattcccttgtcaacataattggcagatctactctcaaacacacttaagagtattccacacaacatgttcggaattcagatttattgatttccatcgtattgactttaaaaatggtatgaagctgactgcaagaaagggaactggtaattttaagttaaaattaagctaatggtgaaagtacatcacctctggcttcagtcaccacatcacctcagattgaatatagattttttatgaacaaagttccagaactctgaaatccagggatgctgcaggcctctcccggcaatgtccttcactttgggtcagtctcctgggccagaggtgaaagtgctttcaaaaatactgccatttccccagcacagtgtctttgattgcatccacatattgagttggaacccagtacacccagtagtaagaggcttccgtggggcccaactgaaacgccatcatgtggtagtcttcatgtccttcgataggttcactgaccacattttttatggagcccatgggcaatttctcagtccgctctcgaacactgaatacctacagtgctggtcagaaacaggtgatttaggcatgttcggttccctccaggaatctttagtgccaatccacagctggtcttgttctagtttaaaggtgagtctcacttttcctccagatttattgtacatgccggacagcggtaccgttggcaggcgctcctgggcccccttaacagatggcatcacatcttcaggttttcctttatccaacactttcctgtgttgtttctgcctgcagagaggctccttcttgttctcttcggcctttgcatcctgctgcgcagcatctttgggtgtgtttactgctaaaacatcattgatggtggagccaaccaccatgatcttggccccactggtcacttttatttctctcaatgttttatcctcggggacgagtcccttatacatgactttctgcatggcaggcgggagacctgtaatcgagtggatcttctgtttcagctcggagcctgtgctgtccagggggaacttcacgtcatgcttggtcttattccagatgatcttcaagtccaccagctccctgcccgcgccgccgcccgcgtcttcgccgttgctgaccgaggcctgggctgcggggtccccagggggctgggccggggccggctgcaggctgcctcgtgcggcgccggagtcctcggccgccgcccccgccgcggcttcagcctccaggcagttgacgggccgcgcgggagcctcagtagccacagtctcggcctccgtgtccatgccaggttcctccatgccatccggggccccggccgccgccatgatgattgtgtacaacacccaccgctcccgcagaggccgctgggaagaggcgagctggctgagattggcccccgcagcagcccctaatctctcacagcccggccggaaacaggtggaggtttctatggagacccgcctcctccgctcccaggtccggcccctgccacgctttcgctttcccaagct

SEQ ID NO: 19188 - RNA, 4892 nt, Homo sapiens
  source 1..4892: mol_type = other RNA
tgtcttctctcctcccaaacaggcatttgatttgaaaacagaaaccagaacagagcatacaccacaaggaaacatggtacttacaaatattgtcaaataattcagcagaactctttaagaaaaaaaaaaggttcttagaaattgagaaagcagtagaaccacccagcctggcagatcaatctaccagatgttctgcatgcgagagggctcccaaccacctgtaacttcagaaaggccgccaggcactattacgaaggaaacaggtgcagatcctaactggagatgactttatcacaaagccttaagacaaagggaccatcctcttccaagacaacaggtgtgaacagaggcaaggagcgagaggagagggctccctcagcagatgggtggaaagcaagcctgcccttgcacggcccttggcacactcaatctaccccctttcccttctctgcccctggcaaagaaaggctgggcaagtgcaagagcccagaatggctcctccaggcacatggttaaagtaagagtaagaggaaaacaagccccttctgggtgaaatatggcaacttttctgagacatggcaacgaggcagagttaatctctttggccctcatcaggtaaagcagcaactaaggagcctactcagggccttacgtgggccccttctatgtccacaagaaagtgcatccttagctcagttcaacatttaaaaagagctaacgctacttgcaaaaggcccaccatggattcaaacacttaataccaaagaggtccagcaactcgcgagtctgtctgtgttctgtgatctgaagcagagctaaggggggcctggctcacagggtcacgctcttctgccaaggcgcctcagggagggaaaaaaaggcatgatgatgtctgtgagccagaacctgcaggaggaccaccggtagagattctagaagacaaagaagccctcaggaggctctgagaggtgtccaatgtctaagagacggccaccccctccatctctagcttcgagtcaacgctgttacagtcactctccggaaaccagctcttcctttatccacctgcacggcccctgccacagtgagggaaagatctggtccctctgacagtaaggaaattgtatagaaattatcctgaggaaaaaaaaaaccactgtgacgctacctaaaagaaagagtatttcaatttgcttacacagatttagtcagtacactccagactgtaagaaatgtatgaagagactgcttacggaactcaaagactaaacagtgaatactactgtggcccagacacggatcgaaaacacttctcccagtggcttctggtgctatgtctgctctcccgagagcgtccagcaaggtcttccatgcagacagggtgaggagccacagagctcaagattgttgaagctgatttagtgagctctgtaaagcaatactcaaacagctccgtacgaaaaggtgtcatttacattattatttatatatagtatctcgaagtaaggaaaaaagcaccattttactgaaaataaaaaggctcacgcaggctttggtcctcctgaaatgacaccagcctgagtgagaagcagttggcccttggggagcggggagatgatggaacgctgtcaccggcaagaagggaggccaagtggcccggcaagccacaagaatggggcaataaggggagcaggtggaggggcctcggagagcagccaggctagtctggggatggagccacctgctctgagagatcaaaagtaggtgtgcggcactgtcaggacaagtctctaggactggggcattggcaaacaaaaggggcaatgtctgacccgagatgatgttctacttaatgcatctcatttcccccaaaacctgtcacctgcagacagaggcttggacaagtagctcagatgtactcttttccccaggaactgcaggccgacaaggacagaaaagctgcaatgactgctcctttctcaagggatgaaaaaacaggctgtttcttggatgctgcacttcacaaatgtactaattgcccccaaaaaagcaaagagtagattttcctgcctagatgcatcacttggcattgactacaccatggaaagcaagagtctgtctatgtgggctggattcctgaactacagcttagaagggaagggcgtagaatatcatcattaactggctcacaaggaatagtcatcttgggcgaacacatgctaatacgtttcacagaatgaggggtgacagcctagaatccaaaatgtgatgtttggaacatttctcgccaaaccttactatgaaagcctgcaaccagtgagaggagaactgcaaagacggcagcagagaaacagcaaacagcacaaaagagataatttaccaagagactttccctcctttcagaggcaaccaagccagaaggagatgacagaagttcacgtgtacagagaacagaagggctaaaaccagaagaaggtgagctaatcatgaaagcaatttatcccatttttgttgttcaataacactggccaacctgctagggtcagatgtcttcttcagaaaggcagcatctctgaacctgggataaaggacacttgaactgaatgcatgagcagaaggacccaatggagaagcataattgaaatcatccttggactgcttaagaatttcttgaaaacttccaaagaaagaaggttatctggatctgcagctatatggctgtataactatcttctacctggctcctcctggaagaggtctttgtctgcttgggagctggggctgttgagcggcacagcccaggcacaaccatgccaggctgggcctctaggccaagctcagtgaggggtgcagacaatcatccaaccagcaatggaactccttggagatgggggcccaaagggcaagacatttaaacaggagtcactgggagatactctgctgctcaacgaacaccacagcaagtgtgagagctccttgcccaagactgagcagctcttcctctcccaccgtgcgttcacaggcagcagcagcacggcgggagggagcccaggaaaggaagcgttgatgaggtaccaaaagaagaactgacatctttgggttcttaaaacaaaaactcaaattgaggaagcgagagaatgaaaaagggaaagaattaaatctgaatcaatggacagaaatatgtggcttactaacccacccccattttgcatacaattttatacaaaaaaggaaaaaaaaaacaccccaactcattgcaatgcagtccaaatgtttgcaaccaaagatgtatgaaaatatttcaattgaaactgctttttttttttttaaaaaaaacaaagcttttgatcattcccttgtcaacataattggcagatctactctcaaacacacttaagagtattccacacaacatgttcggaattcagatttattgatttccatcgtattgactttaaaaatggtatgaagctgactgcaagaaagggaactggtaattttaagttaaaattaagctaatggtgaaagtacatcacctctggcttcagtcaccacatcacctcagattgaatatagattttttatgaacaaagttccagaactctgaaatccagggatgctgcaggcctctcccggcaatgtccttcactttgggtcagtctcctgggccagaggtgaaagtgctttcaaaaatactgccatttccccagcacagtgtctttgattgcatccacatattgagttggaacccagtacacccagtagtaagaggcttccgtggggcccaactgaaacgccatcatgtggtagtcttcatgtccttcgataggttcactgaccacattttttatggagcccatgggcaatttctcagtccgctctttagtgccaatccacagctggtcttgttctagtttaaaggtgagtctcacttttcctccagatttattgtacatgccggacagcggtaccgttggcaggcgctcctgggcccccttaacagatggcatcacatcttcaggttttcctttatccaacactttcctgtgttgccgccagatgagacaaagttgcaaatctcaggtagttgtcacctccactctgcggcacccaactgctgccataaatttccatcatgggcctttctgcctgcagagaggctccttcttgttctcttcggcctttgcatcctgctgcgcagcatctttgggtgtgtttactgctaaaacatcattgatggtggagccaaccaccatgatcttggccccactggtcacttttatttctctcaatgttttatcctcggggacgagtcccttatacatgactttctgcatggcaggcgggagacctgtaatcgagtggatcttctgtttcagctcggagcctgtgctgtccagggggaacttcacgtcatgcttggtcttattccagatgatcttcaagtccaccagctccctgcccgcgccgccgcccgcgtcttcgccgttgctgaccgaggcctgggctgcggggtccccagggggctgggccggggccggctgcaggctgcctcgtgcggcgccggagtcctcggccgccgcccccgccgcggcttcagcctccaggcagttgacgggccgcgcgggagcctcagtagccacagtctcggcctccgtgtccatgccaggttcctccatgccatccggggccccggccgccgccatgatgattgtgtacaacacccaccgctcccgcagaggccgctgggaagaggcgagctggctgagattggcccccgcagcagcccctaatctctcacagcccggccggaaacaggtggaggtttctatggagacccgcctcctccgctcccaggtccggcccctgccacgctttcgctttcccaagct

SEQ ID NO: 19189 - RNA, 4632 nt, Homo sapiens
  source 1..4632: mol_type = other RNA
tgtcttctctcctcccaaacaggcatttgatttgaaaacagaaaccagaacagagcatacaccacaaggaaacatggtacttacaaatattgtcaaataattcagcagaactctttaagaaaaaaaaaaggttcttagaaattgagaaagcagtagaaccacccagcctggcagatcaatctaccagatgttctgcatgcgagagggctcccaaccacctgtaacttcagaaaggccgccaggcactattacgaaggaaacaggtgcagatcctaactggagatgactttatcacaaagccttaagacaaagggaccatcctcttccaagacaacaggtgtgaacagaggcaaggagcgagaggagagggctccctcagcagatgggtggaaagcaagcctgcccttgcacggcccttggcacactcaatctaccccctttcccttctctgcccctggcaaagaaaggctgggcaagtgcaagagcccagaatggctcctccaggcacatggttaaagtaagagtaagaggaaaacaagccccttctgggtgaaatatggcaacttttctgagacatggcaacgaggcagagttaatctctttggccctcatcaggtaaagcagcaactaaggagcctactcagggccttacgtgggccccttctatgtccacaagaaagtgcatccttagctcagttcaacatttaaaaagagctaacgctacttgcaaaaggcccaccatggattcaaacacttaataccaaagaggtccagcaactcgcgagtctgtctgtgttctgtgatctgaagcagagctaaggggggcctggctcacagggtcacgctcttctgccaaggcgcctcagggagggaaaaaaaggcatgatgatgtctgtgagccagaacctgcaggaggaccaccggtagagattctagaagacaaagaagccctcaggaggctctgagaggtgtccaatgtctaagagacggccaccccctccatctctagcttcgagtcaacgctgttacagtcactctccggaaaccagctcttcctttatccacctgcacggcccctgccacagtgagggaaagatctggtccctctgacagtaaggaaattgtatagaaattatcctgaggaaaaaaaaaaccactgtgacgctacctaaaagaaagagtatttcaatttgcttacacagatttagtcagtacactccagactgtaagaaatgtatgaagagactgcttacggaactcaaagactaaacagtgaatactactgtggcccagacacggatcgaaaacacttctcccagtggcttctggtgctatgtctgctctcccgagagcgtccagcaaggtcttccatgcagacagggtgaggagccacagagctcaagattgttgaagctgatttagtgagctctgtaaagcaatactcaaacagctccgtacgaaaaggtgtcatttacattattatttatatatagtatctcgaagtaaggaaaaaagcaccattttactgaaaataaaaaggctcacgcaggctttggtcctcctgaaatgacaccagcctgagtgagaagcagttggcccttggggagcggggagatgatggaacgctgtcaccggcaagaagggaggccaagtggcccggcaagccacaagaatggggcaataaggggagcaggtggaggggcctcggagagcagccaggctagtctggggatggagccacctgctctgagagatcaaaagtaggtgtgcggcactgtcaggacaagtctctaggactggggcattggcaaacaaaaggggcaatgtctgacccgagatgatgttctacttaatgcatctcatttcccccaaaacctgtcacctgcagacagaggcttggacaagtagctcagatgtactcttttccccaggaactgcaggccgacaaggacagaaaagctgcaatgactgctcctttctcaagggatgaaaaaacaggctgtttcttggatgctgcacttcacaaatgtactaattgcccccaaaaaagcaaagagtagattttcctgcctagatgcatcacttggcattgactacaccatggaaagcaagagtctgtctatgtgggctggattcctgaactacagcttagaagggaagggcgtagaatatcatcattaactggctcacaaggaatagtcatcttgggcgaacacatgctaatacgtttcacagaatgaggggtgacagcctagaatccaaaatgtgatgtttggaacatttctcgccaaaccttactatgaaagcctgcaaccagtgagaggagaactgcaaagacggcagcagagaaacagcaaacagcacaaaagagataatttaccaagagactttccctcctttcagaggcaaccaagccagaaggagatgacagaagttcacgtgtacagagaacagaagggctaaaaccagaagaaggtgagctaatcatgaaagcaatttatcccatttttgttgttcaataacactggccaacctgctagggtcagatgtcttcttcagaaaggcagcatctctgaacctgggataaaggacacttgaactgaatgcatgagcagaaggacccaatggagaagcataattgaaatcatccttggactgcttaagaatttcttgaaaacttccaaagaaagaaggttatctggatctgcagctatatggctgtataactatcttctacctggctcctcctggaagaggtctttgtctgcttgggagctggggctgttgagcggcacagcccaggcacaaccatgccaggctgggcctctaggccaagctcagtgaggggtgcagacaatcatccaaccagcaatggaactccttggagatgggggcccaaagggcaagacatttaaacaggagtcactgggagatactctgctgctcaacgaacaccacagcaagtgtgagagctccttgcccaagactgagcagctcttcctctcccaccgtgcgttcacaggcagcagcagcacggcgggagggagcccaggaaaggaagcgttgatgaggtaccaaaagaagaactgacatctttgggttcttaaaacaaaaactcaaattgaggaagcgagagaatgaaaaagggaaagaattaaatctgaatcaatggacagaaatatgtggcttactaacccacccccattttgcatacaattttatacaaaaaaggaaaaaaaaaacaccccaactcattgcaatgcagtccaaatgtttgcaaccaaagatgtatgaaaatatttcaattgaaactgctttttttttttttaaaaaaaacaaagcttttgatcattcccttgtcaacataattggcagatctactctcaaacacacttaagagtattccacacaacatgttcggaattcagatttattgatttccatcgtattgactttaaaaatggtatgaagctgactgcaagaaagggaactggtaattttaagttaaaattaagctaatggtgaaagtacatcacctctggcttcagtcaccacatcacctcagattgaatatagattttttatgaacaaagttccagaactctgaaatccagggatgctgcaggcctctcccggcaatgtccttcactttgggtcagtctcctgggccagaggtgaaagtgctttcaaaaatactgccatttccccagcacagtgtctttgattgcatccacatattgagttggaacccagtacacccagtagtaagaggcttccgtggggcccaactgaaacgccatcatgtggtagtcttcatgtccttcgataggttcactgaccacattttttatggagcccatgggcaatttctcagtccgctctttagtgccaatccacagctggtcttgttctagtttaaaggtgagtctcacttttcctccagatttattgtacatgccggacagcggtaccgttggcaggcgctcctgggcccccttaacagatggcatcacatcttcaggttttcctttatccaacactttcctgtgttgtttctgcctgcagagaggctccttcttgttctcttcggcctttgcatcctgctgcgcagcatctttgggtgtgtttactgctaaaacatcattgatggtggagccaaccaccatgatcttggccccactggtcacttttatttctctcaatgttttatcctcggggacgagtcccttatacatgactttctgcatggcaggcgggagacctgtaatcgagtggatcttctgtttcagctcggagcctgtgctgtccagggggaacttcacgtcatgcttggtcttattccagatgatcttcaagtccaccagctccctgcccgcgccgccgcccgcgtcttcgccgttgctgaccgaggcctgggctgcggggtccccagggggctgggccggggccggctgcaggctgcctcgtgcggcgccggagtcctcggccgccgcccccgccgcggcttcagcctccaggcagttgacgggccgcgcgggagcctcagtagccacagtctcggcctccgtgtccatgccaggttcctccatgccatccggggccccggccgccgccatgatgattgtgtacaac

SEQ ID NO: 19190 - RNA, 4719 nt, Homo sapiens
  source 1..4719: mol_type = other RNA
tgtcttctctcctcccaaacaggcatttgatttgaaaacagaaaccagaacagagcatacaccacaaggaaacatggtacttacaaatattgtcaaataattcagcagaactctttaagaaaaaaaaaaggttcttagaaattgagaaagcagtagaaccacccagcctggcagatcaatctaccagatgttctgcatgcgagagggctcccaaccacctgtaacttcagaaaggccgccaggcactattacgaaggaaacaggtgcagatcctaactggagatgactttatcacaaagccttaagacaaagggaccatcctcttccaagacaacaggtgtgaacagaggcaaggagcgagaggagagggctccctcagcagatgggtggaaagcaagcctgcccttgcacggcccttggcacactcaatctaccccctttcccttctctgcccctggcaaagaaaggctgggcaagtgcaagagcccagaatggctcctccaggcacatggttaaagtaagagtaagaggaaaacaagccccttctgggtgaaatatggcaacttttctgagacatggcaacgaggcagagttaatctctttggccctcatcaggtaaagcagcaactaaggagcctactcagggccttacgtgggccccttctatgtccacaagaaagtgcatccttagctcagttcaacatttaaaaagagctaacgctacttgcaaaaggcccaccatggattcaaacacttaataccaaagaggtccagcaactcgcgagtctgtctgtgttctgtgatctgaagcagagctaaggggggcctggctcacagggtcacgctcttctgccaaggcgcctcagggagggaaaaaaaggcatgatgatgtctgtgagccagaacctgcaggaggaccaccggtagagattctagaagacaaagaagccctcaggaggctctgagaggtgtccaatgtctaagagacggccaccccctccatctctagcttcgagtcaacgctgttacagtcactctccggaaaccagctcttcctttatccacctgcacggcccctgccacagtgagggaaagatctggtccctctgacagtaaggaaattgtatagaaattatcctgaggaaaaaaaaaaccactgtgacgctacctaaaagaaagagtatttcaatttgcttacacagatttagtcagtacactccagactgtaagaaatgtatgaagagactgcttacggaactcaaagactaaacagtgaatactactgtggcccagacacggatcgaaaacacttctcccagtggcttctggtgctatgtctgctctcccgagagcgtccagcaaggtcttccatgcagacagggtgaggagccacagagctcaagattgttgaagctgatttagtgagctctgtaaagcaatactcaaacagctccgtacgaaaaggtgtcatttacattattatttatatatagtatctcgaagtaaggaaaaaagcaccattttactgaaaataaaaaggctcacgcaggctttggtcctcctgaaatgacaccagcctgagtgagaagcagttggcccttggggagcggggagatgatggaacgctgtcaccggcaagaagggaggccaagtggcccggcaagccacaagaatggggcaataaggggagcaggtggaggggcctcggagagcagccaggctagtctggggatggagccacctgctctgagagatcaaaagtaggtgtgcggcactgtcaggacaagtctctaggactggggcattggcaaacaaaaggggcaatgtctgacccgagatgatgttctacttaatgcatctcatttcccccaaaacctgtcacctgcagacagaggcttggacaagtagctcagatgtactcttttccccaggaactgcaggccgacaaggacagaaaagctgcaatgactgctcctttctcaagggatgaaaaaacaggctgtttcttggatgctgcacttcacaaatgtactaattgcccccaaaaaagcaaagagtagattttcctgcctagatgcatcacttggcattgactacaccatggaaagcaagagtctgtctatgtgggctggattcctgaactacagcttagaagggaagggcgtagaatatcatcattaactggctcacaaggaatagtcatcttgggcgaacacatgctaatacgtttcacagaatgaggggtgacagcctagaatccaaaatgtgatgtttggaacatttctcgccaaaccttactatgaaagcctgcaaccagtgagaggagaactgcaaagacggcagcagagaaacagcaaacagcacaaaagagataatttaccaagagactttccctcctttcagaggcaaccaagccagaaggagatgacagaagttcacgtgtacagagaacagaagggctaaaaccagaagaaggtgagctaatcatgaaagcaatttatcccatttttgttgttcaataacactggccaacctgctagggtcagatgtcttcttcagaaaggcagcatctctgaacctgggataaaggacacttgaactgaatgcatgagcagaaggacccaatggagaagcataattgaaatcatccttggactgcttaagaatttcttgaaaacttccaaagaaagaaggttatctggatctgcagctatatggctgtataactatcttctacctggctcctcctggaagaggtctttgtctgcttgggagctggggctgttgagcggcacagcccaggcacaaccatgccaggctgggcctctaggccaagctcagtgaggggtgcagacaatcatccaaccagcaatggaactccttggagatgggggcccaaagggcaagacatttaaacaggagtcactgggagatactctgctgctcaacgaacaccacagcaagtgtgagagctccttgcccaagactgagcagctcttcctctcccaccgtgcgttcacaggcagcagcagcacggcgggagggagcccaggaaaggaagcgttgatgaggtaccaaaagaagaactgacatctttgggttcttaaaacaaaaactcaaattgaggaagcgagagaatgaaaaagggaaagaattaaatctgaatcaatggacagaaatatgtggcttactaacccacccccattttgcatacaattttatacaaaaaaggaaaaaaaaaacaccccaactcattgcaatgcagtccaaatgtttgcaaccaaagatgtatgaaaatatttcaattgaaactgctttttttttttttaaaaaaaacaaagcttttgatcattcccttgtcaacataattggcagatctactctcaaacacacttaagagtattccacacaacatgttcggaattcagatttattgatttccatcgtattgactttaaaaatggtatgaagctgactgcaagaaagggaactggtaattttaagttaaaattaagctaatggtgaaagtacatcacctctggcttcagtcaccacatcacctcagattgaatatagattttttatgaacaaagttccagaactctgaaatccagggatgctgcaggcctctcccggcaatgtccttcactttgggtcagtctcctgggccagaggtgaaagtgctttcaaaaatactgccatttccccagcacagtgtctttgattgcatccacatattgagttggaacccagtacacccagtagtaagaggcttccgtggggcccaactgaaacgcctttagtgccaatccacagctggtcttgttctagtttaaaggtgagtctcacttttcctccagatttattgtacatgccggacagcggtaccgttggcaggcgctcctgggcccccttaacagatggcatcacatcttcaggttttcctttatccaacactttcctgtgttgtttctgcctgcagagaggctccttcttgttctcttcggcctttgcatcctgctgcgcagcatctttgggtgtgtttactgctaaaacatcattgatggtggagccaaccaccatgatcttggccccactggtcacttttatttctctcaatgttttatcctcggggacgagtcccttatacatgactttctgcatggcaggcgggagacctgtaatcgagtggatcttctgtttcagctcggagcctgtgctgtccagggggaacttcacgtcatgcttggtcttattccagatgatcttcaagtccaccagctccctgcccgcgccgccgcccgcgtcttcgccgttgctgaccgaggcctgggctgcggggtccccagggggctgggccggggccggctgcaggctgcctcgtgcggcgccggagtcctcggccgccgcccccgccgcggcttcagcctccaggcagttgacgggccgcgcgggagcctcagtagccacagtctcggcctccgtgtccatgccaggttcctccatgccatccggggccccggccgccgccatgatgattgtgtacaacacccaccgctcccgcagaggccgctgggaagaggcgagctggctgagattggcccccgcagcagcccctaatctctcacagcccggccggaaacaggtggaggtttctatggagacccgcctcctccgctcccaggtccggcccctgccacgctttcgctttcccaagct

SEQ ID NO: 19191 - RNA, 3956 nt, Homo sapiens
  source 1..3956: mol_type = other RNA
tgtcttctctcctcccaaacaggtcccgccacacctccttgccttggtccatttcctccgtcctcattgagtcctttgcttccttttgttcctgagctgcctttcatgttacctccacacttggaataaaaatgcctcccacttcccaagcacaaagagctgcccactcccctgattaacatcctccaggggggtttttctcctgaaaagcccatctggcctcccctcctcctcacgcccagcacatccactgcagagggctgttccagagattattgtgcccaatgtgccgcctgccctgccctgccgactctgcatgaagggtttcatctctggcttccttctaaaacccaactgactgactgactcactccctcactcactcaaaagagctaccgttccatcatcttgctttatcctcccaaatacgccagttacactactaatgatagtaatattccagtgagtcattgaaatatcttattttgcagtacctacagtttgcttgttgaatttacatgggtgtgcacggagctttgcattttaaaattaacagaagacgtcatttcttctgtttaagcagtggaaccgtcgaaataatcctctaaagtatttaggttcccagattttcacaaccaagcaaaggagaaagagggatttatttctagaatcatggaatgataacgctggaatggctctttgcactcagtgggtctattttacagacactgaaactaaggccccaagaagtcaacacacttctcaaagtcatagactaagttcatatggctattttaaatatgtaataataaggaataagacgctatttatctcacaggcactgcagggagggaggtgattaaacagaacgctcaaagtagaggaacttgtagctagcaaaactcctgaaaatacgacagtcctgggagttgcagtggagaggaagcagaggctatgctgtagaggaaggtcacaggagggacgtggaaaggccccagggctgtgcttctcacattcaggtgactcacctgtggtcttgttgcaatgcagattctgatttaccaggtgagtcagggcccaagagtctgcatttctaataactcccaggcgatgctgacattactcttccatgggcctcagtttgagtagcaaagatttagatattctgtttcaggagccaggaagttaaaggagggctatatatacctggacttggaaccagaccccatgccagggtcccaggcctgtcactgattggctctgttgtcagtgggtggagttacacctgtctctgagcctcagtttactcatctgtaaaccaaaggagttgtccagggtgacctccatgactgctgaggtccctttaagctggaatgtcccatgactcagagccctgcagtggccagcaccccaggaggaagggaggggacacggaaagctgttgtgagagatggacagacccacaagtcatcacctctcttgatgcccttggctgggtaggggtgggcctggaattttcactaacatgctccagaccactctctccatgctttgactgtattcttgaaccatgcatgtggtcccaagttttccatcctcttcatgccacttggtcctttactccccactacaccacaacctctgtgttccttgccctcaggatgaccttctcctcaccctggttatgccatcatccttccccttccatggccctgtatataagaactgattataatcacagtatattctgtgttttagcagagcatgtcaacattgctgtacgccatcatcgtgccagctcaacacaaactctaaagaaagtgacattggtgcagtaagagaaagatagacttccccttacctgaaaggaagtggtatcctggctttagggaggagttcatcaattctacagaggagatttcacatctttacacaggtacacaaactacacaaagagggacattcaggaggggaaacactgtggtcgctagaatccctatgtgacaccatggtctctctagagtgtctgtgtgacaccatgttctctctagagtgtctgtgtgacaccgtgttctctctagagtgtctgtgtgacactgtggtctctctggagtgcctgtgtgacgctgtggtctctctagagtgcctgtgtgacgctgtggtctctctagagtgcctgtgtgatgccgtggtctctctagagcgtgtgtgtgacactgtggtctctctagaatgcctgtgtgacactgcagtctctctagaatgtctgtgtgacactgtggtctctctagaatgcctgtgtgacgctgtggtctctctagaatgcctgtgtgacactgtggtctctctagcgtgtcttgtgatgctgtggtctctctagagtgtctgtgtgatgctgcggtcgctagctagaatgactatgtgatgctgtggtctctctagaatgcctatgtgaacttaggaattcacactcctaggctcagtgcaggctgagcaccaaagtgtgatctcatcaagtgaaataacccccttctctcaatttctcttcctgtaaggaggaaaatgccactttccacccacaaagctctctagaggaccaagaagacaattctgtgaaggacgtccaccaggagacaggagctacaagacagctttctggagctgtcctcctaagtccccatgccaatcagtgtatagtaatgtcgccaacttcaaaatcacggaaatatgtttgcatcagacaatggcttcaattccaacacatggtacattcccacaagtttggatttccataggaagaataaataacactggcttccttgaatgtcctggatgaaaaccacacatccttccaaatcctgtggaaaaacatctctggctccctccttcccttagaatcagacccttcaaaatcttgtggtatttccccaaataccataattttgagttgtgacatctggtttccagttctcccaggctggggtttcttgttaaagggacatcggaatctcgacatcccgagctgccaccctgaccttgtgcaggagtctcactgccccacttcctggcatccatgcactctagatggttctggcacttcccccagacaaggaagctacatttttttctaggatgtacctttttagaagcctttgtctcttccagaaggtatgtccggcacgatgggactcccccactctcccttgcctcaaacatcacggaacatctagacatcagtgagcgtcccactagaaaaaggcccctgaatcttcaagaagctccaagaggggagttagattgtctggaaattccccgaagttcttcctgctacacccactggagcccaggatttgagaaccaagcccgccggccgcggcatactaggctcggctttctgtttcgaagctcgaggctgtaccggggagagaggatgtggtccatgggaaggggaagtgccactgctccagggagccaagcatggcttcctcagggcctggctcctcaggcagcaggaggtgggcagcactgtgcagcgggtaagagcacacgctgtgatatcagataggcaggtgttggactcccagctctggccaagtgacctctggcaaacccctttcctcccaagcactggcatcctcacaggtataacaggatacagatggtgggcaaatgccgcggccacatcctacacggggagagacgcttcatcaacaacagccatgaacactgtctggcctgttcatcagggcccagcagacccatcacacagacacatggtaaaagcacgaggaatatttcatttcatggtcacaggtaagtgcttaagctggtagtgaaggaggaagcccaaaggctactgaggcggcatcacagtgacggtcaagaacaggccagaggctggctgcagtggctcaagcctgtaatcccagcactttgggaggcccaggcgggcagat

SEQ ID NO: 19192 - RNA, 4125 nt, Homo sapiens
  source 1..4125: mol_type = other RNA
tgtcttgcaggccgtcatgcaggccacactgacggtaacgttgcaggtcgtcttgcagggcttctcgcaagacgacatcctcatcaccaacgacgtgcagctccaggtagcggttctgacgcagggcagggaggtggccctcctggggggtgactctgacaccgaagaactcacacagcgtcagccagaagccaggggtgaactgcaggcctcggtgggcctgggagtgcagagcatttcgctgccagcggccagggcccaggaacagctcagccagctcctgggctgggatggtgtttgcacctacgagagcgggcatctgggtgagcagctgggtgatggctgtcgtgatgctgctgcctgcgatgagggacgaatccaggatgagtcgtagggagcgctggggctggggccgagccacccgcatggcgggtgccggccgcagcgagaggcattgcctcacgcgcagtagcacgaggatggctgccagggctagggtgttcttccagtacaggaggcctcggaagaagtgcagaatgacggccctgatctgggccatgctgaagtgggcgaggaagctgttgaggatctggtcgatgggtatcatggccagcagctcttgccgtaggatctgttcattgagctcatcctgttcttcattctcttcttccccggattccgtcgatggatccctggggaatccccttgaggccagcagcagggtttgcctggcggcagtgttcctctggaaggctctcctccaccggaggtttctcacaggtggcagagctcggccgccgtcttgttctggcagctccatgacgtcaaagttgaagtgggagaagaagaagacccaatgcccggggagaagtacggtgagcctgtcattattcagagaggctagatcctctgtgttgagaaggatcatgatgggctcctcggtgttctccaggtagcggcaccacaccatgaaggcagcccgtattggaagaatcttcatctccgcttgagagtactcaacctcgataggggagatgttgcgggagtagaaagcgcagcaggctctcttgccggtttggtcgtcgatttggatcagggaggcgtgcagggccgtgccggtgacgccggtttccaagtagaatgggttctggggcttggggtggtggaggagaggcgccttgcggaaagccctcttcaggcactcgaaggcctcttgctcctcgactccccagtagaactggtaggagctcagcagctgccgcaccaggggctctgcgatgatgctgaagcgctccacgaagtggcggtaggggaagacgaattcgatgaagtttcgcagagatagcttggagccaggggtagggtaccctgttatgatggtcatgacgttcttgttcagtttcacccctttgggggtgacgacgaagcccaggaattccacggtttggcggtggaactggctcttgtccagggagcagtagacgttgtgatggcggaagcggaccaggacttggcggacgtggtggaggtgctcctcctgactcattgagtagatcaggacttcctggccataagaaagcacaaagaaccctagcatgtcctttaggatgaagtgaatcacgttctgaggtatgatagggtctggggagagcgcaaacggctggtagctcttcatctcttcaagctccaaaccaaacgctgctttccacacatcttcggtgcggtgcccgttcacgctttcctccacaatggtcccacgcagctccagttttgtgaaccactcggctccgtgtaactggtcaaacagttccggaatcatctgtatgtagtcctgtctgttggtcagcatgtcctgcaggtcccagtattcctcctgtagcctggctctttcttgcatcctggcacccacaggttcccaaggcgcggtggagggacactcgtaaaaggtctcgctgtgatcactgtctccagcctgctgaagctcagagggctctgattcagaaagatcatcggatccgtctgagcttggctggtcggaagtctcatcatctgcttccttcgggttaaacacgtcggccaggtctgagtatgggtgtggcagtccgggtagcaggctcatgccgtgcctctctagggcaatgcatggcgggggcgggcggaagcagttcttcaggcagtagggagagtggaaggtgcagcggcctttgatccagtcgacttcgggggcgtggactcggagccagcggatgcctaggaccacagagaagttcggtgaaggtacgatgtcaaattcgatggactcctggtggttctggtggatacacaccaggggctccgtgtagagccagacaggctcgttgccaatcagcgagccgtccacggattggaccggctgtgggtacggcttctcgtagagctcgacgtagtgctcttgggcgaacttctcatccatgaagttgccgtcagctcccgaatccaccagggcctggaccgcgacgctgtggtaggggttcactctcaccatgagcagcaggaagaggtgggcgcgattgatgtccggatggacttcgctgggcaaccagctgctgaccatccacctctctggagcaggtgagtcgatccaggtcaggttccgggggcgggcctcggggggcagcctgagcatagctcttctctctgccagcttctcttctatttgcaggatgagcacaatcagactgtctagggaatccggctgagggacccggaatagatagtgcctgatctcctcgttgagcccctggcacaagtgggcctgcaggacttcatctggccagcccaagatgggtaccaggctctggaactcatcgatgtactcagtggcagagcggccgccctgcctgatggtgaacatggcctcttctgccacacgcagtgcctggcggtactcaaacacttcggacatggcctccaggaaggctgggaagtctccgatcagggggctgttttcctgcagtagagctttggcccattctaatgccaagccggacaggtgattgatgacatagccaactctcagacggtcgttatagaacattcttgggtagctctgtaaggtcagttggcagagtacgatgaactcgtggaattctctgcgatcgccagagaagtgctttggggcgggcagttggcctgcattgatccctttgatcaagatctcttctgctactctctgttgctctttgaggtcttgcattcggaagtacagcgagatgatggacctcaccatggccataagttctgcggttgagtgctcggtctggttttgctcttgaggagtctcctcccttcccgattccttcaggtcagtgtgagcctcttgttcttctcgggctcccgatgggttgactgatgcttctttcatcctatcagatgctccactgagtggatccccccttgcctggtgtgaaccgttgcatgactcctccaggtcttggagtaggtcattgggtggatcctctatttccttacgtgggccactggatggctcctccatgtcttggagtagatcagtgggcagctcttccatttcctggagtgggccactggggggctccttcttttcctgggctgggccgctggctggccctgcctctccccgcactccactgcccgacgtcgcctcggtggtgttggatgagccctcggaggactccatttgttttgatgatggattcttatgctccatcatcgtctcaaatgagtcttcagagggttctatcatttcgtcggatggaaaggagtgtattctgaagattggtaaggttgtgatggcgtccagtcagtagctgggaccgtggagatcagaaccttggctgcaagcgttcaagtggatctcctcccgtcctgtgccactcgatcctcgctgcttgcttccccgggcccagtcccaagcgtgaggctggggatgaagtgatgccggtggcttagtgatgccggtggcttcctgtcctcgaagctcagtcggtcgtctctcagctggtgtgaggctgggccaggatggaaccccagactctccgaggctccccaccacaccctgctgctgaaggctgctcagcgaggctgtgccgagtgctgggggggtgt

SEQ ID NO: 19193 - RNA, 74 nt, Homo sapiens
  source 1..74: mol_type = other RNA
tgtgaccctagaataattacccaacgtctctgagtctcggttttgagagggtgagtaattattctagggtcaca

SEQ ID NO: 19194 - RNA, 772 nt, Homo sapiens
  source 1..772: mol_type = other RNA
tgtgaccctagaataattaccttccaagtgactatttccaaggatctgctgcgtctgaaaaattatagctaaaaagtgctaggcttatataccaaaaatgatgggtttacctcttttaaaactaaaacaaaaccatcatagtgtgtaccaagcacctcacctcatttaagaaaatgtcatttttcaccaaagtcacttgactgtactgaaaaccatgctcagatgaagagtccaagtaagaagtatggaggagtgaaactgccctctggaagagagagtctgaactcaaggacactgtctcaaaaatcttttctgatagggaccctgtctcgatcttctctaagagagaatgtagctgggagggtggtcttaattcattttcaccaagtataccctcagaattcttgacatagtcctgttctctgttaatgtcataaatgccgtccttggcgtggccgccgcccccgaggacctgagatcccggctcggcctccttcccatgcttctcccggccgtgctctgcgtcctcccgggccctcgcgacaccggcgcacgtgggaagcaccagtcgccggctccgcgctcccgcggggacccccctcaggggcacgccgtccgccccagccccggggtcctcgccgcgggcgctgacagggacgccgcggccgcccgcgctctgtctcccgtcagggtcacgggcaagaggcaaccccgggacgcccggcagcctgcgagaacatgccgactttctctctgaccggcgctagcaacc

SEQ ID NO: 19195 - RNA, 74 nt, Homo sapiens
  source 1..74: mol_type = other RNA
tgtgaccctagaataattactcaccctctcaaaaccgagactcagagacgttgggtaattattctagggtcaca

SEQ ID NO: 19196 - RNA, 6980 nt, Homo sapiens
  source 1..6980: mol_type = other RNA
tgtgactgcattatgaaaattcttcacatggcccatttttacatcaattactacaaaaaatggacatttatcaagtatctgactcacaacatcaagaatgtgcctgtacaaataaatgttaacgaaattacacatttttcacactatctttttccacgattaatatgtatttccttcaattttcagtgaagacttttctaataatactattattaccttcaccccatttcctgtcctcatctactatttagatcacctacatcaaagaaataaaaataggctgggcccagtggcccatacctgtaatcccagcactttgggaggctgagataggcagatcacaaggtcaggagttcgaaaccagccttgccaacatgatgaaaccccatctctactaaaaatacaaaaattagctgggtgtggtggtgcgtgcctatagttccagctactcgggaggctgaggaagaagaatcgcttgaacctgggaggcggaggttgcagtgagccgagatcgcaccactgcactccagcctgggcaacagagcgagactccgtctcaaaaaagaaaaaaaaacaaaggtatttatttattgtttttgttccttttcctttgtgtaaacaaaaacaatatatttgggagaactttcaataaagctgaaattgacaaagttttattcccaataatgccaaagaactagtatcctccttactgaaggctaaaaagaaacagtgatgattaaattacagtagaacaggaattctagcaacagtattgtttctagttatttgtaaaaaataacaatgagttctgtcaattagttattgaatattagatagtacattactgcttttaagaacattttagaatttataggctgaaatactaaagttaataggtctagctacagaataaatgtcgtttatatggttgattttaatcaataatactgagagaacttaacacgtttaatataaatcctcacaacacccctgtgaggtaagtattgcttacacccactttacggatgggaaatcagaaagagcaagaagtaacaatctcaagagttataaataaaaaaattttttgttttcttataaggcagactgtgctgagttctgatgatacgctaataagaacaaatactaaaacagtctctatttttctccagaaaacaactgcgtgagatttcaaaagaaggaaaaattttaagctgactcaaggggaaaatgtttagtatctgcctgatacacacgaaagtgcatatgacatttccagtttcaagcttggtaatcattatgcaaactgcactatactattaggatactggctaacagtatagctccattttgtggagatgtagtcaaaaaataaaggttttagctggaagaacttttttttttttgagatggagtctcgctctgtcacccaggctggagtgcagtggtgcgatctccgctcactgcaacctctgcctcccgggttcaagctattccactgcctcagcctctcgagtagctgggattacaggtgtgtgccaccacacccggctaattttttgtatttttagtagagacgcggtttcactgtgttagccaggatggtctggatcttctgacctcgtgacccgcccgcctcggcctcccaaagtgctgggattacaagcatgagccaccacgcctggcctagctggaagaacttttaaaatacaaagcaaattttctcagtgagcaatcatgtctttaaaaaataatactcagggcacagtgttaggcatatgacagttactttaaaaaatgcctgcagacccgggcgcggtggctcatgcctgtaatctgaggcaggcagatcatgaggtcaggagctcgagaccatcctggccaacatggtgaaaccctgtctctactaaaaatacaaaaattagctgggcatggtggcacatgctcaggaggctgaggcaggagaatcacttgaattcgagaggcggaggttgcagtgagctgagattgcaccactgcactccagcctggcgacacagcacgactgtctcaaaaaaaaaaaaaaaaaaaaaaaaaaaagcctgcagaataaatgaaaacaacaataacaaaaactgggggtcagtcccacaccactattcactgcatctctggaattcagcttttgggattttttttctataaaatgaagttgatattttcccacttcctaaacagaatgaatgttttaaggaacaaggaaagagcatttgctttgaatttctaatattaaaaggaactataagaatagaaatacagttaaccactattttcttaactctcaacgaacagatatatttctgctttaaatgagtgttgtctatcacggccaatcagctgctagcaaactcttaccatttatccaaactctgccctgaggcacttgctgtcttatccaaccaaccatgtacaactctacctccaccctttagctatatacaaggatttcctgtgtcaaagaataatgagtgggcctggcacggtggctcacacctgtaatcccagcactatgggaggccgaggctggtgcatgacctgaggtcaggagttccagaccagcctgaccaagatggtgaaaccctgtctctgctaaaaacacaaaattagctgggtatggtggtgcatgcctgtaatcccaagctacttgggaggctaaggcaggagaatcgcttgaacccaggcagcagagattgcagtgagccgagatcacgccattgcactccagcctgggcaacaagggtgaaactccatcttaaaaaaaaattaaattaaaaaaataataataatgagtaggcaaacagggaagaatatagaggagaaaaattatcttaataagaacaatagaatttgaattgaagaaggctaggaaatatatcttaactagcctaaaatacaaaaaatcaatgttaatacttgtgttcttccaatgagatgatatttttgagggcagtacaaatttcaatagttgcttaagtgaattggtagaaaaaagtttaagattagacaaagttctgaccccaaagaacatacatttgttttaattactcccaatacaattgatcttatcaagttagatgtgctctcaacacacatcagtcttaaccataggagcctttactcacttgtttaaggcagaaactcaactgccttacacaatatccagtagctttcttcattcaatcctcaagaaaaacttaccactttgtaatttacctaaactgtttacctagagaaaacctttgtgtccttagaattagctggattactctttgagctccctcctgattggacgctgatgctgttgaatgtgtcaggaaacgtcctcagaagtggagggagctcaagagttttgtaagtggttaaattctaaggctcacaaaccaaattttttagatgtattcaaatgcccgtgaagcttagaatttaacaagagggcaaaaaaagatgagtctgttttattatccttgactatgcggggtttgaaatttaaacatttcagaaacaatttagatctatcctttgtggtgaagcttaaccagctatttcccaggtatatagagccggggaatctgttatttctttcatcaactttaattttcctggggttttagctttgtaagtgtcaccattataaaagagagttaagttgatttatagaggaaaagctaacatcatggatcttaaatgtagttatagaacactgaatgtatccactttgctggttttatggatcaggaaaaaagtgaaaactgtgccactgaaaaattactttttcagtgatttttagaaaattaaaatcaacccaggaagccccaaaaatcctgacgctgagggtagaaacatgatttatattttatcatcattctctttcaactcatgtaaacctctggtcataaaatctcaaattactttttaaggtgtctaagaaaacactctagaccaagttaacaaccctggggtttttagtcaatgcagttctagctcagtctctgtctctgcatgcttatttatctatgtgtgtatatcttactgtttcttaaatattttttaatgtctctctgactcttctccctttaactgttttttttattaaaaatgagatataccacatctgtaatcccagcactttgggaggccaaggcgggcagatgacgaggtcaggagatcgagaccatcctggctaacacggtgaaaccccgtctctactaaaaaaatacaaaaaaattagctgggcgtggtggcgggcgcctgtagtcccagctgctcaggaggctgaggcaggagaatggcgtgaacccgggaggcggagcttgcagtcagccgagatcgcgccactgcgccccagcctgggcgacacagagagactctgtctcaaaaaaaaaaagaggtatactcaatgttaaaaagtaaagagaagccatgtaggtaagatgttgtggagctagtagttaaaaaataaaactactcatgatttggtatatcttaaaataaatttttatacattataacatatgtataacatacagttatgcattaaagtaactattaatttcctatatggaagaaaatatttaaaaataatcctggtaggagtgaattcatgtgaaatgtaggcagaagtgatagtttagaatatgctttaaaacagatttcatttactttatattcaatttgattttactgattctataactggaaaaacttagaattctataaataactatttaaggtttccatatttctacattgatttctgatttctaaattgttatttcgtttgtgaaaagttcacagtagtaattgaatgttacattttaatagccacatattaatatgtcttatgagaagatctaatatatacaaccttaaaaccatggataagctgtgaagaaaaaaagtcaatgaaacttgaggaggaaaataatttatgaattaaaaatgccacgcaaattttctttttcagaattggtataaaaattctgaaagagaagctgctactcaactaggatagtatccacattttcttgtgtgagctctgactctaaggcacaaggcaagtctaagtgttcttgtgacaagcgagaacttttcagggagacatcagaccagctgtcacagtatggctgaaatctctgggccaatgcattaccaaacctttggcatcggttatatctgtaagatttacctttgtgtgtatacatgtgttccaacaattggctctttcgagggaatttatgaccacagatggtacagctcatttttcttttccttgaaaaagaaaaattacagtttaattctactggctctgtgtctttggagatcaaagatacttgactgatctgcaaaggctctgtggtaccccggttggtgtggtctggctgctgttcattctccttaacaatgaaggagctgagcctgcggcattcaagggcctcgctgttttcattaaggggatgcacttcaccaaggtcattactttccagaatggaagcagggacaccgaatggcagggatccagacacatgtgtatggagatgttgccttaggttactacgggaatcaaaacgttccccacagtaatggcataagtgtattttgacactgttttcagtaaaagtggggcctgtcacctctgatgagggtgaggggtggctctgggagatcacagattctgggtcacatctctcctgcttgatggaaactgggggcttctggtgctcctccagggcctgggtggcaggacaggccctctgctggtctgcagtgccatcatccagaccaatagcaagagacaactgcaactgggggtggtcaccctggacagcagctctgtttccactgttactggaaggagcttctttgacctccagtccttgtttgacaactgttttttgggttgttgagatctgaatgccatataaatttgaggactgcacagtctctggtgagaacacttgattcatttcagttgcaatgtgagaaaggtagtcggcgtgaagaaatcgaatcccttcctccaaacgactatgatccacaatctgttttggccctttccccgtgtacataatgtgcaacaaatagctgaatatgtcaggttggatgtcagttggttgtatttttatgcattcacttgtttggtgaataaatatcatcttgaaatagttagaaaaagcagcaagcactgctctgtgggctttgaagtaaacatctccaattgcaactgtgcaatcacacagaaaaccaaattctcgctgcatgttcagctgctggagaagaacaaggctatggctggcagtgtccattgtggttatgacagaatcttgtgagaggatcaacagctctgccaggacttgagtctcaagagaaagaatgccaaatttaatcccttggggtgatgcgggcgctaactgttgaaacatgctaggtgccgtcaggttccaggtactacgttgtgctatgcgctgcctccgcaactggtaacaactgattactccaaatactgagtgccagagaagacggtgataagatgggtcaagatctgtcccgcgactggtgcagctgcaggccgccgccctgggtggctcgcggcaggagggactgagcccggggcagcccacaggggcaggaccgcgtcgcttacccagatgccgccgcggcggcaggccgactcctccgtgcaggaggggcgggctcccaagccgcgcactgcaagcagtggcgccggctcacgcacccctcggccgcctctcgcgcggcttcccgcgccggcagcccgcgatggccccacgtgaccgcgtgtctggtagcaggggaaagaggggcgccagggccggggtgtgcgtgcgtgcgtgcgtgcgtacgtgcgcgccctcccgcccgcccgcctcagtggccgggcgggggtcggcccgcgctctgagtgccgccgccacagttcgcagttg

SEQ ID NO: 19197 - RNA, 6523 nt, Homo sapiens
  source 1..6523: mol_type = other RNA
tgtgactgcattatgaaaattcttcacatggcccatttttacatcaattactacaaaaaatggacatttatcaagtatctgactcacaacatcaagaatgtgcctgtacaaataaatgttaacgaaattacacatttttcacactatctttttccacgattaatatgtatttccttcaattttcagtgaagacttttctaataatactattattaccttcaccccatttcctgtcctcatctactatttagatcacctacatcaaagaaataaaaataggctgggcccagtggcccatacctgtaatcccagcactttgggaggctgagataggcagatcacaaggtcaggagttcgaaaccagccttgccaacatgatgaaaccccatctctactaaaaatacaaaaattagctgggtgtggtggtgcgtgcctatagttccagctactcgggaggctgaggaagaagaatcgcttgaacctgggaggcggaggttgcagtgagccgagatcgcaccactgcactccagcctgggcaacagagcgagactccgtctcaaaaaagaaaaaaaaacaaaggtatttatttattgtttttgttccttttcctttgtgtaaacaaaaacaatatatttgggagaactttcaataaagctgaaattgacaaagttttattcccaataatgccaaagaactagtatcctccttactgaaggctaaaaagaaacagtgatgattaaattacagtagaacaggaattctagcaacagtattgtttctagttatttgtaaaaaataacaatgagttctgtcaattagttattgaatattagatagtacattactgcttttaagaacattttagaatttataggctgaaatactaaagttaataggtctagctacagaataaatgtcgtttatatggttgattttaatcaataatactgagagaacttaacacgtttaatataaatcctcacaacacccctgtgaggtaagtattgcttacacccactttacggatgggaaatcagaaagagcaagaagtaacaatctcaagagttataaataaaaaaattttttgttttcttataaggcagactgtgctgagttctgatgatacgctaataagaacaaatactaaaacagtctctatttttctccagaaaacaactgcgtgagatttcaaaagaaggaaaaattttaagctgactcaaggggaaaatgtttagtatctgcctgatacacacgaaagtgcatatgacatttccagtttcaagcttggtaatcattatgcaaactgcactatactattaggatactggctaacagtatagctccattttgtggagatgtagtcaaaaaataaaggttttagctggaagaacttttttttttttgagatggagtctcgctctgtcacccaggctggagtgcagtggtgcgatctccgctcactgcaacctctgcctcccgggttcaagctattccactgcctcagcctctcgagtagctgggattacaggtgtgtgccaccacacccggctaattttttgtatttttagtagagacgcggtttcactgtgttagccaggatggtctggatcttctgacctcgtgacccgcccgcctcggcctcccaaagtgctgggattacaagcatgagccaccacgcctggcctagctggaagaacttttaaaatacaaagcaaattttctcagtgagcaatcatgtctttaaaaaataatactcagggcacagtgttaggcatatgacagttactttaaaaaatgcctgcagacccgggcgcggtggctcatgcctgtaatctgaggcaggcagatcatgaggtcaggagctcgagaccatcctggccaacatggtgaaaccctgtctctactaaaaatacaaaaattagctgggcatggtggcacatgctcaggaggctgaggcaggagaatcacttgaattcgagaggcggaggttgcagtgagctgagattgcaccactgcactccagcctggcgacacagcacgactgtctcaaaaaaaaaaaaaaaaaaaaaaaaaaaagcctgcagaataaatgaaaacaacaataacaaaaactgggggtcagtcccacaccactattcactgcatctctggaattcagcttttgggattttttttctataaaatgaagttgatattttcccacttcctaaacagaatgaatgttttaaggaacaaggaaagagcatttgctttgaatttctaatattaaaaggaactataagaatagaaatacagttaaccactattttcttaactctcaacgaacagatatatttctgctttaaatgagtgttgtctatcacggccaatcagctgctagcaaactcttaccatttatccaaactctgccctgaggcacttgctgtcttatccaaccaaccatgtacaactctacctccaccctttagctatatacaaggatttcctgtgtcaaagaataatgagtgggcctggcacggtggctcacacctgtaatcccagcactatgggaggccgaggctggtgcatgacctgaggtcaggagttccagaccagcctgaccaagatggtgaaaccctgtctctgctaaaaacacaaaattagctgggtatggtggtgcatgcctgtaatcccaagctacttgggaggctaaggcaggagaatcgcttgaacccaggcagcagagattgcagtgagccgagatcacgccattgcactccagcctgggcaacaagggtgaaactccatcttaaaaaaaaattaaattaaaaaaataataataatgagtaggcaaacagggaagaatatagaggagaaaaattatcttaataagaacaatagaatttgaattgaagaaggctaggaaatatatcttaactagcctaaaatacaaaaaatcaatgttaatacttgtgttcttccaatgagatgatatttttgagggcagtacaaatttcaatagttgcttaagtgaattggtagaaaaaagtttaagattagacaaagttctgaccccaaagaacatacatttgttttaattactcccaatacaattgatcttatcaagttagatgtgctctcaacacacatcagtcttaaccataggagcctttactcacttgtttaaggcagaaactcaactgccttacacaatatccagtagctttcttcattcaatcctcaagaaaaacttaccactttgtaatttacctaaactgtttacctagagaaaacctttgtgtccttagaattagctggattactctttgagctccctcctgattggacgctgatgctgttgaatgtgtcaggaaacgtcctcagaagtggagggagctcaagagttttgtaagtggttaaattctaaggctcacaaaccaaattttttagatgtattcaaatgcccgtgaagcttagaatttaacaagagggcaaaaaaagatgagtctgttttattatccttgactatgcggggtttgaaatttaaacatttcagaaacaatttagatctatcctttgtggtgaagcttaaccagctatttcccaggtatatagagccggggaatctgttatttctttcatcaactttaattttcctggggttttagctttgtaagtgtcaccattataaaagagagttaagttgatttatagaggaaaagctaacatcatggatcttaaatgtagttatagaacactgaatgtatccactttgctggttttatggatcaggaaaaaagtgaaaactgtgccactgaaaaattactttttcagtgatttttagaaaattaaaatcaacccaggaagccccaaaaatcctgacgctgagggtagaaacatgatttatattttatcatcattctctttcaactcatgtaaacctctggtcataaaatctcaaattactttttaaggtgtctaagaaaacactctagaccaagttaacaaccctggggtttttagtcaatgcagttctagctcagtctctgtctctgcatgcttatttatctatgtgtgtatatcttactgtttcttaaatattttttaatgtctctctgactcttctccctttaactgttttttttattaaaaatgagatataccacatctgtaatcccagcactttgggaggccaaggcgggcagatgacgaggtcaggagatcgagaccatcctggctaacacggtgaaaccccgtctctactaaaaaaatacaaaaaaattagctgggcgtggtggcgggcgcctgtagtcccagctgctcaggaggctgaggcaggagaatggcgtgaacccgggaggcggagcttgcagtcagccgagatcgcgccactgcgccccagcctgggcgacacagagagactctgtctcaaaaaaaaaaagaggtatactcaatgttaaaaagtaaagagaagccatgtaggtaagatgttgtggagctagtagttaaaaaataaaactactcatgatttggtatatcttaaaataaatttttatacattataacatatgtataacatacagttatgcattaaagtaactattaatttcctatatggaagaaaatatttaaaaataatcctggtaggagtgaattcatgtgaaatgtaggcagaagtgatagtttagaatatgctttaaaacagatttcatttactttatattcaatttgattttactgattctataactggaaaaacttagaattctataaataactatttaaggtttccatatttctacattgatttctgatttctaaattgttatttcgtttgtgaaaagttcacagtagtaattgaatgttacattttaatagccacatattaatatgtcttatgagaagatctaatatatacaaccttaaaaccatggataagctgtgaagaaaaaaagtcaatgaaacttgaggaggaaaataatttatgaattaaaaatgccacgcaaattttctttttcagaattggtataaaaattctgaaagagaagctgctactcaactaggatagtatccacattttcttgtgtgagctctgactctaaggcacaaggcaagtctaagtgttcttgtgacaagcgagaacttttcagggagacatcagaccagctgtcacagtatggctgaaatctctgggccaatgcattaccaaacctttggcatcggttatatctgtaagatttacctttgtgtgtatacatgtgttccaacaattggctctttcgagggaatttatgaccacagatggtacagctcatttttcttttccttgaaaaagaaaaattacagtttaattctactggctctgtgtctttggagatcaaagatacttgactgatctgcaaaggctctgtggtaccccggttggtgtggtctggctgctgttcattctccttaacaatgaaggagctgagcctgcggcattcaagggcctcgctgttttcattaaggggatgcacttcaccaaggtcattactttccagaatggaagcagggacaccgaatggcagggatccagacacatgtgtatggagatgttgccttaggttactacgggaatcaaaacgttccccacagtaatggcataagtgtattttgacactgttttcagtaaaagtggggcctgtcacctctgatgagggtgaggggtggctctgggagatcacagattctgggtcacatctctcctgcttgatggaaactgggggcttctggtgctcctccagggcctgggtggcaggacaggccctctgctggtctgcagtgccatcatccagaccaatagcaagagacaactgcaactgggggtggtcaccctggacagcagctctgtttccactgttactggaaggagcttctttgacctccagtccttgtttgacaactgttttttgggttgttgagatctgaatgccatataaatttgaggactgcacagtctctggtgagaacacttgattcatttcagttgcaatgtgagaaaggtagtcggcgtgaagaaatcgaatcccttcctccaaacgactatgatccacaatctgttttggccctttccccgtgtacataatgtgcaacaaatagctgaatatgtcaggttggatgtcagttggttgtatttttatgcattcacttgtttggtgaataaatatcatcttgaaatagttagaaaaagcagcaagcactgctctgtgggctttgaagtaaacatctccaattgcaactgtgcaatcacacagaaaaccaaattctcgctgcatgttcagctgctggagaagaacaaggctatggctggcagtgtccattgtggttccagatgccgccgcggcggcaggccgactcctccgtgcaggaggggcgggctcccaagccgcgcactgcaagcagtggcgccggctcacgcacccctcggccgcctctcgcgcggcttcccgcgccggcagcccgcgatggccccacgtgaccgcgtgtctggtagcaggggaaagag

SEQ ID NO: 19198 - RNA, 7266 nt, Homo sapiens
  source 1..7266: mol_type = other RNA
tgtgactgcattatgaaaattcttcacatggcccatttttacatcaattactacaaaaaatggacatttatcaagtatctgactcacaacatcaagaatgtgcctgtacaaataaatgttaacgaaattacacatttttcacactatctttttccacgattaatatgtatttccttcaattttcagtgaagacttttctaataatactattattaccttcaccccatttcctgtcctcatctactatttagatcacctacatcaaagaaataaaaataggctgggcccagtggcccatacctgtaatcccagcactttgggaggctgagataggcagatcacaaggtcaggagttcgaaaccagccttgccaacatgatgaaaccccatctctactaaaaatacaaaaattagctgggtgtggtggtgcgtgcctatagttccagctactcgggaggctgaggaagaagaatcgcttgaacctgggaggcggaggttgcagtgagccgagatcgcaccactgcactccagcctgggcaacagagcgagactccgtctcaaaaaagaaaaaaaaacaaaggtatttatttattgtttttgttccttttcctttgtgtaaacaaaaacaatatatttgggagaactttcaataaagctgaaattgacaaagttttattcccaataatgccaaagaactagtatcctccttactgaaggctaaaaagaaacagtgatgattaaattacagtagaacaggaattctagcaacagtattgtttctagttatttgtaaaaaataacaatgagttctgtcaattagttattgaatattagatagtacattactgcttttaagaacattttagaatttataggctgaaatactaaagttaataggtctagctacagaataaatgtcgtttatatggttgattttaatcaataatactgagagaacttaacacgtttaatataaatcctcacaacacccctgtgaggtaagtattgcttacacccactttacggatgggaaatcagaaagagcaagaagtaacaatctcaagagttataaataaaaaaattttttgttttcttataaggcagactgtgctgagttctgatgatacgctaataagaacaaatactaaaacagtctctatttttctccagaaaacaactgcgtgagatttcaaaagaaggaaaaattttaagctgactcaaggggaaaatgtttagtatctgcctgatacacacgaaagtgcatatgacatttccagtttcaagcttggtaatcattatgcaaactgcactatactattaggatactggctaacagtatagctccattttgtggagatgtagtcaaaaaataaaggttttagctggaagaacttttttttttttgagatggagtctcgctctgtcacccaggctggagtgcagtggtgcgatctccgctcactgcaacctctgcctcccgggttcaagctattccactgcctcagcctctcgagtagctgggattacaggtgtgtgccaccacacccggctaattttttgtatttttagtagagacgcggtttcactgtgttagccaggatggtctggatcttctgacctcgtgacccgcccgcctcggcctcccaaagtgctgggattacaagcatgagccaccacgcctggcctagctggaagaacttttaaaatacaaagcaaattttctcagtgagcaatcatgtctttaaaaaataatactcagggcacagtgttaggcatatgacagttactttaaaaaatgcctgcagacccgggcgcggtggctcatgcctgtaatctgaggcaggcagatcatgaggtcaggagctcgagaccatcctggccaacatggtgaaaccctgtctctactaaaaatacaaaaattagctgggcatggtggcacatgctcaggaggctgaggcaggagaatcacttgaattcgagaggcggaggttgcagtgagctgagattgcaccactgcactccagcctggcgacacagcacgactgtctcaaaaaaaaaaaaaaaaaaaaaaaaaaaagcctgcagaataaatgaaaacaacaataacaaaaactgggggtcagtcccacaccactattcactgcatctctggaattcagcttttgggattttttttctataaaatgaagttgatattttcccacttcctaaacagaatgaatgttttaaggaacaaggaaagagcatttgctttgaatttctaatattaaaaggaactataagaatagaaatacagttaaccactattttcttaactctcaacgaacagatatatttctgctttaaatgagtgttgtctatcacggccaatcagctgctagcaaactcttaccatttatccaaactctgccctgaggcacttgctgtcttatccaaccaaccatgtacaactctacctccaccctttagctatatacaaggatttcctgtgtcaaagaataatgagtgggcctggcacggtggctcacacctgtaatcccagcactatgggaggccgaggctggtgcatgacctgaggtcaggagttccagaccagcctgaccaagatggtgaaaccctgtctctgctaaaaacacaaaattagctgggtatggtggtgcatgcctgtaatcccaagctacttgggaggctaaggcaggagaatcgcttgaacccaggcagcagagattgcagtgagccgagatcacgccattgcactccagcctgggcaacaagggtgaaactccatcttaaaaaaaaattaaattaaaaaaataataataatgagtaggcaaacagggaagaatatagaggagaaaaattatcttaataagaacaatagaatttgaattgaagaaggctaggaaatatatcttaactagcctaaaatacaaaaaatcaatgttaatacttgtgttcttccaatgagatgatatttttgagggcagtacaaatttcaatagttgcttaagtgaattggtagaaaaaagtttaagattagacaaagttctgaccccaaagaacatacatttgttttaattactcccaatacaattgatcttatcaagttagatgtgctctcaacacacatcagtcttaaccataggagcctttactcacttgtttaaggcagaaactcaactgccttacacaatatccagtagctttcttcattcaatcctcaagaaaaacttaccactttgtaatttacctaaactgtttacctagagaaaacctttgtgtccttagaattagctggattactctttgagctccctcctgattggacgctgatgctgttgaatgtgtcaggaaacgtcctcagaagtggagggagctcaagagttttgtaagtggttaaattctaaggctcacaaaccaaattttttagatgtattcaaatgcccgtgaagcttagaatttaacaagagggcaaaaaaagatgagtctgttttattatccttgactatgcggggtttgaaatttaaacatttcagaaacaatttagatctatcctttgtggtgaagcttaaccagctatttcccaggtatatagagccggggaatctgttatttctttcatcaactttaattttcctggggttttagctttgtaagtgtcaccattataaaagagagttaagttgatttatagaggaaaagctaacatcatggatcttaaatgtagttatagaacactgaatgtatccactttgctggttttatggatcaggaaaaaagtgaaaactgtgccactgaaaaattactttttcagtgatttttagaaaattaaaatcaacccaggaagccccaaaaatcctgacgctgagggtagaaacatgatttatattttatcatcattctctttcaactcatgtaaacctctggtcataaaatctcaaattactttttaaggtgtctaagaaaacactctagaccaagttaacaaccctggggtttttagtcaatgcagttctagctcagtctctgtctctgcatgcttatttatctatgtgtgtatatcttactgtttcttaaatattttttaatgtctctctgactcttctccctttaactgttttttttattaaaaatgagatataccacatctgtaatcccagcactttgggaggccaaggcgggcagatgacgaggtcaggagatcgagaccatcctggctaacacggtgaaaccccgtctctactaaaaaaatacaaaaaaattagctgggcgtggtggcgggcgcctgtagtcccagctgctcaggaggctgaggcaggagaatggcgtgaacccgggaggcggagcttgcagtcagccgagatcgcgccactgcgccccagcctgggcgacacagagagactctgtctcaaaaaaaaaaagaggtatactcaatgttaaaaagtaaagagaagccatgtaggtaagatgttgtggagctagtagttaaaaaataaaactactcatgatttggtatatcttaaaataaatttttatacattataacatatgtataacatacagttatgcattaaagtaactattaatttcctatatggaagaaaatatttaaaaataatcctggtaggagtgaattcatgtgaaatgtaggcagaagtgatagtttagaatatgctttaaaacagatttcatttactttatattcaatttgattttactgattctataactggaaaaacttagaattctataaataactatttaaggtttccatatttctacattgatttctgatttctaaattgttatttcgtttgtgaaaagttcacagtagtaattgaatgttacattttaatagccacatattaatatgtcttatgagaagatctaatatatacaaccttaaaaccatggataagctgtgaagaaaaaaagtcaatgaaacttgaggaggaaaataatttatgaattaaaaatgccacgcaaattttctttttcagaattggtataaaaattctgaaagagaagctgctactcaactaggatagtatccacattttcttgtgtgagctctgactctaaggcacaaggcaagtctaagtgttcttgtgacaagcgagaacttttcagggagacatcagaccagctgtcacagtatggctgaaatctctgggccaatgcattaccaaacctttggcatcggttatatctgtaagatttacctttgtgtgtatacatgtgttccaacaattggctctttcgagggaatttatgaccacagatggtacagctcatttttcttttccttgaaaaagaaaaattacagtttaattctactggctctgtgtctttggagatcaaagatacttgactgatctgcaaaggctctgtggtaccccggttggtgtggtctggctgctgttcattctccttaacaatgaaggagctgagcctgcggcattcaagggcctcgctgttttcattaaggggatgcacttcaccaaggtcattactttccagaatggaagcagggacaccgaatggcagggatccagacacatgtgtatggagatgttgccttaggttactacgggaatcaaaacgttccccacagtaatggcataagtgtattttgacactgttttcagtaaaagtggggcctgtcacctctgatgagggtgaggggtggctctgggagatcacagattctgggtcacatctctcctgcttgatggaaactgggggcttctggtgctcctccagggcctgggtggcaggacaggccctctgctggtctgcagtgccatcatccagaccaatagcaagagacaactgcaactgggggtggtcaccctggacagcagctctgtttccactgttactggaaggagcttctttgacctccagtccttgtttgacaactgttttttgggttgttgagatctgaatgccatataaatttgaggactgcacagtctctggtgagaacacttgattcatttcagttgcaatgtgagaaaggtagtcggcgtgaagaaatcgaatcccttcctccaaacgactatgatccacaatctgttttggccctttccccgtgtacataatgtgcaacaaatagctgaatatgtcaggttggatgtcagttggttgtatttttatgcattcacttgtttggtgaataaatatcatcttgaaatagttagaaaaagcagcaagcactgctctgtgggctttgaagtaaacatctccaattgcaactgtgcaatcacacagaaaaccaaattctcgctgcatgttcagctgctggagaagaacaaggctatggctggcagtgtccattgtggttctataatcccggctactcgggaggctgaggcgggagaatcgcttgaacccaggaggcagaggttgtggtgagctgagattgtgtcattgcactccagtctgggcaacaagagtgaaactccatctccgccggatacattctctacaggtgagtggggtaaactggcactgcggtcctggcatggtggagagtgcaatcaccaaggtgtctggagccttggagtcttagctatcaagaggtgtagctagctccagctacatcacgctcttcaggcctggtgtcttctatgacagaatcttgtgagaggatcaacagctctgccaggacttgagtctcaagagaaagaatgccaaatttaatcccttggggtgatgcgggcgctaactgttgaaacatgctaggtgccgtcaggttccaggtactacgttgtgctatgcgctgcctccgcaactggtaacaactgattactccaaatactgagtgccagagaagacggtgataagatgggtcaagatctgtcccgcgactggtgcagctgcaggccgccgccctgggtggctcgcggcaggagggactgagcccggggcagcccacaggggcaggaccgcgtcgcttacccagatgccgccgcggcggcaggccgactcctccgtgcaggaggggcgggctcccaagccgcgcactgcaagcagtggcgccggctcacgcacccctcggccgcctctcgcgcggcttcccgcgccggcagcccgcgatggccccacgtgaccgcgtgtctggtagcaggggaaagaggggcgccagggccggggtgtgcgtgcgtgcgtgcgtgcgtacgtgcgcgccctcccgcccgcccgcctcagtggccgggcgggggtcggcccgcgctctgagtgccgccgccacagttcgcagttg

SEQ ID NO: 19199 - RNA, 7067 nt, Homo sapiens
  source 1..7067: mol_type = other RNA
tgtgactgcattatgaaaattcttcacatggcccatttttacatcaattactacaaaaaatggacatttatcaagtatctgactcacaacatcaagaatgtgcctgtacaaataaatgttaacgaaattacacatttttcacactatctttttccacgattaatatgtatttccttcaattttcagtgaagacttttctaataatactattattaccttcaccccatttcctgtcctcatctactatttagatcacctacatcaaagaaataaaaataggctgggcccagtggcccatacctgtaatcccagcactttgggaggctgagataggcagatcacaaggtcaggagttcgaaaccagccttgccaacatgatgaaaccccatctctactaaaaatacaaaaattagctgggtgtggtggtgcgtgcctatagttccagctactcgggaggctgaggaagaagaatcgcttgaacctgggaggcggaggttgcagtgagccgagatcgcaccactgcactccagcctgggcaacagagcgagactccgtctcaaaaaagaaaaaaaaacaaaggtatttatttattgtttttgttccttttcctttgtgtaaacaaaaacaatatatttgggagaactttcaataaagctgaaattgacaaagttttattcccaataatgccaaagaactagtatcctccttactgaaggctaaaaagaaacagtgatgattaaattacagtagaacaggaattctagcaacagtattgtttctagttatttgtaaaaaataacaatgagttctgtcaattagttattgaatattagatagtacattactgcttttaagaacattttagaatttataggctgaaatactaaagttaataggtctagctacagaataaatgtcgtttatatggttgattttaatcaataatactgagagaacttaacacgtttaatataaatcctcacaacacccctgtgaggtaagtattgcttacacccactttacggatgggaaatcagaaagagcaagaagtaacaatctcaagagttataaataaaaaaattttttgttttcttataaggcagactgtgctgagttctgatgatacgctaataagaacaaatactaaaacagtctctatttttctccagaaaacaactgcgtgagatttcaaaagaaggaaaaattttaagctgactcaaggggaaaatgtttagtatctgcctgatacacacgaaagtgcatatgacatttccagtttcaagcttggtaatcattatgcaaactgcactatactattaggatactggctaacagtatagctccattttgtggagatgtagtcaaaaaataaaggttttagctggaagaacttttttttttttgagatggagtctcgctctgtcacccaggctggagtgcagtggtgcgatctccgctcactgcaacctctgcctcccgggttcaagctattccactgcctcagcctctcgagtagctgggattacaggtgtgtgccaccacacccggctaattttttgtatttttagtagagacgcggtttcactgtgttagccaggatggtctggatcttctgacctcgtgacccgcccgcctcggcctcccaaagtgctgggattacaagcatgagccaccacgcctggcctagctggaagaacttttaaaatacaaagcaaattttctcagtgagcaatcatgtctttaaaaaataatactcagggcacagtgttaggcatatgacagttactttaaaaaatgcctgcagacccgggcgcggtggctcatgcctgtaatctgaggcaggcagatcatgaggtcaggagctcgagaccatcctggccaacatggtgaaaccctgtctctactaaaaatacaaaaattagctgggcatggtggcacatgctcaggaggctgaggcaggagaatcacttgaattcgagaggcggaggttgcagtgagctgagattgcaccactgcactccagcctggcgacacagcacgactgtctcaaaaaaaaaaaaaaaaaaaaaaaaaaaagcctgcagaataaatgaaaacaacaataacaaaaactgggggtcagtcccacaccactattcactgcatctctggaattcagcttttgggattttttttctataaaatgaagttgatattttcccacttcctaaacagaatgaatgttttaaggaacaaggaaagagcatttgctttgaatttctaatattaaaaggaactataagaatagaaatacagttaaccactattttcttaactctcaacgaacagatatatttctgctttaaatgagtgttgtctatcacggccaatcagctgctagcaaactcttaccatttatccaaactctgccctgaggcacttgctgtcttatccaaccaaccatgtacaactctacctccaccctttagctatatacaaggatttcctgtgtcaaagaataatgagtgggcctggcacggtggctcacacctgtaatcccagcactatgggaggccgaggctggtgcatgacctgaggtcaggagttccagaccagcctgaccaagatggtgaaaccctgtctctgctaaaaacacaaaattagctgggtatggtggtgcatgcctgtaatcccaagctacttgggaggctaaggcaggagaatcgcttgaacccaggcagcagagattgcagtgagccgagatcacgccattgcactccagcctgggcaacaagggtgaaactccatcttaaaaaaaaattaaattaaaaaaataataataatgagtaggcaaacagggaagaatatagaggagaaaaattatcttaataagaacaatagaatttgaattgaagaaggctaggaaatatatcttaactagcctaaaatacaaaaaatcaatgttaatacttgtgttcttccaatgagatgatatttttgagggcagtacaaatttcaatagttgcttaagtgaattggtagaaaaaagtttaagattagacaaagttctgaccccaaagaacatacatttgttttaattactcccaatacaattgatcttatcaagttagatgtgctctcaacacacatcagtcttaaccataggagcctttactcacttgtttaaggcagaaactcaactgccttacacaatatccagtagctttcttcattcaatcctcaagaaaaacttaccactttgtaatttacctaaactgtttacctagagaaaacctttgtgtccttagaattagctggattactctttgagctccctcctgattggacgctgatgctgttgaatgtgtcaggaaacgtcctcagaagtggagggagctcaagagttttgtaagtggttaaattctaaggctcacaaaccaaattttttagatgtattcaaatgcccgtgaagcttagaatttaacaagagggcaaaaaaagatgagtctgttttattatccttgactatgcggggtttgaaatttaaacatttcagaaacaatttagatctatcctttgtggtgaagcttaaccagctatttcccaggtatatagagccggggaatctgttatttctttcatcaactttaattttcctggggttttagctttgtaagtgtcaccattataaaagagagttaagttgatttatagaggaaaagctaacatcatggatcttaaatgtagttatagaacactgaatgtatccactttgctggttttatggatcaggaaaaaagtgaaaactgtgccactgaaaaattactttttcagtgatttttagaaaattaaaatcaacccaggaagccccaaaaatcctgacgctgagggtagaaacatgatttatattttatcatcattctctttcaactcatgtaaacctctggtcataaaatctcaaattactttttaaggtgtctaagaaaacactctagaccaagttaacaaccctggggtttttagtcaatgcagttctagctcagtctctgtctctgcatgcttatttatctatgtgtgtatatcttactgtttcttaaatattttttaatgtctctctgactcttctccctttaactgttttttttattaaaaatgagatataccacatctgtaatcccagcactttgggaggccaaggcgggcagatgacgaggtcaggagatcgagaccatcctggctaacacggtgaaaccccgtctctactaaaaaaatacaaaaaaattagctgggcgtggtggcgggcgcctgtagtcccagctgctcaggaggctgaggcaggagaatggcgtgaacccgggaggcggagcttgcagtcagccgagatcgcgccactgcgccccagcctgggcgacacagagagactctgtctcaaaaaaaaaaagaggtatactcaatgttaaaaagtaaagagaagccatgtaggtaagatgttgtggagctagtagttaaaaaataaaactactcatgatttggtatatcttaaaataaatttttatacattataacatatgtataacatacagttatgcattaaagtaactattaatttcctatatggaagaaaatatttaaaaataatcctggtaggagtgaattcatgtgaaatgtaggcagaagtgatagtttagaatatgctttaaaacagatttcatttactttatattcaatttgattttactgattctataactggaaaaacttagaattctataaataactatttaaggtttccatatttctacattgatttctgatttctaaattgttatttcgtttgtgaaaagttcacagtagtaattgaatgttacattttaatagccacatattaatatgtcttatgagaagatctaatatatacaaccttaaaaccatggataagctgtgaagaaaaaaagtcaatgaaacttgaggaggaaaataatttatgaattaaaaatgccacgcaaattttctttttcagaattggtataaaaattctgaaagagaagctgctactcaactaggatagtatccacattttcttgtgtgagctctgactctaaggcacaaggcaagtctaagtgttcttgtgacaagcgagaacttttcagggagacatcagaccagctgtcacagtatggctgaaatctctgggccaatgcattaccaaacctttggcatcggttatatctgtaagatttacctttgtgtgtatacatgtgttccaacaattggctctttcgagggaatttatgaccacagatggtacagctcatttttcttttccttgaaaaagaaaaattacagtttaattctactggctctgtgtctttggagatcaaagatacttgactgatctgcaaaggctctgtggtaccccggttggtgtggtctggctgctgttcattctccttaacaatgaaggagctgagcctgcggcattcaagggcctcgctgttttcattaaggggatgcacttcaccaaggtcattactttccagaatggaagcagggacaccgaatggcagggatccagacacatgtgtatggagatgttgccttaggttactacgggaatcaaaacgttccccacagtaatggcataagtgtattttgacactgttttcagtaaaagtggggcctgtcacctctgatgagggtgaggggtggctctgggagatcacagattctgggtcacatctctcctgcttgatggaaactgggggcttctggtgctcctccagggcctgggtggcaggacaggccctctgctggtctgcagtgccatcatccagaccaatagcaagagacaactgcaactgggggtggtcaccctggacagcagctctgtttccactgttactggaaggagcttctttgacctccagtccttgtttgacaactgttttttgggttgttgagatctgaatgccatataaatttgaggactgcacagtctctggtgagaacacttgattcatttcagttgcaatgtgagaaaggtagtcggcgtgaagaaatcgaatcccttcctccaaacgactatgatccacaatctgttttggccctttccccgtgtacataatgtgcaacaaatagctgaatatgtcaggttggatgtcagttggttgtatttttatgcattcacttgtttggtgaataaatatcatcttgaaatagttagaaaaagcagcaagcactgctctgtgggctttgaagtaaacatctccaattgcaactgtgcaatcacacagaaaaccaaattctcgctgcatgttcagctgctggagaagaacaaggctatggctggcagtgtccattgtggttcttagctggacttaaactccaagttctgcctcccctatggtggacagcagctgaaatctctgctcctttagccttaagtgtgctgtttggaggctgctccacacatgtacagttgaggggtttgcaagaaattcaagcagagtttataaacagtgtttggggttctgccactccaacattctttctaggattttctcctgcactttccagctgcatgatcactgtgagctctgtcctcttttcttcaagagagattacaggttgttattacagttgtagccacctcttcatatcaccagctgggaccttatgccagtatgacagaatcttgtgagaggatcaacagctctgccaggacttgagtctcaagagaaagaatgccaaatttaatcccttggggtgatgcgggcgctaactgttgaaacatgctaggtgccgtcaggttccaggtactacgttgtgctatgcgctgcctccgcaactggtaacaactgattactccaaatactgagtgccagagaagacggtgataagatgggtcaagccagatgccgccgcggcggcaggccgactcctccgtgcaggaggggcgggctcccaagccgcgcactgcaagcagtggcgccggctcacgcacccctcggccgcctctcgcgcggcttcccgcgccggcagcccgcgatggccccacgtgaccgcgtgtctggtagcaggggaaagag

SEQ ID NO: 19200 - RNA, 6722 nt, Homo sapiens
  source 1..6722: mol_type = other RNA
tgtgactgcattatgaaaattcttcacatggcccatttttacatcaattactacaaaaaatggacatttatcaagtatctgactcacaacatcaagaatgtgcctgtacaaataaatgttaacgaaattacacatttttcacactatctttttccacgattaatatgtatttccttcaattttcagtgaagacttttctaataatactattattaccttcaccccatttcctgtcctcatctactatttagatcacctacatcaaagaaataaaaataggctgggcccagtggcccatacctgtaatcccagcactttgggaggctgagataggcagatcacaaggtcaggagttcgaaaccagccttgccaacatgatgaaaccccatctctactaaaaatacaaaaattagctgggtgtggtggtgcgtgcctatagttccagctactcgggaggctgaggaagaagaatcgcttgaacctgggaggcggaggttgcagtgagccgagatcgcaccactgcactccagcctgggcaacagagcgagactccgtctcaaaaaagaaaaaaaaacaaaggtatttatttattgtttttgttccttttcctttgtgtaaacaaaaacaatatatttgggagaactttcaataaagctgaaattgacaaagttttattcccaataatgccaaagaactagtatcctccttactgaaggctaaaaagaaacagtgatgattaaattacagtagaacaggaattctagcaacagtattgtttctagttatttgtaaaaaataacaatgagttctgtcaattagttattgaatattagatagtacattactgcttttaagaacattttagaatttataggctgaaatactaaagttaataggtctagctacagaataaatgtcgtttatatggttgattttaatcaataatactgagagaacttaacacgtttaatataaatcctcacaacacccctgtgaggtaagtattgcttacacccactttacggatgggaaatcagaaagagcaagaagtaacaatctcaagagttataaataaaaaaattttttgttttcttataaggcagactgtgctgagttctgatgatacgctaataagaacaaatactaaaacagtctctatttttctccagaaaacaactgcgtgagatttcaaaagaaggaaaaattttaagctgactcaaggggaaaatgtttagtatctgcctgatacacacgaaagtgcatatgacatttccagtttcaagcttggtaatcattatgcaaactgcactatactattaggatactggctaacagtatagctccattttgtggagatgtagtcaaaaaataaaggttttagctggaagaacttttttttttttgagatggagtctcgctctgtcacccaggctggagtgcagtggtgcgatctccgctcactgcaacctctgcctcccgggttcaagctattccactgcctcagcctctcgagtagctgggattacaggtgtgtgccaccacacccggctaattttttgtatttttagtagagacgcggtttcactgtgttagccaggatggtctggatcttctgacctcgtgacccgcccgcctcggcctcccaaagtgctgggattacaagcatgagccaccacgcctggcctagctggaagaacttttaaaatacaaagcaaattttctcagtgagcaatcatgtctttaaaaaataatactcagggcacagtgttaggcatatgacagttactttaaaaaatgcctgcagacccgggcgcggtggctcatgcctgtaatctgaggcaggcagatcatgaggtcaggagctcgagaccatcctggccaacatggtgaaaccctgtctctactaaaaatacaaaaattagctgggcatggtggcacatgctcaggaggctgaggcaggagaatcacttgaattcgagaggcggaggttgcagtgagctgagattgcaccactgcactccagcctggcgacacagcacgactgtctcaaaaaaaaaaaaaaaaaaaaaaaaaaaagcctgcagaataaatgaaaacaacaataacaaaaactgggggtcagtcccacaccactattcactgcatctctggaattcagcttttgggattttttttctataaaatgaagttgatattttcccacttcctaaacagaatgaatgttttaaggaacaaggaaagagcatttgctttgaatttctaatattaaaaggaactataagaatagaaatacagttaaccactattttcttaactctcaacgaacagatatatttctgctttaaatgagtgttgtctatcacggccaatcagctgctagcaaactcttaccatttatccaaactctgccctgaggcacttgctgtcttatccaaccaaccatgtacaactctacctccaccctttagctatatacaaggatttcctgtgtcaaagaataatgagtgggcctggcacggtggctcacacctgtaatcccagcactatgggaggccgaggctggtgcatgacctgaggtcaggagttccagaccagcctgaccaagatggtgaaaccctgtctctgctaaaaacacaaaattagctgggtatggtggtgcatgcctgtaatcccaagctacttgggaggctaaggcaggagaatcgcttgaacccaggcagcagagattgcagtgagccgagatcacgccattgcactccagcctgggcaacaagggtgaaactccatcttaaaaaaaaattaaattaaaaaaataataataatgagtaggcaaacagggaagaatatagaggagaaaaattatcttaataagaacaatagaatttgaattgaagaaggctaggaaatatatcttaactagcctaaaatacaaaaaatcaatgttaatacttgtgttcttccaatgagatgatatttttgagggcagtacaaatttcaatagttgcttaagtgaattggtagaaaaaagtttaagattagacaaagttctgaccccaaagaacatacatttgttttaattactcccaatacaattgatcttatcaagttagatgtgctctcaacacacatcagtcttaaccataggagcctttactcacttgtttaaggcagaaactcaactgccttacacaatatccagtagctttcttcattcaatcctcaagaaaaacttaccactttgtaatttacctaaactgtttacctagagaaaacctttgtgtccttagaattagctggattactctttgagctccctcctgattggacgctgatgctgttgaatgtgtcaggaaacgtcctcagaagtggagggagctcaagagttttgtaagtggttaaattctaaggctcacaaaccaaattttttagatgtattcaaatgcccgtgaagcttagaatttaacaagagggcaaaaaaagatgagtctgttttattatccttgactatgcggggtttgaaatttaaacatttcagaaacaatttagatctatcctttgtggtgaagcttaaccagctatttcccaggtatatagagccggggaatctgttatttctttcatcaactttaattttcctggggttttagctttgtaagtgtcaccattataaaagagagttaagttgatttatagaggaaaagctaacatcatggatcttaaatgtagttatagaacactgaatgtatccactttgctggttttatggatcaggaaaaaagtgaaaactgtgccactgaaaaattactttttcagtgatttttagaaaattaaaatcaacccaggaagccccaaaaatcctgacgctgagggtagaaacatgatttatattttatcatcattctctttcaactcatgtaaacctctggtcataaaatctcaaattactttttaaggtgtctaagaaaacactctagaccaagttaacaaccctggggtttttagtcaatgcagttctagctcagtctctgtctctgcatgcttatttatctatgtgtgtatatcttactgtttcttaaatattttttaatgtctctctgactcttctccctttaactgttttttttattaaaaatgagatataccacatctgtaatcccagcactttgggaggccaaggcgggcagatgacgaggtcaggagatcgagaccatcctggctaacacggtgaaaccccgtctctactaaaaaaatacaaaaaaattagctgggcgtggtggcgggcgcctgtagtcccagctgctcaggaggctgaggcaggagaatggcgtgaacccgggaggcggagcttgcagtcagccgagatcgcgccactgcgccccagcctgggcgacacagagagactctgtctcaaaaaaaaaaagaggtatactcaatgttaaaaagtaaagagaagccatgtaggtaagatgttgtggagctagtagttaaaaaataaaactactcatgatttggtatatcttaaaataaatttttatacattataacatatgtataacatacagttatgcattaaagtaactattaatttcctatatggaagaaaatatttaaaaataatcctggtaggagtgaattcatgtgaaatgtaggcagaagtgatagtttagaatatgctttaaaacagatttcatttactttatattcaatttgattttactgattctataactggaaaaacttagaattctataaataactatttaaggtttccatatttctacattgatttctgatttctaaattgttatttcgtttgtgaaaagttcacagtagtaattgaatgttacattttaatagccacatattaatatgtcttatgagaagatctaatatatacaaccttaaaaccatggataagctgtgaagaaaaaaagtcaatgaaacttgaggaggaaaataatttatgaattaaaaatgccacgcaaattttctttttcagaattggtataaaaattctgaaagagaagctgctactcaactaggatagtatccacattttcttgtgtgagctctgactctaaggcacaaggcaagtctaagtgttcttgtgacaagcgagaacttttcagggagacatcagaccagctgtcacagtatggctgaaatctctgggccaatgcattaccaaacctttggcatcggttatatctgtaagatttacctttgtgtgtatacatgtgttccaacaattggctctttcgagggaatttatgaccacagatggtacagctcatttttcttttccttgaaaaagaaaaattacagtttaattctactggctctgtgtctttggagatcaaagatacttgactgatctgcaaaggctctgtggtaccccggttggtgtggtctggctgctgttcattctccttaacaatgaaggagctgagcctgcggcattcaagggcctcgctgttttcattaaggggatgcacttcaccaaggtcattactttccagaatggaagcagggacaccgaatggcagggatccagacacatgtgtatggagatgttgccttaggttactacgggaatcaaaacgttccccacagtaatggcataagtgtattttgacactgttttcagtaaaagtggggcctgtcacctctgatgagggtgaggggtggctctgggagatcacagattctgggtcacatctctcctgcttgatggaaactgggggcttctggtgctcctccagggcctgggtggcaggacaggccctctgctggtctgcagtgccatcatccagaccaatagcaagagacaactgcaactgggggtggtcaccctggacagcagctctgtttccactgttactggaaggagcttctttgacctccagtccttgtttgacaactgttttttgggttgttgagatctgaatgccatataaatttgaggactgcacagtctctggtgagaacacttgattcatttcagttgcaatgtgagaaaggtagtcggcgtgaagaaatcgaatcccttcctccaaacgactatgatccacaatctgttttggccctttccccgtgtacataatgtgcaacaaatagctgaatatgtcaggttggatgtcagttggttgtatttttatgcattcacttgtttggtgaataaatatcatcttgaaatagttagaaaaagcagcaagcactgctctgtgggctttgaagtaaacatctccaattgcaactgtgcaatcacacagaaaaccaaattctcgctgcatgttcagctgctggagaagaacaaggctatggctggcagtgtccattgtggttcttagctggacttaaactccaagttctgcctcccctatggtggacagcagctgaaatctctgctcctttagccttaagtgtgctgtttggaggctgctccacacatgtacagttgaggggtttgcaagaaattcaagcagagtttataaacagtgtttggggttctgccactccaacattctttctaggattttctcctgcactttccagctgcatgatcactgtgagctctgtcctcttttcttcaagagagattacaggttgttattacagttgtagccacctcttcatatcaccagctgggaccttatgccagtcactgagactttatgatgaattttcattcagacaaggagacaggaaagttggcagaggaa

SEQ ID NO: 19201 - RNA, 7675 nt, Homo sapiens
  source 1..7675: mol_type = other RNA
tgtgactgcattatgaaaattcttcacatggcccatttttacatcaattactacaaaaaatggacatttatcaagtatctgactcacaacatcaagaatgtgcctgtacaaataaatgttaacgaaattacacatttttcacactatctttttccacgattaatatgtatttccttcaattttcagtgaagacttttctaataatactattattaccttcaccccatttcctgtcctcatctactatttagatcacctacatcaaagaaataaaaataggctgggcccagtggcccatacctgtaatcccagcactttgggaggctgagataggcagatcacaaggtcaggagttcgaaaccagccttgccaacatgatgaaaccccatctctactaaaaatacaaaaattagctgggtgtggtggtgcgtgcctatagttccagctactcgggaggctgaggaagaagaatcgcttgaacctgggaggcggaggttgcagtgagccgagatcgcaccactgcactccagcctgggcaacagagcgagactccgtctcaaaaaagaaaaaaaaacaaaggtatttatttattgtttttgttccttttcctttgtgtaaacaaaaacaatatatttgggagaactttcaataaagctgaaattgacaaagttttattcccaataatgccaaagaactagtatcctccttactgaaggctaaaaagaaacagtgatgattaaattacagtagaacaggaattctagcaacagtattgtttctagttatttgtaaaaaataacaatgagttctgtcaattagttattgaatattagatagtacattactgcttttaagaacattttagaatttataggctgaaatactaaagttaataggtctagctacagaataaatgtcgtttatatggttgattttaatcaataatactgagagaacttaacacgtttaatataaatcctcacaacacccctgtgaggtaagtattgcttacacccactttacggatgggaaatcagaaagagcaagaagtaacaatctcaagagttataaataaaaaaattttttgttttcttataaggcagactgtgctgagttctgatgatacgctaataagaacaaatactaaaacagtctctatttttctccagaaaacaactgcgtgagatttcaaaagaaggaaaaattttaagctgactcaaggggaaaatgtttagtatctgcctgatacacacgaaagtgcatatgacatttccagtttcaagcttggtaatcattatgcaaactgcactatactattaggatactggctaacagtatagctccattttgtggagatgtagtcaaaaaataaaggttttagctggaagaacttttttttttttgagatggagtctcgctctgtcacccaggctggagtgcagtggtgcgatctccgctcactgcaacctctgcctcccgggttcaagctattccactgcctcagcctctcgagtagctgggattacaggtgtgtgccaccacacccggctaattttttgtatttttagtagagacgcggtttcactgtgttagccaggatggtctggatcttctgacctcgtgacccgcccgcctcggcctcccaaagtgctgggattacaagcatgagccaccacgcctggcctagctggaagaacttttaaaatacaaagcaaattttctcagtgagcaatcatgtctttaaaaaataatactcagggcacagtgttaggcatatgacagttactttaaaaaatgcctgcagacccgggcgcggtggctcatgcctgtaatctgaggcaggcagatcatgaggtcaggagctcgagaccatcctggccaacatggtgaaaccctgtctctactaaaaatacaaaaattagctgggcatggtggcacatgctcaggaggctgaggcaggagaatcacttgaattcgagaggcggaggttgcagtgagctgagattgcaccactgcactccagcctggcgacacagcacgactgtctcaaaaaaaaaaaaaaaaaaaaaaaaaaaagcctgcagaataaatgaaaacaacaataacaaaaactgggggtcagtcccacaccactattcactgcatctctggaattcagcttttgggattttttttctataaaatgaagttgatattttcccacttcctaaacagaatgaatgttttaaggaacaaggaaagagcatttgctttgaatttctaatattaaaaggaactataagaatagaaatacagttaaccactattttcttaactctcaacgaacagatatatttctgctttaaatgagtgttgtctatcacggccaatcagctgctagcaaactcttaccatttatccaaactctgccctgaggcacttgctgtcttatccaaccaaccatgtacaactctacctccaccctttagctatatacaaggatttcctgtgtcaaagaataatgagtgggcctggcacggtggctcacacctgtaatcccagcactatgggaggccgaggctggtgcatgacctgaggtcaggagttccagaccagcctgaccaagatggtgaaaccctgtctctgctaaaaacacaaaattagctgggtatggtggtgcatgcctgtaatcccaagctacttgggaggctaaggcaggagaatcgcttgaacccaggcagcagagattgcagtgagccgagatcacgccattgcactccagcctgggcaacaagggtgaaactccatcttaaaaaaaaattaaattaaaaaaataataataatgagtaggcaaacagggaagaatatagaggagaaaaattatcttaataagaacaatagaatttgaattgaagaaggctaggaaatatatcttaactagcctaaaatacaaaaaatcaatgttaatacttgtgttcttccaatgagatgatatttttgagggcagtacaaatttcaatagttgcttaagtgaattggtagaaaaaagtttaagattagacaaagttctgaccccaaagaacatacatttgttttaattactcccaatacaattgatcttatcaagttagatgtgctctcaacacacatcagtcttaaccataggagcctttactcacttgtttaaggcagaaactcaactgccttacacaatatccagtagctttcttcattcaatcctcaagaaaaacttaccactttgtaatttacctaaactgtttacctagagaaaacctttgtgtccttagaattagctggattactctttgagctccctcctgattggacgctgatgctgttgaatgtgtcaggaaacgtcctcagaagtggagggagctcaagagttttgtaagtggttaaattctaaggctcacaaaccaaattttttagatgtattcaaatgcccgtgaagcttagaatttaacaagagggcaaaaaaagatgagtctgttttattatccttgactatgcggggtttgaaatttaaacatttcagaaacaatttagatctatcctttgtggtgaagcttaaccagctatttcccaggtatatagagccggggaatctgttatttctttcatcaactttaattttcctggggttttagctttgtaagtgtcaccattataaaagagagttaagttgatttatagaggaaaagctaacatcatggatcttaaatgtagttatagaacactgaatgtatccactttgctggttttatggatcaggaaaaaagtgaaaactgtgccactgaaaaattactttttcagtgatttttagaaaattaaaatcaacccaggaagccccaaaaatcctgacgctgagggtagaaacatgatttatattttatcatcattctctttcaactcatgtaaacctctggtcataaaatctcaaattactttttaaggtgtctaagaaaacactctagaccaagttaacaaccctggggtttttagtcaatgcagttctagctcagtctctgtctctgcatgcttatttatctatgtgtgtatatcttactgtttcttaaatattttttaatgtctctctgactcttctccctttaactgttttttttattaaaaatgagatataccacatctgtaatcccagcactttgggaggccaaggcgggcagatgacgaggtcaggagatcgagaccatcctggctaacacggtgaaaccccgtctctactaaaaaaatacaaaaaaattagctgggcgtggtggcgggcgcctgtagtcccagctgctcaggaggctgaggcaggagaatggcgtgaacccgggaggcggagcttgcagtcagccgagatcgcgccactgcgccccagcctgggcgacacagagagactctgtctcaaaaaaaaaaagaggtatactcaatgttaaaaagtaaagagaagccatgtaggtaagatgttgtggagctagtagttaaaaaataaaactactcatgatttggtatatcttaaaataaatttttatacattataacatatgtataacatacagttatgcattaaagtaactattaatttcctatatggaagaaaatatttaaaaataatcctggtaggagtgaattcatgtgaaatgtaggcagaagtgatagtttagaatatgctttaaaacagatttcatttactttatattcaatttgattttactgattctataactggaaaaacttagaattctataaataactatttaaggtttccatatttctacattgatttctgatttctaaattgttatttcgtttgtgaaaagttcacagtagtaattgaatgttacattttaatagccacatattaatatgtcttatgagaagatctaatatatacaaccttaaaaccatggataagctgtgaagaaaaaaagtcaatgaaacttgaggaggaaaataatttatgaattaaaaatgccacgcaaattttctttttcagaattggtataaaaattctgaaagagaagctgctactcaactaggatagtatccacattttcttgtgtgagctctgactctaaggcacaaggcaagtctaagtgttcttgtgacaagcgagaacttttcagggagacatcagaccagctgtcacagtatggctgaaatctctgggccaatgcattaccaaacctttggcatcggttatatctgtaagatttacctttgtgtgtatacatgtgttccaacaattggctctttcgagggaatttatgaccacagatggtacagctcatttttcttttccttgaaaaagaaaaattacagtttaattctactggctctgtgtctttggagatcaaagatacttgactgatctgcaaaggctctgtggtaccccggttggtgtggtctggctgctgttcattctccttaacaatgaaggagctgagcctgcggcattcaagggcctcgctgttttcattaaggggatgcacttcaccaaggtcattactttccagaatggaagcagggacaccgaatggcagggatccagacacatgtgtatggagatgttgccttaggttactacgggaatcaaaacgttccccacagtaatggcataagtgtattttgacactgttttcagtaaaagtggggcctgtcacctctgatgagggtgaggggtggctctgggagatcacagattctgggtcacatctctcctgcttgatggaaactgggggcttctggtgctcctccagggcctgggtggcaggacaggccctctgctggtctgcagtgccatcatccagaccaatagcaagagacaactgcaactgggggtggtcaccctggacagcagctctgtttccactgttactggaaggagcttctttgacctccagtccttgtttgacaactgttttttgggttgttgagatctgaatgccatataaatttgaggactgcacagtctctggtgagaacacttgattcatttcagttgcaatgtgagaaaggtagtcggcgtgaagaaatcgaatcccttcctccaaacgactatgatccacaatctgttttggccctttccccgtgtacataatgtgcaacaaatagctgaatatgtcaggttggatgtcagttggttgtatttttatgcattcacttgtttggtgaataaatatcatcttgaaatagttagaaaaagcagcaagcactgctctgtgggctttgaagtaaacatctccaattgcaactgtgcaatcacacagaaaaccaaattctcgctgcatgttcagctgctggagaagaacaaggctatggctggcagtgtccattgtggttcttagctggacttaaactccaagttctgcctcccctatggtggacagcagctgaaatctctgctcctttagccttaagtgtgctgtttggaggctgctccacacatgtacagttgaggggtttgcaagaaattcaagcagagtttataaacagtgtttggggttctgccactccaacattctttctaggattttctcctgcactttccagctgcatgatcactgtgagctctgtcctcttttcttcaagagagattacaggttgttattacagttgtagccacctcttcatatcaccagctgggaccttatgccagtctataatcccggctactcgggaggctgaggcgggagaatcgcttgaacccaggaggcagaggttgtggtgagctgagattgtgtcattgcactccagtctgggcaacaagagtgaaactccatctcaaaaaaaaaaagaaaaagaaaaaaaagaatcaaaagtgctcctaaactggcaggatgggcatgggtgggggggtggaggaacacactattttcagacttcttttcaaatagtatttaggaaaaagaaatatttactctcttactccattacacctagattggatttcataacacctaaaaatgatacagaaattctaaatctgaaaatactgtttgaggtaaaatctgctgtaattccagacatctgcttattaagatctactgagaatgttagcaaagagggtatggagggggtagatgaaacaggaagagtagttatgctctagaaacctttaatggaactgggaaacgttagtttggggcctcctgcctgttggcagacatagccaacctccaagcacctctaattcccatctaaccaacattacattgtaggatgcctgataaagccaagcacacaagaatactaacaacagtaagcacaaattgttaatagacctttaaaaaaaatcagaacccggagaaagaaaggaaaagattcctctcagtccattaaagacaaaccaaatttctaaaagaaaaaataaggtactcaaaggacaggagaaagatggaaaattataatgctagtacagacctagaatacagtacaggcaagagtaactaaaacttctggatacaagtaaaccaatacttctttcgcaatggaagtatactcccatgaacacactactcaagtgggctaataaaaacctttgcttaaagtgcttggagatttcagaaaaaataaaacatccatgcatgactgatttgtaaccagagaagaaatgaattagaaaaatataaaaaataactgaacactctaagcactttttctcccaataaag

SEQ ID NO: 19202 - RNA, 5168 nt, Homo sapiens
  source 1..5168: mol_type = other RNA
tgtgactgcattatgaaaattcttcgctttttcacactgccttaaattctcccaataaaatgaaattcatctatgctaactcatcttcttttagagcaggggtctttaaccttttgtgtgggcctgttgccagcctgggaaacctatggactcctccaaatagcacatttcaaagaaggaggtaaaatagataagatttctaaggaagccagtaatattaaaatatagttaccaaaatatttttaaatacttgcatttgcaatatagtaatatatgtactttgttagcacattaaatgacaagatctagtggcagcctaaacattaccatcattccaaaatatgagctgaaacaatatttcaaatgcctgcaacaattgtaaagtgatatcaagatgcatgtgctttctgttggtgacaaagtcacaagccacctgacatccctataatctattcctcacttgcaattgaaagtaatacttatttatttatttatttatttatttattgagacagagttttgttcttgttgccaaggctggagcaatggcgtgatcttggctcactgcaacctctgcctcctgggttcaagcgattctcctacctcagccccccaggtaactgggattacagacacccaccaccacactcggttaattttgtatttttagtagagacagggtttctccatgttggtcaggctggtctcaaactcctgacctcaggtcatctacctgcctaggcctcccaaagcactgggattacaggcatgagccaccgcgcctggccaatactaaattttaattagaagttagtgagaatgaagacctaattttccatccgacttcatagattgaattctgtctatggaacccagtttgagaacccctagtttaacaagtgatttacacctagtgtgaaatttttaatcagatttatttcagttaactctgagactaccccctcacacacaggaaggtgaaaagaaggcttggagcaccagctagggaggacagggaggacaggaaggcctctgagggtgggcagagctggagaatggacgcaaaatcaagatgggaaggagccgcctcaagatttcatgggtgtggtggtgggggacctggtttagcttctctcctgttctagacagctctacagagacagagctcaagggagcgttttctacaggttccccgtccggaatgcccagctcctatgggccctaactgaggcactagaggaaggatggacgagcagagccaggagtgggcacgcctttgtgcccagccttctaggtctcctgggttgggcaggacacagagcaaaaccccttccccaactcacacagctccagtcagctgctggctgttggcagggcaaggcccaccccccagagcccaccccccacaagctgtcctctgagacctcactgccacaagggtgaactcccacccagggttctgggctttgcttcagggtgctttgctctctgcccagaaaaacatcccccagaaaaggaaagacaaaggggtggttacctgctgacctccccacaggtttaccctgaaccgaggcccagagaggggaagggacctggccgaggtctccaggaggtcggggatgtgctggtgccctgccagccctgggcttctgccctctcctcccctcagaccagctcccaggggaatgtgaagaaaggagggccacaggcaccagtgaggccaccctggggacaaacaggtggttagaggcagctcagacctcagacattatccagggcacttttataaacaggaaaaatgtggccgggcaaagagtagaggctcctgctaacaccaccagctggtaggtggtgaaaccgcacattagcccttggatacgtgattccccagcctgaccatgtattagaatcacctggattgctcactcaaaacatgtctgctggcatcaggcctgacgctacagaatcagcagctctgtagaggggcctagcatctgcaccatcaatgagcagcccagatagctccagtgtgcagccaggtttggggcccatggcactgagccattcccaagtatagcctaggaagagatcctgagctgtgggcagagggagggaagagctcggggagagcatctggttcaagacacttgattcacttctttttgttggttacatctaaaactaaggatgggtggctggggcgggagccagaatttagtcttagctgagctgggggccaagtggagtgtgccctgaggcttgggacaggagcatgtgggtgggacttcccatccctgacccccacccttatcctgcccttcagtggctatgagagatggcaaccaggtcacagggctggactttgtcgtctcaagccccaaggagtaaagctgggcagggctttggcctggatcaatggccttaggactcagcccacacgtaagtggggtgagtgcagcgcaggacagcgtctgtgttctccagaatctgtcttcactctgactcaatcaccaggggattctgcaccccggtcttagtagaaatgcacctctgagtttcagtttagctccctgcccatcacgtcaccacagtggtccatggaatctgatgcgtcccgcagctcagcccttccaccttgcccagtgtgccctcctcaccgacagctcccgctcccagccccctgcctctccacttctagggctgcaatctgcttctgtctcctccttggatcacacacttggacccagctccctgttttgctctgggctctgctttctcttgtggagttggtgtcaccaaggtctcaggtgagaaactccttcctgccgtgtgactgtctgcggagaagtggggcaccctgtgggggatgggataaaaggggtgtccatgcactccaagctgtggccccttgggttatagatcagtttttatccaaagacccttgtgatgagtccaggcttgagtttagtccctattccaagacatgagtttgcatttcttctttcattggaagatgacatttcaaaaactttccttggctttcaaaaagcttagcattagatgatagaaatcagctcatgggccccttgcttttaggtgatgtttattctgtttcatccttgaatatcaatttgtcgtgcatccaaactcgctatgtcaaaccttttgaatgaatgcagggtatacgtcttaaattaactccataaaacttgagtagctagcatagaaatttaaggagtatgtgagcaggacgttatttcccccagttcacctggccttcttgcactcagtgctttcagcagctgtagggcgttttgtgtgaagttattgacatgaagggatgggagtgaaatcagttatcagataacaaacaagtgctctcatgtctgatgggtagaagagggggcagtcacttcctcaacacgtgagatgacactgactttgcagtgagctctccccaggaaagaggaggagccctgggcaggcgggatggggaaggaccctgcgggaaccatggaggaagtttggagctccctgctggagcatgcagcctgcagggctgcagacagaaaacctcgttccgccctggtttggaggtttgctggctgtgtgaaccttgacaatgtacctctcctctctgaatgtcagttttctcaactgtataaaggaaacagtaatagctactttggttgtttgtgagggtcaaacgcaacacacatacagaagccctataaaatgcaaatacttttatcctcagttctgtgcagaggccactgggtttacttatgtattgattctctctgtcctctctcccacccctatcctcctccccacatgccctcaccttcttggttttgccctcccagaagtaggggagtacagttattcggttagagcagttacactcttgggggtttgcttcagccaagaagacagtgagccgtggggatcgtaattaatggaggcagactgattagaaatgagccactggatcggggtgtttgctgattcatcttggaaacactaggtcctgagtcccaatcggcttctaccacattggtcattgttctacttctgcactgttctgtgcagaagcacctgtgtttactcataaacttacatattgattctgtctcttctcctacccccatcctcctcctcatatcctaagtgctcagcatggtgctaggtacacagcaggcactaaataaatgtttctttaattaaattcccattgatagctacactgtgtgaatggtactttcatgatagatttttctgtcaccccttgagtttctgcagacattaggattcacagagaatgctgtgttccaagtcaaaatattcattatgacacatgctgtttgcaatttccacaatccaagtcattacccataatgtgcttggggaggaaaacaaacctctcttggaaatgctgccgtgtaggggttggggtcagagctctgcctccaaactccgtgacctttcctggagcacttctctgttgaccgtgaccaggaggcattccaggcttgggagcaccagccagaggacccccagccagatgagatccagtcacacatctcaggcaaggtcagacagcccagggaccccaggaatgcagcccaccagatgtgtgctaaggacagcatgcttatttggaacgctgggtaacctgtcatgcattgcagaaacatggagatccccctgtttgacattttctcctgttaatcccattttttaaaaatagctgtgcggtgtagaagtttcctcctggtctcattaggtgtctccttataattgcaggttttaaagcaagctcaaggcagagcctttcagagaaattaaacttcaggtgttgtctaggaccaggggcagccaattatcccattacagaaaccatgtacttggaatactgattgtgcttcagaataatccaattccattcactgtgggctgggggatgcgcctggcaatagaatttcaatagcgaagagtctcagtttatcctcatgaagctttcagtcttcttcctggggttagttcccttcttcttgaaatatattcactagaagttcctcagtggggatattttggtggtaacagggtcaggactagagtgaggcacagttccatatggctggggaggcctcacaatcatggtggaa

SEQ ID NO: 19203 - RNA, 5460 nt, Homo sapiens
  source 1..5460: mol_type = other RNA
tgtgactgcattatgaaaattcttctagtgtgatttacagctctgtcaggtcagttattttcttctttatactcactattttgtctgttagttcctgcaatgttttacaatgatttttagcttccttgtattggattacaacatacttctttcactcaatgaactttgttcctacccatatcctgaactctgcttgtatcatttcagacatctcagcctcagcccagttctgaacacttgctggagagttgatgcagtcatttggagaaaagaaggtatgctgaatttttgagttttcagtgttcttgcacagagtctttttctcatctttatgggcttatccatcttcaatctttgaggttgctgacctttggacagggtatttttcctttattatatctgatgaccttgaggatttgattgtggtgtaaggtggattcagccaacaggttttgtttttggaggattttaaggggccaacatgcagctcccaattcttggactgtgtgctttaactctggggaacttgtattgggccacaactttgtcctctggctcctcgaggtttggagtccactgcactgaggggaccaaagtgcagcagctgtggcagaatgctagcagatgcaaaagtccctgcctccctgtgggcattcacccagtggtggaggcaaaacagctggggtgtgggccacgggcccctgctgactgtgtgtgctgttgcactggaggtagtgctggtttggggtgggtggctggccagtgaaggtgccttctctgatcccccccaagcaacagtggtcactcagggtataagaaggtcccttttcctctgcacagcattacctcaagggtgagatgctagcaggggtggggtttttggttctgtgcccaccatggcttcatcttcagtggcagttggtgtgggttggggtgtgtgctgcattcccatatgctgttagggcaagtacaacaaaacccacctgtgtaaacacacacagcaaagtgatgtaggaagtttccatataaagggctgcagtatggaatggtaatgtgcaggctagtgcgtggctgtagaggtcaccttgctgcagctctccactgatcaggcacggtccgcttgtacagaagctatggtgtgggcacccgaaagtgccctctaagcaggtgtggcctggctggggtcctgggagaggcaagcagactaaggggtgctgaggtcagaccagccccatctcatgtgcaagactgcccagcacagatcaggtctcagaggagaactctctcaaaagtgaatcctcagcacagcacaactgctctacacaaacgtggccagacttcttttttaagcaagtccccttttttacgaagagaactcttagacctgatctgtgctgggcaatcttgcacgtgagatggggctggtctgacctcagcactcctaaagtgctgggataaagtgtctcataagagcaagtggagcctagagacatagctgtccctgccctccaggctccacatcagctgacttgctgctccactactttccttgtctcctgggggctccaccccagagaggtgtaagttagcagttacttaatgtaatcaccccaggatggagggtctgtgttgtgggcccaagccacggttccttgtctggtgatgagcagtaaggggtgtgttgtacctgtggaagatggactgacttgttccttgtgtcaactgcagcttgttggaggtgtcaatatggcacttagggtctttgctcccttgatattctgagggtagcaagggcagttccactgcagaggcagtggcagagaggatttctgttgctcctggaagctctgtccagggagttgctgagttgctactggcttgaaagctcaagtggggggctggctggagacccaggccaggaagacctgcccatcgaggagatatggaaatgggcacccacataacagtctggccacttttctgtggggctgccgtggtatgctgggggtccactccagtcgccaattgcctcgtattttccagtggctgaaggtatcagcagtgaagcctgagaaaaagcaaagacgatagcctgcccttccctctgggagctctgtacctctgaggtatgaacctgttgccaatctcaacacacctgtaggatgtgactggaagcaagttgagaagtcttgcctagtaaggaggaacaggaatagggacttgtttaaaaaagaagtctggccacgtttttgtagagtggctatgctgtgtggggggttcacttcagcccctggtctcctcagacactctgaaactctaagactgaactggctgagtcatccaaacagcaaagatgacagtctggtcctccccctgggagctctgactcaggaggcctgaaacctctgtgagccagagaacagcagtgaaggtggctggagaccctggttgaaaggctccacccagtgattagaaatgtggttggggactggcttaaacaagaatctggccacgttttcgcagggtggctgttctgtgctgaggtaccacttccacccctggtcagcttgggctctccaaagcccacaggccagaagggctagttgcccaaacaacaaaggtcatggcccacccctctctctgggaactctgtcccaggaaggtttcaaatctccattggccagggaacactggtgggtgtagctggaggcctcaggtgggagatcctgtccagtgacgaggaacaggatcagaggcctgcttacagaagcattctggacatgatttggtaaagcagctgtgctatgccacaggatctcttctgcccctggtgggtttgtactctccaaagcccgcacgctggaatcgctaagttgcccaaacaggaaagatggtggcctgcctcatcttttctctcagaatttatcctgtgtgatggagcttaatttttaggttgttaattttactgtcagcgttagagttgttcagaaagaatctcactgttatcttttaggtgagatatatgagaattcattttctcctgtaaataaacctgttcatgtttgttctctggaaagaagtccctttcagctatctgactttgatcacaatcatgtagagcagtagtcagtctacaatgacatgattgaatttccatttccagtgtttcctagctgtgtcttacattctccagttcagaactgagcattctcagttgtcaaaatcctaagctgtccactgtacttaaatattggttttcgttaatgcttcttcattcaattgcatagcccttagaagtttatcagtcttttctttcacactttcaatttcctccaaaattttattttcccttagctggttctgatgttttgtttcatctagttccagtctccagaaattagcatggcaatttcttcctgcaacatgctgttttcacgcaagagatcttcttctttcttatgactaagagaaagctcagaattcattttcttttcagccacttctatctgcttttgtttattagtcagaatctcatcttgtgatattccagtgttctgttcttcagaaagttgtttccgggtatcattttgttcgtcactgtgatactcttcattctcagtgtcaggaaattgctgattttcaggttttctgctcctcctttgtggaattaatccatcatcaccattgccagcactggcaccattagtcaggttttctggtaatcccacaggattacttccatgcttctttatttcttcttcaacctctctatcacagtccttatttatttctggttcttgagacattttctctggctggctattttcactgactttaagcctttgtgactcttcctctgatgttagctttaagtcttgttctggattgctgttttcagaagagatttttagcatctgtttttctttatagtcagaaagtaattcacaaattacatgatgatgactagaaacagcatactctctggccgtctgtccagatagatcttgagaagatacatcaacattttgctcaaggagaagattgactatacttgctgatccacaacatacagcaagtatgagggcagttcttccatatctatcaagtgcatttaaattagcttttttcttgattaaaaatttcaccacttgctgtttttgttcatgtacgccaagcaaaagtggtgtgaggccacacttgttttttgattcaatatcagcaccatataagagcagtgctttggccattaatttatcttcattgtggacagcatagtgtagagtggtatttccatactcatctggaatattttgatcagcgccatgttccagcaacattaacacacattcatcttcctggcattgtacggcctttatcagagctgtcctttttttgttgtcaaggacattaagttgacatcgtctgtccagcaggagttgtactacttctgaatttccattggcagaggccaaatgtagagcagtcctcttttgcttgtccctcttgttcatgtccgtgtccctgagcatgacgatgagatcctttctggggaccttaccccaccaggcagctctgtggagcttgtccagatcttctcgacggacgtggtacctcggctccatgaaggcgctgtcgtcgtagtctccccaagcgcccacgttgctcttgccgctccccctgcagcaggggaagcagtgacagcaccacttgcccatcttgctcctgagcgtcttcataaaggagttgtcatggtctccagaagtgcccacgttgctcgtgccgctccccctgcagcaggggaagcagtggtggcaacacttgcccatcttgctcctgagcatcttcataaaggagtcgtcgtggtctccagaagtgcccatgttgctcttgccgctccccttgcagcaggggaagcggtggtgaaaccacttgcccatcttgctcctgagatcgaatggcttcttcacagcagaggcagcgggcattgaacaaacctcagtcaccatctgcttttaacagcccggggaggccggtagtagcgaacagatcgcgtctaccaaccagtttcaccaactagcaggaaaccctgggtttccaatctgtttgaagagaaaggtcaatcccagccaaaacttgccaaccccagcaagggagcccagtccaccccacccagggaaaacccacacccacccggggaaagcccacgcccaccagggggacccaacgcccaccccaggaaaggccaagccccccctcccaaggaaacacccagcccagtcaagggaatgccaaacccagcagagaaaaagtcaagcccagcaaaggaatgcgagggaggaaacgccaatccaagcaagaaacaccaggcaaagcgactaacgccaagccaagctaggaacgcaaggccaagcgaggaacgcaaagcgaagcgtacccgttacaggtaagccaagccgttat

SEQ ID NO: 19204 - RNA, 5389 nt, Homo sapiens
  source 1..5389: mol_type = other RNA
tgtgactgcattatgaaaattcttctagtgtgatttacagctctgtcaggtcagttattttcttctttatactcactattttgtctgttagttcctgcaatgttttacaatgatttttagcttccttgtattggattacaacatacttctttcactcaatgaactttgttcctacccatatcctgaactctgcttgtatcatttcagacatctcagcctcagcccagttctgaacacttgctggagagttgatgcagtcatttggagaaaagaaggtatgctgaatttttgagttttcagtgttcttgcacagagtctttttctcatctttatgggcttatccatcttcaatctttgaggttgctgacctttggacagggtatttttcctttattatatctgatgaccttgaggatttgattgtggtgtaaggtggattcagccaacaggttttgtttttggaggattttaaggggccaacatgcagctcccaattcttggactgtgtgctttaactctggggaacttgtattgggccacaactttgtcctctggctcctcgaggtttggagtccactgcactgaggggaccaaagtgcagcagctgtggcagaatgctagcagatgcaaaagtccctgcctccctgtgggcattcacccagtggtggaggcaaaacagctggggtgtgggccacgggcccctgctgactgtgtgtgctgttgcactggaggtagtgctggtttggggtgggtggctggccagtgaaggtgccttctctgatcccccccaagcaacagtggtcactcagggtataagaaggtcccttttcctctgcacagcattacctcaagggtgagatgctagcaggggtggggtttttggttctgtgcccaccatggcttcatcttcagtggcagttggtgtgggttggggtgtgtgctgcattcccatatgctgttagggcaagtacaacaaaacccacctgtgtaaacacacacagcaaagtgatgtaggaagtttccatataaagggctgcagtatggaatggtaatgtgcaggctagtgcgtggctgtagaggtcaccttgctgcagctctccactgatcaggcacggtccgcttgtacagaagctatggtgtgggcacccgaaagtgccctctaagcaggtgtggcctggctggggtcctgggagaggcaagcagactaaggggtgctgaggtcagaccagccccatctcatgtgcaagactgcccagcacagatcaggtctcagaggagaactctctcaaaagtgaatcctcagcacagcacaactgctctacacaaacgtggccagacttcttttttaagcaagtccccttttttacgaagagaactcttagacctgatctgtgctgggcaatcttgcacgtgagatggggctggtctgacctcagcactcctaaagtgctgggataaagtgtctcataagagcaagtggagcctagagacatagctgtccctgccctccaggctccacatcagctgacttgctgctccactactttccttgtctcctgggggctccaccccagagaggtgtaagttagcagttacttaatgtaatcaccccaggatggagggtctgtgttgtgggcccaagccacggttccttgtctggtgatgagcagtaaggggtgtgttgtacctgtggaagatggactgacttgttccttgtgtcaactgcagcttgttggaggtgtcaatatggcacttagggtctttgctcccttgatattctgagggtagcaagggcagttccactgcagaggcagtggcagagaggatttctgttgctcctggaagctctgtccagggagttgctgagttgctactggcttgaaagctcaagtggggggctggctggagacccaggccaggaagacctgcccatcgaggagatatggaaatgggcacccacataacagtctggccacttttctgtggggctgccgtggtatgctgggggtccactccagtcgccaattgcctcgtattttccagtggctgaaggtatcagcagtgaagcctgagaaaaagcaaagacgatagcctgcccttccctctgggagctctgtacctctgaggtatgaacctgttgccaatctcaacacacctgtaggatgtgactggaagcaagttgagaagtcttgcctagtaaggaggaacaggaatagggacttgtttaaaaaagaagtctggccacgtttttgtagagtggctatgctgtgtggggggttcacttcagcccctggtctcctcagacactctgaaactctaagactgaactggctgagtcatccaaacagcaaagatgacagtctggtcctccccctgggagctctgactcaggaggcctgaaacctctgtgagccagagaacagcagtgaaggtggctggagaccctggttgaaaggctccacccagtgattagaaatgtggttggggactggcttaaacaagaatctggccacgttttcgcagggtggctgttctgtgctgaggtaccacttccacccctggtcagcttgggctctccaaagcccacaggccagaagggctagttgcccaaacaacaaaggtcatggcccacccctctctctgggaactctgtcccaggaaggtttcaaatctccattggccagggaacactggtgggtgtagctggaggcctcaggtgggagatcctgtccagtgacgaggaacaggatcagaggcctgcttacagaagcattctggacatgatttggtaaagcagctgtgctatgccacaggatctcttctgcccctggtgggtttgtactctccaaagcccgcacgctggaatcgctaagttgcccaaacaggaaagatggtggcctgcctcatcttttctctcagaatttatcctgtgtgatggagcttaatttttaggttgttaattttactgtcagcgttagagttgttcagaaagaatctcactgttatcttttaggtgagatatatgagaattcattttctcctgtaaataaacctgttcatgtttgttctctggaaagaagtccctttcagctatctgactttgatcacaatcatgtagagcagtagtcagtctacaatgacatgattgaatttccatttccagtgtttcctagctgtgtcttacattctccagttcagaactgagcattctcagttgtcaaaatcctaagctgtccactgtacttaaatattggttttcgttaatgcttcttcattcaattgcatagcccttagaagtttatcagtcttttctttcacactttcaatttcctccaaaattttattttcccttagctggttctgatgttttgtttcatctagttccagtctccagaaattagcatggcaatttcttcctgcaacatgctgttttcacgcaagagatcttcttctttcttatgactaagagaaagctcagaattcattttcttttcagccacttctatctgcttttgtttattagtcagaatctcatcttgtgatattccagtgttctgttcttcagaaagttgtttccgggtatcattttgttcgtcactgtgatactcttcattctcagtgtcaggaaattgctgattttcaggttttctgctcctcctttgtggaattaatccatcatcaccattgccagcactggcaccattagtcaggttttctggtaatcccacaggattacttccatgcttctttatttcttcttcaacctctctatcacagtccttatttatttctggttcttgagacattttctggattgctgttttcagaagagatttttagcatctgtttttctttatagtcagaaagtaattcacaaattacatgatgatgactagaaacagcatactctctggccgtctgtccagatagatcttgagaagatacatcaacattttgctcaaggagaagattgactatacttgctgatccacaacatacagcaagtatgagggcagttcttccatatctatcaagtgcatttaaattagcttttttcttgattaaaaatttcaccacttgctgtttttgttcatgtacgccaagcaaaagtggtgtgaggccacacttgttttttgattcaatatcagcaccatataagagcagtgctttggccattaatttatcttcattgtggacagcatagtgtagagtggtatttccatactcatctggaatattttgatcagcgccatgttccagcaacattaacacacattcatcttcctggcattgtacggcctttatcagagctgtcctttttttgttgtcaaggacattaagttgacatcgtctgtccagcaggagttgtactacttctgaatttccattggcagaggccaaatgtagagcagtcctcttttgcttgtccctcttgttcatgtccgtgtccctgagcatgacgatgagatcctttctggggaccttaccccaccaggcagctctgtggagcttgtccagatcttctcgacggacgtggtacctcggctccatgaaggcgctgtcgtcgtagtctccccaagcgcccacgttgctcttgccgctccccctgcagcaggggaagcagtgacagcaccacttgcccatcttgctcctgagcgtcttcataaaggagttgtcatggtctccagaagtgcccacgttgctcgtgccgctccccctgcagcaggggaagcagtggtggcaacacttgcccatcttgctcctgagcatcttcataaaggagtcgtcgtggtctccagaagtgcccatgttgctcttgccgctccccttgcagcaggggaagcggtggtgaaaccacttgcccatcttgctcctgagatcgaatggcttcttcacagcagaggcagcgggcattgaacaaacctcagtcaccatctgcttttaacagcccggggaggccggtagtagcgaacagatcgcgtctaccaaccagtttcaccaactagcaggaaaccctgggtttccaatctgtttgaagagaaaggtcaatcccagccaaaacttgccaaccccagcaagggagcccagtccaccccacccagggaaaacccacacccacccggggaaagcccacgcccaccagggggacccaacgcccaccccaggaaaggccaagccccccctcccaaggaaacacccagcccagtcaagggaatgccaaacccagcagagaaaaagtcaagcccagcaaaggaatgcgagggaggaaacgccaatccaagcaagaaacaccaggcaaagcgactaacgccaagccaagctaggaacgcaaggccaagcgaggaacgcaaagcgaagcgtacccgttacaggtaagccaagccgttat

SEQ ID NO: 19205 - RNA, 4789 nt, Homo sapiens
  source 1..4789: mol_type = other RNA
tgtgactgcattatgaaaattcttctagtgtgatttacagctctgtcaggtcagttattttcttctttatacttgctattttgtctgttagttcctgcaatgttttacaatgatttttagcttccttgtattggattacaacatacttctttcactcagggaactttgttcctacccatatcctgaactctgcttgtatcatttcagacatctcagcctcagcccagttctgaacacttgctggagagttgatgcagtcatttggagaaaagaaagcatgctgaatttttgagttttcagtgttcttgcacagagtctttttctcatctttatgggcttatccaccttcaatctttgaggctgctgacctttggacagggtatttttcctttattatatctgatgaccttgaggatttgattgtggtgtaaggtggattcagccaacaggttttgtctttggaggattttaaggggccaacatgcagctcccaattcttggactgtgtgctttaactctggggaacttgtattgggccacaactttgttctctggctcatcgaggtttggagtccaccgcactgaggggaccaaagtgtggcagctgtggcagaatgctagcagatgcaaaagtccctgcctccctgtgggcattcacctagtggtggaggcaaaacagctggggtgtgggccagggggcccctgctgactgtgtgtgctgttgcactggaggtagttctggtttggggtgggtggctggccagtgaaggtgccttctctgatcccccccaagcaacagtggtcactcagggtataagaaggtcccttttcctctgcacagcattacctcaagggtgagatgctagcaggggtggggtttttggttctgtgcccaccatggcttcatcttcagtggcagttggtgtgggttggggtgtgtgctgcattcccatatgctgttagggcaagtacaacaaaacccacctgtgtaaacacacacagctaagtgatgtaggaagtttccatataaagggctgcagtatggagaggtaatgtgcaggctggtacgtggctgtagaggtcaccttgctgcagctctccactgatcagccacggtctgcttgtacagaagctatggtgtgggcacccaaaagtgccctctaagcaggtgtggcctggctggggtcctgggagaggcaagcagactaaggggtgctgaggtcagaccagccccatctcatgtgcaagactgcccagcagagatcaggtctcagaggagaactctctcaaaagtgaatcctcagcacagcacaactgctctacacaaacgcggccagacttcttttttaagcaagtccccctttttaggaagagaactcttagacctgatctgtgctgggcaatcttgcacgtgagatggggctggtctgacctcagcactccttaagtgctgggataaagtgtctcataagagcaagtggagcctagagacatagatgtccctgccctccaggctccacatcagctgacttgctgctccaccactttccttgtctcctgggggctacaccccagagaggtgtaagttaggagttacttaatgtaatcaccccaggatggagggtctgtgctgtgggcccaagccagggttccttgtctgttgatgagcagtaaggggtgtgttgtacccgtggaagatggactgacttgttccttgtgtcaactgcagcttgttggaggtgtcaatatggcacttagggtctttgctcccttgacattctgagggtagcaagggcagttccactgcagaggcagtggcagagaggatttctgttgctcctggaagctctgtccagggagttgctgagttgctactggcttgaaggctcaagtggggggctggctggagacccaggccaggaagacctgcccatcatggcccacccctctctctgggaactctgtcccaggaaggtttcaaatctccattggccagggaacactggtgggtgtagctggaggcctcaggtgggagatcctgtccagtgacgaggaacaggatcaggggcctgcttacagaagcattctggccatgatttggtaaagcagctgtgctatgccacaggatctcttctgtccctggtgagtttgtactctccaaagcccgcacgctggaatgactaagttgcccaaacaggaaagatggtggcctgcctcatcttttctctcagaatttatcctgtgtgatggagcttaatttttaggttgttaattttactgtcagcgttagagttgttcagaaagaatctcactgttatcttttaggtgagatatataagaattcattttctcctgtaaataaacctgttgatgtttgttctctggaaagaagtccctttcagctatctgactttgatcacaatcatgtagagcagtagtcagtctacaatgacatgattgaatttccatttccagtgtttcctagctgtgtcttacattctccagttcagaactgagcattctcagttgtcaaaatcctaagctgtccactgtacttaaatactggttttcgttaatgcttcttcattcagttgtatagcctttagaagtttttcttttacactttcaatttcctccaaaattttattttcccttagctggttctgatgttttgtttcatctagttccagtcttagcatggcaatttcttcccgcaacatgctgttttcacgcaagagatcttcttctttcttatgactaagagaaagcttagaattcatttccttttcagccacttctatctgcttttgtttattagtcagaatctcatcttgtgatattccagtgttctgttcttcagaaagttgtttctgggtatcattttgttcgtcactgtgatactcttcattctcagtgtcaggaaattgctgattttcaggttttctgctcttcctttgtggaattaatccatcatcaccattgccagcactggcaccattagtcaggttttctggtaatcccacaggattacttccatgcttctttatttcttcttcaacctctctatcacagtccttatttatttctggttcttgagacattttctctggctggctattttcactgactttaagcctttgtgactcttcctctgatgtcagctttaagtcttgttctggattgctgttttcagaagagatttttagcatctgtttttctttatagtcagaaagtaattcacaaattacatgatgatgactagaaacagcatactctctggccgtctgtccagatagatcttgagaagatacatcaacattttgctcaagtagaagattgactatacttgctgatccacaacatacagcaagtatgagggcagttcttccatatctatcaagtgcatttaaattagcttttttcttgattaaaaatttcaccacttgctgtttttgttcatgtacgccaagcaaaagtggtgtgaggccacacttgttttttgattcaatatcagcaccatataagagcagtgctttggccattaatttatcttcattgtagatagcatagtgtagagcggtatttccatactcatcttgaatatttccatcagcgccatgttccagcaacattaacacacattcatcttcctggcattgtacggcctttatcagagctgtcctttttttgttgtcaaggacgttaagttgacatcgtctgtccagcaggagttgtactacttctgaatttccattggcagaggccaaatgtagagcagtcctcttttgcttgtccctcttgttcatgtcagtgtccctgagcatgacgatgagatcctttctggggactttaccccaccaggcagctctgtggagcttgtccagatcttctcgacggacgtggtacctcggctccatgaaggcgctgtcgtcgtagtctccccaagtgcccacgttgctcttgccgctccccctgcagcaggggaagcagtgacagcaccacttgcccatcttgctcctgagtgtcttcataaaggagttgtcatggtctccagaagtgcccacattgctcgtgccgctccccctgcagcaggggaagcagtggtggcaacacttgcccatcttgctcctgagcgtcttcataaaggagtcgtcgtggtctccagaagtgcccatgttgctcttgccgctccccctgcagcaggggaagcggtggtggcaccacttgcccatcttgctcctgagatcaaatggcttcttcacagcagaggcagcgggcattgaacaaacctcagccaccatctgcttttaacagccaggggaggccggtagtagcgaacagatcgcgtctaccaaccagtttcaccaactagcaggaaaccctgggtttccaatctgtttgaagagaaaggtcaatcccagccaaaacttgccaagcccagcaagggagcccagcccaccccacccagggaaaacccacacccacccggggaaagcccacgcccaccagggggaccccacgcccaccccaggaaaggccaagccccccctcccaaggaaacacccagcccagtcaagggaatgccaaacccagcagagaaaaggtcaagtccagcaaaggaatgcgagggaggaaacgccaatccaagcaagaaacaccaggcaaagctactaacagccaagccaagctaggaacgcaaggccaagcgaggaacgcgaagcgaagtgtacccgttacaggtaagccaagccgttatgcgcgtgcggggcgcgcgtgcggggcgcgcgcc

SEQ ID NO: 19206 - RNA, 4448 nt, Homo sapiens
  source 1..4448: mol_type = other RNA
tgtgactgcattatgaaaattcttctagtgtgatttacagctctgtcaggtcagttattttcttctttatacttgctattttgtctgttagttcctgcaatgttttacaatgatttttagcttccttgtattggattacaacatacttctttcactcagggaactttgttcctacccatatcctgaactctgcttgtatcatttcagacatctcagcctcagcccagttctgaacacttgctggagagttgatgcagtcatttggagaaaagaaagcatgctgaatttttgagttttcagtgttcttgcacagagtctttttctcatctttatgggcttatccaccttcaatctttgaggctgctgacctttggacagggtatttttcctttattatatctgatgaccttgaggatttgattgtggtgtaaggtggattcagccaacaggttttgtctttggaggattttaaggggccaacatgcagctcccaattcttggactgtgtgctttaactctggggaacttgtattgggccacaactttgttctctggctcctcgaggtttggagtccaccgcactgaggggaccaaagtgcggcagctgtggcagaatgctagcagatgcaaaagtccctgcctccctgtgggcattcacctagtggtggaggcaaaacagctggggtgtgggccagggggcccctgctgactgtgtgtgctgttgcactggaggtagttctggtttggggtgggtggctggccagtgaaggtgccttctctgatcccccccaagcaacagtggtcactcagggtataagaaggtcccttttcctctgcacagcattacctcaagggtgagatgctagcaggggtggggtttttggttctgtgcccaccatggcttcatcttcagtggcagttggtgtgggttggggtgtgtgctgcattcccatatgctgttagggcaagtacaacaaaacccacctgtgtaaacacacacagctaagtgatgtaggaagtttccatataaagggctgcagtatggagaggtaatgtgtaggctggtacgtggctgtagaggtcaccttgctgcagctctccactgatcagccacggtccgcttgtacagaagctatggtgtgggcacccagaagtgccctctaagcaggtgtggcctggctggggtcctgggagaggcaagcagactaaggggtgctgaggtcagaccagccccatctcatgtgcaagactgcccagcagagatcaggtctcagaggagaactctctcaaaagtgaatcctcagcacagcacaactgctctacacaaacgcggccagacttcttttttaagcaagtccccctttttaggaagagaactcttagacctgatctgtgctgggcaatcttgcacgtgagatggggctggtctgacctcagcactccttaagtgctgggataaagtgtctcataagagcaagtggagcctagagacatagatgtccctgccctccgggctccacatcagctgacttgctgctccaccactttccttgtctcctgggggctacaccccagagaggtgtaagttaggagttacttaatgtaatcaccccaggatggagggtctgtgctgtgggcccaagccagggttccttgtctggtgatgagcagtaaggagtgtgttgtacccgtggaaggtggactgacttgttccttgtgtcaactgcagcttgttggaggtgtcaatatggcacttagggtctttgctcccttgatattctgagggtagcaagggcagttccactgcagaggcagtggcagagaggatttctgttgctcctggaagctctgtccagggagttgctgagttgctactggcttgaaggctcaagtggggggctggctggagacccaggccaggaagacctgcccatcatggcccacccctctctctgggaactctgtcccaggaaggtttcaaatctccattggccagggaacactggtgggtgtagctggaggcctcaggtgggagatcctgtccagtgatgaggaacaggatcaggggcctgcttacagaagcattctggccatgatttggtaaagcagctgtgctatgccacaggatctcttctgtccctggtgagtttgtactctccaaagcccgcacgctggaatgactaagttgcccaaacaggaaagatggtggcctgcctcatcttttctctcagaatttatcctgtgtgatggagcttaatttttaggttgttaattttactgtcagcgttagagttgttcagaaagaatctcactgttatcttttaggtgagatatataagaattcattttctcctgtaaataaacctgttgatgtttgctctctggaaagaagtccctttcagctatctgactttgatcacaatcatgtagagcagtagtcagtctacaatgacatgattgaatttccatttccagtgtttcctagctgtgtcttacattctccagttcagaactgagcattctcagttgtcaaaatcctaagctgtccactgtacttaaatactggttttcgttaatgcttcttcattcagttgtatagcctttagaagtttttcttttacactttcaatttcctccaaaattttattttcccttagctggttctgatgttttgtttcatctagttccagtcttagcatggcaatttcttcccgcaacatgctgttttcacgcaagagatcttcttctttcttatgactaagagaaagctcagaattcatttccttttcagccacttctatctgcttttgtttattagtcagaatctcatcttgtgatattccagtgttctgttcttcagaaagttgtttctgggtatcattttgttcgtcactgtgatactcttcattctcagtgtcaggaaattgctgattttcaggttttctgctcttcctttgtggaattaatccatcatcaccattgccagcactggcaccattagtcaggttttctggtaatcccacaggattacttccatgcttctttatttcttcttcaacctctctatcacagtccttatttatttctggttcttgagacattttctctggctggctattttcactgactttaagcctttgtgactcttcctctgatgtcagctttaagtcttgttctggattgctgttttcagaagagatttttagcatctgtttttctttatagtcagaaagtaattcacaaattacatgatgatgactagaaacagcatactctctggccgtctgtccagatagatcttgagaagatacatcaacattttgctcaagtagaagattgactatacttgctgatccacaacatacagcaagtatgagggcagttcttccatatctatcaagtgcatttaaattagcttttttcttgattaaaaatttcaccacttcctgtttttgttcatgtacgccaagcaaaagtggtgtgaggccacacttgttttttgattcaatatcagcaccatataagagcagtgctttggccattaatttatcttcattgtagatagcatagtgtagagcggtatttccatactcatcttgaatatttccatcagcgccatgttccagcaacattaacacacattcatcttcctggcattgtacggcctttatcagagctgtcctttttttgttgtcaaggacgttaagttgacatcgtctgtccagcaggagttgtactacttctgaatttccattggcagaggccaaatgtagagcagtcctcttttgcttgtccctcttgttcatgtcagtgtccctgagcatgacgatgagatcctttctggggactttaccccaccaggcagctctgtggagcttgtccagatcttctcgacggacgtggtacctcggctccatgaaggcgctgtcgtcgtagtctccccaagtgcccacgttgctcttgccgctccccctgcagcaggggaagcagtgacagcaccacttgcccatcttgctcctgagtgtcttcataaaggagttgtcatggtctccagaagtgcccacattgctcgtgccgctccccctgcagcaggggaagcagtgatggcaacacttgcccatcttgctcctgagcgtcttcataaaggagtcgtcgtggtctccagaagtgcccatgttgctcttgccgctccccctgcagcaggggaagcggtggtggcaccacttgcccatcttgcttctgagatcaaatggcttcttcacagcagaggcagcgggcattgaacaaacctcagccaccatctgcttttaacagccaggggaggccggtagtagcgaacagatcgcgtctaccaaccagtttcaccaactagcaggaaaccctgggtttccaatctgtttgaagagaaaggtcaatcccagccaaaacttgccaagcccagcaaggga

SEQ ID NO: 19207 - RNA, 5447 nt, Homo sapiens
  source 1..5447: mol_type = other RNA
tgtgactgcattatgaaaattcttctagtgtgatttacagctctgtcaggtcagttattttcttctttatacttgctcttttgtctgttacttcctgcaatgttttacaatgatttttagcttccttgtattggattacaacatacttctttcacgcaatgaactttgttcctacccatatcctgaactctgcttgtatcatttcagacatctcagcctcagcccagttctgaacacttgctggagagttgatgcagtcatttggagaaaagaaggcatgctgaatttttgagtttttagtgttcttgcacagagtctttttctcatctttatgggcttatccatcttcaatctttgaggttgctgacgtttggacagggtatttttcctttattatatctgatgaccttgaggatttgattgtggtgtaaggtggattcagccaacaggttttgtttttggaggattttaaggggccaacatgcagctcccaattcttggactgtgtgctttaactctggggaacttgtattgggccacaactttgttctctggctcctcgaggtttggagtccactgcactgaggggaccaaagtgcggcagctgtggcagaatgctaccagatgcaaaagtccctgcctccctgtgggcattcacccagtggtggaggcaaaacagctggggtgtgggccagggggcccctgctgtgtgtgctgttgcactggaggtagtgctggtttggggtgggtggctggccagtgaaggtgccttctttgatcccccccaagcaacagtggtcactcagggtataagaaggtcccttttcctctgcacagcattacctcaagggtgagatgctagcaggggtggggtttttggttctgtgcccaccatggcttcatcttcagtggcagttggtgtgggttggggtgtgtgctgcattcccatatgctgttagggcaagtacaacaaaacccacctgtgtaaacacacacagcaaagtgatgtaggaagtttccatataaagggctgcagtatggagaggtaatgtgcaggctagtgcgtggctgtagaggtcaccttgctgcagctctccattgatcaggcatggtccgcttgtacagaagctatggtgtgggcacccgaaagtgccctctaagcaggtgtggcctggctggggtcctgggagaggcaagcagactaaggggtgctgaggtcagaccagccccatctcatgtgcaagactgcccagcacagatcaggtctcagaggagaactctctcaaaagtgaatcctcagcacagcacaactgctctacacaaacgtggccagacttcttttttaagcaagtccccttttttacgaagagaactcttagacctgatctgtgctgggcaatcctgcatgtgagatggggctggtctgacctcagcactcctaaagtgctgggataaagtgtctcataagagcaagtggagcctagagacatagctgtccctgccctccgggctccacatcagctgacttgctgctccaccactttccttgtctcctgggggctccaccccagagaggtgtaagttagcagttacttaatgtaatcaccccaggatggagggtctgtgttgtgggcccaagccagggttccttgtctggtgatgagcagtaaggggtgtgttgtacctgtggaagatggactgacttgttccttgtgtcaactgcagcttgttggaggtgtcaatatggtacttagggtctttgctcccttgatattctgagggtagcaagggcagttccactgcagaggcagtggcagagaggatttctgttgctcctggaagctctgtccagggagttgctgagttgctactggcttgaaagctcaagtggggggctggctggagacccaggccaggaagacctgcccatcgaggagatatggaaatgggcacccacataacagtctggccacttttctgtggggctgccgtggtatgctgggggtccactccagtcgccaattgcctcgtattttccagtggctgaaggtatcagcagtgaagcctgcgaaaaagcaaagacgataacctgcccttccctctgggagctctgtacctctgaggtatgaacctgttgccaatctgaacacacctgtaggatgtgactggaagcaagttgagaagtcttgcctagtaaggaggaacaggaatagggacttgtttaaaaaagaagtctggccacgtttttgtagagtggctatgctgtgcggggggttcacttcagcccctggtctcctcagacactctgaaactctaagactgaactggctgagtcatccaaacagcaaagatgacagtctggtcctccccctgggagctctcactcaggaggcctgaaacctctgtcagccagagaacagcagtgaaggtggctggagaccctggttgaaaggctccagccagtgattagaaatgtggttggggactggcttaaacaagaatctggccacgttttcgcagggtggctgttctgtgctgaggtaccacttccacccctggtcagcttgggctctccaaagcccacaggccagaagggctagttgcccaaacaacaaaggtcatggcccacccctctctctgggaactctgtcccaggaaggtttcaaatctccattggccagggaacactggtgggtgtagctggaggcctcaggtgggagatcctgtccagtgacaaggaacaggatcaggggcctgcttacagaagcattctggccatgatttggtaaagcagctgtgctatgccacaggatctcttctgcccctggtgggtttgtactctccaaagcccgcacgctggaatggctaagttgcccaaacaggaaagatggtggcctgcctcatcttttctctcagaatttatcctgtgtgatggagcttaatttttaggttgttaattttactgtcagcgttagagttgttcagaaagaatctcactgttatcttttaggtgagatatatgagaattcattttctcctgtaaataaacctgttcatgtttgttctctggaaagaagtccctttcagctatctgactttgatcacaatcatgtagagcagtagtcagtctacaatgacatgattgaatttccatttccagtgtttcctagctgtgtcttacactctccagttcagaactgagcattctcagttgtcaaaatcctaagctgtccactgtacttaaatattggttttcgttaatgcttcttcattcaattgcatagcccttagaagtttatcagtcttttctttcacactttcaatttcctccaaaattttattttcccttagctggttctgatgttttgtttcatctagttccagtcttagcatggcaatttcttcctgcaacacgctgttttcacgcaagagatcttcttctttcttatgactaagagaaagctcagaattcattttctgttcagccacttctatctgcttttgtttattagtcagaatctcatcttgtgatattccagtgttctgttcttcagaaagttgtttccgggtatcattttgttcatcactgtgatactcttcattctcagtgtcaggaaattgctgattttcaggttttctgctcctcctttgtggaattaatccatcatcaccattgccagcactggcaccattagtcaggttttctggtaatcccacaggattacttccatgcttctttatttcttcttcaacctctctatcacagtccttatttatttctggttcttgagacattttctctggctggctattttcactgactttaagcctttgtgactcttcctctgatgtcagctttaagtcttgttctggattgctgttttcagaagagatttttagcatctgtttttctttatagtcagaaagtaattcacaaattacatgatgatgactagaaacagcatactctctggccgtctgtccagatagatcttgagaagatacatcaacattttgctcaagtagaagattgactatacttgctgatccacaacatacagcaagtatgagggcagttcttccatatctatcaagtacatttaaattagcttttttcttgattaaaaatttcaccacttgctgtttttgttcatgtacgccaagcaaaagtggtgtgaggccacacttgttttttgattcaatatcagcaccatataagagcagtgctttggccattaatttatcttcattgtagatagcatagtgtagagcggtatttccatactcatctggaatatttcgatcagcgccatgttccagcaacattaacacacattcatcttcctggcattgtatggcctttatcagagctgtcctttttttgttgtcaaggacattaagttgacatcgtctgtccagcaggagttgtactacttctgaatttccattggcagaggccaaatgtagagcagtcctcttttccttgtccctcttgttcatgtcagtgtccctgagcatgacgatgagatcctttctggggactttaccccaccaggcagctctgtggagcttgtccagatcttctcgacggatgtggtacctcggctccatgaaggcgctgtggtcgtagtctccccaagcgcccacgttgctcttgccgctccccctgcagcaggggaagcagtgacagcaccacttgcccatcttgctcctgagcatcttcataaaggagttttcatggtctccagaagtgcccacgttgctcgtgccgctccccctgcagcaggggaagcagtggcggcaacacttgcccatcttgctcctgagcatcttcataaaggagtcgtcgtggtctccagaagtgcccatgttgctcttgccgctccccctgcagcaggggaagcggtggtggcaccacttgcccatcttgctcctgagatcaaatggcttcttcacagtagaggcagtgggcattgaacaaacctcagccaccatctgcttttaacagccaggggaggccggtagtagcgaacagatcgcgtctaccaaccagtttcaccaactagcaggaaaccttgggtttccaatctgtttgaagagaaaggtcaatcccagccaaaacttgccaaccccagcaagggagcccagcccaccccacccagggaaaacccacacccacccggggaaagcccacgcccaccagggggaccccaggcccaccccaggaaaggccaagccccccctccgaaggaaacacccagcccagtcaagggaatgccaaacccagcagagaaaaattcaggcccagcaaaggaatgcgagggagaaaacgccaatccaagcaagaaacaccaggcaaagcgactaacgccaagccaagctaggaacgcaaggccaagcgaggaacgcaaagcgaagcgcacccattacaggtaagccaagccgtc

SEQ ID NO: 19208 - RNA, 656 nt, Homo sapiens
  source 1..656: mol_type = other RNA
tgtgacttctcccctgccacagatgcacccacacatgtctgtggacctgtgctccatcacctaaaccaaggcagcttcatactccccccagaactacgccaagctgcagcttcctcacttgaaaagcagaagggataaattagtgcctcctggggcaaccataggattaaactgagattgctttttcttcctcaagcacatttatttcatcaccctcaaacttttacacttcactttctttttaaaggccatctttcctgtttagcagttataatgctaacacatgctcaaaatacaaaacttgggagatgtaggaaagtagaaagaaggaagaaaagtccgatgccagtgaccagaggtagcagcacacccccaaggaacgaagtgagaatatgcggcatgcaagtgtcatattctgttctttccattaacagcatacaccggattttttactcgagttttcagatgcagactcatgccctgatctcttgattttttatgtgaacacacgtttggcactcaatatgtcccaccaggaagttcctcttccttaaaactcctgggcggaggaagggagtcctgtgaagttgggagacctgggttcaaggtgtcctacaatgcccccacctttccttcagcttccaggcaggctgcag

SEQ ID NO: 19209 - RNA, 135 nt, Homo sapiens
  source 1..135: mol_type = other RNA
tgtgacttctcccctgccacaggaagcctggtgcggcagtggacggccccacccgagcaggagctgtgcctgcagctgaagtcctcccaggcactggtggccagtctccaggagcagctgtccgaaagccggcgg

SEQ ID NO: 19210 - RNA, 1436 nt, Homo sapiens
  source 1..1436: mol_type = other RNA
tgtgaggttggcattgttgtctgtgggtgagtacctctcttcattttcacctcctcctgatcttttggacactgaaagcatttctgctgagtgacatcgttccattgtatatgtttttgcttgagactgactattagaagtgccagatctatcagaggaataagctctacgaaggtatcgagaatgtggcctttcttctgcatcttgaattactcttccccttccactattactggtttcttgatttccccactgagtataaaaactgtttccatctcctgaagaagaaaaatcagttgaacttttattctttggaaatacagtcattttatttgggagtggctgaccaatcaaaagtcttcttttgtcaaataaactaccacttatactggtactggaagaagctgtaattgcagtagaaattgtggcatgcccactatcaattgagtcttccacagttcctaaatctttactttttgttgaagaatttcgggacataaaaggatggtccaatactgaagacagacttaaacgatctgctggatttctacgaagtaactggtgaataaggtccttggcctctattgacaaaaaagatggcatttcataatctgccaatactactttatttaatgtgttcttgactgtgtcagtgtcgaagggtggtctcccgataagtaatgtataaaacatacagcccagggaccaaacatcagattcaaggccatgtgcacttcgagtggcaatttctggtgaaatgtagttaggagttccacataatgtatagtgcttttcatgtggcattttcagttgagttgccagcccaaaatcagcaatcttgatgttcatattacgagtcagtaggaggttagaaagtgtgaggtcccggtgtagtataccatgagaatgaagatacaacatccctgtgatgatctggtgcatgaagtgtcgagcttcattttctgagaagggtttcactctattctttagatacctgttcatttctccattatggcacatttctaataccagatacacataattgctatcttcaaaatagttataaagcattttgattgcaacttccaaaccagtgtgaatggactcagctctgtagacaccagcaaatgatcctttaccaagcagatttccaactttaaaatcctcgatcttctccccgatgcaggtcgccatatttccaggctctggcctgggttctccggattagcttccttcacgcagtcccttcgaggcagcgctccaagcagccagccggccttggcgcccatcaggctcggctctctaaaccgccgctccaggcgacgacgctgaaaccacggaaagttctccctgacaccttccgaggcctgggcggtgcctctgggctcccattttgaaaatctcccgccgcttgccgtccgagctaggctggtggt

SEQ ID NO: 19211 - RNA, 1532 nt, Homo sapiens
  source 1..1532: mol_type = other RNA
tgtgaggttggcattgttgtctgtgggtgagtacctctcttcattttcacctcctcctgatcttttggacactgaaagcatttctgctgagtgacatcgttccattgtatatgtttttgcttgagactgactattagaagtgccagatctatcagaggaataagctctacgaaggtatcgagaatgtggcctttcttctgcatcttgaattactcttccccttccactattactggtttcttgatttccccactgagtataaaaactgtttccatctcctgaagaagaaaaatcagttgaacttttattctttggaaatacagtcattttatttgggagtggctgaccaatcaaaagtcttcttttgtcaaataaactaccacttatactggtactggaagaagctgtaattgcagtagaaattgtggcatgcccactatcaattgagtcttccacagttcctaaatctttactttttgttgaagaatttcgggacataaaaggatggtccaatactgaagacagacttaaacgatctgctggatttctacgaagtaactggtgaataaggtccttggcctctattgacaaaaaagatggcatttcataatctgccaatactactttatttaatgtgttcttgactgtgtcagtgtcgaagggtggtctcccgataagtaatgtataaaacatacagcccagggaccaaacatcagattcaaggccatgtgcacttcgagtggcaatttctggtgaaatgtagttaggagttccacataatgtatagtgcttttcatgtggcattttcagttgagttgccagcccaaaatcagcaatcttgatgttcatattacgagtcagtaggaggttagaaagtgtgaggtcccggtgtagtataccatgagaatgaagatacaacatccctgtgatgatctggtgcatgaagtgtcgagcttcattttctgagaagggtttcactctattctttagatacctgttcatttctccattatggcacatttctaataccagatacacataattgctatcttcaaaatagttataaagctccaagatagaaggatgtttcaattggcaatgtattttcacctcattttggactctctgtaccattcctgctttgtacatggctttcttatctatcattttgattgcaacttccaaaccagtgtgaatggactcagctctgtagacaccagcaaatgatcctttaccaagcagatttccaactttaaaatcctcgatcttctccccgatgcaggtcgccatatttccaggctctggcctgggttctccggattagcttccttcacgcagtcccttcgaggcagcgctccaagcagccagccggccttggcgcccatcaggctcggctctctaaaccgccgctccaggcgacgacgctgaaaccacggaaagttctccctgacaccttccgaggcctgggcggtgcctctgggctcccattttgaaaatctcccgccgcttgccgtccgagctaggctggtggt

SEQ ID NO: 19212 - RNA, 1723 nt, Homo sapiens
  source 1..1723: mol_type = other RNA
tgtgaggttggcattgttgtctgtgggtgagtacctctcttcattttcacctcctcctgatcttttggacactgaaagcatttctgctgagtgacatcgttccattgtatatgtttttgcttgagactgactattagaagtgccagatctatcagaggaataagctctacgaaggtatcgagaatgtggcctttcttctgcatcttgaattactcttccccttccactattactggtttcttgatttccccactgagtataaaaactgtttccatctcctgaagaagaaaaatcagttgaacttttattctttggaaatacagtcattttatttgggagtggctgaccaatcaaaagtcttcttttgtcaaataaactaccacttatactggtactggaagaagctgtaattgcagtagaaattgtggcatgcccactatcaattgagtcttccacagttcctaaatctttactttttgttgaagaatttcgggacataaaaggatggtccaatactgaagacagacttaaacgatctgctggatttctacgaagtaactggtgaataaggtccttggcctctattgacaaaaaagatggcatttcataatctgccaatactactttatttaatgtgttcttgactgtgtcagtgtcgaagggtggtctcccgataagtaatgtataaaacatacagcccagggaccaaacatcagattcaaggccatgtgcacttcgagtggcaatttctggtgaaatgtagttaggagttccacataatgtatagtgcttttcatgtggcattttcagttgagttgccagcccaaaatcagcaatcttgatgttcatattacgagtcagtaggaggttagaaagtgtgaggtcccggtgtagtataccatgagaatgaagatacaacatccctgtgatgatctggtgcatgaagtgtcgagcttcattttctgagaagggtttcactctattctttagatacctgttcatttctccattatggcacatttctaataccagatacacataattgctatcttcaaaatagttataaagctccaagatagaaggatgtttcaattggcaatgtattttcacctcattttggactctctgtaccattcctgctttgtacatggctttcttatctatcattttgattgcaacttccaaaccagtgtgaatggactcagctctgtagacaccagcaaatgatcctttaccaagcagatttccaactttaaaatcctcgatgcagcaggtgtctagggtggaaggcatgttgactccgtgcggggatacctgcgcttccaggctggactggaagctcagggtgatggtgcaccctagtgatctggttcctcaacctcagtgcagcctaagcgccctcctcccatctccagccaatccccgggagcggagggctcggtcagaatcccgccgcagctcccgccggagataaccgccatccccttggagaagtgggaggtagccctgccctgctctaacgcggtagctcgggcgggattgctgaaagaaagccgcagtgcctcgggacactgccgggcggggagggactcacctgtcccgccttccctactcttgtctcttgaggggcgggccgctccgcccctaaacagcaggggtctgggccgttgggaccctccctaagcacctcggtgcccgccccgcagccgttagcttcgttcgc

SEQ ID NO: 19213 - RNA, 1399 nt, Homo sapiens
  source 1..1399: mol_type = other RNA
tgtgaggttggcattgttgtctgtgggtgagtacctctcttcattttcacctcctcctgatcttttggacactgaaagcatttctgctgagtgacatcgttccattgtatatgtttttgcttgagactgactattagaagtgccagatctatcagaggaataagctctacgaaggtatcgagaatgtggcctttcttctgcatcttgaattactcttccccttccactattactggtttcttgatttccccactgagtataaaaactgtttccatctcctgaagaagaaaaatcagttgaacttttattctttggaaatacagtcattttatttgggagtggctgaccaatcaaaagtcttcttttgtcaaataaactaccacttatactggtactggaagaagctgtaattgcagtagaaattgtggcatgcccactatcaattgagtcttccacagttcctaaatctttactttttgttgaagaatttcgggacataaaaggatggtccaatactgaagacagacttaaacgatctgctggatttctacgaagtaactggtgaataaggtccttggcctctattgacaaaaaagatggcatttcataatctgccaatactactttatttaatgtgttcttgactgtgtcagtgtcgaagggtggtctcccgataagtaatgtataaaacatacagcccagggaccaaacatcagattcaaggccatgtgcacttcgagtggcaatttctggtgaaatgtagttaggagttccacataatgtatagtgcttttcatgtggcattttcagttgagttgccagcccaaaatcagcaatcttgatgttcatattacgagtcagtaggaggttagaaagtgtgaggtcccggtgtagtataccatgagaatgaagatacaacatccctgtgatgatctggtgcatgaagtgtcgagcttcattttctgagaagggtttcactctattctttagatacctgttcatttctccattatggcacatttctaataccagatacacataattgctatcttcaaaatagttataaagctccaagatagaaggatgtttcaattggcaatgtattttcacctcattttggactctctgtaccattcctgctttgtacatggctttcttatctatcattttgattgcaacttccaaaccagtgtgaatggactcagctctgtagacaccagcaaatgatcctttaccaagcagatttccaactttaaaatcctgtcccgccttccctactcttgtctcttgaggggcgggccgctccgcccctaaacagcaggggtctgggccgttgggaccctccctaagcacctcggtgcccgccccgcagccgttagcttcgttcgctccccttccc

SEQ ID NO: 19214 - RNA, 1391 nt, Homo sapiens
  source 1..1391: mol_type = other RNA
tgtgaggttggcattgttgtcttggttgccatggacgatgaccaccaggggcagagacagggcctggagctggatggggagtttgccggggccaagtgtgaagctggcagagaagagcacagcgcacttctcctctgtgacagactcagtgcccttccgctcacaccgcttgatcttcttgagaagcaggttcttgaacagggcagagcagcagttcccaggaatgctgttctccaagggcacagtgttgttgatgatttctccagtgctttctgctccagccccaggaccctgaggcacactcagctcccgcgcctgcttctctgtcaccatgtcggccctgaccagcggaggcttggctggggcccccaggaacctcaagcccaacaggaatcgaactccagcctggaacttggtctgagtcttcagtacctgggggggctgcttctccaccaggaagcaactggtgacgagggttctcaggacttcatccagccggccagtcagcgatgcccgggtcttgggctcaagctccccaccagccgcccctacctcctgctgtagctgggaataaatgtccaccaggctttcacacctctcctggagtggggccaggctctcctcaaacggtgcgccattccctgccagctgctgctgccgtttccaaatctggatcctcttcagcactagggctttggctgcctctagctctccagtggtctcctgcagtagcatggccagggcctcacttggcccagtcccattagcaggagtttctatcaagctgtgcagagacacttggccagcctcagcccccttctgcagggcttctcggagaaggtggatctcccctactcggtgctgcagcctccgcaagcctgtcttaaacttgagttcttcctgcttccagtggaaaggcattggcaagtggcggaactgttccataacagcttttttctctccttgaagtatttgtctgaaagtggccaccagcttcagggggtccctctgatatatgctcagggctggctctccagccagtcacccagaagatgccgcaggtgttggggaaagtcgacatagagccgctgcactttttctgggggcatcttggagaccagaccccacagagacatgatctgggacttggaggttgcctcggcaacccctctgctgtcttctccctttctcagcgggcacttccaggccccataggtctgtagctctgtccagcgagttcaaggctggccctgctagcacctccccccttccaccaccaccaccaaaaagaaaaataagataaagcacacacatacatacacacacacacacacacacacacacacactcctctcccgtcctccctcttcagtgtaagcagtggctgcccc

SEQ ID NO: 19215 - RNA, 1420 nt, Homo sapiens
  source 1..1420: mol_type = other RNA
tgtgaggttggcattgttgtcttggttgccatggacgatgaccaccaggggcagagacagggcctggagctggatggggagtttgccggggccaagtgtgaagctggcagagaagagcacagcgcacttctcctctgtgacagactcagtgcccttccgctcacaccgcttgatcttcttgagaagcaggttcttgaacagggcagagcagcagttcccaggaatgctgttctccaagggcacagtgttgttgatgatttctccagtgctttctgctccagccccaggaccctgaggcacactcagctcccgcgcctgcttctctgtcaccatgtcggccctgaccagcggaggcttggctggggcccccaggaacctcaagcccaacaggaatcgaactccagcctggaacttggtctgagtcttcagtacctgggggggctgcttctccaccaggaagcaactggtgacgagggttctcaggacttcatccagccggccagtcagcgatgcccgggtcttgggctcaagctccccaccagccgcccctacctcctgctgtagctgggaataaatgtccaccaggctttcacacctctcctggagtggggccaggctctcctcaaacggtgcgccattccctgccagctgctgctgccgtttccaaatctggatcctcttcagcactagggctttggctgcctctagctctccagtggtctcctgcagtagcatggccagggcctcacttggcccagtcccattagcaggagtttctatcaagctgtgcagagacacttggccagcctcagcccccttctgcagggcttctcggagaaggtggatctcccctactcggtgctgcagcctccgcaagcctgtcttaaacttgagttcttcctgcttccagtggaaaggcattggcaagtggcggaactgttccataacagcttttttctctccttgaagtatttgtctgaaagtggccaccagcttcagggggtccctctgatatatgctcagggctggctctccagccagtcacccagaagatgccgcaggtgttggggaaagtcgacatagagccgctgcactttttctgggggcatcttggagaccagaccccacagagacatgatctgggacttggaggttgcctcggcaacccctctgctgtcttctccctttctcagcgggcacttccaggccccataggtctgtagctctgtccagcgagttcaaggctggccctgctagcacctccccccttccaccaccaccaccaaaaagaaaaataagataaagcacacacatacatacacacacacacacacacacacacacacactcctctcccgtcctccctcttcagtgtaagcagtggctgccccagcccgctgtttccggcttctccttctac

SEQ ID NO: 19216 - RNA, 1596 nt, Homo sapiens
  source 1..1596: mol_type = other RNA
tgtgaggttggcattgttgtcttggttgccatggacgatgaccaccaggggcagagacagggcctggagctggatggggagtttgccggggccaagtgtgaagctggcagagaagagcacagcgcacttctcctctgtgacagactcagtgcccttccgctcacaccgcttgatcttcttgagaagcaggttcttgaacagggcagagcagcagttcccaggaatgctgttctccaagggcacagtgttgttgatgatttctccagtgctttctgctccagccccaggaccctgaggcacactcagctcccgcgcctgcttctctgtcaccatgtcggccctgaccagcggaggcttggctggggcccccaggaacctcaagcccaacaggaatcgaactccagcctggaacttggtctgagtcttcagtacctgggggggctgcttctccaccaggaagcaactggtgacgagggttctcaggacttcatccagccggccagtcagcgatgcccgggtcttgggctcaagctccccaccagccgcccctacctcctgctgtagctgggaataaatgtccaccaggctttcacacctctcctggagtggggccaggctctcctcaaacggtgcgccattccctgccagctgctgctgccgtttccaaatctggatcctcttcagcactagggctttggctgcctctagctctccagtggtctcctgcagtagcatggccagggcctcacttggcccagtcccattagcaggagtttctatcaagctgtgcagagacacttggccagcctcagcccccttctgcagggcttctcggagaaggtggatctcccctactcggtgctgcagcctccgcaagcctgtcttaaacttgagttcttcctgcttccagtggaaaggcattggcaagtggcggaactgttccataacagcttttttctctccttgaagtatttgtctgaaagtggccaccagcttcagggggtccctctgatatatgctctcaagggtgctgatgtgttgcaagatggtgctcccctccccctgctctcccaccgaggcctgaaggtgctggacagtgtctgaaagtagggcactagccaagttgcagcagaaggcgtcggagccgaccaggaactcccagggctggctctccagccagtcacccagaagatgccgcaggtgttggggaaagtcgacatagagccgctgcactttttctgggggcatcttggagaccagaccccacagagacatgatctgggacttggaggttgccccagctcttttctcctcaaggcagaatccttacccctcctgctcaggttcctccaataggcctttctctcggcaacccctctgctgtcttctccctttctcagcgggcacttccaggccccataggtctgtagctctgtccagcgagttcaaggctggccctgctagcacctccccccttccaccaccaccaccaaaaagaaaaataagataaagcacacacatacatacacacacacacacacacacacacacacactcctctcccgtcctccctcttcagtgtaagcagtggctgcc

SEQ ID NO: 19217 - RNA, 1509 nt, Homo sapiens
  source 1..1509: mol_type = other RNA
tgtgaggttggcattgttgtcttggttgccatggacgatgaccaccaggggcagagacagggcctggagctggatggggagtttgccggggccaagtgtgaagctggcagagaagagcacagcgcacttctcctctgtgacagactcagtgcccttccgctcacaccgcttgatcttcttgagaagcaggttcttgaacagggcagagcagcagttcccaggaatgctgttctccaagggcacagtgttgttgatgatttctccagtgctttctgctccagccccaggaccctgaggcacactcagctcccgcgcctgcttctctgtcaccatgtcggccctgaccagcggaggcttggctggggcccccaggaacctcaagcccaacaggaatcgaactccagcctggaacttggtctgagtcttcagtacctgggggggctgcttctccaccaggaagcaactggtgacgagggttctcaggacttcatccagccggccagtcagcgatgcccgggtcttgggctcaagctccccaccagccgcccctacctcctgctgtagctgggaataaatgtccaccaggctttcacacctctcctggagtggggccaggctctcctcaaacggtgcgccattccctgccagctgctgctgccgtttccaaatctggatcctcttcagcactagggctttggctgcctctagctctccagtggtctcctgcagtagcatggccagggcctcacttggcccagtcccattagcaggagtttctatcaagctgtgcagagacacttggccagcctcagcccccttctgcagggcttctcggagaaggtggatctcccctactcggtgctgcagcctccgcaagcctgtcttaaacttgagttcttcctgcttccagtggaaaggcattggcaagtggcggaactgttccataacagcttttttctctccttgaagtatttgtctgaaagtggccaccagcttcagggggtccctctgatatatgctctcaagggtgctgatgtgttgcaagatggtgctcccctccccctgctctcccaccgaggcctgaaggtgctggacagtgtctgaaagtagggcactagccaagttgcagcagaaggcgtcggagccgaccaggaactcccagggctggctctccagccagtcacccagaagatgccgcaggtgttggggaaagtcgacatagagccgctgcactttttctgggggcatcttggagaccagaccccacagagacatgatctgggacttggaggttgcccctcctgctcaggttcctccaataggcctttctctagcccaagagagaaaggtcctctggagtgagtgggcaccgctttcctctgcatccccttgcagagtgaccagcctcctggcatggccctggctagaaatatccaacccctcttcttccccagccatcaggaggacacatttctccccaccccaacccataacaaggctgggtcgatt

SEQ ID NO: 19218 - RNA, 1549 nt, Homo sapiens
  source 1..1549: mol_type = other RNA
tgtgaggttggcattgttgtcttggttgccatggacgatgaccaccaggggcagagacagggcctggagctggatggggagtttgccggggccaagtgtgaagctggcagagaagagcacagcgcacttctcctctgtgacagactcagtgcccttccgctcacaccgcttgatcttcttgagaagcaggttcttgaacagggcagagcagcagttcccaggaatgctgttctccaagggcacagtgttgttgatgatttctccagtgctttctgctccagccccaggaccctgaggcacactcagctcccgcgcctgcttctctgtcaccatgtcggccctgaccagcggaggcttggctggggcccccaggaacctcaagcccaacaggaatcgaactccagcctggaacttggtctgagtcttcagtacctgggggggctgcttctccaccaggaagcaactggtgacgagggttctcaggacttcatccagccggccagtcagcgatgcccgggtcttgggctcaagctccccaccagccgcccctacctcctgctgtagctgggaataaatgtccaccaggctttcacacctctcctggagtggggccaggctctcctcaaacggtgcgccattccctgccagctgctgctgccgtttccaaatctggatcctcttcagcactagggctttggctgcctctagctctccagtggtctcctgcagtagcatggccagggcctcacttggcccagtcccattagcaggagtttctatcaagctgtgcagagacacttggccagcctcagcccccttctgcagggcttctcggagaaggtggatctcccctactcggtgctgcagcctccgcaagcctgtcttaaacttgagttcttcctgcttccagtggaaaggcattggcaagtggcggaactgttccataacagcttttttctctccttgaagtatttgtctgaaagtggccaccagcttcagggggtccctctgatatatgctctcaagggtgctgatgtgttgcaagatggtgctcccctccccctgctctcccaccgaggcctgaaggtgctggacagtgtctgaaagtagggcactagccaagttgcagcagaaggcgtcggagccgaccaggaactcccagggctggctctccagccagtcacccagaagatgccgcaggtgttggggaaagtcgacatagagccgctgcactttttctgggggcatcttggagaccagaccccacagagacatgatctgggacttggaggttgcctcggaggcaacccctcacctcggcaacccctctgctgtcttctccctttctcagcgggcacttccaggccccataggtctgtagctctgtccagcgagttcaaggctggccctgctagcacctccccccttccaccaccaccaccaaaaagaaaaataagataaagcacacacatacatacacacacacacacacacacacacacacactcctctcccgtcctccctcttcagtgtaagcagtggctgcccc

SEQ ID NO: 19219 - RNA, 1561 nt, Homo sapiens
  source 1..1561: mol_type = other RNA
tgtgaggttggcattgttgtcttggttgccatggacgatgaccaccaggggcagagacagggcctggagctggatggggagtttgccggggccaagtgtgaagctggcagagaagagcacagcgcacttctcctctgtgacagactcagtgcccttccgctcacaccgcttgatcttcttgagaagcaggttcttgaacagggcagagcagcagttcccaggaatgctgttctccaagggcacagtgttgttgatgatttctccagtgctttctgctccagccccaggaccctgaggcacactcagctcccgcgcctgcttctctgtcaccatgtcggccctgaccagcggaggcttggctggggcccccaggaacctcaagcccaacaggaatcgaactccagcctggaacttggtctgagtcttcagtacctgggggggctgcttctccaccaggaagcaactggtgacgagggttctcaggacttcatccagccggccagtcagcgatgcccgggtcttgggctcaagctccccaccagccgcccctacctcctgctgtagctgggaataaatgtccaccaggctttcacacctctcctggagtggggccaggctctcctcaaacggtgcgccattccctgccagctgctgctgccgtttccaaatctggatcctcttcagcactagggctttggctgcctctagctctccagtggtctcctgcagtagcatggccagggcctcacttggcccagtcccattagcaggagtttctatcaagctgtgcagagacacttggccagcctcagcccccttctgcagggcttctcggagaaggtggatctcccctactcggtgctgcagcctccgcaagcctgtcttaaacttgagttcttcctgcttccagtggaaaggcattggcaagtggcggaactgttccataacagcttttttctctccttgaagtatttgtctgaaagtggccaccagcttcagggggtccctctgatatatgctctcaagggtgctgatgtgttgcaagatggtgctcccctccccctgctctcccaccgaggcctgaaggtgctggacagtgtctgaaagtagggcactagccaagttgcagcagaaggcgtcggagccgaccaggaactcccagggctggctctccagccagtcacccagaagatgccgcaggtgttggggaaagtcgacatagagccgctgcactttttctgggggcatcttggagaccagaccccacagagacatgatctgggacttggaggttgcctcggaggcaacccctcacctcggcaacccctctgctgtcttctccctttctcagcgggcacttccaggccccataggtctgtagctctgtccagcgagttcaaggctggccctgctagcacctccccccttccaccaccaccaccaaaaagaaaaataagataaagcacacacatacatacacacacacacacacacacacacacacactcctctcccgtcctccctcttcagtgtaagcagtggctgccccagcccgctgttt

SEQ ID NO: 19220 - RNA, 1530 nt, Homo sapiens
  source 1..1530: mol_type = other RNA
tgtgaggttggcattgttgtcttggttgccatggacgatgaccaccaggggcagagacagggcctggagctggatggggagtttgccggggccaagtgtgaagctggcagagaagagcacagcgcacttctcctctgtgacagactcagtgcccttccgctcacaccgcttgatcttcttgagaagcaggttcttgaacagggcagagcagcagttcccaggaatgctgttctccaagggcacagtgttgttgatgatttctccagtgctttctgctccagccccaggaccctgaggcacactcagctcccgcgcctgcttctctgtcaccatgtcggccctgaccagcggaggcttggctggggcccccaggaacctcaagcccaacaggaatcgaactccagcctggaacttggtctgagtcttcagtacctgggggggctgcttctccaccaggaagcaactggtgacgagggttctcaggacttcatccagccggccagtcagcgatgcccgggtcttgggctcaagctccccaccagccgcccctacctcctgctgtagctgggaataaatgtccaccaggctttcacacctctcctggagtggggccaggctctcctcaaacggtgcgccattccctgccagctgctgctgccgtttccaaatctggatcctcttcagcactagggctttggctgcctctagctctccagtggtctcctgcagtagcatggccagggcctcacttggcccagtcccattagcaggagtttctatcaagctgtgcagagacacttggccagcctcagcccccttctgcagggcttctcggagaaggtggatctcccctactcggtgctgcagcctccgcaagcctgtcttaaacttgagttcttcctgcttccagtggaaaggcattggcaagtggcggaactgttccataacagcttttttctctccttgaagtatttgtctgaaagtggccaccagcttcagggggtccctctgatatatgctctcaagggtgctgatgtgttgcaagatggtgctcccctccccctgctctcccaccgaggcctgaaggtgctggacagtgtctgaaagtagggcactagccaagttgcagcagaaggcgtcggagccgaccaggaactcccagggctggctctccagccagtcacccagaagatgccgcaggtgttggggaaagtcgacatagagccgctgcactttttctgggggcatcttggagaccagaccccacagagacatgatctgggacttggaggttgcctcggcaacccctctgctgtcttctccctttctcagcgggcacttccaggccccataggtctgtagctctgtccagcgagttcaaggctggccctgctagcacctccccccttccaccaccaccaccaaaaagaaaaataagataaagcacacacatacatacacacacacacacacacacacacacacactcctctcccgtcctccctcttcagtgtaagcagtggctgcccc

SEQ ID NO: 19221 - RNA, 1557 nt, Homo sapiens
  source 1..1557: mol_type = other RNA
tgtgaggttggcattgttgtcttggttgccatggacgatgaccaccaggggcagagacagggcctggagctggatggggagtttgccggggccaagtgtgaagctggcagagaagagcacagcgcacttctcctctgtgacagactcagtgcccttccgctcacaccgcttgatcttcttgagaagcaggttcttgaacagggcagagcagcagttcccaggaatgctgttctccaagggcacagtgttgttgatgatttctccagtgctttctgctccagccccaggaccctgaggcacactcagctcccgcgcctgcttctctgtcaccatgtcggccctgaccagcggaggcttggctggggcccccaggaacctcaagcccaacaggaatcgaactccagcctggaacttggtctgagtcttcagtacctgggggggctgcttctccaccaggaagcaactggtgacgagggttctcaggacttcatccagccggccagtcagcgatgcccgggtcttgggctcaagctccccaccagccgcccctacctcctgctgtagctgggaataaatgtccaccaggctttcacacctctcctggagtggggccaggctctcctcaaacggtgcgccattccctgccagctgctgctgccgtttccaaatctggatcctcttcagcactagggctttggctgcctctagctctccagtggtctcctgcagtagcatggccagggcctcacttggcccagtcccattagcaggagtttctatcaagctgtgcagagacacttggccagcctcagcccccttctgcagggcttctcggagaaggtggatctcccctactcggtgctgcagcctccgcaagcctgtcttaaacttgagttcttcctgcttccagtggaaaggcattggcaagtggcggaactgttccataacagcttttttctctccttgaagtatttgtctgaaagtggccaccagcttcagggggtccctctgatatatgctctcaagggtgctgatgtgttgcaagatggtgctcccctccccctgctctcccaccgaggcctgaaggtgctggacagtgtctgaaagtagggcactagccaagttgcagcagaaggcgtcggagccgaccaggaactcccagggctggctctccagccagtcacccagaagatgccgcaggtgttggggaaagtcgacatagagccgctgcactttttctgggggcatcttggagaccagaccccacagagacatgatctgggacttggaggttgcctcggcaacccctctgctgtcttctccctttctcagcgggcacttccaggccccataggtctgtagctctgtccagcgagttcaaggctggccctgctagcacctccccccttccaccaccaccaccaaaaagaaaaataagataaagcacacacatacatacacacacacacacacacacacacacacactcctctcccgtcctccctcttcagtgtaagcagtggctgccccagcccgctgtttccggcttctccttct

SEQ ID NO: 19222 - RNA, 1751 nt, Homo sapiens
  source 1..1751: mol_type = other RNA
tgtgaggttggcattgttgtcttggttgccatggacgatgaccaccaggggcagagacagggcctggagctggatggggagtttgccggggccaagtgtgaagctggcagagaagagcacagcgcacttctcctctgtgacagactcagtgcccttccgctcacaccgcttgatcttcttgagaagcaggttcttgaacagggcagagcagcagttcccaggaatgctgttctccaagggcacagtgttgttgatgatttctccagtgctttctgctccagccccaggaccctgaggcacactcagctcccgcgcctgcttctctgtcaccatgtcggccctgaccagcggaggcttggctggggcccccaggaacctcaagcccaacaggaatcgaactccagcctggaacttggtctgagtcttcagtacctgggggggctgcttctccaccaggaagcaactggtgacgagggttctcaggacttcatccagccggccagtcagcgatgcccgggtcttgggctcaagctccccaccagccgcccctacctcctgctgtagctgggaataaatgtccaccaggctttcacacctctcctggagtggggccaggctctcctcaaacggtgcgccattccctgccagctgctgctgccgtttccaaatctggatcctcttcagcactagggctttggctgcctctagctctccagtggtctcctgcagtagcatggccagggcctcacttggcccagtcccattagcaggagtttctatcaagctgtgcagagacacttggccagcctcagcccccttctgcagggcttctcggagaaggtggatctcccctactcggtgctgcagcctccgcaagcctgtcttaaacttgagttcttcctgcttccagtggaaaggcattggcaagtggcggaactgttccataacagcttttttctctccttgaagtatttgtctgaaagtggccaccagcttcagggggtccctctgatatatgctctcaagggtgctgatgtgttgcaagatggtgctcccctccccctgctctcccaccgaggcctgaaggtgctggacagtgtctgaaagtagggcactagccaagttgcagcagaaggcgtcggagccgaccaggaactcccagggctggctctccagccagtcacccagaagatgccgcaggtgttggggaaagtcgacatagagccgctgcactttttctgggggcatcttggagaccagaccccacagagacatgatctgggacttggaggttgcctctcccaggcctctcagagggatggaaaatggagaggtcccttctctggacgtttctgctccaagaccttcatgcccctctttcctccagtgcccacttaccccagctcttttctcctcaaggcagaatccttacccctcctgctcaggttcctccaataggcctttctctcggcaacccctctgctgtcttctccctttctcagcgggcacttccaggccccataggtctgtagctctgtccagcgagttcaaggctggccctgctagcacctccccccttccaccaccaccaccaaaaagaaaaataagataaagcacacacatacatacacacacacacacacacacacacacacactcctctcccgtcctccctcttcagtgtaagcagtggctgccccagcccgctgtttccggcttctccttctacccaggtccctccctggagctct

SEQ ID NO: 19223 - RNA, 1393 nt, Homo sapiens
  source 1..1393: mol_type = other RNA
tgtgaggttggcattgttgtcttggttgccatggacgatgaccaccaggggcagagacagggcctggagctggatggggagtttgccggggccaagtgtgaagctggcagagaagagcacagcgcacttctcctctgtgacagactcagtgcccttccgctcacaccgcttgatcttcttgagaagcaggttcttgaacagggcagagcagcagttcccaggaatgctgttctccaagggcacagtgttgttgatgatttctccagtgctttctgctccagccccaggaccctgaggcacactcagctcccgcgcctgcttctctgtcaccatgtcggccctgaccagcggaggcttggctggggcccccaggaacctcaagcccaacaggaatcgaactccagcctggaacttggtctgagtcttcagtacctgggggggctgcttctccaccaggaagcaactggtgacgagggttctcaggacttcatccagccggccagtcagcgatgcccgggtcttgggctcaagctccccaccagccgcccctacctcctgctgtagctgggaataaatgtccaccaggctttcacacctctcctggagtggggccaggctctcctcaaacggtgcgccattccctgccagctgctgctgccgtttccaaatctggatcctcttcagcactagggctttggctgcctctagctctccagtggtctcctgcagtagcatggccagggcctcacttggcccagtcccattagcaggagtttctatcaagctgtgcagagacacttggccagcctcagcccccttctgcagggcttctcggagaaggtggatctcccctactcggtgctgcagcctccgcaagcctgtcttaaacttgagttcttcctgcttccagtggaaaggcattggcaagtggcggaactgttccataacagcttttttctctccttgaagtatttgtctgaaagtggccaccagcttcagggggtccctctgatatatgctctcaagggtgctgatgtgttgcaagatggtgctcccctccccctgctctcccaccgaggcctgaaggtgctggacagtgtctgaaagtagggcactagccaagttgcagcagaaggcgtcggagccgaccaggaactccctcggcaacccctctgctgtcttctccctttctcagcgggcacttccaggccccataggtctgtagctctgtccagcgagttcaaggctggccctgctagcacctccccccttccaccaccaccaccaaaaagaaaaataagataaagcacacacatacatacacacacacacacacacacacacacacactcctctcccgtcctccctcttcagtgtaagcagtggctgcccc

SEQ ID NO: 19224 - RNA, 1254 nt, Homo sapiens
  source 1..1254: mol_type = other RNA
tgtgaggttggcattgttgtcttggttgccatggacgatgaccaccaggggcagagacagggcctggagctggatggggagtttgccggggccaagtgtgaagctggcagagaagagcacagcgcacttctcctctgtgacagactcagtgcccttccgctcacaccgcttgatcttcttgagaagcaggttcttgaacagggcagagcagcagttcccaggaatgctgttctccaagggcacagtgttgttgatgatttctccagtgctttctgctccagccccaggaccctgaggcacactcagctcccgcgcctgcttctctgtcaccatgtcggccctgaccagcggaggcttggctggggcccccaggaacctcaagcccaacaggaatcgaactccagcctggaacttggtctgagtcttcagtacctgggggggctgcttctccaccaggaagcaactggtgacgagggttctcaggacttcatccagccggccagtcagcgatgcccgggtcttgggctcaagctccccaccagccgcccctacctcctgctgtagctgggaataaatgtccaccaggctttcacacctctcctggagtggggccaggctctcctcaaacggtgcgccattccctgccagctgctgctgccgtttccaaatctggatcctcttcagcactagggctttggctgcctctagctctccagtggtctcctgcagtagcatggccagggcctcacttggcccagtcccattagcaggagtttctatcaagctgtgcagagacacttggccagcctcagcccccttctgcagggcttctcggagaaggtggatctcccctactcggtgctgcagcctccgcaagcctgtcttaaacttgagttcttcctgcttccagtggaaaggcattggcaagtggcggaactgttccataacagcttttttctctccttgaagtatttgtctgaaagtggccaccagcttcagggggtccctctgatatatgctctcggcaacccctctgctgtcttctccctttctcagcgggcacttccaggccccataggtctgtagctctgtccagcgagttcaaggctggccctgctagcacctccccccttccaccaccaccaccaaaaagaaaaataagataaagcacacacatacatacacacacacacacacacacacacacacactcctctcccgtcctccctcttcagtgtaagcagtggctgcccc

SEQ ID NO: 19225 - RNA, 79 nt, Homo sapiens
  source 1..79: mol_type = other RNA
tgtgaggttgtcatgcctgctggcatagctgtagtaatagcaggcatgacaacctcacactttttgcaaaatacttctt

SEQ ID NO: 19226 - RNA, 1333 nt, Homo sapiens
  source 1..1333: mol_type = other RNA
tgtgcaaatccatgcaaaactgaatccccaggtgtgtccagggccccagagccggagcacaggaggcactggcttggctgccgtcctttcttgtaactgcccaccaagtgccgcctgacgtgaatcccagcctcctcgcggtgccgtccgagctctgggctttgtgtgtgtcatgtccaagttgacaagtggctgtgctgtgagcgtcactgtcctcctccccctcatctttcaggaaactgctgtgactttaaagccggtcctcgccgcttcccgcacacctcgccgcttcccgcgcacctcgccgcttcccgcacaccaccaggcttgtgcttcccggagctgggtctgtgcacgtggcatccgtgcctctaaaggcgttgcaggccggtaagaggccctgctattttccattcatcccataagcgtttttaaatctcagggactgtgctcagcactggaaataatttctagaacatgattcttgaccagccaagcctgcaccggtggttccactctcaaggcattttaaagcaaggtaacaaatgtatgttgaccagctgggcacccatttctgttctggcatgagtaggagcagccacaggctgtggggcgggcaccctctaaacagagccctgcagaaggggctcctccatcacgcgccgagcctgccacacagaggagaggacgctccggagagagaggagcgcagagcctgtgcagatctgccatctcctcctccctaggggatgctcctggcccttgtgtgggtgaacgggtgccgtgatgtggccatgaggcgcacggacctctggactcaacgtggcctctccataggcgtgttaaaaatggtgccgagaatcaggcagggaggacaaggcctttgcagagctggtgagcaggaccgggacggagactccacggttaagcagcacagctgacttcctccacccggtccgccgtgtggggcagcttttcagctgcaggagccttaaatcaagtactgagataaccctgcacttccggccaggcctccagtgacctttctcagggcctcagcagcccccaaggccccgagggacatggcagcctgctctgtgaaacgtcctgtctgttctgcattgtcctgggcctcctcccagcccttcccacaacgcccaggccagctccaacagaggggaagttggccttcaccatccagcgaggcagggtcctggggtcgggcatctttgagccaggggctggggcagtcctgacagctccacctgctcatgccatgccttgcagcctccctgcccgtccgatcgcctgagtcaggcgtggtcctggcctc

SEQ ID NO: 19227 - RNA, 32 nt, Homo sapiens
  source 1..32: mol_type = other RNA
tgtggaaggtagacggccagagaggtgacccc

SEQ ID NO: 19228 - RNA, 605 nt, Homo sapiens
  source 1..605: mol_type = other RNA
tgtggacagtgaggtagagggagttggcgagacccttgtcctctgaggggtagcggcccggcctctccctgctggccccactgccactgcctcgggggccagggaaactgccctggctgcccccaccccctgtgcgggtacccacgctcttcatggcaaactcctgggcatgggccaccccactgcccacgctgcccatggccaggcgggggtccgggggtccaagctcggagggccgtggggcaaaggccaggagaggatcccgccctgggtcagcgcgcacaggcagcgtctccagcttcgccatgactaagccaggggggcacagcgcaggcttctctccttgcctttccaaggggttgaggggccgacgggtcctcaagcctgggaccctccgaggcccggtctgcaggggccatgtgcctcactctcgcagtcggggctcggcccgaaccagctgcgcgactttggaggggccgactgagccatcccggactgcagttttctccttcgctgcctcagggtccggcgcggggtctccgacacgggcgccaccggccccgcttgctggcgcagcccgaagcacgcccggcggggcgcgctgc

SEQ ID NO: 19229 - RNA, 644 nt, Homo sapiens
  source 1..644: mol_type = other RNA
tgtggacagtgaggtagagggagttggcgagacccttgtcctctgaggggtagcggcccggcctctccctgctggccccactgccactgcctcgggggccagggaaactgccctggctgcccccaccccctgtgcgggtacccacgctcttcatggcaaactcctgggcatgggccaccccactgcccacgctgcccatggccaggcgggggtccgggggtccaagctcggagggccgtggggcaaaggccaggagaggatcccgccctgggtcagcgcgcacaggcagcgtctccagcttcgccatgactaagccaggggggcactaagtgttgcagtcagggcagaagtggaagctcactaccagcgcaggcttctctccttgcctttccaaggggttgaggggccgacgggtcctcaagcctgggaccctccgaggcccggtctgcaggggccatgtgcctcactctcgcagtcggggctcggcccgaaccagctgcgcgactttggaggggccgactgagccatcccggactgcagttttctccttcgctgcctcagggtccggcgcggggtctccgacacgggcgccaccggccccgcttgctggcgcagcccgaagcacgcccggcggggcgcgctgc

SEQ ID NO: 19230 - RNA, 639 nt, Homo sapiens
  source 1..639: mol_type = other RNA
tgtggacagtgaggtagagggagttggcgagacccttgtcctctgaggggtagcggcccggcctctccctgctggccccactgccactgcctcgggggccagggaaactgccctggctgcccccaccccctgtgcgggtacccacgctcttcatggcaaactcctgggcatgggccaccccactgcccacgctgcccatggccaggcgggggtccgggggtccaagctcggagggccgtggggcaaaggccaggagaggatcccgccctgggtcagcgcgcacaggcagcgtctccagcttcgccatgactaagccaggggggcacttgcggggctgccgcgtgccaggcgccccgaggcggcgagcgcctgaggaaacgggggtctgggggagggtgggtaggcgacgcacatctgggtcgcgggtgggcgccgccaagggcacagcctgtccctcccggatggacgggggccgcggctgcagtaggtggcaggcctgccctccccaaggtcttcccagctcggccgcaccggggccctgggaagacagggcccccttcccgggatcagtcctccgcagaggtcccagggctggctgaggccggggcaggggacgcagtggcgccagctgctggcact

SEQ ID NO: 19231 - RNA, 2267 nt, Homo sapiens
  source 1..2267: mol_type = other RNA
tgtggacagtgaggtagagggagttggcgagacccttgtcctctgaggggtagcggcccggcctctccctgctggccccactgccactgcctcgggggccagggaaactgccctggctgcccccaccccctgtgcgggtacccacgctcttcatggcaaactcctgggcatgggccaccccactgcccacgctgcccatggccaggcgggggtccgggggtccaagctcggagggccgtggggcaaaggccaggagaggatcccgccctgggtcagcgcgcacaggcagcgtctccagcttcgccatgactaagccaggggggcactttccaaggggttgaggggccgacgggtcctcaagcctgggaccctccgaggcccggtctgcaggggccatgtgcctcactctcgcagtcggggctcggcccgaaccagctgcgcgactttggaggggccgactgagccatcccggactgcagttttctcctatctgggtcgcgggtgggcgccgccaagggcacagcctgtccctcccggatggacgggggccgcggctgcagtaggtggcaggcctgccctccccaaggtcttcccagctcggccgcaccggggccctgggaagacagggcccccttcccgggatcagtcctccgcagaggtcccagggctggctgaggccggggcaggggacgcagtggcgccagctgctggcactgacggagcctctctcagggcctgcgtttcccacaggtgggaggggggaggggaggggaggggccgctgcagggtgcgcggccccaaggatcctgcgcctgccgaaccccgcaaagaattcactgccaccaggaagacttcccggattactaccctctcccgctccctgtggaccttgaccctgctcagcttaccgtgaagccctctgagtccttctgtgggtgcgcgtccccctcccccaaggccggcccacaagcgcagggggagccaggcctcgggttacctgtgctcagggaggccgtgcttcctcgttcctttgtctcaagttcgcacctgggaacacctgccccagagatctgcataatgcagccgggcaggagcaccaggcagtgtctgcctcgggttagaccctcaaataagtgtgtgggaaatgggagagggcgcccttcaggccttttcccactacaccctgcataaaccaggcagggagccctccttccctatcaagttaaggggcccacgtggcaccctatggccccacagaccgtcttctacccagatgcccagttctaatgctgagtccctggcccagaccaagggcacctgacaaaactgttgtccttcgggagtcttctggcccccacaccaggaatgagagctctaggttgttggaaagttcactaccaagcctgtccactgtctctgtagaattccattctcagcatctgtccccacaggtgtggagaagagcacttcgccaccctcctcccttggacccgtctgtccccataagcaagggccaggactaggatgaggacagagagccacgtagggcacaaatgaagggcacaaacagcaagtacacagccctgagggtgacagcctccttccctttgtgccttgggtccctctctggcctcactctagtccctgctctgcctctactccccagcatactccagccccctatgcctcagccctgcaaccccctcctaccttaagtatggacccttctcttgccacctctgggtgcaatgtggggagcagctggggactgggaggatgaagcctgaaaggcctgaggcttggaaccagtaggaaggcctgggcagggtttgggaaagaactggcaaaatttcatacagatgaggtcaggtggtggggacaagggataatgctggactgggcaccagcgtgcgtgtgacactgttaacatgatagggggagactgcttggggaaaatagttgctttgggaaacaccagaggaagatacctctcaagcactaaatggaggccaagcaaggtggctcatgcctgtaatcccagcactttgggaggtcaaggtgggcagattacttgaggccaagagttcaagaccatcctggccaaattggtggaaccccatctctactaaaaatacaaaaattagctgggtgcggtatgcattcctgtaatcccagctacttgggaggctgaggcacgagaacccccttgaacccaggaggcagaggttgcagtgagctgtaattgcaccactgcactccagcctggg

SEQ ID NO: 19232 - RNA, 1847 nt, Homo sapiens
  source 1..1847: mol_type = other RNA
tgtggacagtgaggtagagggagttggcgagacccttgtcctctgaggggtagcggcccggcctctccctgctggccccactgccactgcctcgggggccagggaaactgccctggctgcccccaccccctgtgcgggtacccacgctcttcatggcaaactcctgggcatgggccaccccactgcccacgctgcccatggccaggcgggggtccgggggtccaagctcggagggccgtggggcaaaggccaggagaggatcccgccctgggtcagcgcgcacaggcagcgtctccagcttcgccatgactaagccaggggggcactttccaaggggttgaggggccgacgggtcctcaagcctgggaccctccgaggcccggtctgcaggggccatgtgcctcactctcgcagtcggggctcggcccgaaccagctgcgcgactttggaggggccgactgagccatcccggactgcagttttctcctcgtgaagccctctgagtccttctgtgggtgcgcgtccccctcccccaaggccggcccacaagcgcagggggagccaggcctcgggttacctgtgctcagggaggccgtgcttcctcgttcctttgtctcaagttcgcacctgggaacacctgccccagagatctgcataatgcagccgggcaggagcaccaggcagtgtctgcctcgggttagaccctcaaataagtgtgtgggaaatgggagagggcgcccttcaggccttttcccactacaccctgcataaaccaggcagggagccctccttccctatcaagttaaggggcccacgtggcaccctatggccccacagaccgtcttctacccagatgcccagttctaatgctgagtccctggcccagaccaagggcacctgacaaaactgttgtccttcgggagtcttctggcccccacaccaggaatgagagctctaggttgttggaaagttcactaccaagcctgtccactgtctctgtagaattccattctcagcatctgtccccacaggtgtggagaagagcacttcgccaccctcctcccttggacccgtctgtccccataagcaagggccaggactaggatgaggacagagagccacgtagggcacaaatgaagggcacaaacagcaagtacacagccctgagggtgacagcctccttccctttgtgccttgggtccctctctggcctcactctagtccctgctctgcctctactccccagcatactccagccccctatgcctcagccctgcaaccccctcctaccttaagtatggacccttctcttgccacctctgggtgcaatgtggggagcagctggggactgggaggatgaagcctgaaaggcctgaggcttggaaccagtaggaaggcctgggcagggtttgggaaagaactggcaaaatttcatacagatgaggtcaggtggtggggacaagggataatgctggactgggcaccagcgtgcgtgtgacactgttaacatgatagggggagactgcttggggaaaatagttgctttgggaaacaccagaggaagatacctctcaagcactaaatggaggccaagcaaggtggctcatgcctgtaatcccagcactttgggaggtcaaggtgggcagattacttgaggccaagagttcaagaccatcctggccaaattggtggaaccccatctctactaaaaatacaaaaattagctgggtgcggtatgcattcctgtaatcccagctacttgggaggctgaggcacgagaacccccttgaacccaggaggcagaggttgcagtgagctgtaattgcaccactgcactccagcctggg

SEQ ID NO: 19233 - RNA, 583 nt, Homo sapiens
  source 1..583: mol_type = other RNA
tgtggacagtgaggtagagggagttggcgagacccttgtcctctgaggggtagcggcccggcctctccctgctggccccactgccactgcctcgggggccagggaaactgccctggctgcccccaccccctgtgcgggtacccacgctcttcatggcaaactcctgggcatgggccaccccactgcccacgctgcccatggccaggcgggggtccgggggtccaagctcggagggccgtggggcaaaggccaggagaggatcccgccctgggtcagcgcgcacaggcagcgtctccagcttcgccatgactaagccaggggggcactttccaaggggttgaggggccgacgggtcctcaagcctgggaccctccgaggcccggtctgcaggggccatgtgcctcactctcgcagtcggggctcggcccgaaccagctgcgcgactttggaggggccgactgagccatcccggactgcagttttctccttcgctgcctcagggtccggcgcggggtctccgacacgggcgccaccggccccgcttgctggcgcagcccgaagcacgcccggcggggcgcgctgc

SEQ ID NO: 19234 - RNA, 420 nt, Homo sapiens
  source 1..420: mol_type = other RNA
tgtggacagtgaggtagagggagttggcgagacccttgtcctctgaggggtagcggcccggcctctccctgctggccccactgccactgcctcgggggccagggaaactgccctggctgcccccaccccctgtgcgggtacccacgctcttcatggcaaactcctgggcatgggccaccccactgcccacgctgcccatggccaggcgggggtccgggggtccaagctcggagggccgtggggcaaaggccaggagaggatcccgccctgggtcagcgcgcacaggcagcgtctccagcttcgccatgactaagccaggggggcatcgctgcctcagggtccggcgcggggtctccgacacgggcgccaccggccccgcttgctggcgcagcccgaagcacgcccggcggggcgcgctgc

SEQ ID NO: 19235 - RNA, 87 nt, Homo sapiens
  source 1..87: mol_type = other RNA
tgtggtagatatatgcacgatataggtatgtatgtatgtatgtataaaagcagggcagtatatatatcgtgcatatatctaccacat

SEQ ID NO: 19236 - RNA, 87 nt, Homo sapiens
  source 1..87: mol_type = other RNA
tgtggtagatatatgcacgatatatatactgccctgcttttatacatacatacatacatacctatatcgtgcatatatctaccacat

SEQ ID NO: 19237 - RNA, 51 nt, Homo sapiens
  source 1..51: mol_type = other RNA
tgtgtcccattattggtgatttcagatttcattatttaattatgggacaca

SEQ ID NO: 19238 - RNA, 2854 nt, Homo sapiens
  source 1..2854: mol_type = other RNA
tgtgtccgggaagtggaggaggaagaggaaagagaggggactaaggttctcccagtttaaggttttgttccaatgaggggatgaggaagtatgaagatatttttgttgtcttttcatctttatactgtgttaagtaatgcttacaacataaattcagcaggcttttcctgagctgtaactcagaagttttcgtcctgcaaacaatgtatttacaaatgtgtttattagcttacacagcaatctcacaataactagtaaagattaaaagggcacactcctagtatatttgtttgcagtgttttaagggaaatacatattgccatggtgaagctctaaatagattcaacgaaacatctgaagattgaaagttgttaaaaaaaaaaaaggcaaagaaataaatatcaccaaagaaaaaagattaattgtagcttaaatataaaactaaatcaccagttaattaaactatacagatctaatacaaaccaaaaccagcctgaaagacccaaccttaaaaaatgctaaaaaataaggcataaatctgcataatattgagttttatttccattctctcctttccctctactatgtatgctttacctgatctgcctctaggggcttacaagaaaacggtttccggtttccgtcttcaatttgacctcaaatgtcctgagcaaagtttttgttattctgctgagggttcttttgttggtaagctttagacatcattatttctactaattcagtagttttgatcgtagcgccaaatttaaattcttccactggttcttctggaaggaattaaaacttttacagtgccttgcctgcacagtattatgtttttaaaaaagaaaacccaagcaaaatctattgcttaaagaggtttcttattttttaaacaaacagaataactcttgacaattttaaaaccttgggagaaacagttcattagaacttcattttcttaccgtgaagaattaaatactaaaaacctgttctgaagcacttggttaattttctctcccagagtctaataaagcacatgtgaaagagccatttgttttagtcagaaatacatcttatgttcttctacttctaagtactcagtatgttctttaggactcattttgaagatgcaccaggagccttttctcattcaagcactgcctaccatgatggctgaattttgacctcaaagaagaccgtaatttatatcagtgctcaagaataattttggacatcttggtccgtagcctacagcaagtggtatctgtaaaattaaaggataattccaatgggcttggtagaactgctgctttgccatctcttgtttgttttgaggaagtcgggggaggctaggtaagaatagggtaatagggaatgggggtaagtgagaggtgagaaaagcaaggagagataaagtaggctgtgaacataccgctcgttaaccaagccatactcatactgttgagatttccatcattttgaagtacattatcataacattaaaaaagaaaaaaatgttaagaaaatgtatctaatttttaaagttatcactggaatatgctgaaatattttggctttttgtaaaatataaataatgaagacactgacttttgttgtgcttgtgaagctaatagatcatctccacgagacaggcagcaatgatgaattgcaatacgttattactgaagggaaaaggttcaagccaatattcacactgcagtcaatgaaagagtaagggggccaaagcagtgagcttctgaagaaggttgaagatgacatgggagattagcaggaacagcctccttcactgactggttgctcctgaggcttttccagttttatgtcaatcatatcttctctgcttctgtcctgtgtgctttccattcccggcaaagctgctgctacacgtcgaaagagctgctttacattgtatccagcttttgcactagtttcaataaacataacattcagctctttggctttcctctctccctcctcaattgacacttgcctcttgtcagcaagatctgttttatttcctactagcatgatgataacatcacttcctctttctgttctgacatcatcaatccactttgtagtttgctggaatgagttaacatttgtgatatcataaacaacaactgccacagtggagtcacgaatgtagctaggaatcaagctcctgaaccgctcttgacctgctgtgtcccataattgcaatcgtactgttcgatcctccaagtacatagtttttgataaaaagtcaatgccaattgttgcctgataggtgttgtcaaaactgtcatacatgaatctggtgatcaaagatgtctttccaacgctttgctcccccaggaacaccagcttgaatttcctcagcggattcccgaagtctccgcccgtggacattgtggaactagaggagcggccgccgcctcagcctagagacctcccggaccgatgctgctccagccagctgacgaaaaaggcgagcggaagggcgggcaccgagctctctcggcccctgcaaggcccggtggaggagcccggctggagggcagcaggactctccacagactggcagccgccgccgcctcccggcagagtagcctagcaccgagcgaggcccgcggctgggaagggaaggagggcggtgtcggcaggagccaggggtgtcctctggcttcccaaagctagggccgttccctccttccgcactcggctcccagacctggggaagagaagctgagggtggcggagccggaaccgcagacgtatctgggacctctcacgcgcagcgcctgagcttccacagctgccgccgccgccgcagcccaacctgctgagt

SEQ ID NO: 19239 - RNA, 2854 nt, Homo sapiens
  source 1..2854: mol_type = other RNA
tgtgtccgggaagtggaggaggaagaggaaagagaggggactaaggttctcccagtttaaggttttgttccaatgaggggatgaggaagtatgaagatatttttgttgtcttttcatctttatactgtgttaagtaatgcttacaacataaattcagcaggcttttcctgagctgtaactcagaagttttcgtcctgcaaacaatgtatttacaaatgtgtttattagcttacacagcaatctcacaataactagtaaagattaaaagggcacactcctagtatatttgtttgcagtgttttaagggaaatacatattgccatggtgaagctctaaatagattcaacgaaacatctgaagattgaaagttgttaaaaaaaaaaaaggcaaagaaataaatatcaccaaagaaaaaagattaattgtagcttaaatataaaactaaatcaccagttaattaaactatacagatctaatacaaaccaaaaccagcctgaaagacccaaccttaaaaaatgctaaaaaataaggcataaatctgcataatattgagttttatttccattctctcctttccctctactatgtatgctttacctgatctgcctctaggggcttacaagaaaacggtttccggtttccgtcttcaatttgacctcaaatgtcctgagcaaagtttttgttattctgctgagggttcttttgttggtaagctttagacatcattatttctactaattcagtagttttgatcgtagcgccaaatttaaattcttccactggttcttctggaaggaattaaaacttttacagtgccttgcctgcacagtattatgtttttaaaaaagaaaacccaagcaaaatctattgcttaaagaggtttcttattttttaaacaaacagaataactcttgacaattttaaaaccttgggagaaacagttcattagaacttcattttcttaccgtgaagaattaaatactaaaaacctgttctgaagcacttggttaattttctctcccagagtctaataaagcacatgtgaaagagccatttgttttagtcagaaatacatcttatgttcttctacttctaagtactcagtatgttctttaggactcattttgaagatgcaccaggagccttttctcattcaagcactgcctaccatgatggctgaattttgacctcaaagaagaccgtaatttatatcagtgctcaagaataattttggacatcttggtccgtagcctacagcaagtggtatctgtaaaattaaaggataattccaatgggcttggtagaactgctgctttgccatctcttgtttgttttgaggaagtcgggggaggctaggtaagaatagggtaatagggaatgggggtaagtgagaggtgagaaaagcaaggagagataaagtaggctgtgaacataccgctcgttaaccaagccatactcatactgttgagatttccatcattttgaagtacattatcataacattaaaaaagaaaaaaatgttaagaaaatgtatctaatttttaaagttatcactggaatatgctgaaatattttggctttttgtaaaatataaataatgaagacactgacttttgttgtgcttgtgaagctaatagatcatctccacgagacaggcagcaatgatgaattgcaatacgttattactgaagggaaaaggttcaagccaatattcacactgcagtcaatgaaagagtaagggggccaaagcagtgagcttctgaagaaggttgaagatgacatgggagattagcaggaacagcctccttcactgactggttgctcctgaggcttttccagttttatgtcaatcatatcttctctgcttctgtcctgtgtgctttccattcccggcaaagctgctgctacacgtcgaaagagctgctttacattgtatccagcttttgcactagtttcaataaacataacattcagctctttggctttcctctctccctcctcaattgacacttgcctcttgtcagcaagatctgttttatttcctactagcatgatgataacatcacttcctctttctgttctgacatcatcaatccactttgtagtttgctggaatgagttaacatttgtgatatcgtaaactactacagctgcagcagaatcacggatgtaactgggaatgaggctacggaaacgttcctgacccgcagtatcccacagctgaagcctgattgttcgatcctccaagtacatagtttttgataaaaagtcaatgccaattgttgcctgataggtgttgtcaaaactgtcatacatgaatctggtgatcaaagatgtctttccaacgctttgctcccccaggaacaccagcttgaatttcctcagcggattcccgaagtctccgcccgtggacattgtggaactagaggagcggccgccgcctcagcctagagacctcccggaccgatgctgctccagccagctgacgaaaaaggcgagcggaagggcgggcaccgagctctctcggcccctgcaaggcccggtggaggagcccggctggagggcagcaggactctccacagactggcagccgccgccgcctcccggcagagtagcctagcaccgagcgaggcccgcggctgggaagggaaggagggcggtgtcggcaggagccaggggtgtcctctggcttcccaaagctagggccgttccctccttccgcactcggctcccagacctggggaagagaagctgagggtggcggagccggaaccgcagacgtatctgggacctctcacgcgcagcgcctgagcttccacagctgccgccgccgccgcagcccaacctgctgagt

SEQ ID NO: 19240 - RNA, 2393 nt, Homo sapiens
  source 1..2393: mol_type = other RNA
tgtgtccgggaagtggaggaggaagaggaaagagaggggactaaggttctcccagtttaaggttttgttccaatgaggggatgaggaagtatgaagatatttttgttgtcttttcatctttatactgtgttaagtaatgcttacaacataaattcagcaggcttttcctgagctgtaactcagaagttttcgtcctgcaaacaatgtatttacaaatgtgtttattagcttacacagcaatctcacaataactagtaaagattaaaagggcacactcctagtatatttgtttgcagtgttttaagggaaatacatattgccatggtgaagctctaaatagattcaacgaaacatctgaagattgaaagttgttaaaaaaaaaaaaggcaaagaaataaatatcaccaaagaaaaaagattaattgtagcttaaatataaaactaaatcaccagttaattaaactatacagatctaatacaaaccaaaaccagcctgaaagacccaaccttaaaaaatgctaaaaaataaggcataaatctgcataatattgagttttatttccattctctcctttccctctactatgtatgctttacctgatctgcctctaggggcttacaagaaaacggtttccggtttccgtcttcaatttgacctcaaatgtcctgagcaaagtttttgttattctgctgagggttcttttgttggtaagctttagacatcattatttctactaattcagtagttttgatcgtagcgccaaatttaaattcttccactggttcttctggaaggaattaaaacttttacagtgccttgcctgcacagtattatgtttttaaaaaagaaaacccaagcaaaatctattgcttaaagaggtttcttattttttaaacaaacagaataactcttgacaattttaaaaccttgggagaaacagttcattagaacttcattttcttaccgtgaagaattaaatactaaaaacctgttctgaagcacttggttaattttctctcccagagtctaataaagcacatgtgaaagagccatttgttttagtcagaaatacatcttatgttcttctacttctaagtactcagtatgttctttaggactcattttgaagatgcaccaggagccttttctcattcaagcactgcctaccatgatggctgaattttgacctcaaagaagaccgtaatttatatcagtgctcaagaataattttggacatcttggtccgtagcctacagcaagtggtatctgtaaaattaaaggataattccaatgggcttggtagaactgctgctttgccatctcttgtttgttttgaggaagtcgggggaggctaggtaagaatagggtaatagggaatgggggtaagtgagaggtgagaaaagcaaggagagataaagtaggctgtgaacataccgctcgttaaccaagccatactcatactgttgagatttccatcattttgaagtacattatcataacattaaaaaagaaaaaaatgttaagaaaatgtatctaatttttaaagttatcactggaatatgctgaaatattttggctttttgtaaaatataaataatgaagacactgacttttgttgtgcttgtgaagctaatagatcatctccacgagacaggcagcaatgatgaattgcaatacgttattactgaagggaaaaggttcaagccaatattcacactgcagtcaatgaaagagtaagggggccaaagcagtgagcttctgaagaaggttgaagatgacatgggagattagcaggaacagcctccttcactgactggttgctcctgaggcttttccagttttatgtcaatcatatcttctctgcttctgtcctgtgtgctttccattcccggcaaagctgctgctacacgtcgaaagagctgctttacattgtatccagcttttgcactagtttcaataaacataacattcagctctttggctttcctctctccctcctcaattgacacttgcctcttgtcagcaagatctgttttatttcctactagcatgatgataacatcacttcctctttctgttctgacatcatcaatccactttgtagtttgctggaatgagttaacatttgtgatatcgtaaactactacagctgcagcagaatcacggatgtaactgggaatgaggctacggaaacgttcctgacccgcagtatcccacagctgaagcctgattgttcgatcctccaagtacatagtttttgataaaaagtcaatgccaattgttgcctgataggtgttgtcaaaactgtcatacatgaatctggtgatcaaagatgtctttccaacttccacgacatcagcacttcgcagggccaagcctctggggaaaacaa

SEQ ID NO: 19241 - RNA, 2542 nt, Homo sapiens
  source 1..2542: mol_type = other RNA
tgtgtccgggaagtggaggaggaagaggaaagagaggggactaaggttctcccagtttaaggttttgttccaatgaggggatgaggaagtatgaagatatttttgttgtcttttcatctttatactgtgttaagtaatgcttacaacataaattcagcaggcttttcctgagctgtaactcagaagttttcgtcctgcaaacaatgtatttacaaatgtgtttattagcttacacagcaatctcacaataactagtaaagattaaaagggcacactcctagtatatttgtttgcagtgttttaagggaaatacatattgccatggtgaagctctaaatagattcaacgaaacatctgaagattgaaagttgttaaaaaaaaaaaaggcaaagaaataaatatcaccaaagaaaaaagattaattgtagcttaaatataaaactaaatcaccagttaattaaactatacagatctaatacaaaccaaaaccagcctgaaagacccaaccttaaaaaatgctaaaaaataaggcataaatctgcataatattgagttttatttccattctctcctttccctctactatgtatgctttacctgatctgcctctaggggcttacaagaaaacggtttccggtttccgtcttcaatttgacctcaaatgtcctgagcaaagtttttgttattctgctgagggttcttttgttggtaagctttagacatcattatttctactaattcagtagttttgatcgtagcgccaaatttaaattcttccactggttcttctggaaggaattaaaacttttacagtgccttgcctgcacagtattatgtttttaaaaaagaaaacccaagcaaaatctattgcttaaagaggtttcttattttttaaacaaacagaataactcttgacaattttaaaaccttgggagaaacagttcattagaacttcattttcttaccgtgaagaattaaatactaaaaacctgttctgaagcacttggttaattttctctcccagagtctaataaagcacatgtgaaagagccatttgttttagtcagaaatacatcttatgttcttctacttctaagtactcagtatgttctttaggactcattttgaagatgcaccaggagccttttctcattcaagcactgcctaccatgatggctgaattttgacctcaaagaagaccgtaatttatatcagtgctcaagaataattttggacatcttggtccgtagcctacagcaagtggtatctgtaaaattaaaggataattccaatgggcttggtagaactgctgctttgccatctcttgtttgttttgaggaagtcgggggaggctaggtaagaatagggtaatagggaatgggggtaagtgagaggtgagaaaagcaaggagagataaagtaggctgtgaacataccgctcgttaaccaagccatactcatactgttgagatttccatcattttgaagtacattatcataacattaaaaaagaaaaaaatgttaagaaaatgtatctaatttttaaagttatcactggaatatgctgaaatattttggctttttgtaaaatataaataatgaagacactgacttttgttgtgcttgtgaagctaatagatcatctccacgagacaggcagcaatgatgaattgcaatacgttattactgaagggaaaaggttcaagccaatattcacactgcagtcaatgaaagagtaagggggccaaagcagtgagcttctgaagaaggttgaagatgacatgggagattagcaggaacagcctccttcactgactggttgctcctgaggcttttccagttttatgtcaatcatatcttctctgcttctgtcctgtgtgctttccattcccggcaaagctgctgctacacgtcgaaagagtgttcgatcctccaagtacatagtttttgataaaaagtcaatgccaattgttgcctgataggtgttgtcaaaactgtcatacatgaatctggtgatcaaagatgtctttccaacgctttgctcccccaggaacaccagcttgaatttcctcagcggattcccgaagtctccgcccgtggacattgtggaactagaggagcggccgccgcctcagcctagagacctcccggaccgatgctgctccagccagctgacgaaaaaggcgagcggaagggcgggcaccgagctctctcggcccctgcaaggcccggtggaggagcccggctggagggcagcaggactctccacagactggcagccgccgccgcctcccggcagagtagcctagcaccgagcgaggcccgcggctgggaagggaaggagggcggtgtcggcaggagccaggggtgtcctctggcttcccaaagctagggccgttccctccttccgcactcggctcccagacctggggaagagaagctgagggtggcggagccggaaccgcagacgtatctgggacctctcacgcgcagcgcctgagcttccacagctgccgccgccgccgcagcccaacctgctgagt

SEQ ID NO: 19242 - RNA, 2859 nt, Homo sapiens
  source 1..2859: mol_type = other RNA
tgtgtccgggaagtggaggaggaagaggaaagagaggggactaaggttctcccagtttaaggttttgttgcaatgaggggatgaggaagtatgaagatacttttgttgtcttttcatctttatactgtgttaagtaacgtttacaacataaattcagcaggcttttcctgacctgtaactcgaagttttcttcctgcaaacaatgtatttacaaatgtgtttattagcttacacagcaatctcacaataactagtaaagattaaaagggcacactcctagtatatttgtttgcagtgttttaagggaaatacatattgccatggtgaagctctaaatagattcaacgaaacatctaaaaatggaaagttgttaaaaaaaaaaaaagcaaagaaatatcgccaaagaaaaaatattaatcgtagcttaaatataaaactaaatcactagttaaactatacagatctaatacaaaccaaaaccagcctgaaagacccaaccttaaaaaatgctaaaaaataaggcataaatctgcataatattcagttttatttccattctctcctttccctctactatgtatgctttacctgatctgcctctaggggcttacaagaaaacggtttccggtttccgtcttccgtcttccgtcttcaatttgacctcaaatgtcctgagcaaagtttttgctattctgctgagggttcttttgctggtaagctttagatatcgttatttctgctaattcagtagttttgatcgtagtgccaaatttaaattcttccactggttcttctgtaaggaattaaacttttatggtgtcttgcctgcatagtattatttttttaagaaagaaaacccaagcaaaatctattgcttacagaggtttcttactttttaaacaaacagaataactcttgacaattttaaaaccttgggagaaatagttcattagaacttcattatcttaccatgaagaagtaaatactaaaaacctgttctgaagcacttggttacttttctctcccagagtctaataaagcacatgtgaaaggaccatttgtgttagtcagaaatacattttatgttctgctacttataagtactcagtatgttctttaggactcattttgaagatgcaccaggaggcttttctcattcaagcactgcctaccgtgatcgctgaattctgacctcaaagaagatctaagtaatttacatcagtgctcaagaataattctggacatcttggtccacagcctacagcaagtggtatctgtaaaattaaaggataattccagtgggcttggtcggactgctgctttgccatctcttgtttgttttgaggaagtggggggaggctaggtaagaacacggaaatagggaacggggtaagggagaggtgagaagagcaaggagagataaagcaggctgtgaacatactgctcgttaaccaagccatactcatactgttgagatttccatcattttgaagtacattatcataacattaaaaaagaaaaaaatgttaagaaaatgtatctaatttttaaagttatcaccggaatatgctgaaataatttggctttttgtaaaatataaataatgaagacgctgactttttttgtgcttgtgaagctaatagatcacctccacgagacaggcagcaatgatgaattgcaaaacgttattaatgaagggaaaaggttcaagccaatattcacactgcagtcaatgaaagagtaagggggcttctgaggaagggttgaagatgacatgggagagtagcaggaacaacccccttcgctgactgtttgctcctgaggcttttccagttttatgtcactcatgtcttctctgcttccgtcctgtgtgctttccattcccggcaaagctgctgctacacgtcgaaagagctgctttacattgtatccagcttttgccctagtttcaataaacgtaacattcagccctttggctttcctctctccctcctcaactgacacttgcctcttgtcagcaagatctgttctatttcctactagcgtgatgataacatcacttcctctttctgttctgacatcatcaatccactttgtagtttgctggaatgagttaacatttgtgatatcgtaaactactacagctgcagcagaatcacggatgtacctgggaatgaggctacggagacgttcctgacccgccgtatcccacagccgaagcccgattgttccatcctccaagtacatagtttttgataaaaagtcaatgccaattattgcctgataggtgttgtcaaaactgtcatacctgaatctggtgatcaaagatgtctttgcaacgctttgctcccccaggaacaccagcttgaatttcctcagcggattcccgaagtctccgcccgcggacatggtggaactagaggagctgtcgccgcctcagcccagagacctcccggaccgatgctcctccagccggctgacgaaaaaggcgagcggaagggcgggcgccgagctctctgcgcccctgcaagggccggtggaggagcccggctggaggagcccggctggagggcagcagggctcgccacagactggcagccgccgccgcctcccggcagagtagccgagcacggagcgaggcccgcggctgggaagggaaggagggcggtgtcggcaggagccaggggtgtgctttggcttcccaaggctagggccgttccctccttccgcacccggctcagagacctgcgggagagagacggagggtggcggagcccaaaccgcagatgtatccgggatctctcacgcgcggcgcttcggcttccccagccgccgccgccgcagcccaacctgctgagt

SEQ ID NO: 19243 - RNA, 2845 nt, Homo sapiens
  source 1..2845: mol_type = other RNA
tgtgtccgggaagtggaggaggaagaggaaagagaggggactaaggttctcccagtttaaggttttgttgcaatgaggggatgaggaagtatgaagatatttttgttgtcttttcatctttatactgtgttaagtaacgtttacaacataaattcagcaggcttttcctgacctataactcgaagttttcttcctgcaaacaatgtatttacaaatgtgtttattagcttacacagcaatctcacaataactagtgaagattaaaagggcacactcctagtatatttgtttgcagtgtttcaagggaaatacatattgccatggtgaagctctaaatagattcaacgaaacatctaaaaattgaaagttgttaaaaaaaaagcaaagaaatatcaccaaagaaaaaagattaatcgtagcttaaatataaaactaaatcattagttaattaaactatacagatctcatacaaacgaaaaccagcctgaaagacccaaccttaaaaaaatgctaaaaaataaggcataaatctgcataatattcagttttatttccattctctcctttccctctactatgtatgctttacctgatctgcctctaggggcttacaagaaaatggtttccggtttccatcttcaatttgacctcaaatgtcctgagcaaagtttttgctcttctgctgagggttcttttgttggtaagctttagatatcgttatttctgctaattcagtagttttgatcgtagtgccaaatttaaattcttccactggttcttctgtaaggaattaaacttttatggtgtcttgcctgcatagtattattttttaaaaaaagaaaacccaagcaaaatctattgcttaaagaggtttcttattttttaaacaaacagaataactcttgacaattttaaaaccttgggagaaatagttcattagaacgtcattatcttaccatgaagaattaaatactaaaaacctgttctgaagcacttggttaattttctctcccagagtctaataaagcacatgtgaaaggaccatttgttttagtcagaaatacattttatgttctgctacttataagtactcagtatgttctttaggactcattttgaagatgcaccaggaggcttttctcattcaagcactgcctaccgtgatcgctgaattctgacctcaaagaggatctaagtaatttatatcagtgctcaagaataattctggacatcttggtccacagcctacagcaagtggtatctgtaaaattaaaggataattccagtgggcttggtcggactgctgctttgccatctcttgtttgttttgaggaagtggggggaggctaggtaagaacacggaaatagggaacggggtaagggagaggtgagaagagcaaggagagataaagcaggctgtgaacatactgctcgttaaccaagccatactcatactgttgagatttccatcattttgaagtacattatcataacattaaaaaagaaaaaaaatgttaagaaaatgtatctaatttttaaagttatcactggaatacgctgaaatagtttggctttttgtaaaatataaataatgaagacgctgactttttttgtgcttgtcaagctaatagatcatctccacgagacaggcagcaatgatgaattgcaaaacgttattaatgaagggaaaaggttcaagccaatattcacactgcagtcaatgaaagagtaagggggcttctgaggaagggttgaagatgacatgggagagtagcaggaacaacccccttcgctgactgtttgctcctgaggcttttccagttttatgtcactcatgtcttctctgcttccgtcctgtgtgctttccattcccggcaaagctgctgctacacgtcgaaagagctgctttacattgtatccagcttttgccctagtttcaataaacgtaacattcagccctttggctttcctctctccctcctcaattgacacttgcctcttgtcagcaagatctgttttatttcctactagcgtgatgataacatcacttcctccttctgttctgacatcatcaatccactttgtagtttgctggaatgagttaacatttgtgatatcgtaaactactacagctgcagcagaatcacggatgtacctgggaatgaggctacggagacgttcctgacccgccgtatcccacagccgaagcccgattgttccatcctccaagtacatagtttttgataaaaagtcaatgccaattattgcctgataggtgttgtcaaaactgtcatacctgaatctggtgatcaaagatgtctttgcaacgctttgctcccccaggaacaccagcttgaatttcctcagcggattcccgaagtctccgcccgcggacatggtggaactagaggagctgtcgccgcctcagcccagagacctcccggaccgatgctgctccagccggctgacgaaaaaggcgagcggaagggcgggcgccgagctctctgcgcccctgcaagggccggtggaggagcccggctggagggcagcaggactctccacagactggcagccgccgccgcctcccggcagagtagccgagcaccgagcgaggcccgcggctgggaagggaaggagggcggtgtcggcaggagccaggggtgtgctttggcttcccaaggctagggccgttcccttcttcctcacccggctccaagacctgcgggagaaaggcggagggtggcggagccggaaccgcagacgtatctgggatctctcacgcgcggcgcttcggcttccccagccgccgccgccgcagcccaacctgctgagtgcgcgagcctct

SEQ ID NO: 19244 - RNA, 733 nt, Homo sapiens
  source 1..733: mol_type = other RNA
tgtgtccgggaagtggaggaggaataggcatcatgtaactgttaatgtttggaagttgatatgaattcattctctgtgaattgcctatggagttcctgaacttcatcactgccttcttgcccccaatgggaaacagagcttcattttccagcaatgaggtttttgatctggaccttgaagttacctttggaacagtttctactgcaggattactgggaagaggctgtaatcgaattggaggctgcatatttcctggagcagtatatggtcgaggggctgtcagtgctaacggactggaatgtccttcatcaaccagaacactatggccacgattactctttgggccaactggtgggtggggagacaggattggcatgttattttcaacagaccttcttgtgtgctctcccttaaacctctggattcgctccttcctagctaaggtctccaatttcttttttatttcaagctgatggtaacgctccatatcaagaactttatgaaaaattgcctgggctaagcattcccggatatatttttgatgatcccgcttcatcatatttagtttatattctttttcagaaagtattcttccacttcttgtgatcagtcctgatcttaagagatgacgccttatccttgtattgttaaaatacccagccaggtgtttatccataaggctattatatgcagcaagtaacattggaatccagtacatggaatgcagggctta

SEQ ID NO: 19245 - RNA, 943 nt, Homo sapiens
  source 1..943: mol_type = other RNA
tgtgtccgggaagtggaggaggaataggcatcatgtaactgttaatgtttggaagttgatatgaattcattctctgtgaattgcctatggagttcctgaacttcatcactgccttcttgcccccaatgggaaacagagcttcattttccagcaatgaggtttttgatctggaccttgaagttacctttggaacagtttctactgcaggattactgggaagaggctgtaatcgaattggaggctgcatatttcctggagcagtatatggtcgaggggctgtcagtgctaacggactggaatgtccttcatcaaccagaacactatggccacgattactctttgggccaactggtgggtggggagacaggattggcatgttattttcaacagaccttcttgtgtgctctcccttaaacctctggattcgctccttcctagctaaggtctccaatttcttttttatttcaagctgatggtaacgctccatatcaagaactttatgaaaaattgcctgggctaagcattcccggatatatttttgatgatcccgcttcatcatatttagtttatattctttttcagaaagtattcttccacttcttgtgatcagtcctgatcttaagagatgacgccttatccttgtattgttaaaatacccagccaggtgtttatccataaggctattatatgcagcaagtaacccagcggggtgagaatggctcatttttgcaggatcccttttggaccccgcggcaggtgcggagggtgggtgcgtggggccccgtgcgcgctggcgctgcgacagtcgcgctcgaggggtggctccgcaccgaggtcccctgtgcgcgggcacctgggctgggccgccgccgcccctgggcgcccgggctacccgcagcctcccgggctcccaccctccgttggtatccacagcttccctgtt

SEQ ID NO: 19246 - RNA, 997 nt, Homo sapiens
  source 1..997: mol_type = other RNA
tgtgtccgggaagtggaggaggaataggcatcatgtaactgttaatgtttggaagttgatatgaattcattctctgtgaattgcctatggagttcctgaacttcatcactgccttcttgcccccaatgggaaacagagcttcattttccagcaatgaggtttttgatctggaccttgaagttacctttggaacagtttctactgcaggattactgggaagaggctgtaatcgaattggaggctgcatatttcctggagcagtatatggtcgaggggctgtcagtgctaacggactggaatgtccttcatcaaccagaacactatggccacgattactctttgggccaactggtgggtggggagacaggattggcatgttattttcaacagaccttcttgtgtgctctcccttaaacctctggattcgctccttcctagctaaggtctccaatttcttttttatttcaagctgatggtaacgctccatatcaagaactttatgaaaaattgcctgggctaagcattcccggatatatttttgatgatcccgcttcatcatatttagtttatattctttttcagaaagtattcttccacttcttgtgatcagtcctgatcttaagagatgacgccttatccttgtattgttaaaatacccagccaggtgtttatccataaggctattatatgcagcaagtaacccagcggggtgagaatggctcatttttgcaggatcccttttggaccccgcggcaggtgcggagggtgggtgcgtggggccccgtgcgcgctggcgctgcgacagtcgcgctcgaggggtggctccgcaccgaggtcccctgtgcgcgggcacctgggctgggccgccgccgcccctgggcgcccgggctacccgcagcctcccgggctcccaccctccgttggtatccacagcttccctgttgctaagggaggagagaggcaagcgcccagggtctggagaagcggaggcgctact

SEQ ID NO: 19247 - RNA, 3242 nt, Homo sapiens
  source 1..3242: mol_type = other RNA
tgtgtccgggaagtggaggaggacacaggactagcccaccaccttctcctcccggtctcccaagatgactgcttatagagtggaggaggcaaacaggtcccctcaatgtaccagatggtcacctatagcaccagctccagatggccacgtggctgcagctggactcaatgaaactctgtgacaaccagaagatacctgctttgggatgagagggaggataaagccatgcagggaggatatttaccatccctaccctaagcacagtgcaagcagtgagcccccggctcccagtacctgaaaaaccaggtcctactgccttctggatgctctcttgggccaggaagggaaaagtgtgggaggaatgtcttccagctgctaacgagaagtctgcacccacttgaaagggttaggagaataaaaagcagcattctttaaagaactgcaagtggagcaccaccaggccccttccttggactttcccgtcctgggcagcctcagagcctgcacactgaagctgggttcaaatcctgggtccttcctgcctgacagactgacccctggaaacatgagtctctggtttttttcactgggctagcctcaagcaaatcttgggagctcttgagtatcttcggcatgtgccttttccagcacttgctactgattttgcagagctcccagaaccgtgctccccaactggctccagctctgccagcctggattctcttcactcccaaccagcaggggaccactcagtgacaacactggcctggtcattcagggactgcctgggctctgaagtttcgtcccaactgtctgcgcctatgctggggaaacaccttgcctggtagagctgccctgctcccttgactcctcctcctctgccaaggcaggaaaataatcctctggtcatggatggatggggtcactcacataagtgggaacaaacagtgccccttggtggcagctggatatatgcctccaggcatccctgaccactgtcctgtagacaactgaggccagaaatggagagccaggaacaaactgacctcttccattcaaataagctccaaacccaagcactgcacaatgggaggctgagcctttcaaaggcccaaccagaagagagctggcggctacacaaaaccagggtgtggttaagtgccaggcgaggtgagaaccgggagggctcacaacacagccccctcccagcaaagacacccagaagggaaagagagctggggtggggcattcagcacaactcaaggaaaagggaaaggtgaactctggagaacttcctctgggtggagacgacacgggactccaagccaagagcttagatagactcttcccagcggtgcagcctcatcctgcccttgccactagtgaggcctggagccactggggagaggacaagaggcctgagacctgctccccacccaggcacctccactgacaagacagaggagcggcacagctctcaggccgacctggctcccgtcaggacaccagggctctccatcccctccattgtttgaaaagcttaatacacacaaaggaaaggcagcccctcggcccctggaaaaagcagggtccttcagacagcccccacgctgcatcccatggggccacaagaaagccacccagagaattcagtgtaccatttccagataagaaatcagcttggggctgaggctcggggaggcacacactgaaaaacacaagcctaccttggcgatgagatgaagaaacatactacaggaaacgttaacgtagagagaagagcacagggcagaacacaacacagaaaggcgggtcccatccagtgaggaagctctttatccctggcaacccttcccacaatcaggggtctccagtccgatggcccattggtcataagctttgccttggggaaacagagccaccctcctctgcccccacttctggctgcctcactcccctgctcaaagcttgattttgaattctgtgggctgcgtggtcacagaggcccctgaggacttgaagagtgccttcaggatggtgtcagggtccacttcggcaggggggttggaggaggaggcagagttcaccctgcgaggcagctcgctctcctttttcattgatgggctgtcactcagccgcagcaggatgggctggtctgaggtgataacattcccattcatgtgaaggttgcacttcatcggctgcccgtccagacaccggttgttgtacttcttatatgcggtgatggcatcgtcctttttcacaaacaccacctccgctaccccaggatggaccagtcgagctcgcttgagggccccacacacacagaaaagctcaacaatgtcctcctcagtgactcgagggtgcagattattcacagtcatcttggtgccttccaatgggctcagcagctggcagctctttggggggttcttccttgttcaccagtgtccgggacatgttggtcaaggcttttgttcgaatagaggaagggagagcaggagctgtgtatgcatcattctgaaccactttggtgagagggagggccttggacatggaaagcttggaactgcttagcccagccatgtggtggagaaagccgcctgaggctgcaaacttcatctgtttagtaggaacggaagctataccatcatcatcttcatccaggtcatataaattctgtttggcctggtggttattgacaacattgattctcattccggcaggatggggatgaagtggtgccatggctttctgctgtggaacctggatggttttggtgagcttcagagcaggggtcactgtcccaatgggtgggtttatgaaggcagcaggggaactcctcttcaagctgatcttctcccgggcatcagcaacctggcggggcttctggggcaccgtggtctgctgcttgcgagagttcaacatctctctggcatcctgcactttccctttgattcgaaatcgggcatctttctgcaaaagcttctcccgggcatccttgactcccagtttgagccgggcatctgagaggccaatcttctgccgggcatcaaatctctgctggaaggtggctgtgcgtgttgactggctgagaaggccttgctggatcccaactcgagatcggacacctccaactcccggtctggcattaagccgtcctttcgccgccgccccgcgcttcctgatgagttcgtccagggagatgtccgccatcttgctccgccgagcaagccgaaagc

SEQ ID NO: 19248 - RNA, 3166 nt, Homo sapiens
  source 1..3166: mol_type = other RNA
tgtgtccgggaagtggaggaggacacaggactagcccaccaccttctcctcccggtctcccaagatgactgcttatagagtggaggaggcaaacaggtcccctcaatgtaccagatggtcacctatagcaccagctccagatggccacgtggctgcagctggactcaatgaaactctgtgacaaccagaagatacctgctttgggatgagagggaggataaagccatgcagggaggatatttaccatccctaccctaagcacagtgcaagcagtgagcccccggctcccagtacctgaaaaaccaggtcctactgccttctggatgctctcttgggccaggaagggaaaagtgtgggaggaatgtcttccagctgctaacgagaagtctgcacccacttgaaagggttaggagaataaaaagcagcattctttaaagaactgcaagtggagcaccaccaggccccttccttggactttcccgtcctgggcagcctcagagcctgcacactgaagctgggttcaaatcctgggtccttcctgcctgacagactgacccctggaaacatgagtctctggtttttttcactgggctagcctcaagcaaatcttgggagctcttgagtatcttcggcatgtgccttttccagcacttgctactgattttgcagagctcccagaaccgtgctccccaactggctccagctctgccagcctggattctcttcactcccaaccagcaggggaccactcagtgacaacactggcctggtcattcagggactgcctgggctctgaagtttcgtcccaactgtctgcgcctatgctggggaaacaccttgcctggtagagctgccctgctcccttgactcctcctcctctgccaaggcaggaaaataatcctctggtcatggatggatggggtcactcacataagtgggaacaaacagtgccccttggtggcagctggatatatgcctccaggcatccctgaccactgtcctgtagacaactgaggccagaaatggagagccaggaacaaactgacctcttccattcaaataagctccaaacccaagcactgcacaatgggaggctgagcctttcaaaggcccaaccagaagagagctggcggctacacaaaaccagggtgtggttaagtgccaggcgaggtgagaaccgggagggctcacaacacagccccctcccagcaaagacacccagaagggaaagagagctggggtggggcattcagcacaactcaaggaaaagggaaaggtgaactctggagaacttcctctgggtggagacgacacgggactccaagccaagagcttagatagactcttcccagcggtgcagcctcatcctgcccttgccactagtgaggcctggagccactggggagaggacaagaggcctgagacctgctccccacccaggcacctccactgacaagacagaggagcggcacagctctcaggccgacctggctcccgtcaggacaccagggctctccatcccctccattgtttgaaaagcttaatacacacaaaggaaaggcagcccctcggcccctggaaaaagcagggtccttcagacagcccccacgctgcatcccatggggccacaagaaagccacccagagaattcagtgtaccatttccagataagaaatcagcttggggctgaggctcggggaggcacacactgaaaaacacaagcctaccttggcgatgagatgaagaaacatactacaggaaacgttaacgtagagagaagagcacagggcagaacacaacacagaaaggcgggtcccatccagtgaggaagctctttatccctggcaacccttcccacaatcaggggtctccagtccgatggcccattggtcataagctttgccttggggaaacagagccaccctcctctgcccccacttctggctgcctcactcccctgctcaaagcttgattttgaattctgtgggctgcgtggtcacagaggcccctgaggacttgaagagtgccttcaggatggtgtcagggtccacttcggcaggggggttggaggaggaggcagagttcaccctgcgaggcagctcgctctcctttttcattgatgggctgtcactcagccgcagcaggatgggctggtctgaggtgataacattcccattcatgtgaaggttgcacttcatcggctgcccgtccagacaccggttgttgtacttcttatatgcggtgatggcatcgtcctttttcacaaacaccacctccgctaccccaggatggaccagtcgagctcgcttgagggccccacacacacagaaaagctcaacaatgtcctcctcagtgactcgagggtgcagattattcacagtcatcttggtgccttccaatgggctgagaacaggctcagcagctggcagctctttggggggttcttccttgttcaccagtgtccgggacatgttggtcaaggcttttgttcgaatagaggaagggagagcaggagctgtgtatgcatcattctgaaccactttggtgagagggagggccttggacatggaaagcttggaactgcttagcccagccatgtggtggagaaagccgcctgaggctgcaaacttcatctgtttagtaggaacggaagctataccatcatcatcttcatccaggtcatataaattctggatggttttggtgagcttcagagcaggggtcactgtcccaatgggtgggtttatgaaggcagcaggggaactcctcttcaagctgatcttctcccgggcatcagcaacctggcggggcttctggggcaccgtggtctgctgcttgcgagagttcaacatctctctggcatcctgcactttccctttgattcgaaatcgggcatctttctgcaaaagcttctcccgggcatccttgactcccagtttgagccgggcatctgagaggccaatcttctgccgggcatcaaatctctgctggaaggtggctgtgcgtgttgactggctgagaaggccttgctggatcccaactcgagatcggacacctccaactcccggtctggcattaagccgtcctttcgccgccgccccgcgcttcctgatgagttcgtccagggagatgtccgccatcttgctccgccgagcaagccgaaagc

SEQ ID NO: 19249 - RNA, 3304 nt, Homo sapiens
  source 1..3304: mol_type = other RNA
tgtgtccgggaagtggaggaggacacaggactagcccaccaccttctcctcccggtctcccaagatgactgcttatagagtggaggaggcaaacaggtcccctcaatgtaccagatggtcacctatagcaccagctccagatggccacgtggctgcagctggactcaatgaaactctgtgacaaccagaagatacctgctttgggatgagagggaggataaagccatgcagggaggatatttaccatccctaccctaagcacagtgcaagcagtgagcccccggctcccagtacctgaaaaaccaggtcctactgccttctggatgctctcttgggccaggaagggaaaagtgtgggaggaatgtcttccagctgctaacgagaagtctgcacccacttgaaagggttaggagaataaaaagcagcattctttaaagaactgcaagtggagcaccaccaggccccttccttggactttcccgtcctgggcagcctcagagcctgcacactgaagctgggttcaaatcctgggtccttcctgcctgacagactgacccctggaaacatgagtctctggtttttttcactgggctagcctcaagcaaatcttgggagctcttgagtatcttcggcatgtgccttttccagcacttgctactgattttgcagagctcccagaaccgtgctccccaactggctccagctctgccagcctggattctcttcactcccaaccagcaggggaccactcagtgacaacactggcctggtcattcagggactgcctgggctctgaagtttcgtcccaactgtctgcgcctatgctggggaaacaccttgcctggtagagctgccctgctcccttgactcctcctcctctgccaaggcaggaaaataatcctctggtcatggatggatggggtcactcacataagtgggaacaaacagtgccccttggtggcagctggatatatgcctccaggcatccctgaccactgtcctgtagacaactgaggccagaaatggagagccaggaacaaactgacctcttccattcaaataagctccaaacccaagcactgcacaatgggaggctgagcctttcaaaggcccaaccagaagagagctggcggctacacaaaaccagggtgtggttaagtgccaggcgaggtgagaaccgggagggctcacaacacagccccctcccagcaaagacacccagaagggaaagagagctggggtggggcattcagcacaactcaaggaaaagggaaaggtgaactctggagaacttcctctgggtggagacgacacgggactccaagccaagagcttagatagactcttcccagcggtgcagcctcatcctgcccttgccactagtgaggcctggagccactggggagaggacaagaggcctgagacctgctccccacccaggcacctccactgacaagacagaggagcggcacagctctcaggccgacctggctcccgtcaggacaccagggctctccatcccctccattgtttgaaaagcttaatacacacaaaggaaaggcagcccctcggcccctggaaaaagcagggtccttcagacagcccccacgctgcatcccatggggccacaagaaagccacccagagaattcagtgtaccatttccagataagaaatcagcttggggctgaggctcggggaggcacacactgaaaaacacaagcctaccttggcgatgagatgaagaaacatactacaggaaacgttaacgtagagagaagagcacagggcagaacacaacacagaaaggcgggtcccatccagtgaggaagctctttatccctggcaacccttcccacaatcaggggtctccagtccgatggcccattggtcataagctttgccttggggaaacagagccaccctcctctgcccccacttctggctgcctcactcccctgctcaaagcttgattttgaattctgtgggctgcgtggtcacagaggcccctgaggacttgaagagtgccttcaggatggtgtcagggtccacttcggcaggggggttggaggaggaggcagagttcaccctgcgaggcagctcgctctcctttttcattgatgggctgtcactcagccgcagcaggatgggctggtctgaggtgataacattcccattcatgtgaaggttgcacttcatcggctgcccgtccagacaccggttgttgtacttcttatatgcggtgatggcatcgtcctttttcacaaacaccacctccgctaccccaggatggaccagtcgagctcgcttgagggccccacacacacagaaaagctcaacaatgtcctcctcagtgactcgagggtgcagattattcacagtcatcttggtgccttccaatgggctgagaacaggctcagcagctggcagctctttggggggttcttccttgttcaccagtgtccgggacatgttggtcaaggcttttgttcgaatagaggaagggagagcaggagctgtgtatgcatcattctgaaccactttggtgagagggagggccttggacatggaaagcttggaactgcttagcccagccatgtggtggagaaagccgcctgaggctgcaaacttcatctgtttagtaggaacggaagctataccatcatcatcttcatccaggtcatataaattctgtttggcctggtggttattgacaacattgattctcattccggcaggatggggatgaagtggtgccatggctttctgctgtggaacctggaaacactcagtggtcagaatccaccccacagggtccacatgcattctctggatggttttggtgagcttcagagcaggggtcactgtcccaatgggtgggtttatgaaggcagcaggggaactcctcttcaagctgatcttctcccgggcatcagcaacctggcggggcttctggggcaccgtggtctgctgcttgcgagagttcaacatctctctggcatcctgcactttccctttgattcgaaatcgggcatctttctgcaaaagcttctcccgggcatccttgactcccagtttgagccgggcatctgagaggccaatcttctgccgggcatcaaatctctgctggaaggtggctgtgcgtgttgactggctgagaaggccttgctggatcccaactcgagatcggacacctccaactcccggtctggcattaagccgtcctttcgccgccgccccgcgcttcctgatgagttcgtccagggagatgtccgccatcttgctccgccgagcaagccgaaagc

SEQ ID NO: 19250 - RNA, 3253 nt, Homo sapiens
  source 1..3253: mol_type = other RNA
tgtgtccgggaagtggaggaggacacaggactagcccaccaccttctcctcccggtctcccaagatgactgcttatagagtggaggaggcaaacaggtcccctcaatgtaccagatggtcacctatagcaccagctccagatggccacgtggctgcagctggactcaatgaaactctgtgacaaccagaagatacctgctttgggatgagagggaggataaagccatgcagggaggatatttaccatccctaccctaagcacagtgcaagcagtgagcccccggctcccagtacctgaaaaaccaggtcctactgccttctggatgctctcttgggccaggaagggaaaagtgtgggaggaatgtcttccagctgctaacgagaagtctgcacccacttgaaagggttaggagaataaaaagcagcattctttaaagaactgcaagtggagcaccaccaggccccttccttggactttcccgtcctgggcagcctcagagcctgcacactgaagctgggttcaaatcctgggtccttcctgcctgacagactgacccctggaaacatgagtctctggtttttttcactgggctagcctcaagcaaatcttgggagctcttgagtatcttcggcatgtgccttttccagcacttgctactgattttgcagagctcccagaaccgtgctccccaactggctccagctctgccagcctggattctcttcactcccaaccagcaggggaccactcagtgacaacactggcctggtcattcagggactgcctgggctctgaagtttcgtcccaactgtctgcgcctatgctggggaaacaccttgcctggtagagctgccctgctcccttgactcctcctcctctgccaaggcaggaaaataatcctctggtcatggatggatggggtcactcacataagtgggaacaaacagtgccccttggtggcagctggatatatgcctccaggcatccctgaccactgtcctgtagacaactgaggccagaaatggagagccaggaacaaactgacctcttccattcaaataagctccaaacccaagcactgcacaatgggaggctgagcctttcaaaggcccaaccagaagagagctggcggctacacaaaaccagggtgtggttaagtgccaggcgaggtgagaaccgggagggctcacaacacagccccctcccagcaaagacacccagaagggaaagagagctggggtggggcattcagcacaactcaaggaaaagggaaaggtgaactctggagaacttcctctgggtggagacgacacgggactccaagccaagagcttagatagactcttcccagcggtgcagcctcatcctgcccttgccactagtgaggcctggagccactggggagaggacaagaggcctgagacctgctccccacccaggcacctccactgacaagacagaggagcggcacagctctcaggccgacctggctcccgtcaggacaccagggctctccatcccctccattgtttgaaaagcttaatacacacaaaggaaaggcagcccctcggcccctggaaaaagcagggtccttcagacagcccccacgctgcatcccatggggccacaagaaagccacccagagaattcagtgtaccatttccagataagaaatcagcttggggctgaggctcggggaggcacacactgaaaaacacaagcctaccttggcgatgagatgaagaaacatactacaggaaacgttaacgtagagagaagagcacagggcagaacacaacacagaaaggcgggtcccatccagtgaggaagctctttatccctggcaacccttcccacaatcaggggtctccagtccgatggcccattggtcataagctttgccttggggaaacagagccaccctcctctgcccccacttctggctgcctcactcccctgctcaaagcttgattttgaattctgtgggctgcgtggtcacagaggcccctgaggacttgaagagtgccttcaggatggtgtcagggtccacttcggcaggggggttggaggaggaggcagagttcaccctgcgaggcagctcgctctcctttttcattgatgggctgtcactcagccgcagcaggatgggctggtctgaggtgataacattcccattcatgtgaaggttgcacttcatcggctgcccgtccagacaccggttgttgtacttcttatatgcggtgatggcatcgtcctttttcacaaacaccacctccgctaccccaggatggaccagtcgagctcgcttgagggccccacacacacagaaaagctcaacaatgtcctcctcagtgactcgagggtgcagattattcacagtcatcttggtgccttccaatgggctgagaacaggctcagcagctggcagctctttggggggttcttccttgttcaccagtgtccgggacatgttggtcaaggcttttgttcgaatagaggaagggagagcaggagctgtgtatgcatcattctgaaccactttggtgagagggagggccttggacatggaaagcttggaactgcttagcccagccatgtggtggagaaagccgcctgaggctgcaaacttcatctgtttagtaggaacggaagctataccatcatcatcttcatccaggtcatataaattctgtttggcctggtggttattgacaacattgattctcattccggcaggatggggatgaagtggtgccatggctttctgctgtggaacctggatggttttggtgagcttcagagcaggggtcactgtcccaatgggtgggtttatgaaggcagcaggggaactcctcttcaagctgatcttctcccgggcatcagcaacctggcggggcttctggggcaccgtggtctgctgcttgcgagagttcaacatctctctggcatcctgcactttccctttgattcgaaatcgggcatctttctgcaaaagcttctcccgggcatccttgactcccagtttgagccgggcatctgagaggccaatcttctgccgggcatcaaatctctgctggaaggtggctgtgcgtgttgactggctgagaaggccttgctggatcccaactcgagatcggacacctccaactcccggtctggcattaagccgtcctttcgccgccgccccgcgcttcctgatgagttcgtccagggagatgtccgccatcttgctccgccgagcaagccgaaagc

SEQ ID NO: 19251 - RNA, 3108 nt, Homo sapiens
  source 1..3108: mol_type = other RNA
tgtgtccgggaagtggaggaggacacaggactagcccaccaccttctcctcccggtctcccaagatgactgcttatagagtggaggaggcaaacaggtcccctcaatgtaccagatggtcacctatagcaccagctccagatggccacgtggctgcagctggactcaatgaaactctgtgacaaccagaagatacctgctttgggatgagagggaggataaagccatgcagggaggatatttaccatccctaccctaagcacagtgcaagcagtgagcccccggctcccagtacctgaaaaaccaggtcctactgccttctggatgctctcttgggccaggaagggaaaagtgtgggaggaatgtcttccagctgctaacgagaagtctgcacccacttgaaagggttaggagaataaaaagcagcattctttaaagaactgcaagtggagcaccaccaggccccttccttggactttcccgtcctgggcagcctcagagcctgcacactgaagctgggttcaaatcctgggtccttcctgcctgacagactgacccctggaaacatgagtctctggtttttttcactgggctagcctcaagcaaatcttgggagctcttgagtatcttcggcatgtgccttttccagcacttgctactgattttgcagagctcccagaaccgtgctccccaactggctccagctctgccagcctggattctcttcactcccaaccagcaggggaccactcagtgacaacactggcctggtcattcagggactgcctgggctctgaagtttcgtcccaactgtctgcgcctatgctggggaaacaccttgcctggtagagctgccctgctcccttgactcctcctcctctgccaaggcaggaaaataatcctctggtcatggatggatggggtcactcacataagtgggaacaaacagtgccccttggtggcagctggatatatgcctccaggcatccctgaccactgtcctgtagacaactgaggccagaaatggagagccaggaacaaactgacctcttccattcaaataagctccaaacccaagcactgcacaatgggaggctgagcctttcaaaggcccaaccagaagagagctggcggctacacaaaaccagggtgtggttaagtgccaggcgaggtgagaaccgggagggctcacaacacagccccctcccagcaaagacacccagaagggaaagagagctggggtggggcattcagcacaactcaaggaaaagggaaaggtgaactctggagaacttcctctgggtggagacgacacgggactccaagccaagagcttagatagactcttcccagcggtgcagcctcatcctgcccttgccactagtgaggcctggagccactggggagaggacaagaggcctgagacctgctccccacccaggcacctccactgacaagacagaggagcggcacagctctcaggccgacctggctcccgtcaggacaccagggctctccatcccctccattgtttgaaaagcttaatacacacaaaggaaaggcagcccctcggcccctggaaaaagcagggtccttcagacagcccccacgctgcatcccatggggccacaagaaagccacccagagaattcagtgtaccatttccagataagaaatcagcttggggctgaggctcggggaggcacacactgaaaaacacaagcctaccttggcgatgagatgaagaaacatactacaggaaacgttaacgtagagagaagagcacagggcagaacacaacacagaaaggcgggtcccatccagtgaggaagctctttatccctggcaacccttcccacaatcaggggtctccagtccgatggcccattggtcataagctttgccttggggaaacagagccaccctcctctgcccccacttctggctgcctcactcccctgctcaaagcttgattttgaattctgtgggctgcgtggtcacagaggcccctgaggacttgaagagtgccttcaggatggtgtcagggtccacttcggcaggggggttggaggaggaggcagagttcaccctgcgaggcagctcgctctcctttttcattgatgggctgtcactcagccgccgtccagacaccggttgttgtacttcttatatgcggtgatggcatcgtcctttttcacaaacaccacctccgctaccccaggatggaccagtcgagctcgcttgagggccccacacacacagaaaagctcaacaatgtcctcctcagtgactcgagggtgcagattattcacagtcatcttggtgccttccaatgggctgagaacaggctcagcagctggcagctctttggggggttcttccttgttcaccagtgtccgggacatgttggtcaaggcttttgttcgaatagaggaagggagagcaggagctgtgtatgcatcattctgaaccactttggtgagagggagggccttggacatggaaagcttggaactgcttagcccagccatgtggtggagaaagccgcctgaggctgcaaacttcatctgtttagtaggaacggaagctataccatcatcatcttcatccaggtcatataaattctggatggttttggtgagcttcagagcaggggtcactgtcccaatgggtgggtttatgaaggcagcaggggaactcctcttcaagctgatcttctcccgggcatcagcaacctggcggggcttctggggcaccgtggtctgctgcttgcgagagttcaacatctctctggcatcctgcactttccctttgattcgaaatcgggcatctttctgcaaaagcttctcccgggcatccttgactcccagtttgagccgggcatctgagaggccaatcttctgccgggcatcaaatctctgctggaaggtggctgtgcgtgttgactggctgagaaggccttgctggatcccaactcgagatcggacacctccaactcccggtctggcattaagccgtcctttcgccgccgccccgcgcttcctgatgagttcgtccagggagatgtccgccatcttgctccgccgagcaagccgaaagcagtcgagac

SEQ ID NO: 19252 - RNA, 3186 nt, Homo sapiens
  source 1..3186: mol_type = other RNA
tgtgtccgggaagtggaggaggacacaggactagcccaccaccttctcctcccggtctcccaagatgactgcttatagagtggaggaggcaaacaggtcccctcaatgtaccagatggtcacctatagcaccagctccagatggccacgtggctgcagctggactcaatgaaactctgtgacaaccagaagatacctgctttgggatgagagggaggataaagccatgcagggaggatatttaccatccctaccctaagcacagtgcaagcagtgagcccccggctcccagtacctgaaaaaccaggtcctactgccttctggatgctctcttgggccaggaagggaaaagtgtgggaggaatgtcttccagctgctaacgagaagtctgcacccacttgaaagggttaggagaataaaaagcagcattctttaaagaactgcaagtggagcaccaccaggccccttccttggactttcccgtcctgggcagcctcagagcctgcacactgaagctgggttcaaatcctgggtccttcctgcctgacagactgacccctggaaacatgagtctctggtttttttcactgggctagcctcaagcaaatcttgggagctcttgagtatcttcggcatgtgccttttccagcacttgctactgattttgcagagctcccagaaccgtgctccccaactggctccagctctgccagcctggattctcttcactcccaaccagcaggggaccactcagtgacaacactggcctggtcattcagggactgcctgggctctgaagtttcgtcccaactgtctgcgcctatgctggggaaacaccttgcctggtagagctgccctgctcccttgactcctcctcctctgccaaggcaggaaaataatcctctggtcatggatggatggggtcactcacataagtgggaacaaacagtgccccttggtggcagctggatatatgcctccaggcatccctgaccactgtcctgtagacaactgaggccagaaatggagagccaggaacaaactgacctcttccattcaaataagctccaaacccaagcactgcacaatgggaggctgagcctttcaaaggcccaaccagaagagagctggcggctacacaaaaccagggtgtggttaagtgccaggcgaggtgagaaccgggagggctcacaacacagccccctcccagcaaagacacccagaagggaaagagagctggggtggggcattcagcacaactcaaggaaaagggaaaggtgaactctggagaacttcctctgggtggagacgacacgggactccaagccaagagcttagatagactcttcccagcggtgcagcctcatcctgcccttgccactagtgaggcctggagccactggggagaggacaagaggcctgagacctgctccccacccaggcacctccactgacaagacagaggagcggcacagctctcaggccgacctggctcccgtcaggacaccagggctctccatcccctccattgtttgaaaagcttaatacacacaaaggaaaggcagcccctcggcccctggaaaaagcagggtccttcagacagcccccacgctgcatcccatggggccacaagaaagccacccagagaattcagtgtaccatttccagataagaaatcagcttggggctgaggctcggggaggcacacactgaaaaacacaagcctaccttggcgatgagatgaagaaacatactacaggaaacgttaacgtagagagaagagcacagggcagaacacaacacagaaaggcgggtcccatccagtgaggaagctctttatccctggcaacccttcccacaatcaggggtctccagtccgatggcccattggtcataagctttgccttggggaaacagagccaccctcctctgcccccacttctggctgcctcactcccctgctcaaagcttgattttgaattctgtgggctgcgtggtcacagaggcccctgaggacttgaagagtgccttcaggatggtgtcagggtccacttcggcaggggggttggaggaggaggcagagttcaccctgcgaggcagctcgctctcctttttcattgatgggctgtcactcagccgccgtccagacaccggttgttgtacttcttatatgcggtgatggcatcgtcctttttcacaaacaccacctccgctaccccaggatggaccagtcgagctcgcttgagggccccacacacacagaaaagctcaacaatgtcctcctcagtgactcgagggtgcagattattcacagtcatcttggtgccttccaatgggctgagaacaggctcagcagctggcagctctttggggggttcttccttgttcaccagtgtccgggacatgttggtcaaggcttttgttcgaatagaggaagggagagcaggagctgtgtatgcatcattctgaaccactttggtgagagggagggccttggacatggaaagcttggaactgcttagcccagccatgtggtggagaaagccgcctgaggctgcaaacttcatctgtttagtaggaacggaagctataccatcatcatcttcatccaggtcatataaattctgtttggcctggtggttattgacaacattgattctcattccggcaggatggggatgaagtggtgccatggctttctgctgtggaacctggatggttttggtgagcttcagagcaggggtcactgtcccaatgggtgggtttatgaaggcagcaggggaactcctcttcaagctgatcttctcccgggcatcagcaacctggcggggcttctggggcaccgtggtctgctgcttgcgagagttcaacatctctctggcatcctgcactttccctttgattcgaaatcgggcatctttctgcaaaagcttctcccgggcatccttgactcccagtttgagccgggcatctgagaggccaatcttctgccgggcatcaaatctctgctggaaggtggctgtgcgtgttgactggctgagaaggccttgctggatcccaactcgagatcggacacctccaactcccggtctggcattaagccgtcctttcgccgccgccccgcgcttcctgatgagttcgtccagggagatgtccgccatcttgctccgccgagcaagccgaaagc

SEQ ID NO: 19253 - RNA, 571 nt, Homo sapiens
  source 1..571: mol_type = other RNA
tgtgtccgggaagtggaggaggctgctccgagctagcctgagccctgcttgggagggcctgagacaactcctccagggaaccatgaaacaacttcggcccaggagtccagagcaattggccggggatgacggtagttggactctgggaagggatggattcctctatcatataggctgctgggacgaagatgggtcgagaggtggagggagcttctaggcgtcttgccaaccaccagtcggagttggtctttcgaagcagtaggaacctatccccttcagccagagacacctgctggccatctgccccagtataagtaaaggcatagagggcacagagctgggatccccgaggagggcttcgggggcccagccctaggatcccccaggaacttggccaccaccggctggatagcattgtagccagcactgtcacctgtgagaaaaagggacactggagacccagaagggaataggcctggctgtctccaggtagacagacatggttctaggagcagtgttgcagggaggtgaggacgggagcccttgagttgggggagagggtagagcaaac

SEQ ID NO: 19254 - RNA, 616 nt, Homo sapiens
  source 1..616: mol_type = other RNA
tgtgtccgggaagtggaggaggctgctccgagctagcctgagccctgcttgggagggcctgagacaactcctccagggaaccatgaaacaacttcggcccaggagtccagagcaattggccggggatgacggtagttggactctgggaagggatggattcctctatcatataggctgctgggacgaagatgggtcgagaggtggagggagcttctaggcgtcttgccaaccaccagtcggagttggtctttcgaagcagtaggaacctatccccttcagccagagacacctgctggccatctgccccagtataagtaaaggcatagagggcacagagctgggatccccgaggagggcttcgggggcccagccctaggatcccccaggaacttggccaccaccggctggatagcattgtagccagcactgtcacctgtgagaaaaagggacactggagacccagaagggaataggcctggctgtctccaggtagacagacatggttctaggagcagtgttgcagggaggtgaggacgggagcccttgagttgggggagagggtagagcaaacagcctggtgaggatcggtgacaggttttgggggctgagaactcct

SEQ ID NO: 19255 - RNA, 489 nt, Homo sapiens
  source 1..489: mol_type = other RNA
tgtgtccgggaagtggaggaggctgctccgagctagcctgagccctgcttgggagggcctgagacaactcctccagggaaccatgaaacaacttcggcccaggagtccagagcaattggccggggatgacggtagttggactctgggaagggatggattcctctatcatataggctgctgggacgaagatgggtcgagaggtggagggagcttctaggcgtcttgccaaccaccagtcggagttggtctttcgaagcagtaggaacctatccccttcagccagagacacctgctggccatctgccccagtataagtaaaggcatagagggcacagagctgggatccccgaggagggcttcgggggcccagccctaggatcccccaggaacttggccaccaccggctggatagcattgtagccagcactgtcaccttgtggggcccatcagaagattcaggagcaggagttggtcctgggtagtggtggg

SEQ ID NO: 19256 - RNA, 490 nt, Homo sapiens
  source 1..490: mol_type = other RNA
tgtgtccgggaagtggaggaggctgctccgagctagcctgagccctgcttgggagggcctgagacaactcctccagggaaccatgaaacaacttcggcccaggagtccagagcaattggccggggatgacggtagttggactctgggaagggatggattcctctatcatataggctgctgggacgaagatgggtcgagaggtggagggagcttctaggcgtcttgccaaccaccagtcggagttggtctttcgaagcagtaggaacctatccccttcagccagagacacctgctggccatctgccccagtataagtaaaggcatagagggcacagagctgggatccccgaggagggcttcgggggcccagccctaggatcccccaggaacttggccaccaccggctggatagcattgtagccagcactgtcaccttgtggggcccatcagaagattcaggagcaggagttggtcctgggtagtggtggga

SEQ ID NO: 19257 - RNA, 492 nt, Homo sapiens
  source 1..492: mol_type = other RNA
tgtgtccgggaagtggaggaggctgctccgagctagcctgagccctgcttgggagggcctgagacaactcctccagggaaccatgaaacaacttcggcccaggagtccagagcaattggccggggatgacggtagttggactctgggaagggatggattcctctatcatataggctgctgggacgaagatgggtcgagaggtggagggagcttctaggcgtcttgccaaccaccagtcggagttggtctttcgaagcagtaggaacctatccccttcagccagagacacctgctggccatctgccccagtataagtaaaggcatagagggcacagagctgggatccccgaggagggcttcgggggcccagccctaggatcccccaggaacttggccaccaccggctggatagcattgtagccagcactgtcaccttgtggggcccatcagaagattcaggagcaggagttggtcctgggtagtggtgggagt

SEQ ID NO: 19258 - RNA, 613 nt, Homo sapiens
  source 1..613: mol_type = other RNA
tgtgtccgggaagtggaggaggctgctccgagctagcctgagccctgcttgggagggcctgagacaactcctccagggaaccatgaaacaacttcggcccaggagtccagagcaattggccggggatgacggtagttggactctgggaagggatggattcctctatcatataggctgctgggacgaagatgggtcgagaggtggagggagcttctaggcgtcttgccaaccaccagtcggagttggtctttcgaagcagtaggaacctatccccttcagccagagacacctgctggccatctgccccagtataagtaaaggcatagagggcacagagctgggatccccgaggagggcttcgggggcccagccctaggatcccccaggaacttggccaccaccggctggatagcattgtagccagcactgtcaccttgtggggcccatcagaagattcaggagcaggagttggtcctgggtagtggtgggagtctggccactcctcttttcctcttctctcagcttctccactgcacaatgtgaggctttctgggtgtgctggcccagctactgtagtcccagctacttgggagcctgaggcacaagaatcact

SEQ ID NO: 19259 - RNA, 831 nt, Homo sapiens
  source 1..831: mol_type = other RNA
tgtgtccgggaagtggaggaggctgctccgagctagcctgagccctgcttgggagggcctgagacaactcctccagggaaccatgaaacaacttcggcccaggagtccagagcaattggccggggatgacggtagttggactctgggaagggatggattcctctatcatataggctgctgggacgaagatgggtcgagaggtggagggagcttctaggcgtcttgccaaccaccagtcggagttggtctttcgaagcagtaggaacctatccccttcagccagagacacctgctggccatctgccccagtataagtaaaggcatagagggcacagagctgggatccccgaggagggcttcgggggcccagccctaggatcccccaggaacttggccaccaccggctggatagcattgtagccagcactgtcaccttgtggggcccatcagaagattcaggagcaggagttggtcctgggtagtggtgggagtctggccactcctcttttcctcttctctcagcttctccactgcacaatgtgaggctttctgggtgtgctggcccagctactgtagtcccagctacttgggagcctgaggcacaagaatcacttgaacctcttctcattctcagccgattgtttgggtgactcttaggaggttctcttgtaagtcttctcagttcttttaattttgttctcccactgtgaccttcagataattatgaagatatcccagttactttcagtcgttaagttcttggctgcagcactatcccaataccaccacctcctctgcagtccccatctgttgcttccagctggcagtttc

SEQ ID NO: 19260 - RNA, 570 nt, Homo sapiens
  source 1..570: mol_type = other RNA
tgtgtccgggaagtggaggaggctgctccgagctagcctgagccctgcttgggagggcctgagacaactcctccagggaaccatgaaacaacttcggcccaggagtccagagcaattggccggggatgacggtagttggactctgggaagggatggattcctctatcatataggctgctgggacgaagatgggtcgagaggtggagggagcttctaggcgtcttgccaaccaccagtcggagttggtctttcgaagcagtaggaacctatccccttcagccagagacacctgctggccatctgccccagtataagtaaaggcatagagggcacagagctgggatccccgaggagggcttcgggggcccagccctaggatcccccaggaacttggccaccaccggctggatagcattgtagccagcactgtcaccttgtggggcccatcagaagattcaggagcaggagttggtcctgggtagtggtgggagtcttgaggtggacacaggaaggagataagaagaaagaatcaggttcaagacagaaacagggagacacaaggttaatgac

SEQ ID NO: 19261 - RNA, 435 nt, Homo sapiens
  source 1..435: mol_type = other RNA
tgtgtccgggaagtggaggagggtatacagcgtccgcagacctgaaatcaaatgagaaagtgtgagcaccccgatggaggagccagctggatctcggttgtccttctccgagattcccggtgtcccggcgtttgaggatagaaccagcggatgggaagccgccagcaccgaagacatgacgccgagggggccagagccctttccctcttcctccgtacattacggggagcggcaccacaagcccgatccccgccaagaaaaggagggtcctgagaccccgcccagagccttccacccggcacccccaccactcccggccgcccaatctggctactacagctaaaaccacacttactagctcaccaccctccgaaaggcctcccgcaccgcggagctcctttatatagcccgaggacccgcccccgagttgcgatt

SEQ ID NO: 19262 - RNA, 62 nt, Homo sapiens
  source 1..62: mol_type = other RNA
tgtgtccgggaagtggaggagggtatacagcgtccgcagactagctcaccaccctccgaaag

SEQ ID NO: 19263 - RNA, 502 nt, Homo sapiens
  source 1..502: mol_type = other RNA
tgtgtccgggaagtggaggagggtcctctgcaagccagtcgccacggcagcgctaccataacgcaaagagaggcggcaggccgggggatccggtaccccaaaggcacacctctcagatcgctagagaaggctttctcaccgagggtgggtcacactccccacacgccagtcgcccctcgtcgggcccgcagaggcgctcagggacgcctggggaagggagggggcctgcggtaccaggaaaaatctgcgtgcggcaaccttgagccttcgcggtctgggcagggggcctggccgctgcgcgtgcgcgcaatccccgaagggccccctagtccaccagcctcctttctcccaggcaaagcacctccaagtaaacccacacacaacctgtcggaggcagaacggtagcccctcggcggccggccggcgcacgcgtcatctgccccagcccaccgcaatagctcacacggcccgtgcgcagccgccagaggggagcacgggacct

SEQ ID NO: 19264 - RNA, 1259 nt, Homo sapiens
  source 1..1259: mol_type = other RNA
tgtgtccgggaagtggaggaggtgtgtcctctgcaggggtggggatgtccacgtcgtcatagtcatcgtcagacgactctgacagttgcttcctggggctgctgctcctgaggtctcgaggaggctgtaggcgagcggtgttggctgggggtctggtctccattcctcggagcttcctgaactccatgtgccgccgacagcagtctgcatctgggatccccagagagctggagcggtgggtggatctgatccgccgagggatagcagggggtagctcgggctcctcatcctcaatgtccccaatggagggtcctttcccgggattcttcagtttgtcaagaagatccaggatcaggcctcgattcagcccaggctgggataccagttgatgactgagcatcttggtggcgctgggtcgtttcttgggactcttagtcagagtgactttgatgaagttgtggaaggcagccgaccatttgcctttttccttcagtcggggaggctggtagccactcttggtcatgaggaagagaactctgagagggtgcacatcaaagagcggtggctgtagctcggccagttcgatggccgtgatgcccagggaccagatgtcacacagctcattgtatcctcccttcagggccacagctgccacttccggagccatccagtagggtgtcccaatgaaagagaggcgtctggccagtgtagccccaatctgggccgagatgccaaagtcagccaatctgacctccccagcatcattgatgaggatgttagctcccttgatgtccctgtgtatcttcttctgtgagtgcaaataggccagtccctggagcacttcccggcagacatagctaatctggagctctgacagggagcctgtcacttggtagatgtcctggagagaaccagccccacagaattccatgcagatccagagtttctgcaaccagagataactcccatggtaggccacgatgttggcgtgccggcaagttttcaatatgaggatttccttctgaagggtggagacatcatcatcaggctccatcttcaccatcttcagtgccaccaggtcccctgacaccttgtctcgagccttaaagacttccccatacgtgccgccacccagccgctgtagcaggtcatagtggtcccgggggtctctattgaaaatgtcagggtccacgacgtccatccctgggggcctgagctgggcctgcgcccaggggccagcagggcctcagggctcaact

SEQ ID NO: 19265 - RNA, 1359 nt, Homo sapiens
  source 1..1359: mol_type = other RNA
tgtgtccgggaagtggaggaggtgtgtcctctgcaggggtggggctggatggagcctgactcggcctgtgggctggggagtatgggggcctgggctgactgttgggtctggatctggggctcagtatctggtctttgggagatttccaggtgccaaggttcagcatgtccacgtcgtcatagtcatcgtcagacgactctgacagttgcttcctggggctgctgctcctgaggtctcgaggaggctgtaggcgagcggtgttggctgggggtctggtctccattcctcggagcttcctgaactccatgtgccgccgacagcagtctgcatctgggatccccagagagctggagcggtgggtggatctgatccgccgagggatagcagggggtagctcgggctcctcatcctcaatgtccccaatggagggtcctttcccgggattcttcagtttgtcaagaagatccaggatcaggcctcgattcagcccaggctgggataccagttgatgactgagcatcttggtggcgctgggtcgtttcttgggactcttagtcagagtgactttgatgaagttgtggaaggcagccgaccatttgcctttttccttcagtcggggaggctggtagccactcttggtcatgaggaagagaactctgagagggtgcacatcaaagagcggtggctgtagctcggccagttcgatggccgtgatgcccagggaccagatgtcacacagctcattgtatcctcccttcagggccacagctgccacttccggagccatccagtagggtgtcccaatgaaagagaggcgtctggccagtgtagccccaatctgggccgagatgccaaagtcagccaatctgacctccccagcatcattgatgaggatgttagctcccttgatgtccctgtgtatcttcttctgtgagtgcaaataggccagtccctggagcacttcccggcagacatagctaatctggagctctgacagggagcctgtcacttggtagatgtcctggagagaaccagccccacagaattccatgcagatccagagtttctgcaaccagagataactcccatggtaggccacgatgttggcgtgccggcaagttttcaatatgaggatttccttctgaagggtggagacatcatcatcaggctccatcttcaccatcttcagtgccaccaggtcccctgacaccttgtctcgagccttaaagacttccccatacgtgccgccacccagccgctgtagcaggtcatagtggtcccgggggtctctattgaaaatgtcagggtccacgacgtccatccctgggggcctgagctgggcctgcgcccaggggccag

SEQ ID NO: 19266 - RNA, 1367 nt, Homo sapiens
  source 1..1367: mol_type = other RNA
tgtgtccgggaagtggaggaggtgtgtcctctgcaggggtggggctggatggagcctgactcggcctgtgggctggggagtatgggggcctgggctgactgttgggtctggatctggggctcagtatctggtctttgggagatttccaggtgccaaggttcagcatgtccacgtcgtcatagtcatcgtcagacgactctgacagttgcttcctggggctgctgctcctgaggtctcgaggaggctgtaggcgagcggtgttggctgggggtctggtctccattcctcggagcttcctgaactccatgtgccgccgacagcagtctgcatctgggatccccagagagctggagcggtgggtggatctgatccgccgagggatagcagggggtagctcgggctcctcatcctcaatgtccccaatggagggtcctttcccgggattcttcagtttgtcaagaagatccaggatcaggcctcgattcagcccaggctgggataccagttgatgactgagcatcttggtggcgctgggtcgtttcttgggactcttagtcagagtgactttgatgaagttgtggaaggcagccgaccatttgcctttttccttcagtcggggaggctggtagccactcttggtcatgaggaagagaactctgagagggtgcacatcaaagagcggtggctgtagctcggccagttcgatggccgtgatgcccagggaccagatgtcacacagctcattgtatcctcccttcagggccacagctgccacttccggagccatccagtagggtgtcccaatgaaagagaggcgtctggccagtgtagccccaatctgggccgagatgccaaagtcagccaatctgacctccccagcatcattgatgaggatgttagctcccttgatgtccctgtgtatcttcttctgtgagtgcaaataggccagtccctggagcacttcccggcagacatagctaatctggagctctgacagggagcctgtcacttggtagatgtcctggagagaaccagccccacagaattccatgcagatccagagtttctgcaaccagagataactcccatggtaggccacgatgttggcgtgccggcaagttttcaatatgaggatttccttctgaagggtggagacatcatcatcaggctccatcttcaccatcttcagtgccaccaggtcccctgacaccttgtctcgagccttgcaaaggggaagttggcagtcaggcaggctccatttgccagagtccctccacagcatcccttaaagacttccccatacgtgccgccacccagccgctgtagcaggtcatagtggtcccgggggtctctattgaaaatgtcag

SEQ ID NO: 19267 - RNA, 1191 nt, Homo sapiens
  source 1..1191: mol_type = other RNA
tgttcctctgtctcccagacggtatccattgaggctagctatcgccatggcagcctcatcatagtttgtcatagtcacaaatccaaaacctttgcatttattggtgttaaagtcacggatgaccttcacattggtgacagctccaaaaggcccaaacatttgccacaggatactctcatctgcgtcaggagccaggttgtacacaaatatacaccaccctgttccagggtgcccagggatattaattccagccaaactggtcattccgtcaatggtcattggagaaaacctaaaacgctgtgcctgctgagctagcggtcctggataccttctgtttggagactggtacagctgggaaaggatggcctgattggttttttggcttgggttattagcaaactttacagtgattggctccgtggcaccgggaggtttctggccatttaggcctttgatagcttcttctgcctcaattcgcttgtcaaatcgaataaaccctacaccccttgatatgccagtgacctggtcgacaagaatacgagaagtaataatgcgtccatattgtgaaaaaagctgttccaactccttctgggtcattgtttttggaagtccgctgacatataaatttgcatctctgatagaagctgaacttgggcgagcataggaaacttttattgttttggtttgaagtctcaatccattcagggtgttgatagctttctctgcatccttggggtcaatgtagttcacaaagccatatcccaagctctgccctgttattttgtctcttacaagcttacaggactctatttcaccaatgctcccaaagagactctttagttcctcctgtgtcatgttctgaggaaggtagttgactattaagttggtcttgctgtcttctgtgttcccagagtcaactggtgacgaacagttgttgtttatggtggttggaccattggctgtgttattgcaagttggcccattagacagttgtgtttccatggcagcaattacctgcccggtccaaggctctgctgcccacgaaccacttctaagcagagaagccacatcacacagtctgactgccatgttagtttggagttgccgtctgcgtctcaacagtttccttcttgcgctacacgcggccgcacccgggcacgtccacgcccgtgcacgctgccaggcgcgact

SEQ ID NO: 19268 - RNA, 1324 nt, Homo sapiens
  source 1..1324: mol_type = other RNA
tgttcctctgtctcccagacggtatccattgaggctagctatcgccatggcagcctcatcatagtttgtcatagtcacaaatccaaaacctttgcatttattggtgttaaagtcacggatgaccttcacattggtgacagctccaaaaggcccaaacatttgccacaggatactctcatctgcgtcaggagccaggttgtacacaaatatacaccaccctgttccagggtgcccagggatattaattccagccaaactggtcattccgtcaatggtcattggagaaaacctaaaacgctgtgcctgctgagctagcggtcctggataccttctgtttggagactggtacagctgggaaaggatggcctgattggttttttggcttgggttattagcaaactttacagtgattggctccgtggcaccgggaggtttctggccatttaggcctttgatagcttcttctgcctcaattcgcttgtcaaatcgaataaaccctacaccccttgatatgccagtgacctggtcgacaagaatacgagaagtaataatgcgtccatattgtgaaaaaagctgttccaactccttctgggtcattgtttttggaagtccgctgacatataaatttgcatctctgatagaagctgaacttgggcgagcataggaaacttttattgttttggtttgaagtctcaatccattcagggtgttgatagctttctctgcatccttggggtcaatgtagttcacaaagccatatcccaagctctgccctgttattttgtctcttacaagcttacaggactctatttcaccaatgctcccaaagagactctttagttcctcctgtgtcatgttctgaggaaggtagttgactattaagttggtcttgctgtcttctgtgttcccagagtcaactggtgacgaacagttgttgtttatggtggttggaccattggctgtgttattgcaagttggcccattagacagttgtgtttccatggcagcaattacctgcccggtccaaggctctgctgcccacgaaccacttctaagcagagaagccacatcacacagtctgactgccatgttagtttggagttgccgtctgctgtgactcgaagctgcagctactacggctcgtgccgctggccgtcagcactgccgcggaggagtcgctcggggcgagctccgcggagaggcggtggcggcggcggcggcgggaaaggggactggaagccggcggaacccccgccccacccgcgccgcgccgcgccgcgccggcaaccgccctcctcacccggccggctactgcctcagtgac

SEQ ID NO: 19269 - RNA, 1543 nt, Homo sapiens
  source 1..1543: mol_type = other RNA
tgttcctctgtctcccagacggtatccattgaggctagctatcgccatggcagcctcatcatagtttgtcatagtcacaaatccaaaacctttgcatttattggtgttaaagtcacggatgaccttcacattggtgacagctccaaaaggcccaaacatttgccacaggatactctcatctgcgtcaggagccaggttgtacacaaatatacaccaccctgttccagggtgcccagggatattaattccagccaaactggtcattccgtcaatggtcattggagaaaacctaaaacgctgtgcctgctgagctagcggtcctggataccttctgtttggagactggtacagctgggaaaggatggcctgattggttttttggcttgggttattagcaaactttacagtgattggctccgtggcaccgggaggtttctggccatttaggcctttgatagcttcttctgcctcaattcgcttgtcaaatcgaataaaccctacaccccttgatatgccagtgacctggtcgacaagaatacgagaagtaataatgcgtccatattgtgaaaaaagctgttccaactccttctgggtcattgtttttggaagtccgctgacatataaatttgcatctctgatagaagctgaacttgggcgagcataggaaacttttattgttttggtttgaagtctcaatccattcagggtgttgatagctttctctgcatccttggggtcaatgtagttcacaaagccatatcccaagctctgccctgttattttgtctcttacaagcttacaggactctatttcaccaatgctcccaaagagactctttagttcctcctgtgtcatgttctgaggaaggtagttgactattaagttggtcttgctgtcttctgtgttcccagagtcaactggtgacgaacagttgttgtttatggtggttggaccattggctgtgttattgcaagttggcccattagacagttgtgtttccatggcagcaattacctgcccggtccaaggctctgctgcccacgaaccacttctaagcagagaagccacatcacacagtctgactgccatgttagtttggagttgccgtctttctcccttaaggtttttgtgtatgtgtgtttttaaagtaacggtgcagttctcccaataaggatgagcaagaagctgctggatagttctcttaagacagcacgaaacctaaactgtgctcggcttaaaagaagcaaataaaaagaaacgctttcgaccccaaagtccaatgctaaaagaaatggcgaaaaaaaatatgaaaggggaggggaaacttaaaaaagagtttaaaaagacggagagactaccctcctattgccgttcaactaaacaaaaaggggcaagaaaaacaaaccaaggaacaaagaaaagagacgaaagaacgttttttcaaaaagacgatgtctttctccttgttgctttttagtaggtcgctacaggagtaagctgctgcatctctaactaagaacagaaataggggggaggacgtctt

SEQ ID NO: 19270 - RNA, 1384 nt, Homo sapiens
  source 1..1384: mol_type = other RNA
tgttcctctgtctcccagacggtatccattgaggctagctatcgccatggcagcctcatcatagtttgtcatagtcacaaatccaaaacctttgcatttattggtgttaaagtcacggatgaccttcacattggtgacagctccaaaaggcccaaacatttgccacaggatactctcatctgcgtcaggagccaggttgtacacaaatatacaccaccctgttccagggtgcccagggatattaattccagccaaactggtcattccgtcaatggtcattggagaaaacctaaaacgctgtgcctgctgagctagcggtcctggataccttctgtttggagactggtacagctgggaaaggatggcctgattggttttttggcttgggttattagcaaactttacagtgattggctccgtggcaccgggaggtttctggccatttaggcctttgatagcttcttctgcctcaattcgcttgtcaaatcgaataaaccctacaccccttgatatgccagtgacctggtcgacaagaatacgagaagtaataatgcgtccatattgtgaaaaaagctgttccaactccttctgggtcattgtttttggaagtccgctgacatataaatttgcatctctgatagaagctgaacttgggcgagcataggaaacttttattgttttggtttgaagtctcaatccattcagggtgttgatagctttctctgcatccttggggtcaatgtagttcacaaagccatatcccaagctctgccctgttattttgtctcttacaagcttacaggactctatttcaccaatgctcccaaagagactctttagttcctcctgtgtcatgttctgaggaaggtagttgactattaagttggtcttgctgtcttctgtgttcccagagtcaactggtgacgaacagttgttgtttatggtggttggaccattggctgtgttattgcaagttggcccattagacagttgtgtttccatggcagcaattacctgctgaaattgtaggaggtaagagaaaggaaccgagcagtgggcgacccagtcgccgcaagaacgtgaccgaggttacagcttcaagggcatgatgcaggtttgatgcagcaaggtccgctaagggcgtccagcgctccccgcccccatgcgacgggcggagcggggttggggggaagggaggggactcgtctaacccagggcgggtgtgggagaggcaaatttgccctcttgggcgaagtctaatcagcatagtgaagtagggggctcaaccaaggtcaaaagcgagataggccatcccttaatttgtgcgacccagtctggggacaccggatacagctaactgattctatatcagcatttccgtgtc

SEQ ID NO: 19271 - RNA, 1100 nt, Homo sapiens
  source 1..1100: mol_type = other RNA
tgttcctctgtctcccagacggtatccattgaggctagctatcgccatggcagcctcatcatagtttgtcatagtcacaaatccaaaacctttgcatttattggtgttaaagtcacggatgaccttcacattggtgacagctccaaaaggcccaaacatttgccacaggatactctcatctgcgtcaggagccaggttgtacacaaatatacaccaccctgttccagggtgcccagggatattaattccagccaaactggtcattccgtcaatggtcattggagaaaacctaaaacgctgtgcctgctgagctagcggtcctggataccttctgtttggagactggtacagctgggaaaggatggcctgattggttttttggcttgggttattagcaaactttacagtgattggctccgtggcaccgggaggtttctggccatttaggcctttgatagcttcttctgcctcaattcgcttgtcaaatcgaataaaccctacaccccttgatatgccagtgacctggtcgacaagaatacgagaagtaataatgcgtccatattgtgaaaaaagctgttccaactccttctgggtcattgtttttggaagtccgctgacatataaatttgcatctctgatagaagctgaacttgggcgagcataggaaacttttattgttttggtttgaagtctcaatccattcagggtgttgatagctttctctgcatccttggggtcaatgtagttcacaaagccatatcccaagctctgccctgttattttgtctcttacaagcttacaggactctatttcaccaatgctcccaaagagactctttagttcctcctgtgtcatgttctgaggaaggtagttgactattaagttggtcttgctgtcttctgtgttcccagagtcaactggtgacgaacagttgttgtttatggtggttggaccattggctgtgttattgcaagttggcccattagacagttgtgtttccatggcagcaattacctgctgcgtctcaacagtttccttcttgcgctacacgcggccgcacccgggcacgtccacgcccgtgcacgctgccaggcgcgact

SEQ ID NO: 19272 - RNA, 1233 nt, Homo sapiens
  source 1..1233: mol_type = other RNA
tgttcctctgtctcccagacggtatccattgaggctagctatcgccatggcagcctcatcatagtttgtcatagtcacaaatccaaaacctttgcatttattggtgttaaagtcacggatgaccttcacattggtgacagctccaaaaggcccaaacatttgccacaggatactctcatctgcgtcaggagccaggttgtacacaaatatacaccaccctgttccagggtgcccagggatattaattccagccaaactggtcattccgtcaatggtcattggagaaaacctaaaacgctgtgcctgctgagctagcggtcctggataccttctgtttggagactggtacagctgggaaaggatggcctgattggttttttggcttgggttattagcaaactttacagtgattggctccgtggcaccgggaggtttctggccatttaggcctttgatagcttcttctgcctcaattcgcttgtcaaatcgaataaaccctacaccccttgatatgccagtgacctggtcgacaagaatacgagaagtaataatgcgtccatattgtgaaaaaagctgttccaactccttctgggtcattgtttttggaagtccgctgacatataaatttgcatctctgatagaagctgaacttgggcgagcataggaaacttttattgttttggtttgaagtctcaatccattcagggtgttgatagctttctctgcatccttggggtcaatgtagttcacaaagccatatcccaagctctgccctgttattttgtctcttacaagcttacaggactctatttcaccaatgctcccaaagagactctttagttcctcctgtgtcatgttctgaggaaggtagttgactattaagttggtcttgctgtcttctgtgttcccagagtcaactggtgacgaacagttgttgtttatggtggttggaccattggctgtgttattgcaagttggcccattagacagttgtgtttccatggcagcaattacctgctgctgtgactcgaagctgcagctactacggctcgtgccgctggccgtcagcactgccgcggaggagtcgctcggggcgagctccgcggagaggcggtggcggcggcggcggcgggaaaggggactggaagccggcggaacccccgccccacccgcgccgcgccgcgccgcgccggcaaccgccctcctcacccggccggctactgcctcagtgac

SEQ ID NO: 19273 - RNA, 1230 nt, Homo sapiens
  source 1..1230: mol_type = other RNA
tgttcctctgtctcccagacggtatccattgaggctagctatcgccatggcagcctcatcatagtttgtcatagtcacaaatccaaaacctttgcatttattggtgttaaagtcacggatgaccttcacattggtgacagctccaaaaggcccaaacatttgccacaggatactctcatctgcgtcaggagccaggttgtacacaaatatacaccaccctgttccagggtgcccagggatattaattccagccaaactggtcattccgtcaatggtcattggagaaaacctaaaacgctgtgcctgctgagctagcggtcctggataccttctgtttggagactggtacagctgggaaaggatggcctgattggttttttggcttgggttattagcaaactttacagtgattggctccgtggcaccgggaggtttctggccatttaggcctttgatagcttcttctgcctcaattcgcttgtcaaatcgaataaaccctacaccccttgatatgccagtgacctggtcgacaagaatacgagaagtaataatgcgtccatattgtgaaaaaagctgttccaactccttctgggtcattgtttttggaagtccgctgacatataaatttgcatctctgatagaagctgaacttgggcgagcataggaaacttttattgttttggtttgaagtctcaatccattcagggtgttgatagctttctctgcatccttggggtcaatgtagttcacaaagccatatcccaagctctgccctgttattttgtctcttacaagcttacaggactctatttcaccaatgctcccaaagagactctttagttcctcctgtgtcatgttctgaggaaggtagttgactattaagttggtcttgctgtcttctgtgttcccagagtcaactggtgacgaacagttgttgtttatggtggttggaccattggctgtgttattgcaagttggcccattagacagttgtgtttccatggcagcaattacctgctgtgactcgaagctgcagctactacggctcgtgccgctggccgtcagcactgccgcggaggagtcgctcggggcgagctccgcggagaggcggtggcggcggcggcggcgggaaaggggactggaagccggcggaacccccgccccacccgcgccgcgccgcgccgcgccggcaaccgccctcctcacccggccggctactgcctcagtgac

SEQ ID NO: 19274 - RNA, 1452 nt, Homo sapiens
  source 1..1452: mol_type = other RNA
tgttcctctgtctcccagacggtatccattgaggctagctatcgccatggcagcctcatcatagtttgtcatagtcacaaatccaaaacctttgcatttattggtgttaaagtcacggatgaccttcacattggtgacagctccaaaaggcccaaacatttgccacaggatactctcatctgcgtcaggagccaggttgtacacaaatatacaccaccctgttccagggtgcccagggatattaattccagccaaactggtcattccgtcaatggtcattggagaaaacctaaaacgctgtgcctgctgagctagcggtcctggataccttctgtttggagactggtacagctgggaaaggatggcctgattggttttttggcttgggttattagcaaactttacagtgattggctccgtggcaccgggaggtttctggccatttaggcctttgatagcttcttctgcctcaattcgcttgtcaaatcgaataaaccctacaccccttgatatgccagtgacctggtcgacaagaatacgagaagtaataatgcgtccatattgtgaaaaaagctgttccaactccttctgggtcattgtttttggaagtccgctgacatataaatttgcatctctgatagaagctgaacttgggcgagcataggaaacttttattgttttggtttgaagtctcaatccattcagggtgttgatagctttctctgcatccttggggtcaatgtagttcacaaagccatatcccaagctctgccctgttattttgtctcttacaagcttacaggactctatttcaccaatgctcccaaagagactctttagttcctcctgtgtcatgttctgaggaaggtagttgactattaagttggtcttgctgtcttctgtgttcccagagtcaactggtgacgaacagttgttgtttatggtggttggaccattggctgtgttattgcaagttggcccattagacagttgtgtttccatggcagcaattacctgctttctcccttaaggtttttgtgtatgtgtgtttttaaagtaacggtgcagttctcccaataaggatgagcaagaagctgctggatagttctcttaagacagcacgaaacctaaactgtgctcggcttaaaagaagcaaataaaaagaaacgctttcgaccccaaagtccaatgctaaaagaaatggcgaaaaaaaatatgaaaggggaggggaaacttaaaaaagagtttaaaaagacggagagactaccctcctattgccgttcaactaaacaaaaaggggcaagaaaaacaaaccaaggaacaaagaaaagagacgaaagaacgttttttcaaaaagacgatgtctttctccttgttgctttttagtaggtcgctacaggagtaagctgctgcatctctaactaagaacagaaataggggggaggacgtctt

SEQ ID NO: 19275 - RNA, 893 nt, Homo sapiens
  source 1..893: mol_type = other RNA
tgttcctctgtctcccagacggtatccattgaggctagctatcgccatggcagcctcatcatagtttgtcatagtcacaaatccaaaacctttgcatttattggtgttaaagtcacggatgaccttcacattggtgacagctccaaaaggcccaaacatttgccacaggatactctcatctgcgtcaggagccaggttgtacacaaatatacaccaccctgttccagggtgcccagggatattaattccagccaaactggtcattccgtcaatggtcattggagaaaacctaaaacgctgtgcctgctgagctagcggtcctggataccttctgtttggagactggtacagctgggaaaggatggcctgattggttttttggcttgggttattagcaaactttacagtgattggctccgtggcaccgggaggtttctggccatttaggcctttgatagcttcttctgcctcaattcgcttgtcaaatcgaataaaccctacaccccttgatatgccagtgacctggtcgacaagaatacgagaagtaataatgcgtccatattgtgaaaaaagctgttccaactccttctgggtcattgtttttggaagtccgctgacatataaatttgcatctctgatagaagctgaacttgggcgagcataggaaacttttattgttttggtttgaagtctcaatccattcagggtgttgatagctttctctgcatccttggggtcaatgtagttcacaaagccatatcccaagctctgcccttttagctacatggtattttactgtttaattgtagcttcacattaaccatgttcggtattcagattcttctcctacaaggtagaaatgatatctgaagcttggcaaggtcaatcagctt

SEQ ID NO: 19276 - RNA, 1559 nt, Homo sapiens
  source 1..1559: mol_type = other RNA
tgttcctctgtctcccagacggtatccattgaggctagctatcgccatggcagcctcatcatagtttgtcatagtcacaaatccaaaacctttgcatttattggtgttaaagtcacggatgaccttcacattggtgacagctccaaaaggcccaaacatttgccacaggatactctcatctgcgtcaggagccaggttgtacacaaatatacaccaccctgttccagggtgcccagggatattaattccagccaaactggtcattccgtcaatggtcattggagaaaacctctttactccataagccatattgagcagattgtccaacctaaaacgctgtgcctgctgagctagcggtcctggataccttctgtttggagactggtacagctgggaaaggatggcctgattggttttttggcttgggttattagcaaactttacagtgattggctccgtggcaccgggaggtttctggccatttaggcctttgatagcttcttctgcctcaattcgcttgtcaaatcgaataaaccctacaccccttgatatgccagtgacctggtcgacaagaatacgagaagtaataatgcgtccatattgtgaaaaaagctgttccaactccttctgggtcattgtttttggaagtccgctgacatataaatttgcatctctgatagaagctgaacttgggcgagcataggaaacttttattgttttggtttgaagtctcaatccattcagggtgttgatagctttctctgcatccttggggtcaatgtagttcacaaagccatatcccaagctctgccctgttattttgtctcttacaagcttacaggactctatttcaccaatgctcccaaagagactctttagttcctcctgtgtcatgttctgaggaaggtagttgactattaagttggtcttgctgtcttctgtgttcccagagtcaactggtgacgaacagttgttgtttatggtggttggaccattggctgtgttattgcaagttggcccattagacagttgtgtttccatggcagcaattaccccggtccaaggctctgctgcccacgaaccacttctaagcagagaagccacatcacacagtctgactgccatgttagtttggagttgccgtcacggcaacctcatattgctttgtcatgctttttgcacttaaattttcaaaactgcttgtgctgggcgcagaactgggaaggcagggctaaagtatctctccagccagctcaactgcaggagaggaaagccccatctaagttcactagccctgccacagtcttccactgcctgatgggttccttcaggaaaacacttccagaggcattcatccacttgaggtctggggttggctgctgctgcgaggctgctgcagccgaggctcccgcgagcagctgctaggatccttgccgtctcgttcctgcctctttcgagctgcacaatagccccggctgggtgcacctcattaagccagccgagagccccaggagcagggcaagccgtgtgacagcgctacctctttgtaatgactgtat

SEQ ID NO: 19277 - RNA, 1579 nt, Homo sapiens
  source 1..1579: mol_type = other RNA
tgttcctctgtctcccagacggtatccattgaggctagctatcgccatggcagcctcatcatagtttgtcatagtcacaaatccaaaacctttgcatttattggtgttaaagtcacggatgaccttcacattggtgacagctccaaaaggcccaaacatttgccacaggatactctcatctgcgtcaggagccaggttgtacacaaatatacaccaccctgttccagggtgcccagggatattaattccagccaaactggtcattccgtcaatggtcattggagaaaacctctttactccataagccatattgagcagattgtccaacctaaaacgctgtgcctgctgagctagcggtcctggataccttctgtttggagactggtacagctgggaaaggatggcctgattggttttttggcttgggttattagcaaactttacagtgattggctccgtggcaccgggaggtttctggccatttaggcctttgatagcttcttctgcctcaattcgcttgtcaaatcgaataaaccctacaccccttgatatgccagtgacctggtcgacaagaatacgagaagtaataatgcgtccatattgtgaaaaaagctgttccaactccttctgggtcattgtttttggaagtccgctgacatataaatttgcatctctgatagaagctgaacttgggcgagcataggaaacttttattgttttggtttgaagtctcaatccattcagggtgttgatagctttctctgcatccttggggtcaatgtagttcacaaagccatatcccaagctctgccctgttattttgtctcttacaagcttacaggactctatttcaccaatgctcccaaagagactctttagttcctcctgtgtcatgttctgaggaaggtagttgactattaagttggtcttgctgtcttctgtgttcccagagtcaactggtgacgaacagttgttgtttatggtggttggaccattggctgtgttattgcaagttggcccattagacagttgtgtttccatggcagcaattaccccggtccaaggctctgctgcccacgaaccacttctaagcagagaagccacatcacacagtctgactgccatgttagtttggagttgccgtctttctcccttaaggtttttgtgtatgtgtgtttttaaagtaacggtgcagttctcccaataaggatgagcaagaagctgctggatagttctcttaagacagcacgaaacctaaactgtgctcggcttaaaagaagcaaataaaaagaaacgctttcgaccccaaagtccaatgctaaaagaaatggcgaaaaaaaatatgaaaggggaggggaaacttaaaaaagagtttaaaaagacggagagactaccctcctattgccgttcaactaaacaaaaaggggcaagaaaaacaaaccaaggaacaaagaaaagagacgaaagaacgttttttcaaaaagacgatgtctttctccttgttgctttttagtaggtcgctacaggagtaagctgctgcatctctaactaagaacagaaataggggggaggacgtctt

SEQ ID NO: 19278 - RNA, 1471 nt, Homo sapiens
  source 1..1471: mol_type = other RNA
tgttcctctgtctcccagacggtatccattgaggctagctatcgccatggcagcctcatcatagtttgtcatagtcacaaatccaaaacctttgcatttattggtgttaaagtcacggatgaccttcacattggtgacagctccaaaaggcccaaacatttgccacaggatactctcatctgcgtcaggagccaggttgtacacaaatatacaccaccctgttccagggtgcccagggatattaattccagccaaactggtcattccgtcaatggtcattggagaaaacctctttactccataagccatattgagcagattgtccaacctaaaacgctgtgcctgctgagctagcggtcctggataccttctgtttggagactggtacagctgggaaaggatggcctgattggttttttggcttgggttattagcaaactttacagtgattggctccgtggcaccgggaggtttctggccatttaggcctttgatagcttcttctgcctcaattcgcttgtcaaatcgaataaaccctacaccccttgatatgccagtgacctggtcgacaagaatacgagaagtaataatgcgtccatattgtgaaaaaagctgttccaactccttctgggtcattgtttttggaagtccgctgacatataaatttgcatctctgatagaagctgaacttgggcgagcataggaaacttttattgttttggtttgaagtctcaatccattcagggtgttgatagctttctctgcatccttggggtcaatgtagttcacaaagccatatcccaagctctgccctgttattttgtctcttacaagcttacaggactctatttcaccaatgctcccaaagagactctttagttcctcctgtgtcatgttctgaggaaggtagttgactattaagttggtcttgctgtcttctgtgttcccagagtcaactggtgacgaacagttgttgtttatggtggttggaccattggctgtgttattgcaagttggcccattagacagttgtgtttccatggcagcaattacctgcacggcaacctcatattgctttgtcatgctttttgcacttaaattttcaaaactgcttgtgctgggcgcagaactgggaaggcagggctaaagtatctctccagccagctcaactgcaggagaggaaagccccatctaagttcactagccctgccacagtcttccactgcctgatgggttccttcaggaaaacacttccagaggcattcatccacttgaggtctggggttggctgctgctgcgaggctgctgcagccgaggctcccgcgagcagctgctaggatccttgccgtctcgttcctgcctctttcgagctgcacaatagccccggctgggtgcacctcattaagccagccgagagccccaggagcagggcaagccgtgtgacagcgctacctctttgtaatgactgtat

SEQ ID NO: 19279 - RNA, 1562 nt, Homo sapiens
  source 1..1562: mol_type = other RNA
tgttcctctgtctcccagacggtatccattgaggctagctatcgccatggcagcctcatcatagtttgtcatagtcacaaatccaaaacctttgcatttattggtgttaaagtcacggatgaccttcacattggtgacagctccaaaaggcccaaacatttgccacaggatactctcatctgcgtcaggagccaggttgtacacaaatatacaccaccctgttccagggtgcccagggatattaattccagccaaactggtcattccgtcaatggtcattggagaaaacctctttactccataagccatattgagcagattgtccaacctaaaacgctgtgcctgctgagctagcggtcctggataccttctgtttggagactggtacagctgggaaaggatggcctgattggttttttggcttgggttattagcaaactttacagtgattggctccgtggcaccgggaggtttctggccatttaggcctttgatagcttcttctgcctcaattcgcttgtcaaatcgaataaaccctacaccccttgatatgccagtgacctggtcgacaagaatacgagaagtaataatgcgtccatattgtgaaaaaagctgttccaactccttctgggtcattgtttttggaagtccgctgacatataaatttgcatctctgatagaagctgaacttgggcgagcataggaaacttttattgttttggtttgaagtctcaatccattcagggtgttgatagctttctctgcatccttggggtcaatgtagttcacaaagccatatcccaagctctgccctgttattttgtctcttacaagcttacaggactctatttcaccaatgctcccaaagagactctttagttcctcctgtgtcatgttctgaggaaggtagttgactattaagttggtcttgctgtcttctgtgttcccagagtcaactggtgacgaacagttgttgtttatggtggttggaccattggctgtgttattgcaagttggcccattagacagttgtgtttccatggcagcaattacctgcccggtccaaggctctgctgcccacgaaccacttctaagcagagaagccacatcacacagtctgactgccatgttagtttggagttgccgtcacggcaacctcatattgctttgtcatgctttttgcacttaaattttcaaaactgcttgtgctgggcgcagaactgggaaggcagggctaaagtatctctccagccagctcaactgcaggagaggaaagccccatctaagttcactagccctgccacagtcttccactgcctgatgggttccttcaggaaaacacttccagaggcattcatccacttgaggtctggggttggctgctgctgcgaggctgctgcagccgaggctcccgcgagcagctgctaggatccttgccgtctcgttcctgcctctttcgagctgcacaatagccccggctgggtgcacctcattaagccagccgagagccccaggagcagggcaagccgtgtgacagcgctacctctttgtaatgactgtat

SEQ ID NO: 19280 - RNA, 1369 nt, Homo sapiens
  source 1..1369: mol_type = other RNA
tgttcctctgtctcccagacggtatccattgaggctagctatcgccatggcagcctcatcatagtttgtcatagtcacaaatccaaaacctttgcatttattggtgttaaagtcacggatgaccttcacattggtgacagctccaaaaggcccaaacatttgccacaggatactctcatctgcgtcaggagccaggttgtacacaaatatacaccaccctgttccagggtgcccagggatattaattccagccaaactggtcattccgtcaatggtcattggagaaaacctctttactccataagccatattgagcagattgtccaacctaaaacgctgtgcctgctgagctagcggtcctggataccttctgtttggagactggtacagctgggaaaggatggcctgattggttttttggcttgggttattagcaaactttacagtgattggctccgtggcaccgggaggtttctggccatttaggcctttgatagcttcttctgcctcaattcgcttgtcaaatcgaataaaccctacaccccttgatatgccagtgacctggtcgacaagaatacgagaagtaataatgcgtccatattgtgaaaaaagctgttccaactccttctgggtcattgtttttggaagtccgctgacatataaatttgcatctctgatagaagctgaacttgggcgagcataggaaacttttattgttttggtttgaagtctcaatccattcagggtgttgatagctttctctgcatccttggggtcaatgtagttcacaaagccatatcccaagctctgccctgttattttgtctcttacaagcttacaggactctatttcaccaatgctcccaaagagactctttagttcctcctgtgtcatgttctgaggaaggtagttgactattaagttggtcttgctgtcttctgtgttcccagagtcaactggtgacgaacagttgttgtttatggtggttggaccattggctgtgttattgcaagttggcccattagacagttgtgtttccatggcagcaattacctgcccggtccaaggctctgctgcccacgaaccacttctaagcagagaagccacatcacacagtctgactgccatgttagtttggagttgccgtctaacgcgcacgaggggatcatcattgctcctgccctgggcgcccgcggccctacaccacctccgcacacaacgcggccggtgttaagtctccaaacgccccgagagctccaaggaccgcgcgcgcgaaggcgccgtagcaagtgggcacacaccagacaccaccccggcgtgttccgcgggagaagccagtgcacacatcctcccgcaaggcggggttgcc

SEQ ID NO: 19281 - RNA, 1514 nt, Homo sapiens
  source 1..1514: mol_type = other RNA
tgttcctctgtctcccagacggtatccattgaggctagctatcgccatggcagcctcatcatagtttgtcatagtcacaaatccaaaacctttgcatttattggtgttaaagtcacggatgaccttcacattggtgacagctccaaaaggcccaaacatttgccacaggatactctcatctgcgtcaggagccaggttgtacacaaatatacaccaccctgttccagggtgcccagggatattaattccagccaaactggtcattccgtcaatggtcattggagaaaacctctttactccataagccatattgagcagattgtccaacctaaaacgctgtgcctgctgagctagcggtcctggataccttctgtttggagactggtacagctgggaaaggatggcctgattggttttttggcttgggttattagcaaactttacagtgattggctccgtggcaccgggaggtttctggccatttaggcctttgatagcttcttctgcctcaattcgcttgtcaaatcgaataaaccctacaccccttgatatgccagtgacctggtcgacaagaatacgagaagtaataatgcgtccatattgtgaaaaaagctgttccaactccttctgggtcattgtttttggaagtccgctgacatataaatttgcatctctgatagaagctgaacttgggcgagcataggaaacttttattgttttggtttgaagtctcaatccattcagggtgttgatagctttctctgcatccttggggtcaatgtagttcacaaagccatatcccaagctctgccctgttattttgtctcttacaagcttacaggactctatttcaccaatgctcccaaagagactctttagttcctcctgtgtcatgttctgaggaaggtagttgactattaagttggtcttgctgtcttctgtgttcccagagtcaactggtgacgaacagttgttgtttatggtggttggaccattggctgtgttattgcaagttggcccattagacagttgtgtttccatggcagcaattacctgcccggtccaaggctctgctgcccacgaaccacttctaagcagagaagccacatcacacagtctgactgccatgttagtttggagttgccgtctgaaattgtaggaggtaagagaaaggaaccgagcagtgggcgacccagtcgccgcaagaacgtgaccgaggttacagcttcaagggcatgatgcaggtttgatgcagcaaggtccgctaagggcgtccagcgctccccgcccccatgcgacgggcggagcggggttggggggaagggaggggactcgtctaacccagggcgggtgtgggagaggcaaatttgccctcttgggcgaagtctaatcagcatagtgaagtagggggctcaaccaaggtcaaaagcgagataggccatcccttaatttgtgcgacccagtctggggacaccggatacagctaactgattctatatcagcatttccgtgtc

SEQ ID NO: 19282 - RNA, 1230 nt, Homo sapiens
  source 1..1230: mol_type = other RNA
tgttcctctgtctcccagacggtatccattgaggctagctatcgccatggcagcctcatcatagtttgtcatagtcacaaatccaaaacctttgcatttattggtgttaaagtcacggatgaccttcacattggtgacagctccaaaaggcccaaacatttgccacaggatactctcatctgcgtcaggagccaggttgtacacaaatatacaccaccctgttccagggtgcccagggatattaattccagccaaactggtcattccgtcaatggtcattggagaaaacctctttactccataagccatattgagcagattgtccaacctaaaacgctgtgcctgctgagctagcggtcctggataccttctgtttggagactggtacagctgggaaaggatggcctgattggttttttggcttgggttattagcaaactttacagtgattggctccgtggcaccgggaggtttctggccatttaggcctttgatagcttcttctgcctcaattcgcttgtcaaatcgaataaaccctacaccccttgatatgccagtgacctggtcgacaagaatacgagaagtaataatgcgtccatattgtgaaaaaagctgttccaactccttctgggtcattgtttttggaagtccgctgacatataaatttgcatctctgatagaagctgaacttgggcgagcataggaaacttttattgttttggtttgaagtctcaatccattcagggtgttgatagctttctctgcatccttggggtcaatgtagttcacaaagccatatcccaagctctgccctgttattttgtctcttacaagcttacaggactctatttcaccaatgctcccaaagagactctttagttcctcctgtgtcatgttctgaggaaggtagttgactattaagttggtcttgctgtcttctgtgttcccagagtcaactggtgacgaacagttgttgtttatggtggttggaccattggctgtgttattgcaagttggcccattagacagttgtgtttccatggcagcaattacctgcccggtccaaggctctgctgcccacgaaccacttctaagcagagaagccacatcacacagtctgactgccatgttagtttggagttgccgtctgcgtctcaacagtttccttcttgcgctacacgcggccgcacccgggcacgtccacgcccgtgcacgctgccaggcgcgact

SEQ ID NO: 19283 - RNA, 1363 nt, Homo sapiens
  source 1..1363: mol_type = other RNA
tgttcctctgtctcccagacggtatccattgaggctagctatcgccatggcagcctcatcatagtttgtcatagtcacaaatccaaaacctttgcatttattggtgttaaagtcacggatgaccttcacattggtgacagctccaaaaggcccaaacatttgccacaggatactctcatctgcgtcaggagccaggttgtacacaaatatacaccaccctgttccagggtgcccagggatattaattccagccaaactggtcattccgtcaatggtcattggagaaaacctctttactccataagccatattgagcagattgtccaacctaaaacgctgtgcctgctgagctagcggtcctggataccttctgtttggagactggtacagctgggaaaggatggcctgattggttttttggcttgggttattagcaaactttacagtgattggctccgtggcaccgggaggtttctggccatttaggcctttgatagcttcttctgcctcaattcgcttgtcaaatcgaataaaccctacaccccttgatatgccagtgacctggtcgacaagaatacgagaagtaataatgcgtccatattgtgaaaaaagctgttccaactccttctgggtcattgtttttggaagtccgctgacatataaatttgcatctctgatagaagctgaacttgggcgagcataggaaacttttattgttttggtttgaagtctcaatccattcagggtgttgatagctttctctgcatccttggggtcaatgtagttcacaaagccatatcccaagctctgccctgttattttgtctcttacaagcttacaggactctatttcaccaatgctcccaaagagactctttagttcctcctgtgtcatgttctgaggaaggtagttgactattaagttggtcttgctgtcttctgtgttcccagagtcaactggtgacgaacagttgttgtttatggtggttggaccattggctgtgttattgcaagttggcccattagacagttgtgtttccatggcagcaattacctgcccggtccaaggctctgctgcccacgaaccacttctaagcagagaagccacatcacacagtctgactgccatgttagtttggagttgccgtctgctgtgactcgaagctgcagctactacggctcgtgccgctggccgtcagcactgccgcggaggagtcgctcggggcgagctccgcggagaggcggtggcggcggcggcggcgggaaaggggactggaagccggcggaacccccgccccacccgcgccgcgccgcgccgcgccggcaaccgccctcctcacccggccggctactgcctcagtgac

SEQ ID NO: 19284 - RNA, 1582 nt, Homo sapiens
  source 1..1582: mol_type = other RNA
tgttcctctgtctcccagacggtatccattgaggctagctatcgccatggcagcctcatcatagtttgtcatagtcacaaatccaaaacctttgcatttattggtgttaaagtcacggatgaccttcacattggtgacagctccaaaaggcccaaacatttgccacaggatactctcatctgcgtcaggagccaggttgtacacaaatatacaccaccctgttccagggtgcccagggatattaattccagccaaactggtcattccgtcaatggtcattggagaaaacctctttactccataagccatattgagcagattgtccaacctaaaacgctgtgcctgctgagctagcggtcctggataccttctgtttggagactggtacagctgggaaaggatggcctgattggttttttggcttgggttattagcaaactttacagtgattggctccgtggcaccgggaggtttctggccatttaggcctttgatagcttcttctgcctcaattcgcttgtcaaatcgaataaaccctacaccccttgatatgccagtgacctggtcgacaagaatacgagaagtaataatgcgtccatattgtgaaaaaagctgttccaactccttctgggtcattgtttttggaagtccgctgacatataaatttgcatctctgatagaagctgaacttgggcgagcataggaaacttttattgttttggtttgaagtctcaatccattcagggtgttgatagctttctctgcatccttggggtcaatgtagttcacaaagccatatcccaagctctgccctgttattttgtctcttacaagcttacaggactctatttcaccaatgctcccaaagagactctttagttcctcctgtgtcatgttctgaggaaggtagttgactattaagttggtcttgctgtcttctgtgttcccagagtcaactggtgacgaacagttgttgtttatggtggttggaccattggctgtgttattgcaagttggcccattagacagttgtgtttccatggcagcaattacctgcccggtccaaggctctgctgcccacgaaccacttctaagcagagaagccacatcacacagtctgactgccatgttagtttggagttgccgtctttctcccttaaggtttttgtgtatgtgtgtttttaaagtaacggtgcagttctcccaataaggatgagcaagaagctgctggatagttctcttaagacagcacgaaacctaaactgtgctcggcttaaaagaagcaaataaaaagaaacgctttcgaccccaaagtccaatgctaaaagaaatggcgaaaaaaaatatgaaaggggaggggaaacttaaaaaagagtttaaaaagacggagagactaccctcctattgccgttcaactaaacaaaaaggggcaagaaaaacaaaccaaggaacaaagaaaagagacgaaagaacgttttttcaaaaagacgatgtctttctccttgttgctttttagtaggtcgctacaggagtaagctgctgcatctctaactaagaacagaaataggggggaggacgtctt

SEQ ID NO: 19285 - RNA, 1136 nt, Homo sapiens
  source 1..1136: mol_type = other RNA
tgttcctctgtctcccagacggtatccattgaggctagctatcgccatggcagcctcatcatagtttgtcatagtcacaaatccaaaacctttgcatttattggtgttaaagtcacggatgaccttcacattggtgacagctccaaaaggcccaaacatttgccacaggatactctcatctgcgtcaggagccaggttgtacacaaatatacaccaccctgttccagggtgcccagggatattaattccagccaaactggtcattccgtcaatggtcattggagaaaacctctttactccataagccatattgagcagattgtccaacctaaaacgctgtgcctgctgagctagcggtcctggataccttctgtttggagactggtacagctgggaaaggatggcctgattggttttttggcttgggttattagcaaactttacagtgattggctccgtggcaccgggaggtttctggccatttaggcctttgatagcttcttctgcctcaattcgcttgtcaaatcgaataaaccctacaccccttgatatgccagtgacctggtcgacaagaatacgagaagtaataatgcgtccatattgtgaaaaaagctgttccaactccttctgggtcattgtttttggaagtccgctgacatataaatttgcatctctgatagaagctgaacttgggcgagcataggaaacttttattgttttggtttgaagtctcaatccattcagggtgttgatagctttctctgcatccttggggtcaatgtagttcacaaagccatatcccaagctctgccctgttattttgtctcttacaagcttacaggactctatttcaccaatgctcccaaagagactctttagttcctcctgtgtcatgttctgaggaaggtagttgactattaagttggtcttgctgtcttctgtgttcccagagtcaactggtgacgaacagttgttgtttatggtggttggaccattggctgtgttattgcaagttggcccattagacagttgtgtttccatggcagcaattacctgcgtctcaacagtttccttcttgcgctacacgcggccgcacccgggcacgtccacgcccgtgcacgctgccaggcgcgact

SEQ ID NO: 19286 - RNA, 1133 nt, Homo sapiens
  source 1..1133: mol_type = other RNA
tgttcctctgtctcccagacggtatccattgaggctagctatcgccatggcagcctcatcatagtttgtcatagtcacaaatccaaaacctttgcatttattggtgttaaagtcacggatgaccttcacattggtgacagctccaaaaggcccaaacatttgccacaggatactctcatctgcgtcaggagccaggttgtacacaaatatacaccaccctgttccagggtgcccagggatattaattccagccaaactggtcattccgtcaatggtcattggagaaaacctctttactccataagccatattgagcagattgtccaacctaaaacgctgtgcctgctgagctagcggtcctggataccttctgtttggagactggtacagctgggaaaggatggcctgattggttttttggcttgggttattagcaaactttacagtgattggctccgtggcaccgggaggtttctggccatttaggcctttgatagcttcttctgcctcaattcgcttgtcaaatcgaataaaccctacaccccttgatatgccagtgacctggtcgacaagaatacgagaagtaataatgcgtccatattgtgaaaaaagctgttccaactccttctgggtcattgtttttggaagtccgctgacatataaatttgcatctctgatagaagctgaacttgggcgagcataggaaacttttattgttttggtttgaagtctcaatccattcagggtgttgatagctttctctgcatccttggggtcaatgtagttcacaaagccatatcccaagctctgccctgttattttgtctcttacaagcttacaggactctatttcaccaatgctcccaaagagactctttagttcctcctgtgtcatgttctgaggaaggtagttgactattaagttggtcttgctgtcttctgtgttcccagagtcaactggtgacgaacagttgttgtttatggtggttggaccattggctgtgttattgcaagttggcccattagacagttgtgtttccatggcagcaattacctgctgaaaacaacgaggttcattattgaataaaggcatcaggaattcttggagatggagctttcaaataaggctttagt

SEQ ID NO: 19287 - RNA, 1423 nt, Homo sapiens
  source 1..1423: mol_type = other RNA
tgttcctctgtctcccagacggtatccattgaggctagctatcgccatggcagcctcatcatagtttgtcatagtcacaaatccaaaacctttgcatttattggtgttaaagtcacggatgaccttcacattggtgacagctccaaaaggcccaaacatttgccacaggatactctcatctgcgtcaggagccaggttgtacacaaatatacaccaccctgttccagggtgcccagggatattaattccagccaaactggtcattccgtcaatggtcattggagaaaacctctttactccataagccatattgagcagattgtccaacctaaaacgctgtgcctgctgagctagcggtcctggataccttctgtttggagactggtacagctgggaaaggatggcctgattggttttttggcttgggttattagcaaactttacagtgattggctccgtggcaccgggaggtttctggccatttaggcctttgatagcttcttctgcctcaattcgcttgtcaaatcgaataaaccctacaccccttgatatgccagtgacctggtcgacaagaatacgagaagtaataatgcgtccatattgtgaaaaaagctgttccaactccttctgggtcattgtttttggaagtccgctgacatataaatttgcatctctgatagaagctgaacttgggcgagcataggaaacttttattgttttggtttgaagtctcaatccattcagggtgttgatagctttctctgcatccttggggtcaatgtagttcacaaagccatatcccaagctctgccctgttattttgtctcttacaagcttacaggactctatttcaccaatgctcccaaagagactctttagttcctcctgtgtcatgttctgaggaaggtagttgactattaagttggtcttgctgtcttctgtgttcccagagtcaactggtgacgaacagttgttgtttatggtggttggaccattggctgtgttattgcaagttggcccattagacagttgtgtttccatggcagcaattacctgctgaaattgtaggaggtaagagaaaggaaccgagcagtgggcgacccagtcgccgcaagaacgtgaccgaggttacagcttcaagggcatgatgcaggtttgatgcagcaaggtccgctaagggcgtccagcgctccccgcccccatgcgacgggcggagcggggttggggggaagggaggggactcgtctaacccagggcgggtgtgggagaggcaaatttgccctcttgggcgaagtctaatcagcatagtgaagtagggggctcaaccaaggtcaaaagcgagataggccatcccttaatttgtgcgacccagtctggggacaccggatacagctaactgattctatatcagcatttccgtgtc

SEQ ID NO: 19288 - RNA, 1139 nt, Homo sapiens
  source 1..1139: mol_type = other RNA
tgttcctctgtctcccagacggtatccattgaggctagctatcgccatggcagcctcatcatagtttgtcatagtcacaaatccaaaacctttgcatttattggtgttaaagtcacggatgaccttcacattggtgacagctccaaaaggcccaaacatttgccacaggatactctcatctgcgtcaggagccaggttgtacacaaatatacaccaccctgttccagggtgcccagggatattaattccagccaaactggtcattccgtcaatggtcattggagaaaacctctttactccataagccatattgagcagattgtccaacctaaaacgctgtgcctgctgagctagcggtcctggataccttctgtttggagactggtacagctgggaaaggatggcctgattggttttttggcttgggttattagcaaactttacagtgattggctccgtggcaccgggaggtttctggccatttaggcctttgatagcttcttctgcctcaattcgcttgtcaaatcgaataaaccctacaccccttgatatgccagtgacctggtcgacaagaatacgagaagtaataatgcgtccatattgtgaaaaaagctgttccaactccttctgggtcattgtttttggaagtccgctgacatataaatttgcatctctgatagaagctgaacttgggcgagcataggaaacttttattgttttggtttgaagtctcaatccattcagggtgttgatagctttctctgcatccttggggtcaatgtagttcacaaagccatatcccaagctctgccctgttattttgtctcttacaagcttacaggactctatttcaccaatgctcccaaagagactctttagttcctcctgtgtcatgttctgaggaaggtagttgactattaagttggtcttgctgtcttctgtgttcccagagtcaactggtgacgaacagttgttgtttatggtggttggaccattggctgtgttattgcaagttggcccattagacagttgtgtttccatggcagcaattacctgctgcgtctcaacagtttccttcttgcgctacacgcggccgcacccgggcacgtccacgcccgtgcacgctgccaggcgcgact

SEQ ID NO: 19289 - RNA, 1272 nt, Homo sapiens
  source 1..1272: mol_type = other RNA
tgttcctctgtctcccagacggtatccattgaggctagctatcgccatggcagcctcatcatagtttgtcatagtcacaaatccaaaacctttgcatttattggtgttaaagtcacggatgaccttcacattggtgacagctccaaaaggcccaaacatttgccacaggatactctcatctgcgtcaggagccaggttgtacacaaatatacaccaccctgttccagggtgcccagggatattaattccagccaaactggtcattccgtcaatggtcattggagaaaacctctttactccataagccatattgagcagattgtccaacctaaaacgctgtgcctgctgagctagcggtcctggataccttctgtttggagactggtacagctgggaaaggatggcctgattggttttttggcttgggttattagcaaactttacagtgattggctccgtggcaccgggaggtttctggccatttaggcctttgatagcttcttctgcctcaattcgcttgtcaaatcgaataaaccctacaccccttgatatgccagtgacctggtcgacaagaatacgagaagtaataatgcgtccatattgtgaaaaaagctgttccaactccttctgggtcattgtttttggaagtccgctgacatataaatttgcatctctgatagaagctgaacttgggcgagcataggaaacttttattgttttggtttgaagtctcaatccattcagggtgttgatagctttctctgcatccttggggtcaatgtagttcacaaagccatatcccaagctctgccctgttattttgtctcttacaagcttacaggactctatttcaccaatgctcccaaagagactctttagttcctcctgtgtcatgttctgaggaaggtagttgactattaagttggtcttgctgtcttctgtgttcccagagtcaactggtgacgaacagttgttgtttatggtggttggaccattggctgtgttattgcaagttggcccattagacagttgtgtttccatggcagcaattacctgctgctgtgactcgaagctgcagctactacggctcgtgccgctggccgtcagcactgccgcggaggagtcgctcggggcgagctccgcggagaggcggtggcggcggcggcggcgggaaaggggactggaagccggcggaacccccgccccacccgcgccgcgccgcgccgcgccggcaaccgccctcctcacccggccggctactgcctcagtgac

SEQ ID NO: 19290 - RNA, 1249 nt, Homo sapiens
  source 1..1249: mol_type = other RNA
tgttcctctgtctcccagacggtatccattgaggctagctatcgccatggcagcctcatcatagtttgtcatagtcacaaatccaaaacctttgcatttattggtgttaaagtcacggatgaccttcacattggtgacagctccaaaaggcccaaacatttgccacaggatactctcatctgcgtcaggagccaggttgtacacaaatatacaccaccctgttccagggtgcccagggatattaattccagccaaactggtcattccgtcaatggtcattggagaaaacctctttactccataagccatattgagcagattgtccaacctaaaacgctgtgcctgctgagctagcggtcctggataccttctgtttggagactggtacagctgggaaaggatggcctgattggttttttggcttgggttattagcaaactttacagtgattggctccgtggcaccgggaggtttctggccatttaggcctttgatagcttcttctgcctcaattcgcttgtcaaatcgaataaaccctacaccccttgatatgccagtgacctggtcgacaagaatacgagaagtaataatgcgtccatattgtgaaaaaagctgttccaactccttctgggtcattgtttttggaagtccgctgacatataaatttgcatctctgatagaagctgaacttgggcgagcataggaaacttttattgttttggtttgaagtctcaatccattcagggtgttgatagctttctctgcatccttggggtcaatgtagttcacaaagccatatcccaagctctgccctgttattttgtctcttacaagcttacaggactctatttcaccaatgctcccaaagagactctttagttcctcctgtgtcatgttctgaggaaggtagttgactattaagttggtcttgctgtcttctgtgttcccagagtcaactggtgacgaacagttgttgtttatggtggttggaccattggctgtgttattgcaagttggcccattagacagttgtgtttccatggcagcaattacctgctgtgcggggtgctgtactctgcttcaaacgcaaagtaggaaatcctgcactcgactatgcaaacgcttgccgctagccgcatccttctatcgccccccaactcaagacccgaaatggccaactcttcaccgagggggcgtcccatcgctgccttgccttggcccgccccttcgccaagctcaatcccttttc

SEQ ID NO: 19291 - RNA, 1491 nt, Homo sapiens
  source 1..1491: mol_type = other RNA
tgttcctctgtctcccagacggtatccattgaggctagctatcgccatggcagcctcatcatagtttgtcatagtcacaaatccaaaacctttgcatttattggtgttaaagtcacggatgaccttcacattggtgacagctccaaaaggcccaaacatttgccacaggatactctcatctgcgtcaggagccaggttgtacacaaatatacaccaccctgttccagggtgcccagggatattaattccagccaaactggtcattccgtcaatggtcattggagaaaacctctttactccataagccatattgagcagattgtccaacctaaaacgctgtgcctgctgagctagcggtcctggataccttctgtttggagactggtacagctgggaaaggatggcctgattggttttttggcttgggttattagcaaactttacagtgattggctccgtggcaccgggaggtttctggccatttaggcctttgatagcttcttctgcctcaattcgcttgtcaaatcgaataaaccctacaccccttgatatgccagtgacctggtcgacaagaatacgagaagtaataatgcgtccatattgtgaaaaaagctgttccaactccttctgggtcattgtttttggaagtccgctgacatataaatttgcatctctgatagaagctgaacttgggcgagcataggaaacttttattgttttggtttgaagtctcaatccattcagggtgttgatagctttctctgcatccttggggtcaatgtagttcacaaagccatatcccaagctctgccctgttattttgtctcttacaagcttacaggactctatttcaccaatgctcccaaagagactctttagttcctcctgtgtcatgttctgaggaaggtagttgactattaagttggtcttgctgtcttctgtgttcccagagtcaactggtgacgaacagttgttgtttatggtggttggaccattggctgtgttattgcaagttggcccattagacagttgtgtttccatggcagcaattacctgctttctcccttaaggtttttgtgtatgtgtgtttttaaagtaacggtgcagttctcccaataaggatgagcaagaagctgctggatagttctcttaagacagcacgaaacctaaactgtgctcggcttaaaagaagcaaataaaaagaaacgctttcgaccccaaagtccaatgctaaaagaaatggcgaaaaaaaatatgaaaggggaggggaaacttaaaaaagagtttaaaaagacggagagactaccctcctattgccgttcaactaaacaaaaaggggcaagaaaaacaaaccaaggaacaaagaaaagagacgaaagaacgttttttcaaaaagacgatgtctttctccttgttgctttttagtaggtcgctacaggagtaagctgctgcatctctaactaagaacagaaataggggggaggacgtctt

SEQ ID NO: 19292 - RNA, 1488 nt, Homo sapiens
  source 1..1488: mol_type = other RNA
tgttcctctgtctcccagacggtatccattgaggctagctatcgccatggcagcctcatcatagtttgtcatagtcacaaatccaaaacctttgcatttattggtgttaaagtcacggatgaccttcacattggtgacagctccaaaaggcccaaacatttgccacaggatactctcatctgcgtcaggagccaggttgtacacaaatatacaccaccctgttccagggtgcccagggatattaattccagccaaactggtcattccgtcaatggtcattggagaaaacctctttactccataagccatattgagcagattgtccaacctaaaacgctgtgcctgctgagctagcggtcctggataccttctgtttggagactggtacagctgggaaaggatggcctgattggttttttggcttgggttattagcaaactttacagtgattggctccgtggcaccgggaggtttctggccatttaggcctttgatagcttcttctgcctcaattcgcttgtcaaatcgaataaaccctacaccccttgatatgccagtgacctggtcgacaagaatacgagaagtaataatgcgtccatattgtgaaaaaagctgttccaactccttctgggtcattgtttttggaagtccgctgacatataaatttgcatctctgatagaagctgaacttgggcgagcataggaaacttttattgttttggtttgaagtctcaatccattcagggtgttgatagctttctctgcatccttggggtcaatgtagttcacaaagccatatcccaagctctgccctgttattttgtctcttacaagcttacaggactctatttcaccaatgctcccaaagagactctttagttcctcctgtgtcatgttctgaggaaggtagttgactattaagttggtcttgctgtcttctgtgttcccagagtcaactggtgacgaacagttgttgtttatggtggttggaccattggctgtgttattgcaagttggcccattagacagttgtgtttccatggcagcaattacctttctcccttaaggtttttgtgtatgtgtgtttttaaagtaacggtgcagttctcccaataaggatgagcaagaagctgctggatagttctcttaagacagcacgaaacctaaactgtgctcggcttaaaagaagcaaataaaaagaaacgctttcgaccccaaagtccaatgctaaaagaaatggcgaaaaaaaatatgaaaggggaggggaaacttaaaaaagagtttaaaaagacggagagactaccctcctattgccgttcaactaaacaaaaaggggcaagaaaaacaaaccaaggaacaaagaaaagagacgaaagaacgttttttcaaaaagacgatgtctttctccttgttgctttttagtaggtcgctacaggagtaagctgctgcatctctaactaagaacagaaataggggggaggacgtctt

SEQ ID NO: 19293 - RNA, 1435 nt, Homo sapiens
  source 1..1435: mol_type = other RNA
tgttcctctgtctcccagacggtatccattgaggctagctatcgccatggcagcctcatcatagtttgtcatagtcacaaatccaaaacctttgcatttattggtgttaaagtcacggatgaccttcacattggtgacagctccaaaaggcccaaacatttgccacaggatactctcatctgcgtcaggagccaggttgtacacaaatatacaccaccctgttccagggtgcccagggatattaattccagccaaactggtcattccgtcaatggtcattggagaaaacctgctaaaacgctgtgcctgctgagctagcggtcctggataccttctgtttggagactggtacagctgggaaaggatggcctgattggttttttggcttgggttattagcaaactttacagtgattggctccgtggcaccgggaggtttctggccatttaggcctttgatagcttcttctgcctcaattcgcttgtcaaatcgaataaaccctacaccccttgatatgccagtgacctggtcgacaagaatacgagaagtaataatgcgtccatattgtgaaaaaagctgttccaactccttctgggtcattgtttttggaagtccgctgacatataaatttgcatctctgatagaagctgaacttgggcgagcataggaaacttttattgttttggtttgaagtctcaatccattcagggtgttgatagctttctctgcatccttggggtcaatgtagttcacaaagccatatcccaagctctgccctgttattttgtctcttacaagcttacaggactctatttcaccaatgctcccaaagagactctttagttcctcctgtgtcatgttctgaggaaggtagttgactattaagttggtcttgctgtcttctgtgttcccagagtcaactggtgacgaacagttgttgtttatggtggttggaccattggctgtgttattgcaagttggcccattagacagttgtgtttccatggcagcaattacctgcacggcaacctcatattgctttgtcatgctttttgcacttaaattttcaaaactgcttgtgctgggcgcagaactgggaaggcagggctaaagtatctctccagccagctcaactgcaggagaggaaagccccatctaagttcactagccctgccacagtcttccactgcctgatgggttccttcaggaaaacacttccagaggcattcatccacttgaggtctggggttggctgctgctgcgaggctgctgcagccgaggctcccgcgagcagctgctaggatccttgccgtctcgttcctgcctctttcgagctgcacaatagccccggctgggtgcacctcattaagccagccgagagccccaggagcagggcaagccgtgtgacagcgctacctctttgtaatgactgtat

SEQ ID NO: 19294 - RNA, 1526 nt, Homo sapiens
  source 1..1526: mol_type = other RNA
tgttcctctgtctcccagacggtatccattgaggctagctatcgccatggcagcctcatcatagtttgtcatagtcacaaatccaaaacctttgcatttattggtgttaaagtcacggatgaccttcacattggtgacagctccaaaaggcccaaacatttgccacaggatactctcatctgcgtcaggagccaggttgtacacaaatatacaccaccctgttccagggtgcccagggatattaattccagccaaactggtcattccgtcaatggtcattggagaaaacctgctaaaacgctgtgcctgctgagctagcggtcctggataccttctgtttggagactggtacagctgggaaaggatggcctgattggttttttggcttgggttattagcaaactttacagtgattggctccgtggcaccgggaggtttctggccatttaggcctttgatagcttcttctgcctcaattcgcttgtcaaatcgaataaaccctacaccccttgatatgccagtgacctggtcgacaagaatacgagaagtaataatgcgtccatattgtgaaaaaagctgttccaactccttctgggtcattgtttttggaagtccgctgacatataaatttgcatctctgatagaagctgaacttgggcgagcataggaaacttttattgttttggtttgaagtctcaatccattcagggtgttgatagctttctctgcatccttggggtcaatgtagttcacaaagccatatcccaagctctgccctgttattttgtctcttacaagcttacaggactctatttcaccaatgctcccaaagagactctttagttcctcctgtgtcatgttctgaggaaggtagttgactattaagttggtcttgctgtcttctgtgttcccagagtcaactggtgacgaacagttgttgtttatggtggttggaccattggctgtgttattgcaagttggcccattagacagttgtgtttccatggcagcaattacctgcccggtccaaggctctgctgcccacgaaccacttctaagcagagaagccacatcacacagtctgactgccatgttagtttggagttgccgtcacggcaacctcatattgctttgtcatgctttttgcacttaaattttcaaaactgcttgtgctgggcgcagaactgggaaggcagggctaaagtatctctccagccagctcaactgcaggagaggaaagccccatctaagttcactagccctgccacagtcttccactgcctgatgggttccttcaggaaaacacttccagaggcattcatccacttgaggtctggggttggctgctgctgcgaggctgctgcagccgaggctcccgcgagcagctgctaggatccttgccgtctcgttcctgcctctttcgagctgcacaatagccccggctgggtgcacctcattaagccagccgagagccccaggagcagggcaagccgtgtgacagcgctacctctttgtaatgactgtat

SEQ ID NO: 19295 - RNA, 1562 nt, Homo sapiens
  source 1..1562: mol_type = other RNA
tgttcctctgtctcccagacggtatccattgaggctagctatcgccatggcagcctcatcatagtttgtcatagtcacaaatccaaaacctttgcatttattggtgttaaagtcacggatgaccttcacattggtgacagctccaaaaggcccaaacatttgccacaggatactctcatctgcgtcaggagccaggttgtacacaaatatacaccaccctgttccagggtgcccagggatattaattccagccaaactggtcattccgtcaatggtcattggagaaaacctgctctttactccataagccatattgagcagattgtccaacctaaaacgctgtgcctgctgagctagcggtcctggataccttctgtttggagactggtacagctgggaaaggatggcctgattggttttttggcttgggttattagcaaactttacagtgattggctccgtggcaccgggaggtttctggccatttaggcctttgatagcttcttctgcctcaattcgcttgtcaaatcgaataaaccctacaccccttgatatgccagtgacctggtcgacaagaatacgagaagtaataatgcgtccatattgtgaaaaaagctgttccaactccttctgggtcattgtttttggaagtccgctgacatataaatttgcatctctgatagaagctgaacttgggcgagcataggaaacttttattgttttggtttgaagtctcaatccattcagggtgttgatagctttctctgcatccttggggtcaatgtagttcacaaagccatatcccaagctctgccctgttattttgtctcttacaagcttacaggactctatttcaccaatgctcccaaagagactctttagttcctcctgtgtcatgttctgaggaaggtagttgactattaagttggtcttgctgtcttctgtgttcccagagtcaactggtgacgaacagttgttgtttatggtggttggaccattggctgtgttattgcaagttggcccattagacagttgtgtttccatggcagcaattaccccggtccaaggctctgctgcccacgaaccacttctaagcagagaagccacatcacacagtctgactgccatgttagtttggagttgccgtcacggcaacctcatattgctttgtcatgctttttgcacttaaattttcaaaactgcttgtgctgggcgcagaactgggaaggcagggctaaagtatctctccagccagctcaactgcaggagaggaaagccccatctaagttcactagccctgccacagtcttccactgcctgatgggttccttcaggaaaacacttccagaggcattcatccacttgaggtctggggttggctgctgctgcgaggctgctgcagccgaggctcccgcgagcagctgctaggatccttgccgtctcgttcctgcctctttcgagctgcacaatagccccggctgggtgcacctcattaagccagccgagagccccaggagcagggcaagccgtgtgacagcgctacctctttgtaatgactgtat

SEQ ID NO: 19296 - RNA, 1363 nt, Homo sapiens
  source 1..1363: mol_type = other RNA
tgttcctctgtctcccagacggtatccattgaggctagctatcgccatggcagcctcatcatagtttgtcatagtcacaaatccaaaacctttgcatttattggtgttaaagtcacggatgaccttcacattggtgacagctccaaaaggcccaaacatttgccacaggatactctcatctgcgtcaggagccaggttgtacacaaatatacaccaccctgttccagggtgcccagggatattaattccagccaaactggtcattccgtcaatggtcattggagaaaacctgctctttactccataagccatattgagcagattgtccaacctaaaacgctgtgcctgctgagctagcggtcctggataccttctgtttggagactggtacagctgggaaaggatggcctgattggttttttggcttgggttattagcaaactttacagtgattggctccgtggcaccgggaggtttctggccatttaggcctttgatagcttcttctgcctcaattcgcttgtcaaatcgaataaaccctacaccccttgatatgccagtgacctggtcgacaagaatacgagaagtaataatgcgtccatattgtgaaaaaagctgttccaactccttctgggtcattgtttttggaagtccgctgacatataaatttgcatctctgatagaagctgaacttgggcgagcataggaaacttttattgttttggtttgaagtctcaatccattcagggtgttgatagctttctctgcatccttggggtcaatgtagttcacaaagccatatcccaagctctgccctgttattttgtctcttacaagcttacaggactctatttcaccaatgctcccaaagagactctttagttcctcctgtgtcatgttctgaggaaggtagttgactattaagttggtcttgctgtcttctgtgttcccagagtcaactggtgacgaacagttgttgtttatggtggttggaccattggctgtgttattgcaagttggcccattagacagttgtgtttccatggcagcaattaccccggtccaaggctctgctgcccacgaaccacttctaagcagagaagccacatcacacagtctgactgccatgttagtttggagttgccgtctgctgtgactcgaagctgcagctactacggctcgtgccgctggccgtcagcactgccgcggaggagtcgctcggggcgagctccgcggagaggcggtggcggcggcggcggcgggaaaggggactggaagccggcggaacccccgccccacccgcgccgcgccgcgccgcgccggcaaccgccctcctcacccggccggctactgcctcagtgac

SEQ ID NO: 19297 - RNA, 1582 nt, Homo sapiens
  source 1..1582: mol_type = other RNA
tgttcctctgtctcccagacggtatccattgaggctagctatcgccatggcagcctcatcatagtttgtcatagtcacaaatccaaaacctttgcatttattggtgttaaagtcacggatgaccttcacattggtgacagctccaaaaggcccaaacatttgccacaggatactctcatctgcgtcaggagccaggttgtacacaaatatacaccaccctgttccagggtgcccagggatattaattccagccaaactggtcattccgtcaatggtcattggagaaaacctgctctttactccataagccatattgagcagattgtccaacctaaaacgctgtgcctgctgagctagcggtcctggataccttctgtttggagactggtacagctgggaaaggatggcctgattggttttttggcttgggttattagcaaactttacagtgattggctccgtggcaccgggaggtttctggccatttaggcctttgatagcttcttctgcctcaattcgcttgtcaaatcgaataaaccctacaccccttgatatgccagtgacctggtcgacaagaatacgagaagtaataatgcgtccatattgtgaaaaaagctgttccaactccttctgggtcattgtttttggaagtccgctgacatataaatttgcatctctgatagaagctgaacttgggcgagcataggaaacttttattgttttggtttgaagtctcaatccattcagggtgttgatagctttctctgcatccttggggtcaatgtagttcacaaagccatatcccaagctctgccctgttattttgtctcttacaagcttacaggactctatttcaccaatgctcccaaagagactctttagttcctcctgtgtcatgttctgaggaaggtagttgactattaagttggtcttgctgtcttctgtgttcccagagtcaactggtgacgaacagttgttgtttatggtggttggaccattggctgtgttattgcaagttggcccattagacagttgtgtttccatggcagcaattaccccggtccaaggctctgctgcccacgaaccacttctaagcagagaagccacatcacacagtctgactgccatgttagtttggagttgccgtctttctcccttaaggtttttgtgtatgtgtgtttttaaagtaacggtgcagttctcccaataaggatgagcaagaagctgctggatagttctcttaagacagcacgaaacctaaactgtgctcggcttaaaagaagcaaataaaaagaaacgctttcgaccccaaagtccaatgctaaaagaaatggcgaaaaaaaatatgaaaggggaggggaaacttaaaaaagagtttaaaaagacggagagactaccctcctattgccgttcaactaaacaaaaaggggcaagaaaaacaaaccaaggaacaaagaaaagagacgaaagaacgttttttcaaaaagacgatgtctttctccttgttgctttttagtaggtcgctacaggagtaagctgctgcatctctaactaagaacagaaataggggggaggacgtctt

SEQ ID NO: 19298 - RNA, 1474 nt, Homo sapiens
  source 1..1474: mol_type = other RNA
tgttcctctgtctcccagacggtatccattgaggctagctatcgccatggcagcctcatcatagtttgtcatagtcacaaatccaaaacctttgcatttattggtgttaaagtcacggatgaccttcacattggtgacagctccaaaaggcccaaacatttgccacaggatactctcatctgcgtcaggagccaggttgtacacaaatatacaccaccctgttccagggtgcccagggatattaattccagccaaactggtcattccgtcaatggtcattggagaaaacctgctctttactccataagccatattgagcagattgtccaacctaaaacgctgtgcctgctgagctagcggtcctggataccttctgtttggagactggtacagctgggaaaggatggcctgattggttttttggcttgggttattagcaaactttacagtgattggctccgtggcaccgggaggtttctggccatttaggcctttgatagcttcttctgcctcaattcgcttgtcaaatcgaataaaccctacaccccttgatatgccagtgacctggtcgacaagaatacgagaagtaataatgcgtccatattgtgaaaaaagctgttccaactccttctgggtcattgtttttggaagtccgctgacatataaatttgcatctctgatagaagctgaacttgggcgagcataggaaacttttattgttttggtttgaagtctcaatccattcagggtgttgatagctttctctgcatccttggggtcaatgtagttcacaaagccatatcccaagctctgccctgttattttgtctcttacaagcttacaggactctatttcaccaatgctcccaaagagactctttagttcctcctgtgtcatgttctgaggaaggtagttgactattaagttggtcttgctgtcttctgtgttcccagagtcaactggtgacgaacagttgttgtttatggtggttggaccattggctgtgttattgcaagttggcccattagacagttgtgtttccatggcagcaattacctgcacggcaacctcatattgctttgtcatgctttttgcacttaaattttcaaaactgcttgtgctgggcgcagaactgggaaggcagggctaaagtatctctccagccagctcaactgcaggagaggaaagccccatctaagttcactagccctgccacagtcttccactgcctgatgggttccttcaggaaaacacttccagaggcattcatccacttgaggtctggggttggctgctgctgcgaggctgctgcagccgaggctcccgcgagcagctgctaggatccttgccgtctcgttcctgcctctttcgagctgcacaatagccccggctgggtgcacctcattaagccagccgagagccccaggagcagggcaagccgtgtgacagcgctacctctttgtaatgactgtat

SEQ ID NO: 19299 - RNA, 1220 nt, Homo sapiens
  source 1..1220: mol_type = other RNA
tgttcctctgtctcccagacggtatccattgaggctagctatcgccatggcagcctcatcatagtttgtcatagtcacaaatccaaaacctttgcatttattggtgttaaagtcacggatgaccttcacattggtgacagctccaaaaggcccaaacatttgccacaggatactctcatctgcgtcaggagccaggttgtacacaaatatacaccaccctgttccagggtgcccagggatattaattccagccaaactggtcattccgtcaatggtcattggagaaaacctgctctttactccataagccatattgagcagattgtccaacctaaaacgctgtgcctgctgagctagcggtcctggataccttctgtttggagactggtacagctgggaaaggatggcctgattggttttttggcttgggttattagcaaactttacagtgattggctccgtggcaccgggaggtttctggccatttaggcctttgatagcttcttctgcctcaattcgcttgtcaaatcgaataaaccctacaccccttgatatgccagtgacctggtcgacaagaatacgagaagtaataatgcgtccatattgtgaaaaaagctgttccaactccttctgggtcattgtttttggaagtccgctgacatataaatttgcatctctgatagaagctgaacttgggcgagcataggaaacttttattgttttggtttgaagtctcaatccattcagggtgttgatagctttctctgcatccttggggtcaatgtagttcacaaagccatatcccaagctctgccctgttattttgtctcttacaagcttacaggactctatttcaccaatgctcccaaagagactctttagttcctcctgtgtcatgttctgaggaaggtagttgactattaagttggtcttgctgtcttctgtgttcccagagtcaactggtgacgaacagttgttgtttatggtggttggaccattggctgtgttattgcaagttggcccattagacagttgtgtttccatggcagcaattacctgcccggtccaaggctctgctgcccacgaaccacttctaagcagagaagccacatcacacagtctgactgccatgttagtttggagttgccgtcacggcaacctcatattgctttgtcatgctttttgcacttaaattttcaaaactgcttgtgctgggcgca

SEQ ID NO: 19300 - RNA, 1517 nt, Homo sapiens
  source 1..1517: mol_type = other RNA
tgttcctctgtctcccagacggtatccattgaggctagctatcgccatggcagcctcatcatagtttgtcatagtcacaaatccaaaacctttgcatttattggtgttaaagtcacggatgaccttcacattggtgacagctccaaaaggcccaaacatttgccacaggatactctcatctgcgtcaggagccaggttgtacacaaatatacaccaccctgttccagggtgcccagggatattaattccagccaaactggtcattccgtcaatggtcattggagaaaacctgctctttactccataagccatattgagcagattgtccaacctaaaacgctgtgcctgctgagctagcggtcctggataccttctgtttggagactggtacagctgggaaaggatggcctgattggttttttggcttgggttattagcaaactttacagtgattggctccgtggcaccgggaggtttctggccatttaggcctttgatagcttcttctgcctcaattcgcttgtcaaatcgaataaaccctacaccccttgatatgccagtgacctggtcgacaagaatacgagaagtaataatgcgtccatattgtgaaaaaagctgttccaactccttctgggtcattgtttttggaagtccgctgacatataaatttgcatctctgatagaagctgaacttgggcgagcataggaaacttttattgttttggtttgaagtctcaatccattcagggtgttgatagctttctctgcatccttggggtcaatgtagttcacaaagccatatcccaagctctgccctgttattttgtctcttacaagcttacaggactctatttcaccaatgctcccaaagagactctttagttcctcctgtgtcatgttctgaggaaggtagttgactattaagttggtcttgctgtcttctgtgttcccagagtcaactggtgacgaacagttgttgtttatggtggttggaccattggctgtgttattgcaagttggcccattagacagttgtgtttccatggcagcaattacctgcccggtccaaggctctgctgcccacgaaccacttctaagcagagaagccacatcacacagtctgactgccatgttagtttggagttgccgtctgaaattgtaggaggtaagagaaaggaaccgagcagtgggcgacccagtcgccgcaagaacgtgaccgaggttacagcttcaagggcatgatgcaggtttgatgcagcaaggtccgctaagggcgtccagcgctccccgcccccatgcgacgggcggagcggggttggggggaagggaggggactcgtctaacccagggcgggtgtgggagaggcaaatttgccctcttgggcgaagtctaatcagcatagtgaagtagggggctcaaccaaggtcaaaagcgagataggccatcccttaatttgtgcgacccagtctggggacaccggatacagctaactgattctatatcagcatttccgtgtc

SEQ ID NO: 19301 - RNA, 1233 nt, Homo sapiens
  source 1..1233: mol_type = other RNA
tgttcctctgtctcccagacggtatccattgaggctagctatcgccatggcagcctcatcatagtttgtcatagtcacaaatccaaaacctttgcatttattggtgttaaagtcacggatgaccttcacattggtgacagctccaaaaggcccaaacatttgccacaggatactctcatctgcgtcaggagccaggttgtacacaaatatacaccaccctgttccagggtgcccagggatattaattccagccaaactggtcattccgtcaatggtcattggagaaaacctgctctttactccataagccatattgagcagattgtccaacctaaaacgctgtgcctgctgagctagcggtcctggataccttctgtttggagactggtacagctgggaaaggatggcctgattggttttttggcttgggttattagcaaactttacagtgattggctccgtggcaccgggaggtttctggccatttaggcctttgatagcttcttctgcctcaattcgcttgtcaaatcgaataaaccctacaccccttgatatgccagtgacctggtcgacaagaatacgagaagtaataatgcgtccatattgtgaaaaaagctgttccaactccttctgggtcattgtttttggaagtccgctgacatataaatttgcatctctgatagaagctgaacttgggcgagcataggaaacttttattgttttggtttgaagtctcaatccattcagggtgttgatagctttctctgcatccttggggtcaatgtagttcacaaagccatatcccaagctctgccctgttattttgtctcttacaagcttacaggactctatttcaccaatgctcccaaagagactctttagttcctcctgtgtcatgttctgaggaaggtagttgactattaagttggtcttgctgtcttctgtgttcccagagtcaactggtgacgaacagttgttgtttatggtggttggaccattggctgtgttattgcaagttggcccattagacagttgtgtttccatggcagcaattacctgcccggtccaaggctctgctgcccacgaaccacttctaagcagagaagccacatcacacagtctgactgccatgttagtttggagttgccgtctgcgtctcaacagtttccttcttgcgctacacgcggccgcacccgggcacgtccacgcccgtgcacgctgccaggcgcgact

SEQ ID NO: 19302 - RNA, 1366 nt, Homo sapiens
  source 1..1366: mol_type = other RNA
tgttcctctgtctcccagacggtatccattgaggctagctatcgccatggcagcctcatcatagtttgtcatagtcacaaatccaaaacctttgcatttattggtgttaaagtcacggatgaccttcacattggtgacagctccaaaaggcccaaacatttgccacaggatactctcatctgcgtcaggagccaggttgtacacaaatatacaccaccctgttccagggtgcccagggatattaattccagccaaactggtcattccgtcaatggtcattggagaaaacctgctctttactccataagccatattgagcagattgtccaacctaaaacgctgtgcctgctgagctagcggtcctggataccttctgtttggagactggtacagctgggaaaggatggcctgattggttttttggcttgggttattagcaaactttacagtgattggctccgtggcaccgggaggtttctggccatttaggcctttgatagcttcttctgcctcaattcgcttgtcaaatcgaataaaccctacaccccttgatatgccagtgacctggtcgacaagaatacgagaagtaataatgcgtccatattgtgaaaaaagctgttccaactccttctgggtcattgtttttggaagtccgctgacatataaatttgcatctctgatagaagctgaacttgggcgagcataggaaacttttattgttttggtttgaagtctcaatccattcagggtgttgatagctttctctgcatccttggggtcaatgtagttcacaaagccatatcccaagctctgccctgttattttgtctcttacaagcttacaggactctatttcaccaatgctcccaaagagactctttagttcctcctgtgtcatgttctgaggaaggtagttgactattaagttggtcttgctgtcttctgtgttcccagagtcaactggtgacgaacagttgttgtttatggtggttggaccattggctgtgttattgcaagttggcccattagacagttgtgtttccatggcagcaattacctgcccggtccaaggctctgctgcccacgaaccacttctaagcagagaagccacatcacacagtctgactgccatgttagtttggagttgccgtctgctgtgactcgaagctgcagctactacggctcgtgccgctggccgtcagcactgccgcggaggagtcgctcggggcgagctccgcggagaggcggtggcggcggcggcggcgggaaaggggactggaagccggcggaacccccgccccacccgcgccgcgccgcgccgcgccggcaaccgccctcctcacccggccggctactgcctcagtgac

SEQ ID NO: 19303 - RNA, 1585 nt, Homo sapiens
  source 1..1585: mol_type = other RNA
tgttcctctgtctcccagacggtatccattgaggctagctatcgccatggcagcctcatcatagtttgtcatagtcacaaatccaaaacctttgcatttattggtgttaaagtcacggatgaccttcacattggtgacagctccaaaaggcccaaacatttgccacaggatactctcatctgcgtcaggagccaggttgtacacaaatatacaccaccctgttccagggtgcccagggatattaattccagccaaactggtcattccgtcaatggtcattggagaaaacctgctctttactccataagccatattgagcagattgtccaacctaaaacgctgtgcctgctgagctagcggtcctggataccttctgtttggagactggtacagctgggaaaggatggcctgattggttttttggcttgggttattagcaaactttacagtgattggctccgtggcaccgggaggtttctggccatttaggcctttgatagcttcttctgcctcaattcgcttgtcaaatcgaataaaccctacaccccttgatatgccagtgacctggtcgacaagaatacgagaagtaataatgcgtccatattgtgaaaaaagctgttccaactccttctgggtcattgtttttggaagtccgctgacatataaatttgcatctctgatagaagctgaacttgggcgagcataggaaacttttattgttttggtttgaagtctcaatccattcagggtgttgatagctttctctgcatccttggggtcaatgtagttcacaaagccatatcccaagctctgccctgttattttgtctcttacaagcttacaggactctatttcaccaatgctcccaaagagactctttagttcctcctgtgtcatgttctgaggaaggtagttgactattaagttggtcttgctgtcttctgtgttcccagagtcaactggtgacgaacagttgttgtttatggtggttggaccattggctgtgttattgcaagttggcccattagacagttgtgtttccatggcagcaattacctgcccggtccaaggctctgctgcccacgaaccacttctaagcagagaagccacatcacacagtctgactgccatgttagtttggagttgccgtctttctcccttaaggtttttgtgtatgtgtgtttttaaagtaacggtgcagttctcccaataaggatgagcaagaagctgctggatagttctcttaagacagcacgaaacctaaactgtgctcggcttaaaagaagcaaataaaaagaaacgctttcgaccccaaagtccaatgctaaaagaaatggcgaaaaaaaatatgaaaggggaggggaaacttaaaaaagagtttaaaaagacggagagactaccctcctattgccgttcaactaaacaaaaaggggcaagaaaaacaaaccaaggaacaaagaaaagagacgaaagaacgttttttcaaaaagacgatgtctttctccttgttgctttttagtaggtcgctacaggagtaagctgctgcatctctaactaagaacagaaataggggggaggacgtctt

SEQ ID NO: 19304 - RNA, 1559 nt, Homo sapiens
  source 1..1559: mol_type = other RNA
tgttcctctgtctcccagacggtatccattgaggctagctatcgccatggcagcctcatcatagtttgtcatagtcacaaatccaaaacctttgcatttattggtgttaaagtcacggatgaccttcacattggtgacagctccaaaaggcccaaacatttgccacaggatactctcatctgcgtcaggagccaggttgtacacaaatatacaccaccctgttccagggtgcccagggatattaattccagccaaactggtcattccgtcaatggtcattggagaaaacctgctctttactccataagccatattgagcagattgtccaacctaaaacgctgtgcctgctgagctagcggtcctggataccttctgtttggagactggtacagctgggaaaggatggcctgattggttttttggcttgggttattagcaaactttacagtgattggctccgtggcaccgggaggtttctggccatttaggcctttgatagcttcttctgcctcaattcgcttgtcaaatcgaataaaccctacaccccttgatatgccagtgacctggtcgacaagaatacgagaagtaataatgcgtccatattgtgaaaaaagctgttccaactccttctgggtcattgtttttggaagtccgctgacatataaatttgcatctctgatagaagctgaacttgggcgagcataggaaacttttattgttttggtttgaagtctcaatccattcagggtgttgatagctttctctgcatccttggggtcaatgtagttcacaaagccatatcccaagctctgccctgttattttgtctcttacaagcttacaggactctatttcaccaatgctcccaaagagactctttagttcctcctgtgtcatgttctgaggaaggtagttgactattaagttggtcttgctgtcttctgtgttcccagagtcaactggtgacgaacagttgttgtttatggtggttggaccattggctgtgttattgcaagttggcccattagacagttgtgtttccatggcagcaattacctgcccggtccaaggctctgctgcccacgaaccacttctaagcagagaagccacatcacacagtctgactgccatgttagtttggagttgccgtttcacactttttctgctgcttttggtttaccccagtagaatcccatgaaaacctgcttcacactggcaaagtgggcagacagaggaacaaaggcaattccagggcctgcagaaagtcttcaaaggcaagggaagaaagcaacgccctgcctaaacactggctatttatagcacagcaatggaagatctgggaggtggctgagggaatatgaaagctagagagtgggtgggcgggcttccttctggcttccttagactcagaaactaatgcattcttccctgcctccaaagctgctattttgtttcctgtgtaaggtttcaaaatactgcaacactgtccctaggtgcatttgacaatatcagagcaattacagtttggttaaaatctgaaggtaatcaactcaccattc

SEQ ID NO: 19305 - RNA, 1243 nt, Homo sapiens
  source 1..1243: mol_type = other RNA
tgttcctctgtctcccagacggtatccattgaggctagctatcgccatggcagcctcatcatagtttgtcatagtcacaaatccaaaacctttgcatttattggtgttaaagtcacggatgaccttcacattggtgacagctccaaaaggcccaaacatttgccacaggatactctcatctgcgtcaggagccaggttgtacacaaatatacaccaccctgttccagggtgcccagggatattaattccagccaaactggtcattccgtcaatggtcattggagaaaacctgctctttactccataagccatattgagcagattgtccaacctaaaacgctgtgcctgctgagctagcggtcctggataccttctgtttggagactggtacagctgggaaaggatggcctgattggttttttggcttgggttattagcaaactttacagtgattggctccgtggcaccgggaggtttctggccatttaggcctttgatagcttcttctgcctcaattcgcttgtcaaatcgaataaaccctacaccccttgatatgccagtgacctggtcgacaagaatacgagaagtaataatgcgtccatattgtgaaaaaagctgttccaactccttctgggtcattgtttttggaagtccgctgacatataaatttgcatctctgatagaagctgaacttgggcgagcataggaaacttttattgttttggtttgaagtctcaatccattcagggtgttgatagctttctctgcatccttggggtcaatgtagttcacaaagccatatcccaagctctgccctgttattttgtctcttacaagcttacaggactctatttcaccaatgctcccaaagagactctttagttcctcctgtgtcatgttctgaggaaggtagttgactattaagttggtcttgctgtcttctgtgttcccagagtcaactggtgacgaacagttgttgtttatggtggttggaccattggctgtgttattgcaagttggcccattagacagttgtgtttccatggcagcaattacctgccctttaaaaacagtcctccaagagctctttcctggtaacttagcatgcactatatcatacagccatttgtaaggccccatcaatgactccacctgtatgtggtcatctttatatagaaacccaaccagaatggagacataaaattctagaagagctttagttctttcatcattgtgatctaaa

SEQ ID NO: 19306 - RNA, 1139 nt, Homo sapiens
  source 1..1139: mol_type = other RNA
tgttcctctgtctcccagacggtatccattgaggctagctatcgccatggcagcctcatcatagtttgtcatagtcacaaatccaaaacctttgcatttattggtgttaaagtcacggatgaccttcacattggtgacagctccaaaaggcccaaacatttgccacaggatactctcatctgcgtcaggagccaggttgtacacaaatatacaccaccctgttccagggtgcccagggatattaattccagccaaactggtcattccgtcaatggtcattggagaaaacctgctctttactccataagccatattgagcagattgtccaacctaaaacgctgtgcctgctgagctagcggtcctggataccttctgtttggagactggtacagctgggaaaggatggcctgattggttttttggcttgggttattagcaaactttacagtgattggctccgtggcaccgggaggtttctggccatttaggcctttgatagcttcttctgcctcaattcgcttgtcaaatcgaataaaccctacaccccttgatatgccagtgacctggtcgacaagaatacgagaagtaataatgcgtccatattgtgaaaaaagctgttccaactccttctgggtcattgtttttggaagtccgctgacatataaatttgcatctctgatagaagctgaacttgggcgagcataggaaacttttattgttttggtttgaagtctcaatccattcagggtgttgatagctttctctgcatccttggggtcaatgtagttcacaaagccatatcccaagctctgccctgttattttgtctcttacaagcttacaggactctatttcaccaatgctcccaaagagactctttagttcctcctgtgtcatgttctgaggaaggtagttgactattaagttggtcttgctgtcttctgtgttcccagagtcaactggtgacgaacagttgttgtttatggtggttggaccattggctgtgttattgcaagttggcccattagacagttgtgtttccatggcagcaattacctgcgtctcaacagtttccttcttgcgctacacgcggccgcacccgggcacgtccacgcccgtgcacgctgccaggcgcgact

SEQ ID NO: 19307 - RNA, 1281 nt, Homo sapiens
  source 1..1281: mol_type = other RNA
tgttcctctgtctcccagacggtatccattgaggctagctatcgccatggcagcctcatcatagtttgtcatagtcacaaatccaaaacctttgcatttattggtgttaaagtcacggatgaccttcacattggtgacagctccaaaaggcccaaacatttgccacaggatactctcatctgcgtcaggagccaggttgtacacaaatatacaccaccctgttccagggtgcccagggatattaattccagccaaactggtcattccgtcaatggtcattggagaaaacctgctctttactccataagccatattgagcagattgtccaacctaaaacgctgtgcctgctgagctagcggtcctggataccttctgtttggagactggtacagctgggaaaggatggcctgattggttttttggcttgggttattagcaaactttacagtgattggctccgtggcaccgggaggtttctggccatttaggcctttgatagcttcttctgcctcaattcgcttgtcaaatcgaataaaccctacaccccttgatatgccagtgacctggtcgacaagaatacgagaagtaataatgcgtccatattgtgaaaaaagctgttccaactccttctgggtcattgtttttggaagtccgctgacatataaatttgcatctctgatagaagctgaacttgggcgagcataggaaacttttattgttttggtttgaagtctcaatccattcagggtgttgatagctttctctgcatccttggggtcaatgtagttcacaaagccatatcccaagctctgccctgttattttgtctcttacaagcttacaggactctatttcaccaatgctcccaaagagactctttagttcctcctgtgtcatgttctgaggaaggtagttgactattaagttggtcttgctgtcttctgtgttcccagagtcaactggtgacgaacagttgttgtttatggtggttggaccattggctgtgttattgcaagttggcccattagacagttgtgtttccatggcagcaattacctgctaacgcgcacgaggggatcatcattgctcctgccctgggcgcccgcggccctacaccacctccgcacacaacgcggccggtgttaagtctccaaacgccccgagagctccaaggaccgcgcgcgcgaaggcgccgtagcaagtgggcacacaccagacaccaccccggcgtgttccgcgggagaagccagtgcacacatcctcccgcaaggcggggttgcc

SEQ ID NO: 19308 - RNA, 1426 nt, Homo sapiens
  source 1..1426: mol_type = other RNA
tgttcctctgtctcccagacggtatccattgaggctagctatcgccatggcagcctcatcatagtttgtcatagtcacaaatccaaaacctttgcatttattggtgttaaagtcacggatgaccttcacattggtgacagctccaaaaggcccaaacatttgccacaggatactctcatctgcgtcaggagccaggttgtacacaaatatacaccaccctgttccagggtgcccagggatattaattccagccaaactggtcattccgtcaatggtcattggagaaaacctgctctttactccataagccatattgagcagattgtccaacctaaaacgctgtgcctgctgagctagcggtcctggataccttctgtttggagactggtacagctgggaaaggatggcctgattggttttttggcttgggttattagcaaactttacagtgattggctccgtggcaccgggaggtttctggccatttaggcctttgatagcttcttctgcctcaattcgcttgtcaaatcgaataaaccctacaccccttgatatgccagtgacctggtcgacaagaatacgagaagtaataatgcgtccatattgtgaaaaaagctgttccaactccttctgggtcattgtttttggaagtccgctgacatataaatttgcatctctgatagaagctgaacttgggcgagcataggaaacttttattgttttggtttgaagtctcaatccattcagggtgttgatagctttctctgcatccttggggtcaatgtagttcacaaagccatatcccaagctctgccctgttattttgtctcttacaagcttacaggactctatttcaccaatgctcccaaagagactctttagttcctcctgtgtcatgttctgaggaaggtagttgactattaagttggtcttgctgtcttctgtgttcccagagtcaactggtgacgaacagttgttgtttatggtggttggaccattggctgtgttattgcaagttggcccattagacagttgtgtttccatggcagcaattacctgctgaaattgtaggaggtaagagaaaggaaccgagcagtgggcgacccagtcgccgcaagaacgtgaccgaggttacagcttcaagggcatgatgcaggtttgatgcagcaaggtccgctaagggcgtccagcgctccccgcccccatgcgacgggcggagcggggttggggggaagggaggggactcgtctaacccagggcgggtgtgggagaggcaaatttgccctcttgggcgaagtctaatcagcatagtgaagtagggggctcaaccaaggtcaaaagcgagataggccatcccttaatttgtgcgacccagtctggggacaccggatacagctaactgattctatatcagcatttccgtgtc

SEQ ID NO: 19309 - RNA, 1142 nt, Homo sapiens
  source 1..1142: mol_type = other RNA
tgttcctctgtctcccagacggtatccattgaggctagctatcgccatggcagcctcatcatagtttgtcatagtcacaaatccaaaacctttgcatttattggtgttaaagtcacggatgaccttcacattggtgacagctccaaaaggcccaaacatttgccacaggatactctcatctgcgtcaggagccaggttgtacacaaatatacaccaccctgttccagggtgcccagggatattaattccagccaaactggtcattccgtcaatggtcattggagaaaacctgctctttactccataagccatattgagcagattgtccaacctaaaacgctgtgcctgctgagctagcggtcctggataccttctgtttggagactggtacagctgggaaaggatggcctgattggttttttggcttgggttattagcaaactttacagtgattggctccgtggcaccgggaggtttctggccatttaggcctttgatagcttcttctgcctcaattcgcttgtcaaatcgaataaaccctacaccccttgatatgccagtgacctggtcgacaagaatacgagaagtaataatgcgtccatattgtgaaaaaagctgttccaactccttctgggtcattgtttttggaagtccgctgacatataaatttgcatctctgatagaagctgaacttgggcgagcataggaaacttttattgttttggtttgaagtctcaatccattcagggtgttgatagctttctctgcatccttggggtcaatgtagttcacaaagccatatcccaagctctgccctgttattttgtctcttacaagcttacaggactctatttcaccaatgctcccaaagagactctttagttcctcctgtgtcatgttctgaggaaggtagttgactattaagttggtcttgctgtcttctgtgttcccagagtcaactggtgacgaacagttgttgtttatggtggttggaccattggctgtgttattgcaagttggcccattagacagttgtgtttccatggcagcaattacctgctgcgtctcaacagtttccttcttgcgctacacgcggccgcacccgggcacgtccacgcccgtgcacgctgccaggcgcgact

SEQ ID NO: 19310 - RNA, 1275 nt, Homo sapiens
  source 1..1275: mol_type = other RNA
tgttcctctgtctcccagacggtatccattgaggctagctatcgccatggcagcctcatcatagtttgtcatagtcacaaatccaaaacctttgcatttattggtgttaaagtcacggatgaccttcacattggtgacagctccaaaaggcccaaacatttgccacaggatactctcatctgcgtcaggagccaggttgtacacaaatatacaccaccctgttccagggtgcccagggatattaattccagccaaactggtcattccgtcaatggtcattggagaaaacctgctctttactccataagccatattgagcagattgtccaacctaaaacgctgtgcctgctgagctagcggtcctggataccttctgtttggagactggtacagctgggaaaggatggcctgattggttttttggcttgggttattagcaaactttacagtgattggctccgtggcaccgggaggtttctggccatttaggcctttgatagcttcttctgcctcaattcgcttgtcaaatcgaataaaccctacaccccttgatatgccagtgacctggtcgacaagaatacgagaagtaataatgcgtccatattgtgaaaaaagctgttccaactccttctgggtcattgtttttggaagtccgctgacatataaatttgcatctctgatagaagctgaacttgggcgagcataggaaacttttattgttttggtttgaagtctcaatccattcagggtgttgatagctttctctgcatccttggggtcaatgtagttcacaaagccatatcccaagctctgccctgttattttgtctcttacaagcttacaggactctatttcaccaatgctcccaaagagactctttagttcctcctgtgtcatgttctgaggaaggtagttgactattaagttggtcttgctgtcttctgtgttcccagagtcaactggtgacgaacagttgttgtttatggtggttggaccattggctgtgttattgcaagttggcccattagacagttgtgtttccatggcagcaattacctgctgctgtgactcgaagctgcagctactacggctcgtgccgctggccgtcagcactgccgcggaggagtcgctcggggcgagctccgcggagaggcggtggcggcggcggcggcgggaaaggggactggaagccggcggaacccccgccccacccgcgccgcgccgcgccgcgccggcaaccgccctcctcacccggccggctactgcctcagtgac

SEQ ID NO: 19311 - RNA, 1494 nt, Homo sapiens
  source 1..1494: mol_type = other RNA
tgttcctctgtctcccagacggtatccattgaggctagctatcgccatggcagcctcatcatagtttgtcatagtcacaaatccaaaacctttgcatttattggtgttaaagtcacggatgaccttcacattggtgacagctccaaaaggcccaaacatttgccacaggatactctcatctgcgtcaggagccaggttgtacacaaatatacaccaccctgttccagggtgcccagggatattaattccagccaaactggtcattccgtcaatggtcattggagaaaacctgctctttactccataagccatattgagcagattgtccaacctaaaacgctgtgcctgctgagctagcggtcctggataccttctgtttggagactggtacagctgggaaaggatggcctgattggttttttggcttgggttattagcaaactttacagtgattggctccgtggcaccgggaggtttctggccatttaggcctttgatagcttcttctgcctcaattcgcttgtcaaatcgaataaaccctacaccccttgatatgccagtgacctggtcgacaagaatacgagaagtaataatgcgtccatattgtgaaaaaagctgttccaactccttctgggtcattgtttttggaagtccgctgacatataaatttgcatctctgatagaagctgaacttgggcgagcataggaaacttttattgttttggtttgaagtctcaatccattcagggtgttgatagctttctctgcatccttggggtcaatgtagttcacaaagccatatcccaagctctgccctgttattttgtctcttacaagcttacaggactctatttcaccaatgctcccaaagagactctttagttcctcctgtgtcatgttctgaggaaggtagttgactattaagttggtcttgctgtcttctgtgttcccagagtcaactggtgacgaacagttgttgtttatggtggttggaccattggctgtgttattgcaagttggcccattagacagttgtgtttccatggcagcaattacctgctttctcccttaaggtttttgtgtatgtgtgtttttaaagtaacggtgcagttctcccaataaggatgagcaagaagctgctggatagttctcttaagacagcacgaaacctaaactgtgctcggcttaaaagaagcaaataaaaagaaacgctttcgaccccaaagtccaatgctaaaagaaatggcgaaaaaaaatatgaaaggggaggggaaacttaaaaaagagtttaaaaagacggagagactaccctcctattgccgttcaactaaacaaaaaggggcaagaaaaacaaaccaaggaacaaagaaaagagacgaaagaacgttttttcaaaaagacgatgtctttctccttgttgctttttagtaggtcgctacaggagtaagctgctgcatctctaactaagaacagaaataggggggaggacgtctt

SEQ ID NO: 19312 - RNA, 1457 nt, Homo sapiens
  source 1..1457: mol_type = other RNA
tgttcctctgtctcccagacggtatccattgaggctagctatcgccatggcagcctcatcatagtttgtcatagtcacaaatccaaaacctttgcatttattggtgttaaagtcacggatgaccttcacattggtgacagctccaaaaggcccaaacatttgccacaggatactctcatctgcgtcaggagccaggttgtacacaaatatacaccaccctgttccagggtgcccagggatattaattccagccaaactggtcattccgtcaatggtcattggagaaaacctgctctttactccataagccatattgagcagattgtccaacctaaaacgctgtgcctgctgagctagcggtcctggataccttctgtttggagactggtacagctgggaaaggatggcctgattggttttttggcttgggttattagcaaactttacagtgattggctccgtggcaccgggaggtttctggccatttaggcctttgatagcttcttctgcctcaattcgcttgtcaaatcgaataaaccctacaccccttgatatgccagtgacctggtcgacaagaatacgagaagtaataatgcgtccatattgtgaaaaaagctgttccaactccttctgggtcattgtttttggaagtccgctgacatataaatttgcatctctgatagaagctgaacttgggcgagcataggaaacttttattgttttggtttgaagtctcaatccattcagggtgttgatagctttctctgcatccttggggtcaatgtagttcacaaagccatatcccaagctctgccctgttattttgtctcttacaagcttacaggactctatttcaccaatgctcccaaagagactctttagttcctcctgtgtcatgttctgaggaaggtagttgactattaagttggtcttgctgtcttctgtgttcccagagtcaactggtgacgaacagttgttgtttatggtggttggaccattggctgtgttattgcaagttggcccattagacagttgtgtttccatggcagcaattacctgttcacactttttctgctgcttttggtttaccccagtagaatcccatgaaaacctgcttcacactggcaaagtgggcagacagaggaacaaaggcaattccagggcctgcagaaagtcttcaaaggcaagggaagaaagcaacgccctgcctaaacactggctatttatagcacagcaatggaagatctgggaggtggctgagggaatatgaaagctagagagtgggtgggcgggcttccttctggcttccttagactcagaaactaatgcattcttccctgcctccaaagctgctattttgtttcctgtgtaaggtttcaaaatactgcaacactgtccctaggtgcatttgacaatatcagagcaattacagtttggttaaaatctgaaggtaatca

SEQ ID NO: 19313 - RNA, 1491 nt, Homo sapiens
  source 1..1491: mol_type = other RNA
tgttcctctgtctcccagacggtatccattgaggctagctatcgccatggcagcctcatcatagtttgtcatagtcacaaatccaaaacctttgcatttattggtgttaaagtcacggatgaccttcacattggtgacagctccaaaaggcccaaacatttgccacaggatactctcatctgcgtcaggagccaggttgtacacaaatatacaccaccctgttccagggtgcccagggatattaattccagccaaactggtcattccgtcaatggtcattggagaaaacctgctctttactccataagccatattgagcagattgtccaacctaaaacgctgtgcctgctgagctagcggtcctggataccttctgtttggagactggtacagctgggaaaggatggcctgattggttttttggcttgggttattagcaaactttacagtgattggctccgtggcaccgggaggtttctggccatttaggcctttgatagcttcttctgcctcaattcgcttgtcaaatcgaataaaccctacaccccttgatatgccagtgacctggtcgacaagaatacgagaagtaataatgcgtccatattgtgaaaaaagctgttccaactccttctgggtcattgtttttggaagtccgctgacatataaatttgcatctctgatagaagctgaacttgggcgagcataggaaacttttattgttttggtttgaagtctcaatccattcagggtgttgatagctttctctgcatccttggggtcaatgtagttcacaaagccatatcccaagctctgccctgttattttgtctcttacaagcttacaggactctatttcaccaatgctcccaaagagactctttagttcctcctgtgtcatgttctgaggaaggtagttgactattaagttggtcttgctgtcttctgtgttcccagagtcaactggtgacgaacagttgttgtttatggtggttggaccattggctgtgttattgcaagttggcccattagacagttgtgtttccatggcagcaattacctttctcccttaaggtttttgtgtatgtgtgtttttaaagtaacggtgcagttctcccaataaggatgagcaagaagctgctggatagttctcttaagacagcacgaaacctaaactgtgctcggcttaaaagaagcaaataaaaagaaacgctttcgaccccaaagtccaatgctaaaagaaatggcgaaaaaaaatatgaaaggggaggggaaacttaaaaaagagtttaaaaagacggagagactaccctcctattgccgttcaactaaacaaaaaggggcaagaaaaacaaaccaaggaacaaagaaaagagacgaaagaacgttttttcaaaaagacgatgtctttctccttgttgctttttagtaggtcgctacaggagtaagctgctgcatctctaactaagaacagaaataggggggaggacgtctt

SEQ ID NO: 19314 - RNA, 1454 nt, Homo sapiens
  source 1..1454: mol_type = other RNA
tgttcctctgtctcccagacggtatccattgaggctagctatcgccatggcagcctcatcatagtttgtcatagtcacaaatccaaaacctttgcatttattggtgttaaagtcacggatgaccttcacattggtgacagctccaaaaggcccaaacatttgccacaggatactctcatctgcgtcaggagccaggttgtacacaaatatacaccaccctgttccagggtgcccagggatattaattccagccaaactggtcattccgtcaatggtcattggagaaaacctgctctttactccataagccatattgagcagattgtccaacctaaaacgctgtgcctgctgagctagcggtcctggataccttctgtttggagactggtacagctgggaaaggatggcctgattggttttttggcttgggttattagcaaactttacagtgattggctccgtggcaccgggaggtttctggccatttaggcctttgatagcttcttctgcctcaattcgcttgtcaaatcgaataaaccctacaccccttgatatgccagtgacctggtcgacaagaatacgagaagtaataatgcgtccatattgtgaaaaaagctgttccaactccttctgggtcattgtttttggaagtccgctgacatataaatttgcatctctgatagaagctgaacttgggcgagcataggaaacttttattgttttggtttgaagtctcaatccattcagggtgttgatagctttctctgcatccttggggtcaatgtagttcacaaagccatatcccaagctctgccctgttattttgtctcttacaagcttacaggactctatttcaccaatgctcccaaagagactctttagttcctcctgtgtcatgttctgaggaaggtagttgactattaagttggtcttgctgtcttctgtgttcccagagtcaactggtgacgaacagttgttgtttatggtggttggaccattggctgtgttattgcaagttggcccattagacagttgtgtttccatggcagcaattacttcacactttttctgctgcttttggtttaccccagtagaatcccatgaaaacctgcttcacactggcaaagtgggcagacagaggaacaaaggcaattccagggcctgcagaaagtcttcaaaggcaagggaagaaagcaacgccctgcctaaacactggctatttatagcacagcaatggaagatctgggaggtggctgagggaatatgaaagctagagagtgggtgggcgggcttccttctggcttccttagactcagaaactaatgcattcttccctgcctccaaagctgctattttgtttcctgtgtaaggtttcaaaatactgcaacactgtccctaggtgcatttgacaatatcagagcaattacagtttggttaaaatctgaaggtaatca

SEQ ID NO: 19315 - RNA, 935 nt, Homo sapiens
  source 1..935: mol_type = other RNA
tgttcctctgtctcccagacggtatccattgaggctagctatcgccatggcagcctcatcatagtttgtcatagtcacaaatccaaaacctttgcatttattggtgttaaagtcacggatgaccttcacattggtgacagctccaaaaggcccaaacatttgccacaggatactctcatctgcgtcaggagccaggttgtacacaaatatacaccaccctgttccagggtgcccagggatattaattccagccaaactggtcattccgtcaatggtcattggagaaaacctgctctttactccataagccatattgagcagattgtccaacctaaaacgctgtgcctgctgagctagcggtcctggataccttctgtttggagactggtacagctgggaaaggatggcctgattggttttttggcttgggttattagcaaactttacagtgattggctccgtggcaccgggaggtttctggccatttaggcctttgatagcttcttctgcctcaattcgcttgtcaaatcgaataaaccctacaccccttgatatgccagtgacctggtcgacaagaatacgagaagtaataatgcgtccatattgtgaaaaaagctgttccaactccttctgggtcattgtttttggaagtccgctgacatataaatttgcatctctgatagaagctgaacttgggcgagcataggaaacttttattgttttggtttgaagtctcaatccattcagggtgttgatagctttctctgcatccttggggtcaatgtagttcacaaagccatatcccaagctctgcccttttagctacatggtattttactgtttaattgtagcttcacattaaccatgttcggtattcagattcttctcctacaaggtagaaatgatatctgaagcttggcaaggtcaatcagctt

SEQ ID NO: 19316 - RNA, 1545 nt, Homo sapiens
  source 1..1545: mol_type = other RNA
tgttcctctgtctcccagacgtacaagtaaaatctgttggttccatccatcagcagggtgtccgggaggttgtgcccctctgtgaaggtgatgaccacggggatgatgcccactgcagcaagctccagtgtggctgtattgatggaagctgcatcataggcccagcccgcctggaagaacacagccaccttcctcatgagaagacccgagcgtacacgtttgaacacgtctcgccataaacctcatggtggccccgaggttcctgcggccagatgactgctccagggggatgttcctgacagcctccaggagtgcaaccttccccttgtagtctgagaaacgaaccaagtaattggttttggcattgtaggaaacaatggccacatgggcacctgttgggcagttactgtcacttatttccatcttcatcaacagagacaataaaatgtctctcatcctctcaaaatccaacagggagacatcatttgacatgtccaaggcaaaggccacttcagttgggaatgctgggcatttggaaatacctcttgaacaaactcctttgttttgtgataagaagcagcaagatgtaggcacacaggtgtgcagttatgacatctcctggggcacagtattgctcagtggagcttctcttcatcgttgagatggcatgctgtcaatccactttatttggcagttttcacgtgtgaaatcaacaattttgcaaggcatttgtcctggtgggccttggtcacccgaagttccaacaaatccaggaaagccagcattacccctcttccctcttattccctttgcccccttttctccttgatggcccgggtcaccatcttctccttgtgcaccaggatagccagggaatccatgttcaccctttgttccttttgttcctggatgtccttatccatcagaaccaggaagaccaggttgccctcttggtccttgtcgactctgtgggcctctttctcctacatcaccaatctctcccttcactcctcttggtccagcttttccttttgaaccatttggccctggaggcccaggattcccctgagcacccactaagcctttttgtccagaagttcctggtggtccttgccttcctcttggtccctttaatcctggcagacctcgccttcctattgtcccccaagggccgacatttccagtttctccctgaggtccatcaacattagaacttccctgacgcccacgccttcctttttctcccttagggccttggatatagctattagttccaggatccccaggatctccccttaacccaggctctccacgctctccaggttgtcctggcagtcccgtcaagccccgatttcccctatttcctttttctccagatgaccctgggattccgtgattaccctgttctccatgcaagccatcaactccctcaccagggttgcccttctctcctgaaaatcctcttgctcccttaggtcccctcataccagggcatccttcctcacctcggagtccaggaagacctcaggggcctcgttctccctg

SEQ ID NO: 19317 - RNA, 24 nt, Homo sapiens
  source 1..24: mol_type = other RNA
tgttcctctgtctcccagactgga

SEQ ID NO: 19318 - RNA, 2237 nt, Homo sapiens
  source 1..2237: mol_type = other RNA
tgttctctttgccaaggacaggatgggtgtgaaaggacctcaggcttgtgacggaaggaagtaataagctcgattggaaattctattacattaagaaaaggcagccatggaaataaagctaaataatcctactgagctcagcaagataaatatatatgtattttatccgtgttgaaaatagaggaaggagaaagaatggaagacaacttgtatagtttgttatctctaaagcatctacatcttgttgcttgggagggtctccagtagatgtgccagctggggcttcaagatcagaatttgcatttaggaagttcactttcatggggtttatccatctgtgttaaaatggtagctgttcttgagggtgaggtggactcccacaggtaggtctcggcggtgcccttccatgctgtcttcattagctctggttcccttgaaactttgtggccaagaatcaggtgaaatctttcttgatgactcaggtgggcagtgttcaggatgagctgtggtgggaggaacttcatggattgactacactttgaggtcagcatggttgggttatcaaattgcagaatcagcagctttatccttttgattcaccaggagcaatcacacattgtagagtcacacaatcctgtttcttctgcttgggcacatagggagactatattccacagcctcacttgcagttaggtgaaacaatgtgattgagttctacccaggtgaatgtgggcagaagtgatatatgccacttgtagatatacccaaaaaatgtctcaggtgctggaagtgaaggacttcgcaatggaggagaaacacagtagaaggatcctggatacataagtcaccacatggaagacagccaccaggagagatgcctgactcacattggacataaatgaaatcccaagttctgatagtggtttccatgatctgtgcccctgcttcatgagaagaggaacttagtctgttttgttctgttttgtttaatgctgtgttcccagcaagaatgctgcctggcacacattaggattgactaaatatttattgaatgatggacatagaggtagagactctgctttatgtcatccttcaggttctagcttaaatgtctcttctcagagaaaccatccctgaccactatctaaagtaggcagcctctacctggtaattctccttcatagagtcctcttgttttcctttgcagcacttatcaatgatctgtaatcacatattggtttcttgccatttattcaatgttacctatcttcccagagtgtaagccccttgaggtcaggaccatgtctattttgtcacaatgggatgcctagtgcttgacttcagtagacactccatagtagacgctgcataggtattcggtggatacgagagtgaaacagtgaatgaaggaaggtggacctgggccaaggagctgggcggccaaggtcaggtttatgccatcagccccactcaggacaaatgtcccgactcctgctcggagccctcttcctactactctgtgcttcccacagctgttgatcatctcactgacaagcaggctcagccaagaaagtggaaagaggaaaagaaaaatgaggcacaggagggtagaatggaaaatctcagctcttttagcagccactcttccttatttcttgctagagtattggcacctttaaaagccttggctgtcctccccaacctccccactcaatcacaaaccgcagcacctagaaaaaaataaaggcaaaaatcaatgtgctaaatctcagttgggctcagtagcaactccctgcagcttccctctgcaagccatggaactgagctctccagccctctccctgaacttgactgcagggttggggaacttgcatgctaaaaatatgccctctccccttcggcaacccattcccaacctggtgaagaccaaggaggaagcttctgagattctcctccttgccttccatttgcagctcagattctctgtccaatgacttcatctaccctctcctgctgtccactctctgctccctttcttctcagccctcacttggtctctgccctacttacccagccagtggcctctaaagttttccattcagaatttccctctttaccttctcttttagatatgtagaaagtgaaagggaaaaggggattgttatctgggtacagacggttgagttgggaagagaatcatattttgattattaaaatattaaaatgatacagtttca

SEQ ID NO: 19319 - RNA, 2146 nt, Homo sapiens
  source 1..2146: mol_type = other RNA
tgttctctttgccaaggacaggatgggtgtgaaaggacctcaggcttgtgacggaaggaagtaataagctcgattggaaattctattacattaagaaaaggcagccatggaaataaagctaaataatcctactgagctcagcaagataaatatatatgtattttatccgtgttgaaaatagaggaaggagaaagaatggaagacaacttgtatagtttgttatctctaaagcatctacatcttgttgcttgggagggtctccagtagatgtgccagctggggcttcaagatcagaatttgcatttaggaagttcactttcatggggtttatccatctgtgttaaaatggtagctgttcttgagggtgaggtggactcccacaggtaggtctcggcggtgcccttccatgctgtcttcattagctctggttcccttgaaactttgtggccaagaatcaggtgaaatctttcttgatgactcaggtgggcagtgttcaggatgagctgtggtgggaggaacttcatggattgactacactttgaggtcagcatggttgggttatcaaattgcagaatcagcagctttatccttttgattcaccaggagcaatcacacattgtagagtcacacaatcctgtttcttctgcttgggcacatagggagactatattccacagcctcacttgcagttaggtgaaacaatgtgattgagttctacccaggtgaatgtgggcagaagtgatatatgccacttgtagatatacccaaaaaatgtctcaggtgctggaagtgaaggacttcgcaatggaggagaaacacagtagaaggatcctggatacataagtcaccacatggaagacagccaccaggagagatgcctgactcacattggacataaatgaaatcccaagttctgatagtggtttccatgatctgtgcccctgcttcatgagaagaggaacttagtctgttttgttctgttttgtttaatgctgtgttcccagcaagaatgctgcctggcacacattaggattgactaaatatttattgaatgatggacatagaggtagagactggtaattctccttcatagagtcctcttgttttcctttgcagcacttatcaatgatctgtaatcacatattggtttcttgccatttattcaatgttacctatcttcccagagtgtaagccccttgaggtcaggaccatgtctattttgtcacaatgggatgcctagtgcttgacttcagtagacactccatagtagacgctgcataggtattcggtggatacgagagtgaaacagtgaatgaaggaaggtggacctgggccaaggagctgggcggccaaggtcaggtttatgccatcagccccactcaggacaaatgtcccgactcctgctcggagccctcttcctactactctgtgcttcccacagctgttgatcatctcactgacaagcaggctcagccaagaaagtggaaagaggaaaagaaaaatgaggcacaggagggtagaatggaaaatctcagctcttttagcagccactcttccttatttcttgctagagtattggcacctttaaaagccttggctgtcctccccaacctccccactcaatcacaaaccgcagcacctagaaaaaaataaaggcaaaaatcaatgtgctaaatctcagttgggctcagtagcaactccctgcagcttccctctgcaagccatggaactgagctctccagccctctccctgaacttgactgcagggttggggaacttgcatgctaaaaatatgccctctccccttcggcaacccattcccaacctggtgaagaccaaggaggaagcttctgagattctcctccttgccttccatttgcagctcagattctctgtccaatgacttcatctaccctctcctgctgtccactctctgctccctttcttctcagccctcacttggtctctgccctacttacccagccagtggcctctaaagttttccattcagaatttccctctttaccttctcttttagatatgtagaaagtgaaagggaaaaggggattgttatctgggtacagacggttgagttgggaagagaatcatattttgattattaaaatattaaaatgatacagtttca

SEQ ID NO: 19320 - RNA, 1976 nt, Homo sapiens
  source 1..1976: mol_type = other RNA
tgttctctttgccaaggacaggatgggtgtgaaaggacctcaggcttgtgacggaaggaagtaataagctcgattggaaattctattacattaagaaaaggcagccatggaaataaagctaaataatcctactgagctcagcaagataaatatatatgtattttatccgtgttgaaaatagaggaaggagaaagaatggaagacaacttgtatagtttgttatctctaaagcatctacatcttgttgcttgggagggtctccagtagatgtgccagctggggcttcaagatcagaatttgcatttaggaagttcactttcatggggtttatccatctgtgttaaaatggtagctgttcttgagggtgaggtggactcccacaggtaggtctcggcggtgcccttccatgctgtcttcattagctctggttcccttgaaactttgtggccaagaatcaggtgaaatctttcttgatgactcaggtgggcagtgttcaggatgagctgtggtgggaggaacttcatggattgactacactttgaggtcagcatggttgggttatcaaattgcagaatcagcagctttatccttttgattcaccaggagcaatcacacattgtagagtcacacaatcctgtttcttctgcttgggcacatagggagactatattccacagcctcacttgcagttaggtgaaacaatgtgattgagttctacccaggtgaatgtgggcagaagtgatatatgccacttgtagatatacccaaaaaatgtctcaggtgctggaagtgaaggacttcgcaatggaggagaaacacagtagaaggatcctggatacataagtcaccacatggaagacagccaccaggagagatgcctgactcacattggacattttagaggccagaagtcaggaatcaaggtatctgcaaggccaggctccctctgatacctgcacaggagaatactcgcccccatcaagcctctggtgtttgctggcagtgcttggcatccctcagctgatcgatgcgtcagtcccacttctgcctccatggtcagcaggcatcctcccctcgtgtgtctgtgtctccatgtggtattctcctgcccatgtgtctttctccctgcctctgctttgtagttacaggcaaacaggggctgggaaggtgaagagtggatgtctgaacaaaatttaattcctgttaggaaagaagaaaggggcaatggatgttaggtaaggagataaaatgtacaatacactttaatgatacaacataacagttacgaaagaagctaagaatggtgaagggggctccacttacctttggtttatttattccaccagtcttccttccttcctttttgttttacacctgtaagcttcagactctagagtggtgggttcaccaaccactccaaatcctacccctgcaatggattttattataccaccaggttgagtgaagctgaccaacttcaggggcttcagggaggtggtaaaggcagggaggggataactgagaggtgagagtcacacagtgcccactttctaggtaatcaattgacagcaattcagcatgccatcattgctgttctagctgtatgtagttgatgtacacaactgagagggaggttgcaagtatgagaattttttatacacatataaaaaattatatatctctatatatcttgtcaatgagcaaaaaattgaaatgtgagactaccttaaaccttgattctttctctcgtcttatgttcttgaacactcttccacagtagggggcaatctgactggagagtgaaatactctttcttgttgaatgaccatggcactcctgtcttagtttcttctcaccctatttctaggccaaggtcatttccctgtaacatccttaataacggattctgagcccagaccaggcacggtggctcatgcctgtaatcccagcactttgggaggctgagacaggcggat

SEQ ID NO: 19321 - RNA, 1365 nt, Homo sapiens
  source 1..1365: mol_type = other RNA
tgttctctttgccaaggacaggatgggtgtgaaaggacctcaggcttgtgacggaaggaagtaataagctcgattggaaattctattacattaagaaaaggcagccatggaaataaagctaaataatcctactgagctcagcaagataaatatatatgtattttatccgtgttgaaaatagaggaaggagaaagaatggaagacaacttgtatagtttgttatctctaaagcatctacatcttgttgcttgggagggtctccagtagatgtgccagctggggcttcaagatcagaatttgcatttaggaagttcactttcatggggtttatccatctgtgttaaaatggtagctgttcttgagggtgaggtggactcccacaggtaggtctcggcggtgcccttccatgctgtcttcattagctctggttcccttgaaactttgtggccaagaatcaggtgaaatctttcttgatgactcaggtgggcagtgttcaggatgagctgtggtgggaggaacttcatggattgactacactttgaggtcagcatggttgggttatcaaattgcagaatcagcagctttatccttttgattcaccaggagcaatcacacattgtagagtcacacaatcctgtttcttctgcttgggcacatagggagactatattccacagcctcacttgcagttaggtgaaacaatgtgattgagttctacccaggtgaatgtgggcagaagtgatatatgccacttgtagatatacccaaaaaatgtctcaggtgctggaagtgaaggacttcgcaatggaggagaaacacagtagaaggatcctggatacataagtcaccacatggaagacagccaccaggagagatgcctgactcacattggacattttagaggccagaagtcaggaatcaaggtatctgcaaggccaggctccctctgatacctgcacaggagaatactcgcccccatcaagcctctggtgtttgctggcagtgcttggcatccctcagctgatcgatgcgtcagtcccacttctgcctccatggtcagcaggcatcctcccctcgtgtgtctgtgtctccatgtggtattctcctgcccatgtgtctttctccctgcctctgctttgtagttacaggcaaacaggggctgggaaggtgaagagtggatgtctgaacaaaatttaattccttggcaggcttcccatcaaatattgttgcgcaaaggatggatggatgaaaggaagagtgagccaataaacgagggaacgccgggaaaggcagcctcaagccggtgggccctgccacccccaccgtccctgagcatccgagccggttcccgcccccggcccgaac

SEQ ID NO: 19322 - RNA, 1467 nt, Homo sapiens
  source 1..1467: mol_type = other RNA
tgttctctttgccaaggacaggatgggtgtgaaaggacctcaggcttgtgacggaaggaagtaataagctcgattggaaattctattacattaagaaaaggcagccatggaaataaagctaaataatcctactgagctcagcaagataaatatatatgtattttatccgtgttgaaaatagaggaaggagaaagaatggaagacaacttgtatagtttgttatctctaaagcatctacatcttgttgcttgggagggtctccagtagatgtgccagctggggcttcaagatcagaatttgcatttaggaagttcactttcatggggtttatccatctgtgttaaaatggtagctgttcttgagggtgaggtggactcccacaggtaggtctcggcggtgcccttccatgctgtcttcattagctctggttcccttgaaactttgtggccaagaatcaggtgaaatctttcttgatgactcaggtgggcagtgttcaggatgagctgtggtgggaggaacttcatggattgactacactttgaggtcagcatggttgggttatcaaattgcagaatcagcagctttatccttttgattcaccaggagcaatcacacattgtagagtcacacaatcctgtttcttctgcttgggcacatagggagactatattccacagcctcacttgcagttaggtgaaacaatgtgattgagttctacccaggtgaatgtgggcagaagtgatatatgccacttgtagatatacccaaaaaatgtctcaggtgctggaagtgaaggacttcgcaatggaggagaaacacagtagaaggatcctggatacataagtcaccacatggaagacagccaccaggagagatgcctgactcacattggacattttagaggccagaagtcaggaatcaaggtatctgcaaggccaggctccctctgatacctgcacaggagaatactcgcccccatcaagcctctggtgtttgctggcagtgcttggcatccctcagctgatcgatgcgtcagtcccacttctgcctccatggtcagcaggcatcctcccctcgtgtgtctgtgtctccatgtggtattctcctgcccatgtgtctttctccctgcctctggaaccagaagacctgggttcaagtcattgccttgctgtttattagctgtgtggcctccagaagtcacttgatttctttgacctcgatgaccaatctgtgaactcagggcaattctagtcttttccatttacgatgttcttgtgagaatcaaatggagtaatctgaaaacttggcaggcttcccatcaaatattgttgcgcaaaggatggatggatgaaaggaagagtgagccaataaacgagggaacgccgggaaaggcagcctcaagccggtgggccctgccacccccaccgtccctgagcatccgagccggttcccgcccccggcccgaac

SEQ ID NO: 19323 - RNA, 1296 nt, Homo sapiens
  source 1..1296: mol_type = other RNA
tgttctctttgccaaggacaggatgggtgtgaaaggacctcaggcttgtgacggaaggaagtaataagctcgattggaaattctattacattaagaaaaggcagccatggaaataaagctaaataatcctactgagctcagcaagataaatatatatgtattttatccgtgttgaaaatagaggaaggagaaagaatggaagacaacttgtatagtttgttatctctaaagcatctacatcttgttgcttgggagggtctccagtagatgtgccagctggggcttcaagatcagaatttgcatttaggaagttcactttcatggggtttatccatctgtgttaaaatggtagctgttcttgagggtgaggtggactcccacaggtaggtctcggcggtgcccttccatgctgtcttcattagctctggttcccttgaaactttgtggccaagaatcaggtgaaatctttcttgatgactcaggtgggcagtgttcaggatgagctgtggtgggaggaacttcatggattgactacactttgaggtcagcatggttgggttatcaaattgcagaatcagcagctttatccttttgattcaccaggagcaatcacacattgtagagtcacacaatcctgtttcttctgcttgggcacatagggagactatattccacagcctcacttgcagttaggtgaaacaatgtgattgagttctacccaggtgaatgtgggcagaagtgatatatgccacttgtagatatacccaaaaaatgtctcaggtgctggaagtgaaggacttcgcaatggaggagaaacacagtagaaggatcctggatacataagtcaccacatggaagacagccaccaggagagatgcctgactcacattggacattttagaggccagaagtcaggaatcaaggtatctgcaaggccaggctccctctgatacctgcacaggagaatactcgcccccatcaagcctctggtgtttgctggcagtgcttggcatccctcagctgatcgatgcgtcagtcccacttctgcctccatggtcagcaggcatcctcccctcgtgtgtctgtgtctccatgtggtattctcctgcccatgtgtctttctccctgcctcttggcaggcttcccatcaaatattgttgcgcaaaggatggatggatgaaaggaagagtgagccaataaacgagggaacgccgggaaaggcagcctcaagccggtgggccctgccacccccaccgtccctgagcatccgagccggttcccgcccccggcccgaac

SEQ ID NO: 19324 - RNA, 2057 nt, Homo sapiens
  source 1..2057: mol_type = other RNA
tgttctctttgccaaggacaggatgggtgtgaaaggacctcaggcttgtgacggaaggaagtaataagctcgattggaaattctattacattaagaaaaggcagccatggaaataaagctaaataatcctactgagctcagcaagataaatatatatgtattttatccgtgttgaaaatagaggaaggagaaagaatggaagacaacttgtatagtttgttatctctaaagcatctacatcttgttgcttgggagggtctccagtagatgtgccagctggggcttcaagatcagaatttgcatttaggaagttcactttcatggggtttatccatctgtgttaaaatggtagctgttcttgagggtgaggtggactcccacaggtaggtctcggcggtgcccttccatgctgtcttcattagctctggttcccttgaaactttgtggccaagaatcaggtgaaatctttcttgatgactcaggtgggcagtgttcaggatgagctgtggtgggaggaacttcatggattgactacactttgaggtcagcatggttgggttatcaaattgcagaatcagcagctttatccttttgattcaccaggagcaatcacacattgtagagtcacacaatcctgtttcttctgcttgggcacatagggagactatattccacagcctcacttgcagttaggtgaaacaatgtgattgagttctacccaggtgaatgtgggcagaagtgatatatgccacttgtagatatacccaaaaaatgtctcaggtgctggaagtgaaggacttcgcaatggaggagaaacacagtagaaggatcctggatacataagtcaccacatggaagacagccaccaggagagatgcctgactcacattggactctgctttatgtcatccttcaggttctagcttaaatgtctcttctcagagaaaccatccctgaccactatctaaagtaggcagcctctacctggtaattctccttcatagagtcctcttgttttcctttgcagcacttatcaatgatctgtaatcacatattggtttcttgccatttattcaatgttacctatcttcccagagtgtaagccccttgaggtcaggaccatgtctattttgtcacaatgggatgcctagtgcttgacttcagtagacactccatagtagacgctgcataggtattcggtggatacgagagtgaaacagtgaatgaaggaaggtggacctgggccaaggagctgggcggccaaggtcaggtttatgccatcagccccactcaggacaaatgtcccgactcctgctcggagccctcttcctactactctgtgcttcccacagctgttgatcatctcactgacaagcaggctcagccaagaaagtggaaagaggaaaagaaaaatgaggcacaggagggtagaatggaaaatctcagctcttttagcagccactcttccttatttcttgctagagtattggcacctttaaaagccttggctgtcctccccaacctccccactcaatcacaaaccgcagcacctagaaaaaaataaaggcaaaaatcaatgtgctaaatctcagttgggctcagtagcaactccctgcagcttccctctgcaagccatggaactgagctctccagccctctccctgaacttgactgcagggttggggaacttgcatgctaaaaatatgccctctccccttcggcaacccattcccaacctggtgaagaccaaggaggaagcttctgagattctcctccttgccttccatttgcagctcagattctctgtccaatgacttcatctaccctctcctgctgtccactctctgctccctttcttctcagccctcacttggtctctgccctacttacccagccagtggcctctaaagttttccattcagaatttccctctttaccttctcttttagatatgtagaaagtgaaagggaaaaggggattgttatctgggtacagacggttgagttgggaagagaatcatattttgattattaaaatattaaaatgatacagtttca

SEQ ID NO: 19325 - RNA, 3279 nt, Homo sapiens
  source 1..3279: mol_type = other RNA
tgttgggattcagcaggaccatgcccctccctgcggggctccagctagatgcaggctgggcttcccttcagcccacctcatcctctgcccatgattccctcaagccagcccaggattgcccatctttctcatccaagataattcatcctagtgtctcagatgttgtgtcaaacttataatctctggccccatcccagctctcacaacacccctgtgtcacatgaagctcttcatctgctgagtttagtagtacgtctccctttccacccagccatccgggtgctgacggatgaggagttttctgatttcatcatagacgaagatgagaatactgtagggaatggcacagagccaccaggttatcttgagtgggtacattcgcagggccacgtccatgcctggagtgtaggacagaaatgcagccaagagtgtctcctccaggatcccaaatattaagactttgtttctcatgccctgctggaaaagtgagttgcggcgagtcttggagatgatgagatccgcccactgcacaaccacgatggtgacaaaaaaggccgtttggcatgtgaactccacaacttttcgttgctcataggtccactgctgtccgtagctgtcctccaggtcattcaagtatttatcttcccagtggaggcggatgcccagcagatcaacaggcctaaaaccattctcagccaggattacaaagtaggtaaagaatccagccagagcctggatcatcccaatctgtccataggccatgccaatgagacggtggttcaccagattatccgtctttgggttccttggaagcctcttcatgatgtcgctttcagctgactcataagccaaggagatggcagggaccatgtcagtgccgagatcaatgcagaggatggttatggttcccagaggcaggggtataccgaggatgatgaacatcaggaagggcgtgatctcggggatgttgctggtcagggtgtacatgatggatttcttcaggttgtcaaagatcaggcggccctcctccacccccgtgacgatggaggcaaagttgtcatccagcaggatcatgtcggctgcctgcttagagacgtcagagccagagatgcccatggcaatgccaatgtcagccttcttcagcgcaggggagtcgttcaccccgtcacctgtcacggccacaacggctcccagcctctgacatccctcgacaatgatgagcttctgctgaggggaggtccgagcaaacacgatctcagggtggttctggaggatctgatcaagctgcttggactgtatgtccttcagttctgcaccatgcaccacaatggctttggcagcactggcatcgaccttgctgatagggatcttaagccgggcagcgacttcctctgccgtctcagtgccttctgagatgatgcccacacccttggcaatggccttagctgtaatgggatgatctcctgttaccatgatcaccttaattcctgcactgcgacacttgctcacagcatcaggcactgcagctcggggagggtcaatcatggatatgaggcccacaaaacaaaggttgtccatggggaaatttatttcatctgtattaaatgggaatcccttggagaagctgctaggcagattcaagaagcagaagcctagcacacgttcccccagacctcccagttctaagtaggcattttggaaggcttccttcatttcatcgttcattgagtactcctgcccattcagaagaaaggtagaacaaaactccaagatcctctccggagcacccttcatcatcagtacgtgggtctgggagctgtcctcccgaaggtggatggacatctggtacttgttggtagaattaaagggaatctctgccaccttggggtttttctctctcatctccgccacagagctgtaagactgctcgatgaacttgaggagggctgactcggaagcatcacctgttgtggccctcttagcaatgggcaggatctcctgattagccttaaagtcagcccggttgcagaggccagcgattcgggccagcataaaccaggtatcagagctcttggtaaatgtttttccagtctgttcttcagtggtgtcggcctcatacacggtcatatcaaaccacatgtgggcgacggtcatgcggttctgggtgagggtgcccgtcttgtctgagcagatggtggacgtggagcccagcgtctccaccgcctccaggttcttcaccaggcagttcttccgcgccatgcgcttggctgtgagggtcaggcacacagtgactgtggccaacagcccctcaggcacattggccacaatgatgccaatgagaaaaatgatagcctccagccaaccatagcccaagagaagtgagagcgcaaaaaaagtgacaccaaggaagacggccaccacagtgatcagatggatgaagtgttcgatctcagcagcgataggtgtctggccaaccgccaggcctgacgtcagggaggcaattctgcccatcactgtggagtctcccgtagcaatcacaataccccgggcggttccttccacacagttggtggaaaagaagcagatgtttcgggtctccagagggttctcatgggtgaagtcaggggagcggctctggggttctgactccccagtcaaggatgagttgtccaccttacatccttgtgcagagataagccggaggtcagcagggactcggtctccacccttgatttccaccaggtctcccaacaccacctcttgtacattaatttgcatcttctctcctcctcgaattaccagagcttgctgaggcaccatgttcttaaaagactccatgatcttggagctcttggcctcctgataataggagaagcagccagtgacgatgaccacgacggacagtacgatgctcaggtagaggttgtctttggtaggctcctcattgaaatatatctggatgctgtaggccacaaagcagagaatggccccagtccatagtaggagggagaagcctccgaacagttgcttacagaatttgacccattctggagtggtggggggtggggtaacagtattgggtccacctcgagtcaggatttcctttgccctttggtggctatggcccatttgcagctttttccaggtagtgtccatggaacgtggccaggcagagggtgaggggtgggaacgttggacttgaagttagggggctggattcctagttcagcttttgtcctggcagcctcacagtcagagttggagactctctgcctcctc

SEQ ID NO: 19326 - RNA, 3771 nt, Homo sapiens
  source 1..3771: mol_type = other RNA
tgttgggattcagcaggaccatgcccctccctgcggggctccagctagatgcaggctgggcttcccttcagcccacctcatcctctgcccatgattccctcaagccagcccaggattgcccatctttctcatccaagataattcatcctagtgtctcagatgttgtgtcaaacttataatctctggccccatcccagctctcacaacacccctgtgtcacatgaagctcttcatctgctgagtttagtagtacgtctccctttccacccagccatccgggtgctgacggatgaggagttttctgatttcatcatagacgaagatgagaatactgtagggaatggcacagagccaccaggttatcttgagtgggtacattcgcagggccacgtccatgcctggagtgtaggacagaaatgcagccaagagtgtctcctccaggatcccaaatattaagactttgtttctcatgccctgctggaaaagtgagttgcggcgagtcttggagatgatgagatccgcccactgcacaaccacgatggtgacaaaaaaggccgtttggcatgtgaactccacaacttttcgttgctcataggtccactgctgtccgtagctgtcctccaggtcattcaagtatttatcttcccagtggaggcggatgcccagcagatcaacaggcctaaaaccattctcagccaggattacaaagtaggtaaagaatccagccagagcctggatcatcccaatctgtccataggccatgccaatgagacggtggttcaccagattatccgtctttgggttccttggaagcctcttcatgatgtcgctttcagctgactcataagccaaggagatggcagggaccatgtcagtgccgagatcaatgcagaggatggttatggttcccagaggcaggggtataccgaggatgatgaacatcaggaagggcgtgatctcggggatgttgctggtcagggtgtacatgatggatttcttcaggttgtcaaagatcaggcggccctcctccacccccgtgacgatggaggcaaagttgtcatccagcaggatcatgtcggctgcctgcttagagacgtcagagccagagatgcccatggcaatgccaatgtcagccttcttcagcgcaggggagtcgttcaccccgtcacctgtcacggccacaacggctcccagcctctgacatccctcgacaatgatgagcttctgctgaggggaggtccgagcaaacacgatctcagggtggttctggaggatctgatcaagctgcttggactgtatgtccttcagttctgcaccatgcaccacaatggctttggcagcactggcatcgaccttgctgatagggatcttaagccgggcagcgacttcctctgccgtctcagtgccttctgagatgatgcccacacccttggcaatggccttagctgtaatgggatgatctcctgttaccatgatcaccttaattcctgcactgcgacacttgctcacagcatcaggcactgcagctcggggagggtcaatcatggatatgaggcccacaaaacaaaggttgtccatggggaaatttatttcatctgtattaaatgggaatcccttggagaagctgctaggcagattcaagaagcagaagcctagcacacgttcccccagacctcccagttctaagtaggcattttggaaggcttccttcatttcatcgttcattgagtactcctgcccattcagaagaaaggtagaacaaaactccaagatcctctccggagcacccttcatcatcagtacgtgggtctgggagctgtcctcccgaaggtggatggacatctggtacttgttggtagaattaaagggaatctctgccaccttggggtttttctctctcatctccgccacagagctgtaagactgctcgatgaacttgaggagggctgactcggaagcatcacctgttgtggccctcttagcaatgggcaggatctcctgattagccttaaagtcagcccggttgcagaggccagcgattcgggccagcataaaccaggtatcagagctcttggtaaatgtttttccagtctgttcttcagtggtgtcggcctcatacacggtcatatcaaaccacatgtgggcgacggtcatgcggttctgggtgagggtgcccgtcttgtctgagcagatggtggacgtggagcccagcgtctccaccgcctccaggttcttcaccaggcagttcttccgcgccatgcgcttggctgtgagggtcaggcacacagtgactgtggccaacagcccctcaggcacattggccacaatgatgccaatgagaaaaatgatagcctccagccaaccatagcccaagagaagtgagagcgcaaaaaaagtgacaccaaggaagacggccaccacagtgatcagatggatgaagtgttcgatctcagcagcgataggtgtctggccaaccgccaggcctgacgtcagggaggcaattctgcccatcactgtggagtctcccgtagcaatcacaataccccgggcggttccttccacacagttggtggaaaagaagcagatgtttcgggtctccagagggttctcatgggtgaagtcaggggagcggctctggggttctgactccccagtcaaggatgagttgtccaccttacatccttgtgcagagataagccggaggtcagcagggactcggtctccacccttgatttccaccaggtctcccaacaccacctcttgtacattaatttgcatcttctctcctcctcgaattaccagagcttgctgaggcaccatgttcttaaaagactccatgatcttggagctcttggcctcctgataataggagaagcagccagtgacgatgaccacgacggacagtacgatgctcaggtagaggttgtctttggtaggctcctcattgaaatatatctggatgctgtaggccacaaagcagagaatggccccagtccatagtaggagggagaagcctccgaacagttgcttacagaatttgacccattctggagtggtggggggtggggtaacagtattgggtccacctcgagtcaggatttcctttgccctttggtggctatggccctttgtcaggtccacggagtacttggtgctcagctcttccaaggttaatttgtgatcatccatgaccacttccttcttcagttcctccatattgcgcttctgtttttccctcttcaccatttttttcttgataagcccttttttaggtcttcgtcttggactctggtcatggggagccactgtccctttcttcccccaaagccccatagctatccccagaaagagctgcccgagctcaactgtgggaagaaagctgagagagtgaggcaaggggaagggaagagggcgcgcgggcaagggggccacgagaagagagtggtggggagagaatgagggagcagaaagaaagaggcagggagggaggtgttgggtggtgaaggtgagagagaggaagggaagtgagagaggagagactgagcggtcctccagccgtccgctgggaagaggaagagtcaggagtgagggaagagggaggagagaagcctagggtggaaggataaaaaggtagaggtgagggaatgcagtgagggcaggaaacaagaggtgaagcgtaaccaggtgcctcagtgatgaagatgccgcaaggcccacaggaaggtgggaaatgcagtgagagtgaggaggcggagtgagcttcaaggatct

SEQ ID NO: 19327 - RNA, 858 nt, Homo sapiens
  source 1..858: mol_type = other RNA
tgttgggattcagcaggaccatgcccctccctgcggggctccagctagatgcaggctgggcttcccttcagcccacctcatcctctgcccatgattccctcaagccagcccaggattgcccatctttctcatccaagataattcatcctagtgtctcagatgttgtgtcaaacttataatctctggccccatcccagctctcacaacacccctgtgtcacatgaagctcttcatctgctgagtttagtagtacgtctccctttccacccagccatccgggtgctgacggatgaggagttttctgatttcatcatagacgaagatgagaatactgtagggaatggcacagagccaccaggttatcttgagtgggtacattcgcagggccacgtccatgcctggagtgtaggacagaaatgcagccaagagtgtctcctccaggatcccaaatattaagactttgtttctcatgccctgctggaaaagtgagttgcggcgagtcttggagatgatgagatccgcccactgcacaaccacgatggtgacaaaaaaggccgtttggcatgtgaactccacaacttttcgttgctcataggtccactgctgtccgtagctgtcctccaggtcattcaagtatttatcttcccagtggaggcggatgcccagcagatcaacaggcctaaaaccattctcagccaggattacaaagtaggtaaagaatccagccagagcctggatcatccctgtgaatgacagagttgcaggacaggggagcctggttcagagaagggccccaaaaggtaggccaggggagggctgggggctgggacttgcttctggctgggctggtgtgtgtct

SEQ ID NO: 19328 - RNA, 832 nt, Homo sapiens
  source 1..832: mol_type = other RNA
tgttgtcatgttttttccctagagataaaagttttcctttttgcctgactctctgatatctaaatataatattaacttgggagacaacaaaacaaaaatctaatttaaaagactcctcaacgattcaggaggcagtgattataaccgaacagtggtgatttcctaagattctgggcaagaacttccttcttcctatttcacatgctttgagagaattctaagattatgaaatattacttatgtaaatttcagccatcttacttctttgactacctaactagcaaattataggctgcatttttctgtgcattatttgttgtaaagaaaacatttttttttcaatttataaatgtatgtttgttgccatttcatggaaacaatgaaaaatgtgaaactcccttatttactgattcttggaacctttcacacaccaaatctcaggtttagcctctaaagcgcaaaggttttcagggtgaggtttgactcagtaggcctttcaaagtcacatctgtccatttctttttcgtgcatatacccccaagcaggcacaaatgcctgtaatgctgagaaccacacctaacaaaagggcgattgcatcaccggcttctactgcttccacaacaggcagcaccaaaagcagtgacatgaggactaaggacaactgtgttgaaactgaggtcatgatgttggaatcttgagggctgaaggttccaaagaaatggtatatatagaattctatctgacttgaaattttcccttcctggagctccggatgctgagattaagaggttccacgtgacacgaccttctaggaagcagccattacaggaat

SEQ ID NO: 19329 - RNA, 920 nt, Homo sapiens
  source 1..920: mol_type = other RNA
tgttgtcatgttttttccctagagataaaagttttcctttttgcctgactctctgatatctaaatataatattaacttgggagacaacaaaacaaaaatctaatttaaaagactcctcaacgattcaggaggcagtgattataaccgaacagtggtgatttcctaagattctgggcaagaacttccttcttcctatttcacatgctttgagagaattctaagattatgaaatattacttatgtaaatttcagccatcttacttctttgactacctaactagcaaattataggctgcatttttctgtgcattatttgttgtaaagaaaacatttttttttcaatttataaatgtatgtttgttgccatttcatggaaacaatgaaaaatgtgaaactcccttatttactgattcttggaacctttcacacaccaaatctcaggtttagcctctaaagcgcaaaggttttcagggtgaggtttgactcagtaggcctttcaaagtcacatctgtccatttctttttcgtgcatatacccccaagcaggcacaaatgcctgtaatgctgagaaccacacctaacaaaagggcgattgcatcaccggcttctactgcttccacaacaggcagcaccaaaagcagtgacatgaggactaaggacaactgtgttgaaactgaggtcatgatgttggaatcttgagggctgaaggttccaaagaaatggtatatatagaattctatctgacttgaaattttcccttcctggagctccggatgctgagattaagaggttccacgtgacacgactttggcccggcaaggtccaaatttgctcctgttttacaaatacactggtgcaacctaagtatcctttggagacgagttcgtacattaccttctaggaagcagccattacaggaat

SEQ ID NO: 19330 - RNA, 33 nt, Homo sapiens
  source 1..33: mol_type = other RNA
tgtttcggggctcatggcctgtgtaaatgggga

SEQ ID NO: 19331 - RNA, 65 nt, Homo sapiens
  source 1..65: mol_type = other RNA
ttaagacttgcagtgatgtttaactcctctccacgtgaacatcacagcaagtctgtgctgcttcc

SEQ ID NO: 19332 - RNA, 5665 nt, Homo sapiens
  source 1..5665: mol_type = other RNA
ttaagacttgcagtgatgtttctgaaaatttcccttttgcaagattaaatacacagcttataaaatgaaaatcctcaggtatacattagagattcacaggggttacagtgcatttcctatcacttccaatggccttccaatatttatttatttatttttcttaagtggctattatattgagagtgattcaccaaaaaatcttgagaatttggcattcttagttcccaaatttgtggaaaattttaatagggcagacagcgtggtaaatgtattacaaaattattaaactttacatatggaacacttattttctaggctattttctaggctcataaacacatacgacataacaaataaagacataaacatacaaacataaagaggtagaggggccatccagaggactccctgacctacctataatattgcttatacaactaaaattcagtcacttgctctctcaataatatgtaacatgctgaactctttgaagctgcttgagtttacgttatctgacatcaaataggatgtttaataaatatggacttctgataaacgtagtccataaagaacagaaagccacatattccttccgaatgtgactacagtgactttagcaaatgaaagtgaaaagttctaaattttcttaaagaattaaaaaataaattcaaaaatgatataaatatcttggtcactatttcaagattaagaaaaaaatcaatccattacagtgcccattataaatataaaaaattaatttctcaaacttgttttacagacaatatttttataaatattgctcaaagttccagcatatatatatatatacacacacacacacacacatatatggaaacacacacaaacacacaaaacagcatttaaaaatacacacacagaatgagcaaaagatattatccttcactctaacaaaactatctgacaggcctgtgattacatggcacttaaaaatattgatcaatttagatttttattcaaaatcagtatttaatgtattaaagacaaagacataagaggctgaatttccctttgttcacacaaagtctcaaacttattgttgcaatatgcttttggattttttaaaagacatcactgttacgtctaataggtgctaaccgcctctttaagaatggaatttctggtgactcagacatccattagtagcacatttctgcattaatactgtttcatacatttattttattttcatactatttttctgtatatgagaaagaaaaagactcaaaaataaaatgtacaacaagtggaacaagcagtgattggctgacaccccacggccaagggcaggctccagcaggtttcggagtagaaaggtcatcacagtatggtgcataatggagcatcatattagagtggaattcagccaaacacagtaatgtatggatgtagacgcatctgtttgctgtacttgttattggtttgacagctgtactcagagcagtgatctgatccaattgaaatgttgtctcctgctcccacaaatgtgttggctggtggtagatcttgtacggcctggtgtttttttcctgcagttggtgactggggatgaagctgaacagtaggcaatggggaactagatttgtaatgccttgccaggtcaggactgccgggcccaccattaacggacctgtatcgccccatgcttgggctgtctgacagcttctcattgacactatcatacctctgtccatttggcttagaagcctccacagtgacaatgctgctgtagagaggctgcttagattttttgtttttcttgtcctttttaggctttttagatttgtcatgctgttggggtgtaaaaaagtcttcgtgatcttttttgccggcttcatagccatttttatttttggacctgcagtaccttgccatcactacaattaagatgattagaatcaccgtcataatgccagcaaccacgccaatgacaatactgagtctctgtttgctaatttcatagcttgggtcaccagctatatcctgggtgagtgggatgtgcaaacttctagctatctgggagtcaatcgcagttgcattagaaacactttcattgacaaacacgtgcaccagagtcgtggtggactgggaaggctgcccactgtcattcacttgcaccaccaacctgtgcaagccataatgcttttgggtgagttttcccactaaggaaaccacaccactagtgggatcaatttcaaacagcttgaagggatttcctcccacaatgctgtagttcaggtctgcattgatgccatcatcactgtctgttgccaacactgtagctactactgtcctgacattactcgaaggtggcagtaaagtgtaggaaatgtttttgggaagggtaactgtgggagcattgtcattttcatccatcacaaaaagcgagactgtagctgtggcagatctgggaggatctcccccatccacagccttgactctgaaagtgtatgtggtctgatgttcccggtcaaaagacattgtggagtaaatggtccccgtgtcattttcaatagaaaaaatgttattgttctcctctatgtacaggctcatctctgcattccgccccttgtcagcatccatcacggtgaccatccccacagggctgttgggctgcaagttttctttcacataaaaggtgaagacgtcctgcataaacttagggtcattgtcatttttatcagccacctgcacaatcaccgtagtgctgccctgcagcacggggatgcctttgtctttggcgttaactttaaactcatacctgtcagtctgctcgcggtccagcacggtattgaccaggatgtccccagaatcgggatcgatggcaaagatccccatcacagaggagtccagcgagtaggcgatctcggcgttcttaccgctgtctgcgtctgtcgccagcaccgtggccaccctctcgcccgggatgttgttctcagggaagtaaacctccaccaccgactggccgaacatgggcgggttgtcgttggtgtctcccaccttgacaatcagggagttgttgctcgagaggctggggctgcctgagtccaccgccacgatgaccacgttgaactcccgggtggcctcatagtccagaggggtcgaggtgtgcaagaagtactttttcttgttctggtcgccctcggtgtcgctggctggcttgagctggaagggcacgtcgcccaccacggtgcaggtgaccaccccgttctcgccttggtctcggtcggacacctgcaccagagcgatgggggtgtcgaccagaacgtcctcggccacgttggccaccccgtccttgagggggatgcgcccaatcttgcggatttcaatggacggcacgttgtcgttctcgtctttgatgttaaggaccacggtggccttgtcggtcttggggggctgcccgcggtcgcgggccatgaccgtgaagcgcagctggttcacctcctcgcggtcgatccggtgcaggacgctgagccagccggacgtctcgtcaaggcgcagcagccgcctcaccgactcggtggccgccccgaacacgtattcgatctgcccgttgacccccacgtccaagtcggctgcgcgcagttgcaggatgggggtccccggggcgctgttctcagccaagtcggcctcgtacacgctcttctcgaagcgggggctgttgtcgttcacgtcggtgatgaggacccgtaggatggcctgcgaggagcgaggcgggtcgccgccgtcgcgcactcgcagggtcagctcgtaggagtcgcgctgctcgcggtccagcgcccccttcacgatcagctgcggctgcttctcgccgtccggggtgtccgccacctgcagctcgaacacgctgctgcggccgccggggttggtgccgccgccgccctctgatgcgtccagccgccgcttggagcctcccgagccgccgccgctcgcgccgttcccgccgcccccggggtagggggcgctgtcggccgccccggcgcgccggctctcgccgccgctgccgccgcctccgggctcctggagcagctcgtagcgctcgatgccgttgcggccgaagtcgcggtcggtggctgtgggcagcaggtaaagtgtgcccaccggccgattctcctccaccgtgagcgtgagcacgggcgacgggaaggtgggcgtgttgtcgttgatgtcaagcacgatgacctgaccctcaaacaggtccacccagctctgcgagggcccgatcaccgacacctcgaagtccaggaagcactcgttctcgtcgaagatcatctgacactggggcagcttctcgcggtcgatgcgccgctcgctcgtgctcagctcgccagtgaggttgtcgatcttcaggtactcggaaccggactccaggctgaaagtcacctcacccgatccggtcacgatgcccaggtctgaagccacgttgccgatgcggacgtcggcggggccctcctcggccagccggtaccggaggagctgcttggcggccgccaggctgagcgagagcggcaggaggaggcagcagcccaagcaccagccgcgcgcccatcccgcggtccgcatcctcagcatcttctcctgctgctgctgctactgctccttctaaccacagccccctcggcgcccccctcctccggggccggccgcctgccctcccccgagtcctctcccctctcccggaaaggaaggagcgagagggaggggagggagggggcaaaagcggcgtggagagttggccgggaatgggggtgggagggcagcgatagatgcttctttttttcctcctgcttcttccgaaagttattgtttcataattcatgcaatgggtgctaatcgcccgctcgcctgccgccgttcagtcgcagtactcacagttcacgggacactgcgcgccgcgggttcggcgctcccccaacccagagtcatcccctcagcgggcggagaatccccggctctagtccccgctctgtcggaaggggccagaaccgctccggcagacgggcagtggggctgggaagaggtggggaatgagcctgcagcctcccccgcctgccagcccgctggtctttgctgctactcgagttgagtccaattcacgttccaggcactcactccaaacccaggctctgctccggctccggccacccagacaaacgtgagtcgcttcctgcaccaggcgctggggccagcaacaagccagtctcaactccgactctgctcatgcagcgggggagccagtcaacagatcgagaatgaaaaatcccccggcacgtcgcttcgggcacggtgcaggggagactactcgcgtcacagagcggtcagtgtcagggtccccccggcgcgccaaagagaagcccgagccatcttcagagacgcccagagtcagtcccttctcaccccggagagcgcgggtttctcttttttcttaacaactctgcgcaaggtcattagtcacgaagcagccgcctgaaaccgcagcagcctttcgcccacgggggcgaaggctgagcagtgcgcaccgtgcggtgcccaagtttgggttcgcagccgcagagtccgtgccttttctcacctgcattcggcccgcatgtcggagcagtgggatctgcagcgctgtgcgcgattc

SEQ ID NO: 19333 - RNA, 7987 nt, Homo sapiens
  source 1..7987: mol_type = other RNA
ttaattttttgtttcggtcactcttgatagcagacattgactgaaacaaaaaattaaaagctttatattcaaaatttgcaaaatgaagctgggtgtggtggtgcacgcctatagtcccagctacttgggaggctgaggctggaggattgcttgaggtcaagtattggaggctgcagtgtaccatgatggtgcctataggaatagctactacactccaacctggacaacgttatcaagaccccatctcttagaaaaatgcaaaattaaatgcaaaagaaatgggctgggcatagtgattcatgcctgtaatctcagtaccctgggaggctgaggtggaaggattgcttgagtgcaggagttcaagaccagtctaggcaacatagtgagaccctgcctgtaaaaaaaaataataaaaatagttggatatggtggcatgtgtctgtagtcccagccactctggaggctaaggtgggaggatcagtagagcccaggaggtcaaggctgcagtgggccatgatcatgtcactgctctccaacctgggcgacatccagaccctgcctctcatcagctgaaagtgcctgtgaaaaacaaagcttctctaaaggcagtgtggtgtcctgcactggatcttatgtctcagagcgttggtggagaacactgacatcccaggcattaaaatgaggtggtgtttggtagatggtggctaatctgcattttgccaaagcagcatcagtaggtggtccaacaatagtatctcaggcttactaagcatctgtccagataacagggaagagccagctcagtcagtgttactgtctcttctgggctccctgacttgtatttagagcgcaataccaagttgcagatccaactgctggatgacaaagttttgggagttcctgccctccaaccggacgcacaaaacagcatcatctctaatcaaattggttcagtgtaaatggagggtttataaaatagaacgcaatctcaggcaaagtctctgttcttccacgtatctgccttcatcaagtgactcatgagacaatcacaggatcggcaggagtgagacctaggaaagatattcaagtaaaacatgtttcttaactagttctgtttctggtgattggaatttgcttgattttacttactaataaaatttttgctgcttatattttaagtacatctgaaaaacctgattatgaagttagaatccgtattatctcctcgaatactcttagaaagcaatgtctctctataaaaacatgaggagaaaaagacttctacagcatctttttattgtctttaccattactttaatgcattttaaaatttatctacattaattgggaacaaagaaaaatagacatttctttgtttttcataaataactaatcttcatatttgataaaaatctcaaatgattattttaccttcccacaaatataatacatacaaaatttttctgaagtaaggtcaacaaattaagtatcttgagactaacataaccacatacaactgctgtttctactgactcccaggaacgaagcagaaacaaaaactcatcaagctgctctgggtttccttttgtaagtgttacagattcagaactgtaatcatgtatcatctgccagtaataacatatggattcaaattgattgtctacaaataaagtatcgctggctctagtgtaacttctggatttaacataacagtgactacagcatgggataggcactatacatatatggaaatcataaacagtatcgaatgccctggacttcaactactgactcggtatgtgcctcatttggctcagtaataaattcacctgcaccaaacccgtatcaaaagtcaccaaatctctcatatatatatataatatatattatgtatatatacaacccacaaaacatacatactatacatagtttgtaacaacatgaagtcatactgtcttaaaatgatgcactcacagacagacactatcctggctgaaataaatcctattgtcatcaggctgctagcttttgagagtcttgactcaggttagctacttatattctgcctactcttcacccttctttaacgtcttggcagttctttcagaaccaccctccgcaatccagacagatttgtttcccaggatcacttgattggactttggaaacaagaaagagcatgcagagggagcaggcaattcttagccactgtccctcacacctgcctatacgtgtgatgtgctctgtcctgttggccacatttagtgttagaaagcagttattcaaagctctgtccctcctaccccccttgggctttctgtagagcacaaaagtgaaagaagcttctttggctggggtagcagttcattaaaatatacaactacatttcctagctctggggttcccattctgtactggagagtgcaggtcacggatgctgttattaaggtttggtgtgtgatccatgaggttttctcctggcagccggtgtcaggattagcgcagctccagcccaggaggcaacagcctaatgaataccaactttgaaacagtgctgtcggcacgttatttaagcttgtacatgcccacaattacacacaacacacacatgggccttggtcactggcaatggtcatgagaaaatatgagaaaggtttgcaaggaaaaccaataaggcaccaagaaaaattatttccagtcaattttaccatttcaaaatgtgagaaggaaaatcatagaaattaaaaagatttcctaaaatctggtcagctaattcactgagaggtcccattagttcctttagacaacctacctgaatggaatccttaccccctaagctatgaagtgaggcattgcttaaaatcaaactgaaagggacagccctgaagctgtacacataagagactccaatgggccctaagtcctccccagctccacaaagctggctgtgaagaagttgctgaactactccataaccttttattttacagttgctttcatgagcatgacttgtttccataatcacatgcaaattgggggaagtaactatatggatggaaacagggggtggctgtaagtagatccagtttctctcccctggggtggctgatctcagtaagacttagggatgcaggtgggcttttatctttgtctctcttaggggatgagggaagagagggacagcagaggtgagaacagagacaaagaagtgcttctgaaagttggtctggaattagaccccaaagatcctgactaatattgccccccacttgggcttagcgtcctttgttttaactggcttatttttaaagtaaattagttgttcagcatgttgctaaaacaaaacaaaaaaaaattctaaaaatgaattaaatcactttcatccacttcatcccacaacttttggatacactgtgcatcatttccagatttctccacaaagaaggagggacaacccaaatgaggcacaatgactgaaggcagcagagcagtctgtctactttctgggaagacatatgaaatgagggaaaaggtcaaggtgatcagaaaaggttctctcatttgaaaaacaggagaggaattggcattcagtcaagggatctatttcaagattctaggaagaggcttcttcctagaagaataaatagaggaataaaataggcacaaagttctgtagctatttgtacgaggttttgtagaatccactgaaattttaattcagaggataaattgggtaagagcagtgcattttaataaatgtgaagtttttgagagtccttacaactttaatactaggtttcttcccaccagtaaagtgtttaaattccccctgggaactatgcatttgtctatttaacatccatgaagtaaaaattgtcctaggcttaaattttacttttccaactttggtataagtgaattacaaatgcctacactcaagttgttttcctagacaggattttctcaaatgttaattgctctggccattttagcttcctaaatttagtccccaatcctggtcattggtattttgctggctgaggcactgtcaccccccttccccagtaatggccccacactcttcatgaatgaatgcttaaacagattaggaaagcaaacagaattttctaatagcaaagaaacctctgtgtgtatgttcatcaatataagcgttcataatgaatgaaggaatagttaaacagattagtaaagcaaaccaaattctctaattgcaaagtgtgtgtgtgtgtgatcatcaatatacaggctttctcagaagaggaagaaaactatagaggtagcactatactgatctatattttaaaaggttgtgcaagcatgttatgcatctcttttgttttcagagacggcagagagcaacgtcttgctgctcttggaatatctggctataaactagtccaaagtccaggaacacttattttcccttatttgggccaatgtttgttcacaggtagccagcctccctcccccagttcaagcacttcattcaagggtgggtgtggtttctaatcacagctctccaggagaggaggaataagaaaagcaaaaaggctgtttaacatgataaagggggaggggggaggggggagggggtggagcaaataagtgttggaaatttacttattagaagtatatccatttcagtccttacatttaaaaaggagccccctttagcaactgtcgctaagtattgtccagagggagtgggtttatacttttaccaaaattataacacaagttccttaaaaaaaaaaaaaaaaaaaaaaaaaggggatcactgaagcttaagaaccacccactacctctcaggcacaaagctgccatctcaccagcctaaaattcaagctccaccaatcaccatcgcttaggctctcactactgcaaatatttatgccagatcctctataatgctacctctaacttattcaagacacaacgatggtgctgttaggagtgagaattattacaagcactacagaaaagaaactgaacctccctctataaacaaagctaaggctgaacacaaaaccgctaagcactccctaaccttgtcactttggggaggccctgagctcattatgctcccctcctaggtatgacctggggctataaactgcagctcaccttaaagaatcatggacactttaagcagtggaaggagaagctggctgaaaaagcacacccaacaacttcccagtcacagcaaccgaaacgttcactgttcacatttttttttaaagacacacgtataggaaatatattttcccaattgagaccacacagttcaaagaaacctgaaccaagtggaacttcattacaacgccaaccttaggattgtaaagcccccaaagcaaaggtaaattgttgccaaaatgcaacaaagttacaaattaagaaaaatacatataaattaaaaagagggttcccataaagaaggcagtaagaaacgcaaaatagaatacacgtgagctgggccccttggagaagacctgggacaggttcttcctcgaaaacgcccctcttccctctctccaagtcgccgcgggagggggcaacagcaccatgaaggtaaacggaagtgaccttggcaaaactaccaaacaaaacgcccccctcccctcagctctccggccgagtccctcggcggcagcctcctacacgtgcgacagggacacctgcttgtggtaggtggcggcggggcccggcggcccggtcctgcctgtgagcgcggcgctcgcctcggggtagtcccctgcggccatggcgcccccgctcttgtggccgcgccgcgggcggcagcagcagcggctggtgaaacgccgccacgactccaccgtcttgcccgaccagatccagacgcccgacgtgatgcccaccaccaggcacatgaagtacttgagcatgagcacccagtactcgggcttggcgcgcggctggccggtgtcgtggcccgggcaggcgcaggtgagcgccgcctcccagctctcgcggtagtgctgctcgtacaggtagcaggccaccacaatgctggcggggaccgtgtagagcagcgtgaagatgccgatgcggatcatgagcttctccagcttgtccgtcttggtgccgccctgcttgatgacgctgcggatgcggaagagcgacacgaagcccgccagcaggaagagcgtgcccaccagcaggtagagcaccagcgggcccagcacgaagccgcgcagcgagttcaggttctggttgcccacgtagcagatgccggccactgggtccccgtccacggagctcagcgccagtgccgtgatggacttgacgctggggatgagccacgcagccaggtggaagtactgcgcgtagcccgcgatggcctcgttgccccacttcatgccggcggccaggaaccaggtgagcgacaggatgacccaccagatggagctggccatgccgaagaagtagaccaggaggaagacgatggtgcacagtgcagggcccgtggtctcgtagtggatgtggttgtgctcgcggctgcaggccacgctggcatggcccacgaccagacgcaccaggaagcccagcgacacgcacaggtagcaggctgacaggaagatgatggggcgctcaggatagcggaagcgttccatgtcgatgaggaaggtggccactgtggtggacgtggagatgaagcacagcaccgaccacaggcctatccagaaggtggcgaacgtgcgctcgtcggcactgaaggacggctggtagcagggtaccgcgcagttgggcacctggcccgtccgcaccttgttgtagagcgggtgtgactccttcagaatgggcacgaagggctcgcgacacttgcacacgaacgggcccccagcggggcattcgccccccgaggccggcgcccctggcgggcctggaagggtgggcttggctgggaaaggcctggggggcgccgtggtggcctcgctgcggttgtaatccatgcagaggacctcggcgtcgcggcccagcaccgggaggcggtcgcagctcatgcgctcgggccaggcgaagccgtactggcgcatcagcggcgagcagccggccttggcgcgctcgcacaccgagcggcagggcggcagcggcttgtggtagtcgggcagacagatgggcgtgtacatagagcataggaagaagcgcaggtccggcgagcattggatctccaccagcggccagaactggtgcacctccaggcccgcctcgtcctgcgtgtcgtggttgaactggttgggcatgtgcgtcaggttgtagccgatgccgcggcacatgggcaccgtgatttcctggcacaccggggccttggacgcggcggccgcccggcccaccagctgcgctaggagcagcagcaacagcgagggcggcgcggatgggtcaggccgagccatcgccccctccctcccctcgcctccagcagcccgcgagggacgcacacaggcagaggaatccgggccggggcttctccctccggcgtctcgtgtgtggcgccggggctggcaacctgttggttgctttttcctttaaagaaaaccgtccaaagataaactgcttcgggaaggcgctgcctccgctggcagcgctccgctcctcgccggatagggctggggagagacggttagggctcggattccagggaaaggactctccacggatcccgccgagaagagcagacagtccccagccagcctgggtcctccgtccctgggtcactccgctgagaagcgcgactcagagccgggctggcgcccggaaagtttagcgacaggctgggtacccgtggcagcggcacatggcagcaggtgggggcgactcagagtggggggcgcccccagaacaggggcggcgcaggccggtcactcgccctctcctcctcgggagccccccgcatgatccagacggagccgggcaggggcaggccgtgcgttctccccggggccgggag

SEQ ID NO: 19334 - RNA, 71 nt, Homo sapiens
  source 1..71: mol_type = other RNA
ttacacagctggacagaggcagcagcgacagtgacagcgatagtggcagcagcggtggcagcgagagctat

SEQ ID NO: 19335 - RNA, 268 nt, Homo sapiens
  source 1..268: mol_type = other RNA
ttacacagctggacagaggcagcagcgacagtgacagcgatagtggcagcagcggtggcagcgagagctatgcggggccagggtccacccctttctagctttggcgtctggttggcttccagggcagcctccgatccatcccgcccgaggaggcaaggttcgttttccgattggcctattttctccgcgcattttatttccggttctgaggacgccgcggaagcgggacgggattggagtgctctgctccggacgcactacgtaggtg

SEQ ID NO: 19336 - RNA, 69 nt, Homo sapiens
  source 1..69: mol_type = other RNA
ttagccaattgtccatctttagctattctgaatgcctaaagatagacaattggctaaatagaaattgtg

SEQ ID NO: 19337 - RNA, 1365 nt, Homo sapiens
  source 1..1365: mol_type = other RNA
ttagcttaaggagtaccagatcagggcagagacttcccagctgggtaaggcatgctttgagggaagactccaccagccctgccaggaaagggcagcaggcgcagtgcccctatggggcccacatggctggtaacagcagcaggacacctcttccaaagctgtccaccagccccactaggggctcctactcatggcaaaaaagactacatgagcccacaactgtcaactaacacagtgccacctcctcccaaagcaaacacatatacatacaatgttaagaacctattatcagaacagcagtgcagcagaccctggccttggtctctgaaagtcctgtgtcactggctgtaaggacgcttggccacaggttcctcctccttctcccgcttcagccattgctctaggagtcctgcagtgcctctcttggtggggagtggactcttctgcaggaactgactggaccactggggaacatctgactcttccttttgaggtgtttttgagtcttcctttttgggtgactttgtggccaaccactgcaacatcctctggctactgccacttgccctgagctcctttttgaccaccaagtcgacaggagccagacactcaggagtgttgtttcgcgagttgttcaccacagaagagactgcatggaaggtgatgttctctgttgggtggattaatttcagagcttcctgagttgagacttcaccaaagtcaagccatttagaaactgcctcctctccatctaatatggcaggcatcctgtggtggatgtcactcaagcctttgcaggaatccactgtgatgatggtataggaatacaggacatctcctccctctgggggctcccagcagtcaaagatcccggccattgtcagcagcctccagttgtcccagactttctcccagttctcaggactatctgcagcaccaatgctacctgacttaaatgaccgtttctccattacggtatcactacgacagttggtagtattgaactgcagcttggaaggatcactttctttgaaccaagaagggaccaagccccagcgcatgggagcaatgatacgctcagatgagtctgcatccttctcaaagtgcagtcgagacagaagcactgggctgttggattgaggactcttgttgtaagaggggcagtacttatcagggtccctccactccgggagccgctgctggccccgccgatcctggtaggcgcaagctctcgtgagaacatctctaggtaagtgacaggatgttcgcccacacattcttcaacaccgcccctcgcaacctcgccccggcagcgcgcgtcacctccctcgactctcctcacccccgctccgctccgctttggcc

SEQ ID NO: 19338 - RNA, 1462 nt, Homo sapiens
  source 1..1462: mol_type = other RNA
ttagcttaaggagtaccagatcagggcagagacttcccagctgggtaaggcatgctttgagggaagactccaccagccctgccaggaaagggcagcaggcgcagtgcccctatggggcccacatggctggtaacagcagcaggacacctcttccaaagctgtccaccagccccactaggggctcctactcatggcaaaaaagactacatgagcccacaactgtcaactaacacagtgccacctcctcccaaagcaaacacatatacatacaatgttaagaacctattatcagaacagcagtgcagcagaccctggccttggtctctgaaagtcctgtgtcactggctgtaaggacgcttggccacaggttcctcctccttctcccgcttcagccattgctctaggagtcctgcagtgcctctcttggtggggagtggactcttctgcaggaactgactggaccactggggaacatctgactcttccttttgaggtgtttttgagtcttcctttttgggtgactttgtggccaaccactgcaacatcctctggctactgccacttgccctgagctcctttttgaccaccaagtcgacaggagccagacactcaggagtgttgtttcgcgagttgttcaccacagaagagactgcatggaaggtgatgttctctgttgggtggattaatttcagagcttcctgagttgagacttcaccaaagtcaagccatttagaaactgcctcctctccatctaatatggcaggcatcctgtggtggatgtcactcaagcctttgcaggaatccactgtgatgatggtataggaatacaggacatctcctccctctgggggctcccagcagtcaaagatcccggccattgtcagcagcctccagttgtcccagactttctcccagttctcaggactatctgcagcaccaatgctacctgacttctctgtcttgatttgaggaaaatagatgaagtatggctgcctctggtttgttccctgacatcgctgccactcatagaatccatctgctaaaacgacacagcgtcttccctttcccagaggcaccttaaatgaccgtttctccattacggtatcactacgacagttggtagtattgaactgcagcttggaaggatcactttctttgaaccaagaagggaccaagccccagcgcatgggagcaatgatacgctcagatgagtctgcatccttctcaaagtgcagtcgagacagaagcactgggctgttggattgaggactcttgttgtaagaggggcagtacttatcagggtccctccactccgggagccgctgctggccccgccgatcctggtaggcgcaagctctcgtgagaacatctctaggtaagtgacaggatgttcgcccacacattcttcaacaccgcccctcgcaacctcgccccggcagcgcgcgtcacctccctcgactct

SEQ ID NO: 19339 - RNA, 1664 nt, Homo sapiens
  source 1..1664: mol_type = other RNA
ttagcttaaggagtaccagatcagggcagagacttcccagctgggtaaggcatgctttgagggaagactccaccagccctgccaggaaagggcagcaggcgcagtgcccctatggggcccacatggctggtaacagcagcaggacacctcttccaaagctgtccaccagccccactaggggctcctactcatggcaaaaaagactacatgagcccacaactgtcaactaacacagtgccacctcctcccaaagcaaacacatatacatacaatgttaagaacctattatcagaacagcagtgcagcagaccctggccttggtctctgaaagtcctgtgtcactggctgtaaggacgcttggccacaggttcctcctccttctcccgcttcagccattgctctaggagtcctgcagtgcctctcttggtggggagtggactcttctgcaggaactgactggaccactggggaacatctgactcttccttttgaggtgtttttgagtcttcctttttgggtgactttgtggccaaccactgcaacatcctctggctactgccacttgccctgagctcctttttgaccaccaagtcgacaggagccagacactcaggagtgttgtttcgcgagttgttcaccacagaagagactgcatggaaggtgatgttctctgttgggtggattaatttcagagcttcctgagttgagacttcaccaaagtcaagccatttagaaactgcctcctctccatctaatatggcaggcatcctgtggtggatgtcactcaagcctttgcaggaatccactgtgatgatggtataggaatacaggacatctcctccctctgggggctcccagcagtcaaagatcccggccattgtcagcagcctccagttgtcccagactttctcccagttctcaggactatctgcagcaccaatgctacctgacttctctgtcttgatttgaggaaaatagatgaagtatggctgcctctggtttgttccctgacatcgctgccactcatagaatccatctgctaaaacgacacagcgtcttccctttcccagaggcaccttaaatgaccgtttctccattacggtatcactacgacagttggtagtattgaactgcagcttggaaggatcactttctttgaaccaagaagggaccaagccccagcgcatgggagcaatgatacgctcagatgagtctgcatccttctcaaagtgcagtcgagacagaagcactgggctgttggattgaggactcttgttgtaagaggggcagtacttatcagggtccctccactccgggagccgctgctggccccgccgatcctggtaggcgcaagctctcgtgagaacatctctaggtaagtgacaggatgttcgcccacacattcttcaacaccgcccctcgcaacctgcgaacctgtgggccgcggatcccgctccggactctgctccccggagcgggggccggtgctcggggagcaggtggcccccagccaccggccgcgatccctcgcccctccccgcgtcgcctccgctccgctccggccctcagactccgccgccccgcgtcgcctcacttcggcccaggccgccctctccgcgtcgcctcgcgtccgctcgggcctctgctcccctctgtcagctcgc

SEQ ID NO: 19340 - RNA, 1636 nt, Homo sapiens
  source 1..1636: mol_type = other RNA
ttagcttaaggagtaccagatcagggcagagacttcccagctgggtaaggcatgctttgagggaagactccaccagccctgccaggaaagggcagcaggcgcagtgcccctatggggcccacatggctggtaacagcagcaggacacctcttccaaagctgtccaccagccccactaggggctcctactcatggcaaaaaagactacatgagcccacaactgtcaactaacacagtgccacctcctcccaaagcaaacacatatacatacaatgttaagaacctattatcagaacagcagtgcagcagaccctggccttggtctctgaaagtcctgtgtcactggctgtaaggacgcttggccacaggttcctcctccttctcccgcttcagccattgctctaggagtcctgcagtgcctctcttggtggggagtggactcttctgcaggaactgactggaccactggggaacatctgactcttccttttgaggtgtttttgagtcttcctttttgggtgactttgtggccaaccactgcaacatcctctggctactgccacttgccctgagctcctttttgaccaccaagtcgacaggagccagacactcaggagtgttgtttcgcgagttgttcaccacagaagagactgcatggaaggtgatgttctctgttgggtggattaatttcagagcttcctgagttgagacttcaccaaagtcaagccatttagaaactgcctcctctccatctaatatggcaggcatcctgtggtggatgtcactcaagcctttgcaggaatccactgtgatgatggtataggaatacaggacatctcctccctctgggggctcccagcagtcaaagatcccggccattgtcagcagcctccagttgtcccagactttctcccagttctcaggactatctgcagcaccaatgctacctgacttctctgtcttgatttgaggaaaatagatgaagtatggctgcctctggtttgttccctgacatcgctgccactcatagaatccatctgctaaaacgacacagcgtcttccctttcccagaggcaccttaaatgaccgtttctccattacggtatcactacgacagttggtagtattgaactgcagcttggaaggatcactttctttgaaccaagaagggaccaagccccagcgcatgggagcaatgatacgctcagatgagtctgcatccttctcaaagtgcagtcgagacagaagcactgggctgttggattgaggactcttgttgtaagaggggcagtacttatcagggtccctccactccgggagccgctgctggccccgccgatcctggtaggcgcaagctctcgtgagaacatctctaggtaagtgacaggatgttcgcccacacattcttcaacaccgcccctcgcaacctgtgggccgcggatcccgctccggactctgctccccggagcgggggccggtgctcggggagcaggtggcccccagccaccggccgcgatccctcgcccctccccgcgtcgcctccgctccgctccggccctcagactccgccgccccgcgtcgcctcacttcggcccaggccgccctctccgcgtcgcctcgcgtccgctcgggcctct

SEQ ID NO: 19341 - RNA, 1476 nt, Homo sapiens
  source 1..1476: mol_type = other RNA
ttagcttaaggagtaccagatcagggcagagacttcccagctgggtaaggcatgctttgagggaagactccaccagccctgccaggaaagggcagcaggcgcagtgcccctatggggcccacatggctggtaacagcagcaggacacctcttccaaagctgtccaccagccccactaggggctcctactcatggcaaaaaagactacatgagcccacaactgtcaactaacacagtgccacctcctcccaaagcaaacacatatacatacaatgttaagaacctattatcagaacagcagtgcagcagaccctggccttggtctctgaaagtcctgtgtcactggctgtaaggacgcttggccacaggttcctcctccttctcccgcttcagccattgctctaggagtcctgcagtgcctctcttggtggggagtggactcttctgcaggaactgactggaccactggggaacatctgactcttccttttgaggtgtttttgagtcttcctttttgggtgactttgtggccaaccactgcaacatcctctggctactgccacttgccctgagctcctttttgaccaccaagtcgacaggagccagacactcaggagtgttgtttcgcgagttgttcaccacagaagagactgcatggaaggtgatgttctctgttgggtggattaatttcagagcttcctgagttgagacttcaccaaagtcaagccatttagaaactgcctcctctccatctaatatggcaggcatcctgtggtggatgtcactcaagcctttgcaggaatccactgtgatgatggtataggaatacaggacatctcctccctctgggggctcccagcagtcaaagatcccggccattgtcagcagcctccagttgtcccagactttctcccagttctcaggactatctgcagcaccaatgctacctgacttctctgtcttgatttgaggaaaatagatgaagtatggctgcctctggtttgttccctgacatcgctgccactcatagaatccatctgctaaaacgacacagcgtcttccctttcccagaggcaccttaaatgaccgtttctccattacggtatcactacgacagttggtagtattgaactgcagcttggaaggatcactttctttgaaccaagaagggaccaagccccagcgcatgggagcaatgatacgctcagatgagtctgcatccttctcaaagtgcagtcgagacagaagcactgggctgttggattgaggactcttgttgtaagaggggcagtacttatcagggtccctccactccgggagccgctgctggccccgccgatcctggtaggcgcaagctctcgtgagaacatctctaggtaagtgacaggatgttcgcccacacattcttcaacaccgcccctcgcaacttcggcccaggccgccctctccgcgtcgcctcgcgtccgctcgggcctct

SEQ ID NO: 19342 - RNA, 1356 nt, Homo sapiens
  source 1..1356: mol_type = other RNA
ttagcttaaggagtaccagatcagggcagagacttcccagctgggtaaggcatgctttgagggaagactccaccagccctgccaggaaagggcagcaggcgcagtgcccctatggggcccacatggctggtaacagcagcaggacacctcttccaaagctgtccaccagccccactaggggctcctactcatggcaaaaaagactacatgagcccacaactgtcaactaacacagtgccacctcctcccaaagcaaacacatatacatacaatgttaagaacctattatcagaacagcagtgcagcagaccctggccttggtctctgaaagtcctgtgtcactggctgtaaggacgcttggccacaggttcctcctccttctcccgcttcagccattgctctaggagtcctgcagtgcctctcttggtggggagtggactcttctgcaggaactgactggaccactggggaacatctgactcttccttttgaggtgtttttgagtcttcctttttgggtgactttgtggccaaccactgcaacatcctctggctactgccacttgccctgagctcctttttgaccaccaagtcgacaggagccagacactcaggagtgttgtttcgcgagttgttcaccacagaagagactgcatggaaggtgatgttctctgttgggtggattaatttcagagcttcctgagttgagacttcaccaaagtcaagccatttagaaactgcctcctctccatctaatatggcaggcatcctgtggtggatgtcactcaagcctttgcaggaatccactgtgatgatggtataggaatacaggacatctcctccctctgggggctcccagcagtcaaagatcccggccattgtcagcagcctccagttgtcccagactttctcccagttctcaggactatctgcagcaccaatgctacctgacttctctgtcttgatttgaggaaaatagatgaagtatggctgcctctggtttgttccctgacatcgctgccactcatagaatccatctgctaaaacgacacagcgtcttccctttcccagaggcaccttctcaaagtgcagtcgagacagaagcactgggctgttggattgaggactcttgttgtaagaggggcagtacttatcagggtccctccactccgggagccgctgctggccccgccgatcctggtaggcgcaagctctcgtgagaacatctctaggtaagtgacaggatgttcgcccacacattcttcaacaccgcccctcgcaacctcgccccggcagcgcgcgtcacctccctcgactctcctcacccccgctccgctccgctttggccacccgcgtc

SEQ ID NO: 19343 - RNA, 400 nt, Homo sapiens
  source 1..400: mol_type = other RNA
ttaggccgcagatctgggtgaggaggctgctggggttggtggtgttgaccccaactgtgagcggctggatctccaggggtaggtccaggaagctctggggggtgaggcgggcacggaactgggcctggggcggccctgagctgctaaacaccacggccaccgtcatgccctgctcgccctgccccggacccagccctgcccaggcaccgaagagcgaggtgagcaacagggccggccccagggccccacccatgtccaccggagggtcactcgggctgtgaagttcggggtatttttaggccggcgataaataattcatagggaacgtggcatcaggctccccccgcgggaggagggggcgcgagcagcgagagccaccgtcacccgcggctcaaggaca

SEQ ID NO: 19344 - RNA, 410 nt, Homo sapiens
  source 1..410: mol_type = other RNA
ttaggccgcagatctgggtgaggaggctgctggggttggtggtgttgaccccaactgtgagcggctggatctccaggggtaggtccaggaagctctggggggtgaggcgggcacggaactgggcctggggcggccctgagctgctaaacaccacggccaccgtcatgccctgctcgccctgccccggacccagccctgcccaggcaccgaagagcgaggtgagcaacagggccggccccagggccccacccatgtccaccggagggtcactcgggctgtgaagttcggggtatttttaggccggcgataaataattcatagggaacgtggcatcaggctccccccgcgggaggagggggcgcgagcagcgagagccaccgtcacccgcggctcaaggacactcgcgatgc

SEQ ID NO: 19345 - RNA, 663 nt, Homo sapiens
  source 1..663: mol_type = other RNA
ttaggccgcagatctgggtgaggaggctgctggggttggtggtgttgaccccaactgtgagcggctggatctccaggggtaggtccaggaagctctggggggtgaggcgggcacggaactgggcctggggcggccctgagctgctaaacaccacggccaccgtcatgccctgctcgccctgccccggacccagccctgcccaggcaccgaagagcgaggtgagcaacagggccggccccagggccccacccatgtccaccggagggtcccagcagctccttgcagggtcgcgggacgcacctgggggttcaggttgccgggtgcctttgctccgcgtgtccccgccctgcccgcgtaggcaggaaacaggagactcggggcttcccctccccgccgtcggggatcctgggcgaagcccccagagaccggcgcaggcggctggtgcgcagccagggcccagcgccaggtcttgctcgcccagtgccctctctgcctacccttccctttgcgctctggaagcccgggagccgggcacgggccagcatctgcaagatgccactactctggaagcccactccgattctcccaggtcgcaggaaggagagagctaggctggggcaaaggagatggggcagagctggaaggggaagaagcgggactcgc

SEQ ID NO: 19346 - RNA, 3763 nt, Homo sapiens
  source 1..3763: mol_type = other RNA
ttaggccgcagatctgggtgaggaggctgctggggttggtggtgttgaccccaactgtgagcggctggatctccaggggtaggtccaggaagctctggggggtgaggcgggcacggaactgggcctggggcggccctgagctgctaaacaccacggccaccgtcatgccctgctcgccctgccccggacccagccctgcccaggcaccgaagagcgaggtgagcaacagggccggccccagggccccacccatgtccaccggagggtcctgcggagagaccagaacaagcacagggagagagacagaggtttggagagaggcagatggacagacaggagggacagagggacacacatacggaagatgaaagagaagaggggaaaacctccctccccgaagagaggcggagagagagggagacagacagacacggacaaagagaaagagacagaggttagttgagcatcccaagggcatcccagaagagcaagggctggggaagaacaggagccatgaccgggacccagccctccagtctactgatgccttccaaaactcagccagtgggttctgccctaggaagtcatactgaaaatgctagtctggggttcaagtgcatggatttgagtcagacagatctgagttcgtgtcccagttctgccactaactggctgtgtgatcttagggaagtcacttagcctctctgagccatgttttcttgcctgaaataatcacagcagtgtgaggacttagatgagctaacaggctatttgctgggattagtgacctcatcccgcaggtgacaggcccccagccaggtgaaggaagacagctcttgcatcacccccaacccccacccccaccggccagtcctcctcatagtctaaaccggatcttccatctgtctctcaccagggcctgtgctactggtcagtgtgccctgcttgccatggggccagccccaagggccctcctctgcatggttctgcctggcacagagccccctcctcctgggcactggacgtcactacagcccttccttctgtggcctcagctagtagcagctcttccgcagcagggtgcaacagcactgacttgttcagagctcaggggtaccggaaaacccaagctggtgagctggggtttggtcttgttacacatgagctggtgagctggcctctcgggccatcactggcgtgcaggatcttttgaacccaacccaggggcctgacacgtatccttgctaaatgtcattattttggattgggaccaagagccacagcagtgagggtaacacaaagcctgagtggagtggtgcccacggatgtcactctccctcccagctggccatcggccatggcactgccatctctcccatcttcatcacatccccagcaaaacttctgagcagggaagagctaaagggtggacagggtgagcctgccactccagccctcccgcctcccccaggatctgcacatctctgctacagaaatgctcacgaaaatcaagcagttgccagaaaccacgcctccgaaagacagatgcccttcagggatggggcccgagacaactgctgggcaggctccagctttctcacagggccttccttttgcctgccaccaaatttctctctctctctttttttttttttttgagacagagtcttgctctgtcacccagactggagtgcagtggtgcgatctcggctcactgcaagctccacctcccgggttcatgccatcctcctgcctcggcctcccaagtagctgggactacaggcgcccaccaccatgcccggctaattttttgtattttttagtacagatagggtttcaccgtgttagccaggatggtctcgatctcctgacctcatgatctgcccacctcggcctcccaaagtgctgggattacaggcgtcagccaccacacccagctatctctctctttttttttaatccaaagcctaatgtcttacagacatatgggccttcttgtatctctagttctctctaaggaatccagagagcggggaagtgcaagaggctaccaggaacattcaggaaagttcctcttctccccagggtggcactgaaaggatccctccagggaacccactaaaccaactttagtgtagaaacatcaattggcccgtgtgtgctgagccccttccctgcagcaggcgctggatggtggaatgtccctatgggtgagacatggtccctgccctccaggaacttagagtcaaatctgcagaatgagcatgctgctgttagcacctccaacctccttttttctaaatatatttctctttccaaccttctctccctacttccctcaaactccccagcctccccgtcaagatcttctcttagctaagcatctagagctcattcacaggaaggtatgagggactgatcatagctgaaagggttctcattcccaagagagatgtagtttaaccacaatcagagccttaagctaaagtgccaggtggtagaatttcaggccaagaagacaagagttttggcaaggaagggaatattgctctcatggtggcgcccttgaaatcttcccatgtgtacggttccctagtacagtgacacagaagtgacagaagtgacagaactgacagcccagagacatgtttgagtctggcaagggatcgatcctagccatgccatgccatgcctcagctgccaccaccaatcagggatgtcagatctcaaccacaaaggacactgacatgcttgtcgctccccttgcacggcctctgtctgctcacctctgcccacacctccaggtcctagaggttccttgccctctggggagccccaaacctcctactacccctgcctcccagtaatgagctctagatctgtgctgcccagtataggagccgccagtcatacacgactattgggtaccagaaacatctctcacccaaacggagtttgctatcagtgtaaaatttcatgccacactgcacattgaagacaacagggaaaaagaatgtaaaaaatctcgtaaacacttgtatcttgattacatgttgaaataataacatttggggtatgtttagtcaaagaaaatatactattaaaattaacgtcacctgtttctatttgttttaatgtggttactagaaaattttaaattgtacttgtggctcccattttatttctttggacagtgtgaccctggatgaagggcccaggctctccctcaactgcaaaggggcagaataagcagtctgccattagcatctccaacctcctttttctaaatgtatttctctttccaactccctactcccctcaagcttccaccctccccagtcaagaccttttcttagccaaggacctagagctcattcacatgaaggaataagggtctggtaatagctgaaaatgttctcattcccactctctccaataggaagacatcctcatgggctggggacaccagagactctctccaaagggaaggtgtcctgctgggttgggggttgggggtcggggggtgggggagttgaggcaggttgtacctctaatcaaggggcctaaaatgggggagggatcccagaatacctccagagccaggggccaaaactaggtaagtccctgggctccaaatagcaaggggcagactcaaggagcttccgaattctgtctcatcaccccgtctaacccagccaccctacagaggtaggagggacaaactccactttcccccgccacaatctcctcccttgcctccccc

SEQ ID NO: 19347 - RNA, 786 nt, Homo sapiens
  source 1..786: mol_type = other RNA
ttaggcttccccctcctcctgcaggcccagggccaggccctcaaagaccgagtgggccgacagcgcgaaggccaggctgagcaggcgcacggggctggcgcgcgagaggccctgcacgctcaggctggggccgtggccgtggggctccacgtacagcgcgtggccccgcgcgccccccatgaaggggctctcatactccgagtcgctgcccacgtccgatccggcgttgaaggtctccaggtcgatgaaggacggcttctccttgcggaaggtcaggatcagctgctccaggaagacggtcatgaagaagcccagcaggaggatggtttcggccagcgggtagtcggtgctgatgtggccgaggctcaggaccttctggagcttttccctcacagcgggcagcagagcgttgaagcacgtggccagaaacacccctcctccaaaggtgttgcagagagagaggatctttttcgagcgatgggccttctcaaaatctgtctcgatgatcttcacggggagcagggagccgagcagcatgaagaagaacacgcccaccatgcacaggattttggccactagcaatttcaccatggtggcggcttgggctgctctggtcactgcagggccaaaccatctgtgggcgcacacccaagtcccacgatgtgctaccgagcccaaccacacagttggaggctcatgtctcagtccagcaactcccgggggcccctcgtccgccgactggcgccgctgcacgcccaacggccgcgcagtctcgaccccacagac

SEQ ID NO: 19348 - RNA, 1554 nt, Homo sapiens
  source 1..1554: mol_type = other RNA
ttaggcttccccctcctcctgcccctgagcccccaaaagaggagtttttttaaaaaacggaaaaagcagtgtttcagggaatctgttacaagtgagcgactgaaactgagaaaaaggagaggcaaggagaccagaggtcaccctgagggcgcacgtggggtctgtctgtcctgcttagatctcccctctccctgaaaggaagcaggtgccgagagccggggaggccttcccgggggcatcagcacagtgagatccgcccgctggagagggtagaatggttgtatcttgctgaatgactgaagagtgagtctgagttttgttttcagcggtattattatttgtgagtctaacctagcgggtggtcctggctgtcaccggtgcttgggcgggatcaccaccagcggctgcccgtacttgggccgccacatgaggacctgggcatcgttggcattgggcttgaccagggcgctgggcgggatgggctcattcttgctcaggattttgggctggtcctgggcgatgggctcccgcagccgggcgcgctggcccaggggccggttggggttcacctcgatgctgagctgcatgcgccagtgcagcgtctgcaggatgatcatgtcgttggtggaggtgttggtggccaccagccaggtggtgaagctctggtcccggtagatattggtgagcttggccacgttgctctcgctgacgggcacggcccatgtgacgctggggtaaaagttgtcattcatgctgatgatgaacttggagtccctcttggtggggcccacgatggtgcaggtctctgtggtgttgccgtaccaggggtagttcaccccatccgagtcgctgatggcttggatcttgccctcctggaggtcggggagctcccagctggacatgccctgctcgccgtactggttgtagaactccatgtggctgcacgcctggatccagccaactacccaagtctccttcttggggatgggcggcatgaccacctgggccgaggcccggaagtggggtgtccggtagcggagcaccacgctggaggactcatcgatgctagtggggacggggtcgatggaggctttcacatcaatcaccgtgatcccttcccggaagactctggctttgcctccgatgctctgaatacagcccatggcatacaggagcgctctgatctccagggaaggccagcagtcacagaaaaaaccaggcattgaaaggacagaggctgcaggacccagtacagacggcgctgctctccaatctcaactctcaagaccgatatccataggatagaaaactcactgagtagactggggttgcatatatcactaccgcggcctgtttataaataaggattctgctgcatttcatgagccctgggctctctcttcttctcctcgcagtggacaaaaatcaccgatattctttgggttaaaaaaagtttgtagtttaatgaataattatgcggttctgacatccagcccttctgtgcctcacacgcggggacggcagctcgcagactctccctgaagtcttcggagg

SEQ ID NO: 19349 - RNA, 1807 nt, Homo sapiens
  source 1..1807: mol_type = other RNA
ttaggcttccccctcctcctgcccctgagcccccaaaagaggagtttttttaaaaaacggaaaaagcagtgtttcagggaatctgttacaagtgagcgactgaaactgagaaaaaggagaggcaaggagaccagaggtcaccctgagggcgcacgtggggtctgtctgtcctgcttagatctcccctctccctgaaaggaagcaggtgccgagagccggggaggccttcccgggggcatcagcacagtgagatccgcccgctggagagggtagaatggttgtatcttgctgaatgactgaagagtgagtctgagttttgttttcagcggtattattatttgtgagtctaacctagcgggtggtcctggctgtcaccggtgcttgggcgggatcaccaccagcggctgcccgtacttgggccgccacatgaggacctgggcatcgttggcattgggcttgaccagggcgctgggcgggatgggctcattcttgctcaggattttgggctggtcctgggcgatgggctcccgcagccgggcgcgctggcccaggggccggttggggttcacctcgatgctgagctgcatgcgccagtgcagcgtctgcaggatgatcatgtcgttggtggaggtgttggtggccaccagccaggtggtgaagctctggtcccggtagatattggtgagcttggccacgttgctctcgctgacgggcacggcccatgtgacgctggggtaaaagttgtcattcatgctgatgatgaacttggagtccctcttggtggggcccacgatggtgcaggtctctgtggtgttgccgtaccaggggtagttcaccccatccgagtcgctgatggcttggatcttgccctcctggaggtcggggagctcccagctggaccagcattccttgcagtatagggaccttgttttcagtggccaccagagacagtcccaaggctctttctctctcatggaccactctgcattcagagtttcagcgggtcctccaagggcttgccaccttcaaggctggggtcatcagaggccaaaaaggaatctcaagagagggaaaagtttttgttctgcagatggaaatgttcggtgctggaattctgttgccctgggagacagcgttctctccccaactgttggggaccagaccgaaagccaatgacgaagcttggaatgtccaccagggaggtgggtggggccaaagagccaaacaggtgtctgaaggtgggagacattgagaggctaggtggcagatggaggcgtagggcatgtctgcatccctgacctgcctaactgggacagggggcaggctgagcctggccaggggagtagggacaagatctcagagagagctggtccagcagcctcccctacaggtggggaacagaggcccagtgaagtcctccagggaggcttccttcactagaacccgggtcttctggccctgcactcagtgagagcgtcactctccactgagggccatggtgccgcatgggtatggcagggcatgggacaagggattgaaaccgctgcctgtgctggctgcaaatctggaggctggggccttttcagccgaagctcagaaccacatggcttatagggcaagttaggcttggggcacctgcccactgttccagctcattccttccccagtgtggaccggacacgtccgccgggccaggcactgagaagatatagcggaggagtcacagccaggcccagacaacagcactcacatccccttccctgagatgtcggggataatgccaggagccatgaatgagggtattgat

SEQ ID NO: 19350 - RNA, 1106 nt, Homo sapiens
  source 1..1106: mol_type = other RNA
ttaggcttccccctcctcctgcccctgagcccccaaaagaggagtttttttaaaaaacggaaaaagcagtgtttcagggaatctgttacaagtgagcgactgaaactgagaaaaaggagaggcaaggagaccagaggtcaccctgagggcgcacgtggggtctgtctgtcctgcttagatctcccctctccctgaaaggaagcaggtgccgagagccggggaggccttcccgggggcatcagcacagtgagatccgcccgctggagagggtagaatggttgtatcttgctgaatgactgaagagtgagtctgagttttgttttcagcggtattattatttgtgagtctaacctagcgggtggtcctggctgtcaccggtgcttgggcgggatcaccaccagcggctgcccgtacttgggccgccacatgaggacctgggcatcgttggcattgggcttgaccagggcgctgggcgggatgggctcattcttgctcaggattttgggctggtcctgggcgatgggctcccgcagccgggcgcgctggcccaggggccggttggggttcacctcgatgctgagctgcatgcgccagtgcagcgtctgcaggatgatcatgtcgttggtggaggtgttggtggccaccagccaggtggtgaagctctggtcccggtagatattggtgagcttggccacgttgctctcgctgacgggcacggcccatgtgacgctggggtaaaagttgtcattcatgctgatgatgaacttggagtccctcttggtggggcccacgatggtgcaggtctctgtggtgttgccgtaccaggggtagttcaccccatccgagtcgctgatggcttggatcttgccctcctggaggtcggggagctcccagctggactgcctggtgcagccaacagcagtcagtggaagcttctggagaccctgcctcaactgtcctcccacaaacaacaggtgaagacgcttccttcccccaaacactgggcacgactgatctttttcaatgcacccaactccaatcagcaaaacaaaggatatcagtatgtaacttgtcatttccctgattactacggctgttgagtgacg

SEQ ID NO: 19351 - RNA, 88 nt, Homo sapiens
  source 1..88: mol_type = other RNA
ttaggcttccccctcctcctgccgcctggcctggaggcaagcaggccagggggcaggaggagggggaagcctaagaagaaccaaaggc

SEQ ID NO: 19352 - RNA, 34 nt, Homo sapiens
  source 1..34: mol_type = other RNA
ttaggcttccccctcctcctgcgcaacctaacct

SEQ ID NO: 19353 - RNA, 170 nt, Homo sapiens
  source 1..170: mol_type = other RNA
ttaggcttccccctcctcctgctccgggcagcagcggcctccccccgggtgcgcgcgcatccagccccctccccagccggcgctgcgcttcttccgtaaccgagcccttggaatcccggagacccgccccgcccgcagcgcggcgcgcgggggacgcgcgcaagcatcat

SEQ ID NO: 19354 - RNA, 174 nt, Homo sapiens
  source 1..174: mol_type = other RNA
ttaggcttccccctcctcctgctccgtctccccttttctcaatgagaactgggagggagctggcagggctgcggttgctcctcaccaaggctgtggctgcggctgcttccagtgcccgccggtcacattcagcaggtgcagtcacaacaggatgaggggaggagggagaatgcc

SEQ ID NO: 19355 - RNA, 1391 nt, Homo sapiens
  source 1..1391: mol_type = other RNA
ttaggcttccccctcctcctgctccgtgctctcactggctgcccgctgccgctggaagtggtgccgcttgggggaacctctcgtgtccagactggctgcccgctggctgggctccagcttccacttcttgaccttgaaataggggctggccccatccaggctggcatggcggcgcaggcgggtgaggaactgcagaacggtacctgccccggatcccgggcccgcctccccaggccctgctgcagccccgggccctccagccttggtgctcctggtaccggcatccaacgaggtgccttccccagagtcgctagatgccgaggggctgatctctgcgaagtcagtggcgcccgcggctgagttgtaggggtcacctggcagggcggagctggaagatggccagagtggccttgggagaggtggccgggtggggcgtggtggctgagctggcctcgcctgagtcacactcgtggatggtgacaatcttgaggggcggcaggtgcaggtgcgtgagccgggcattcttcaggtggtggaagtccccctccgtcagtgtgtaccggcgacccttgtcctgcgtcttgcggctctgctcaaacagcgccgcctcattgaaggagacccggcggcccgtggagctggtggacaggaagcgttcggtctccgcatcctggcactcggggtcctctccccggaagtcggggtcttgggctgggtgggtgccgttgtccaggtaggtggtggtggtcttctccgcttcctccatggccctgttgaggcgctggtggacgtcccagcagcgcttgcagaggagcaggacgccagacaacaccaccagcgtgccccccacgaacagcgacatcaccaccaccagcagcacgtagttgtccaggatggggtctggctctgccgtggggcgtccagtggcattgtcccacgacgtcgtcagggctactgtggcagtggtggtggtggtggtggtggcggctgtggccatggtggctgtgggctgcattctgaactggggaggagggccctcgcccggtcctgaggtcccagggacgcagctgggggtgtcctggaattcacgactctgcagcccgaggtgcgccgcgtgcgcaggagggggtggggtccgggggggcacggactcccctctcacgttgcttggtccgtgggggttctggggcggcacagccagggcccctcggccacaattcccctttaagctgcacagcccagggtctctggacacaggcgccccgcctgcttccccacgcaggtcccctctggcactgtggaggactcgccatgcctctcctgccccctcccctgtgtgacagcgatcacagaccccggcacaaagctgagcagagcccatcggggcccaa

SEQ ID NO: 19356 - RNA, 1734 nt, Homo sapiens
  source 1..1734: mol_type = other RNA
ttaggcttccccctcctcctgctccgtgctctcactggctgcccgctgccgctggaagtggtgccgcttgggggaacctctcgtgtccagactggctgcccgctggctgggctccagcttccacttcttgaccttgaaataggggctggccccatccaggctggcatggcggcgcaggcgggtgaggaactgcagaacggtacctgccccggatcccgggcccgcctccccaggccctgctgcagccccgggccctccagccttggtgctcctggtaccggcatccaacgaggtgccttccccagagtcgctagatgccgaggggctgatctctgcgaagtcagtggcgcccgcggctgagttgtaggggtcacctggcagggcggagctggaagatggccagagtggccttgggagaggtggccgggtggggcgtggtggctgagctggcctcgcctgagtcacactcgtggatggtgacaatcttgaggggcggcaggtgcaggtgcgtgagccgggcattcttcaggtggtggaagtccccctccgtcagtgtgtaccggcgacccttgtcctgcgtcttgcggctctgctcaaacagcgccgcctcattgaaggagacccggcggcccgtggagctggtggacaggaagcgttcggtctccgcatcctggcactcggggtcctctccccggaagtcggggtcttgggctgggtgggtgccgttgtccaggtaggtggtggtggtcttctccgcttcctccatggccctgttgaggcgctggtggacgtcccagcagcgcttgcagaggagcaggacgccagacaacaccaccagcgtgccccccacgaacagcgacatcaccaccaccagcagcacgtagttgtccaggatggggtctggctctgccgtggggcgtccagtggcattgtcccacgacgtcgtcagggctactgtggcagtggtggtggtggtggtggtggcggctgtggccatggtggctgtgggctgcattctgaactggggaggagggccctgtggggaggaagcctggtcagctccagctagacctacttctcctgcaggagccactgcagacaagctgggtcttccctgcaggagcaggagcccacacagggggcagtgactcatggagaggtagcagagccggaggcagcctccacccggcttggctctgcccagcgggccccgggggctctctctggacctccatctcccatccccatggcgggggaggaggcctggccctctgagggtgcgcctgtacccatcacaactgcacacagccggtgcggcctgtcctgcaaggtagcgccaggccctggagctcagcgctgggcagggcaagcactcggaggaatggggacgccaaggcggtgcagccggctcgagaaggactccagacgccctgtccgccccatcacgggggtggggggctacccccaccccaagaagttcagctacaccctggcagggcccacccggccatggttgggtagagggagacctcccgctgcctgcgcgccagggagggtgcaggggctgggcgcgtgctcccgggtcacgactccgggaggtggaggtctccccggtgctgagtgctggtgggagtgcaagggacaaagaaggcgcatctgttcccagccccggagaagctggttcccatggcgactgcggagcaggccgcggctgggggggcgggttgccaggga

SEQ ID NO: 19357 - RNA, 877 nt, Homo sapiens
  source 1..877: mol_type = other RNA
ttaggcttccccctcctcctgctccgtgctctcactggctgcccgctgccgctggaagtggtgccgcttgggggaacctctcgtgtccagactggctgcccgctggctgggctccagcttccacttcttgaccttgaaataggggctggccccatccaggctggcatggcggcgcaggcgggtgaggaactgcagaacggtacctgccccggatcccgggcccgcctccccaggccctgctgcagccccgggccctccagccttggtgctcctggtaccggcatccaacgaggtgccttccccagagtcgctagatgccgaggggctgatctctgcgaagtcagtggcgcccgcggctgagttgtaggggtcacctggcagggcggagctggaagatggccagagtggccttgggagaggtggccgggtggggcgtggtggctgagctggcctcgcctgagtcacactcgtggatggtgacaatcttgaggggcggcaggtgcaggtgcgtgagccgggcattcttcaggtggtggaagtccccctccgtcagtgtgtaccggcgacccttgtcctgcgtcttgcggctctgctcaaacagcgccgcctcattgaaggagacccggcggcccgtggagctggtggacaggaagcgttcggtctccgcatcctggcactcggggtcctctccccggaagtcggggttcgctcagcacgcgcctgggcccacctacgcctgggcgttaaggaaacagagatgagtcggaatcgagctgcgcccagtcttgggctgggtgggtgccgttgtccaggtaggtggtggtggtcttctccgcttcctccatggccctgttgaggcgctggtggacgtcccagc

SEQ ID NO: 19358 - RNA, 1287 nt, Homo sapiens
  source 1..1287: mol_type = other RNA
ttaggcttccccctcctcctgctccgtgctctcactggctgcccgctgccgctggaagtggtgccgcttgggggaacctctcgtgtccagactggctgcccgctggctgggctccagcttccacttcttgaccttgaaataggggctggccccatccaggctggcatggcggcgcaggcgggtgaggaactgcagaacggtacctgccccggatcccgggcccgcctccccaggccctgctgcagccccgggccctccagccttggtgctcctggtaccggcatccaacgaggtgccttccccagagtcgctagatgccgaggggctgatctctgcgaagtcagtggcgcccgcggctgagttgtaggggtcacctggcagggcggagctggggcccacagagcggccggtgagggccttccccgggggctggaagatggccagagtggccttgggagaggtggccgggtggggcgtggtggctgagctggcctcgcctgagtcacactcgtggatggtgacaatcttgaggggcggcaggtgcaggtgcgtgagccgggcattcttcaggtggtggaagtccccctccgtcagtgtgtaccggcgacccttgtcctgcgtcttgcggctctgctcaaacagcgccgcctcattgaaggagacccggcggcccgtggagctggtggacaggaagcgttcggtctccgcatcctggcactcggggtcctctccccggaagtcggggtcttgggctgggtgggtgccgttgtccaggtaggtggtggtggtcttctccgcttcctccatggccctgttgaggcgctggtggacgtcccagcagcgcttgcagaggagcaggacgccagacaacaccaccagcgtgccccccacgaacagcgacatcaccaccaccagcagcacgtagttgtccaggatggggtctggctctgccgtggggcgtccagtggcattgtcccacgacgtcgtcagggctactgtggcagtggtggtggtggtggtggtggcggctgtggccatggtggctgtgggctgcattctgaactggggaggagggccctcagcgccgggacgagcggcccatgggcggcgggctggcggcgggcggctgcgtggcgctcgcggctggctccggcgcccggtggccgcggagcaggcggagaatttatgaatggagagcgcggcgcgggggaggccggcgcgagaggaggggccgcgcacgtgaccgcgttggcggcgcgcccgctccgcgcgcccggtgctgcccgg

SEQ ID NO: 19359 - RNA, 1327 nt, Homo sapiens
  source 1..1327: mol_type = other RNA
ttaggcttccccctcctcctgctccgtgctctcactggctgcccgctgccgctggaagtggtgccgcttgggggaacctctcgtgtccagactggctgcccgctggctgggctccagcttccacttcttgaccttgaaataggggctggccccatccaggctggcatggcggcgcaggcgggtgaggaactgcagaacggtacctgccccggatcccgggcccgcctccccaggccctgctgcagccccgggccctccagccttggtgctcctggtaccggcatccaacgaggtgccttccccagagtcgctagatgccgaggggctgatctctgcgaagtcagtggcgcccgcggctgagttgtaggggtcacctggcagggcggagctggggcccacagagcggccggtgagggccttccccgggggctggaagatggccagagtggccttgggagaggtggccgggtggggcgtggtggctgagctggcctcgcctgagtcacactcgtggatggtgacaatcttgaggggcggcaggtgcaggtgcgtgagccgggcattcttcaggtggtggaagtccccctccgtcagtgtgtaccggcgacccttgtcctgcgtcttgcggctctgctcaaacagcgccgcctcattgaaggagacccggcggcccgtggagctggtggacaggaagcgttcggtctccgcatcctggcactcggggtcctctccccggaagtcggggtcttgggctgggtgggtgccgttgtccaggtaggtggtggtggtcttctccgcttcctccatggccctgttgaggcgctggtggacgtcccagcagcgcttgcagaggagcaggacgccagacaacaccaccagcgtgccccccacgaacagcgacatcaccaccaccagcagcacgtagttgtccaggatggggtctggctctgccgtggggcgtccagtggcattgtcccacgacgtcgtcagggctactgtggcagtggtggtggtggtggtggtggcggctgtggccatggtggctgtgggctgcattctgaactggggaggagggccctcagcgccgggacgagcggcccatgggcggcgggctggcggcgggcggctgcgtggcgctcgcggctggctccggcgcccggtggccgcggagcaggcggagaatttatgaatggagagcgcggcgcgggggaggccggcgcgagaggaggggccgcgcacgtgaccgcgttggcggcgcgcccgctccgcgcgcccggtgctgcccggtccccggcccgccgcccccgctgcgctcgccgctgggtct

SEQ ID NO: 19360 - RNA, 1432 nt, Homo sapiens
  source 1..1432: mol_type = other RNA
ttaggcttccccctcctcctgctccgtgctctcactggctgcccgctgccgctggaagtggtgccgcttgggggaacctctcgtgtccagactggctgcccgctggctgggctccagcttccacttcttgaccttgaaataggggctggccccatccaggctggcatggcggcgcaggcgggtgaggaactgcagaacggtacctgccccggatcccgggcccgcctccccaggccctgctgcagccccgggccctccagccttggtgctcctggtaccggcatccaacgaggtgccttccccagagtcgctagatgccgaggggctgatctctgcgaagtcagtggcgcccgcggctgagttgtaggggtcacctggcagggcggagctggggcccacagagcggccggtgagggccttccccgggggctggaagatggccagagtggccttgggagaggtggccgggtggggcgtggtggctgagctggcctcgcctgagtcacactcgtggatggtgacaatcttgaggggcggcaggtgcaggtgcgtgagccgggcattcttcaggtggtggaagtccccctccgtcagtgtgtaccggcgacccttgtcctgcgtcttgcggctctgctcaaacagcgccgcctcattgaaggagacccggcggcccgtggagctggtggacaggaagcgttcggtctccgcatcctggcactcggggtcctctccccggaagtcggggtcttgggctgggtgggtgccgttgtccaggtaggtggtggtggtcttctccgcttcctccatggccctgttgaggcgctggtggacgtcccagcagcgcttgcagaggagcaggacgccagacaacaccaccagcgtgccccccacgaacagcgacatcaccaccaccagcagcacgtagttgtccaggatggggtctggctctgccgtggggcgtccagtggcattgtcccacgacgtcgtcagggctactgtggcagtggtggtggtggtggtggtggcggctgtggccatggtggctgtgggctgcattctgaactggggaggagggccctcgcccggtcctgaggtcccagggacgcagctgggggtgtcctggaattcacgactctgcagcccgaggtgcgccgcgtgcgcaggagggggtggggtccgggggggcacggactcccctctcacgttgcttggtccgtgggggttctggggcggcacagccagggcccctcggccacaattcccctttaagctgcacagcccagggtctctggacacaggcgccccgcctgcttccccacgcaggtcccctctggcactgtggaggactcgccatgcctctcctgccccctcccctgtgtgacagcgatcacagaccccggcacaaagctgagcagagcccatcggggcccaa

SEQ ID NO: 19361 - RNA, 358 nt, Homo sapiens
  source 1..358: mol_type = other RNA
ttaggcttccccctcctcctgctcctgcgtcggctcgcctgccgtccgccgccgcccgccgcccgccgggctgggcgctgggccgggctagcggcgcgcctggggccggcaggagcgccgcctggctgcctgcgcggagccaagctgctcgcggcgccccgcgcgcgcccctgcccgccgcccgcgctcctcgccgtcccggcttcgctgctgccgcccgagccgccgccgccgccagcagcaggagcagcagcggccgccgcggcgctcctcggacctgcacattcctctcctcccctcgcgcgcgctccctcctcccgcttcctctcctccaccagctgactccgagggagaggat

SEQ ID NO: 19362 - RNA, 57 nt, Homo sapiens
  source 1..57: mol_type = other RNA
ttatggtttgcctgggactgaggcaaccagaaggagcaggaaagccctgatgaaatc

SEQ ID NO: 19363 - RNA, 1791 nt, Homo sapiens
  source 1..1791: mol_type = other RNA
ttatggtttgcctgggactgaggcgattcctgggatgcagaactttcagctttaaagccaatatagtctcagacaaatcatgatggattggtcacattgtgtatgcattggtctgtgtggcaggcataataacagccacccaaagacgtccaaattctaatttctggaatctgcaagtatgtcaccttataggccaagacggactttgcagatgtgattaagtaaaggattttgaaatggggagattatcctgtactacaattgtccttataagggaaagaaagaagagggtgagagtcagaaaagggagacgtgctatggttgcagaggttagagtgatgcagttgctggaagtgccccacagccaaagcaagcaggtgacttccaggaactggagaaggcatggaacagattctccccaagggccttccaaaggaacacagcccttctgacatcttgatttgagctccatgagacccattttgggctctgacctccagaactttaagacaacaaatgtgtgttgttttaagccactaaatttatggtaatttgttacagcagcaatagcagactaatacactctgctttccaaaaaatcccccaaagacttgaatgcaggttgctttgctgcctttctattgccccagggcagattctggtttctcccaaaataccattcctttattaatgaaggaggcagtgtgggaagtgttgagagcacattgaaaagcaaccatttactgatcatccaggttaagctggagcactagagtgggaattcagatgcttcagctgcatgtctggctctgcctttccttgctctgtcagcttggtctacctctctggaatctctggttcttacttatctctaaaatgaactaaataacatagaattatcatctcaaatttataaactttggtaacattcttaagtgatcatgcattcgtaatgtgtttgtgactgactccagagcatatgcatttttggggggtgacatcacacccaagaggattaaaatggattcttggatggggggctcttactgtttctgtgttttagaaacagatgtacagatgatacataaccgaatacacagtatacctgtggtatggaaggttcatggggtggtgacaaggaaaagtgtccaacacgtctccttccgggagtgctaatggcaaagaaaaaggctgagaatcatttgtctagttattgcaccacctgttgctatttgataacgtgttttaaagggcatgggaaagatgatgaagcagaggaatctcaggaactttctggagtcagatgaatataaatccaattcttcacgtggttgtagatctgtaccactctgagatcagtctctttatatttcagtgttatttaccagcaggaaaagacgattttgactgattgagttgaatgtgctgagttgatggtgagttcaatatggctgtaaagctcggtactgtcctggtcattgtgccttccgggagagggagaacgactgtgagttcctgagcccaaaggtgatcttttcttgctttgtagttctgaggagactgcacctggacaagttgtagaaatttgggctgtgcggtatgagatgcatgtatgcagactaaaaggcattcagccaacggatctgcatttggtaagagccggggattgggacgaggcagagagcaagaccaagctggtttcctctccggtttcctccggggtggctgggtcccaggtcctgcccccgcctcgccctgtgcaagctcggtgcagtgcagcccctccggctc

SEQ ID NO: 19364 - RNA, 1946 nt, Homo sapiens
  source 1..1946: mol_type = other RNA
ttatggtttgcctgggactgaggcgattcctgggatgcagaactttcagctttaaagccaatatagtctcagacaaatcatgatggattggtcacattgtgtatgcattggtctgtgtggcaggcataataacagccacccaaagacgtccaaattctaatttctggaatctgcaagtatgtcaccttataggccaagacggactttgcagatgtgattaagtaaaggattttgaaatggggagattatcctgtactacaattgtccttataagggaaagaaagaagagggtgagagtcagaaaagggagacgtgctatggttgcagaggttagagtgatgcagttgctggaagtgccccacagccaaagcaagcaggtgacttccaggaactggagaaggcatggaacagattctccccaagggccttccaaaggaacacagcccttctgacatcttgatttgagctccatgagacccattttgggctctgacctccagaactttaagacaacaaatgtgtgttgttttaagccactaaatttatggtaatttgttacagcagcaatagcagactaatacactctgctttccaaaaaatcccccaaagacttgaatgcaggttgctttgctgcctttctattgccccagggcagattctggtttctcccaaaataccattcctttattaatgaaggaggcagtgtgggaagtgttgagagcacattgaaaagcaaccatttactgatcatccaggttaagctggagcactagagtgggaattcagatgcttcagctgcatgtctggctctgcctttccttgctctgtcagcttggtctacctctctggaatctctggttcttacttatctctaaaatgaactaaataacatagaattatcatctcaaatttataaactttggtaacattcttaagtgatcatgcattcgtaatgtgtttgtgactgactccagagcatatgcatttttggggggtgacatcacacccaagaggattaaaatggattcttggatggggggctcttactgtttctgtgttttagaaacagatgtacagatgatacataaccgaatacacagtatacctgtggtatggaaggttcatggggtggtgacaaggaaaagtgtccaacacgtctccttccgggagtgctaatggcaaagaaaaaggctgagaatcatttgtctagttattgcaccacctgttgctatttgataacgtgttttaaagggcatgggaaagatgatgaagcagaggaatctcaggaactttctggagtcagatgaatataaatccaattcttcacgtggttgtagatctgtaccactctgagatcagtctctttatcttccatcaggccatggtccaaatgcagggggagctgagggttcagcatggaggtcgttccaccgggtctgcttgtgttacgatcaatttgtcttcagagacagcgcccgtgcttccagagacagactttgttcttaccatcccatcttcccacaatttcagtgttatttaccagcaggaaaagacgattttgactgattgagttgaatgtgctgagttgatggtgagttcaatatggctgtaaagctcggtactgtcctggtcattgtgccttccgggagagggagaacgactgtgagttcctgagcccaaaggtgatcttttcttgctttgtagttctgaggagactgcacctggacaagttgtagaaatttgggctgtgcggtatgagatgcatgtatgcagactaaaaggcattcagccaacggatctgcatttggtaagagccggggattgggacgaggcagagagcaagaccaagctggtttcctctccggtttcctccggggtggctgggtcccaggtcctgcccccgcctcgccctgtgcaagctcggtgcagtgcagcccctccggctc

SEQ ID NO: 19365 - RNA, 72 nt, Homo sapiens
  source 1..72: mol_type = other RNA
ttattcattcacaaaagctttactgagtatataaataaagcttttgtgaatgaataaataagcgaatgtatt

SEQ ID NO: 19366 - RNA, 825 nt, Homo sapiens
  source 1..825: mol_type = other RNA
ttcaacgggtatttattgagcaactactatctgccaagccctgggataaagcattgaatgagacagacgcagcccttaccctgccctttaaagagctccagtagacccaccctcttcccacagcactgttatcacacatcacacagatatacgacagacactgccgcgcacacaaaggaggccagattctgaaagaaggaccgattgctcatcgttaactgattcaaagttgggcttgagtaagctagctgaggtgggcaaggaggctggcaaacccccgcaacccctcaagggcaggagtagggttcaagaggttggtctcggaggcagacggcctggatccaaatcctggttgcatcgctgatgagctgtaaggtccttcaggtcttgaagcctcaggttaggccttttgcaaactggggatagcaggacctgctcatgggccactgggctctgggcacgctggcttgtgacctctggctggccctggactatgtggccagcaatgcctccgtcatgaatctgctgctcatcagctttgaccgctacttctccgtgactcggcccctgagctaccgtgccaagcgcacaccccgccgggcagctctgatgatcggcctggcctggctggtttcctttgtgctctgggccccagccatcctcttctggcagtacctggcttcccaggaccctgggtcaccttcctgggcagcccagagagaccctgccaactttccagacttcgctattcccaggcagggagggaaacccggggaactggtttttctgttccctgctgggtgggaatgcgctcttcaccaggaa

SEQ ID NO: 19367 - RNA, 688 nt, Homo sapiens
  source 1..688: mol_type = other RNA
ttcaacgggtatttattgagcatatgttgtatgccctcaacattttaagaactgtacttggacgtgcacgcaccctgtccctcaaccaccgctgccgcctccttcttctgtcactcctggtgctgcactgtgttcgttcagtgagaagctggtacctcttttgtgaagcggcagctgagaagactctggcatttgccatggccgaggaaaagcccaaggcattgtcaatggggcagatcagattccgatttgacagtcagccaatcaatgaaacagacacaccttgttcagttggagaattttaatgtttttcacttatccttgttaaaccaatgataattttataacttttttgtatgcagctgttacacgtagggcaatctctctgtaagtagggataaattactctaaagttgctgtctggtgtgagctgcacatcatacagtagtttctgctcatttttcctttctcatataatgaatcaataagtcttcatcataaaggaatgcaccaaggtgaactgtgggttccggctgctgctgcatacttacggttagttcgcatccactgtaacagcgcctggcggtcggcaggagccacagtgcgaagcggccgcagcatcactgcctgcctcgcagtgggaaattttaccttgctggagcaagccgcgcaggcactggctggcatt

SEQ ID NO: 19368 - RNA, 1226 nt, Homo sapiens
  source 1..1226: mol_type = other RNA
ttcacagtggctaagttccgcatgtcccatatggtctctaccagaggaatactgccgacctgccagtcatagcacagggtcacgggtgcaagcagaagccacacattgaaggccaagaggtaggaataggtgaggaatctcatcatggaccacacagctcgtggggacactgggaatccactgctcttgggttctggtggcagtggagagtggcagccaccccaagctcctttgtgagggaaccgctgctgcttcccattctcccggtgaggatggcctggcagtgaggagggctgggggctcccgggctgctgtgggctgcgtggacagagggccccattgctcgacttgtcttgcttgttggaaagggaaaagaggtcataaaccaagcacactccaaacaccgtgatgcctgtctctttcaccagcatcgcacaggtccccagaaacaaactgagcagcaagaagaagggagacaccgtggaagggaaacttcccccaacacagccctgatccagactcctgttgtacgagagaaaggccaatagaaacagcagacacgctaacacgtccgctctgccaacgatcccagccaccgcctcagtatgaataggatgtacagcaaaaagcaatgccgttacaaaagcaagtccacgattcttgaagacagttttatcacaggtgtacatcagcacaagagtcactaagcagtgtaaaattatatttactgcatgaaagtagaatgggttcataccagtcaaaaatatgtttagccttccagggagaaaagtgccgctgcttcccgggaagttcccggcttttcagcacccgggacaacagcagcggcgcccggagagacgctctccacccgccccgcgctcgcgtccagtcgccggctctgtgctctcctgcccgggctttctctcacccgcccggcgcggcgtcccgcttggcggaggaacccgcggggatagggagcaccttcctcaaagccaggagaaggggtctccctggacaaggacatcctgctcgccctgcccgggtgtgttcagaggcgccaccggctctttaactttacagcccctttcttggcccgcacttacaaaaagtaccaggttcgagttttggtttgggcctgggagccgaattgtcttctgaaacatttcttattttattgtttgctcaagataatttgggagatgccaagcaaactactttttctatct

SEQ ID NO: 19369 - RNA, 1267 nt, Homo sapiens
  source 1..1267: mol_type = other RNA
ttcacagtggctaagttccgcatgtcccatatggtctctaccagaggaatactgccgacctgccagtcatagcacagggtcacgggtgcaagcagaagccacacattgaaggccaagaggtaggaataggtgaggaatctcatcatggaccacacagctcgtggggacactgggaatccactgctcttgggttctggtggcagtggagagtggcagccaccccaagctcctttgtgagggaaccgctgctgcttcccattctcccggtgaggatggcctggcagtgaggagggctgggggctcccgggctgctgtgggctgcgtggacagagggccccattgctcgacttgtcttgcttgttggaaagggaaaagaggtcataaaccaagcacactccaaacaccgtgatgcctgtctctttcaccagcatcgcacaggtccccagaaacaaactgagcagcaagaagaagggagacaccgtggaagggaaacttcccccaacacagccctgatccagactcctgttgtacgagagaaaggccaatagaaacagcagacacgctaacacgtccgctctgccaacgatcccagccaccgcctcagtatgaataggatgtacagcaaaaagcaatgccgttacaaaagcaagtccacgattcttgaagacagttttatcacaggtgtacatcagcacaagagtcactaagcagtgtaaaattatatttactgcatgaaagtagaatgggttcataccagtcaaaaatatgtttagcttgaaggtgaggacgcagagcggccggtaggacttgtggctggtgttctcggccatgcccttgccccagaagtcgttggtgaagatgccccagcggagcggggcgccgggccgcacgtcggggttgttcacgatcgcccacacgtcgtcgtgcacgaactcgccctgcagggagcggccgtagcacaggcagcttgccccggccagcagcgccgcggccccggccggcgctagcccgcagccccgccgccgggagggtgtgcggtccccgccgccgcctcgggcagaggtggtcaccaccatcgcgccgccgccgccgctgctgccctggcctctcccgggcgtctggcatcctcccctaccggggccccggcggcgcgcggcgtctgcccggaggggggctcgggcatggtgctgcggcagctggacccgccgcgagctccccgcgctccgccgccgcctgcgccgcggagttggcccagctgcaaataaac

SEQ ID NO: 19370 - RNA, 414 nt, Homo sapiens
  source 1..414: mol_type = other RNA
ttcacagtggctaagttccgcatgtcccatatggtctctaccagaggaatactgccgacctgccagtcatagcacagggtcacgggtgcaagcagaagccacacattgaaggccaagaggtaggaataggtgaggaatctcgtaagaatgtaaggcgaaaatgaagctggattatcctgctctgaaaagaggggcatagatcctcccattatccacagacggaagtacaaaatgacaagcacataacttaggaccaaaatggccctttttaaaaatggtctcatggtaagcaggaaatttctattgctgcttgctctcagatacctacttaatataatttgaaggctccaatgtcttccatccacaaaatacctcacagatctcttacctctaaaaatagaagatgccaaggtt

SEQ ID NO: 19371 - RNA, 1388 nt, Homo sapiens
  source 1..1388: mol_type = other RNA
ttcacagtggctaagttccgcatgtcccatatggtctctaccagaggaatactgccgacctgccagtcatagcacagggtcacgggtgcaagcagaagccacacattgaaggccaagaggtaggaataggtgaggaatctcgtaagaatgtaaggcgaaaatgaagctggattatcctgctctgaaaagaggggcatagatcctcccattatccacagacggaagtacaaaatgacaagcacataacttaggaccaaaatggccctttttaaaaatggtctcatggtaagcaggaaatttctattgctgcttgctctcagatacctcatcatggaccacacagctcgtggggacactgggaatccactgctcttgggttctggtggcagtggagagtggcagccaccccaagctcctttgtgagggaaccgctgctgcttcccattctcccggtgaggatggcctggcagtgaggagggctgggggctcccgggctgctgtgggctgcgtggacagagggccccattgctcgacttgtcttgcttgttggaaagggaaaagaggtcataaaccaagcacactccaaacaccgtgatgcctgtctctttcaccagcatcgcacaggtccccagaaacaaactgagcagcaagaagaagggagacaccgtggaagggaaacttcccccaacacagccctgatccagactcctgttgtacgagagaaaggccaatagaaacagcagacacgctaacacgtccgctctgccaacgatcccagccaccgcctcagtatgaataggatgtacagcaaaaagcaatgccgttacaaaagcaagtccacgattcttgaagacagttttatcacaggtgtacatcagcacaagagtcactaagcagtgtaaaattatatttactgcatgaaagtagaatgggttcataccagtcaaaaatatgtttagcttgaaggtgaggacgcagagcggccggtaggacttgtggctggtgttctcggccatgcccttgccccagaagtcgttggtgaagatgccccagcggagcggggcgccgggccgcacgtcggggttgttcacgatcgcccacacgtcgtcgtgcacgaactcgccctgcagggagcggccgtagcacaggcagcttgccccggccagcagcgccgcggccccggccggcgctagcccgcagccccgccgccgggagggtgtgcggtccccgccgccgcctcgggcagaggtggtcaccaccatcgcgccgccgccgccgctgctgccctggcctctcccgggcgtctggcatcctcccctaccggggccccggcggcgcgcggcgtctgcccggaggggggctcgggcatggtgctgcggcagctggac

SEQ ID NO: 19372 - RNA, 1391 nt, Homo sapiens
  source 1..1391: mol_type = other RNA
ttcacagtggctaagttccgcatgtcccatatggtctctaccagaggaatactgccgacctgccagtcatagcacagggtcacgggtgcaagcagaagccacacattgaaggccaagaggtaggaataggtgaggaatctcgtaagaatgtaaggcgaaaatgaagctggattatcctgctctgaaaagaggggcatagatcctcccattatccacagacggaagtacaaaatgacaagcacataacttaggaccaaaatggccctttttaaaaatggtctcatggtaagcaggaaatttctattgctgcttgctctcagatacctcatcatggaccacacagctcgtggggacactgggaatccactgctcttgggttctggtggcagtggagagtggcagccaccccaagctcctttgtgagggaaccgctgctgcttcccattctcccggtgaggatggcctggcagtgaggagggctgggggctcccgggctgctgtgggctgcgtggacagagggccccattgctcgacttgtcttgcttgttggaaagggaaaagaggtcataaaccaagcacactccaaacaccgtgatgcctgtctctttcaccagcatcgcacaggtccccagaaacaaactgagcagcaagaagaagggagacaccgtggaagggaaacttcccccaacacagccctgatccagactcctgttgtacgagagaaaggccaatagaaacagcagacacgctaacacgtccgctctgccaacgatcccagccaccgcctcagtatgaataggatgtacagcaaaaagcaatgccgttacaaaagcaagtccacgattcttgaagacagttttatcacaggtgtacatcagcacaagagtcactaagcagtgtaaaattatatttactgcatgaaagtagaatgggttcataccagtcaaaaatatgtttagcttgaaggtgaggacgcagagcggccggtaggacttgtggctggtgttctcggccatgcccttgccccagaagtcgttggtgaagatgccccagcggagcggggcgccgggccgcacgtcggggttgttcacgatcgcccacacgtcgtcgtgcacgaactcgccctgcagggagcggccgtagcacaggcagcttgccccggccagcagcgccgcggccccggccggcgctagcccgcagccccgccgccgggagggtgtgcggtccccgccgccgcctcgggcagaggtggtcaccaccatcgcgccgccgccgccgctgctgccctggcctctcccgggcgtctggcatcctcccctaccggggccccggcggcgcgcggcgtctgcccggaggggggctcgggcatggtgctgcggcagctggacccg

SEQ ID NO: 19373 - RNA, 1453 nt, Homo sapiens
  source 1..1453: mol_type = other RNA
ttcacagtggctaagttccgcatgtcccatatggtctctaccagaggaatactgccgacctgccagtcatagcacagggtcacgggtgcaagcagaagccacacattgaaggccaagaggtaggaataggtgaggaatctcgtaagaatgtaaggcgaaaatgaagctggattatcctgctctgaaaagaggggcatagatcctcccattatccacagacggaagtacaaaatgacaagcacataacttaggaccaaaatggccctttttaaaaatggtctcatggtaagcaggaaatttctattgctgcttgctctcagatacctcatcatggaccacacagctcgtggggacactgggaatccactgctcttgggttctggtggcagtggagagtggcagccaccccaagctcctttgtgagggaaccgctgctgcttcccattctcccggtgaggatggcctggcagtgaggagggctgggggctcccgggctgctgtgggctgcgtggacagagggccccattgctcgacttgtcttgcttgttggaaagggaaaagaggtcataaaccaagcacactccaaacaccgtgatgcctgtctctttcaccagcatcgcacaggtccccagaaacaaactgagcagcaagaagaagggagacaccgtggaagggaaacttcccccaacacagccctgatccagactcctgttgtacgagagaaaggccaatagaaacagcagacacgctaacacgtccgctctgccaacgatcccagccaccgcctcagtatgaataggatgtacagcaaaaagcaatgccgttacaaaagcaagtccacgattcttgaagacagttttatcacaggtgtacatcagcacaagagtcactaagcagtgtaaaattatatttactgcatgaaagtagaatgggttcataccagtcaaaaatatgtttagcttgaaggtgaggacgcagagcggccggtaggacttgtggctggtgttctcggccatgcccttgccccagaagtcgttggtgaagatgccccagcggagcggggcgccgggccgcacgtcggggttgttcacgatcgcccacacgtcgtcgtgcacgaactcgccctgcagggagcggccgtagcacaggcagcttgccccggccagcagcgccgcggccccggccggcgctagcccgcagccccgccgccgggagggtgtgcggtccccgccgccgcctcgggcagaggtggtcaccaccatcgcgccgccgccgccgctgctgccctggcctctcccgggcgtctggcatcctcccctaccggggccccggcggcgcgcggcgtctgcccggaggggggctcgggcatggtgctgcggcagctggacccgccgcgagctccccgcgctccgccgccgcctgcgccgcggagttggcccagctgcaaataaac

SEQ ID NO: 19374 - RNA, 1180 nt, Homo sapiens
  source 1..1180: mol_type = other RNA
ttcacagtggctaagttccgcatgtcccatatggtctctaccagaggaatactgccgacctgccagtcatagcacagggtcacgggtgcaagcagaagccacacattgaaggccaagaggtaggaataggtgaggaatctcgtaagaatgtaaggcgaaaatgaagctggattatcctgctctgaaaagaggggcatagatcctcccattatccacagacggaagtacaaaatgacaagcacataacttaggaccaaaatggccctttttaaaaatggtctcatggtaagcaggaaatttctattgctgcttgctctcagatacgacttgtcttgcttgttggaaagggaaaagaggtcataaaccaagcacactccaaacaccgtgatgcctgtctctttcaccagcatcgcacaggtccccagaaacaaactgagcagcaagaagaagggagacaccgtggaagggaaacttcccccaacacagccctgatccagactcctgttgtacgagagaaaggccaatagaaacagcagacacgctaacacgtccgctctgccaacgatcccagccaccgcctcagtatgaataggatgtacagcaaaaagcaatgccgttacaaaagcaagtccacgattcttgaagacagttttatcacaggtgtacatcagcacaagagtcactaagcagtgtaaaattatatttactgcatgaaagtagaatgggttcataccagtcaaaaatatgtttagcttgaaggtgaggacgcagagcggccggtaggacttgtggctggtgttctcggccatgcccttgccccagaagtcgttggtgaagatgccccagcggagcggggcgccgggccgcacgtcggggttgttcacgatcgcccacacgtcgtcgtgcacgaactcgccctgcagggagcggccgtagcacaggcagcttgccccggccagcagcgccgcggccccggccggcgctagcccgcagccccgccgccgggagggtgtgcggtccccgccgccgcctcgggcagaggtggtcaccaccatcgcgccgccgccgccgctgctgccctggcctctcccgggcgtctggcatcctcccctaccggggccccggcggcgcgcggcgtctgcccggaggggggctcgggcatggtgctgcggcagctgga

SEQ ID NO: 19375 - RNA, 690 nt, Homo sapiens
  source 1..690: mol_type = other RNA
ttcacagtggctaagttccgcatgtcccatatggtctctaccagaggaatactgccgacctgccagtcatagcacagggtcacgggtgcaagcagaagccacacattgaaggccaagaggtaggaataggtgaggaatgacttgtcttgcttgttggaaagggaaaagaggtcataaaccaagcacactccaaacaccgtgatgcctgtctctttcaccagcatcgcacaggtccccagaaacaaactgagcagcaagaagaagggagacaccgtggaagggaaacttcccccaacacagccctgatccagactcctgttgtacgagagaaaggccaatagaaacagcagacacgctaacacgtccgctctgccaacgatcccagccaccgcctcagtatgaataggatgtacagcaaaaagcaatgccgttacaaaagcaagtccacgattcttgaagacagttttatcacaggtgtacatcagcacaagagtcactaagcagtgtaaaattatatttactgcatgaaagtagaatgggttcataccagtcaaaaatatgtttagccttccagggagaaaagtgccgctgcttcccgggaagttcccggcttttcagcacccgggacaacagcagcggcgcccggagagacgctctccacccgccccgcgctcgcgtccagtcgccggc

SEQ ID NO: 19376 - RNA, 993 nt, Homo sapiens
  source 1..993: mol_type = other RNA
ttcacagtggctaagttccgcatgtcccatatggtctctaccagaggaatactgccgacctgccagtcatagcacagggtcacgggtgcaagcagaagccacacattgaaggccaagaggtaggaataggtgaggaatgacttgtcttgcttgttggaaagggaaaagaggtcataaaccaagcacactccaaacaccgtgatgcctgtctctttcaccagcatcgcacaggtccccagaaacaaactgagcagcaagaagaagggagacaccgtggaagggaaacttcccccaacacagccctgatccagactcctgttgtacgagagaaaggccaatagaaacagcagacacgctaacacgtccgctctgccaacgatcccagccaccgcctcagtatgaataggatgtacagcaaaaagcaatgccgttacaaaagcaagtccacgattcttgaagacagttttatcacaggtgtacatcagcacaagagtcactaagcagtgtaaaattatatttactgcatgaaagtagaatgggttcataccagtcaaaaatatgtttagcttgaaggtgaggacgcagagcggccggtaggacttgtggctggtgttctcggccatgcccttgccccagaagtcgttggtgaagatgccccagcggagcggggcgccgggccgcacgtcggggttgttcacgatcgcccacacgtcgtcgtgcacgaactcgccctgcagggagcggccgtagcacaggcagcttgccccggccagcagcgccgcggccccggccggcgctagcccgcagccccgccgccgggagggtgtgcggtccccgccgccgcctcgggcagaggtggtcaccaccatcgcgccgccgccgccgctgctgccctggcctctcccgggcgtctggcatcctcccctaccggggccccggcggcgcgcggcgtctgcccggaggggggctcgggcatggtgctgcggcagctgg

SEQ ID NO: 19377 - RNA, 158 nt, Homo sapiens
  source 1..158: mol_type = other RNA
ttcaccaccttctccacccagcagtaacactgatcatgtcccgggcagtcaaggagatcgacgggccgccttcttagggcaggttccccgtagttgtttacttatcaatattccgtgatgaggaaaaaccacaccctgcattagcaaggccaataaaa

SEQ ID NO: 19378 - RNA, 3159 nt, Homo sapiens
  source 1..3159: mol_type = other RNA
ttcaccaccttctccacccagccaccaggataccgccgcaggatgagctttcggacctcatcatagatgaagatgaggaggctgtaggggaaggcgcagaaccaccaggtgactttgagcgggtacatgcggagggctacacccatgcctgggcagtaagagagaaaggcagccaacgccgtctcctccaggagcccaaaaatcaggatcttgttcttcatgccctgctggaagactgagttgcggcgggtcttgcagatgatgaggtcagcccactgcaccaccacgatgctggcaaagaatgccgtgtggcacgtgaactccaccaccttccgctgctcataggtccactcctgtccatagctgtcctccagatcattcatggtccggtcatcccagtcgaggcggattcccagtagccgtgatggcaggaaaccgttctctgccaggatcacaaagtaggtgaagaagccacccagtgcctggatcatcccgatctgtccgtaggccatgctgatgagcctctcattcaccagcttgtccgtctgggagtttcgtggctgccgcttcatgatatcactctcagctgcctcataggccaaggagatggcagggaccatatctgtgcccaggtcaatgcaaaggatggtcacagtgcccagaggtagggggatgttggcaatgatgaacagcaggaagggggtgatctcggggatgttgctggtcagggtgtaggcgatggatttcttcaagttgtcaaagatcaggcggccctcctccacccccgtgacgatggaggcaaagttgtcatccagcaggatcatgtcggctgcctgcttagagacgtcagagccagagatgcccatggcaatgccaatgtcagccttcttcaatgcaggggagtcgttcaccccgtcacccgtcacggccacaatggctccctgcctctgacatccctccacaatgatgagcttctgctggggagacgttcgagcaaagacgatctctgtgtggttcttgaggatctcatcgagctgctccgatgtcatgtccttcaggtcagagccgtgcaccacgcatgccttggcttctctggggttgacttgactcatgggaatgttgagccgggctgcaatgtcctccacagtctcgttaccctctgatatgatgcccacgcctttggcaatggccttggctgtgatagggtgatccccggttaccatgatcaccttgatgcctgcgcttcggcacttgcccacagcatctggcacagcagcccggggagggtcaatcatagacatgagccccacaaagcaaagcttctccgtgggaaagttcagctcatccgtgtcgaatttgaagccccgaggaaactttccagatggcagattcagttgacagaatcccagcacacgctccccaagtccccccagctccatgtaggcattttgaaaggcatcttgcatctccttgtcgagcgggatctccttgccctgcaccaggatggtggagcaccggtccagaatgcgctctggggcccccttcatcaccagcacgtggctctgggggctgtcttctcgctcgtggatagacagctggtacttgttggtagagttgaaaggaatctctgccaccttggggtttctgtctctcattttcctcactgagccacaggagagctcaatgcacttgagcagagctgactcagaggcatcaccagctgtgtcccgcttagacacggagatgttctcctgtcctgccttgaagacggcgcggttgcagagaccagcaattcgagacagggccgtccacgtaggggatcgtttgtcaaaagtggccccagactgatcttcggtggtgtcagcctcatggatttggttgtcgaaccacatgtgggcgacggtcatgcggttctgggtgagggtgcccgtcttgtccgagcagatggtggacgtggagcccagcgtctccaccgcctccaggttcttcaccaggcagttcttccgtgccatgcgcttggctgtcagggtcaggcacacagtgacagtggccagaagcccctcaggcacgttggccactatgatgccgatgaggaagatgactgcctccagccagctgtagcccaggatgagggagagcacgaagaaggagacccccaggaatacagcgacccctgtgatcagctggatgaagtgttcaatctccattgctatgggtgtccgcccaacctccaggcctgaggcgagagtagctatgcggcccatcaccgtccggtctcctgtggcaatcacaatgcccctggcagtgccttcaacacagttggtggagaagaaacagatattgcgggtctccagggggttctcatgggtgaactcgggggagcgggtctggggctccgactctcctgttaaggatgagttatccaccttacagccatgagaagagatgatccggaggtcagcagggacgcggtctccacccttcacctccaccaggtctcccaccaccacttcctctgcgttgatctgcatcttctctccctcccggatcacaagggcttgctgaggtaccatgttcttgaaggaatccatgatcttggagctcttggcctcctggtagtaggagaagcagccagtgacaatgaccacagctgccagcaccacacccagatatagattgtcgttggatggttcatcctccatggcagcctggatgccgtaggccaggaagcagaggatagccccaatccacagcaggatggagaaccccccgaaaagctgacggcagaacttgacccactcaggggttgtgggaggtggtgtgagggcgttgggcccatctcgagccagaacgtcctgagcccgctggttggtgaggcccttggacaggtccacttggtatttgcggcccagctcatccaaggacagcttgtggtcatccattgccacctccttcttcagctcatccagttccttctccttctgtttcttcttgccgcccccattctctgccgtggtggcggcaggtgagtactcacggccagccccacggcccatcttggggcagagtggctgagggaccttagcgggagaggtcaccaggaggatcccaagcccacaccagcccgtctgggacagtcggagaccctggcagacagag

SEQ ID NO: 19379 - RNA, 3237 nt, Homo sapiens
  source 1..3237: mol_type = other RNA
ttcaccaccttctccacccagccgccagggcgtcgcctgatgatgagttttctgacttcgtcatatacgaagatgagaagagagtaggggaaggcacagaaccaccaggtaggtttgaggggatacatcctaagagcaacacccattccagggcagtaggaaaggaaagcagccagggctgtctcttcaaagaggccaaatatcaagatcttgttcttcatcccctgctggaagaccgaattcctcctggtcttacagatgaccaagtcggcccactgcaccaccacgatactgacgaagaaggctgtgtggcaggtgaactccacgattttcctctgctcataggtccactgctgcccgtagctgtcttccacatcgttgatccagcggtcatcccagtccactcggaggcccaacaggtgaattgggaggaagccgttctcagccagaatcacaaagtaagtaaagaagcctcccagggcctggatcattccaatctgcccataggccatgctgatcagccgctcattcacaagtttgtctgttttgggatttctgggctgtctcttcatgatgtcactctcagcctgctcataagccagggagatggcaggaaccatgtcagtgcccaagtcaatgcagaggatggtgacagtccccagtggtagtggaatgtttgcaataataaatatcaggaacggggtgatctcgggaatgttactggttaaggtataagcaatggatttcttcaagttatcaaagatcagacgaccttcctctactccagtcacaattgaggcaaagttgtcatccagaagaatcatgtcagcagcttgcttggacacatctgagccagcaatccccatagcaaccccaatgtctgctttcttcaaagctggagagtcattcacaccgtcaccagtcacagccacgatagcaccctgtctttggcagccttccacaatgatgagcttctgctgaggggaggtcctggcaaacactatctcagtgtggtacttcaaaatgtcatccagctgctcggaggtcatgtcctttagatcactgccgtgtactacgcaggccttggcatccctggggttcacctggctgactgggatgttgaggcgggcagcaatgtcttccacggtctcattgccttctgagatgatgcccacacctttggcaatagctttagctgtgattggatggtctcctgtgaccatgatgaccttaattccagcacttcgacatttgcccacggcatcaggaacggccgcccgtggagggtcaatcatggagatgagcccaacaaagcacagattatcgatagggaaattcacatcgtcagtgtcaaactggaacccttcaggaaactgttcatctggcagaaagaggtggcagaaacctaggactcgttctccgaggccccccagctccaaataggcgttctgaaaggcgtctttcagctcctcatccaggggctgctccttgccgtggaggaggatagagctgcaacggtctaggatcctttctggggcgcccttcatcaccaacaggtgttggggctccgatgtgttggggttcttatgaatagacaactggtacttgttggtggagttgaagggtatctcgacgattttggcgtatctttctctcatctccttcacggaaccacagcacagctctatgcactttaagagtgctgactcagaggcatctcctgcaactgcccgcttaagaataggtaggttttcctggttagcctgaaacactgccctgttacaaagacctgcaattctggacagagcaagccaggtagctgaagtcttgtcaaaagagacaccactctgattctctgtcgtatcagcttcatggatttgattgtcaaaccacatgtgggccactgtcatccggttctgagtcagagttccagttttatcagagcagatggtggacgtggaccccaaggtctccacagcttctaagttcttcactaagcagtttttccttgccatgcgtttggcagtaagtgtcagacagaccgtgacagtggccagcaaaccttccggcacattggctacgatgataccgatgaggaagatgacagcctcaagccaggtgtactcaaggatgagagaaaggatgaagaaagacacacccaggaacacagccacacccgtgatgatgtggataaaatgttcaatttctgcagcaatgggggtctggcctccttccagcccagaagcaagtgtggcaattcttcccatcacagtgcgatccccagtgtagacaacaataccacgtgcggtgccttcaacacaattggttgaaaagaaggcaatgttcctcgtctccagggggttttcatttgtgaaatctggagacctagtctggggttctgattcaccagtgagcgaggagttatccaccttgcagccatttgcagatatgattctgaggtcagcaggaattcggtctcctccttttacttccaccagatccccaaccacaacttcctccgcatttatgctcattttctcaccatttcgaatcacaagggcttgctgagggaccatgtttttgaaggattccatgatctttgaacttttagcttcttgatagtaggagaagcaaccagttatgattacaacggctgatagcaccacacccaggtacagattatcgttttgaggttcctcttctgtagcagcttggatgctataagccaagaaacaaagaatcgctccaatccacagtaacattgagaaccccccaaagagctgccgacaaaacttgatccattcaggagtagtgggagggggagtgagggcgttgggaccatctcgcgccaggatctcagctgcacgagcagatgttaatccccggctcaagtctgttccatatttacgatgaagttcatcaaggctaagtttatgatcatccatagaaacttctttcttcagttcatccatgtccctgtcttttttgccctttttgccctttttatcaccttgttctgaaacagctgcaggctcatacttatcacgtccaaccagcagtgtatccttaggcaagttactaacttctacatttcaatttcctcttccacagcgtggagataaagaatagtgccaacctcatttcatgtttttaaggattaaatgatacaatacatctaaatgctagtacttttatactgtttatattctttgctttgcaaagacattattacatatc

SEQ ID NO: 19380 - RNA, 3333 nt, Homo sapiens
  source 1..3333: mol_type = other RNA
ttcaccaccttctccacccagccgccagggcgtcgcctgatgatgagttttctgacttcgtcatatacgaagatgagaagagagtaggggaaggcacagaaccaccaggtaggtttgaggggatacatcctaagagcaacacccattccagggcagtaggaaaggaaagcagccagggctgtctcttcaaagaggccaaatatcaagatcttgttcttcatcccctgctggaagaccgaattcctcctggtcttacagatgaccaagtcggcccactgcaccaccacgatactgacgaagaaggctgtgtggcaggtgaactccacgattttcctctgctcataggtccactgctgcccgtagctgtcttccacatcgttgatccagcggtcatcccagtccactcggaggcccaacaggtgaattgggaggaagccgttctcagccagaatcacaaagtaagtaaagaagcctcccagggcctggatcattccaatctgcccataggccatgctgatcagccgctcattcacaagtttgtctgttttgggatttctgggctgtctcttcatgatgtcactctcagcctgctcataagccagggagatggcaggaaccatgtcagtgcccaagtcaatgcagaggatggtgacagtccccagtggtagtggaatgtttgcaataataaatatcaggaacggggtgatctcgggaatgttactggttaaggtataagcaatggatttcttcaagttatcaaagatcagacgaccttcctctactccagtcacaattgaggcaaagttgtcatccagaagaatcatgtcagcagcttgcttggacacatctgagccagcaatccccatagcaaccccaatgtctgctttcttcaaagctggagagtcattcacaccgtcaccagtcacagccacgatagcaccctgtctttggcagccttccacaatgatgagcttctgctgaggggaggtcctggcaaacactatctcagtgtggtacttcaaaatgtcatccagctgctcggaggtcatgtcctttagatcactgccgtgtactacgcaggccttggcatccctggggttcacctggctgactgggatgttgaggcgggcagcaatgtcttccacggtctcattgccttctgagatgatgcccacacctttggcaatagctttagctgtgattggatggtctcctgtgaccatgatgaccttaattccagcacttcgacatttgcccacggcatcaggaacggccgcccgtggagggtcaatcatggagatgagcccaacaaagcacagattatcgatagggaaattcacatcgtcagtgtcaaactggaacccttcaggaaactgttcatctggcagaaagaggtggcagaaacctaggactcgttctccgaggccccccagctccaaataggcgttctgaaaggcgtctttcagctcctcatccaggggctgctccttgccgtggaggaggatagagctgcaacggtctaggatcctttctggggcgcccttcatcaccaacaggtgttggggctccgatgtgttggggttcttatgaatagacaactggtacttgttggtggagttgaagggtatctcgacgattttggcgtatctttctctcatctccttcacggaaccacagcacagctctatgcactttaagagtgctgactcagaggcatctcctgcaactgcccgcttaagaataggtaggttttcctggttagcctgaaacactgccctgttacaaagacctgcaattctggacagagcaagccaggtagctgaagtcttgtcaaaagagacaccactctgattctctgtcgtatcagcttcatggatttgattgtcaaaccacatgtgggccactgtcatccggttctgagtcagagttccagttttatcagagcagatggtggacgtggaccccaaggtctccacagcttctaagttcttcactaagcagtttttccttgccatgcgtttggcagtaagtgtcagacagaccgtgacagtggccagcaaaccttccggcacattggctacgatgataccgatgaggaagatgacagcctcaagccaggtgtactcaaggatgagagaaaggatgaagaaagacacacccaggaacacagccacacccgtgatgatgtggataaaatgttcaatttctgcagcaatgggggtctggcctccttccagcccagaagcaagtgtggcaattcttcccatcacagtgcgatccccagtgtagacaacaataccacgtgcggtgccttcaacacaattggttgaaaagaaggcaatgttcctcgtctccagggggttttcatttgtgaaatctggagacctagtctggggttctgattcaccagtgagcgaggagttatccaccttgcagccatttgcagatatgattctgaggtcagcaggaattcggtctcctccttttacttccaccagatccccaaccacaacttcctccgcatttatgctcattttctcaccatttcgaatcacaagggcttgctgagggaccatgtttttgaaggattccatgatctttgaacttttagcttcttgatagtaggagaagcaaccagttatgattacaacggctgatagcaccacacccaggtacagattatcgttttgaggttcctcttctgtagcagcttggatgctataagccaagaaacaaagaatcgctccaatccacagtaacattgagaaccccccaaagagctgccgacaaaacttgatccattcaggagtagtgggagggggagtgagggcgttgggaccatctcgcgccaggatctcagctgcacgagcagatgttaatccccggctcaagtctgttccatatttacgatgaagttcatcaaggctaagtttatgatcatccatagaaacttctttcttcagttcatccatgtccctgtcttttttgccctttttgccctttttatcaccttgttctgaaacagctgcaggctcatacttatcacgtccaacccccttccccatggtggcggtgctcagtgcccggcgccgggtcctgtcgctggagaatcagagagaaaagcacagagcagctcccggccgagcgagcgggaccaggggagccaagtggagggagctagggctgccgcggggcgggagggtgggagggcggccggcggctcgggccgatgccgccgccgctgttgctgccgccgcccgggctgctaccgctgttgccacgtgtccgcctcctcccgccgctgctctgcgccccagaccccgccgcagctcc

SEQ ID NO: 19381 - RNA, 3428 nt, Homo sapiens
  source 1..3428: mol_type = other RNA
ttcaccaccttctccacccagccgccagggcgtcgcctgatgatgagttttctgacttcgtcatatacgaagatgagaagagagtaggggaaggcacagaaccaccaggtaggtttgaggggatacatcctaagagcaacacccattccagggcagtaggaaaggaaagcagccagggctgtctcttcaaagaggccaaatatcaagatcttgttcttcatcccctgctggaagaccgaattcctcctggtcttacagatgaccaagtcggcccactgcaccaccacgatactgacgaagaaggctgtgtggcaggtgaactccacgattttcctctgctcataggtccactgctgcccgtagctgtcttccacatcgttgatccagcggtcatcccagtccactcggaggcccaacaggtgaattgggaggaagccgttctcagccagaatcacaaagtaagtaaagaagcctcccagggcctggatcattccaatctgcccataggccatgctgatcagccgctcattcacaagtttgtctgttttgggatttctgggctgtctcttcatgatgtcactctcagcctgctcataagccagggagatggcaggaaccatgtcagtgcccaagtcaatgcagaggatggtgacagtccccagtggtagtggaatgtttgcaataataaatatcaggaacggggtgatctcgggaatgttactggttaaggtataagcaatggatttcttcaagttatcaaagatcagacgaccttcctctactccagtcacaattgaggcaaagttgtcatccagaagaatcatgtcagcagcttgcttggacacatctgagccagcaatccccatagcaaccccaatgtctgctttcttcaaagctggagagtcattcacaccgtcaccagtcacagccacgatagcaccctgtctttggcagccttccacaatgatgagcttctgctgaggggaggtcctggcaaacactatctcagtgtggtacttcaaaatgtcatccagctgctcggaggtcatgtcctttagatcactgccgtgtactacgcaggccttggcatccctggggttcacctggctgactgggatgttgaggcgggcagcaatgtcttccacggtctcattgccttctgagatgatgcccacacctttggcaatagctttagctgtgattggatggtctcctgtgaccatgatgaccttaattccagcacttcgacatttgcccacggcatcaggaacggccgcccgtggagggtcaatcatggagatgagcccaacaaagcacagattatcgatagggaaattcacatcgtcagtgtcaaactggaacccttcaggaaactgttcatctggcagaaagaggtggcagaaacctaggactcgttctccgaggccccccagctccaaataggcgttctgaaaggcgtctttcagctcctcatccaggggctgctccttgccgtggaggaggatagagctgcaacggtctaggatcctttctggggcgcccttcatcaccaacaggtgttggggctccgatgtgttggggttcttatgaatagacaactggtacttgttggtggagttgaagggtatctcgacgattttggcgtatctttctctcatctccttcacggaaccacagcacagctctatgcactttaagagtgctgactcagaggcatctcctgcaactgcccgcttaagaataggtaggttttcctggttagcctgaaacactgccctgttacaaagacctgcaattctggacagagcaagccaggtagctgaagtcttgtcaaaagagacaccactctgattctctgtcgtatcagcttcatggatttgattgtcaaaccacatgtgggccactgtcatccggttctgagtcagagttccagttttatcagagcagatggtggacgtggaccccaaggtctccacagcttctaagttcttcactaagcagtttttccttgccatgcgtttggcagtaagtgtcagacagaccgtgacagtggccagcaaaccttccggcacattggctacgatgataccgatgaggaagatgacagcctcaagccaggtgtactcaaggatgagagaaaggatgaagaaagacacacccaggaacacagccacacccgtgatgatgtggataaaatgttcaatttctgcagcaatgggggtctggcctccttccagcccagaagcaagtgtggcaattcttcccatcacagtgcgatccccagtgtagacaacaataccacgtgcggtgccttcaacacaattggttgaaaagaaggcaatgttcctcgtctccagggggttttcatttgtgaaatctggagacctagtctggggttctgattcaccagtgagcgaggagttatccaccttgcagccatttgcagatatgattctgaggtcagcaggaattcggtctcctccttttacttccaccagatccccaaccacaacttcctccgcatttatgctcattttctcaccatttcgaatcacaagggcttgctgagggaccatgtttttgaaggattccatgatctttgaacttttagcttcttgatagtaggagaagcaaccagttatgattacaacggctgatagcaccacacccaggtacagattatcgttttgaggttcctcttctgtagcagcttggatgctataagccaagaaacaaagaatcgctccaatccacagtaacattgagaaccccccaaagagctgccgacaaaacttgatccattcaggagtagtgggagggggagtgagggcgttgggaccatctcgcgccaggatctcagctgcacgagcagatgttaatccccggctcaagtctgttccatatttacgatgaagttcatcaaggctaagtttatgatcatccatagaaacttctttcttcagttcatccatgtccctgtcttttttgccctttttgccctttttatcaccttgttctgaaacagctgcaggctcatacttatcacgtccaaccttaaaggccatcttagggcagtgaagacacaccctttctggcaccagcccgcccagccggcttcgcacttagaagcagccagttttttctttgggggagggcggccgcctctgcgcggagcaagctaagccccagcgtccccaggagaaggagccccgaacccggaggctgcccccgccggaaccggggccgcggcgggaacggaggcccgggaggaggccccggcggagcgccccaggggaaggggaggagcgcgcctttcctcagggcacggagggcggagggaaaaggaaggagaaggaggtgacggcggtcgcagggaggggagccaggctcagggatgccggctcagtcccggggccgcccccgctgct

SEQ ID NO: 19382 - RNA, 6623 nt, Homo sapiens
  source 1..6623: mol_type = other RNA
ttcaccaccttctccacccagccgccagggcgtcgcctgatgatgagttttctgacttcgtcatatacgaagatgagaagagagtaggggaaggcacagaaccaccaggtaggtttgaggggatacatcctaagagcaacacccattccagggcagtaggaaaggaaagcagccagggctgtctcttcaaagaggccaaatatcaagatcttgttcttcatcccctgctggaagaccgaattcctcctggtcttacagatgaccaagtcggcccactgcaccaccacgatactgacgaagaaggctgtgtggcaggtgaactccacgattttcctctgctcataggtccactgctgcccgtagctgtcttccacatcgttgatccagcggtcatcccagtccactcggaggcccaacaggtgaattgggaggaagccgttctcagccagaatcacaaagtaagtaaagaagcctcccagggcctggatcattccaatctgcccataggccatgctgatcagccgctcattcacaagtttgtctgttttgggatttctgggctgtctcttcatgatgtcactctcagcctgctcataagccagggagatggcaggaaccatgtcagtgcccaagtcaatgcagaggatggtgacagtccccagtggtagtggaatgtttgcaataataaatatcaggaacggggtgatctcgggaatgttactggttaaggtataagcaatggatttcttcaagttatcaaagatcagacgaccttcctctactccagtcacaattgaggcaaagttgtcatccagaagaatcatgtcagcagcttgcttggacacatctgagccagcaatccccatagcaaccccaatgtctgctttcttcaaagctggagagtcattcacaccgtcaccagtcacagccacgatagcaccctgtctttggcagccttccacaatgatgagcttctgctgaggggaggtcctggcaaacactatctcagtgtggtacttcaaaatgtcatccagctgctcggaggtcatgtcctttagatcactgccgtgtactacgcaggccttggcatccctggggttcacctggctgactgggatgttgaggcgggcagcaatgtcttccacggtctcattgccttctgagatgatgcccacacctttggcaatagctttagctgtgattggatggtctcctgtgaccatgatgaccttaattccagcacttcgacatttgcccacggcatcaggaacggccgcccgtggagggtcaatcatggagatgagcccaacaaagcacagattatcgatagggaaattcacatcgtcagtgtcaaactggaacccttcaggaaactgttcatctggcagaaagaggtggcagaaacctaggactcgttctccgaggccccccagctccaaataggcgttctgaaaggcgtctttcagctcctcatccaggggctgctccttgccgtggaggaggatagagctgcaacggtctaggatcctttctggggcgcccttcatcaccaacaggtgttggggctccgatgtgttggggttcttatgaatagacaactggtacttgttggtggagttgaagggtatctcgacgattttggcgtatctttctctcatctccttcacggaaccacagcacagctctatgcactttaagagtgctgactcagaggcatctcctgcaactgcccgcttaagaataggtaggttttcctggttagcctgaaacactgccctgttacaaagacctgcaattctggacagagcaagccaggtagctgaagtcttgtcaaaagagacaccactctgattctctgtcgtatcagcttcatggatttgattgtcaaaccacatgtgggccactgtcatccggttctgagtcagagttccagttttatcagagcagatggtggacgtggaccccaaggtctccacagcttctaagttcttcactaagcagtttttccttgccatgcgtttggcagtaagtgtcagacagaccgtgacagtggccagcaaaccttccggcacattggctacgatgataccgatgaggaagatgacagcctcaagccaggtgtactcaaggatgagagaaaggatgaagaaagacacacccaggaacacagccacacccgtgatgatgtggataaaatgttcaatttctgcagcaatgggggtctggcctccttccagcccagaagcaagtgtggcaattcttcccatcacagtgcgatccccagtgtagacaacaataccacgtgcggtgccttcaacacaattggttgaaaagaaggcaatgttcctcgtctccagggggttttcatttgtgaaatctggagacctagtctggggttctgattcaccagtgagcgaggagttatccaccttgcagccatttgcagatatgattctgaggtcagcaggaattcggtctcctccttttacttccaccagatccccaaccacaacttcctccgcatttatgctcattttctcaccatttcgaatcacaagggcttgctgagggaccatgtttttgaaggattccatgatctttgaacttttagcttcttgatagtaggagaagcaaccagttatgattacaacggctgatagcaccacacccaggtacagattatcgttttgaggttcctcttctgtagcagcttggatgctataagccaagaaacaaagaatcgctccaatccacagtaacattgagaaccccccaaagagctgccgacaaaacttgatccattcaggagtagtgggagggggagtgagggcgttgggaccatctcgcgccaggatctcagctgcacgagcagatgttaatccccggctcaagtctgttccatatttacgatgaagttcatcaaggctaagtttatgatcatccatagaaacttctttcttcagttcatccatgtccctgtcttttttgccctttttgccctttttatcaccttgttctgaaacagctgcaggctcatacttatcacgtccaacctttttaacttctgtggtcacgtgtgcagcactacttgactaataacttcttccaactgggtgggttctttagtttctatcttatctattaatgaagcaggtctaaagatagtcaacattcttgacattctctccattatggagcaaccacatttgttggtgcctctttcggtacagctctcagtctcaaagctgcaaaattcagagtcagggagtgcacactgcgtgagatgaacagtggtagaatcaggtaggacaatgtttccttattattttttaaggcattagggaaaaacaaaggtcatgggaagggtgaatgataaatacggcatttcctcaatcaactacagtaatcttcccactcatctgggcattgggcacacacttcctactttttcaattagaaagttcaggtcacttcccccctcccagaggactgggagtgattaatcctcactctcatcatgttccatgtaagggcacccccgcccctttgagcatctctgaggaaaggtacaatggaaactcaacggattacactattttctaaagggccactcataaaaatgaagttgggttatggtttttttttttcccccttccattctaatttaggaagtggaaagtcacagcaagggcaggggcttacccacggtgacacagcttagcacagcgtcatcatttcatcctgtgcttcccatggattctatcctctcaaagattaactaagcattttgctatttgatctgggtagagggaaaaggtgcccaagacatgagaagataaaattcttgacaggaggaaccaaggttaaaacatgtaacaaggttcactcacttaaaaatatataccgaatcctcacagtcctcacaatgagtgagacatccccgagacttgctagagctgaagatgttgcttcctcttttttggcaattagccatttaatggggacagggttggggatagatatgacagatttagaaattatcccaaaataagcaggatcttccatcccagaggtatattgcttcaggtctgcataagctatagccaccgccaaaggccttcatacccatcccaaacaccagcctccaacagggcaggatgcgaaggctttctcaacctgcatttttcccaccatatcagcacaatgtcccatggccagcagggagctcagaattcttgagacttctgaaattcctgctgaaaaagtttagagggtacttgaaagttcaagacccaccattccctccagacaggtctgctaatggtgttgagtctgccaatttattctagtgttgccacatgctggctacatgacctttgcctgtcagccttagtttcttcattcctaaaatgggaataacacttggtataactattaaagaacctagagaaggcattttcatagtctgattagtcaagaaaccattaactctgaaaaataaaacaccttaaaaactggactatttccaaagcccacagacaaaagcttttgacgggcaagaagggccagaaggatggcaaaaggaagtgccccaaatgcagcccatttcggagttgccaagaagattgtagaaacaacacctctggacatgatttggcaaataccactttagcaggaaagttgtgtgatggactctgaccttgctggttccctagaggctgccaagtctgggctaccttcaatgtaaaaggtaagggggaggggtgctttctcattttcctggtcgatacattattaaatcatccaacacaattgtgtatgtaaaagtattctcaaagcactacacaaaggctattattataacttggtcttaattaacatatacattactgccatttttcgctttctatgaaaattcttttcaaacctttgaagaaaaaactcctttggcattatttttcatttgatcttaacagtgaaaacttaaagaaaataacagtcaagaaatgatctagcccagtttattacatctccatttgctcctaaatgactaagtagtttagtttatgtgcaaggaattgtctagccagggactggagggctaagggatggccggggttgagggaggacactgtcatagtaccatggctgctatccagccccagcagcagcacatcactgcaggagcagcagttctctgcagaggaggtgagcctgaggggccaccatgccttcatattccttctcttgcccacccaaatatgcatcctggagaatataatttaccaaggccaaagcagtagatccctttgtgagcccagtttagtatatccaaacttgggcagcccagcagccagcaagggtcaaagaacagcgacagttctagccagcaggttccctcaacccaaaagaacatgacttaaccttcctccccaatctgcctgcatgtcaattcttaatgagcctgacagcctaccctacctgcagtagtgtacatccatgatcattcaaaaaataaaaattctaaaaggtgtaaagaatcagtgcactttagatatatttttgcttttacagttattaagaacaatcagacaaaaacttcagtttcttcaatggaaaattctacctctacattaggtgcatgggttatgaagggttaaaactttctacttattccttaactccccctttctgctgaccaccttaccctcctttttttcattttaccagattgctctggttagagacaactgattaataatcagcatatgcgttatgagaggaccagatcaactcccagtaagtcctgatcactcctcaattagtaccctgaagcctaggctaggaaggaaaatgactgccaggctgaagaggataaaggctgtccaaggccctaaagaaatgtcacatgaattgaaataataaaacaaatatggtgccatggaagcatcatgtggaagataaaagaaacacacaagaggataaccccaaagtgcattagggacctgcccctacatggtaacagactagaaagagcaatcacagctcaccgatctacacagcaaggcccactgagtcacaaaatcttacactgattatcaggctcccaaacaatacaagtcccaaggacaaagcacgaactatcatgaatcaacttatcaaatcactgagacagccaatagtcattactaaatagggtttgaataaaactggaaagagatcacgtgcagatatatttcatcataactcacaaaggaactagtaagtgaggtctaaaaccagataaagagattcactgtaaagtcacaaaggaacaaaggaatgaggtctattgatcaaaaatccctttgctcaggatgcaaataaaaaccaaaccaaagagaaagtgtagggtgaagggtacttctttcgtaacagaatctgctatccgaaacacaaaataaatatgaagaacttcttgtggattcctgacaacagatttcagcacaactaatgaggtgagtcatatgctaagaacagtctctctatgactccagccaaagaatacacacttcctctcatacactcaattcatagcaacgtgagaaagttcagacctgactaggttccacatccctccccca

SEQ ID NO: 19383 - RNA, 5965 nt, Homo sapiens
  source 1..5965: mol_type = other RNA
ttcaccaccttctccacccagccgccagggcgtcgcctgatgatgagttttctgacttcgtcatatacgaagatgagaagagagtaggggaaggcacagaaccaccaggtaggtttgaggggatacatcctaagagcaacacccattccagggcagtaggaaaggaaagcagccagggctgtctcttcaaagaggccaaatatcaagatcttgttcttcatcccctgctggaagaccgaattcctcctggtcttacagatgaccaagtcggcccactgcaccaccacgatactgacgaagaaggctgtgtggcaggtgaactccacgattttcctctgctcataggtccactgctgcccgtagctgtcttccacatcgttgatccagcggtcatcccagtccactcggaggcccaacaggtgaattgggaggaagccgttctcagccagaatcacaaagtaagtaaagaagcctcccagggcctggatcattccaatctgcccataggccatgctgatcagccgctcattcacaagtttgtctgttttgggatttctgggctgtctcttcatgatgtcactctcagcctgctcataagccagggagatggcaggaaccatgtcagtgcccaagtcaatgcagaggatggtgacagtccccagtggtagtggaatgtttgcaataataaatatcaggaacggggtgatctcgggaatgttactggttaaggtataagcaatggatttcttcaagttatcaaagatcagacgaccttcctctactccagtcacaattgaggcaaagttgtcatccagaagaatcatgtcagcagcttgcttggacacatctgagccagcaatccccatagcaaccccaatgtctgctttcttcaaagctggagagtcattcacaccgtcaccagtcacagccacgatagcaccctgtctttggcagccttccacaatgatgagcttctgctgaggggaggtcctggcaaacactatctcagtgtggtacttcaaaatgtcatccagctgctcggaggtcatgtcctttagatcactgccgtgtactacgcaggccttggcatccctggggttcacctggctgactgggatgttgaggcgggcagcaatgtcttccacggtctcattgccttctgagatgatgcccacacctttggcaatagctttagctgtgattggatggtctcctgtgaccatgatgaccttaattccagcacttcgacatttgcccacggcatcaggaacggccgcccgtggagggtcaatcatggagatgagcccaacaaagcacagattatcgatagggaaattcacatcgtcagtgtcaaactggaacccttcaggaaactgttcatctggcagaaagaggtggcagaaacctaggactcgttctccgaggccccccagctccaaataggcgttctgaaaggcgtctttcagctcctcatccaggggctgctccttgccgtggaggaggatagagctgcaacggtctaggatcctttctggggcgcccttcatcaccaacaggtgttggggctccgatgtgttggggttcttatgaatagacaactggtacttgttggtggagttgaagggtatctcgacgattttggcgtatctttctctcatctccttcacggaaccacagcacagctctatgcactttaagagtgctgactcagaggcatctcctgcaactgcccgcttaagaataggtaggttttcctggttagcctgaaacactgccctgttacaaagacctgcaattctggacagagcaagccaggtagctgaagtcttgtcaaaagagacaccactctgattctctgtcgtatcagcttcatggatttgattgtcaaaccacatgtgggccactgtcatccggttctgagtcagagttccagttttatcagagcagatggtggacgtggaccccaaggtctccacagcttctaagttcttcactaagcagtttttccttgccatgcgtttggcagtaagtgtcagacagaccgtgacagtggccagcaaaccttccggcacattggctacgatgataccgatgaggaagatgacagcctcaagccaggtgtactcaaggatgagagaaaggatgaagaaagacacacccaggaacacagccacacccgtgatgatgtggataaaatgttcaatttctgcagcaatgggggtctggcctccttccagcccagaagcaagtgtggcaattcttcccatcacagtgcgatccccagtgtagacaacaataccacgtgcggtgccttcaacacaattggttgaaaagaaggcaatgttcctcgtctccagggggttttcatttgtgaaatctggagacctagtctggggttctgattcaccagtgagcgaggagttatccaccttgcagccatttgcagatatgattctgaggtcagcaggaattcggtctcctccttttacttccaccagatccccaaccacaacttcctccgcatttatgctcattttctcaccatttcgaatcacaagggcttgctgagggaccatgtttttgaaggattccatgatctttgaacttttagcttcttgatagtaggagaagcaaccagttatgattacaacggctgatagcaccacacccaggtacagattatcgttttgaggttcctcttctgtagcagcttggatgctataagccaagaaacaaagaatcgctccaatccacagtaacattgagaaccccccaaagagctgccgacaaaacttgatccattcaggagtagtgggagggggagtgagggcgttgggaccatctcgcgccaggatctcagctgcacgagcagatgttaatccccggctcaagtctgttccatatttacgatgaagttcatcaaggctaagtttatgatcatccatagaaacttctttcttcagttcatccatgtccctgtcttttttgccctttttgccctttttatcaccttgttctgaaacagctgcaggctcatacttatcacgtccaacctttttaacttctgtggtcacgtgtgcagcactacttgactaataacttcttccaactgggtgggttctttagtttctatcttatctattaatgaagcaggtctaaagatagtcaacattcttgacattctctccattatggagcaaccacatttgttggtgcctctttcggtacagctttaaaaatatataccgaatcctcacagtcctcacaatgagtgagacatccccgagacttgctagagctgaagatgttgcttcctcttttttggcaattagccatttaatggggacagggttggggatagatatgacagatttagaaattatcccaaaataagcaggatcttccatcccagaggtatattgcttcaggtctgcataagctatagccaccgccaaaggccttcatacccatcccaaacaccagcctccaacagggcaggatgcgaaggctttctcaacctgcatttttcccaccatatcagcacaatgtcccatggccagcagggagctcagaattcttgagacttctgaaattcctgctgaaaaagtttagagggtacttgaaagttcaagacccaccattccctccagacaggtctgctaatggtgttgagtctgccaatttattctagtgttgccacatgctggctacatgacctttgcctgtcagccttagtttcttcattcctaaaatgggaataacacttggtataactattaaagaacctagagaaggcattttcatagtctgattagtcaagaaaccattaactctgaaaaataaaacaccttaaaaactggactatttccaaagcccacagacaaaagcttttgacgggcaagaagggccagaaggatggcaaaaggaagtgccccaaatgcagcccatttcggagttgccaagaagattgtagaaacaacacctctggacatgatttggcaaataccactttagcaggaaagttgtgtgatggactctgaccttgctggttccctagaggctgccaagtctgggctaccttcaatgtaaaaggtaagggggaggggtgctttctcattttcctggtcgatacattattaaatcatccaacacaattgtgtatgtaaaagtattctcaaagcactacacaaaggctattattataacttggtcttaattaacatatacattactgccatttttcgctttctatgaaaattcttttcaaacctttgaagaaaaaactcctttggcattatttttcatttgatcttaacagtgaaaacttaaagaaaataacagtcaagaaatgatctagcccagtttattacatctccatttgctcctaaatgactaagtagtttagtttatgtgcaaggaattgtctagccagggactggagggctaagggatggccggggttgagggaggacactgtcatagtaccatggctgctatccagccccagcagcagcacatcactgcaggagcagcagttctctgcagaggaggtgagcctgaggggccaccatgccttcatattccttctcttgcccacccaaatatgcatcctggagaatataatttaccaaggccaaagcagtagatccctttgtgagcccagtttagtatatccaaacttgggcagcccagcagccagcaagggtcaaagaacagcgacagttctagccagcaggttccctcaacccaaaagaacatgacttaaccttcctccccaatctgcctgcatgtcaattcttaatgagcctgacagcctaccctacctgcagtagtgtacatccatgatcattcaaaaaataaaaattctaaaaggtgtaaagaatcagtgcactttagatatatttttgcttttacagttattaagaacaatcagacaaaaacttcagtttcttcaatggaaaattctacctctacattaggtgcatgggttatgaagggttaaaactttctacttattccttaactccccctttctgctgaccaccttaccctcctttttttcattttaccagattgctctggttagagacaactgattaataatcagcatatgcgttatgagaggaccagatcaactcccagtaagtcctgatcactcctcaattagtaccctgaagcctaggctaggaaggaaaatgactgccaggctgaagaggataaaggctgtccaaggccctaaagaaatgtcacatgaattgaaataataaaacaaatatggtgccatggaagcatcatgtggaagataaaagaaacacacaagaggataaccccaaagtgcattagggacctgcccctacatggtaacagactagaaagagcaatcacagctcaccgatctacacagcaaggcccactgagtcacaaaatcttacactgattatcaggctcccaaacaatacaagtcccaaggacaaagcacgaactatcatgaatcaacttatcaaatcactgagacagccaatagtcattactaaatagggtttgaataaaactggaaagagatcacgtgcagatatatttcatcataactcacaaaggaactagtaagtgaggtctaaaaccagataaagagattcactgtaaagtcacaaaggaacaaaggaatgaggtctattgatcaaaaatccctttgctcaggatgcaaataaaaaccaaaccaaagagaaagtgtagggtgaagggtacttctttcgtaacagaatctgctatccgaaacacaaaataaatatgaagaacttcttgtggattcctgacaacagatttcagcacaactaatgaggtgagtcatatgctaagaacagtctctctatgactccagccaaagaatacacacttcctctcatacactcaattcatagcaacgtgagaaagttcagacctgactaggttccacatccctccccca

SEQ ID NO: 19384 - RNA, 5031 nt, Homo sapiens
  source 1..5031: mol_type = other RNA
ttcaccaccttctccacccagccgccagggcgtcgcctgatgatgagttttctgacttcgtcatatacgaagatgagaagagagtaggggaaggcacagaaccaccaggtaggtttgaggggatacatcctaagagcaacacccattccagggcagtaggaaaggaaagcagccagggctgtctcttcaaagaggccaaatatcaagatcttgttcttcatcccctgctggaagaccgaattcctcctggtcttacagatgaccaagtcggcccactgcaccaccacgatactgacgaagaaggctgtgtggcaggtgaactccacgattttcctctgctcataggtctgaaatgcagaagacagaagatgagctctggctcttcacctgcatggctggtggcagtgtggcctcagtcttctggggcttgaggagctctgacactggtcaggtcagaggtgcccactcacccactgctgcccgtagctgtcttccacatcgttgatccagcggtcatcccagtccactcggaggcccaacaggtgaattgggaggaagccgttctcagccagaatcacaaagtaagtaaagaagcctcccagggcctggatcattcctaagttgggaaaacaacccaattactagaacctcacacacaagggtacctgtatagccttcagctgattactgcagcaggcctgggagagcacatatggaggagtgtttccccctggttgataaaagcacaggaaagaattgcctggtcactcacaggctatgagggatgggatggaggaccccaggcatacactccaatctcagggccctctgctttttgagtcactttttggagcctacacaaagacacatgtgccttgctctcaaaatgcccacctgttacttgaccagctgcttctaagggtatgacctttaggggaaatccacttccctactttttaatctctgacaaatgataacttcttttccatctttcaaaattcctacatgctgccatttttctagccactgtggcactttctgactctcctccccaccttcaggaccctcctccccctggcatccaatttaaccacgctgctccaagttcctcagggcagggtttcatcctaaaccaccagagacctagtcttccttcctctcaaaagcaggcctccttggagaaggtcaggatgggccaccagccaattactttgttgccaacaactgtctaatgaatctttgccataatttccacaatattctatctaatctgttcttctttatccaagcgttcacagttatgtgacccattaatccaggagaataagacatccatggtggctttgccaggttctcttgaaggaaccctaggcagaggatttaaaaacaaatggcatgctgattgcccaccacctggatcacctgttagctagtcatgctgcactgtgggggcagaagtccagtgtgaggtggatggaggatcaccctttggtggtgacctaccagccaaactctcaaacacatatactttctccaatgcctaactccatccaagtgagtgacagataagtgtgtatctccagggaaagcagcctgtgcgtcagtacacacaattccttagaaccatgcctcctgttccgcaaggctcagtgaggaaggacatcctcatttctcaggcagagttgagcccagttccaaggtgctcagtatagaaaaccagtttccacaaaaggtaactgggcaaacagcaacagatgtattctcacatggaagagagttcagagaaactccacaggctcactccgttagggctcatcctagacctgaaagtcgcctggatttgcagtctctgaaatcaacctcaacctgaggtggacaccatcacctcagatgccttagatgtgccagcttcccactccaggctgcagcttaccaatctgcccataggccatgctgatcagccgctcattcacaagtttgtctgttttgggatttctgggctgtctcttcatgatgtcactctcagcctgctcataagccagggagatggcaggaaccatgtcagtgcccaagtcaatgcagaggatggtgacagtccccagtggtagtggaatgtttgcaataataaatatcaggaacggggtgatctcgggaatgttactggttaaggtataagcaatggatttcttcaagttatcaaagatcagacgaccttcctctactccagtcacaattgaggcaaagttgtcatccagaagaatcatgtcagcagcttgcttggacacatctgagccagcaatccccatagcaaccccaatgtctgctttcttcaaagctggagagtcattcacaccgtcaccagtcacagccacgatagcaccctgtctttggcagccttccacaatgatgagcttctgctgaggggaggtcctggcaaacactatctcagtgtggtacttcaaaatgtcatccagctgctcggaggtcatgtcctttagatcactgccgtgtactacgcaggccttggcatccctggggttcacctggctgactgggatgttgaggcgggcagcaatgtcttccacggtctcattgccttctgagatgatgcccacacctttggcaatagctttagctgtgattggatggtctcctgtgaccatgatgaccttaattccagcacttcgacatttgcccacggcatcaggaacggccgcccgtggagggtcaatcatggagatgagcccaacaaagcacagattatcgatagggaaattcacatcgtcagtgtcaaactggaacccttcaggaaactgttcatctggcagaaagaggtggcagaaacctaggactcgttctccgaggccccccagctccaaataggcgttctgaaaggcgtctttcagctcctcatccaggggctgctccttgccgtggaggaggatagagctgcaacggtctaggatcctttctggggcgcccttcatcaccaacaggtgttggggctccgatgtgttggggttcttatgaatagacaactggtacttgttggtggagttgaagggtatctcgacgattttggcgtatctttctctcatctccttcacggaaccacagcacagctctatgcactttaagagtgctgactcagaggcatctcctgcaactgcccgcttaagaataggtaggttttcctggttagcctgaaacactgccctgttacaaagacctgcaattctggacagagcaagccaggtagctgaagtcttgtcaaaagagacaccactctgattctctgtcgtatcagcttcatggatttgattgtcaaaccacatgtgggccactgtcatccggttctgagtcagagttccagttttatcagagcagatggtggacgtggaccccaaggtctccacagcttctaagttcttcactaagcagtttttccttgccatgcgtttggcagtaagtgtcagacagaccgtgacagtggccagcaaaccttccggcacattggctacgatgataccgatgaggaagatgacagcctcaagccaggtgtactcaaggatgagagaaaggatgaagaaagacacacccaggaacacagccacacccgtgatgatgtggataaaatgttcaatttctgcagcaatgggggtctggcctccttccagcccagaagcaagtgtggcaattcttcccatcacagtgcgatccccagtgtagacaacaataccacgtgcggtgccttcaacacaattggttgaaaagaaggcaatgttcctcgtctccagggggttttcatttgtgaaatctggagacctagtctggggttctgattcaccagtgagcgaggagttatccaccttgcagccatttgcagatatgattctgaggtcagcaggaattcggtctcctccttttacttccaccagatccccaaccacaacttcctccgcatttatgctcattttctcaccatttcgaatcacaagggcttgctgagggaccatgtttttgaaggattccatgatctttgaacttttagcttcttgatagtaggagaagcaaccagttatgattacaacggctgatagcaccacacccaggtacagattatcgttttgaggttcctcttctgtagcagcttggatgctataagccaagaaacaaagaatcgctccaatccacagtaacattgagaaccccccaaagagctgccgacaaaacttgatccattcaggagtagtgggagggggagtgagggcgttgggaccatctcgcgccaggatctcagctgcacgagcagatgttaatccccggctcaagtctgttccatatttacgatgaagttcatcaaggctaagtttatgatcatccatagaaacttctttcttcagttcatccatgtccctgtcttttttgccctttttgccctttttatcaccttgttctgaaacagctgcaggctcatacttatcacgtccaacccccttccccatggtggcggtgctcagtgcccggcgccgggtcctgtcgctggagaatcagagagaaaagcacagagcagctcccggccgagcgagcgggaccaggggagccaagtggagggagctagggctgccgcggggcgggagggtgggagggcggccggcggctcgggccgatgccgccgccgctgttgctgccgccgcccgggctgctaccgctgttgccacgtgtccgcctcctcccgccgctgctctgcgccccagaccccgccgcagctccagcccgcgcctcctcctcacttcctaaaatatgcaacctgcgtgctggccccgcccacgccgcgaaacgtcaccgttaccggagcaacctgacaccggccgtgggcctggctccgccccctcccgaaaccccgcccacgggcccggacagcgcctgctgcggccagtcctggctcccggcaggagggcgcccaggtctgggacaagcgtgtccaccgtgtcccgggagggctgcggggcgctcctgctggctgaacag

SEQ ID NO: 19385 - RNA, 3168 nt, Homo sapiens
  source 1..3168: mol_type = other RNA
ttcaccaccttctccacccagctgtcagccttttccaccacccgctggatctccagctgcaggggggtcagacgcctgcggagctcctgcagcagccgctggagctggctcttctgtcgctccgccgtccgggcggtctcctcggcctccgccagccggactcgcagctcctgcatctctgccgccagcgtcttattggttacttcagtggctgagaaacggttatggctctcctccagcttcagctccagtgtgtggatcttgttctctaggtagagccggccgctgtcctgctgctccgcgcgctgcagcaggctccccacgttaatcaggctgccattgtgggacaccaaggctttgtgttctgtgggggcagcacctggcttcgtgcttttcccaggagggggcagcaggtccaggtttccgaagagcacctcctcgggaaggccaccatccaggccctcctggcggctgtactgaaggctccggtactggcagatgttctgggtcaccaccctgctgaccagctgcttggcctgctctgcactgagccggatcccaagggtaaggaggatcctctctaagtctcgccggtgcaagtagccacaccagttggcatcaaagaacacaaaagcaagcagacagtctaaggggagcacagcagagggatccagctccttgggcatgtcctgaagtgaagagaactccatctctgactggtttgaggcaacggaccggacctccgaatcctccagctttgctccaaactcctcctctccatcatccctcagaagcaacagttctgggtccagggccatctcacacaggtcctcagaagcctcgccccggggtttttcttcttcctctcccccagaagagagtggtttgggcaaaagcccatcctccttcagcggggcctctgactctgtagccgggccctcattctgtgcctcatccttgggctccttgaccacctcctctttgatggcttcttcctccttggtggcttcttccttggccgcctcctccttctcaggttcaggtggggacacgaccttttcaggaaggctcagtagcatcttataaactctatagccaaaatccctctggagcatctccagaaacagctcggccagcaccatcacctcaaaagagatcctttcctttggcctccgatcctccacaatcccatggagggacaggtttacacagccagggcgtgcgatgacagcaggttctagggggggtggaggggcctctgggagatcagtgtccgtttcctgctgtgtggtggcctctggagtttctgcgttccgtctagaagtgtctgctgcttgctccaaggcatcaggtgcctgttcagtaggctccgtttccccttgtgcctcctgggttgggggagctgcctctgcagctttctgctggcacagggcctcccactcctccaaagtaggcatgatggtccagacatccggcaggtacaccaccactgtctgaagccgccgggggggtcccggctgcaggtactgaaactcggcaaagcgccaccacttggtacagccgctcaaatcaatgccagtctgggcctgcgcacagcggatggcggtacgcaccagcacctgcgggtcagcctgggggtcgaggccatccagggaaggagaccattcacccccaaccagcactgcctcctcttctttcctgcccagcaaaaacttaatctgcttcagaggatgctctggcgtctcccttggctcagccatgtcatccacaaagagcatgcaacaacgatacaattcctccaaccccggggaagagagcagcagtaccttcgaactataagcggggtcactgtctgcagtgatgggctcagcaccagcgtctggagctgcctccttttcagaagagacctggatccggcttggatgatggagggaaaagggctggctcagggggaaggctgatagccaactcagatgcacggacagaaaatctgaggggaccaggaggctgcggtaacggcgctggagttctaggaagtcacagatggggctgtccacagtgtaaggagtgaggtggacccggtaaggaggcaggtcatgccttggcttcttagcaccccagggctctccaccagcccgctgtttgcgtttcttggagtcatagtcatcacttcggccctgatccaaccgtccatgagggccccgggcaggaaatctgttcaggtggctcaggtgaagtgtgtgggatgtttggaagagactcagaggcttctgaggaaagagtgggggaatccggtgaggctggaagatcaactgaggctgagctcccaggatcccttgcttctggcccagggctgctacatgcagaagaggaggtgctggggacttcagtaggggctggttggagagcgtttgcaccttgacagcattccagggcactgcctggcctgggttgtatgcagccttcaccagcaccttctcacccagctggggcagacggcccttcaccacacttagctgaaaaaagacctcttcatccacaaccccaaagtagtcatgcaagctggtaacaataccagtgaagacccgctgtttctccccaccctgaaggtgcctggcattctgggacagttctgtggccacaggaggagtgagcaaaccaggaggagggcccagaagagatgttgaagctgtgcctgagaagttgcgtccccctggaagcgggttgatccgctggcgcttaaactgggacattgggaacgctgtcctctttcagagtcgtggggaaaaggacccaggcctcccaacaacttagcgctcctctcactatgccacgccacccccagagtagctggcggggtgaggggctcgagagagccccgatgacattccttcgttcaaaaacatccgccaaaaccctccacgcaaggcccggaaaaatggaggaggccggtgccggcgaggagactgtgtgggccctctccccggaagcccgacccgttgtttcctcgaccggctggtgggaaggcagctccctggccgaccaaacgcgaaaccggctgcgcgccaccctcctgctcccacgctcccgggccctccgctccggcctcagcagccgccagcgccgggtctcccagcagagccgcggcgaggccaccaagggaggact

SEQ ID NO: 19386 - RNA, 2877 nt, Homo sapiens
  source 1..2877: mol_type = other RNA
ttcaccaccttctccacccagctgtcagccttttccaccacccgctggatctccagctgcaggggggtcagacgcctgcggagctcctgcagcagccgctggagctggctcttctgtcgctccgccgtccgggcggtctcctcggcctccgccagccggactcgcagctcctgcatctctgccgccagcgtcttattggttacttcagtggctgagaaacggttatggctctcctccagcttcagctccagtgtgtggatcttgttctctaggtagagccggccgctgtcctgctgctccgcgcgctgcagcaggctccccacgttaatcaggctgccattgtgggacaccaaggctttgtgttctgtgggggcagcacctggcttcgtgcttttcccaggagggggcagcaggtccaggtttccgaagagcacctcctcgggaaggccaccatccaggccctcctggcggctgtactgaaggctccggtactggcagatgttctgggtcaccaccctgctgaccagctgcttggcctgctctgcactgagccggatcccaagggtaaggaggatcctctctaagtctcgccggtgcaagtagccacaccagttggcatcaaagaacacaaaagcaagcagacagtctaaggggagcacagcagagggatccagctccttgggcatgtcctgaagtgaagagaactccatctctgactggtttgaggcaacggaccggacctccgaatcctccagctttgctccaaactcctcctctccatcatccctcagaagcaacagttctgggtccagggccatctcacacaggtcctcagaagcctcgccccggggtttttcttcttcctctcccccagaagagagtggtttgggcaaaagcccatcctccttcagcggggcctctgactctgtagccgggccctcattctgtgcctcatccttgggctccttgaccacctcctctttgatggcttcttcctccttggtggcttcttccttggccgcctcctccttctcaggttcaggtggggacacgaccttttcaggaaggctcagtagcatcttataaactctatagccaaaatccctctggagcatctccagaaacagctcggccagcaccatcacctcaaaagagatcctttcctttggcctccgatcctccacaatcccatggagggacaggtttacacagccagggcgtgcgatgacagcaggttctagggggggtggaggggcctctgggagatcagtgtccgtttcctgctgtgtggtggcctctggagtttctgcgttccgtctagaagtgtctgctgcttgctccaaggcatcaggtgcctgttcagtaggctccgtttccccttgtgcctcctgggttgggggagctgcctctgcagctttctgctggcacagggcctcccactcctccaaagtaggcatgatggtccagacatccggcaggtacaccaccactgtctgaagccgccgggggggtcccggctgcaggtactgaaactcggcaaagcgccaccacttggtacagccgctcaaatcaatgccagtctgggcctgcgcacagcggatggcggtacgcaccagcacctgcgggtcagcctgggggtcgaggccatccagggaaggagaccattcacccccaaccagcactgcctcctcttctttcctgcccagcaaaaacttaatctgcttcagaggatgctctggcgtctcccttggctcagccatgtcatccacaaagagcatgcaacaacgatacaattcctccaaccccggggaagagagcagcagtaccttcgaactataagcggggtcactgtctgcagtgatgggctcagcaccagcgtctggagctgcctccttttcagaagagacctggatccggcttggatgatggagggaaaagggctggctcagggggaaggctgatagccaactcagatgcacggacagaaaatctgaggggaccaggaggctgcggtaacggcgctggagttctaggaagtcacagatggggctgtccacagtgtaaggagtgaggtggacccggtaaggaggcaggtcatgccttggcttcttagcaccccagggctctccaccagcccgctgtttgcgtttcttggagtcatagtcatcacttcggccctgatccaaccgtccatgagggccccgggcaggaaatctgttcaggtggctcaggtgaagtgtgtgggatgtttggaagagactcagaggcttctgaggaaagagtgggggaatccggtgaggctggaagatcaactgaggctgagctcccaggatcccttgcttctggcccagggctgctacatgcagaagaggaggtgctggggacttcagtaggggctggttggagagcgtttgcaccttgacagcattccagggcactgcctggcctgggttgtatgcagccttcaccagcaccttctcacccagctggggcagacggcccttcaccacacttagctgaaaaaagacctcttcatccacaaccccaaagtagtcatgcaagctggtaacaataccagtgaagacccgctgtttctccccaccctgaaggtgcctggcattctgggacagttctgtggccacaggaggagtgagcaaaccaggaggagggcccagaagagatgttgaagctgtgcctgagaagttgcgtccccctggaagcgggttgatccgctggcgcttaaactgggacattgggaacgctgtcctctttcagagtcgtggggaaaaggctgcgggccagggcagcgacaccggggggacaaagacacccggaaccaccacagccgctgctgccgccgccaccggaagcgcctct

SEQ ID NO: 19387 - RNA, 3171 nt, Homo sapiens
  source 1..3171: mol_type = other RNA
ttcaccaccttctccacccagctgtcagccttttccaccacccgctggatctccagctgcaggggggtcagacgcctgcggagctcctgcagcagccgctggagctggctcttctgtcgctccgccgtccgggcggtctcctcggcctccgccagccggactcgcagctcctgcatctctgccgccagcgtcttattggttacttcagtggctgagaaacggttatggctctcctccagcttcagctccagtgtgtggatcttgttctctaggtagagccggccgctgtcctgctgctccgcgcgctgcagcaggctccccacgttaatcaggctgccattgtgggacaccaaggctttgtgttctgtgggggcagcacctggcttcgtgcttttcccaggagggggcagcaggtccaggtttccgaagagcacctcctcgggaaggccaccatccaggccctcctggcggctgtactgaaggctccggtactggcagatgttctgggtcaccaccctgctgaccagctgcttggcctgctctgcactgagccggatcccaagggtaaggaggatcctctctaagtctcgccggtgcaagtagccacaccagttggcatcaaagaacacaaaagcaagcagacagtctaaggggagcacagcagagggatccagctccttgggcatgtcctgaagtgaagagaactccatctctgactggtttgaggcaacggaccggacctccgaatcctccagctttgctcctgcaaactcctcctctccatcatccctcagaagcaacagttctgggtccagggccatctcacacaggtcctcagaagcctcgccccggggtttttcttcttcctctcccccagaagagagtggtttgggcaaaagcccatcctccttcagcggggcctctgactctgtagccgggccctcattctgtgcctcatccttgggctccttgaccacctcctctttgatggcttcttcctccttggtggcttcttccttggccgcctcctccttctcaggttcaggtggggacacgaccttttcaggaaggctcagtagcatcttataaactctatagccaaaatccctctggagcatctccagaaacagctcggccagcaccatcacctcaaaagagatcctttcctttggcctccgatcctccacaatcccatggagggacaggtttacacagccagggcgtgcgatgacagcaggttctagggggggtggaggggcctctgggagatcagtgtccgtttcctgctgtgtggtggcctctggagtttctgcgttccgtctagaagtgtctgctgcttgctccaaggcatcaggtgcctgttcagtaggctccgtttccccttgtgcctcctgggttgggggagctgcctctgcagctttctgctggcacagggcctcccactcctccaaagtaggcatgatggtccagacatccggcaggtacaccaccactgtctgaagccgccgggggggtcccggctgcaggtactgaaactcggcaaagcgccaccacttggtacagccgctcaaatcaatgccagtctgggcctgcgcacagcggatggcggtacgcaccagcacctgcgggtcagcctgggggtcgaggccatccagggaaggagaccattcacccccaaccagcactgcctcctcttctttcctgcccagcaaaaacttaatctgcttcagaggatgctctggcgtctcccttggctcagccatgtcatccacaaagagcatgcaacaacgatacaattcctccaaccccggggaagagagcagcagtaccttcgaactataagcggggtcactgtctgcagtgatgggctcagcaccagcgtctggagctgcctccttttcagaagagacctggatccggcttggatgatggagggaaaagggctggctcagggggaaggctgatagccaactcagatgcacggacagaaaatctgaggggaccaggaggctgcggtaacggcgctggagttctaggaagtcacagatggggctgtccacagtgtaaggagtgaggtggacccggtaaggaggcaggtcatgccttggcttcttagcaccccagggctctccaccagcccgctgtttgcgtttcttggagtcatagtcatcacttcggccctgatccaaccgtccatgagggccccgggcaggaaatctgttcaggtggctcaggtgaagtgtgtgggatgtttggaagagactcagaggcttctgaggaaagagtgggggaatccggtgaggctggaagatcaactgaggctgagctcccaggatcccttgcttctggcccagggctgctacatgcagaagaggaggtgctggggacttcagtaggggctggttggagagcgtttgcaccttgacagcattccagggcactgcctggcctgggttgtatgcagccttcaccagcaccttctcacccagctggggcagacggcccttcaccacacttagctgaaaaaagacctcttcatccacaaccccaaagtagtcatgcaagctggtaacaataccagtgaagacccgctgtttctccccaccctgaaggtgcctggcattctgggacagttctgtggccacaggaggagtgagcaaaccaggaggagggcccagaagagatgttgaagctgtgcctgagaagttgcgtccccctggaagcgggttgatccgctggcgcttaaactgggacattgggaacgctgtcctctttcagagtcgtggggaaaaggacccaggcctcccaacaacttagcgctcctctcactatgccacgccacccccagagtagctggcggggtgaggggctcgagagagccccgatgacattccttcgttcaaaaacatccgccaaaaccctccacgcaaggcccggaaaaatggaggaggccggtgccggcgaggagactgtgtgggccctctccccggaagcccgacccgttgtttcctcgaccggctggtgggaaggcagctccctggccgaccaaacgcgaaaccggctgcgcgccaccctcctgctcccacgctcccgggccctccgctccggcctcagcagccgccagcgccgggtctcccagcagagccgcggcgaggccaccaagggaggact

SEQ ID NO: 19388 - RNA, 2880 nt, Homo sapiens
  source 1..2880: mol_type = other RNA
ttcaccaccttctccacccagctgtcagccttttccaccacccgctggatctccagctgcaggggggtcagacgcctgcggagctcctgcagcagccgctggagctggctcttctgtcgctccgccgtccgggcggtctcctcggcctccgccagccggactcgcagctcctgcatctctgccgccagcgtcttattggttacttcagtggctgagaaacggttatggctctcctccagcttcagctccagtgtgtggatcttgttctctaggtagagccggccgctgtcctgctgctccgcgcgctgcagcaggctccccacgttaatcaggctgccattgtgggacaccaaggctttgtgttctgtgggggcagcacctggcttcgtgcttttcccaggagggggcagcaggtccaggtttccgaagagcacctcctcgggaaggccaccatccaggccctcctggcggctgtactgaaggctccggtactggcagatgttctgggtcaccaccctgctgaccagctgcttggcctgctctgcactgagccggatcccaagggtaaggaggatcctctctaagtctcgccggtgcaagtagccacaccagttggcatcaaagaacacaaaagcaagcagacagtctaaggggagcacagcagagggatccagctccttgggcatgtcctgaagtgaagagaactccatctctgactggtttgaggcaacggaccggacctccgaatcctccagctttgctcctgcaaactcctcctctccatcatccctcagaagcaacagttctgggtccagggccatctcacacaggtcctcagaagcctcgccccggggtttttcttcttcctctcccccagaagagagtggtttgggcaaaagcccatcctccttcagcggggcctctgactctgtagccgggccctcattctgtgcctcatccttgggctccttgaccacctcctctttgatggcttcttcctccttggtggcttcttccttggccgcctcctccttctcaggttcaggtggggacacgaccttttcaggaaggctcagtagcatcttataaactctatagccaaaatccctctggagcatctccagaaacagctcggccagcaccatcacctcaaaagagatcctttcctttggcctccgatcctccacaatcccatggagggacaggtttacacagccagggcgtgcgatgacagcaggttctagggggggtggaggggcctctgggagatcagtgtccgtttcctgctgtgtggtggcctctggagtttctgcgttccgtctagaagtgtctgctgcttgctccaaggcatcaggtgcctgttcagtaggctccgtttccccttgtgcctcctgggttgggggagctgcctctgcagctttctgctggcacagggcctcccactcctccaaagtaggcatgatggtccagacatccggcaggtacaccaccactgtctgaagccgccgggggggtcccggctgcaggtactgaaactcggcaaagcgccaccacttggtacagccgctcaaatcaatgccagtctgggcctgcgcacagcggatggcggtacgcaccagcacctgcgggtcagcctgggggtcgaggccatccagggaaggagaccattcacccccaaccagcactgcctcctcttctttcctgcccagcaaaaacttaatctgcttcagaggatgctctggcgtctcccttggctcagccatgtcatccacaaagagcatgcaacaacgatacaattcctccaaccccggggaagagagcagcagtaccttcgaactataagcggggtcactgtctgcagtgatgggctcagcaccagcgtctggagctgcctccttttcagaagagacctggatccggcttggatgatggagggaaaagggctggctcagggggaaggctgatagccaactcagatgcacggacagaaaatctgaggggaccaggaggctgcggtaacggcgctggagttctaggaagtcacagatggggctgtccacagtgtaaggagtgaggtggacccggtaaggaggcaggtcatgccttggcttcttagcaccccagggctctccaccagcccgctgtttgcgtttcttggagtcatagtcatcacttcggccctgatccaaccgtccatgagggccccgggcaggaaatctgttcaggtggctcaggtgaagtgtgtgggatgtttggaagagactcagaggcttctgaggaaagagtgggggaatccggtgaggctggaagatcaactgaggctgagctcccaggatcccttgcttctggcccagggctgctacatgcagaagaggaggtgctggggacttcagtaggggctggttggagagcgtttgcaccttgacagcattccagggcactgcctggcctgggttgtatgcagccttcaccagcaccttctcacccagctggggcagacggcccttcaccacacttagctgaaaaaagacctcttcatccacaaccccaaagtagtcatgcaagctggtaacaataccagtgaagacccgctgtttctccccaccctgaaggtgcctggcattctgggacagttctgtggccacaggaggagtgagcaaaccaggaggagggcccagaagagatgttgaagctgtgcctgagaagttgcgtccccctggaagcgggttgatccgctggcgcttaaactgggacattgggaacgctgtcctctttcagagtcgtggggaaaaggctgcgggccagggcagcgacaccggggggacaaagacacccggaaccaccacagccgctgctgccgccgccaccggaagcgcctct

SEQ ID NO: 19389 - RNA, 2777 nt, Homo sapiens
  source 1..2777: mol_type = other RNA
ttcaccaccttctccacccagctgtcagccttttccaccacccgctggatctccagctgcaggggggtcagacgcctgcggagctcctgcagcagccgctggagctggctcttctgtcgctccgccgtccgggcggtctcctcggcctccgccagccggactcgcagctcctgcatctctgccgccagcgtcttattggttacttcagtggctgagaaacggttatggctctcctccagcttcagctccagtgtgtggatcttgttctctaggtagagccggccgctgtcctgctgctccgcgcgctgcagcaggctccccacgttaatcaggctgccattgtgggacaccaaggctttgtgttctgtgggggcagcacctggcttcgtgcttttcccaggagggggcagcaggtccaggtttccgaagagcacctcctcgggaaggccaccatccaggccctcctggcggctgtactgaaggctccggtactggcagatgttctgggtcaccaccctgctgaccagctgcttggcctgctctgcactgagccggatcccaagggtaaggaggatcctctctaagtctcgccggtgcaagtagccacaccagttggcatcaaagaacacaaaagcaagcagacagtctaaggggagcacagcagagggatccagctccttgggcatgtcctgaagtgaagagaactccatctctgactggtttgaggcaacggaccggacctccgaatcctccagctttgctcctgcaaactcctcctctccatcatccctcagaagcaacagttctgggtccagggccatctcacacaggtcctcagaagcctcgccccggggtttttcttcttcctctcccccagaagagagtggtttgggcaaaagcccatcctccttcagcggggcctctgactctgtagccgggccctcattctgtgcctcatccttgggctccttgaccacctcctctttgatggcttcttcctccttggtggcttcttccttggccgcctcctccttctcaggttcaggtggggacacgaccttttcaggaaggctcagtagcatcttataaactctatagccaaaatccctctggagcatctccagaaacagctcggccagcaccatcacctcaaaagagatcctttcctttggcctccgatcctccacaatcccatggagggacaggtttacacagccagggcgtgcgatgacagcaggttctagggggggtggaggggcctctgggagatcagtgtccgtttcctgctgtgtggtggcctctggagtttctgcgttccgtctagaagtgtctgctgcttgctccaaggcatcaggtgcctgttcagtaggctccgtttccccttgtgcctcctgggttgggggagctgcctctgcagctttctgctggcacagggcctcccactcctccaaagtaggcatgatggtccagacatccggcaggtacaccaccactgtctgaagccgccgggggggtcccggctgcaggtactgaaactcggcaaagcgccaccacttggtacagccgctcaaatcaatgccagtctgggcctgcgcacagcggatggcggtacgcaccagcacctgcgggtcagcctgggggtcgaggccatccagggaaggagaccattcacccccaaccagcactgcctcctcttctttcctgcccagcaaaaacttaatctgcttcagaggatgctctggcgtctcccttggctcagccatgtcatccacaaagagcatgcaacaacgatacaattcctccaaccccggggaagagagcagcagtaccttcgaactataagcggggtcactgtctgcagtgatgggctcagcaccagcgtctggagctgcctccttttcagaagagacctggatccggcttggatgatggagggaaaagggctggctcagggggaaggctgatagccaactcagatgcacggacagaaaatctgaggggaccaggaggctgcggtaacggcgctggagttctaggaagtcacagatggggcttcggccctgatccaaccgtccatgagggccccgggcaggaaatctgttcaggtggctcaggtgaagtgtgtgggatgtttggaagagactcagaggcttctgaggaaagagtgggggaatccggtgaggctggaagatcaactgaggctgagctcccaggatcccttgcttctggcccagggctgctacatgcagaagaggaggtgctggggacttcagtaggggctggttggagagcgtttgcaccttgacagcattccagggcactgcctggcctgggttgtatgcagccttcaccagcaccttctcacccagctggggcagacggcccttcaccacacttagctgaaaaaagacctcttcatccacaaccccaaagtagtcatgcaagctggtaacaataccagtgaagacccgctgtttctccccaccctgaaggtgcctggcattctgggacagttctgtggccacaggaggagtgagcaaaccaggaggagggcccagaagagatgttgaagctgtgcctgagaagttgcgtccccctggaagcgggttgatccgctggcgcttaaactgggacattgggaacgctgtcctctttcagagtcgtggggaaaaggctgcgggccagggcagcgacaccggggggacaaagacacccggaaccaccacagccgctgctgccgccgccaccggaagcgcctctccggaagcgcgaccact

SEQ ID NO: 19390 - RNA, 405 nt, Homo sapiens
  source 1..405: mol_type = other RNA
ttcagcaggaacagcttccttttcgtgtcttaccactgtaatcgtttgtttgaacaagagttttattgctctggcttcccagggcttcgtgaggcctcccctgcatggccaggctgatgtggattctccctagtgtgacttcgctggtgcctcttcctctgtcttgcactggtgggttcatgtttcacttctccaccagggcggtgggtggaggccacgagggctgtcccatcacctcatgtttggcagctgtggtgggcctggtgccagcgctgccaaggaaaccgtctggaccactagggaaccttgggtctggatggggaggcggtgaagagcctctggggtggaagtggtccagccaaggctggtctccatcgccttctgctggcaaaaggaagagttgct

SEQ ID NO: 19391 - RNA, 698 nt, Homo sapiens
  source 1..698: mol_type = other RNA
ttcagccaggctagtgcagtcttagtttaggttgctcggaggttgaattatgctctgaggtcaccccaaccaaaaattttaatgcagggatagtaggctagggcctgtaggcttaagtttttatttgcattaataaattaaagctccatacatagggtcttctcgtcttatttgtttatatccgcctcttcgcggataggtcaatttccctgattaaaagtaggagacagctgaaccctcgtgtggtcattcatacaagttcctatttaaggaacaagtgattatgctacctttgcacagtcaggatactgcggccattgaacgtatgtcactgggcaggcagtgcctctaatactggtaatgctagaggtgatgtttttggtaaacaggcggggtaaaatttgcggagttccttttactttttgtattctttccttagagcatacctgtgttgggttaacagtgtaaataataaagagcttattatatcgtttattaatattaggctaactgtcagtgggttattccagtctgatgtaagcttatgcaatggagaatgttttcatattacttatattaacattattgcttctattaagtaatagattagtccaatgtgatgttaggagttcagtagagtgactagaatttaagatagatgttgagcttaaacgctttcttaattggtgattgctttt

SEQ ID NO: 19392 - RNA, 850 nt, Homo sapiens
  source 1..850: mol_type = other RNA
ttcaggtctggggctgaaacctcctctgatccactgaggtgtctctggaaatcctccaccacagccacagcctcctcaccactctcagggtgatgcagctgcacccaggtccggagctccccagggaggatgctcaggaactgctcaagcaccagcagctccaggatctgctccttggtgtgcacctctggcatgagccaccagcggcagagctcccgaagccggctcaatgcttcctgcggcccagacatctcgtggtaacacaattgcctgaagtgtagccggaagatttcgcagacaggaggatagttcttctggagactgctgccctgcccccaggtctggtttgctggctcctgcttcacagtcaggcgcccctcttgcttctggaaagcagtgctcctggggatgaggcctaaatttcccctgcctgcagtggtcattgtgaccccaaagagaagcttgttacagctgcagttggtccgattaaaatgatggtcaatagttcaggtctcaggaactgtttttcagggttggagaaaggggtgatggtagtgtggcctggccacgtctgccctgttcatcgctgtacccgcagatacccggctccgtgccacgcacgaatggtcaggggtatgagacaaagaagcggctctacatcgggcggcttctgagagtcacggggaccgcgccgcctgccgccgggaagaagcgcggtcctggccagcgtcggcgacccgagctccggccgcgcctccctccgcgtctcggcccactcgcggtggcactcggcaccgaagccggacactctactgcccgttagaccaaaaacaatggccgagccggaagc

SEQ ID NO: 19393 - RNA, 887 nt, Homo sapiens
  source 1..887: mol_type = other RNA
ttcaggtctggggctgaaacctcctctgatccactgaggtgtctctggaaatcctccaccacagccacagcctcctcaccactctcagggtgatgcagctgcacccaggtccggagctccccagggaggatgctcaggaactgctcaagcaccagcagctccaggatctgctccttggtgtgcacctctggcatgagccaccagcggcagagctcccgaagccggctcaatgcttcctgcggcccagacatctcgtggtaacacaattgcctgaagtgtagccggaagatttcgcagacaggaggatagttcttctggagactgctgccctgcccccaggtctggtttgctggctcctgcttcacagtcaggcgcccctcttgcttctggaaagcagtgctcctggggatgaggcctaaatttcccctgcctgcagtggtcattgtgaccccaaagagaagcttgttacagctgcagttggtccgattaaaatgatggtcaatagttcaggtctcaggaactgtttttcagggttggagaaaggggtgatggtagtgtggcctttcgtgttaaaccaggcttcagcagcgccgctcacctggccacgtctgccctgttcatcgctgtacccgcagatacccggctccgtgccacgcacgaatggtcaggggtatgagacaaagaagcggctctacatcgggcggcttctgagagtcacggggaccgcgccgcctgccgccgggaagaagcgcggtcctggccagcgtcggcgacccgagctccggccgcgcctccctccgcgtctcggcccactcgcggtggcactcggcaccgaagccggacactctactgcccgttagaccaaaaacaatggccgagccggaagc

SEQ ID NO: 19394 - RNA, 309 nt, Homo sapiens
  source 1..309: mol_type = other RNA
ttcaggtctggggctgaaacctggccacgtctgccctgttcatcgctgtacccgcagatacccggctccgtgccacgcacgaatggtcaggggtatgagacaaagaagcggctctacatcgggcggcttctgagagtcacggggaccgcgccgcctgccgccgggaagaagcgcggtcctggccagcgtcggcgacccgagctccggccgcgcctccctccgcgtctcggcccactcgcggtggcactcggcaccgaagccggacactctactgcccgttagaccaaaaacaatggccgagccggaagc

SEQ ID NO: 19395 - RNA, 2513 nt, Homo sapiens
  source 1..2513: mol_type = other RNA
ttcatgaactgggtctagcttgggaagactgtgggtctctcagagttgtcctcactcagtatagcatcatgtcaatctggcatggaagcaaaagcctgccatggcagagggaagtgtctagaatgatgatcccaatagagcaatctcagattccatacctatatgtggcgtcagcagatccagttctgactttgttccagtaggggaacatagaagtgcagagaggcttgttggatgggaagaggcctgaggtcagagggaacagagggtccttgtgggcacaggcaatgatgagatccatagtctttggcagtgagagccactaaaaatgtcttaaataacataacacatctctaagaatcatcaaaactacaatgctgagacaagcagcattgccttgttgatttcagtttttggaatgtaaatttctgaacagtaactgctgctgtaactgaatggaatggcttcaaaatgctaaaaatttgttaaataacctaggcaggttcagccagggccgtgataactcttctaattgagggttgagagatactgaggacaaaggccttggagttagactgatctgggtctaatcttggttctgctatttacttgctctgcaactttgggaacataatttctctcctaagtgaaacagagataggaatatctaccttgcagcgttgtggtgaggattagcaagtatgcatgtaaatagccttaaccctgggtattcactgaatacctagaagatacttgagaaatggaagctctttttatattgatttgggctttgcaagctgctaagaaactgacaccctcctctttcagttctactttctttagagaaagaagcaaaagattctcattaaatgtattccacgaagaacagactgacaccaacctcttcatatgcctgagatttctattttcagcagagcccactccaacttcagagggagagtgtattacagttttactattaatcagcattatctgatgacagacttgttgactgtgaaagtctggttttacttatttcttttgttttattttagtagacagaatgccgtattttttttaaacagctttattgagttgtaatttatgtaccataccatttactaatttaatgtgtgcaagtcaatggcttttagtacattgataaaatcatgcatccatcaccaatctcaaattctagaacattttcatctccccacaaaagaaaccttacacccactagcagtcaaagccatttccccaccttacccctcagcctctgataagaatgaatctactttctgtctctatagatttgcctattctggacatttcatataaatgaaatcatataatatgtgaccttctacaatttggtttctttcaattagcataatattttcaaggaaaatcccttattcaatggtgaagatatcttattatgtcacaggagttcagtgagggccattcattccttggtagtgtcttcttgaggcccaggcactctttggatcctttctcaagcccaagtttactgtcacaggaaccccaggtccacaacagccacttaagagcatcaacttgcaccccagacttggatttaaacactttggatcactgaatccatattggcagtggagctgatgtgcttgaaattaagatgcattctaatgctcagtctccgttcaggcactatcatgtagatctcccaaggggtctatagacccacacaggaagctggcatagtggtggcttttgaggcagactctataatcttgagaggtaggtgtgtcattcaagctcctgtggttagatagctctgggggctgctgtagcctggctcaaaccgtgtctcacctggagtagacctgcccagggagggccatgcatgctctgtggctggcaaagtggcttttccatttgttttgggatttccctctctcctttcccatccagcacagaggtatggatgggtcaggaccaggcgtttactttggttagattccaaatgactaagatattttatgatggaaaactccatttgacaatcccagggagttgagtgtttttcaccctcctaagtgaataattcactttggctgtttagatatcagagctgaacaagtggctctggagcccaagatgacctcctggccagaaagggcctaaccgcactgctctgatgaccagtacttatttctatttagggattctgggcatcttccgcagccctaaaccacctaaatggacttataagagctgttccttaaatgcgtcagtgacttgggtaaatgagctgaattctcagggctttatttttttttctttctgcatcactcaatgactccacaataagtgtgctacaagttttaaatgctaatattggattttggacactgttacagttatatctgaagtaagatgtcaggctgtttggcgttaacagtgcccaagagtttatattcgtatctattcaacgctgacctccattactctctcccttttgcagccttaac

SEQ ID NO: 19396 - RNA, 2510 nt, Homo sapiens
  source 1..2510: mol_type = other RNA
ttcatgaactgggtctagcttgggaagactgtgggtctctcagagttgtcctcactcagtatagcatcatgtcaatctggcatggaagcaaaagcctgccatggcagagggaagtgtctagaatgatgatcccaatagagcaatctcagattccatacctatatgtggcgtcagcagatccagttctgactttgttccagtaggggaacatagaagtgcagagaggcttgttggatgggaagaggcctgaggtcagagggaacagagggtccttgtgggcacaggcaatgatgagatccatagtctttggcagtgagagccactaaaaatgtcttaaataacataacacatctctaagaatcatcaaaactacaatgctgagacaagcagcattgccttgttgatttcagtttttggaatgtaaatttctgaacagtaactgctgctgtaactgaatggaatggcttcaaaatgctaaaaatttgttaaataacctaggcaggttcagccagggccgtgataactcttctaattgagggttgagagatactgaggacaaaggccttggagttagactgatctgggtctaatcttggttctgctatttacttgctctgcaactttgggaacataatttctctcctaagtgaaacagagataggaatatctaccttgcagcgttgtggtgaggattagcaagtatgcatgtaaatagccttaaccctgggtattcactgaatacctagaagatacttgagaaatggaagctctttttatattgatttgggctttgcaagctgctaagaaactgacaccctcctctttcagttctactttctttagagaaagaagcaaaagattctcattaaatgtattccacgaagaacagactgacaccaacctcttcatatgcctgagatttctattttcagcagagcccactccaacttcagagggagagtgtattacagttttactattaatcagcattatctgatgacagacttgttgactgtgaaagtctggttttacttatttcttttgttttattttagtagacagaatgccgtattttttttaaacagctttattgagttgtaatttatgtaccataccatttactaatttaatgtgtgcaagtcaatggcttttagtacattgataaaatcatgcatccatcaccaatctcaaattctagaacattttcatctccccacaaaagaaaccttacacccactagcagtcaaagccatttccccaccttacccctcagcctctgataagaatgaatctactttctgtctctatagatttgcctattctggacatttcatataaatgaaatcatataatatgtgaccttctacaatttggtttctttcaattagcataatattttcaaggaaaatcccttattcaatggtgaagatatcttattatgtcacaggagttcagtgagggccattcattccttggtagtgtcttcttgaggcccaggcactctttggatcctttctcaagcccaagtttactgtcacaggaaccccaggtccacaacagccacttaagagcatcaacttgcaccccagacttggatttaaacactttggatcactgaatccatattggcagtggagctgatgtgcttgaaattaagatgcattctaatgctcagtctccgttcaggcactatcatgtagatctcccaaggggtctatagacccacacaggaagctggcatagtggtggcttttgaggcagactctataatcttgagaggtaggtgtgtcattcaagctcctgtggttagatagctctgggggctgtagcctggctcaaaccgtgtctcacctggagtagacctgcccagggagggccatgcatgctctgtggctggcaaagtggcttttccatttgttttgggatttccctctctcctttcccatccagcacagaggtatggatgggtcaggaccaggcgtttactttggttagattccaaatgactaagatattttatgatggaaaactccatttgacaatcccagggagttgagtgtttttcaccctcctaagtgaataattcactttggctgtttagatatcagagctgaacaagtggctctggagcccaagatgacctcctggccagaaagggcctaaccgcactgctctgatgaccagtacttatttctatttagggattctgggcatcttccgcagccctaaaccacctaaatggacttataagagctgttccttaaatgcgtcagtgacttgggtaaatgagctgaattctcagggctttatttttttttctttctgcatcactcaatgactccacaataagtgtgctacaagttttaaatgctaatattggattttggacactgttacagttatatctgaagtaagatgtcaggctgtttggcgttaacagtgcccaagagtttatattcgtatctattcaacgctgacctccattactctctcccttttgcagccttaac

SEQ ID NO: 19397 - RNA, 708 nt, Homo sapiens
  source 1..708: mol_type = other RNA
ttcatttgcctcccagcctacatctatctcctgtgctggatgcttcctgcccttgaacattgaactccaagtttgtcatctttgggattcagactggcttccttgttcctcagcttacagatggcccggcctgttgtgggaccttgtgattgtgtgagttaatactccttaataaactcccttttatttatatgtatatatatgtgtgtgtgtgtgtgtttgtgtgtgtatatatattctattagttctgtcccttagagaatcctgactaatacacttagcttctccttgtctctttcttttgatcttctgtgaagccctggcttgacttttcctggaaacttttcctgtgacagtgcatgtatcacaagatggccccattggacatttatgcctttaaatgaatggtacaaacactttcacctatgtcctgtatcttccaagctacaggcttcacaatcttgtgaagacataaagagaaggcgccatctgcaaatcaggaacagccctccctggactctgaatctgctggctccttggtcttggacttacccacatcagacaatggaggactcaccaccagaccgggaagcaacagcctgggctccagagtcggctggacactctgtgtccggctcctctttcgtgcacagacgaggagaggtctcatgaagcttcagcacagtctgggatcctggctctttctgt

SEQ ID NO: 19398 - RNA, 1093 nt, Homo sapiens
  source 1..1093: mol_type = other RNA
ttcatttgcctcccagcctacatctatctcctgtgctggatgcttcctgcccttgaacattgaactccaagtttgtcatctttgggattcagactggcttccttgttcctcagcttacagatggcccggcctgttgtgggaccttgtgattgtgtgagttaatactccttaataaactcccttttatttatatgtatatatatgtgtgtgtgtgtgtgtttgtgtgtgtatatatattctattagttctgtcccttagagaatcctgactaatacacttagcttctccttgtctctttcttttgatcttctgtgaagccctggcttgacttttcctggaaacttttcctgtgacagtgcatgtatcacaagatggccctaatgtcctttttcagtttctgtatcccatacggtataccacatcacatttagttgccgtgtatcttgactgtaataatttttttaaaccttctttatttctgaagaccttgactgtttcaggagtagtggtcaggtgttttgtagaacgtgtctcaattagaatttgctgacttggtctcacagttagcatttaaaatttaattgcccagatatataacgatctaccactacagcggtagctattagtgcattggggtaattccatggttgattcattttacttttgcagctgaaaaaacctcatgctgagcagagaggcatctaatttgctcatcatccatgctggaagctttttttgtctattagctttgacctttatgacccattggacatttatgcctttaaatgaatggtacaaacactttcacctatgtcctgtatcttccaagctacaggcttcacaatcttgtgaagacataaagagaaggcgccatctgcaaatcaggaacagccctccctggactctgaatctgctggctccttggtcttggacttacccacatcagacaatggaggactcaccaccagaccgggaagcaacagcctgggctccagagtcggctggacactctgtgtccggctcctctttcgtgcacagacgaggagaggtctcatgaagcttcagcacagtctgggatcctggctctttctgt

SEQ ID NO: 19399 - RNA, 144 nt, Homo sapiens
  source 1..144: mol_type = other RNA
ttcatttgcctcccagcctacatctttctcctgtgctggatgcttcctggcctcaaaaatcggactccacgttcttcagttttggaagctggactggctctctttgctcctcagcctgcagacagcctattgtgggatcttgtg

SEQ ID NO: 19400 - RNA, 1248 nt, Homo sapiens
  source 1..1248: mol_type = other RNA
ttcatttgcctcccagcctacatctttctcctgtgttgaatgcttcctgtcctcaaacatcagaatccaagttcttcagctttgggactcagactggcctctttgcttgcagatggcctattgtggaaccttgtgatcatgtgagttaatactccttaataaactctcttttatatattcatcctattcgttctgtgcctctagagaaccctgactaatacagacactaacatggcaaggagggaactgggtgtcttgtaacagccaggtcagcatgtagattgattgcctgcatggtctccactgacactacgaaggtgtgacaggagttaccttgggacaggaatgaaggtcttggtttcttactccaccttctctgatattatcatgtgggggaatttgggtaccatgtttccatctaatgagggtggagtccaagctcccgtctagcctttgctgatggggttgggagggagactgcgttatgcatttccattaatgtttgactggagttgtgctgttattatctaaaagttttctgtcttgctaggcgcccttttcgtcctcttttggttagagagagcaggcttttcatgagaaaaatctcttagctgcagccgatgatatttctgggttgctggattctttagcacccaatccaggatatatgagataaaagggaaactcaggaaacacactgctgtcattctttggtcccacggtccctagccagtcttgtctccactttcagagtcttcttatgtttcttttacatataatgtctgaggttttgatctgtacttaatgagaggaatagggtaaagtatgtccactccatcttttgagacttatgttttagtatagtaaaaatttgacttttatctcttctttccaaacagttgattgcatatccgaagagtagtactgctaaagtgacagtctggagactgaggtaggaggatcgctggaggccagaagtttgaggctgcagtgagaaataatgacaccactgcacttcagcctgggtagcagagcgaaacaccatttttgttttctgttctctgccacattccttccctgaggcattcagcacagagctgatttcatgcttccattaacgttttcaattttgaatatgttttcatttattctagtctcttgaagttaaatcatttcctttatatgtaagaaatttgctaatcattcatgggtattgttttctctaggttatttggtttcctatgtatc

SEQ ID NO: 19401 - RNA, 4237 nt, Homo sapiens
  source 1..4237: mol_type = other RNA
ttcatttgcctcccagcctacatgtttctcctgtgctgaatgcttcctgcccttaaacataggacttaaagttcttcagctctgggactcgggctggcttccttgctcctcagtttgcagacggcctattgtgggaccttgtgatcgtattagtttaatactctttaataaactcctatatatataataggtgatatatatatatacaaaataggctatatatacatatcgcctattagttctgtccctctacagaaccctgacttatacacatggcttctttttattttttatgtttgtgggcacatagtaggtgtatatatttaagggatgcatgatgcttgctactttgtctcacaactctcatgtactcagctatgggaaccacagtctctggcacctgaaatggctcaaaggaccccaagcataagcaaataagtactgcgagtcacatatttgtccccaattctcctgaggtcatcagtttaatttttcccctaaggggacctggaagtattgttatgtgggctctaatatccaagagcccccagaaaagtccgagttcctttcttttctcctcttgttttaacaggattatagggacattggcattgacctccagttgagaacctaatttctcaggctgactggccccatttctaactgtaccattctgcctgagacatttggatttgcaatgtcccttgatttaaaaaaaaaaaaaatcaaccaggctgcatgagattcctctggcctttctctatatttatgctttagataatgagtctctctttctgtgaaggcccacatagcacacgtgttagttccctttcagggttcttctgagtactcactttcccagttctctagccaggaatgaacagtcacataagtgtccaaagccaggggatcctgtgccgtgctcccctgtttctgcattcctctctctctgcctcaatcagcaaccagctcacacatctgggtgggggaggtgacctatgcctaccttatcacccttctttcctgatcaaacatccagctgcacatccagcccctgtttgcccaggctgatgcttattggcaaagtgggtagagcagtaacccccagtgccagcctgggggttatttgctgcccctactttgcccataagccatggttctttcagaccagcctctactcactatgtcaattttgtaaagcaggtttactaattaccatttgtctgagtctggtgagacaaaacatacacacaacaagttatgtgcaacagatttattactcacagataggcagcaagagacaaaagaagcttaggatctgttgtgagccaatccctccatgcctcaacaaagctgcacagggcaagtgaagtctcaactgagcatgtcccacttgcattacagctgaggaaccccaacaggaagcccaccctggattatatacatcagaggcacgtaactcatcaggcaaatctttgaaagacatctggcttccagggaaaagtggagtaaagccaaggctgtaccagagtagttcctccctaactcaagacgttgcattcccatcacaatctacagctgttcctgagaactccaagcaagaaaagggagagaactaggtcactccaaggccacccagacaactgacctgcagcaccaaatgtctatacaatgttggtttcacttctctgtggtaccctttttccagggccttggcctagctgacttttttattccttgattataatttttcccaggagacttttaaaactgttcagtctctactttctgcttggcttctctgacacactcaggaaacacacagaggggaaagcacagtagacaaggtcagcctatgctctctctgtagccttgacttttcaggtcctggttttctttctttgttcttcaatctaggctttcttgttgtctcagtgtgatagttgatttgataaaagctactatgatgtagcaagaaatggacgtcttaataatttatggttttagaagttattaatttttagttttattgcccaaacgttttccaagaaagttttaaaaattaataatgcttaagtacatgatacatgtaatgcgctctgtggtttcttcagcttatgcagaattcacaggggactaactgacatatttagctagtacgcacctattttctatgtaaccaatgtatatgtcctccttttttataaagattttctagacatgtaggcccatttaaatgtgaaaatatatgtattttcatatatacatgtatacaaaattttttccaagtgttcaaggatattcacaattttttaatgttttcaatatgcttaaataattacaagcaattaagtgtatatttagtatattcttgcttgggaatttagatcagtattgggttatagatgtctcaaatcttatataatctaatgtgggaatttgtatgttgtataaaatgtatttaaatgtagaactgccttcccaaattaggttaaatgtgattaaacataacctcaagcatgcctaaagaaattctaaacttaactagtgtaataatttttgtaaaagatatggaacaattatttgataaaatttattatgccagaaaaatccagccttgctgctgcagcaactataaatctggcctgattttaaaattcgacaggtaacatttttacaaccacaagatttgagatactagttataaatgaggattctctgtgggaccactattcctgctgaagaaaatgaattcttcaaagtcctctacatattatgtgactttaatatctgaatagtcactgacataaagggttgacttacttttaagttattagtgccagctttctattggctttaagctcagaaatgtaaaaaattcaccttctgagaaatatgacacactttgattaattaatttttaaccaaaaaaaatcaggatgggaaatttgattggcaaggtataatgaaaaatgtacccaatgtcttttgcatgttagtttcatcaagggagatagcttcagtcacataaggtcctaccatattttgaaaagtaaaacacaacagagtaccatcaccatcttaatattgtgttactttctggccttgtcttcttcagctattcagatcttgaatgtctgtaggacattctggcttctatcagaaagaaggctaaactttttcttcttagtataaggagtgaccataaacaatggcttgccaaatcaaggcattcctcgtggtgcagtattacaaaataaagcttcaccctccttggatgtgtaaattgcatgctaggtgagagcacttagaaccacaccttaggtctttactctaaaatacatggtctggattcaccaaaatggcatgaaccctcagtcatactgcaggaaaactgacctcacatcaactattcagcccaatgttggtggcaagattgtccagatcacatccaaagactcttcagctttctgccatcaagcatataaagctcctagaaaaacttccatataatttaaaacaccaaaccttctcagtgaagcagaaccccatggaaagcaggtttagagaattgctccaattctatgagacctctcaaaatatagagctaagaaccaacaaaagataagacagcagctccttagatagcataaacatcagtgacattcacagtttacatctcatacatgtagaataaagataaaaccatcagttttaactattcaataatgcagtgttaaagtctcagatactcatagagtattatctaatagtgacctccttatctatatgaatccaacttcttccagtttatgttaagcttttatttattttttatgcattttttcttgtatgcatttatctcagcagtgtatagtgatgtcttgtatacaaacatttggaaaagataactataaaaaatcaaaatgagtttgtgactgcaattttctacttggcaatttttaatatacattagggcacatgtatgaagatatgtttgatgaaagaaatgaaatgtctgggggaatttgaagtagcttcttccttcatttactgacagaaataattcagataagatcttaaaatattctgtaacatttgcagagtgctttaaacatgaggtagatcttatttttttatttaacatcaaattggctcccattctcaaaaaatctattgtcactaaatctttctgaaacagaaatatacacatatatacatgtctgaataataaaat

SEQ ID NO: 19402 - RNA, 4239 nt, Homo sapiens
  source 1..4239: mol_type = other RNA
ttcatttgcctcccagcctacatgtttctcctgtgctgaatgcttcctgcccttaaacataggacttaaagttcttcagctctgggactcgggctggcttccttgctcctcagtttgcagacggcctattgtgggaccttgtgatcgtattagtttaatactctttaataaactcctatatatataataggtgatatatatatatacaaaataggctatatatacatatcgcctattagttctgtccctctacagaaccctgacttatacacatggcttctttttattttttatgtttgtgggcacatagtaggtgtatatatttaagggatgcatgatgcttgctactttgtctcacaactctcatgtactcagctatgggaaccacagtctctggcacctgaaatggctcaaaggaccccaagcataagcaaataagtactgcgagtcacatatttgtccccaattctcctgaggtcatcagtttaatttttcccctaaggggacctggaagtattgttatgtgggctctaatatccaagagcccccagaaaagtccgagttcctttcttttctcctcttgttttaacaggattatagggacattggcattgacctccagttgagaacctaatttctcaggctgactggccccatttctaactgtaccattctgcctgagacatttggatttgcaatgtcccttgatttaaaaaaaaaaaaaatcaaccaggctgcatgagattcctctggcctttctctatatttatgctttagataatgagtctctctttctgtgaaggcccacatagcacacgtgttagttccctttcagggttcttctgagtactcactttcccagttctctagccaggaatgaacagtcacataagtgtccaaagccaggggatcctgtgccgtgctcccctgtttctgcattcctctctctctgcctcaatcagcaaccagctcacacatctgggtgggggaggtgacctatgcctaccttatcacccttctttcctgatcaaacatccagctgcacatccagcccctgtttgcccaggctgatgcttattggcaaagtgggtagagcagtaacccccagtgccagcctgggggttatttgctgcccctactttgcccataagccatggttctttcagaccagcctctactcactatgtcaattttgtaaagcaggtttactaattaccatttgtctgagtctggtgagacaaaacatacacacaacaagttatgtgcaacagatttattactcacagataggcagcaagagacaaaagaagcttaggatctgttgtgagccaatccctccatgcctcaacaaagctgcacagggcaagtgaagtctcaactgagcatgtcccacttgcattacagctgaggaaccccaacaggaagcccaccctggattatatacatcagaggcacgtaactcatcaggcaaatctttgaaagacatctggcttccagggaaaagtggagtaaagccaaggctgtaccagagtagttcctccctaactcaagacgttgcattcccatcacaatctacagctgttcctgagaactccaagcaagaaaagggagagaactaggtcactccaaggccacccagacaactgacctgcagcaccaaatgtctatacaatgttggtttcacttctctgtggtaccctttttccagggccttggcctagctgacttttttattccttgattataatttttcccaggagacttttaaaactgttcagtctctactttctgcttggcttctctgacacactcaggaaacacacagaggggaaagcacagtagacaaggtcagcctatgctctctctgtagccttgacttttcaggtcctggttttctttctttgttcttcaatctaggctttcttgttgtctcagtgtgatagttgatttgataaaagctactatgatgtagcaagaaatggacgtcttaataatttatggttttagaagttattaatttttagttttattgcccaaacgttttccaagaaagttttaaaaattaataatgcttaagtacatgatacatgtaatgcgctctgtggtttcttcagcttatgcagaattcacaggggactaactgacatatttagctagtacgcacctattttctatgtaaccaatgtatatgtcctccttttttataaagattttctagacatgtaggcccatttaaatgtgaaaatatatgtattttcatatatacatgtatacaaaattttttccaagtgttcaaggatattcacaattttttaatgttttcaatatgcttaaataattacaagcaattaagtgtatatttagtatattcttgcttgggaatttagatcagtattgggttatagatgtctcaaatcttatataatctaatgtgggaatttgtatgttgtataaaatgtatttaaatgtagaactgccttcccaaattaggttaaatgtgattaaacataacctcaagcatgcctaaagaaattctaaacttaactagtgtaataatttttgtaaaagatatggaacaattatttgataaaatttattatgccagaaaaatccagccttgctgctgcagcaactataaatctggcctgattttaaaattcgacaggtaacatttttacaaccacaagatttgagatactagttataaatgaggattctctgtgggaccactattcctgctgaagaaaatgaattcttcaaagtcctctacatattatgtgactttaatatctgaatagtcactgacataaagggttgacttacttttaagttattagtgccagctttctattggctttaagctcagaaatgtaaaaaattcaccttctgagaaatatgacacactttgattaattaatttttaaccaaaaaaaatcaggatgggaaatttgattggcaaggtataatgaaaaatgtacccaatgtcttttgcatgttagtttcatcaagggagatagcttcagtcacataaggtcctaccatattttgaaaagtaaaacacaacagagtaccatcaccatcttaatattgtgttactttctggccttgtcttcttcagctattcagatcttgaatgtctgtaggacattctggcttctatcagaaagaaggctaaactttttcttcttagtataaggagtgaccataaacaatggcttgccaaatcaaggcattcctcgtggtgcagtattacaaaataaagcttcaccctccttggatgtgtaaattgcatgctaggtgagagcacttagaaccacaccttaggtctttactctaaaatacatggtctggattcaccaaaatggcatgaaccctcagtcatactgcaggaaaactgacctcacatcaactattcagcccaatgttggtggcaagattgtccagatcacatccaaagactcttcagctttctgccatcaagcatataaagctcctagaaaaacttccatataatttaaaacaccaaaccttctcagtgaagcagaaccccatggaaagcaggtttagagaattgctccaattctatgagacctctcaaaatatagagctaagaaccaacaaaagataagacagcagctccttagatagcataaacatcagtgacattcacagtttacatctcatacatgtagaataaagataaaaccatcagttttaactattcaataatgcagtgttaaagtctcagatactcatagagtattatctaatagtgacctccttatctatatgaatccaacttcttccagtttatgttaagcttttatttattttttatgcattttttcttgtatgcatttatctcagcagtgtatagtgatgtcttgtatacaaacatttggaaaagataactataaaaaatcaaaatgagtttgtgactgcaattttctacttggcaatttttaatatacattagggcacatgtatgaagatatgtttgatgaaagaaatgaaatgtctgggggaatttgaagtagcttcttccttcatttactgacagaaataattcagataagatcttaaaatattctgtaacatttgcagagtgctttaaacatgaggtagatcttatttttttatttaacatcaaattggctcccattctcaaaaaatctattgtcactaaatctttctgaaacagaaatatacacatatatacatgtctgaataataaaatgg

SEQ ID NO: 19403 - RNA, 4240 nt, Homo sapiens
  source 1..4240: mol_type = other RNA
ttcatttgcctcccagcctacatgtttctcctgtgctgaatgcttcctgcccttaaacataggacttaaagttcttcagctctgggactcgggctggcttccttgctcctcagtttgcagacggcctattgtgggaccttgtgatcgtattagtttaatactctttaataaactcctatatatataataggtgatatatatatatacaaaataggctatatatacatatcgcctattagttctgtccctctacagaaccctgacttatacacatggcttctttttattttttatgtttgtgggcacatagtaggtgtatatatttaagggatgcatgatgcttgctactttgtctcacaactctcatgtactcagctatgggaaccacagtctctggcacctgaaatggctcaaaggaccccaagcataagcaaataagtactgcgagtcacatatttgtccccaattctcctgaggtcatcagtttaatttttcccctaaggggacctggaagtattgttatgtgggctctaatatccaagagcccccagaaaagtccgagttcctttcttttctcctcttgttttaacaggattatagggacattggcattgacctccagttgagaacctaatttctcaggctgactggccccatttctaactgtaccattctgcctgagacatttggatttgcaatgtcccttgatttaaaaaaaaaaaaaatcaaccaggctgcatgagattcctctggcctttctctatatttatgctttagataatgagtctctctttctgtgaaggcccacatagcacacgtgttagttccctttcagggttcttctgagtactcactttcccagttctctagccaggaatgaacagtcacataagtgtccaaagccaggggatcctgtgccgtgctcccctgtttctgcattcctctctctctgcctcaatcagcaaccagctcacacatctgggtgggggaggtgacctatgcctaccttatcacccttctttcctgatcaaacatccagctgcacatccagcccctgtttgcccaggctgatgcttattggcaaagtgggtagagcagtaacccccagtgccagcctgggggttatttgctgcccctactttgcccataagccatggttctttcagaccagcctctactcactatgtcaattttgtaaagcaggtttactaattaccatttgtctgagtctggtgagacaaaacatacacacaacaagttatgtgcaacagatttattactcacagataggcagcaagagacaaaagaagcttaggatctgttgtgagccaatccctccatgcctcaacaaagctgcacagggcaagtgaagtctcaactgagcatgtcccacttgcattacagctgaggaaccccaacaggaagcccaccctggattatatacatcagaggcacgtaactcatcaggcaaatctttgaaagacatctggcttccagggaaaagtggagtaaagccaaggctgtaccagagtagttcctccctaactcaagacgttgcattcccatcacaatctacagctgttcctgagaactccaagcaagaaaagggagagaactaggtcactccaaggccacccagacaactgacctgcagcaccaaatgtctatacaatgttggtttcacttctctgtggtaccctttttccagggccttggcctagctgacttttttattccttgattataatttttcccaggagacttttaaaactgttcagtctctactttctgcttggcttctctgacacactcaggaaacacacagaggggaaagcacagtagacaaggtcagcctatgctctctctgtagccttgacttttcaggtcctggttttctttctttgttcttcaatctaggctttcttgttgtctcagtgtgatagttgatttgataaaagctactatgatgtagcaagaaatggacgtcttaataatttatggttttagaagttattaatttttagttttattgcccaaacgttttccaagaaagttttaaaaattaataatgcttaagtacatgatacatgtaatgcgctctgtggtttcttcagcttatgcagaattcacaggggactaactgacatatttagctagtacgcacctattttctatgtaaccaatgtatatgtcctccttttttataaagattttctagacatgtaggcccatttaaatgtgaaaatatatgtattttcatatatacatgtatacaaaattttttccaagtgttcaaggatattcacaattttttaatgttttcaatatgcttaaataattacaagcaattaagtgtatatttagtatattcttgcttgggaatttagatcagtattgggttatagatgtctcaaatcttatataatctaatgtgggaatttgtatgttgtataaaatgtatttaaatgtagaactgccttcccaaattaggttaaatgtgattaaacataacctcaagcatgcctaaagaaattctaaacttaactagtgtaataatttttgtaaaagatatggaacaattatttgataaaatttattatgccagaaaaatccagccttgctgctgcagcaactataaatctggcctgattttaaaattcgacaggtaacatttttacaaccacaagatttgagatactagttataaatgaggattctctgtgggaccactattcctgctgaagaaaatgaattcttcaaagtcctctacatattatgtgactttaatatctgaatagtcactgacataaagggttgacttacttttaagttattagtgccagctttctattggctttaagctcagaaatgtaaaaaattcaccttctgagaaatatgacacactttgattaattaatttttaaccaaaaaaaatcaggatgggaaatttgattggcaaggtataatgaaaaatgtacccaatgtcttttgcatgttagtttcatcaagggagatagcttcagtcacataaggtcctaccatattttgaaaagtaaaacacaacagagtaccatcaccatcttaatattgtgttactttctggccttgtcttcttcagctattcagatcttgaatgtctgtaggacattctggcttctatcagaaagaaggctaaactttttcttcttagtataaggagtgaccataaacaatggcttgccaaatcaaggcattcctcgtggtgcagtattacaaaataaagcttcaccctccttggatgtgtaaattgcatgctaggtgagagcacttagaaccacaccttaggtctttactctaaaatacatggtctggattcaccaaaatggcatgaaccctcagtcatactgcaggaaaactgacctcacatcaactattcagcccaatgttggtggcaagattgtccagatcacatccaaagactcttcagctttctgccatcaagcatataaagctcctagaaaaacttccatataatttaaaacaccaaaccttctcagtgaagcagaaccccatggaaagcaggtttagagaattgctccaattctatgagacctctcaaaatatagagctaagaaccaacaaaagataagacagcagctccttagatagcataaacatcagtgacattcacagtttacatctcatacatgtagaataaagataaaaccatcagttttaactattcaataatgcagtgttaaagtctcagatactcatagagtattatctaatagtgacctccttatctatatgaatccaacttcttccagtttatgttaagcttttatttattttttatgcattttttcttgtatgcatttatctcagcagtgtatagtgatgtcttgtatacaaacatttggaaaagataactataaaaaatcaaaatgagtttgtgactgcaattttctacttggcaatttttaatatacattagggcacatgtatgaagatatgtttgatgaaagaaatgaaatgtctgggggaatttgaagtagcttcttccttcatttactgacagaaataattcagataagatcttaaaatattctgtaacatttgcagagtgctttaaacatgaggtagatcttatttttttatttaacatcaaattggctcccattctcaaaaaatctattgtcactaaatctttctgaaacagaaatatacacatatatacatgtctgaataataaaatgga

SEQ ID NO: 19404 - RNA, 4273 nt, Homo sapiens
  source 1..4273: mol_type = other RNA
ttcatttgcctcccagcctacatgtttctcctgtgctgaatgcttcctgcccttaaacataggacttaaagttcttcagctctgggactcgggctggcttccttgctcctcagtttgcagacggcctattgtgggaccttgtgatcgtattagtttaatactctttaataaactcctatatatataataggtgatatatatatatacaaaataggctatatatacatatcgcctattagttctgtccctctacagaaccctgacttatacacatggcttctttttattttttatgtttgtgggcacatagtaggtgtatatatttaagggatgcatgatgcttgctactttgtctcacaactctcatgtactcagctatgggaaccacagtctctggcacctgaaatggctcaaaggaccccaagcataagcaaataagtactgcgagtcacatatttgtccccaattctcctgaggtcatcagtttaatttttcccctaaggggacctggaagtattgttatgtgggctctaatatccaagagcccccagaaaagtccgagttcctttcttttctcctcttgttttaacaggattatagggacattggcattgacctccagttgagaacctaatttctcaggctgactggccccatttctaactgtaccattctgcctgagacatttggatttgcaatgtcccttgatttaaaaaaaaaaaaaatcaaccaggctgcatgagattcctctggcctttctctatatttatgctttagataatgagtctctctttctgtgaaggcccacatagcacacgtgttagttccctttcagggttcttctgagtactcactttcccagttctctagccaggaatgaacagtcacataagtgtccaaagccaggggatcctgtgccgtgctcccctgtttctgcattcctctctctctgcctcaatcagcaaccagctcacacatctgggtgggggaggtgacctatgcctaccttatcacccttctttcctgatcaaacatccagctgcacatccagcccctgtttgcccaggctgatgcttattggcaaagtgggtagagcagtaacccccagtgccagcctgggggttatttgctgcccctactttgcccataagccatggttctttcagaccagcctctactcactatgtcaattttgtaaagcaggtttactaattaccatttgtctgagtctggtgagacaaaacatacacacaacaagttatgtgcaacagatttattactcacagataggcagcaagagacaaaagaagcttaggatctgttgtgagccaatccctccatgcctcaacaaagctgcacagggcaagtgaagtctcaactgagcatgtcccacttgcattacagctgaggaaccccaacaggaagcccaccctggattatatacatcagaggcacgtaactcatcaggcaaatctttgaaagacatctggcttccagggaaaagtggagtaaagccaaggctgtaccagagtagttcctccctaactcaagacgttgcattcccatcacaatctacagctgttcctgagaactccaagcaagaaaagggagagaactaggtcactccaaggccacccagacaactgacctgcagcaccaaatgtctatacaatgttggtttcacttctctgtggtaccctttttccagggccttggcctagctgacttttttattccttgattataatttttcccaggagacttttaaaactgttcagtctctactttctgcttggcttctctgacacactcaggaaacacacagaggggaaagcacagtagacaaggtcagcctatgctctctctgtagccttgacttttcaggtcctggttttctttctttgttcttcaatctaggctttcttgttgtctcagtgtgatagttgatttgataaaagctactatgatgtagcaagaaatggacgtcttaataatttatggttttagaagttattaatttttagttttattgcccaaacgttttccaagaaagttttaaaaattaataatgcttaagtacatgatacatgtaatgcgctctgtggtttcttcagcttatgcagaattcacaggggactaactgacatatttagctagtacgcacctattttctatgtaaccaatgtatatgtcctccttttttataaagattttctagacatgtaggcccatttaaatgtgaaaatatatgtattttcatatatacatgtatacaaaattttttccaagtgttcaaggatattcacaattttttaatgttttcaatatgcttaaataattacaagcaattaagtgtatatttagtatattcttgcttgggaatttagatcagtattgggttatagatgtctcaaatcttatataatctaatgtgggaatttgtatgttgtataaaatgtatttaaatgtagaactgccttcccaaattaggttaaatgtgattaaacataacctcaagcatgcctaaagaaattctaaacttaactagtgtaataatttttgtaaaagatatggaacaattatttgataaaatttattatgccagaaaaatccagccttgctgctgcagcaactataaatctggcctgattttaaaattcgacaggtaacatttttacaaccacaagatttgagatactagttataaatgaggattctctgtgggaccactattcctgctgaagaaaatgaattcttcaaagtcctctacatattatgtgactttaatatctgaatagtcactgacataaagggttgacttacttttaagttattagtgccagctttctattggctttaagctcagaaatgtaaaaaattcaccttctgagaaatatgacacactttgattaattaatttttaaccaaaaaaaatcaggatgggaaatttgattggcaaggtataatgaaaaatgtacccaatgtcttttgcatgttagtttcatcaagggagatagcttcagtcacataaggtcctaccatattttgaaaagtaaaacacaacagagtaccatcaccatcttaatattgtgttactttctggccttgtcttcttcagctattcagatcttgaatgtctgtaggacattctggcttctatcagaaagaaggctaaactttttcttcttagtataaggagtgaccataaacaatggcttgccaaatcaaggcattcctcgtggtgcagtattacaaaataaagcttcaccctccttggatgtgtaaattgcatgctaggtgagagcacttagaaccacaccttaggtctttactctaaaatacatggtctggattcaccaaaatggcatgaaccctcagtcatactgcaggaaaactgacctcacatcaactattcagcccaatgttggtggcaagattgtccagatcacatccaaagactcttcagctttctgccatcaagcatataaagctcctagaaaaacttccatataatttaaaacaccaaaccttctcagtgaagcagaaccccatggaaagcaggtttagagaattgctccaattctatgagacctctcaaaatatagagctaagaaccaacaaaagataagacagcagctccttagatagcataaacatcagtgacattcacagtttacatctcatacatgtagaataaagataaaaccatcagttttaactattcaataatgcagtgttaaagtctcagatactcatagagtattatctaatagtgacctccttatctatatgaatccaacttcttccagtttatgttaagcttttatttattttttatgcattttttcttgtatgcatttatctcagcagtgtatagtgatgtcttgtatacaaacatttggaaaagataactataaaaaatcaaaatgagtttgtgactgcaattttctacttggcaatttttaatatacattagggcacatgtatgaagatatgtttgatgaaagaaatgaaatgtctgggggaatttgaagtagcttcttccttcatttactgacagaaataattcagataagatcttaaaatattctgtaacatttgcagagtgctttaaacatgaggtagatcttatttttttatttaacatcaaattggctcccattctcaaaaaatctattgtcactaaatctttctgaaacagaaatatacacatatatacatgtctgaataataaaatggaaacattttaaaatttttgataaatatttcatga

SEQ ID NO: 19405 - RNA, 7629 nt, Homo sapiens
  source 1..7629: mol_type = other RNA
ttccactgccactacctaatttatctattgttttgctaagaggtagataaaacaaaagtgaaatggggcttctatgaggaggtccattagagggtgggtggggaggggctgggatcgcccagtggaactcccccaactacaaagacggcctgaatgagtccaaggaccgcgccctcagactcccccagggcaaaggatcctgcttcacctcttctccttctagagccaactgggcccccattgaagactgaaaaagggcccaatggaggtgtaggatctcaaagaaaccctgttgaagaggtctcagctctggtttccccaggcttcctgactttggggctgtgtggtgggttccaggccaagccccaggtctcactccagccagccccctctagaagggaagaggccattcctttcctcaccatctggtccaacaaagctatagaaagtgagagagggacaagctggaggccaaaggggtgacacatgggcaaggaaagcagaaagtggggacctcatggccagccctcccagcccaatcgatatgggggggatcctggcaggcctgcctgttccccaaggacaaaccttttgtggcacaagcctcaactcacttgtcctggctgggattcatacccttatgcatgagtccctgcccttagttccaatcttactgtaaggattgaggtagttaatccatttatactcgtagcatccatcacctgcggttaatcaaaacacatgctcccgaggagcttcctgctatttcattcaagaaaaaaaattttttttcttttgtccatccggagtcaaccatactaaggcgccagcaaaggcgccatcagactgtgccccaaagcggtgcacaggaccgagggtcagggctggggctctcgcccctaaatcccccttcagacatgaggcctcctccctgtcccgtaccccgatagagaagccttatgtatccaaaggaaagaaactgcagttttcagctggtgttactctaagtctgaatacagagaaatgttctgcatctaaattgtcgagtatttggaagggaaatggcttttatgtcccctggcattgatgaggatttttcttcaatcttcctgcaattactgtgacaggctgtgctgtttcccttctactggttttcaagaaacaggcaaacagtcgagtggtttgaatggcaaagccactaggatctccccataaacacttcaggggaaagaaaggagaacccccacccctgatgagaggtgggaggaaggggttgcctagaggcaccagcttctcctgtggagcaagaaggctcaagcaggccctctggggctctgtgaggtagttactagcactgctggttcccagtttggcagagggtatgtctgggttgggaggaggggaaggcacccttgagagctaactgaggcccctcctcactgcccgtctgccaggcctgaagggaactcggcagtgctatctctgcagtaggggcaggggacagagcagtcccacaacagggagctacctggagccccaaacttcctctccttccccaaagtgcaaccaggagccgacagaccaatttctcggctccctaccccttggcttggcaaacaccacaccctaatcccccaggagcctctgaagggaagggcctcgcccttagctcccagtttccaggaggccttcctcctcagacagccaggtatgtgtcgaaagctggctattgctttgattcaggaacagcctctctcagcctctgtctgtctgtctttggcacagaggaaaatggacacagaaccaactagagcatccccctccagtgttctctgggttttaaatggggtcttttctgccaatagtgaggcataaacaaggatagctcccaactgcctccagaaggagggggtcaggaaaaaggaaaaaagattgataaggactgggaggaggggaggaaagtagaaaagggctataaaactccctgtccttaaaaatggctctctcctaaccagacccctcacaggagctgagtccacaacccaaactgcaaaaggcaaccagacccgagaggggattaaagccatttggggtgtaactggcagatgcagcttcaaagtcagtcagtgaatcaaaccattttggttatgtgtttcaaagaatttaaaaatatatcctaaagagatggtcctttcttaaaaatatatatgtagcacacacacacacatatatatcttagagcacagaagcattttttttaagtcactcttctcaaatcatccaaatctcccaagtgcttttcgcgatagcttgttatctcaccaaggatggggaaatggaggtgctgagcaggagggcaaggagttgccctaagacctagcctacggggcacaagagggcccggcccaccaagacaggtccttcatcccactaaaccttaaccaccaaaccatgctccttttgctttctggtggtataacttacatgattttcctgctgggcaaatatcaacaatgagtggagccttgcctaatccaagcaagtgaagttttccagtcccttgccacacacttcctcgtctcttctgggagctgaatcagccaacggaaaaggacttgggctcaaggtgtgaagggagcaggcccccaaggaaactgaacactgcaacaatcacatttcaggtactgtgggatttttttttcttcctgatgatagtctgaaccagatatcaaagcatgcttgctgctggaaattcgctttaaattactaaatggccgacgtctgaacgttatctgctttgttttgggataaagcatatagagccagagatggaaagctgggagaccctttttatggttgggacaggtggagaggcttaattctactggcctgatgttatccctaaatgtttttctgcttctattcaatttgggccagacaattctgggggctacaagggaatgtcctagggagaaaatgataaggcaggaacctgtcccagtcacgtccccatatcccctgcccctccttgccaccagccaccctaaatcaagaattccctaagtttgggtccacttttaaaatcaatcagaccgatctaaagaagacagggagacagaggtgggggcagttaactagtatctgtttgccccttagatctatggatatagattaggaagaatagcaagacggaactgaaatgaaacaataacaaaaaaaaaaaatgaaaagcattgcaatgacaaaccaggtggacctctctgagggcgagagggtggccttgtcttttttccacgaacggaatctcagctcccatatttttagacagagaaatataggtttttttaaagggtatattttttagttattatttctctcctcgataaaacggaggcaatattttaaaatatctcaacagcaccactggtgggaaaagctggctgagatgctctttaaccaaaggaggaaagagaggagaccaagggccagctggttggttgttgggcattgtttaaccactgagagcccccagctccactaggccttttaatcctatcaggtaggatattccagcagccgccagcagctggggctctagaagtcagagatcagggccaaacaaggctctgggctctgcccctctgggctctctcaaacctgggccttccctcttagcactagcctcctcctaagggggcagcccccaaagcctttcccaccaggcctgttctccatagagagttcctaaagggttactggctcatgttgtaagaaattatgaaacataactttcttgttttttcttttcattaaaaaaataaaatattcaagactatcagcttctcttttgctttgcttttcttttttatataaaatatcagcaagctgcaaaaaaacaaaaatcaaaaaaaaatttttttaatggggttggggggaacaaaaaggaaaataattgctgaggtaacttcataccttgaggtagtttacttcgcacacagcattgcctgactacgcccacatgttgcggttgtcttgttgttactgttgttgcaatgttgaaaggaggggaactccacgcatgggcttttccatatgtagagaggccttcctcccttcccagcacacttgatagcattgtccagggtagctaaagtgcattacctggctaatatgcattgtcaatcagtatattaggaggagaggcctaacctcatttaactgatggcttctgtctcccacaagggctaaacactccatgggatcttaattaagcctggtaaattaataaattaagcttatttaccccttgctgtacaatgctgctggtattctgaattgttttttagacacacctttcatcatgctgataatgattcatggagacagaagccgtcagttaaaaattcctctcagatacaaacagaagcaagtactctccaatttactgaatttgccagatgatggactttagctttatcgggagctcagggttgggttccaagtcccaccaccaaggtaacagtgccgtggctgggagtgccccacaacccctgcctctaggaaccagcccttatgggagcacatgggctggggtgagggcaccgtggcagcctttggggccactcaagtcctccatggaaccgagactttatcaaggggagttagcgtccccttcccagtgctcatatccaatcattaaaatagactttaaaaaaatataaaatccgcctgagaacgatgggaatcagggacagtggtcagcccctaccctgctgagcattcaataccacctatgtgcacctggacataatgtgaaacctacacgggagagggacatgaatgtggtggggaagccccaacagagtggggaaatttcagttgtgccaatttgaagatggtgatctggcatagatcagccacaagtgcgctccttttaaacgtggattattatgtattttaaccatctttctccccattttcccctcttcttcattccgtattgtacctattggttagggagtgattggaattaatctacagatactgacagttcttttcccttgagtcaatactgtaagcaaagcaatgcattcgttcgcatttttttctggtagcaataaagataaaaaaattagtgtaaatatagaaagaggccgtaaatggaggtattttaatcaattacccaagtagggggaagaagattggaaaaacattaaggtcaagaaatgaaccatcctttaaggctgattaaaacacctctctgcatgtttttaaaacctgaaggaaattttatttttcttcccactgaggtgtgatccaccctcttggtggggcctggagagcttctttaaacaatccacgtttaaaagtgccttgcgctagaatttctgacaccccgaggggcagacagtgttgggccaattgggtgggtgtttggggctgagagatcagggttcctcactggaacatctttctcaatcaagtgggcaaacctgatctacagcccggcccaggtgtcccggattcccactcattctcaggcctgccggggagagcacactctcgatttctgcccgttgttgtcctggactcgaagggacagggaggggctggtcacttcctccgtgcctgggcctggttactctgtcccttctgatgctgctgcttaacctgggccaggatgtctcggatcttccgttgagccatctgactggcatagaaatgtccgatgattttcacgatgacctggtcgttctcatcaggggtctggtctcttggtactaccacctcagctgccgtcaaattctgcaactcgttcaccgtttttccacctttgccaatgacccggccagctgctgatgctggcacacgtatgtgggtctccagcttcacttcctccttgggaccaaagaagttctcctccttgagtttgccatagattcttccctgagccttgaattgggcctctggcggtccagtgatgataaccatacgaactttggagtcaggtgtttcgggtggtgcaatcttgatggaggcgctggcaaaccgggagagctgtttgatgtgctgccccttcttgccgatgatggcgcccactgcctgggcggggataaacacctgcaccatctcctgctcgggagccataaaggagctatagggagcagccccagtaacgctgctgggaggcggcgggactgcgctggatgaagctgggaaaagacctacagcagccaggttcaggccagggatcaggtgagactgcaggctcatggcagccacatcattctcataggcctcccgaactttcttcattatttcctgctcggccctgcaacaattctcgatggcccccttcacagtgatggtcctctcagggttgtaaagggtaaggtcttgcaacgaggagatggtgatttttgtctcggtatcttgctctaccttcttcaggttccgtccttccttgccaatgagacgccctacaaagttattatgggccaggatcttcaggggaacctcgtcagccgttttggtgtccttagcctctttatgcataatctccaagatcatcttacaagcggaggagcagccctcaggggtggagtgcacactgatggctttttcagctgcacctgcgttctccttcctatgcacgtctatcttggactgggtctgttttgtgatgttgcggatggtggccccctccttgccaataatggcacccacatactgggtgggcaccaggagccgaagggggatgtccacttgctgctgcttggctggggcccccgctgccacaggtgagccctggcggggctgaccccgagagccaaagccccctcggcgcccattctcaggtccctgtgctatctgctcatcggggatgtaggagaccttcagggcatggttctccaactggtggccattcagcttcatgatggcttgcctggtctgctcccggttggaataggtgacattcaccactgccgtctcactctcggtgttcacttgctcacagttctctactgtaccatactgagccagcaggctgtccagtacttcccatcggagctggggtggaatatttcggatttgaattttccggctcctttgttttttgggcaccgaatgttcaatctctaagcgttttccttgtaattctactttcccggagaaagtttcgatggccttcatcgcccagtgctcgtccgggcagtccacgaaggcgtagccggatttgaccaagaactggccgctgtaggagatcttgtgctccgcaaacactttctccaagtccgcgggggtcacgctctcgttgaggttgccgatgtaaagcttgttcatggtggcggtctcggggcaggacgcggtcccgggcaaggccgaacgagcgggcgcgggcggcgagcctcctaggccaagaggcggagaggccggcggcaggagccgcaaactttctttgcaccccaccccagaagttgtcccgagcccagggcggggaaggcggcctgagggcgcgcagaggtcgcgggagagttcggggagagcccaggagaagtgcccgcggcgcgcagggagacggacgacacggcgcagcttcttcccttcggtccgaaacccctccgagag

SEQ ID NO: 19406 - RNA, 7404 nt, Homo sapiens
  source 1..7404: mol_type = other RNA
ttccactgccactacctaatttatctattgttttgctaagaggtagataaaacaaaagtgaaatggggcttctatgaggaggtccattagagggtgggtggggaggggctgggatcgcccagtggaactcccccaactacaaagacggcctgaatgagtccaaggaccgcgccctcagactcccccagggcaaaggatcctgcttcacctcttctccttctagagccaactgggcccccattgaagactgaaaaagggcccaatggaggtgtaggatctcaaagaaaccctgttgaagaggtctcagctctggtttccccaggcttcctgactttggggctgtgtggtgggttccaggccaagccccaggtctcactccagccagccccctctagaagggaagaggccattcctttcctcaccatctggtccaacaaagctatagaaagtgagagagggacaagctggaggccaaaggggtgacacatgggcaaggaaagcagaaagtggggacctcatggccagccctcccagcccaatcgatatgggggggatcctggcaggcctgcctgttccccaaggacaaaccttttgtggcacaagcctcaactcacttgtcctggctgggattcatacccttatgcatgagtccctgcccttagttccaatcttactgtaaggattgaggtagttaatccatttatactcgtagcatccatcacctgcggttaatcaaaacacatgctcccgaggagcttcctgctatttcattcaagaaaaaaaattttttttcttttgtccatccggagtcaaccatactaaggcgccagcaaaggcgccatcagactgtgccccaaagcggtgcacaggaccgagggtcagggctggggctctcgcccctaaatcccccttcagacatgaggcctcctccctgtcccgtaccccgatagagaagccttatgtatccaaaggaaagaaactgcagttttcagctggtgttactctaagtctgaatacagagaaatgttctgcatctaaattgtcgagtatttggaagggaaatggcttttatgtcccctggcattgatgaggatttttcttcaatcttcctgcaattactgtgacaggctgtgctgtttcccttctactggttttcaagaaacaggcaaacagtcgagtggtttgaatggcaaagccactaggatctccccataaacacttcaggggaaagaaaggagaacccccacccctgatgagaggtgggaggaaggggttgcctagaggcaccagcttctcctgtggagcaagaaggctcaagcaggccctctggggctctgtgaggtagttactagcactgctggttcccagtttggcagagggtatgtctgggttgggaggaggggaaggcacccttgagagctaactgaggcccctcctcactgcccgtctgccaggcctgaagggaactcggcagtgctatctctgcagtaggggcaggggacagagcagtcccacaacagggagctacctggagccccaaacttcctctccttccccaaagtgcaaccaggagccgacagaccaatttctcggctccctaccccttggcttggcaaacaccacaccctaatcccccaggagcctctgaagggaagggcctcgcccttagctcccagtttccaggaggccttcctcctcagacagccaggtatgtgtcgaaagctggctattgctttgattcaggaacagcctctctcagcctctgtctgtctgtctttggcacagaggaaaatggacacagaaccaactagagcatccccctccagtgttctctgggttttaaatggggtcttttctgccaatagtgaggcataaacaaggatagctcccaactgcctccagaaggagggggtcaggaaaaaggaaaaaagattgataaggactgggaggaggggaggaaagtagaaaagggctataaaactccctgtccttaaaaatggctctctcctaaccagacccctcacaggagctgagtccacaacccaaactgcaaaaggcaaccagacccgagaggggattaaagccatttggggtgtaactggcagatgcagcttcaaagtcagtcagtgaatcaaaccattttggttatgtgtttcaaagaatttaaaaatatatcctaaagagatggtcctttcttaaaaatatatatgtagcacacacacacacatatatatcttagagcacagaagcattttttttaagtcactcttctcaaatcatccaaatctcccaagtgcttttcgcgatagcttgttatctcaccaaggatggggaaatggaggtgctgagcaggagggcaaggagttgccctaagacctagcctacggggcacaagagggcccggcccaccaagacaggtccttcatcccactaaaccttaaccaccaaaccatgctccttttgctttctggtggtataacttacatgattttcctgctgggcaaatatcaacaatgagtggagccttgcctaatccaagcaagtgaagttttccagtcccttgccacacacttcctcgtctcttctgggagctgaatcagccaacggaaaaggacttgggctcaaggtgtgaagggagcaggcccccaaggaaactgaacactgcaacaatcacatttcaggtactgtgggatttttttttcttcctgatgatagtctgaaccagatatcaaagcatgcttgctgctggaaattcgctttaaattactaaatggccgacgtctgaacgttatctgctttgttttgggataaagcatatagagccagagatggaaagctgggagaccctttttatggttgggacaggtggagaggcttaattctactggcctgatgttatccctaaatgtttttctgcttctattcaatttgggccagacaattctgggggctacaagggaatgtcctagggagaaaatgataaggcaggaacctgtcccagtcacgtccccatatcccctgcccctccttgccaccagccaccctaaatcaagaattccctaagtttgggtccacttttaaaatcaatcagaccgatctaaagaagacagggagacagaggtgggggcagttaactagtatctgtttgccccttagatctatggatatagattaggaagaatagcaagacggaactgaaatgaaacaataacaaaaaaaaaaaatgaaaagcattgcaatgacaaaccaggtggacctctctgagggcgagagggtggccttgtcttttttccacgaacggaatctcagctcccatatttttagacagagaaatataggtttttttaaagggtatattttttagttattatttctctcctcgataaaacggaggcaatattttaaaatatctcaacagcaccactggtgggaaaagctggctgagatgctctttaaccaaaggaggaaagagaggagaccaagggccagctggttggttgttgggcattgtttaaccactgagagcccccagctccactaggccttttaatcctatcaggtaggatattccagcagccgccagcagctggggctctagaagtcagagatcagggccaaacaaggctctgggctctgcccctctgggctctctcaaacctgggccttccctcttagcactagcctcctcctaagggggcagcccccaaagcctttcccaccaggcctgttctccatagagagttcctaaagggttactggctcatgttgtaagaaattatgaaacataactttcttgttttttcttttcattaaaaaaataaaatattcaagactatcagcttctcttttgctttgcttttcttttttatataaaatatcagcaagctgcaaaaaaacaaaaatcaaaaaaaaatttttttaatggggttggggggaacaaaaaggaaaataattgctgaggtaacttcataccttgaggtagtttacttcgcacacagcattgcctgactacgcccacatgttgcggttgtcttgttgttactgttgttgcaatgttgaaaggaggggaactccacgcatgggcttttccatatgtagagaggccttcctcccttcccagcacacttgatagcattgtccagggtagctaaagtgcattacctggctaatatgcattgtcaatcagtatattaggaggagaggcctaacctcatttaactgatggcttctgtctcccacaagggctaaacactccatgggatcttaattaagcctggtaaattaataaattaagcttatttaccccttgctgtacaatgctgctggtattctgaattgttttttagacacacctttcatcatgctgataatgattcatggagacagaagccgtcagttaaaaattcctctcagatacaaacagaagcaagtactctccaatttactgaatttgccagatgatggactttagctttatcgggagctcagggttgggttccaagtcccaccaccaaggtaacagtgccgtggctgggagtgccccacaacccctgcctctaggaaccagcccttatgggagcacatgggctggggtgagggcaccgtggcagcctttggggccactcaagtcctccatggaaccgagactttatcaaggggagttagcgtccccttcccagtgctcatatccaatcattaaaatagactttaaaaaaatataaaatccgcctgagaacgatgggaatcagggacagtggtcagcccctaccctgctgagcattcaataccacctatgtgcacctggacataatgtgaaacctacacgggagagggacatgaatgtggtggggaagccccaacagagtggggaaatttcagttgtgccaatttgaagatggtgatctggcatagatcagccacaagtgcgctccttttaaacgtggattattatgtattttaaccatctttctccccattttcccctcttcttcattccgtattgtacctattggttagggagtgattggaattaatctacagatactgacagttcttttcccttgagtcaatactgtaagcaaagcaatgcattcgttcgcatttttttctggtagcaataaagataaaaaaattagtgtaaatatagaaagaggccgtaaatggaggtattttaatcaattacccaagtagggggaagaagattggaaaaacattaaggtcaagaaatgaaccatcctttaaggctgattaaaacacctctctgcatgtttttaaaacctgaaggaaattttatttttcttcccactgaggtgtgatccaccctcttggtggggcctggagagcttctttaaacaatccacgtttaaaagtgccttgcgctagaatttctgacaccccgaggggcagacagtgttgggccaattgggtgggtgtttggggctgagagatcagggttcctcactggaacatctttctcaatcaagtgggcaaacctgatctacagcccggcccaggtgtcccggattcccactcattctcaggcctgccggggagagcacactctcgatttctgcccgttgttgtcctggactcgaagggacagggaggggctggtcacttcctccgtgcctgggcctggttactctgtcccttctgatgctgctgcttaacctgggccaggatgtctcggatcttccgttgagccatctgactggcatagaaatgtccgatgattttcacgatgacctggtcgttctcatcaggggtctggtctcttggtactaccacctcagctgccgtcaaattctgcaactcgttcaccgtttttccacctttgccaatgacccggccagctgctgatgctggcacacgtatgtgggtctccagcttcacttcctccttgggaccaaagaagttctcctccttgagtttgccatagattcttccctgagccttgaattgggcctctggcggtccagtgatgataaccatacgaactttggagtcaggtgtttcgggtggtgcaatcttgatggaggcgctggcaaaccgggagagctgtttgatgtgctgccccttcttgccgatgatggcgcccactgcctgggcggggataaacacctgcaccatctcctgctcgggagcctgcataaaggagctatagggagcagccccagtaacgctgctgggaggcggcgggactgcgctggatgaagctgggaaaagacctacagcagccaggttcaggccagggatcaggtgagactgcaggctcatggcagccacatcattctcataggcctcccgaactttcttcattatttcctgctcggccctgcaacaattctcgatggcccccttcacagtgatggtcctctcagggttgtaaagggtaaggtcttgcaacgaggagatggtgatttttgtctcggtatcttgctctaccttcttcaggttccgtccttccttgccaatgagacgccctacaaagttattatgggccaggatcttcaggggaacctcgtcagccgttttggtgtccttagcctctttatgcataatctccaagatcatcttacaagcggaggagcagccctcaggggtggagtgcacactgatggctttttcagctgcacctgcgttctccttcctatgcacgtctatcttggactgggtctgttttgtgatgttgcggatggtggccccctccttgccaataatggcacccacatactgggtgggcaccaggagccgaagggggatgtccacttgctgctgcttggctggggcccccgctgccacaggtgagccctggcggggctgaccccgagagccaaagccccctcggcgcccattctcaggtccctgtgctatctgctcatcggggatgtaggagaccttcagggcatggttctccaactggtggccattcagcttcatgatggcttgcctggtctgctcccggttggaataggtgacattcaccactgccgtctcactctcggtgttcacttgctcacagttctctactgtaccatactgagccagcaggctgtccagtacttcccatcggagctggggtggaatatttcggatttgaattttccggctccttgaaaacagacagagtcgggctctgtcctccagagggaacagccgaggtggccctctcaggagccaggagaggaaaccagaccagcctccaaagcaatctgtcttcggcagcttcccaccgcaccatgagaaggacccggcagacatccccgtgctcctcggggtccttagtgccccctgatgacgatgggcaaacatctgggcaccagccccgcaagcgtctgcgtgtccataagtggcggccgctgcgcagtagccctcagggatccgcgtctccccctagctgccaac

SEQ ID NO: 19407 - RNA, 7708 nt, Homo sapiens
  source 1..7708: mol_type = other RNA
ttccactgccactacctaatttatctattgttttgctaagaggtagataaaacaaaagtgaaatggggcttctatgaggaggtccattagagggtgggtggggaggggctgggatcgcccagtggaactcccccaactacaaagacggcctgaatgagtccaaggaccgcgccctcagactcccccagggcaaaggatcctgcttcacctcttctccttctagagccaactgggcccccattgaagactgaaaaagggcccaatggaggtgtaggatctcaaagaaaccctgttgaagaggtctcagctctggtttccccaggcttcctgactttggggctgtgtggtgggttccaggccaagccccaggtctcactccagccagccccctctagaagggaagaggccattcctttcctcaccatctggtccaacaaagctatagaaagtgagagagggacaagctggaggccaaaggggtgacacatgggcaaggaaagcagaaagtggggacctcatggccagccctcccagcccaatcgatatgggggggatcctggcaggcctgcctgttccccaaggacaaaccttttgtggcacaagcctcaactcacttgtcctggctgggattcatacccttatgcatgagtccctgcccttagttccaatcttactgtaaggattgaggtagttaatccatttatactcgtagcatccatcacctgcggttaatcaaaacacatgctcccgaggagcttcctgctatttcattcaagaaaaaaaattttttttcttttgtccatccggagtcaaccatactaaggcgccagcaaaggcgccatcagactgtgccccaaagcggtgcacaggaccgagggtcagggctggggctctcgcccctaaatcccccttcagacatgaggcctcctccctgtcccgtaccccgatagagaagccttatgtatccaaaggaaagaaactgcagttttcagctggtgttactctaagtctgaatacagagaaatgttctgcatctaaattgtcgagtatttggaagggaaatggcttttatgtcccctggcattgatgaggatttttcttcaatcttcctgcaattactgtgacaggctgtgctgtttcccttctactggttttcaagaaacaggcaaacagtcgagtggtttgaatggcaaagccactaggatctccccataaacacttcaggggaaagaaaggagaacccccacccctgatgagaggtgggaggaaggggttgcctagaggcaccagcttctcctgtggagcaagaaggctcaagcaggccctctggggctctgtgaggtagttactagcactgctggttcccagtttggcagagggtatgtctgggttgggaggaggggaaggcacccttgagagctaactgaggcccctcctcactgcccgtctgccaggcctgaagggaactcggcagtgctatctctgcagtaggggcaggggacagagcagtcccacaacagggagctacctggagccccaaacttcctctccttccccaaagtgcaaccaggagccgacagaccaatttctcggctccctaccccttggcttggcaaacaccacaccctaatcccccaggagcctctgaagggaagggcctcgcccttagctcccagtttccaggaggccttcctcctcagacagccaggtatgtgtcgaaagctggctattgctttgattcaggaacagcctctctcagcctctgtctgtctgtctttggcacagaggaaaatggacacagaaccaactagagcatccccctccagtgttctctgggttttaaatggggtcttttctgccaatagtgaggcataaacaaggatagctcccaactgcctccagaaggagggggtcaggaaaaaggaaaaaagattgataaggactgggaggaggggaggaaagtagaaaagggctataaaactccctgtccttaaaaatggctctctcctaaccagacccctcacaggagctgagtccacaacccaaactgcaaaaggcaaccagacccgagaggggattaaagccatttggggtgtaactggcagatgcagcttcaaagtcagtcagtgaatcaaaccattttggttatgtgtttcaaagaatttaaaaatatatcctaaagagatggtcctttcttaaaaatatatatgtagcacacacacacacatatatatcttagagcacagaagcattttttttaagtcactcttctcaaatcatccaaatctcccaagtgcttttcgcgatagcttgttatctcaccaaggatggggaaatggaggtgctgagcaggagggcaaggagttgccctaagacctagcctacggggcacaagagggcccggcccaccaagacaggtccttcatcccactaaaccttaaccaccaaaccatgctccttttgctttctggtggtataacttacatgattttcctgctgggcaaatatcaacaatgagtggagccttgcctaatccaagcaagtgaagttttccagtcccttgccacacacttcctcgtctcttctgggagctgaatcagccaacggaaaaggacttgggctcaaggtgtgaagggagcaggcccccaaggaaactgaacactgcaacaatcacatttcaggtactgtgggatttttttttcttcctgatgatagtctgaaccagatatcaaagcatgcttgctgctggaaattcgctttaaattactaaatggccgacgtctgaacgttatctgctttgttttgggataaagcatatagagccagagatggaaagctgggagaccctttttatggttgggacaggtggagaggcttaattctactggcctgatgttatccctaaatgtttttctgcttctattcaatttgggccagacaattctgggggctacaagggaatgtcctagggagaaaatgataaggcaggaacctgtcccagtcacgtccccatatcccctgcccctccttgccaccagccaccctaaatcaagaattccctaagtttgggtccacttttaaaatcaatcagaccgatctaaagaagacagggagacagaggtgggggcagttaactagtatctgtttgccccttagatctatggatatagattaggaagaatagcaagacggaactgaaatgaaacaataacaaaaaaaaaaaatgaaaagcattgcaatgacaaaccaggtggacctctctgagggcgagagggtggccttgtcttttttccacgaacggaatctcagctcccatatttttagacagagaaatataggtttttttaaagggtatattttttagttattatttctctcctcgataaaacggaggcaatattttaaaatatctcaacagcaccactggtgggaaaagctggctgagatgctctttaaccaaaggaggaaagagaggagaccaagggccagctggttggttgttgggcattgtttaaccactgagagcccccagctccactaggccttttaatcctatcaggtaggatattccagcagccgccagcagctggggctctagaagtcagagatcagggccaaacaaggctctgggctctgcccctctgggctctctcaaacctgggccttccctcttagcactagcctcctcctaagggggcagcccccaaagcctttcccaccaggcctgttctccatagagagttcctaaagggttactggctcatgttgtaagaaattatgaaacataactttcttgttttttcttttcattaaaaaaataaaatattcaagactatcagcttctcttttgctttgcttttcttttttatataaaatatcagcaagctgcaaaaaaacaaaaatcaaaaaaaaatttttttaatggggttggggggaacaaaaaggaaaataattgctgaggtaacttcataccttgaggtagtttacttcgcacacagcattgcctgactacgcccacatgttgcggttgtcttgttgttactgttgttgcaatgttgaaaggaggggaactccacgcatgggcttttccatatgtagagaggccttcctcccttcccagcacacttgatagcattgtccagggtagctaaagtgcattacctggctaatatgcattgtcaatcagtatattaggaggagaggcctaacctcatttaactgatggcttctgtctcccacaagggctaaacactccatgggatcttaattaagcctggtaaattaataaattaagcttatttaccccttgctgtacaatgctgctggtattctgaattgttttttagacacacctttcatcatgctgataatgattcatggagacagaagccgtcagttaaaaattcctctcagatacaaacagaagcaagtactctccaatttactgaatttgccagatgatggactttagctttatcgggagctcagggttgggttccaagtcccaccaccaaggtaacagtgccgtggctgggagtgccccacaacccctgcctctaggaaccagcccttatgggagcacatgggctggggtgagggcaccgtggcagcctttggggccactcaagtcctccatggaaccgagactttatcaaggggagttagcgtccccttcccagtgctcatatccaatcattaaaatagactttaaaaaaatataaaatccgcctgagaacgatgggaatcagggacagtggtcagcccctaccctgctgagcattcaataccacctatgtgcacctggacataatgtgaaacctacacgggagagggacatgaatgtggtggggaagccccaacagagtggggaaatttcagttgtgccaatttgaagatggtgatctggcatagatcagccacaagtgcgctccttttaaacgtggattattatgtattttaaccatctttctccccattttcccctcttcttcattccgtattgtacctattggttagggagtgattggaattaatctacagatactgacagttcttttcccttgagtcaatactgtaagcaaagcaatgcattcgttcgcatttttttctggtagcaataaagataaaaaaattagtgtaaatatagaaagaggccgtaaatggaggtattttaatcaattacccaagtagggggaagaagattggaaaaacattaaggtcaagaaatgaaccatcctttaaggctgattaaaacacctctctgcatgtttttaaaacctgaaggaaattttatttttcttcccactgaggtgtgatccaccctcttggtggggcctggagagcttctttaaacaatccacgtttaaaagtgccttgcgctagaatttctgacaccccgaggggcagacagtgttgggccaattgggtgggtgtttggggctgagagatcagggttcctcactggaacatctttctcaatcaagtgggcaaacctgatctacagcccggcccaggtgtcccggattcccactcattctcaggcctgccggggagagcacactctcgatttctgcccgttgttgtcctggactcgaagggacagggaggggctggtcacttcctccgtgcctgggcctggttactctgtcccttctgatgctgctgcttaacctgggccaggatgtctcggatcttccgttgagccatctgactggcatagaaatgtccgatgattttcacgatgacctggtcgttctcatcaggggtctggtctcttggtactaccacctcagctgccgtcaaattctgcaactcgttcaccgtttttccacctttgccaatgacccggccagctgctgatgctggcacacgtatgtgggtctccagcttcacttcctccttgggaccaaagaagttctcctccttgagtttgccatagattcttccctgagccttgaattgggcctctggcggtccagtgatgataaccatacgaactttggagtcaggtgtttcgggtggtgcaatcttgatggaggcgctggcaaaccgggagagctgtttgatgtgctgccccttcttgccgatgatggcgcccactgcctgggcggggataaacacctgcaccatctcctgctcgggagcctgcataaaggagctatagggagcagccccagtaacgctgctgggaggcggcgggactgcgctggatgaagctgggaaaagacctacagcagccaggttcaggccagggatcaggtgagactgcaggctcatggcagccacatcattctcataggcctcccgaactttcttcattatttcctgctcggccctgcaacaattctcgatggcccccttcacagtgatggtcctctcagggttgtaaagggtaaggtcttgcaacgaggagatggtgatttttgtctcggtatcttgctctaccttcttcaggttccgtccttccttgccaatgagacgccctacaaagttattatgggccaggatcttcaggggaacctcgtcagccgttttggtgtccttagcctctttatgcataatctccaagatcatcttacaagcggaggagcagccctcaggggtggagtgcacactgatggctttttcagctgcacctgcgttctccttcctatgcacgtctatcttggactgggtctgttttgtgatgttgcggatggtggccccctccttgccaataatggcacccacatactgggtgggcaccaggagccgaagggggatgtccacttgctgctgcttggctggggcccccgctgccacaggtgagccctggcggggctgaccccgagagccaaagccccctcggcgcccattctcaggtccctgtgctatctgctcatcggggatgtaggagaccttcagggcatggttctccaactggtggccattcagcttcatgatggcttgcctggtctgctcccggttggaataggtgacattcaccactgccgtctcactctcggtgttcacttgctcacagttctctactgtaccatactgagccagcaggctgtccagtacttcccatcggagctggggtggaatatttcggatttgaattttccggctcctttgttttttgggcaccgaatgttcaatctctaagcgttttccttgtaattctactttcccggagaaagtttcgatggccttcatcgcccagtgctcgtccgggcagtccacgaaggcgtagccggatttgaccaagaactggccgctgtaggagatcttgtgctccgcaaacactttctccaagtccgcgggggtcacgctctcgttgaggttgccgatgtaaagcttgttcatggtggcggtctcggggcaggacgcggtcccgggcaaggccgaacgagcgggcgcgggcggcgagcctcctaggccaagaggcggagaggccggcggcaggagccgcaaactttctttgcaccccaccccagaagttgtcccgagcccagggcggggaaggcggcctgagggcgcgcagaggtcgcgggagagttcggggagagcccaggagaagtgcccgcggcgcgcagggagacggacgacacggcgcagcttcttcccttcggtccgaaacccctccgagagggctggtgtgtcacgtttctccgcggccgccctggcgccgcctctaaataaaatcgacttgaaaaaaaatggagcg

SEQ ID NO: 19408 - RNA, 7291 nt, Homo sapiens
  source 1..7291: mol_type = other RNA
ttccactgccactacctaatttatctattgttttgctaagaggtagataaaacaaaagtgaaatggggcttctatgaggaggtccattagagggtgggtggggaggggctgggatcgcccagtggaactcccccaactacaaagacggcctgaatgagtccaaggaccgcgccctcagactcccccagggcaaaggatcctgcttcacctcttctccttctagagccaactgggcccccattgaagactgaaaaagggcccaatggaggtgtaggatctcaaagaaaccctgttgaagaggtctcagctctggtttccccaggcttcctgactttggggctgtgtggtgggttccaggccaagccccaggtctcactccagccagccccctctagaagggaagaggccattcctttcctcaccatctggtccaacaaagctatagaaagtgagagagggacaagctggaggccaaaggggtgacacatgggcaaggaaagcagaaagtggggacctcatggccagccctcccagcccaatcgatatgggggggatcctggcaggcctgcctgttccccaaggacaaaccttttgtggcacaagcctcaactcacttgtcctggctgggattcatacccttatgcatgagtccctgcccttagttccaatcttactgtaaggattgaggtagttaatccatttatactcgtagcatccatcacctgcggttaatcaaaacacatgctcccgaggagcttcctgctatttcattcaagaaaaaaaattttttttcttttgtccatccggagtcaaccatactaaggcgccagcaaaggcgccatcagactgtgccccaaagcggtgcacaggaccgagggtcagggctggggctctcgcccctaaatcccccttcagacatgaggcctcctccctgtcccgtaccccgatagagaagccttatgtatccaaaggaaagaaactgcagttttcagctggtgttactctaagtctgaatacagagaaatgttctgcatctaaattgtcgagtatttggaagggaaatggcttttatgtcccctggcattgatgaggatttttcttcaatcttcctgcaattactgtgacaggctgtgctgtttcccttctactggttttcaagaaacaggcaaacagtcgagtggtttgaatggcaaagccactaggatctccccataaacacttcaggggaaagaaaggagaacccccacccctgatgagaggtgggaggaaggggttgcctagaggcaccagcttctcctgtggagcaagaaggctcaagcaggccctctggggctctgtgaggtagttactagcactgctggttcccagtttggcagagggtatgtctgggttgggaggaggggaaggcacccttgagagctaactgaggcccctcctcactgcccgtctgccaggcctgaagggaactcggcagtgctatctctgcagtaggggcaggggacagagcagtcccacaacagggagctacctggagccccaaacttcctctccttccccaaagtgcaaccaggagccgacagaccaatttctcggctccctaccccttggcttggcaaacaccacaccctaatcccccaggagcctctgaagggaagggcctcgcccttagctcccagtttccaggaggccttcctcctcagacagccaggtatgtgtcgaaagctggctattgctttgattcaggaacagcctctctcagcctctgtctgtctgtctttggcacagaggaaaatggacacagaaccaactagagcatccccctccagtgttctctgggttttaaatggggtcttttctgccaatagtgaggcataaacaaggatagctcccaactgcctccagaaggagggggtcaggaaaaaggaaaaaagattgataaggactgggaggaggggaggaaagtagaaaagggctataaaactccctgtccttaaaaatggctctctcctaaccagacccctcacaggagctgagtccacaacccaaactgcaaaaggcaaccagacccgagaggggattaaagccatttggggtgtaactggcagatgcagcttcaaagtcagtcagtgaatcaaaccattttggttatgtgtttcaaagaatttaaaaatatatcctaaagagatggtcctttcttaaaaatatatatgtagcacacacacacacatatatatcttagagcacagaagcattttttttaagtcactcttctcaaatcatccaaatctcccaagtgcttttcgcgatagcttgttatctcaccaaggatggggaaatggaggtgctgagcaggagggcaaggagttgccctaagacctagcctacggggcacaagagggcccggcccaccaagacaggtccttcatcccactaaaccttaaccaccaaaccatgctccttttgctttctggtggtataacttacatgattttcctgctgggcaaatatcaacaatgagtggagccttgcctaatccaagcaagtgaagttttccagtcccttgccacacacttcctcgtctcttctgggagctgaatcagccaacggaaaaggacttgggctcaaggtgtgaagggagcaggcccccaaggaaactgaacactgcaacaatcacatttcaggtactgtgggatttttttttcttcctgatgatagtctgaaccagatatcaaagcatgcttgctgctggaaattcgctttaaattactaaatggccgacgtctgaacgttatctgctttgttttgggataaagcatatagagccagagatggaaagctgggagaccctttttatggttgggacaggtggagaggcttaattctactggcctgatgttatccctaaatgtttttctgcttctattcaatttgggccagacaattctgggggctacaagggaatgtcctagggagaaaatgataaggcaggaacctgtcccagtcacgtccccatatcccctgcccctccttgccaccagccaccctaaatcaagaattccctaagtttgggtccacttttaaaatcaatcagaccgatctaaagaagacagggagacagaggtgggggcagttaactagtatctgtttgccccttagatctatggatatagattaggaagaatagcaagacggaactgaaatgaaacaataacaaaaaaaaaaaatgaaaagcattgcaatgacaaaccaggtggacctctctgagggcgagagggtggccttgtcttttttccacgaacggaatctcagctcccatatttttagacagagaaatataggtttttttaaagggtatattttttagttattatttctctcctcgataaaacggaggcaatattttaaaatatctcaacagcaccactggtgggaaaagctggctgagatgctctttaaccaaaggaggaaagagaggagaccaagggccagctggttggttgttgggcattgtttaaccactgagagcccccagctccactaggccttttaatcctatcaggtaggatattccagcagccgccagcagctggggctctagaagtcagagatcagggccaaacaaggctctgggctctgcccctctgggctctctcaaacctgggccttccctcttagcactagcctcctcctaagggggcagcccccaaagcctttcccaccaggcctgttctccatagagagttcctaaagggttactggctcatgttgtaagaaattatgaaacataactttcttgttttttcttttcattaaaaaaataaaatattcaagactatcagcttctcttttgctttgcttttcttttttatataaaatatcagcaagctgcaaaaaaacaaaaatcaaaaaaaaatttttttaatggggttggggggaacaaaaaggaaaataattgctgaggtaacttcataccttgaggtagtttacttcgcacacagcattgcctgactacgcccacatgttgcggttgtcttgttgttactgttgttgcaatgttgaaaggaggggaactccacgcatgggcttttccatatgtagagaggccttcctcccttcccagcacacttgatagcattgtccagggtagctaaagtgcattacctggctaatatgcattgtcaatcagtatattaggaggagaggcctaacctcatttaactgatggcttctgtctcccacaagggctaaacactccatgggatcttaattaagcctggtaaattaataaattaagcttatttaccccttgctgtacaatgctgctggtattctgaattgttttttagacacacctttcatcatgctgataatgattcatggagacagaagccgtcagttaaaaattcctctcagatacaaacagaagcaagtactctccaatttactgaatttgccagatgatggactttagctttatcgggagctcagggttgggttccaagtcccaccaccaaggtaacagtgccgtggctgggagtgccccacaacccctgcctctaggaaccagcccttatgggagcacatgggctggggtgagggcaccgtggcagcctttggggccactcaagtcctccatggaaccgagactttatcaaggggagttagcgtccccttcccagtgctcatatccaatcattaaaatagactttaaaaaaatataaaatccgcctgagaacgatgggaatcagggacagtggtcagcccctaccctgctgagcattcaataccacctatgtgcacctggacataatgtgaaacctacacgggagagggacatgaatgtggtggggaagccccaacagagtggggaaatttcagttgtgccaatttgaagatggtgatctggcatagatcagccacaagtgcgctccttttaaacgtggattattatgtattttaaccatctttctccccattttcccctcttcttcattccgtattgtacctattggttagggagtgattggaattaatctacagatactgacagttcttttcccttgagtcaatactgtaagcaaagcaatgcattcgttcgcatttttttctggtagcaataaagataaaaaaattagtgtaaatatagaaagaggccgtaaatggaggtattttaatcaattacccaagtagggggaagaagattggaaaaacattaaggtcaagaaatgaaccatcctttaaggctgattaaaacacctctctgcatgtttttaaaacctgaaggaaattttatttttcttcccactgaggtgtgatccaccctcttggtggggcctggagagcttctttaaacaatccacgtttaaaagtgccttgcgctagaatttctgacaccccgaggggcagacagtgttgggccaattgggtgggtgtttggggctgagagatcagggttcctcactggaacatctttctcaatcaagtgggcaaacctgatctacagcccggcccaggtgtcccggattcccactcattctcaggcctgccggggagagcacactctcgatttctgcccgttgttgtcctggactcgaagggacagggaggggctggtcacttcctccgtgcctgggcctggttactctgtcccttctgatgctgctgcttaacctgggccaggatgtctcggatcttccgttgagccatctgactggcatagaaatgtccgatgattttcacgatgacctggtcgttctcatcaggggtctggtctcttggtactaccacctcagctgccgtcaaattctgcaactcgttcaccgtttttccacctttgccaatgacccggccagctgctgatgctggcacacgtatgtgggtctccagcttcacttcctccttgggaccaaagaagttctcctccttgagtttgccatagattcttccctgagccttgaattgggcctctggcggtccagtgatgataaccatacgaactttggagtcaggtgtttcgggtggtgcaatcttgatggaggcgctggcaaaccgggagagctgtttgatgtgctgccccttcttgccgatgatggcgcccactgcctgggcggggataaacacctgcaccatctcctgctcgggagcctgcataaaggagctatagggagcagccccagtaacgctgctgggaggcggcgggactgcgctggatgaagctgggaaaagacctacagcagccaggttcaggccagggatcaggtgagactgcaggctcatggcagccacatcattctcataggcctcccgaactttcttcattatttcctgctcggccctgcaacaattctcgatggcccccttcacagtgatggtcctctcagggttgtaaagggtaaggtcttgcaacgaggagatggtgatttttgtctcggtatcttgctctaccttcttcaggttccgtccttccttgccaatgagacgccctacaaagttattatgggccaggatcttcaggggaacctcgtcagcctgcctggtctgctcccggttggaataggtgacattcaccactgccgtctcactctcggtgttcacttgctcacagttctctactgtaccatactgagccagcaggctgtccagtacttcccatcggagctggggtggaatatttcggatttgaattttccggctcctttgttttttgggcaccgaatgttcaatctctaagcgttttccttgtaattctactttcccggagaaagtttcgatggccttcatcgcccagtgctcgtccgggcagtccacgaaggcgtagccggatttgaccaagaactggccgctgtaggagatcttgtgctccgcaaacactttctccaagtccgcgggggtcacgctctcgttgaggttgccgatgtaaagcttgttcatggtggcggtctcggggcaggacgcggtcccgggcaaggccgaacgagcgggcgcgggcggcgagcctcctaggccaagaggcggagaggccggcggcaggagccgcaaactttctttgcaccccaccccagaagttgtcccgagcccagggcggggaaggcggcctgagggcgcgcagaggtcgcgggagagttcggggagagcccaggagaagtgcccgcggcgcgcagggagacggacgacacggcgcagcttcttcccttcggtccgaaacccctccgagagggctggtgtgtcacgtttctccgcggccgccctggcgccgcctctaaataaaatcgacttgaaaaaaaatggagcg

SEQ ID NO: 19409 - RNA, 7626 nt, Homo sapiens
  source 1..7626: mol_type = other RNA
ttccactgccactacctaatttatctattgttttgctaagaggtagataaaacaaaagtgaaatggggcttctatgaggaggtccattagagggtgggtggggaggggctgggatcgcccagtggaactcccccaactacaaagacggcctgaatgagtccaaggaccgcgccctcagactcccccagggcaaaggatcctgcttcacctcttctccttctagagccaactgggcccccattgaagactgaaaaagggcccaatggaggtgtaggatctcaaagaaaccctgttgaagaggtctcagctctggtttccccaggcttcctgactttggggctgtgtggtgggttccaggccaagccccaggtctcactccagccagccccctctagaagggaagaggccattcctttcctcaccatctggtccaacaaagctatagaaagtgagagagggacaagctggaggccaaaggggtgacacatgggcaaggaaagcagaaagtggggacctcatggccagccctcccagcccaatcgatatgggggggatcctggcaggcctgcctgttccccaaggacaaaccttttgtggcacaagcctcaactcacttgtcctggctgggattcatacccttatgcatgagtccctgcccttagttccaatcttactgtaaggattgaggtagttaatccatttatactcgtagcatccatcacctgcggttaatcaaaacacatgctcccgaggagcttcctgctatttcattcaagaaaaaaaattttttttcttttgtccatccggagtcaaccatactaaggcgccagcaaaggcgccatcagactgtgccccaaagcggtgcacaggaccgagggtcagggctggggctctcgcccctaaatcccccttcagacatgaggcctcctccctgtcccgtaccccgatagagaagccttatgtatccaaaggaaagaaactgcagttttcagctggtgttactctaagtctgaatacagagaaatgttctgcatctaaattgtcgagtatttggaagggaaatggcttttatgtcccctggcattgatgaggatttttcttcaatcttcctgcaattactgtgacaggctgtgctgtttcccttctactggttttcaagaaacaggcaaacagtcgagtggtttgaatggcaaagccactaggatctccccataaacacttcaggggaaagaaaggagaacccccacccctgatgagaggtgggaggaaggggttgcctagaggcaccagcttctcctgtggagcaagaaggctcaagcaggccctctggggctctgtgaggtagttactagcactgctggttcccagtttggcagagggtatgtctgggttgggaggaggggaaggcacccttgagagctaactgaggcccctcctcactgcccgtctgccaggcctgaagggaactcggcagtgctatctctgcagtaggggcaggggacagagcagtcccacaacagggagctacctggagccccaaacttcctctccttccccaaagtgcaaccaggagccgacagaccaatttctcggctccctaccccttggcttggcaaacaccacaccctaatcccccaggagcctctgaagggaagggcctcgcccttagctcccagtttccaggaggccttcctcctcagacagccaggtatgtgtcgaaagctggctattgctttgattcaggaacagcctctctcagcctctgtctgtctgtctttggcacagaggaaaatggacacagaaccaactagagcatccccctccagtgttctctgggttttaaatggggtcttttctgccaatagtgaggcataaacaaggatagctcccaactgcctccagaaggagggggtcaggaaaaaggaaaaaagattgataaggactgggaggaggggaggaaagtagaaaagggctataaaactccctgtccttaaaaatggctctctcctaaccagacccctcacaggagctgagtccacaacccaaactgcaaaaggcaaccagacccgagaggggattaaagccatttggggtgtaactggcagatgcagcttcaaagtcagtcagtgaatcaaaccattttggttatgtgtttcaaagaatttaaaaatatatcctaaagagatggtcctttcttaaaaatatatatgtagcacacacacacacatatatatcttagagcacagaagcattttttttaagtcactcttctcaaatcatccaaatctcccaagtgcttttcgcgatagcttgttatctcaccaaggatggggaaatggaggtgctgagcaggagggcaaggagttgccctaagacctagcctacggggcacaagagggcccggcccaccaagacaggtccttcatcccactaaaccttaaccaccaaaccatgctccttttgctttctggtggtataacttacatgattttcctgctgggcaaatatcaacaatgagtggagccttgcctaatccaagcaagtgaagttttccagtcccttgccacacacttcctcgtctcttctgggagctgaatcagccaacggaaaaggacttgggctcaaggtgtgaagggagcaggcccccaaggaaactgaacactgcaacaatcacatttcaggtactgtgggatttttttttcttcctgatgatagtctgaaccagatatcaaagcatgcttgctgctggaaattcgctttaaattactaaatggccgacgtctgaacgttatctgctttgttttgggataaagcatatagagccagagatggaaagctgggagaccctttttatggttgggacaggtggagaggcttaattctactggcctgatgttatccctaaatgtttttctgcttctattcaatttgggccagacaattctgggggctacaagggaatgtcctagggagaaaatgataaggcaggaacctgtcccagtcacgtccccatatcccctgcccctccttgccaccagccaccctaaatcaagaattccctaagtttgggtccacttttaaaatcaatcagaccgatctaaagaagacagggagacagaggtgggggcagttaactagtatctgtttgccccttagatctatggatatagattaggaagaatagcaagacggaactgaaatgaaacaataacaaaaaaaaaaaatgaaaagcattgcaatgacaaaccaggtggacctctctgagggcgagagggtggccttgtcttttttccacgaacggaatctcagctcccatatttttagacagagaaatataggtttttttaaagggtatattttttagttattatttctctcctcgataaaacggaggcaatattttaaaatatctcaacagcaccactggtgggaaaagctggctgagatgctctttaaccaaaggaggaaagagaggagaccaagggccagctggttggttgttgggcattgtttaaccactgagagcccccagctccactaggccttttaatcctatcaggtaggatattccagcagccgccagcagctggggctctagaagtcagagatcagggccaaacaaggctctgggctctgcccctctgggctctctcaaacctgggccttccctcttagcactagcctcctcctaagggggcagcccccaaagcctttcccaccaggcctgttctccatagagagttcctaaagggttactggctcatgttgtaagaaattatgaaacataactttcttgttttttcttttcattaaaaaaataaaatattcaagactatcagcttctcttttgctttgcttttcttttttatataaaatatcagcaagctgcaaaaaaacaaaaatcaaaaaaaaatttttttaatggggttggggggaacaaaaaggaaaataattgctgaggtaacttcataccttgaggtagtttacttcgcacacagcattgcctgactacgcccacatgttgcggttgtcttgttgttactgttgttgcaatgttgaaaggaggggaactccacgcatgggcttttccatatgtagagaggccttcctcccttcccagcacacttgatagcattgtccagggtagctaaagtgcattacctggctaatatgcattgtcaatcagtatattaggaggagaggcctaacctcatttaactgatggcttctgtctcccacaagggctaaacactccatgggatcttaattaagcctggtaaattaataaattaagcttatttaccccttgctgtacaatgctgctggtattctgaattgttttttagacacacctttcatcatgctgataatgattcatggagacagaagccgtcagttaaaaattcctctcagatacaaacagaagcaagtactctccaatttactgaatttgccagatgatggactttagctttatcgggagctcagggttgggttccaagtcccaccaccaaggtaacagtgccgtggctgggagtgccccacaacccctgcctctaggaaccagcccttatgggagcacatgggctggggtgagggcaccgtggcagcctttggggccactcaagtcctccatggaaccgagactttatcaaggggagttagcgtccccttcccagtgctcatatccaatcattaaaatagactttaaaaaaatataaaatccgcctgagaacgatgggaatcagggacagtggtcagcccctaccctgctgagcattcaataccacctatgtgcacctggacataatgtgaaacctacacgggagagggacatgaatgtggtggggaagccccaacagagtggggaaatttcagttgtgccaatttgaagatggtgatctggcatagatcagccacaagtgcgctccttttaaacgtggattattatgtattttaaccatctttctccccattttcccctcttcttcattccgtattgtacctattggttagggagtgattggaattaatctacagatactgacagttcttttcccttgagtcaatactgtaagcaaagcaatgcattcgttcgcatttttttctggtagcaataaagataaaaaaattagtgtaaatatagaaagaggccgtaaatggaggtattttaatcaattacccaagtagggggaagaagattggaaaaacattaaggtcaagaaatgaaccatcctttaaggctgattaaaacacctctctgcatgtttttaaaacctgaaggaaattttatttttcttcccactgaggtgtgatccaccctcttggtggggcctggagagcttctttaaacaatccacgtttaaaagtgccttgcgctagaatttctgacaccccgaggggcagacagtgttgggccaattgggtgggtgtttggggctgagagatcagggttcctcactggaacatctttctcaatcaagtgggcaaacctgatctacagcccggcccaggtgtcccggattcccactcattctcaggcctgccggggagagcacactctcgatttctgcccgttgttgtcctggactcgaagggacagggaggggctggtcacttcctccgtgcctgggcctggttactctgtcccttctgatgctgctgcttaacctgggccaggatgtctcggatcttccgttgagccatctgactggcatagaaatgtccgatgattttcacgatgacctggtcgttctcatcaggggtctggtctcttggtactaccacctcagctgccgtcaaattctgcaactcgttcaccgtttttccacctttgccaatgacccggccagctgctgatgctggcacacgtatgtgggtctccagcttcacttcctccttgggaccaaagaagttctcctccttgagtttgccatagattcttccctgagccttgaattgggcctctggcggtccagtgatgataaccatacgaactttggagtcaggtgtttcgggtggtgcaatcttgatggaggcgctggcaaaccgggagagctgtttgatgtgctgccccttcttgccgatgatggcgcccactgcctgggcggggataaacacctgcaccatctcctgctcgggagcctgcataaaggagctatagggagcagccccagtaacgctgctgggaggcggcgggactgcgctggatgaagctgggaaaagacctacagcagccaggttcaggccagggatcaggtgagagctcatggcagccacatcattctcataggcctcccgaactttcttcattatttcctgctcggccctgcaacaattctcgatggcccccttcacagtgatggtcctctcagggttgtaaagggtaaggtcttgcaacgaggagatggtgatttttgtctcggtatcttgctctaccttcttcaggttccgtccttccttgccaatgagacgccctacaaagttattatgggccaggatcttcaggggaacctcgtcagccgttttggtgtccttagcctctttatgcataatctccaagatcatcttacaagcggaggagcagccctcaggggtggagtgcacactgatggctttttcagctgcacctgcgttctccttcctatgcacgtctatcttggactgggtctgttttgtgatgttgcggatggtggccccctccttgccaataatggcacccacatactgggtgggcaccaggagccgaagggggatgtccacttgctgctgcttggctggggcccccgctgccacaggtgagccctggcggggctgaccccgagagccaaagccccctcggcgcccattctcaggtccctgtgctatctgctcatcggggatgtaggagaccttcagggcatggttctccaactggtggccattcagcttcatgatggcttgcctggtctgctcccggttggaataggtgacattcaccactgccgtctcactctcggtgttcacttgctcacagttctctactgtaccatactgagccagcaggctgtccagtacttcccatcggagctggggtggaatatttcggatttgaattttccggctcctttgttttttgggcaccgaatgttcaatctctaagcgttttccttgtaattctactttcccggagaaagtttcgatggccttcatcgcccagtgctcgtccgggcagtccacgaaggcgtagccggatttgaccaagaactggccgctgtaggagatcttgtgctccgcaaacactttctccaagtccgcgggggtcacgctctcgttgaggttgccgatgtaaagcttgttcatggtggcggtctcggggcaggacgcggtcccgggcaaggccgaacgagcgggcgcgggcggcgagcctcctaggccaagaggcggagaggccggcggcaggagccgcaaactttctttgcaccccaccccagaagttgtcccgagcccagggcggggaaggcggcctgagggcgcgcagaggtcgcgggagagttcggggagagcccaggagaagtgcccgcggcgcgcagggagacggacgacacggcgcagcttcttcccttcggtccgaaacccctccgagag

SEQ ID NO: 19410 - RNA, 34 nt, Homo sapiens
  source 1..34: mol_type = other RNA
ttccactgccactacctaatttcacacacaaaaa

SEQ ID NO: 19411 - RNA, 806 nt, Homo sapiens
  source 1..806: mol_type = other RNA
ttccagccctggtaggcgccgcggaagaaggggaagcgcgcctgcaggaactggtagatctcgctgagcgtcaggcgcttgctgggcgagctctggatggccatgacgatgagcgcgatgtacgagtagggcggcttctcgggccgccgcagccccgagctcgccttcttggcgcccccgctcccggcgcccgcgccgccgccgcccgcgctcttgcaggcagccgagggggcgctggccgaattggaggaggacgaggacgaggcgcaggaggcggaggacgacgacgaggaggaggaggtggtctccggggcggcggcggcggcggcggcggcggcgggcggcgggctcatcagggcggcctggagcgcgccggggaccgggctgcacgcgcggcggagcggggccggcggcggcccgccctcggtggtcatctgggacccgggagcgaggccgggccgcgagggcgggccccgggcgggaagcggaggcgccggagcggggtcggcccagaagccctgcgagcgccctagcccgccgcccgggctgcagccgtggccactccgggccagcgcttcggcgtcgcctccctcagctcctctggggcttctggcggcggcggcggcggcgggcgggaggcaacgcccggcgcatccctccccgagccgcgggccctgccttgcgcaacggcctcccaggccgcggggccgagcggccggcgccgggcgactgcgcccgcgagtgggaccgcggcctggaccccggggacgagcccgacgtctcccttcaggagcgctcctcgctct

SEQ ID NO: 19412 - RNA, 2921 nt, Homo sapiens
  source 1..2921: mol_type = other RNA
ttcctatgcatatacttctttgaattcaaattgggcccctgaaggctaaaacagtacattggagctgagctgctactgatttatgctgatattaaatattaagaattaagatgacacgtaacttgacaatttgtttccatcttgcctttggctcctctttattcatgtgcaatgcagaattctctgcccagagcttccatgcttcctggaagaggcagtggaggatggacagtgggagtcatcctccctcttacccctatcttggcaggacaatgacttatgaatatagccaagagaggagacagctgggttgtgctggctgtccgattttacaccctcaaggaatctgtaaccccttcaacatggtgcagtcaatgtgtctaccctccacatatatccttcactctttcttcgtgggatttctttacaactttgacatccaggtctccctctgagatcattttcaaatggattttattcagataaaaatccatgcatgtagggagagggggagttcagaggcccagcatcccttgggtttgctgctatccaaggtaccccccttccccctgtcacacacagcatctggacagctatagattgccacacctcttatttttcacatttcagcacttgttcagtttaattgaatctgagtaaaaaagaaagttttccatagaaccttaaatataacatatgcagaagtttaaggattctgtatagccatagttccttgaaaatcaactgtatctaaatttacccagagagataatcattagcatgtttctcattcgtcaaactattaatgtgtgtcccaacctcaactactgacctttagtcttcaacttgagcacagcagctgccagcagtgtggtctgagatctgcatttttaggggctgctgtaggctttggaattcaagggttcatttgtgaaccagctgcttcatactcacctagctgggcctcccaaagtgctggaattacaggcgtgagccactgtgcctggcctagttttccatcttatttagacacttctggttggttaagaggctggaactggaatagattgtcaagagacagatttttcagaagccgagcaggtggcaccactagatggtgtattttcagcagaagaattcctctcatggatgttaatgtgtcccaggagcactttagtggttgtcttcatgtgaatgaacacatatgagcatttttgacacaatattttaggcactggcttcctgcagacacatttccagaaagctgaggccaagaagagtcgttttgtgtttttctcagggacaagagaagctatttttccaggatatttctagagaaacctgccagtgaaacaagtaatgcaaatggattatctggatgattgtacagtccttttaactttaaaattttataatttcaagtcttgagtagccacttttctgtcctccacgacaatcagcaaatgtttattgaatatttatcatgtgatcagggcagcaaaaaagaaaaaaatacattattattctcttaaaatgcttatggctgaatttgtaaaagaaggccaacctacatgaaacaacttggaactctacagaataatttaatattaaatgccaaattgtgtgagacagactccagtggctgtaagatattcagagaaaagaaatatcagagtggagttgtcaaggagtttcgttcattcatccaacaaagaatttctgagcaattagtgtacaccaggaactgtcctaacactagtgacaggtcctgaataaggcacagtccctgccctcaggaccatgtagcattgagagggagacaaaaggaaaaaaaattgagtaattacaacatagaattgctttaatagaggtatgtgctgaatgctgcgagggcgcataggaggagcatccaaaaggcttcctgcaagaagcctaaggggagagatctaaggagaggtttagctggatgaagtgagatatgaggagtgaagggtagctcatgctaaaaagaacagtacatgtgtgaccaacaactccactcctgagtgtataccccaaaaaagtgaaaacagagattaaaaatatcctcatacgcaaatgtttatagtagccctattcacaatagcaaaaaggtagagaagcctaaatgtgaatcaggagttgaatgaataaccaaattatgatgcagtgaaatattattcagccataagaaggaatgaggtgctgacacgtgctacaacatggatggacctcaaaaatattttgctaagaagccagtcacgaaagaacacagagaatgtgactccatttatataaaataactagaataggcaaatctatagggggaaaaaagcagattggtggttgctaagggctggggatttgggataagaagctgaggagttaatgggtatgggcttttattttgaagtgatggagatatctggggaccagagagaggtggtggctgcataatattgtgaatatactaagtgccactaagtccactttaaaatggttaattttatattacatgaatttcacctcaattaaatttttaaaaagaacagcctgcacaagtgttagacactaacatgtttggctcatttgaaaaatctccaatggtccaatgaaactggagaaggttaaaggggtaaagaggaaaagtactgagagaaaactggggagataactaagtcagattacatggaatttaagctaagccttgaaggataagcatgacttagagacaggcagtggaaagcaaacctagcaatgtggaaaaaggaaacactaacttggaagaataaagaagactcttggaaatctctagaagtaacatggactttggtgacttgttttcaaagcttagaaacaggcataggaaatgactgacttgatttttctttcctagctgtgga

SEQ ID NO: 19413 - RNA, 3142 nt, Homo sapiens
  source 1..3142: mol_type = other RNA
ttcctatgcatatacttctttgaattcaaattgggcccctgaaggctaaaacagtacattggagctgagctgctactgatttatgctgatattaaatattaagaattaagatgacacgtaacttgacaatttgtttccatcttgcctttggctcctctttattcatgtgcaatgcagaattctctgcccagagcttccatgcttcctggaagaggcagtggaggatggacagtgggagtcatcctccctcttacccctatcttggcaggacaatgacttatgaatatagccaagagaggagacagctgggttgtgctggctgtccgattttacaccctcaaggaatctgtaaccccttcaacatggtgcagtcaatgtgtctaccctccacatatatccttcactctttcttcgtgggatttctttacaactttgacatccaggtctccctctgagatcattttcaaatggattttattcagataaaaatccatgcatgtagggagagggggagttcagaggcccagcatcccttgggtttgctgctatccaaggtaccccccttccccctgtcacacacagcatctggacagctatagattgccacacctcttatttttcacatttcagcacttgttcagtttaattgaatctgagtaaaaaagaaagttttccatagaaccttaaatataacatatgcagaagtttaaggattctgtatagccatagttccttgaaaatcaactgtatctaaatttacccagagagataatcattagcatgtttctcattcgtcaaactattaatgtgtgtcccaacctcaactactgacctttagtcttcaacttgagcacagcagctgccagcagtgtggtctgagatctgcatttttaggggctgctgtaggctttggaattcaagggttcatttgtgaaccagctgcttcatactcacctagctgggcctcccaaagtgctggaattacaggcgtgagccactgtgcctggcctagttttccatcttatttagacacttctggttggttaagaggctggaactggaatagattgtcaagagacagatttttcagaagccgagcaggtggcaccactagatggtgtattttcagcagaagaattcctctcatggatgttaatgtgtcccaggagcactttagtggttgtcttcatgtgaatgaacacatatgagcatttttgacacaatattttaggcactggcttcctgcagacacatttccagaaagctgaggccaagaagagtcgttttgtgtttttgtttctgctctggctaagtttctgtgtggctgtagagtttctttctcattccaggtcttgtttaaaatgtttcttggaagtgccaactttggggaagctgcacactttgtctccaccttgggtttcttcaatttgatcttcatctccttcaccccagtcatcttgtatttcaccaaggtggagcactggtcctcttttgctgctctgccatggggctgtctctcagggacaagagaagctatttttccaggatatttctagagaaacctgccagtgaaacaagtaatgcaaatggattatctggatgattgtacagtccttttaactttaaaattttataatttcaagtcttgagtagccacttttctgtcctccacgacaatcagcaaatgtttattgaatatttatcatgtgatcagggcagcaaaaaagaaaaaaatacattattattctcttaaaatgcttatggctgaatttgtaaaagaaggccaacctacatgaaacaacttggaactctacagaataatttaatattaaatgccaaattgtgtgagacagactccagtggctgtaagatattcagagaaaagaaatatcagagtggagttgtcaaggagtttcgttcattcatccaacaaagaatttctgagcaattagtgtacaccaggaactgtcctaacactagtgacaggtcctgaataaggcacagtccctgccctcaggaccatgtagcattgagagggagacaaaaggaaaaaaaattgagtaattacaacatagaattgctttaatagaggtatgtgctgaatgctgcgagggcgcataggaggagcatccaaaaggcttcctgcaagaagcctaaggggagagatctaaggagaggtttagctggatgaagtgagatatgaggagtgaagggtagctcatgctaaaaagaacagtacatgtgtgaccaacaactccactcctgagtgtataccccaaaaaagtgaaaacagagattaaaaatatcctcatacgcaaatgtttatagtagccctattcacaatagcaaaaaggtagagaagcctaaatgtgaatcaggagttgaatgaataaccaaattatgatgcagtgaaatattattcagccataagaaggaatgaggtgctgacacgtgctacaacatggatggacctcaaaaatattttgctaagaagccagtcacgaaagaacacagagaatgtgactccatttatataaaataactagaataggcaaatctatagggggaaaaaagcagattggtggttgctaagggctggggatttgggataagaagctgaggagttaatgggtatgggcttttattttgaagtgatggagatatctggggaccagagagaggtggtggctgcataatattgtgaatatactaagtgccactaagtccactttaaaatggttaattttatattacatgaatttcacctcaattaaatttttaaaaagaacagcctgcacaagtgttagacactaacatgtttggctcatttgaaaaatctccaatggtccaatgaaactggagaaggttaaaggggtaaagaggaaaagtactgagagaaaactggggagataactaagtcagattacatggaatttaagctaagccttgaaggataagcatgacttagagacaggcagtggaaagcaaacctagcaatgtggaaaaaggaaacactaacttggaagaataaagaagactcttggaaatctctagaagtaacatggactttggtgacttgttttcaaagcttagaaacaggcataggaaatgactgacttgatttttctttcctagctgtgga

SEQ ID NO: 19414 - RNA, 7306 nt, Homo sapiens
  source 1..7306: mol_type = other RNA
ttcgccacttccctccctgcagaatcagtgaggctaggggaggagtcagcatgagccccagccagcctcctcagcttcagggcctccccactgcagccacgaagaggagagggcttggcgagcgtgggcttggtcctccagaaggacttggggaggcaagttgcagggatcacaaaacaacctccttcaatacccttttcccattgctcagagggagaaattgaggcccagagagggctagtgacttgcacaaagtcatatagcgagatagtagctgcaaggattcaaacccaagtccctttctttggagccagttatactcccaataagccctatggctgcccaagtaccccaggccactggcaaaattgagaagaaagcaaagcaataggggcagcagtaattcctgtgtgttgtggatttagcaggtattgggtatcacgctgcaacccttcacgtgcaccttgtttagtcctcgctgcagtcctataaggttaaggcacatgatacacattatcagcatcatccccattttagagatgagaaaattgaggatcagagaggttatgtgatttccttcaggtcaattcaagagacttgaacccagacctgctgatcccagagcggcatacaaggacccagccctcaatcctggggtctttctgtggtgtaactcttggggcgtgcccatgggggctgcctcgtgctgaccacagcaaggcccaaggaatgagcatttctccgtccatccatctgtctacctacctatccgtctgttcactcaataaatatttacccagggctttctccatgccaggcaatattcaggcattgggaggcatacagcagtgaacaaagcaggcagtgcctggcttcgtggccctcataccctcgtggggagaggcagactataaacagagaaacaacaaagatgtgtgtcaggtggtggtgagggctatggagaaaaacaaagccagaggagggggcagcgcaggatggcggggtcggagaaggcttctctgaggaggtgacatttgagcggtgatctgaaggaggtgagggcttgggccgtgtggggatcactagagaggggtttctggcagaggaaatagcgggagcaaaggccctgaggcgggagcgtgcctggcatgttggaggaacagagaacaggtcagtgcagctggagacggcaagcaagcggcagggcgttggggaggtggagaggtcagtgggaatcagaccaagggcggccctgtcaggttttcttctgagtgagatggaagccattggaggttctgagcagaagcgtggaatcatctgattgagtttttaagagcatcttctggctgctggagtgaggatgtactacagggctcaaaggaagagggagcgggggttagaaaggcaaggtagtatgtgggtgtcagatggcagaggctagggccacgcagagtgaaggaggtggagagggaggccaagatctgaatatattctaaaggctaagccacaggattagggtctgagaaccctctaggatggctccaggtttttggcttaaaccagaatgaaactgtcatttatgcaggtggggaggactgctggaaaagcagtgcgggcccgggctttgcacatctcagttcgtttgtgccttatattcctcaagcatcagaatcaccggagacacttgttgaagtccagatttctgggatcctccaccagagcttcccattcaatagagctgggtggggcttgagaatgtggatttctaatcagtttccaggtgatggcgatgctgccagtcacaggacctcaccttgagacccacagattgttgcagctggggaagtggaggctcacagctggaaggcgactggtaataaagtcataaattgagccaaagcctcttcagtccttggccagcttctggaccctgatggagagagaagggagccctcagacatttgtccccagagaatgagaagtgggtgtggctggagctcctagggaccctctggtttctgcttctgtttccatggaggccataaaaaagggtagtggccgagcgtgcatgtgacatgcattctctccagcttctccacccccgggtgtaatcctgtctggcttccctgagccctgtgcacaggagggattctggagaagcttgctgcaagacccagcggtgtcctcattcctttgttttacaaccgtttgccgtgttcgcatgccgcagttgtcaggagtgctatccaccatctgggtccatttctgggtctcctcatgtggggtgcgtggagaggctgtactttccagccttcttgaagttaggcacgtccttggcacttgatttctgccaagatctgtgagcagaagtgaggtgtgtctctttctgatgggagcctcaagagctggtgagcaattttttgtctgcatcccctgccagggagactggcgggttcttcaagggagggctcgccagcctgggcccctgactgtggacgttatggaggagaagccttgccaactggagatggacagggaaccggagtaagaagcaaacctgtgtttttttaagccaagggttggcaaattttcttggccagagaatgaatattttaggcttgtcacagctactcaactctgctgttggagcaagaaagcaggcacagacagtacgtaaatgggtggttgtggctgtgtctcgatgaaactttgtttacaagatgagtgaccagcttgcaggctatagtttgccaacctgtttgaagtcttgagaattgggagttgtttgttcctgcagcatgaactagccgtagtgacaactgtaccttccatagtgaccttgctggcatagacaacagaacctactatgcctctgcaagcacaaggcagtagataaggaaagtgtacttgactttggctggagatcttgtggttctcctctcagatcctcttcccatccttctccttgctctctgtcctgagtggttggcctgcagggattatgtcaatcaagggaacccttgttgtctggctttccattgggtctggcccattgggagcactggtgggatctgggaagagagaggatagtgaggctggtgtatttattccccagttctctgccttcaagatcccctcaagctgcctgtgtccttcaactgaaggccacatctcctattgggggctctctcttatctcctggtgacagccaacttctcccttctccctcctctcaccctttgagcccataatagttcgacttgcaccagctctgaggtactaccttatcctttgtggtttgctatactcttttctcatccctcctaagtgatccctttattaaaatcaaatcaaatgacctacctggagggtgccatctgctcctgctgagaccctgactgctgctgctttgaggcacacatgtctgggcttgaattctgattgagtcactgccttagttaaatcatgtcacctctgagacccctgggttttctcttctgcagactgaagcaaaactaacctctaggaaaggaggaggggtttcctaaactatggtatctgtacaatgtcaggaggcatctcaattagtgttaggaaagaaggaaggaatcctcatgacagcttggagagggtggggcctgagtgccacttgccacttgggaaatgaggctaaggctgcgtgggatggagtgttccggggctctgaatgggcctgaaccctggacagacatcagtgcatacacctctggttcagtcccttctggggatattgctggaaaagggtccctcaggacagaaaacgaggcatcagctaggcccaggttcaaatgtgggctttgcactccttgctgtgtgaccttgggcaagtgacactgcctctctgtgcttcatctaaaaatagataacacaaatacctaccacaaatgagaaacagaacataaggcaggcatcctgactctctttttgactgctgtatgcatggtatctaaagcagtacctggtgtataataggtgcttactgcttgttacatgaatgaatgagtgaacaaatgcatttgtgtagagcacttagcacagtgctcacctgcctgaattcagcttctgatgctaccagtttccagctctgtggccttgggtgcctcatttaaatttctttatgtggaagatgggattcaaaaatacctactttgtgggattgctaaggactacatgaatcttcacatgtgccaggcagaaccagcactcactcatgttaaccatcattggtcacacttttgctgggggtcaggctttttaagctgtttaagctcttttgaccatgcatacagcagtcaaaaagagattccggatgcctgccttatgttctaatcctcactcgaggtaagtatttttatccctatttttagatgaagcacagagaggcggtgtcacttgcccaaggtcacacagcaagcagtgcaaagcccacatttgaacctgggtgcctgaccagttggcttactggaattacccctgggctggggacagaaacctgggcaacttgccacatgatattggatgactgttgccctccaagagcctcagtgttcctatctgtgaagtgggaggtggtggctgaagtgggagccttctgagtccccttgtagcttgcacctgcacatgggtcactttcggaccaggctgttgcaggggatgccctatgcacagccccagagatgggacatctggatgtgaatggactcagggcaagttcagggtcagagccctcctcacatgcctgggccagtggcaagcatgtgccaacactactactacactacatcacaaacactactactaatggtattgctgaccttattatcatcatcatcatgaggtgggagctgggaggaagccctcgttggggtaggggtcccagcttctgggccctccgccctgttcccgattcctctatccttggccagtggtgcagcggggaggtggcagcccattggtgctcaaagctggaagagacgttcttcacaagtgccatcgagccttctttttttaaccgccacgagctgactaatgcctgagagtgtcagtccctccagctccgggtggccctgcaggggtgtgaagtgccgagaggagaggaagctgctgccttccagagctgccgggctgcctggggcactgtaggccctcagagcctgagcccaacatctccgagcccctgtccctctgtcagggctcctgtacgctctccaagctctcatgcccctctcagacctcagcctcctttctgagtctccccatccttttcggatctccctgtctgccctccgagccccagctccctctccggagatcagtctcttttttgccctcctcccgctttcctgtagtagtcccttgacagatgctggcagggttgcccgcagggggcccagccctggcctgggtgctgggaatcctggctggagcctcagttcagccagtggctcttaggggactttgtgcagctcctgttcccatttgggtctcgctttccctatctgtgtaatgagagggttggactggatgggtgagaagtccccttcccacactgagccgagaagattccatagaaacccaaaaaccttccagtagggggttaggggtccagcgccccagcacggttccttgcatggtgctggagcccctttcccctttcctcaggggaaagttcattgcctctgaacagcacaggctcttggcagctatctcctgagtagatttttggatgtgcctttccaactcctcccttcctgacgtcagcagtgcctggtccaagtgggcccccagtggtcttgattccatcctattttccaccttgcacaatctaaaacttgaccaaggtgtgcacctcttgatgctggccaagtactctccccatagatgccctggctggttaatgtatcacactgagggcacggaatgctgcatgaactcattttgatgggctgtgcagagtttcggaaccctctggctccagggccaagtctggttactgcggcagccatgaacgtgcactgctcaggtctcctaccgtggggagcatgattgactgacggccccagctgctgtcccttgggatgtgctgccatatctgtgctgaacccacatttcctgtgggctgctgtcagccaaccaccgagcatggcaggaatactaaaggcaggcccactctggagagatgaagaacccttccagtaagtgactttggctcaaggactctccattggcatggcttaaccttttttgaattgtactgcagttcaagactcttcctacgcaatctgccttccttctccctgtccttccccaggtgccagacctgccttctcctgctccctctctcaataaatctcttgtatgttgaactcaatcttgacgtctgcttttcagtgggccatcctaacacagttattacctactaggctactgaagttatgctatacacaggaactgataacagcaacaactaggatttaatgagcacatattgtgggccaggccatatctcatcaactgtttacttcagcctcatgagggaggaactctaactatcccattttataatgaggaaactgaagctcagagaaggaaggaacttactcgaagcagaatttaaaaatgactgtagagtttccaaattttttgttgatatctctctcaccctctatgtaatacaagccggtgagtgtagatatgaagtcgctttttgctaatcgtcgtgtctccctcctcagagactcacgtagtctctggcatgtagaaggctcttgataaatatttgctgcaattgccaatgaataaatgagcagtaaaagagctgtgcacaatggccaagtggcttagccacattgcaaaaaggttgcaaaaagaagaagcttttctttgaaagtcctcggccctggatggctgcagtagcctcctccatccattttccacacagcagccggggggggctcagtcttttggagccttggctttcttgtctggaaaatggggctaacaatgcctatctacatcataggatcgccacggtgcctacaggaggcctcactgcaaagggcttggcacagcacctgagtcagctgctattgtccaacctggagtgtagggtggactgtagtccttctgtgatctcataatccaccagcagacccctcctgtgtacccctctgtgtactcctgctgtgtacctggagacccccaggtctccaggggtcaaaccacaccccacaggcaccttggaagaagaaatccacaggaggaaaaa

SEQ ID NO: 19415 - RNA, 5772 nt, Homo sapiens
  source 1..5772: mol_type = other RNA
ttcgccacttccctccctgcagaatcagtgaggctaggggaggagtcagcatgagccccagccagcctcctcagcttcagggcctccccactgcagccacgaagaggagagggcttggcgagcgtgggcttggtcctccagaaggacttggggaggcaagttgcagggatcacaaaacaacctccttcaatacccttttcccattgctcagagggagaaattgaggcccagagagggctagtgacttgcacaaagtcatatagcgagatagtagctgcaaggattcaaacccaagtccctttctttggagccagttatactcccaataagccctatggctgcccaagtaccccaggccactggcaaaattgagaagaaagcaaagcaataggggcagcagtaattcctgtgtgttgtggatttagcaggtattgggtatcacgctgcaacccttcacgtgcaccttgtttagtcctcgctgcagtcctataaggttaaggcacatgatacacattatcagcatcatccccattttagagatgagaaaattgaggatcagagaggttatgtgatttccttcaggtcaattcaagagacttgaacccagacctgctgatcccagagcggcatacaaggacccagccctcaatcctggggtctttctgtggtgtaactcttggggcgtgcccatgggggctgcctcgtgctgaccacagcaaggcccaaggaatgagcatttctccgtccatccatctgtctacctacctatccgtctgttcactcaataaatatttacccagggctttctccatgccaggcaatattcaggcattgggaggcatacagcagtgaacaaagcaggcagtgcctggcttcgtggccctcataccctcgtggggagaggcagactataaacagagaaacaacaaagatgtgtgtcaggtggtggtgagggctatggagaaaaacaaagccagaggagggggcagcgcaggatggcggggtcggagaaggcttctctgaggaggtgacatttgagcggtgatctgaaggaggtgagggcttgggccgtgtggggatcactagagaggggtttctggcagaggaaatagcgggagcaaaggccctgaggcgggagcgtgcctggcatgttggaggaacagagaacaggtcagtgcagctggagacggcaagcaagcggcagggcgttggggaggtggagaggtcagtgggaatcagaccaagggcggccctgtcaggttttcttctgagtgagatggaagccattggaggttctgagcagaagcgtggaatcatctgattgagtttttaagagcatcttctggctgctggagtgaggatgtactacagggctcaaaggaagagggagcgggggttagaaaggcaaggtagtatgtgggtgtcagatggcagaggctagggccacgcagagtgaaggaggtggagagggaggccaagatctgaatatattctaaaggctaagccacaggattagggtctgagaaccctctaggatggctccaggtttttggcttaaaccagaatgaaactgtcatttatgcaggtggggaggactgctggaaaagcagtgcgggcccgggctttgcacatctcagttcgtttgtgccttatattcctcaagcatcagaatcaccggagacacttgttgaagtccagatttctgggatcctccaccagagcttcccattcaatagagctgggtggggcttgagaatgtggatttctaatcagtttccaggtgatggcgatgctgccagtcacaggacctcaccttgagacccacagattgttgcagctggggaagtggaggctcacagctggaaggcgactggtaataaagtcataaattgagccaaagcctcttcagtccttggccagcttctggaccctgatggagagagaagggagccctcagacatttgtccccagagaatgagaagtgggtgtggctggagctcctagggaccctctggtttctgcttctgtttccatggaggccataaaaaagggtagtggccgagcgtgcatgtgacatgcattctctccagcttctccacccccgggtgtaatcctgtctggcttccctgagccctgtgcacaggagggattctggagaagcttgctgcaagacccagcggtgtcctcattcctttgttttacaaccgtttgccgtgttcgcatgccgcagttgtcaggagtgctatccaccatctgggtccatttctgggtctcctcatgtggggtgcgtggagaggctgtactttccagccttcttgaagttaggcacgtccttggcacttgatttctgccaagatctgtgagcagaagtgaggtgtgtctctttctgatgggagcctcaagagctggtgagcaattttttgtctgcatcccctgccagggagactggcgggttcttcaagggagggctcgccagcctgggcccctgactgtggacgttatggaggagaagccttgccaactggagatggacagggaaccggagtaagaagcaaacctgtgtttttttaagccaagggttggcaaattttcttggccagagaatgaatattttaggcttgtcacagctactcaactctgctgttggagcaagaaagcaggcacagacagtacgtaaatgggtggttgtggctgtgtctcgatgaaactttgtttacaagatgagtgaccagcttgcaggctatagtttgccaacctgtttgaagtcttgagaattgggagttgtttgttcctgcagcatgaactagccgtagtgacaactgtaccttccatagtgaccttgctggcatagacaacagaacctactatgcctctgcaagcacaaggcagtagataaggaaagtgtacttgactttggctggagatcttgtggttctcctctcagatcctcttcccatccttctccttgctctctgtcctgagtggttggcctgcagggattatgtcaatcaagggaacccttgttgtctggctttccattgggtctggcccattgggagcactggtgggatctgggaagagagaggatagtgaggctggtgtatttattccccagttctctgccttcaagatcccctcaagctgcctgtgtccttcaactgaaggccacatctcctattgggggctctctcttatctcctggtgacagccaacttctcccttctccctcctctcaccctttgagcccataatagttcgacttgcaccagctctgaggtactaccttatcctttgtggtttgctatactcttttctcatccctcctaagtgatccctttattaaaatcaaatcaaatgacctacctggagggtgccatctgctcctgctgagaccctgactgctgctgctttgaggcacacatgtctgggcttgaattctgattgagtcactgccttagttaaatcatgtcacctctgagacccctgggttttctcttctgcagactgaagcaaaactaacctctaggaaaggaggaggggtttcctaaactatggtatctgtacaatgtcaggaggcatctcaattagtgttaggaaagaaggaaggaatcctcatgacagcttggagagggtggggcctgagtgccacttgccacttgggaaatgaggctaaggctgcgtgggatggagtgttccggggctctgaatgggcctgaaccctggacagacatcagtgcatacacctctggttcagtcccttctggggatattgctggaaaagggtccctcaggacagaaaacgaggcatcagctaggcccaggttcaaatgtgggctttgcactccttgctgtgtgaccttgggcaagtgacactgcctctctgtgcttcatctaaaaatagataacacaaatacctaccacaaatgagaaacagaacataaggcaggcatcctgactctctttttgactgctgtatgcatggtatctaaagcagtacctggtgtataataggtgcttactgcttgttacatgaatgaatgagtgaacaaatgcatttgtgtagagcacttagcacagtgctcacctgcctgaattcagcttctgatgctaccagtttccagctctgtggccttgggtgcctcatttaaatttctttatgtggaagatgggattcaaaaatacctactttgtgggattgctaaggactacatgaatcttcacatgtgccaggcagaaccagcactcactcatgttaaccatcattggtcacacttttgctgggggtcaggctttttaagctgtttaagctcttttgaccatgcatacagcagtcaaaaagagattccggatgcctgccttatgttctaatcctcactcgaggtaagtatttttatccctatttttagatgaagcacagagaggcggtgtcacttgcccaaggtcacacagcaagcagtgcaaagcccacatttgaacctgggtgcctgaccagttggcttactggaattacccctgggctggggacagaaacctgggcaacttgccacatgatattggatgactgttgccctccaagagcctcagtgttcctatctgtgaagtgggaggtggtggctgaagtgggagccttctgagtccccttgtagcttgcacctgcacatgggtcactttcggaccaggctgttgcaggggatgccctatgcacagccccagagatgggacatctggatgtgaatggactcagggcaagttcagggtcagagccctcctcacatgcctgggccagtggcaagcatgtgccaacactactactacactacatcacaaacactactactaatggtattgctgaccttattatcatcatcatcatgaggtgggagctgggaggaagccctcgttggggtaggggtcccagcttctgggccctccgccctgttcccgattcctctatccttggccagtggtgcagcggggaggtggcagcccattggtgctcaaagctggaagagacgttcttcacaagtgccatcgagccttctttttttaaccgccacgagctgactaatgcctgagagtgtcagtccctccagctccgggtggcctcgaagcagaatttaaaaatgactgtagagtttccaaattttttgttgatatctctctcaccctctatgtaatacaagccggtgagtgtagatatgaagtcgctttttgctaatcgtcgtgtctccctcctcagagactcacgtagtctctggcatgtagaaggctcttgataaatatttgctgcaattgccaatgaataaatgagcagtaaaagagctgtgcacaatggccaagtggcttagccacattgcaaaaaggttgcaaaaagaagaagcttttctttgaaagtcctcggccctggatggctgcagtagcctcctccatccattttccacacagcagccggggggggctcagtcttttggagccttggctttcttgtctggaaaatggggctaacaatgcctatctacatcataggatcgccacggtgcctacaggaggcctcactgcaaagggcttggcacagcacctgagtcagctgctattgtccaacctggagtgtagggtggactgtagtccttctgtgatctcataatccaccagcagacccctcctgtgtacccctctgtgtactcctgctgtgtacctggagacccccaggtctccaggggtcaaaccacaccccacaggcaccttggaagaagaaatccacaggaggaaaaa

SEQ ID NO: 19416 - RNA, 5524 nt, Homo sapiens
  source 1..5524: mol_type = other RNA
ttcgccacttccctccctgcagaatcagtgaggctaggggaggagtcagcatgagccccagccagcctcctcagcttcagggcctccccactgcagccacgaagaggagagggcttggcgagcgtgggcttggtcctccagaaggacttggggaggcaagttgcagggatcacaaaacaacctccttcaatacccttttcccattgctcagagggagaaattgaggcccagagagggctagtgacttgcacaaagtcatatagcgagatagtagctgcaaggattcaaacccaagtccctttctttggagccagttatactcccaataagccctatggctgcccaagtaccccaggccactggcaaaattgagaagaaagcaaagcaataggggcagcagtaattcctgtgtgttgtggatttagcaggtattgggtatcacgctgcaacccttcacgtgcaccttgtttagtcctcgctgcagtcctataaggttaaggcacatgatacacattatcagcatcatccccattttagagatgagaaaattgaggatcagagaggttatgtgatttccttcaggtcaattcaagagacttgaacccagacctgctgatcccagagcggcatacaaggacccagccctcaatcctggggtctttctgtggtgtaactcttggggcgtgcccatgggggctgcctcgtgctgaccacagcaaggcccaaggaatgagcatttctccgtccatccatctgtctacctacctatccgtctgttcactcaataaatatttacccagggctttctccatgccaggcaatattcaggcattgggaggcatacagcagtgaacaaagcaggcagtgcctggcttcgtggccctcataccctcgtggggagaggcagactataaacagagaaacaacaaagatgtgtgtcaggtggtggtgagggctatggagaaaaacaaagccagaggagggggcagcgcaggatggcggggtcggagaaggcttctctgaggaggtgacatttgagcggtgatctgaaggaggtgagggcttgggccgtgtggggatcactagagaggggtttctggcagaggaaatagcgggagcaaaggccctgaggcgggagcgtgcctggcatgttggaggaacagagaacaggtcagtgcagctggagacggcaagcaagcggcagggcgttggggaggtggagaggtcagtgggaatcagaccaagggcggccctgtcaggttttcttctgagtgagatggaagccattggaggttctgagcagaagcgtggaatcatctgattgagtttttaagagcatcttctggctgctggagtgaggatgtactacagggctcaaaggaagagggagcgggggttagaaaggcaaggtagtatgtgggtgtcagatggcagaggctagggccacgcagagtgaaggaggtggagagggaggccaagatctgaatatattctaaaggctaagccacaggattagggtctgagaaccctctaggatggctccaggtttttggcttaaaccagaatgaaactgtcatttatgcaggtggggaggactgctggaaaagcagtgcgggcccgggctttgcacatctcagttcgtttgtgccttatattcctcaagcatcagaatcaccggagacacttgttgaagtccagatttctgggatcctccaccagagcttcccattcaatagagctgggtggggcttgagaatgtggatttctaatcagtttccaggtgatggcgatgctgccagtcacaggacctcaccttgagacccacagattgttgcagctggggaagtggaggctcacagctggaaggcgactggtaataaagtcataaattgagccaaagcctcttcagtccttggccagcttctggaccctgatggagagagaagggagccctcagacatttgtccccagagaatgagaagtgggtgtggctggagctcctagggaccctctggtttctgcttctgtttccatggaggccataaaaaagggtagtggccgagcgtgcatgtgacatgcattctctccagcttctccacccccgggtgtaatcctgtctggcttccctgagccctgtgcacaggagggattctggagaagcttgctgcaagacccagcggtgtcctcattcctttgttttacaaccgtttgccgtgttcgcatgccgcagttgtcaggagtgctatccaccatctgggtccatttctgggtctcctcatgtggggtgcgtggagaggctgtactttccagccttcttgaagttaggcacgtccttggcacttgatttctgccaagatctgtgagcagaagtgaggtgtgtctctttctgatgggagcctcaagagctggtgagcaattttttgtctgcatcccctgccagggagactggcgggttcttcaagggagggctcgccagcctgggcccctgactgtggacgttatggaggagaagccttgccaactggagatggacagggaaccggagtaagaagcaaacctgtgtttttttaagccaagggttggcaaattttcttggccagagaatgaatattttaggcttgtcacagctactcaactctgctgttggagcaagaaagcaggcacagacagtacgtaaatgggtggttgtggctgtgtctcgatgaaactttgtttacaagatgagtgaccagcttgcaggctatagtttgccaacctgtttgaagtcttgagaattgggagttgtttgttcctgcagcatgaactagccgtagtgacaactgtaccttccatagtgaccttgctggcatagacaacagaacctactatgcctctgcaagcacaaggcagtagataaggaaagtgtacttgactttggctggagatcttgtggttctcctctcagatcctcttcccatccttctccttgctctctgtcctgagtggttggcctgcagggattatgtcaatcaagggaacccttgttgtctggctttccattgggtctggcccattgggagcactggtgggatcttattatcatcatcatcatgaggtgggagctgggaggaagccctcgttggggtaggggtcccagcttctgggccctccgccctgttcccgattcctctatccttggccagtggtgcagcggggaggtggcagcccattggtgctcaaagctggaagagacgttcttcacaagtgccatcgagccttctttttttaaccgccacgagctgactaatgcctgagagtgtcagtccctccagctccgggtggccctgcaggggtgtgaagtgccgagaggagaggaagctgctgccttccagagctgccgggctgcctggggcactgtaggccctcagagcctgagcccaacatctccgagcccctgtccctctgtcagggctcctgtacgctctccaagctctcatgcccctctcagacctcagcctcctttctgagtctccccatccttttcggatctccctgtctgccctccgagccccagctccctctccggagatcagtctcttttttgccctcctcccgctttcctgtagtagtcccttgacagatgctggcagggttgcccgcagggggcccagccctggcctgggtgctgggaatcctggctggagcctcagttcagccagtggctcttaggggactttgtgcagctcctgttcccatttgggtctcgctttccctatctgtgtaatgagagggttggactggatgggtgagaagtccccttcccacactgagccgagaagattccatagaaacccaaaaaccttccagtagggggttaggggtccagcgccccagcacggttccttgcatggtgctggagcccctttcccctttcctcaggggaaagttcattgcctctgaacagcacaggctcttggcagctatctcctgagtagatttttggatgtgcctttccaactcctcccttcctgacgtcagcagtgcctggtccaagtgggcccccagtggtcttgattccatcctattttccaccttgcacaatctaaaacttgaccaaggtgtgcacctcttgatgctggccaagtactctccccatagatgccctggctggttaatgtatcacactgagggcacggaatgctgcatgaactcattttgatgggctgtgcagagtttcggaaccctctggctccagggccaagtctggttactgcggcagccatgaacgtgcactgctcaggtctcctaccgtggggagcatgattgactgacggccccagctgctgtcccttgggatgtgctgccatatctgtgctgaacccacatttcctgtgggctgctgtcagccaaccaccgagcatggcaggaatactaaaggcaggcccactctggagagatgaagaacccttccagtaagtgactttggctcaaggactctccattggcatggcttaaccttttttgaattgtactgcagttcaagactcttcctacgcaatctgccttccttctccctgtccttccccaggtgccagacctgccttctcctgctccctctctcaataaatctcttgtatgttgaactcaatcttgacgtctgcttttcagtgggccatcctaacacagttattacctactaggctactgaagttatgctatacacaggaactgataacagcaacaactaggatttaatgagcacatattgtgggccaggccatatctcatcaactgtttacttcagcctcatgagggaggaactctaactatcccattttataatgaggaaactgaagctcagagaaggaaggaacttactcgaagcagaatttaaaaatgactgtagagtttccaaattttttgttgatatctctctcaccctctatgtaatacaagccggtgagtgtagatatgaagtcgctttttgctaatcgtcgtgtctccctcctcagagactcacgtagtctctggcatgtagaaggctcttgataaatatttgctgcaattgccaatgaataaatgagcagtaaaagagctgtgcacaatggccaagtggcttagccacattgcaaaaaggttgcaaaaagaagaagcttttctttgaaagtcctcggccctggatggctgcagtagcctcctccatccattttccacacagcagccggggggggctcagtcttttggagccttggctttcttgtctggaaaatggggctaacaatgcctatctacatcataggatcgccacggtgcctacaggaggcctcactgcaaagggcttggcacagcacctgagtcagctgctattgtccaacctggagtgtagggtggactgtagtccttctgtgatctcataatccaccagcagacccctcctgtgtacccctctgtgtactcctgctgtgtacctggagacccccaggtctccaggggtcaaaccacaccccacaggcaccttggaagaagaaatccacaggaggaaaaa

SEQ ID NO: 19417 - RNA, 4208 nt, Homo sapiens
  source 1..4208: mol_type = other RNA
ttcgccacttccctccctgcagaatcagtgaggctaggggaggagtcagcatgagccccagccagcctcctcagcttcagggcctccccactgcagccacgaagaggagagggcttggcgagcgtgggcttggtcctccagaaggacttggggaggcaagttgcagggatcacaaaacaacctccttcaatacccttttcccattgctcagagggagaaattgaggcccagagagggctagtgacttgcacaaagtcatatagcgagatagtagctgcaaggattcaaacccaagtccctttctttggagccagttatactcccaataagccctatggctgcccaagtaccccaggccactggcaaaattgagaagaaagcaaagcaataggggcagcagtaattcctgtgtgttgtggatttagcaggtattgggtatcacgctgcaacccttcacgtgcaccttgtttagtcctcgctgcagtcctataaggttaaggcacatgatacacattatcagcatcatccccattttagagatgagaaaattgaggatcagagaggttatgtgatttccttcaggtcaattcaagagacttgaacccagacctgctgatcccagagcggcatacaaggacccagccctcaatcctggggtctttctgtggtgtaactcttggggcgtgcccatgggggctgcctcgtgctgaccacagcaaggcccaaggaatgagcatttctccgtccatccatctgtctacctacctatccgtctgttcactcaataaatatttacccagggctttctccatgccaggcaatattcaggcattgggaggcatacagcagtgaacaaagcaggcagtgcctggcttcgtggccctcataccctcgtggggagaggcagactataaacagagaaacaacaaagatgtgtgtcaggtggtggtgagggctatggagaaaaacaaagccagaggagggggcagcgcaggatggcggggtcggagaaggcttctctgaggaggtgacatttgagcggtgatctgaaggaggtgagggcttgggccgtgtggggatcactagagaggggtttctggcagaggaaatagcgggagcaaaggccctgaggcgggagcgtgcctggcatgttggaggaacagagaacaggtcagtgcagctggagacggcaagcaagcggcagggcgttggggaggtggagaggtcagtgggaatcagaccaagggcggccctgtcaggttttcttctgagtgagatggaagccattggaggttctgagcagaagcgtggaatcatctgattgagtttttaagagcatcttctggctgctggagtgaggatgtactacagggctcaaaggaagagggagcgggggttagaaaggcaaggtagtatgtgggtgtcagatggcagaggctagggccacgcagagtgaaggaggtggagagggaggccaagatctgaatatattctaaaggctaagccacaggattagggtctgagaaccctctaggatggctccaggtttttggcttaaaccagaatgaaactgtcatttatgcaggtggggaggactgctggaaaagcagtgcgggcccgggctttgcacatctcagttcgtttgtgccttatattcctcaagcatcagaatcaccggagacacttgttgaagtccagatttctgggatcctccaccagagcttcccattcaatagagctgggtggggcttgagaatgtggatttctaatcagtttccaggtgatggcgatgctgccagtcacaggacctcaccttgagacccacagattgttgcagctggggaagtggaggctcacagctggaaggcgactggtaataaagtcataaattgagccaaagcctcttcagtccttggccagcttctggaccctgatggagagagaagggagccctcagacatttgtccccagagaatgagaagtgggtgtggctggagctcctagggaccctctggtttctgcttctgtttccatggaggccataaaaaagggtagtggccgagcgtgcatgtgacatgcattctctccagcttctccacccccgggtgtaatcctgtctggcttccctgagccctgtgcacaggagggattctggagaagcttgctgcaagacccagcggtgtcctcattcctttgttttacaaccgtttgccgtgttcgcatgccgcagttgtcaggagtgctatccaccatctgggtccatttctgggtctcctcatgtggggtgcgtggagaggctgtactttccagccttcttgaagttaggcacgtccttggcacttgatttctgccaagatctgtgagcagaagtgaggtgtgtctctttctgatgggagcctcaagagctggtgagcaattttttgtctgcatcccctgccagggagactggcgggttcttcaagggagggctcgccagcctgggcccctgactgtggacgttatggaggagaagccttgccaactggagatggacagggaaccggagtaagaagcaaacctgtgtttttttaagccaagggttggcaaattttcttggccagagaatgaatattttaggcttgtcacagctactcaactctgctgttggagcaagaaagcaggcacagacagtacgtaaatgggtggttgtggctgtgtctcgatgaaactttgtttacaagatgagtgaccagcttgcaggctatagtttgccaacctgtttgaagtcttgagaattgggagttgtttgttcctgcagcatgaactagccgtagtgacaactgtaccttccatagtgaccttgctggcatagacaacagaacctactatgcctctgcaagcacaaggcagtagataaggaaagtgtacttgactttggctggagatcttgtggttctcctctcagatcctcttcccatccttctccttgctctctgtcctgagtggttggcctgcagggattatgtcaatcaagggaacccttgttgtctggctttccattgggtctggcccattgggagcactggtgggatcttattatcatcatcatcatgaggtgggagctgggaggaagccctcgttggggtaggggtcccagcttctgggccctccgccctgttcccgattcctctatccttggccagtggtgcagcggggaggtggcagcccattggtgctcaaagctggaagagacgttcttcacaagtgccatcgagccttctttttttaaccgccacgagctgactaatgcctgagagtgtcagtccctccagctccgggtggcctcgaagcagaatttaaaaatgactgtagagtttccaaattttttgttgatatctctctcaccctctatgtaatacaagccggtgagtgtagatatgaagtcgctttttgctaatcgtcgtgtctccctcctcagagactcacgtagtctctggcatgtagaaggctcttgataaatatttgctgcaattgccaatgaataaatgagcagtaaaagagctgtgcacaatggccaagtggcttagccacattgcaaaaaggttgcaaaaagaagaagcttttctttgaaagtcctcggccctggatggctgcagtagcctcctccatccattttccacacagcagccggggggggccttttaaataaaaaaaattagattgtgttaccttcttgcacactcctatagtttcccatcttattcaggataaaaacctgaggatgtgaccaggaaccaccaggccttatgggtccagcccctgccactctgaacccttcctcttgctgtcgcccctccatgcacttggtgggaagccaatgccgttggcctcagtgtatctggaaggctccaccctggcccagccctggagccctcgtatgtacagttccctctgcctagaacacttgtccccagcatccccacggctggtcccttccacccctcatgtctcagcatgatcccctcctcagggagcccggccaacccagtccttccaccgcatcccagctgctctgcctcgccaccctgccccatcctttcacagcacgtacccctgccagaatgatcgttagtcatgcacttaattgtttatcaccaggaagagtggacacttcctgaagacaggggtctgagattccgttatggcctcggtgcctaaaagagtccctg

SEQ ID NO: 19418 - RNA, 1109 nt, Homo sapiens
  source 1..1109: mol_type = other RNA
ttcgggctggcctgctgctccggggccccaccggccaccgcggaggacgaggacgaggacgaagaggcgagggaagggctggatttggcagcagctgggggcttggccagtcctgccttgggcacgagggcggccgcctggtcccggggcctgtgggcccgtctggctcgaggcatctgcatctgcccgtggatccgctccactcggggcggccgggggctccacaccggggccgggacccgcgctggctgtccactcctaaaactccacagccggggcggccggggcggcgaccgcggcaggagccagaactccggccccgggcccagggcctcacaggcgggcaggtccacggcgagctgaaacatggctatcagtatccaggcatggcttccgagggggcggcccggccagcggatggacatggagctgagtcctaaaagctgttgaatccacatggtcacgtttcggggagcggggcctcagacctggctcgcccaggccatctgcgcggcgcccgcgcccgctcgcttccgtcccgcggcgccggtctccggctctcggtccgccgcctcccgccgcccgccggccgcggggcgcacagcgagtcagagcgcggccgcgcggggctccatgccggccggcgcgccgccgccgttggggcgcatggctcaggctgggcggcccgcgggggcgcacatcctccggccggggcgcggggctcgcggccccctccgccggcggcacagcgaaggcggcagcgaggcggggcgtgttccggcgctgtcgcggcgcagcaaagggctggggagccgcggcttcgccctccggggcggcgaggagggaggccggcggcgctgccgctcacggtgcgtgtctcccggcgcgcggctcttgcctccagccggagctccgcgccgatggggcggcgctgcttagggtttggggtgacgcgacgcggacggacgcgagtcccctccgcgctgccgggtcggggggctctgccagaggctccgccgccgatcggcgccactcaagttgcccgggggctccgtctgagcgctcgctctgcagacggccgcggcccggagactggcaggaggcgggca

SEQ ID NO: 19419 - RNA, 1275 nt, Homo sapiens
  source 1..1275: mol_type = other RNA
ttcgggctggcctgctgctccggggccccaccggccaccgcggaggacgaggacgaggacgaagaggcgagggaagggctggatttggcagcagctgggggcttggccagtcctgccttgggcacgagggcggccgcctggtcccggggcctgtgggcccgtctggctcgaggcatctgcatctgcccgtggatccgctccactcggggcggccgggggctccacaccggggccgggacccgcgctggctgtccactcctaaaactccacagccggggcggccggggcggcgaccgcggcaggagccagaactccggccccgggcccagggcctcacaggcgggcaggtccacggcgagctgaaacatggctatcagtatccaggcatggcttccgagggggcggcccggccagcggatggacatggagctgagtcctaaaagctgttgaatccacatggtcacgtttcggggagcggggcctcagacctggctcgcccaggccatctgcgcggcgcccgcgcccgctcgcttccgtcccgcggcgccggtctccggctctcggtccgccgcctcccgccgcccgccggccgcggggcgcacagcgagtcagagcgcggccgcgcggggctccatgccggccggcgcgccgccgccgttggggcgcatggctcaggctgggcggcccgcgggggcgcacatcctccggccggggcgcggggctcgcggccccctccgccggcggcacagcgaaggcggcagcgaggcggggcgtgttccggcgctgtcgcggcgcagcaaagggctggggagccgcggcttcgccctccggggcggcgaggagggaggccggcggcgctgccgctcacggtgcgtgtctcccggcgcgcggctcttgcctccagccggagctccgcgccgatggggcggcgctgcttagggtttggggtgacgcgacgcggacggacgcgagtcccctccgcgctgccgggtcggggggctctgccagaggctccgccgccgatcggcgccactcaagttgcccgggggctccgtctgagcgctcgctctgcagacggccgcggcccggagactggcaggaggcgggcacgagaggcgcgcggggcgagggcgccgtggagcgcggggcgtggggacgcgcggcggcggcgccgcgcggaggaggcgcgcggggatcccggggccccgccgcccgcgcccaccgcgcccgccgcagagccgcccgcgctgctcagccgcctccctcctcgcgtct

SEQ ID NO: 19420 - RNA, 995 nt, Homo sapiens
  source 1..995: mol_type = other RNA
ttcgggctggcctgctgctccggggccccaccggccaccgcggaggacgaggacgaggacgaagaggcgagggaagggctggatttggcagcagctgggggcttggccagtcctgccttgggcacgagggcggccgcctggtcccggggcctgtgggcccgtctggctcgaggcatctgcatctgcccgtggatccgctccactcggggcggccgggggctccacaccggggccgggacccgcgctggctgtccactcctaaaactccacagccggggcggccggggcggcgaccgcggcaggagccagaactccggccccgggcccagggcctcacaggcgggcaggtccacggcgagctgaaacatggctatcagtatccaggcatggcttccgagggggcggcccggccagcggatggacatggagttctggcctcctctggatcgtactcagggaaatgagatctgctccggataaacctaaagtttattgacgcgaagtgtctgttctgttgacatttccgctccccctgtttatctgcagtgccggtgccctttgaaaccctgttatccacctcctcagctccccggagggctgcagaaagggcaaatcctgcgcaaccctgaggagggcggggctgcctctccacgcagcggggctgcaggggagaagtcagggctggcggggcggcccctccccagttcacatggagcggctttgtcaccaggtctggggtcgcctctggaccagtggactctctggtgtcacatgaaaaccagggcgcggcagagagccacgtggaagggctcagaggagccaggcccacgctccctcttccaccagcacagataattgaagactgattataggtgtcattcaaagtcagttctcgtcaccagcctcacgtctgaaagttaaaatgaatcccaaaactgtaatgactgaagcgggtggggggcgcgagggtgttcaggtgccaagcgccagcctga

SEQ ID NO: 19421 - RNA, 8527 nt, Homo sapiens
  source 1..8527: mol_type = other RNA
ttctcaaggaggtgtcgtttatgtgaactaaaatataaatttcacctttctgagaagagtaatgtacagcatgcactgcatatgtggtgtccctagggatggggctgtagctgcgagcatggtgatgcctgttttgcatcctgtgcacccactcctcagtgctgggctacttcaaggaactttttgtgccttctagacgactacacataagaactgtggactcctgagaaaacgcatgcactttggttccttaagaatttatctacttttgccaaatgaggcttggctcaaataagaaatacgttgtatagaggccacagccattcttcgtcagctgagacattttactccagattcctcaattctctaaactcttttcactgatcaactagtcatcatttgcaaggattgtcctttagtgctcccaaaaggctctcctgcctctcaggtcccttcattgctgatccacagtgtccattttctgtcaaagactaaaacattttctcattgactgttaaaatacctttcaaagccttcagtcaccaatttatgaagggttaagcatagtccacccaagaatatttcaccctttttaattatcttttttccccattttttaagagtatatttgaagaatggaagggtatgacagaattgatactcaagagatatctcctaggcttctctccccattttcttttggtgacgcttaactcttaacctaatggagagaaatagagggaaataaacacacacacacacacacacacacacacacacacacacacacagagagagagagagagagagagagaggagagagagagagagagaacatgcaagagaaagacaagcaccagactatgtaaggccatctgcagcattaatctagtatacatgtttgggaagtaggttataaataagctatttatattgtggaaatgtgtaaaaaatgttataaatagtaagtgattaatacaattttgattccaactgaaacagaggctacagcataaacaccgaaagggaaaaactataaaaaacaattactatatggttacaggcaggattttggtttatgtttttttagattcagaatgtatgaatatgtataagaccattaatgtctgaaagtaaaaaaaacagttgaagtatcttttccataatgaaaaacattgtaataatagaatacatacaatctttttggggtgggggcaacattctgaacagtaaaaaaattttgtcactttgcaatactgtatgtacatagaattttccaaagtgataactgtttttagtatataatttctaaaactgtattatagtgatgcatgtttacttatataactttaagtgatatcttaaaatgaaataaaagagaatttagttgttatcatacctctgttatgatttctcaaaagaatagtatatttactggtatttgtgttttttttcagtgaaatactgttttgtattactcagccttttttcttccaatttattaaggtttaactgacataaaaatcatatttaaggtgtacaacatgacgttttgatatatgtgtacattatgcaatgattaaatcaagctaattgaaaaataaaatatgaacataaaatatttatttgaaactctaagaaaaaattacaagatctctgtggtaggcagagtaacagcccccgcccaaacaatgttcacaatgtaacccctgaactcgtaagcatcatattttattgtagaagaaaatttgtagatgttattaaatattttgagattgggattatcctagattatctaggtgagcccaacattatcacaagggcccttatacgttggagaaaggtggttagaatgagaaacattgcaaaatactatagtattgactagaggtagaggtaaaggccatgagccaaagaatggagaaagtaactagaatcttctaaagacaatcaagtagattctcctctagagccaacagaaggaacaaagccctgccaatgccttcattttagccaagagaaacctaatttagatttttgacctttagactctaatataataaatttgtgttgttgtaaacaactaaatctgtggcaatttattacagtatcaatagaaaccccaaaacatctgtatgctaaaactgtaaatatactaaaaaaaaatactaattaagtggcgaggactatcatatttatggattgaaggattcaaatctatagacttttagacttccattaatctctagaagtaatacaattccaaccaatgtcccagaaaaatatttgtagacattagcaagatgattctaaaactgatataaaaggcgaataaactagaatatccaaaacaatctgaaagagaatcacaaagctggaaaatttacacttgtaatttccagatttactgtctaattagattacccaatgtactgtggtactgaagaaaggatggacaaatagaaggaccagaaatatccatatatgtcaccaattcattttgactaagctgtaaagtcaatctaatgaagaaatgatagtatttaaacagtaagatgctgggaaatgtgagatatataaaaaatatgaaccttgatcgtatttcaaaccacatacagaaattaacacaatcttaagccaaaacgtcaaactatcaaattgcatgaaaaaaatgagagaaaatatttttgaccattaaattattacatatgatatcaaaatataaaaataaaatttattaaaaataaattgataaaatagactttgaaaaaattaagacgtcttcaaataagaccactgagataataaaaaggcaaattacagaataaaaatatttatcacattattgaattacatataacatatatccagcataaataactacatataatttagcactcctgtgtatactaagtattttactagttactttgtaaaaattatctgtgttttaaaatgtcagttctgttagcatgtgttgaagctgttttgatctgtgttgtagtcctagcacatgaaaaaccctggtttaatgtttacgtattcattctggaccttccttgctatactataatttcgtcacctcgttaatgtgaatatattagtttatcctcataatatataataaattaaaatgtgttcagcttaggagtcaggaacatggaaaggcaagaactctaactgaacaggctgagtatgtatagattcaggaagctcaaaagaggaaaaataactgccaaaaacaacttttacacctgtccgagttattcttatatcagaattctgccaaagaaaactacatttttattgatgtatttctttttcagaccatgaggataattcctatttattacagaacaatgtggaaagcacatacaaggtgtgaaaaacatgaatagcagtaatgaaataattccagtaacatcataatgtggatacagtgtttgataaaatttagatgtggatctttccacacatttatctgtatttatacttaggttttaggatggggtcaacaattttgtgccattttcttataaatgatttcaaataatgcatcatgaatgttttataaaaacattagcctaataattgtgaaacatggttttatgtgctgtttcattctatcatacaatatttttctgattgatttctgacttttttagcattttaaatattttaaatgttttctaagtgttttctactttcagatttactaaaatattccattttaaatagtattttctttttcttagattttgttccataatttttttcattaagaacatacatgtattatcacatttaatccactcaaaaccctcagaaggcagtagttatttttatcatgaacttacagataaagaatgcagcttagagaagttaaataagttgtttaatgctgtgaaccaagtccgtagtctgatcctagggttatactgtaacacgaaaggatacttacacgcaagactaaagaggatcaaacctgatactcaacctatggctgcattccatcctgaaccacagtgccagaaaacagtgattacagttttctatgattcagtgagttcactgggagtttcttctgcttaggctcacctgggctcaaacatgcaactacagacatctactctggggtggtctagaatgccccctcacaaggatgcagttccaactggaatggcaggaacagctagcatggctgggcctctccctccagctggtctttcattctggaattgttctcagcgtggggagctcaagactccaaaagggcaaagacagaaactgtgaaacatcttaggactcagcctaggaaagtgagcaatgtcacatcagaaagatttcactgatcaaaataaccaagccagcatcaccgcataaggaaatgaattcaaaccctgaaaggagagagacaaaaagtctcattgcaaaatggtgttttcacaggaacacctgactcattgggagtcattgttaccaaagcacacacaaaatctacacagtattttcattctagtttacgggatatgtctttgttgttatttgtaaagtgaaacttcacagggttacattgataaaaggtgggggctctctgacaaataccaagaattattaagaatttttgtacttgtgttagcctggatggagcacctttaacatcgctggcacaagtgatatgtttcacttctttaggcacattttttgcttagagttggaaggagcccaggtggtttgctgacccaatagtgctagattgctgagatacttccgagctgactgcttgggaacatggaattgttcatttatgtgtacccattctgggtcaagagactgctgattgcttgggaacactgagagattcctttatgtgtgcccactctgggtcaagacagaccacttgtcctgtgaaccatctggtccaatctctccctgttctctgtgaccttcatgggtagagaggaacaaagcaactaaggctcctgtcattaaccacagttgtcaggtttccttttattgacaaatttggagttggaatggttttgaggagaggagcctgagctgcctgactcaaaccttgcagcaaattcctggctgctctgagacatcttctccctgcagcctgcatcagagggtacatttcagaacagaggcttaaacaatgggaaggaaaagaacaaaaagacaatcaggaatgagtagtaagaataatcggctgccatgctagtcatgggactcaggagaacacaggaggtgaagggtatcacaaatgccttcatcccccaccccagcctacaccactgccagccttgcccctgctctgtccccctcagaaggacaccaagagacagagggtggcaaaaatccaatgcgttattcttttccgaccccctccccactctcaccagatgcctccgaaaatcagctggacggtgggagggatcaagaatgactgccgtcaccatggaaactccttgatggcgagattgctttgagaaccaggaggggatgagataagcaccagaggaacactgggcagtcagggcccagcatccaccaaccctttcttccagataactcctttgttctctgggctggtctccctcttgctcctataggggccctttctgactcttcacctgttttgattcttcagtggtgcccttcccgggtctgggagggaagggcccgaggcccactcagggctgccccaggatggccacttctcactgcagcccagacaccctggtctataagacacactatccttgccactgagaaggaagggacgtcaacacttttgagccaagccctgtgtcccctgcatcctgcaaggaagaagaaaaataaagacctgactatttttcacaggtgcaacgggtgactaaagacagaaagagagtggtgtggttttcacttcatcttgttgagaagccagggcctgaagtccagagatccccattcacatgcaccctcttgggtgggaaggggaggaactcttacctccctctctgccatgttctcctctcgttgcccatttgtgtactatcctccctgtcccctacctgactgcatgtgccttcaatgcaaaggtcttactgctcatcagctttacatctgcatcacagtcacaattcctgcaccttacaggcctggatcaaattcttgtgaatgagcaaaagcatctctaaaggtcaccagtgccctgcttgtctcaatcctagccggacactaggctataatgctcattataaatgtgaaaataaggaaggagaccacctctcccattgtctcctgtttcaaaaaggaagcagaaagttaaaaagaagcagaagtgaggtcaacagccagacagcttggcaccaaaaaccaggcctggtagttaaacatcaactcctaacctaactgcttgtgttatctgtagatgccagacatcgtatgaggaagcgctgtgaaactttctgttctgttctgctagcccccattactgatgcacgtagccctcaatcccatagcccccgcttgcacaatgtatcacgaccctttcacgtggaccccttagagttgtaagcccttaaaagggacaggaatcttcactttggggagctcagaccttgagatgcgagtctactgatgctcccagctgattaaagcctcttccttccttaaactggtgtccgagaggttttgtctgtgaccagtcctgctacaaaagaagctgtgtgcattttttttgcagtgcataaacagactggcctatgatctgtgcctttccttaagtaatatctatcattacaccaaaaatgaaaataaagcctgtggggattatcacgccttccaaatacctgggctgcctctggaggaaactattgctaaatgcccaaagtgaagaaaataaaaaatgtctggagggtagctccccccaaaatactaagaactcctaaataacataaattatggataaatgaaacatctataatcacaggaaatagcataaaatgctattgcaaacccatgattttggtgtatggatagtgtgttcatgtcacttattaaaaccatgaaacctccgggcctggggaaagggaagccgtgcatcccacttgaccagctcatacctccttccttctgcactcagaatcaactgccctttacctgctttcatgccttgatcactactgtttggttctgagatggtgcttttttctgggtggaaattctgcctgaagggagcagggaatttggtgttctaaatccagaaccagcaaaactcaatgagaggggcctcatcccaatgaacccagcacaaacaaacgtgcaacagtcaggcctattttaaaaagacttctcatctctgaacaaatgataccacattttatgaaactcaattacctgcacagtcctttggagaccctgaggctcctgagccttctccaactatcctaggccatcagattaccctactcacactctttaggaaatctgaagttttagattgcttccatcacctgactgaggtcccaagaaggtggctatatgacaaaaaggatccagcctctgcaactgcctattctcctggcaggcctcacctggtgaggccacaaagcatacgagttaaaagaacacagttcctagggacggtggctttggtcggagttctcatgccgacacataatagctacatggcctgaactggttttctaaaacgggaaaggctcagagctcaagcaagatatgagcagaccccatgaaaggtcaacaaatgctggatatggctagacatgtaaggacacaactcagagccatttccttttctcaggttgtaaaacacattttgaggctggagttggggaggtgtgtagctattttgagattggcaataaaactccataaacaccatttacccatgaaattccctgacatgttataaggaaactcacctgagtaggaggaatcaggataaccccccattcaaaactcagggatgtaaaaatatatcacctgctgcccagacacagaggactgctattgctatttagcacaatgtctgcacatcctgtacttgtatctttctctctctctctctcttccctgtgtaaggaaaggcacacaaaaacagttgaaaaaggaaagtcaaaatggcatttctccattctcactaagcctgacctgtctctcctcctttcattccttcacacaattatgtagagaaaaattttaaaacatttttaaaaaatgagcaaagtggcagctactcaccaatttgtgtcctaggcaatccgttgaaccttgattgtgtggtgacgagtgtgctgctgctatcagcctataagctgacatcaaaatgtctacaaaaacctggccaggccccctctcctgccctccctcttccaccttacccagaatgagtgtcccctcacctgagctgagttgtctaagtccatattcaattgataaggagaaatgacactccaagcagcgtcctgttttccaggcaactttttccaaaagctccttttccagaatt

SEQ ID NO: 19422 - RNA, 650 nt, Homo sapiens
  source 1..650: mol_type = other RNA
ttctccaaaagaaagcactttctgaaactgatcattttgttgagcaaatatgtgaattctgcaatcatcattgccacatgctaatattggtacatcagtatttggcaaaaaagataagcagagagccaaagcaaatccatttccaaagtttaaagtctgaaggcacattacttctggaccctttttagaccagagtcgaacagcagaatctgcagctgcagaaacgatcagtgtacataatgcaggatctgatgtcctcctctggtaaacagcatgcaccgcataaacaggtccttcatggccttgaagatgcactgcttttaaaagctgattatcctctatttcccagtgaatcacttgattatcagatcctccagaaactaattcagtagaaggggagccatcctgtttacaaatccactgtatgcaattgactcgggcggtgtgaccattcaagttggtaacaacaacccttttcagggggtcatagagcaccacggagcaggacgtgccaaaggccagaagtcctctgggcccagagctccagttcaggactccccgcacccggtttgggcagcaaaacacgtgagaagtctccagcacgggtgccaccatgtcgccaactggtcagccgcacaaacaagagacgc

SEQ ID NO: 19423 - RNA, 571 nt, Homo sapiens
  source 1..571: mol_type = other RNA
ttctccaaaagaaagcactttctgaaactgatcattttgttgagcaaatatgtgaattctgcaatcatcattgccacatgctaatattggtacatcagtatttggcaaaaaagataagcagagagccaaagcaaatccatttccaaagtttaaagtctgaaggcacattacttctggaccctttttagaccagagtcgaacagcagaatctgcagctgcagaaacgatcagtgtacataatgcaggatctgatgtcctcctctggtaaacagcatgcaccgcataaacaggtccttcatggccttgaagatgcactgcttttaaaagctgattatcctctatttcccagtgaatcacttgattatcagatcctccagaaactaattcagtagaaggggcagggggtcatagagcaccacggagcaggacgtgccaaaggccagaagtcctctgggcccagagctccagttcaggactccccgcacccggtttgggcagcaaaacacgtgagaagtctccagcacgggtgccaccatgtcgccaactggtcagccgcacaaacaagagacgc

SEQ ID NO: 19424 - RNA, 572 nt, Homo sapiens
  source 1..572: mol_type = other RNA
ttctccaaaagaaagcactttctgaaactgatcattttgttgagcaaatatgtgaattctgcaatcatcattgccacatgctaatattggtacttctggaccctttttagaccagagtcgaacagcagaatctgcagctgcagaaacgatcagtgtacataatgcaggatctgatgtcctcctctggtaaacagcatgcaccgcataaacaggtccttcatggccttgaagatgcactgcttttaaaagctgattatcctctatttcccagtgaatcacttgattatcagatcctccagaaactaattcagtagaaggggagccatcctgtttacaaatccactgtatgcaattgactcgggcggtgtgaccattcaagttggtaacaacaacccttttcagggggtcatagagcaccacggagcaggacgtgccaaaggccagaagtcctctgggcccagagctccagttcaggactccccgcacccggtttgggcagcaaaacacgtgagaagtctccagcacgggtgccaccatgtcgccaactggtcagccgcacaaacaagagacgc

SEQ ID NO: 19425 - RNA, 845 nt, Homo sapiens
  source 1..845: mol_type = other RNA
ttctccaaaagaaagcactttctgaaactgatcattttgttgagcaaatatgtgaattctgcaatcatcattgccacatgctaatattggtattggcctgaatgcagatggaagaaatgaaattctgttatgatgccagaatgtgtgcagcttctccttccacagagccttgcacagaatggaagcgtaacatgaaaccatagagtcgcagctcctgctacagagggcgagagaggctggtggcttccaggccctgcctcgttccacctggccagtcttccaggtaacatcagtatttggcaaaaaagataagcagagagccaaagcaaatccatttccaaagtttaaagtctgaaggcacattacttctggaccctttttagaccagagtcgaacagcagaatctgcagctgcagaaacgatcagtgtacataatgcaggatctgatgtcctcctctggtaaacagcatgcaccgcataaacaggtccttcatggccttgaagatgcactgcttttaaaagctgattatcctctatttcccagtgaatcacttgattatcagatcctccagaaactaattcagtagaaggggagccatcctgtttacaaatccactgtatgcaattgactcgggcggtgtgaccattcaagttggtaacaacaacccttttcagggggtcatagagcaccacggagcaggacgtgccaaaggccagaagtcctctgggcccagagctccagttcaggactccccgcacccggtttgggcagcaaaacacgtgagaagtctccagcacgggtgccaccatgtcgccaactggtcagccgcacaaacaagagacgc

SEQ ID NO: 19426 - RNA, 767 nt, Homo sapiens
  source 1..767: mol_type = other RNA
ttctccaaaagaaagcactttctgaaactgatcattttgttgagcaaatatgtgaattctgcaatcatcattgccacatgctaatattggtattggcctgaatgcagatggaagaaatgaaattctgttatgatgccagaatgtgtgcagcttctccttccacagagccttgcacagaatggaagcgtaacatgaaaccatagagtcgcagctcctgctacagagggcgagagaggctggtggcttccaggccctgcctcgttccacctggccagtcttccaggtaacttctggaccctttttagaccagagtcgaacagcagaatctgcagctgcagaaacgatcagtgtacataatgcaggatctgatgtcctcctctggtaaacagcatgcaccgcataaacaggtccttcatggccttgaagatgcactgcttttaaaagctgattatcctctatttcccagtgaatcacttgattatcagatcctccagaaactaattcagtagaaggggagccatcctgtttacaaatccactgtatgcaattgactcgggcggtgtgaccattcaagttggtaacaacaacccttttcagggggtcatagagcaccacggagcaggacgtgccaaaggccagaagtcctctgggcccagagctccagttcaggactccccgcacccggtttgggcagcaaaacacgtgagaagtctccagcacgggtgccaccatgtcgccaactggtcagccgcacaaacaagagacgc

SEQ ID NO: 19427 - RNA, 14393 nt, Homo sapiens
  source 1..14393: mol_type = other RNA
ttctcgaggaaagaagcactttctatggtcataaatacacaaattagatccactccatggacactcaggaaaaactttttataaaaagtgagttctaatttcagttgtttgaaaataccgtaggacatcagaattaagagaggttgctttccaaataaatgcccttattaagcaaacaaggatactgaagcccaaattgaagtgaccaaataaaatcaagtggtgagtctgtggctagcctggatttagtactagagcttcagttggctgtcgaattattacgtgtgttttcccaccatgtggtacaaggcctctcactgtagtaaaagagtaaatgagaagctgagtagatttttccacaagttgatttttgttcgttagtttgttttgtccaaataatgtctcattttgcactcaaattggtttacttatagcattttcctaaaaggaagatatcattcattcatctattcattcattccacaaacatcttctgagaatcggatacatggcaggcatcttagtgggtgatacaagagcatttataatctagtaatataacccagtgtacagcaacacaagtgtggataaacaaggagcttcctaatacaatcccagcacatgttcctcctactaacctcaaaataagatgtaaaccctgtagctatagtacctggtcttgtctcagctctaccactttcctgcatgccctcaggaaaattactaaatctcactgctgcagtctcctaatatgtataattatagtacttaccttatagagtggctgtaatgattaataattggtaattaattgacataacttgaagatttttcaatcatccagacacataagaagtgttcaataaacagaattattattattacttttgctaccaccaaaaaatgaaaagttttccacagatagcctccaagacaaccaaggtctaaactccatttcctgttattttaatcccttccagttcccctgtctcccctttaattctgacagagcatctaattttaagatacattttaatggctatttctgcaaacagaacatttagcagtttggtgatgaaatcagggcagtttgagatgtcgcacgctaactagttacactgcacaaagcctaacagtttgctttctgtttttaaagaagcgtttcgtttagccatacttgtggcggcacatgtaattgaaaagaggcatatggagaccagcatgcgaagcctaacaaacacttcagagtggcttaaaaactatgctaatcagttttgggaaaccatgttttaatctaaaagaaaaaaaagacaacctcctcaaacctcaggtgatttttaaagaaacggagtcattgttgatattaactaacactggtttatttccctgtgccctggcaaatgtcagaaataaaattgaataatataaaaagaaaggaatgagagcactcgtgacctgtagttttatggagcagaaatgaactcttaatggaggtaagccaggacaccagcacatggtcagagtctgagtgcagactgtctcctccaggacatggagaagcgacacaggctcactcttccctctgcaagaaggcgctgagcattacctgaaaacaaggaaggcatcagatgaacagacctttataacagaatgtgcatctgccaagacaaaaatacacgacaagcttctggtgctggcacgctgacagtatgagcaagctgtcttagtagtgattttgcaaatcatttgagtttaaattctatataggctgtagggcccctggagcatcactttctatatttggcctcctcatttagctatgtttggaataaataggctatggataaaaatcatgccctttaagagttttgcatacacacactagttctgcatatatatcatatgtgaactgagtgattaatgcaagtctatgttctcatgcacacacacatacacacacgcatgcatgcacgcaggctttctaaatgtatttttaagttgttttcctttgtgattttttttcctctctctttttttttaagttcagctctctggcatttagtaacccacaagctgctgtttctttttccaaagaagttcagctcgatggaggggccaagaaaaatgagcccaactgatgattgtaatctcgaaagaaaatatgctttttatcagggaccgcatgttgccaatgccaattaaagtaaaactgggagatttcatcagataccaacctggagagcagacatgacatgccaagtataagaaaggaaaagtatgtttcaggtggaatttcagggatgtctatttgaggtgaaatgtaaaaatatagggtggaaagtgtaacacagattgcagattgagcaattgttaaccatctagagaagaaatagcacaaaagcaatggcatagatttttatttcagctgaggtagatgaacatcgtgactctgccactgactgctggaattatcttcacatctccagggcttagtttcctcatctgtaaatcaggaatcacaaaattctgtttggatttttaaaagtattaataataatgtggattaagagaccagtttcacagtatttatttgataaaagttaagagagagagagagaaattattagtttgtggatagacggatcaagaagatcatgttccttttcaagtgttacgggcaatcatttagacacattcatcctgcaaacactgagtattctgttcattattctagtgtctttcaatggtaggcaaggagtattgcaacggtatggcatcttcttacagttttatttctgacaccaactaataacatattcatgagatcacctgattctaccccatcaacagagattgctttttacatttgctttggaggtacaaaatgttaaaggttaaggaaagcttcacttcaaggttactctgacttagttcattcctaaaatgattacgtcaaccttgaaagagtattgtatgggtaaaatgagagaaccatgcaaaattactgacacccagtatataataaaaatagtttctttctccattcccttaggtgagttgagtgtttttcatattttaagaactagtagaagtttgttagcttttgactgtgtctttgtcttaaaaaattgggtacaagggctgaaattcatgattgaaagactggaaatatttttgtgctttccaaagtgttgaacttgagagagttctttgaacttggtgaaaatgattatttaaaaatttgcagtatgttggacataataattaagatatggaaaccagctattgagcatatattttttcacacatattctttatataaacctaccacattttatttttatgcctcttcaaagtttatagttagtagaaatagatacttacactgtacccatccatcatttatttgagtattgtattatactgatcctgaaattctggaatttggtcatttctttctagaaagattcaccatgcatatttgtgtgaagtaagaaacaagctcttactcaaactcttactcttattctgtgtagatagattcttttaagtcagttaagaagtttcgagtttcaaaagaccaataaccaggtcatacatgtactaatttggcaaaacctgaggcagtgctaaggtcactgaagaagatgggtttgtattaatgtttcattcaactcctcatatttggccccaatcacaataatcatgtatattttgtcaactttcctgggtattctgctctcctatagggagagaatagagttagaagttcaaagaactaaataaagtgcagctgctacaactttggttgaaaagaacatcatttgtttggctcaaaatttctgtgatccttcagggtgtttcattcatcttcccagatagttccagccttctgaaaatgctttaagacattctcaggaaaacaacataaatgtaattcatactgtttatctgaagtagtcacactcaaaaaagctatcttatttccataaatgtagactcaagttgggttcatgcaaagataagattatacctactttttaagcaatctggaccttgctgttatcagttgttgcacagaacacaatgtaatttgttttcatagagtgcatatgtatgtggatttctctatcagttcaatactgttcatctttattgttgccaagttgctatggtttgaatgtgtccaccagagttcatgtgttaaaaacttaatttccaatgattaactttcagtgatattgaaaggagaggcctaacaggaggtgttcaggtcacggggcaccaccttcattagtggattaaagtcattatcacagaagtgggtttcttataaaataatgcattcagtcccttcttattccctcttgctctctctttgcacttctttcatgggatgatgtagcaagaaggtcctcatcagatggcagccccccaagtcttggaattcccagcctccagaatcatgaggcaataaattcctgttcattgtaaattacccagtctgtggtactctgttataaaaacacaactaagacacctgtgttgatggactttgctaacaataatgaagggacattgttaacataattatttattatagaaaaacacaaaagtgatctaaatattcaataaagttaaaataattatgaaacattgtataatattactaatgtctatgtaattaatgttattgaaatttgacttataggtaattgtaaaaaaattttgagggctgcacctcacatctattaaatcagggaaaggactagatagtctgcacttttaagaaatagataaagcaattttggaggattttgtaataaaatgtgagcttaatatgaaggtaagaaccattactgttttgcttgcttctgtaatgttctgtacataacaggcatttaatacattgatgctgaataaatccatggagtattatcctctacagaaaactatgttattttttcaatgattgttgaaagtatataacactaaaaggtaccgttgatataatactcaatgaaaacagagaataaaaattgcatgtattctatggttacaaatgttttaaaacatatttttaaatggataaaaatcacacccaaagaatcatttatatatgataaaaaatgataaatagaacctcaccaaaattaaaatttttctttgcaaaaagacactattaaaggaatgaaaagacaggaccatgctgagagaaaatattttcaaattaatcatccaacaaaggacttgtatcaagaatatgaaaagaactcttaagctcaactgtaggaaaacaaacaatttaaaaatagtcagaagatttgaatttgtattttaccaaagatacttggatggcaaataagcagaagtaaggatgctcaacattttcaattattaagaaaatacaaattaaaactactataaaataccactaatatattaggatagcttaaaaaatgttgacaatatcaagtgctggtgaagaattagattaactagaactctcgtatacatcttgtggggatgcaaaatggtagttgttttagaaacagttttgcaggttcttataaaattaaatatatacttaccacatgactcaacagtccaacttgtaaaaatgaaatcttttatttacacaaaactctatacatgcatgtttatagcaactttagttataatctccaaaaactagaagcaatgcaaatatacttaaactggtgattcataaactgtggtgtatccattcggtggcattctcaaaaataccaaacatatggtatattttgccaatcatttataaatatacatatatgtgtgtgtatgtgtctgtgtgtgtgtgtatgcatgttgatccatgcaaccacatggatgaatcttaactcaaatgcattatgctaagtgatagaatctgtgggcaaattgatacaacttgtttgattccatttatatgacattctatagccatttatatgaaaaaagcaaaactacagggatagtgagtagatcagtagtggctagaggtcaagagtggcagaagggtttgacaacaaaagggcagcatgagtggatttttggagggaaatgaactgttctgtttcttgattgtgccagtggttacatgactacatttgtcaaaacttgaaactatacattaaaaatagtaaatattattattattatattatacaaaataaaaaagtaaatgtaaagaaatgcaaggaactcaaaagtaaaagagtgtcaacgtgttatgtgggtgaacttcttttttaccttcacttcccaattttttttctgtgatataatttaaaatatttatttaagtaacagttaagtaataattatagtaacttctcagtatccataatggatgggttctgggacccccatgggcaccaaaatttacagatgctaaagttcatgatataagatggtgtaatatttgcaaataacctacacacatccctcttgtttactttaaatcatctctaggttacttataatacctaatagaatgtaaatgctatgtaaatagttgttatactgtcttgtttatgaaataatgacaaggaaaaacatctgtacattttccatacagatgcaactttttgtgaatatttttggactacagttggttgaatccatggttgtggaacccacagctacagagggatgactgtatcatatataaaggaaagagttctaccataacactgtgtttaattagcagagtcactggttatttggtcttcctcataaattaacattgcatttgtctttgcaaagttaagtgttacctgcaattggatctatatggctgcaaaccaaccaattaaaaaaatagttaacaaattagatgctttctctataccacatccatctgtttaattgctacatttaataaaatataaactttctctatatgctccttctttacctcaagctatttgcctccctctcttgcctgctaccgctacagctacgttcacacctttgacacttacagtaagacacttccaacctggcaaattcctgcacattgttcaaaatgtggctttgatattttctttcctagaatctgtctgattcatttgcccaatctttcttctaaagatgtcttctctttgcctccttatcagagttcacattaaactcaccatattttattaaaacactccttgcagttgactttattcactacctagattataagttccttaaagcagcttgtctaatacatcttacaccctcaattattagacaaaagcctggtacacggtagctacttgacacatttttattgtccctatatgatacgttttattgcctgtactgaataaacttattattttaagtgtatcctacatatatttttagttttatggccaatacttttcttaggaaattatttttaaaatgaaaagaaaatccctcattgttatatgttaaggtggttggcctatgttttatttgagttggatagattcttagagccacatgccttgcttggttcattcgttcattagaatgggccacgtcctgacagctgagggaaagtacgttgtaataaaccttcaatgatgctcataacctggctgctttctaagattgtgttagttactttattttactgaattgataaagattaaactttcatagaaatgaatagattaaatactatacagataatttgtagggatgatattatgccacttcataggtaatataccaagtcgtatagcctcccaaagtacataagctcataagctcataaaagcaaaaggtgagaaagctgtcatccaatcccattattttatttgtaaaataaacatacccatactttatccagctagttaggagcagaaccatggtcaaaacttttagtgactgaaacatatgtaacttagtaatttgtttgaattttgaaaacagaacactggggagaaatcagaatggattaatgtgcaatatgggctctctgcatttttcaaaaacaaagaataaaaactttaataaagtacagtgatttactaaagtaaatttaagttttctaaagtactgaaggtgaaaagtttgagaaaagataaggtgattcccaatacataaattataccctacaaagatttttatcatagaaactaggtcaatcctattcagaagggcaaagataaagctaatatttgccaggacctgcccaccacaccacccctccatccccgcatagtagacaaagaggagtccggttactagaattttcagtttctgacatatcaacaagacaaagtattcatatataaattttttaaaaatgaccaacttctatctttgagtcttactattccatgacattagttgtcaacaaggatgacttacaagctggttagcagtacatattttccaagacaggtggctaagaaaccgcagcgtgaaccagctccactctgtgctcatcccacagaaacatccactcagtgtgacacttgcatttgacccataagcagagagtttcacctgatacagggtgaccccattacaaataaatacctgtcttttccatcccaagcttccttggttaagtaacacagcttccattaaagacattacaggaggactcaatcacttgtccaaaggggataatgaattgaaaagtacagtggggataaaggtggcatttccatggataacaagagacacatcaggctcatttcaaaagagtagaagtgacaaagccagtccctattgaccaccaattacttctaacaaaaatagcaaccatgcttcacagagagacattctgcatccaactaggtctcacctaagccctactgcatgtcttccaagttccaccatctttgcctcagccccagtgcatgtctcccaagcaccagtgccgttgagtcttctgcccatcagaactcttgcagaagcagtgaatatccaagcttaagtggctcatatccctttgattaaaagattcaaacatatttttctgtcactgtctctttgtgcaagaaatactcttctggctttctttttttacagaaattggattaaacagcatgctttgcaaacaacagataggaatgctaattaaaggacagacctcacaatcacacaaaaagcagctctgcaccaaagtctttttatttcatttcaaatgtgatgcctgtgatttagaaagacggagcttatgtgaactctatttactaaagatagaacaccagcaaatagacttagcaaagaaggtaaagccacaaatttaaacaacaatttccttacatttctattatgattagtaatatttgatcagtatgagtgaaagctaacgtcttgattacagatgccaacaaaagaggtgttagaaaagcctaggttccttctgagaaaggcaaaaatataatgttaaaatgtgatctgactgctgaaatttaaatatactttttattgttactcactgggacaaagaatttgattaaaaagtcttaatttttaaaagcacaaacacaatagaaacattaatatagtacaatccctattatttttcttctaatttggaccacaattattcattcaacatgttgatattgagtgtataaagccctatgttttgtactgagaatacaaaggtgaagaagtcatggtttccactccccaagtatcacactctagggaggatgaatgatgtttgaacagatggttacaaagcaaggtaataaaggcaacaatagttaaatgcacgaagtattctgagtatcttccatagtctaggaaagatgtgagttgctaaggctgcaggggagggaggagcactgatcagggtaaatccttgtaaaggaaaaagaggaggttaactatatttaatatgaacagggcaagaaattgaggcattgtgtcagtgttccaagtaatttgtcattacttgaggatacagaattaaagggcattgcaggagctgatgctaggattgtgcacatcagctagattaggaaggtcccggcacacaatgccaagaaaattaggctctgttctctaggtctggaagctaacagagactctagctgaaagttcatgtgtgcagtgtgaagaatcccaggtatttctgtcatgctctcctggttcagaaccatatattaattccttcaacaaataattgtcatgtgctcaccttaggtcaggcagtgttctgggtaccagggatctgatattgaatagttaaagtcagcctccttgtagagtaattgatggttaacaatttgaagattttaggtgagattttaaaactttctggctgttatgtgaagaatgggaccaagactaggtataggaagacaagttaggaggctcttaaagtaatctgagaggctctaaagattgacagtgataatactggacaaaggagatgaattataaaaatatttaggagtaaagtaaatgggacgtgattattggaggtaagatgaatggagttggaggaggtgaggaaagaaaacgttaagaataaattccaagattttaatttaggttattgagtgaatgttggccccacaaaccaagatagataataaatcaaaagtattcaatctttaccaatgaccataaacaaaaggcatgggaaaaatatatatagcattacatgtaggattagatgtacctacattacatgtagaattaagataaggatggacatacagctgttgatttatggtgtgcaagaaaacaataaaatatttgatgatgtatcaatagaatttcagaaacaggactttttttcacataaaaatgtattatcacattagcagaggatttaatttaaatatttcagaaattccaaaattttgaatatacatcagtcaccacttcatttctgttggtaattgctcatattgacaccagcgtgaactaaccatggctcaggtagaaaacaatgcaactgacactatattttcctctgccaacaactcaggagggaaggaatccacaaattaggttgacacatggtgtctagaaagaattaattcccactcgattctgggcagccttacaagctgggttccatccataaagactgatgggaactctggggtttggtttatatggtgatattttctgttgccatcaacaaccggacataagaatactgatcactgaagaacatttcttttgtttttgctgctatattatatcaagacacttgggaattgttccacacttggaagttgttcttaacctgcattcaatagtttttctgtatttgtcatgttgatatcttctggcaggaacactgagacatttattgtaaaagctttatcaggggacaaaaatattttggatatgccaaatcaaattagagtgcacttgaacagtcatcatccatcttttatccatgattagcattcattatgcagtatcagaaggatttacattagaattaatagacatcatggaaaaaaatatttttaaatgtttcctgctgaaaccaggactacttaaggagcagttattcagcataactgggttaattatgaccgtagtactctcccaaatatttctaacacctattggctggcattcaaattagtgttagacaaaaatggtaaagtaggccacattttatcttttggatccccttgttttcaatttactctcatttattcaaaatttatttattaagtgcccattacacactagacactattccaagcaaaaagtcctaccctcacagagattaccctcgatcctctttcagttcttctaatttccagccctcagtgtgttctttcgctctggttttcctaaaagtataaaattcttacgcttagagtcatgttatgtgtctttgacaaaaacatagaagtgattctgtattcttattgcaccctacttggtggtgcacagtgtcaatttgtcctattactgagaatgttcattttagtcaagtgattaatgatgtgtctgctaggtatccttactgtaaatatagctttatttttctttttaattaatacatattttctggggtggcactttgaaattttatacatttattgttcttcatcaaaattttaatgtattcagctatctgtttttatacatatgtgcttgtggattccaattttatcttacgctttgtaatctatatgaccattctttaattttatgataaaattttcctggtttggccagtgggagccctttcaagtggacttctgagtctttttggcatgtgtccataattttagcagaaccacaattactccagcctcatcttttactttcttggcctcagccctaggaatcaaccatttctccaagaacatcttttcttttgagtagcaaatggaattaagaaaccaatatttgggtgctagctgctattgggttatctcttctcacagatcctcccataatatatatggatattttcatctgtattgatttctatatgtatcaaaatacattgaaaaccatgagatctcatcaataattcaacatccaatccaacaccacagagaaggaaaggaaggaaaatagaaagaaaggaaagggaataggtagggtaaagaaggagagtgaaaggaagggaagagaagggggaaaaaaaggaaaggggaagagaagaaaaaggaaaggagaagtggaattcaatgaagtttagaatatccttttagaaaagcttagaggaaaagcaggaattcacattcacaaccataaatgaaggcacagagaaagtttttgaaagagaaatgagtgagaagggtagaagttttactgattcttttttttttttcagatagcagatactctgagctttttagagctgttaacaatgatcatgtctctatgacatggttgatctggatggaagacaactaatatggtacttttgccttttgaaaatgtatgtggttgttgttagatcaccaaaataatactggaggaataattgtttttcagtaacagtaatctttccctctccagttttgtttttggctctattatagcatttgaatcaaattatgaacacgtactaatgccttgtatgttataggctagaaattggggatacaaacatgagtaaaaactatattcaagaagtttacagatgaatagagaagagacataacagtaaatagaccactgtgatttaactgtaattggatgttagctgttctgacagagtacttcccatgtgtaaagtagtgtgctttaaacttccctggcacattggtcccagtttatgtgcatccccagatccataccactctgcctgttccccacctcagtaatgtccattgcttcttggtcagaggggacctctcaaaatctcgcttcattcacgtggccataaaatcctgcctgctgccctgccataggcccggtagccctcacttgtcgtgccaactggtaaaaggagaccattctacccttgtggtggtcagactaaacccacagaggttacagcttccccattagttgctagacaaaataacttaacctttacttgtgggggagtaagtgacttgaccgatggaagacaggagtgtagaaggagccacagaaaaattgctcatctatcttgtcctgactcagtgatttatgacagatcagttttccctcacatgactgaacaactggctttgttgtattgcaacactgtgcttacttctgtaacgcgccaccttgtgaatatgttctctccttacctgcctcgttcctcttttcttcttcatttgacttcacccttgcctctctaggattttactctgggaggatccagctctccaggatgatggtaagatgtccttgacttcaaagtagagcacctggagaataagttccacctctgtcctgtcctgggctcatgattttttggtgccccttcaagtagcacagaaaccaatcccactggcatcttgatcttggactttctgcatccagcacctttgatgtgtctccaccagcttgcagaataaaatccagaattcttagtccagtagtcagccctatgccatttcatccaaactcctctttttgtcttgagtaacctatgctggatgctgtgagaaactactgcttgctgtagaaaagagagatcttcctttttgttcattcatttcctccttcactagtcaactgctgtttctgaccatgccaaggtggaaccctttttctgttcctcttcttcagtctggaacacaggagctggaagcctggaagggcaacagccatctggtgaccacgatacaatcacaaagtgaagtcccacgataggccatctacaaactgaggagcaaggaagccagtccgagtcccaaacctcaagagcagggaagccaactgtgcagccttcagtctatggccaaaggcccgagagcccctggcaaactact

SEQ ID NO: 19428 - RNA, 3322 nt, Homo sapiens
  source 1..3322: mol_type = other RNA
ttctcgaggaaagaagcactttctgctatcaaaacttgatcatttcccatgagaaaaaatgctcaagaaagttggatggcagcttggcacacttaagagaaagctcactcacaactaaagaacaactgcattctgctacagtaatctgggatgggtatgacagcaccagcataacactggctggagtgtggcaaggagagggagttggcaatctactgatgctggggacattggataccgatttttttctactgttttccagatctttgagttcattctcgatttttgtgattaattccctgagttcatcaagattagtgcaaataagctgaaactctggtacagtaggtgactttatgacagttttcctcttctttgtgattgcttttttagagacggatttttttccagatttgtgcttcttgtgttttgctttttttttgatgatcaataacttattctggatctcaggtttgtaagacttgaatgcaagagaatgaagaccttcacgctttctctgtaagttttcattcaaaacatctttcaatttcttttttttctttttcttcttttttgccctcattttagttagtttgagtttcttgtggctctgtagtgactgctctaatagaatatcccttacaactttgtggcagttaatttctggatgatcactgtgacttccatttacatgtatttggcaagattttagagtattttcttttaatggactgggttcaatctttattctggaagcttcaccgtatttttcctgattttctataaaccttatttcacctggactaagaggctctccaaagccagtaacttcccctggactccttggtttctctaaattttctttacaacaatcagtttttttaatttcacaaggcctgcgaattctaatttcatagttggattttactcccatttcaacagagatgtcatgattatccaagatcattttagcaggacagcaagctggatcaaaattattttcctgctctttcttgaaggaagagggcaggctatctctgctacatctatgttctccattacttgtactaacatagtcacacttcaatttctccaatttaatccgaggtactctttgtattttaatgggtggaattggaaattctggggcctgaaagggtctctgtttataaatccgtacatctgcaccacagaactgtggaaaatgtacataagcattctccaaataatcataaccaagaataacttccctgcattcatggataggctgtccaagtacagcatcttgaacttccttttgtgtttcatacacaaagtcacaaagacccttaagtagccacactttttggtaaaaaggtagttcgtgaaaaggtttttcttccaatggattaacttctccaagaactttaaaaaactgaggacacaaccccagtttttcagcacagttatcaggattttcagtttgccctacagcagtgtaccactgttgtactttctgcctcagcgctgcttcccaggtcctataaggcaaagtaggtcttcgatgtaaggtaggtctgcgatggggaggacttaatagagaagtcattattttcgatagaaaagcattacactgaggcatcagaagacaacgttccaattcgtaaaagactatttctggcaaatttagaatttgctgagctaaacaaaggaaatgcccaatagctggaatttcccacatggtctccatacaagttggagctgcttgagctagaagttttctttcccattcttctatttccttttgactagcttcttctgcttcttttctttcctgctcccgaagccttttttcttcttttgctctcagctgttcttcctgtctcaaaacttgaaccattatagattcaaaaactccacttgtcaagcctgccaaacttcgcggtgttgaccgacgccttgttgaggtacatgcagttcccttctcatcctccaatccataatagcctctagatgtaactgctatcgttgtcttttctctcaagtgccgagagagaagcgctaacttctgctccagcatcatctccagcttctggccctgtttggagatccagtggtccactccgtgcaggcggtagcacgtctccagcatcaacctgaagtccgccacgaactcggtgatgcccccgtactggccgctggcgaacttctcttccatctgcagcagacacatgccctgtccgggctgctgcgggaaggcgcgaccgccccggcccccgctgcgcggcccttccgccacctcctcctccgcggtggcaacgccccccaagggctgcagaaagggggcggtgaggccccggtgcttctcctgcaggaactcgcccaggatgcggtagccctgctgtagctcgtaggtcagctcctgctccttgcagcaaccgcctccgatcaccatcgcctccatctcttcctcctgatcgtccgcgtcctccagcgaggaggcactccttccgtgggccggccctgaggtctgggccgccgctgccacctcctcctcgtcgtcctctccttcggccgccggtggcggccgctcttcctccccagccggctccatcgctcccggcgtcccgggcacactcatgccccggcaggcctaggctgggcggtgtggaacagccgctcgaggtgctgggggacgcgtgagcgcgagccgcttcctcacggctcggccgcggcgcgtagcccccgccacatcgggcctggctctcctcagccgccggctcggctcggtgcgcgcgggggtcttgagctcaccgccggcggggcggggttacatggcgcgcgaggaggggggagagaagaggagagcctaggtgccctcctctcccctcccccccggcggcggcgcgcgcacggccctcgccggcctcacccctccgcaccccgcccgcctgctcttcaccggccaggccctgccgggtcgccgcggcctcggcgccccaccccctcccgggccagcggggggctgggagggggcgaggaggaagggggttctcctctcccctccccggagggggccgcagcggcggctccggctcctcctctccctcacaccccctcccgcccccctctacctgcgggggacacgggcagaaggaggcggtgcacggacggggcccggcgacaactgtcagttagaagccccgctgggcggtgaggggggagaaaggggaggggcagggagagaagggggagggcactcagccccccggctgggaagagctgtggagagaagcaaagaaagaggccctgtcgccatccccggtgcgcatgcgtagtagaa

SEQ ID NO: 19429 - RNA, 3494 nt, Homo sapiens
  source 1..3494: mol_type = other RNA
ttctcgaggaaagaagcactttctgctatcaaaacttgatcatttcccatgagaaaaaatgctcaagaaagttggatggcagcttggcacacttaagagaaagctcactgaatcaaagtgatctttctccaggatatccagaggttctgttgagtctatagacttactgatttctcccttaggagagtcttttccaagatctccttcaccttcatcagtggtccatagttctctattaaatgtatcatgatcaggttgtcttctgaaatcatcatagtctttcttcaggcggctcctgtttctttggaaagccttcattaactttggttcccatggcagcaattcatttaaaagacgtatcaatgtactatgtaattcttttacagcttgcctccgatgataccattttcccgatttttttctactgttttccagatctttgagttcattctcgatttttgtgattaattccctgagttcatcaagattagtgcaaataagctgaaactctggtacagtaggtgactttatgacagttttcctcttctttgtgattgcttttttagagacggatttttttccagatttgtgcttcttgtgttttgctttttttttgatgatcaataacttattctggatctcaggtttgtaagacttgaatgcaagagaatgaagaccttcacgctttctctgtaagttttcattcaaaacatctttcaatttcttttttttctttttcttcttttttgccctcattttagttagtttgagtttcttgtggctctgtagtgactgctctaatagaatatcccttacaactttgtggcagttaatttctggatgatcactgtgacttccatttacatgtatttggcaagattttagagtattttcttttaatggactgggttcaatctttattctggaagcttcaccgtatttttcctgattttctataaaccttatttcacctggactaagaggctctccaaagccagtaacttcccctggactccttggtttctctaaattttctttacaacaatcagtttttttaatttcacaaggcctgcgaattctaatttcatagttggattttactcccatttcaacagagatgtcatgattatccaagatcattttagcaggacagcaagctggatcaaaattattttcctgctctttcttgaaggaagagggcaggctatctctgctacatctatgttctccattacttgtactaacatagtcacacttcaatttctccaatttaatccgaggtactctttgtattttaatgggtggaattggaaattctggggcctgaaagggtctctgtttataaatccgtacatctgcaccacagaactgtggaaaatgtacataagcattctccaaataatcataaccaagaataacttccctgcattcatggataggctgtccaagtacagcatcttgaacttccttttgtgtttcatacacaaagtcacaaagacccttaagtagccacactttttggtaaaaaggtagttcgtgaaaaggtttttcttccaatggattaacttctccaagaactttaaaaaactgaggacacaaccccagtttttcagcacagttatcaggattttcagtttgccctacagcagtgtaccactgttgtactttctgcctcagcgctgcttcccaggtcctataaggcaaagtaggtcttcgatgtaaggtaggtctgcgatggggaggacttaatagagaagtcattattttcgatagaaaagcattacactgaggcatcagaagacaacgttccaattcgtaaaagactatttctggcaaatttagaatttgctgagctaaacaaaggaaatgcccaatagctggaatttcccacatggtctccatacaagttggagctgcttgagctagaagttttctttcccattcttctatttccttttgactagcttcttctgcttcttttctttcctgctcccgaagccttttttcttcttttgctctcagctgttcttcctgtctcaaaacttgaaccattatagattcaaaaactccacttgtcaagcctgccaaacttcgcggtgttgaccgacgccttgttgaggtacatgcagttcccttctcatcctccaatccataatagcctctagatgtaactgctatcgttgtcttttctctcaagtgccgagagagaagcgctaacttctgctccagcatcatctccagcttctggccctgtttggagatccagtggtccactccgtgcaggcggtagcacgtctccagcatcaacctgaagtccgccacgaactcggtgatgcccccgtactggccgctggcgaacttctcttccatctgcagcagacacatgccctgtccgggctgctgcgggaaggcgcgaccgccccggcccccgctgcgcggcccttccgccacctcctcctccgcggtggcaacgccccccaagggctgcagaaagggggcggtgaggccccggtgcttctcctgcaggaactcgcccaggatgcggtagccctgctgtagctcgtaggtcagctcctgctccttgcagcaaccgcctccgatcaccatcgcctccatctcttcctcctgatcgtccgcgtcctccagcgaggaggcactccttccgtgggccggccctgaggtctgggccgccgctgccacctcctcctcgtcgtcctctccttcggccgccggtggcggccgctcttcctccccagccggctccatcgctcccggcgtcccgggcacactcatgccccggcaggcctaggctgggcggtgtggaacagccgctcgaggtgctgggggacgcgtgagcgcgagccgcttcctcacggctcggccgcggcgcgtagcccccgccacatcgggcctggctctcctcagccgccggctcggctcggtgcgcgcgggggtcttgagctcaccgccggcggggcggggttacatggcgcgcgaggaggggggagagaagaggagagcctaggtgccctcctctcccctcccccccggcggcggcgcgcgcacggccctcgccggcctcacccctccgcaccccgcccgcctgctcttcaccggccaggccctgccgggtcgccgcggcctcggcgccccaccccctcccgggccagcggggggctgggagggggcgaggaggaagggggttctcctctcccctccccggagggggccgcagcggcggctccggctcctcctctccctcacaccccctcccgcccccctctacctgcgggggacacgggcagaaggaggcggtgcacggacggggcccggcgacaactgtcagttagaagccccgctgggcggtgaggggggagaaaggggaggggcagggagagaagggggagggcactcagccccccggctgggaagagctgtggagagaagcaaagaaagaggccctgtcgccatccccggtgcgcatgcgtagtaga

SEQ ID NO: 19430 - RNA, 6260 nt, Homo sapiens
  source 1..6260: mol_type = other RNA
ttctcgaggaaagaagcactttctgctatcaaaacttgatcatttcccatgagaaaaaatgctcaagaaagttggatggcagcttggcacacttaagagaaagctcactggacttgttgaaagggacgacaattcagtttgaggtttatttgtgtttacatttgttggcactgtagttgaaatccctggtgaatggaactggagtgaagtccgagattgtcttttagaaatagatacagaacgtgtggctcctggtactgctgccgaatgtggaactgtgtttattattttaggggatgtagtcgcaggtgtaggtaaggcaaccgtaacaggaatttgcaaagctgatgttaaacatttaggagacactactggttgtgtagttgaaatcagaacagatgatgcaaggtgtcctgttttcacagttgatatagccacagtgtttccgagacttgatgagcaaagtctatttgacaaaataggcataattcttgaagaggtatcatttccactgactaaaacaggaggttgtgccccagctgaagcagaggctgaggtcactggaaaggaacccaaagataaatttgctccggtaactgaaagcacatttactgctcttgctgaagaaaccactgattcattaacaggggtaatattctgactcacaaaatttgagcttactggaactgaattaccacttgttgacaatggcaaaatatagcccttgctacttttgtcttctccttttggggttacattttgtaatatgttaattgatggtatagctggcacagtgcctgaagtatttacaattgcttgacctatgtttagtccaattttcacatcctttatctgagacacagctggtgatgaatttatttttattggtgtgcccactgtagacggaatcagtactatttggggttgctctggagtcttaacatatgctttatgcaatggaggaggaagagtttgttttaatgattctgcaacaagagttggggttgatgtaccactaggaactggggcattaataaaaactaatttctgggcagaaacacctgtagatgtcagcgcaggtgtcatattaattgcagttccattgccagaagaaagaatagatggagctgataccagcataagtttctgaactggagtcccactgattacatctccatttgttgctgctgttgcttctgaccttgtaacagggtaactttttgtgatataatctacttgttgctgtttagttggagtatgaataatatttgcattgttttgtccaaaatttgctgctgatatgctaattacacttaccgaactacttgttgttgatggtagtagagtactagaacaaatagaggacttcaagggagaagagggcatgtgtgaagttttatctatcacgtggcccaaatcaccactgccagtggtgtggcctaatgtaagtttgagatttttccccatggatggggcaaagctagctggaatggaaacagaagttggtgtttggctaaaaggtgaaagactagatgtagtagttgttccagctacaggtgaaaaagcagaggaagaagttgttgattttggcaccagaaatgcctgcagctgaggagcaaaagtgaaaactgaacttgaagatacagtattgggtgaattttgatctgggttggtctgtacttttacaactccagtgttcccacctcgtgtcctaacaagaattgactgtgaatctcttatgcacacagttttcagctcttgctttgcttcagaagaatcagcagtctgttgtgcaaaacagttgaaggaactaccaggatttgtagacccatttagtgttgttgttgatgacagaggctgacctgtggaggaaatggtcggtgaagcactgggcaaggagaatgtggctgctgaaactgcattcttggcttttcctgcctcactctggctagtcttaactgatggtgttaataagttacttacagaggttacaggcgacaaaggctgtggtctagcactacttatatttgataaaggtgtaattgttttgttgaaagctgtatttggtagttgggtagaaacagttcctggtgagttgacaaaaactgatgctaaagaagaatttatatttgttgtctgtgggaaagatgaacaatgttgttctgtacctttctgttgaagtggtggcacttcttttgcaactgcttttccttctttatgctgaatcacaaaattcttaggcagaataagaacttgctgcatgattttttctcctgttttaggatccaccataggctgcacctgaatctttacagagctattttgaagatctattggcaaccactggccacagggcattttgtataccatttgtaaaggaccttttgtattggtgtggcaggtcaatgctggctttatcgggcttgcttccggaggagataaaactggtttttccacagcaagagcatttctacctgtggaaggaggcagttgatttgttaaggtcactttattcccaatattctttgcaagcaaagcctgaatgggtttggtccctttctggagagtagacactggtactgaatccaatgaggcaaatgactctggaaatgatggctctgtatgctttgattcactgaaacagtcaatctgcacatcactttctagattctcaactgttgtctcatttgtgcttaactttgccttcttccttggagaaagctcttttgtgctgtcatccacataatcagtttgtttggactgtcgtttaagtgttttaagcagtgtcttcggtaagtcttttgaaggcaattcctttttcaacagcttgcttctagccataggaaaatctatttctgacaacttcatatcatctgaatcaaagtgatctttctccaggatatccagaggttctgttgagtctatagacttactgatttctcccttaggagagtcttttccaagatctccttcaccttcatcagtggtccatagttctctattaaatgtatcatgatcaggttgtcttctgaaatcatcatagtctttcttcaggcggctcctgtttctttggaaagccttcattaactttggttcccatggcagcaattcatttaaaagacgtatcaatgtactatgtaattcttttacagcttgcctccgatgataccattttcccgatttttttctactgttttccagatctttgagttcattctcgatttttgtgattaattccctgagttcatcaagattagtgcaaataagctgaaactctggtacagtaggtgactttatgacagttttcctcttctttgtgattgcttttttagagacggatttttttccagatttgtgcttcttgtgttttgctttttttttgatgatcaataacttattctggatctcaggtttgtaagacttgaatgcaagagaatgaagaccttcacgctttctctgtaagttttcattcaaaacatctttcaatttcttttttttctttttcttcttttttgccctcattttagttagtttgagtttcttgtggctctgtagtgactgctctaatagaatatcccttacaactttgtggcagttaatttctggatgatcactgtgacttccatttacatgtatttggcaagattttagagtattttcttttaatggactgggttcaatctttattctggaagcttcaccgtatttttcctgattttctataaaccttatttcacctggactaagaggctctccaaagccagtaacttcccctggactccttggtttctctaaattttctttacaacaatcagtttttttaatttcacaaggcctgcgaattctaatttcatagttggattttactcccatttcaacagagatgtcatgattatccaagatcattttagcaggacagcaagctggatcaaaattattttcctgctctttcttgaaggaagagggcaggctatctctgctacatctatgttctccattacttgtactaacatagtcacacttcaatttctccaatttaatccgaggtactctttgtattttaatgggtggaattggaaattctggggcctgaaagggtctctgtttataaatccgtacatctgcaccacagaactgtggaaaatgtacataagcattctccaaataatcataaccaagaataacttccctgcattcatggataggctgtccaagtacagcatcttgaacttccttttgtgtttcatacacaaagtcacaaagacccttaagtagccacactttttggtaaaaaggtagttcgtgaaaaggtttttcttccaatggattaacttctccaagaactttaaaaaactgaggacacaaccccagtttttcagcacagttatcaggattttcagtttgccctacagcagtgtaccactgttgtactttctgcctcagcgctgcttcccaggtcctataaggcaaagtaggtcttcgatgtaaggtaggtctgcgatggggaggacttaatagagaagtcattattttcgatagaaaagcattacactgaggcatcagaagacaacgttccaattcgtaaaagactatttctggcaaatttagaatttgctgagctaaacaaaggaaatgcccaatagctggaatttcccacatggtctccatacaagttggagctgcttgagctagaagttttctttcccattcttctatttccttttgactagcttcttctgcttcttttctttcctgctcccgaagccttttttcttcttttgctctcagctgttcttcctgtctcaaaacttgaaccattatagattcaaaaactccacttgtcaagcctgccaaacttcgcggtgttgaccgacgccttgttgaggtacatgcagttcccttctcatcctccaatccataatagcctctagatgtaactgctatcgttgtcttttctctcaagtgccgagagagaagcgctaacttctgctccagcatcatctccagcttctggccctgtttggagatccagtggtccactccgtgcaggcggtagcacgtctccagcatcaacctgaagtccgccacgaactcggtgatgcccccgtactggccgctggcgaacttctcttccatctgcagcagacacatgccctgtccgggctgctgcgggaaggcgcgaccgccccggcccccgctgcgcggcccttccgccacctcctcctccgcggtggcaacgccccccaagggctgcagaaagggggcggtgaggccccggtgcttctcctgcaggaactcgcccaggatgcggtagccctgctgtagctcgtaggtcagctcctgctccttgcagcaaccgcctccgatcaccatcgcctccatctcttcctcctgatcgtccgcgtcctccagcgaggaggcactccttccgtgggccggccctgaggtctgggccgccgctgccacctcctcctcgtcgtcctctccttcggccgccggtggcggccgctcttcctccccagccggctccatcgctcccggcgtcccgggcacactcatgccccggcaggcctaggctgggcggtgtggaacagccgctcgaggtgctgggggacgcgtgagcgcgagccgcttcctcacggctcggccgcggcgcgtagcccccgccacatcgggcctggctctcctcagccgccggctcggctcggtgcgcgcgggggtcttgagctcaccgccggcggggcggggttacatggcgcgcgaggaggggggagagaagaggagagcctaggtgccctcctctcccctcccccccggcggcggcgcgcgcacggccctcgccggcctcacccctccgcaccccgcccgcctgctcttcaccggccaggccctgccgggtcgccgcggcctcggcgccccaccccctcccgggccagcggggggctgggagggggcgaggaggaagggggttctcctctcccctccccggagggggccgcagcggcggctccggctcctcctctccctcacaccccctcccgcccccctctacctgcgggggacacgggcagaaggaggcggtgcacggacggggcccggcgacaactgtcagttagaagccccgctgggcggtgaggggggagaaaggggaggggcagggagagaagggggagggcactcagccccccggctgggaagagctgtggagagaagcaaagaaagaggccctgtcgccatccccggtgcgcatgcgtagtaga

SEQ ID NO: 19431 - RNA, 4199 nt, Homo sapiens
  source 1..4199: mol_type = other RNA
ttctcgaggaaagaagcactttctgctatcaaaacttgatcatttcccatgagaaaaaatgctcaagaaagttggatggcagcttggcacacttaagagaaagctcactttctgttgaagtggtggcacttcttttgcaactgcttttccttctttatgctgaatcacaaaattcttaggcagaataagaacttgctgcatgattttttctcctgttttaggatccaccataggctgcacctgaatctttacagagctattttgaagatctattggcaaccactggccacagggcattttgtataccatttgtaaaggaccttttgtattggtgtggcaggtcaatgctggctttatcgggcttgcttccggaggagataaaactggtttttccacagcaagagcatttctacctgtggaaggaggcagttgatttgttaaggtcactttattcccaatattctttgcaagcaaagcctgaatgggtttggtccctttctggagagtagacactggtactgaatccaatgaggcaaatgactctggaaatgatggctctgtatgctttgattcactgaaacagtcaatctgcacatcactttctagattctcaactgttgtctcatttgtgcttaactttgccttcttccttggagaaagctcttttgtgctgtcatccacataatcagtttgtttggactgtcgtttaagtgttttaagcagtgtcttcggtaagtcttttgaaggcaattcctttttcaacagcttgcttctagccataggaaaatctatttctgacaacttcatatcatctgaatcaaagtgatctttctccaggatatccagaggttctgttgagtctatagacttactgatttctcccttaggagagtcttttccaagatctccttcaccttcatcagtggtccatagttctctattaaatgtatcatgatcaggttgtcttctgaaatcatcatagtctttcttcaggcggctcctgtttctttggaaagccttcattaactttggttcccatggcagcaattcatttaaaagacgtatcaatgtactatgtaattcttttacagcttgcctccgatgataccattttcccgatttttttctactgttttccagatctttgagttcattctcgatttttgtgattaattccctgagttcatcaagattagtgcaaataagctgaaactctggtacagtaggtgactttatgacagttttcctcttctttgtgattgcttttttagagacggatttttttccagatttgtgcttcttgtgttttgctttttttttgatgatcaataacttattctggatctcaggtttgtaagacttgaatgcaagagaatgaagaccttcacgctttctctgtaagttttcattcaaaacatctttcaatttcttttttttctttttcttcttttttgccctcattttagttagtttgagtttcttgtggctctgtagtgactgctctaatagaatatcccttacaactttgtggcagttaatttctggatgatcactgtgacttccatttacatgtatttggcaagattttagagtattttcttttaatggactgggttcaatctttattctggaagcttcaccgtatttttcctgattttctataaaccttatttcacctggactaagaggctctccaaagccagtaacttcccctggactccttggtttctctaaattttctttacaacaatcagtttttttaatttcacaaggcctgcgaattctaatttcatagttggattttactcccatttcaacagagatgtcatgattatccaagatcattttagcaggacagcaagctggatcaaaattattttcctgctctttcttgaaggaagagggcaggctatctctgctacatctatgttctccattacttgtactaacatagtcacacttcaatttctccaatttaatccgaggtactctttgtattttaatgggtggaattggaaattctggggcctgaaagggtctctgtttataaatccgtacatctgcaccacagaactgtggaaaatgtacataagcattctccaaataatcataaccaagaataacttccctgcattcatggataggctgtccaagtacagcatcttgaacttccttttgtgtttcatacacaaagtcacaaagacccttaagtagccacactttttggtaaaaaggtagttcgtgaaaaggtttttcttccaatggattaacttctccaagaactttaaaaaactgaggacacaaccccagtttttcagcacagttatcaggattttcagtttgccctacagcagtgtaccactgttgtactttctgcctcagcgctgcttcccaggtcctataaggcaaagtaggtcttcgatgtaaggtaggtctgcgatggggaggacttaatagagaagtcattattttcgatagaaaagcattacactgaggcatcagaagacaacgttccaattcgtaaaagactatttctggcaaatttagaatttgctgagctaaacaaaggaaatgcccaatagctggaatttcccacatggtctccatacaagttggagctgcttgagctagaagttttctttcccattcttctatttccttttgactagcttcttctgcttcttttctttcctgctcccgaagccttttttcttcttttgctctcagctgttcttcctgtctcaaaacttgaaccattatagattcaaaaactccacttgtcaagcctgccaaacttcgcggtgttgaccgacgccttgttgaggtacatgcagttcccttctcatcctccaatccataatagcctctagatgtaactgctatcgttgtcttttctctcaagtgccgagagagaagcgctaacttctgctccagcatcatctccagcttctggccctgtttggagatccagtggtccactccgtgcaggcggtagcacgtctccagcatcaacctgaagtccgccacgaactcggtgatgcccccgtactggccgctggcgaacttctcttccatctgcagcagacacatgccctgtccgggctgctgcgggaaggcgcgaccgccccggcccccgctgcgcggcccttccgccacctcctcctccgcggtggcaacgccccccaagggctgcagaaagggggcggtgaggccccggtgcttctcctgcaggaactcgcccaggatgcggtagccctgctgtagctcgtaggtcagctcctgctccttgcagcaaccgcctccgatcaccatcgcctccatctcttcctcctgatcgtccgcgtcctccagcgaggaggcactccttccgtgggccggccctgaggtctgggccgccgctgccacctcctcctcgtcgtcctctccttcggccgccggtggcggccgctcttcctccccagccggctccatcgctcccggcgtcccgggcacactcatgccccggcaggcctaggctgggcggtgtggaacagccgctcgaggtgctgggggacgcgtgagcgcgagccgcttcctcacggctcggccgcggcgcgtagcccccgccacatcgggcctggctctcctcagccgccggctcggctcggtgcgcgcgggggtcttgagctcaccgccggcggggcggggttacatggcgcgcgaggaggggggagagaagaggagagcctaggtgccctcctctcccctcccccccggcggcggcgcgcgcacggccctcgccggcctcacccctccgcaccccgcccgcctgctcttcaccggccaggccctgccgggtcgccgcggcctcggcgccccaccccctcccgggccagcggggggctgggagggggcgaggaggaagggggttctcctctcccctccccggagggggccgcagcggcggctccggctcctcctctccctcacaccccctcccgcccccctctacctgcgggggacacgggcagaaggaggcggtgcacggacggggcccggcgacaactgtcagttagaagccccgctgggcggtgaggggggagaaaggggaggggcagggagagaagggggagggcactcagccccccggctgggaagagctgtggagagaagcaaagaaagaggccctgtcgccatccccggtgcgcatgcgtagtaga

SEQ ID NO: 19432 - RNA, 4451 nt, Homo sapiens
  source 1..4451: mol_type = other RNA
ttctctttctttagccttgtgttatttatgtgtaaagttggattatggaaggcaaagaatctctcgtgtgtcattcacgctcaagtaaatggcagtggggtagggatgtaaatgaaactgcgtgataagccctgcaagtcattctgatgtatcaattttgcttactggtgtttaattgcagacattgtcatattaatgcaaccactaatacattatggagtaagatgcaaaaatcacatgagtcttaagagaaaagaaatgtgctttctatggtgggccccttttgtattattctctaacttcttattttatacctctactattagagaaatttcagtagaaaatcgtgaggggcaccgttttagagtttttgttgttataggtatgcttttactacagctaggtccccttgtacatctttatgttctttggcagtctagagaaccagaagagcaaactctatgagatagaaactctaagaatttatttacctccagcatcccttctcttctttcattaaattgaatttgtggccaactcaaagactgacaatttatactatggtttttatgtttttatattataatttatattacggcttatgtcaaaatgttttgttcactgctttgaaagtatcttttgtttacttttgttatttcatattttaattttttcctttctaattgttagaaactcatgtattttatctttcaaagaaaattttttaaaaggcttactctgcttatatgtatattttgcacaaagctttccattcataaacaaaaggtgaataggaatcagaattgaaaactacgtaatttcttttctccttttgagtcaaatcatcacagtatagattagtcattgtgtatgaagtgcattgccaatacatagtcacatttgtgtagaaatgtaaaggctatatctcaatacaaatcaaaaaccaaaaaatgcagaagaccattagctaataatactaataatctagtatagaaagcatgtgccaactgatctagactcttgtgacagttgtatatctacccagctgcatgacctgaggtgtatcaaaatcttgatttcctagactacaaatgagtaaaagggatggaggccccttacagttttaagattctagaattctaagtgtgtgtaactagagcaaattttattttctaaaatttgcataataaatttaaaaataggagaaaaacaaataattaaagtacatatttctagaaatcttttttaggtgacttatactaccaggaatggatttaccactaaatattggttttgcctaattcagcattgctatgtaatttgatggaagtataactccatagacaaagagatttggtcctaacatagcttgtattttatatgtatatacactatttctatttaaatttctgtgtagtcatgttttacccttttaaaatgaagattagttttattatgtattttcttttgtctataaacattcaatgaattcacactgaaaactgattatgaacagatagtctgctaggcactaaggaaacacatacgaaaaactaagtcctcctctgccctcaatatgctcacaagactacagttactgaagcctgacctcaaaacctagctagcaaagtccttgaatcaggtgatagttcagaataccattcgtgctctctcccaagagtatatctgaggaagggcagttctttctagttttctacatcctggtcgtataggtcaaccacaggaaaattaaatgaatctattgttttggtgacctagccttttcatataactctcatctataaatgtattaccaaatactatttatgtaaagggacttgtatgacaaatattttgaaattaaaaccacaatggttagcatagcttttaaattagatagatgttgacctcccattggtaaacatataaagtgctaccaagatctgccaatgacagactttggaagtggaaattcatctttgtaataatcctgttatctgtaggctgacctcaaaccttcataacattcagggccccttattcctaactgtatcttctattttgggcattgtgctcttgccatctaacaggaaaacaactttcagtgctgccaccttttgaacaggagagatttctagagattagaaaattactaaatttaaatatacatagttttaaaatatgatacttttctacccatgcattcaaatatattctaactttaaaatcctgtaaatacttatatttgtaatgattttacttatatgatccaattaattggcaagaatatgtggtgaaagattttttacatgtttgtattgttctgtgtgagacatctattgtaagcattgcttcaggccctcatttttgtctgccttccaggatttgctggcccaagtgctgtgtgctagcttagtgtcagtcacaaaggggagggaaacttgcagttgagccagacagttttgttattcctttaaaattaaaagcatatgaaacagatacagcttattaaggttttttttataaataacataaacttaaataacaaaacaataagttcaaaaacaacttaatatagagtttaatgcagtaaccataggaaaaaagcgtgattatttgtgggaagaacattattaaaagccatattcccaaatatgaattatacaaagatagattatgttacttgaaaaaaacttaaagatttctcaattttactttgaggaattataaaatgttatttagtggcaagtaagatgaagtacagtattatcatcaatcactgttgctatcttatatacaagatttttggaaacatccttttagcaataccctttccacttgagcagcattagaaattttgttcttgttaataggtataagcatgttctaatcctgtacttttgttaaattatctattttattgactttcataatagatttttttgagaatattctttttttctgattagagtttaagtagattataatttttcactagaaagcatttaaaatgctgctcattttccatagttagtgtggcttgattatctgacaaatcctgccagcagcctgtaggtctgatataccttatataacatcatctgcattattattattatagcagccattttataagcagataggaatatttaaataatcattatcagataatcaaatctaacatactcttaagggtaaattaatttaagaaaaaaattactattactaacatcatgattgtacaaccagttttacaattttgtacaacctttagttactaaatctgatttttgtgtatacttttcaaatgtctctttaatgcagtgtcttaaaacaaacataaatgcgcaagtccagcttgatcagtttttcagtagttttccagcctttcttgattactagaaaataaaaggaaagaaaattttgagaagaaagaaaacagtccacttaaagaaatctccctgctggaactggttctttatataccatatgcaattaagttattgccataggaagaaagtgggctgttttttgttctttctttgttttttttcctcttacaggaatccccttttgatttaaggccacaaacatttcccctccgttgtttgtccatttagctgctgcatatgtgttgtaatggttttccagaattagatctttgaagttacaatcttcattgcattccttctttgcatagagttttccttcctcgttcgttgcaagatagaattcactttccacccctttgattgccacaatcccaactgctactgtcctgatttccatgatataagtgtgctcctggtggtctttaactgaagggcactgactgggtcactggtgaagttccccgcaggaactgagtcagaccccatctcagggccctgcacaagataggtgcctgctctaaggcgtggaccctcgccacagccctggcccgtcttgacgggcgagggttactgtacttgtcccaaccgtacagatgagaaagctgagactcagggcgagcaacccgggtcccagcggagcgcccggcacacgccgacacttcagcaccagtcgcggtggccaccactgtgcgcggagatggctgcgacgcgtgcgcaggtaaagtccatccgtgccttgcctcccaccggcgccttccccggcctctggtttttgtacccgccagcggctccgactccatcgcgtcctcttccagtctagtgcttttttccagatctcgatcccaaactccctcctgccagaatctggacccgaatccacccattgcccgttttctgctgccgctggagagaatctctgaggtccccaggagagcctgcctgcacggaagagatgcctcctcagtatggccgcccccggagaggagcgattaagtgcagacctccatgttgctcttgagcctgagcggcttcagggagccatgtttgttactggcgggc

SEQ ID NO: 19433 - RNA, 4548 nt, Homo sapiens
  source 1..4548: mol_type = other RNA
ttctctttctttagccttgtgttatttatgtgtaaagttggattatgggaggcaaataatcttttgtgtctcattcacgctcaagtaaatggcagtggagtagggatgtaaaccaaactgcatgataagccctgcaagtcattctgatgtatcaattttgcttactggtgtttaattgcagacattgtcatattaacgcaaccacaaatatattatggagtaagatgcaaaaatcacatgagtcttaagagaaaagaaatgttccgtctgtggtgggccccctttgcattattctctaacttcttattttacacctctactattagagaaatttcagtagaaaatcgtaaggggcactgttttagagtttttcttgttataggattgcttttactacagctaggtcccctcgcacatctttatgttctttggcagtctagagaaccagaagagcaaactctatgagatagaaaccctaagaatttacctccagcatcccttctcttctgtcattaaattgaatttgtagccaactcaaaggctgacaatttatactatggtttttattttttatattataatttatattatggcttatgtcaaaatgttttgttcactgctttgaaagtatcttttgtttacttttgttatcatttcatgttttaattttttcttttctaattgttagaaactcatgtatttaattttatctttcaaagaacatttttaaaaggcttactctgcttatatgtatattttgcacaaagctttccattcataaacaaaaggtgaataggaatcagaattgaaaactacataatttcttttctccttttgagtcaaatcatcacagtatagattagtcattgtgtatgaagtgcattgccaagacatagtcacatttgtgtacaaatgtaaaggctatatctcaacagaaataaaaaacaaaaacatgccaaagaccattagctaataatactaataatcgaagagtagaaagcatgtgctaactgatctagactcttgtgacagctgtatatctacccagctgcgtgaccttaggtgtatcaaaatctcaatttcctagactacaaatgagtaagagggatggaggccccttacagttttaatattctagaattctaaaggtgtgtaactagagcaaattttattttctaaaatttgcataataaatttaaaaataggagaaaaacaaataattaaagtacatatttctagaagtcttttttaggtgacttatactaccaggaatggatttaccactaaatgttggttttgcctaattcagcattgctatgtaatttgatggaagtataactccatagacaaagagcatttggtcctaacatagcttgtattttatatgtatatacactatttctatttaaatttctgtatagtcatgttttacccttttaaaatgaagattagttttagtgtgtattttcttttgtctataaacattcagtgaattcacactgaaaactgattatgaacagatagtctgctaggcactaaggaaacacatatgaaaaactaagtcctcctctgccctcaatatgctcacaagactacagttactgaagcctgacctcaaaacctagctagcaaagtccttgaatcaggtgatagttcagaataccattcatgctctctcccaagagtatatctgaggaagggcagttctttctagttttctacatcctggtcgtataggtcaaccacaggaaaattaaatgaatctattgtttttgttgacctagccttttcatataactctcatctataaatgtattaccaaatactatttatgtaaagggacttgaatgacaaatattttgaaattaaaaccacagtggttagcataccttttaaattagataaatattgacctcccattggtgaacatataaagtgctaccaagatctgccaatgaaagacttttgaagtggaaattcatccttgtaataatcctgttatctgtaggctgacctcaagccttcatgacattcagggccccttattcttaactgcatcttctattttgggcattgtgctcttgccatctaacaggaaaacaactttcagtgctgccaccttttgaacagcagagatttctagagattagaaaattactaaatttaaatatacatagttttaaaatatgatattttctacccatgcattcaaatatattctaactttaaaatcctgtaaatacttatatttgtaatgattttacttatatgatccaattaattggcaagaatatgtggtgaaagattttttacatatttgtattgttctgtgtgagacatctattgtaagcattgcttcaggctcttatttttgtctgccttccaggatttgctggcccaagtgctgtgtgctagacttagtgtcagtcagaaaagggagggaaacttgccgttgagccagacagttttgttattcctttaaaattaaaagcatatgaaacagatacagcttattaaggttttttttttataaataacataaacttaaataacaaaacaataaagttcaaaaacaacttaaaatagagtttaatgctgtaaccataggaaaaaagcatgattatttgtgggaagaacattattaaaagccatattcccaaatatgaattatacaaagatagattatgttacttgaaaaaaacttaaagatttctcaattttactttgaggatttataaaatgttattttgtggcaagtaagatgaagtacagtattatcatcaatcactgttgctatcttatatacaagatttttggaaacatccttttagcaataccctttccacttgagcagcattagaaattttgttcttatttataggtataagcatgttctaatcctgtacttttgttaaattatctattttattgactttcataatagtttttttgagaattttttttctgattagagtttaagtagattataatttttcactagaaagcatttaaaatgctgctcattttccatagttagtgtggcttgattatctgacaaatcctgccagaagcctgtaggtctgatataccttatataacaacatctgtattattattattatagcagccattttataagcagataggaatatttaaataatcattatcagataatcaaatctaacatactcttaagggtaaattaatttaagaaaaaaattactgttactaacatcatgattgtacaaccagttttacaattttttacaacctttagttactaaatctgatttttgtgtatacttttcaaatctttctttaatgcagtgtcttaaaacaaacataaatgcacaagtccagcttgatcagtttttcagtagttttccagcctttcttgattactaaaaaataaaaggaaagaaaattttgagaagaaagaaaacagtccacttaaagaaatctccctgctggaactggttctttatataccatatgcaattaagttattgccataggaagaaagtgggctgttttttgttctttcttcgttttttttcctcttacaggaatccccttttgatttaaggcaacaaacatttcccctccgttgtgtgtccatttagctgatgcatatgtgttgtaatggttttccagaattagttctttgaagttacaatcttcattgcattctttctttgcatagagttttccttccttgttcattgcaagatagaattcactttccacccctttgattgccacaattccaactgccactgtcctgatttccatgatattgtaattattcttcatctcttgggtcccttttactttgcctcttttatcgatcctcaggtaccactgtgttcgacagaagagtcttctcactcttatatcccctccttccatgtaatcataacttcttgtgtgtcgctcagggctggaacagttcacatttgtagccatttgctctggagtcatgtcattgcaagctaaagatatagtacccactagacagataatgtgaaagcatgatctgtagagcaaagttggcaggatccatgtcagtatccatttgtgcattatagtgtagtgctccgggtgttcatgaataacataatgaaaatgaatcttgagttgattgttactcctaggtcattgacctcttcctatctgtgaattgtagattgatttaagaaagagtagttgctctttccaaattgttagccttatccttttagttcctgataacaacacaggattcctccttaaataactctgttgataaatcctcataaaaacagttcgtagtaagttcagttgctgtgacgctgtttgctatttgacttttgttttgttgctaacagctggatatataagaattccatgtctgttgtctgcctggtgcaacttgagcctttctactgtagctacaaactatttctcagctgaaaagttctccagcagaatcataattgtttccataaatcaacaggcagaaggattttctctctgtgtgtgagcgcgtgtgtgcttgtgtgtgtgtgt

SEQ ID NO: 19434 - RNA, 4891 nt, Homo sapiens
  source 1..4891: mol_type = other RNA
ttctgagctgaggacagctggctgtacctccgaggccacaggcacccccacccacccctgcgcctgcagggaatgtgcagaatctgccagagcggaggccagagcccgcaggcagccacggctgttagaggaagcagatgcagcctcaccccagcccacgtctgtcaccacagccagggcctggcaggcgatggcacccgcgcagctttgggaaagaacacttggcctcccaaagggttctgccacccctgggggccgctacagccaccaaccctggggtctttccatcacttcagacactgagcagaacccagagagggttagtgagctgcaggtagggctgggacggggccccaggttccagcccagggtctcagggatccatggctggcactgcccacagggccaggcatgggcagagcagccttctcagcagcggggcccagcggccaagcctctgtcacacagcaccctgtgccagcatgccccgtgctagggagaagatgctttttaagccctctttagggggtatttcccgtctagtaagtgccagcaggcagacccactcttgacaggctcctaatgtccccaccagcgtgcacctgcacttttttttttttttttttgagacagagtctcgctctgtcgcgcagactggagcgcggtgttgtgatcttggctcactgcaatctctgccttctggcttcaagcatttctcgtgcctcagcctcctgagtagctagggttacaggcacctgccaccacgcccagctaatttttgtatttttagtagagacggggttttcaccatgttggccaggctggtctcgaactcccaatctcaggtgatccacccgcctcagcctcccaaagtgctgggatgacaggtgtgagccaacgtgcctggcctcttttatcttatagcaaaaattagtgctgccttgtttatagaaagtggccattgagggactgggggacaggccacagccaccccgatgagaggagcgggcctgccctcaccgacaccagcctcctgggacccgggccaacaaaagggctgagatgggaagaaaggttggaaatgaaagcctcgccaaagacgcagcggcaatgagtagttgggctgaagggcagcgccacgggccgcccagactacagacaaggcctggctatgcagccctcactggcaccgcggccgtgaagtcagcttctcctcagagccctggaggcaggcctggcagagcagaggtggtgtccccgccttgggggcctgtgcccctgggaaggtgctggcccaaatgtctcaggctttctgcagcccatccccagcagttcaggccagaggctcttcctgcaggtggcggtggcctgatgggctcagcaggcatgcctggagctgctgccctgagctctgctcagggagtctgtttcttcttccccaaatttccacggcctccctgagctctcagattttgagatatagatatatacatatatatgtatatatttcttcacttgcgggcagttccaaggaactgtttgttcctggacctgtataaaggtcacttttgggggacaccctccagctgccccactgccaagctggtgcacagcccttcccttccccgtgcaggcctccagcctacccctgcactccacaactctgggttttcaaggttccctctcctaggaggacactgggggcagatggggacgaggggtcaacacctggaggcaagcaggccagctccctgcccctcacaccagctcgggcagcatctctgcaaaggcagttcccaccctacctgaggaggcatgggcatccctggccccagtccaaccagaaggactgtaggtctagacctggccagagcagaacagaaccagggtttgacaggccctggggccctttcctcctttcaaagtaggcctcccaggagcagcttgtcagccacatccttggcagtcccaggagaggcagaaaagtctgagggtggggaggagagcccacagagggtggcactgcgtattgccctgggggctaatgccagggcctgcttccaggtaagtcaggtggctccaggccctgggactggacagaatggtctgtggctgatgaggaagcaggggaaactctcctgccgttggccaagtcaccagggcccaaagccaggcagctgccaatcccacggaataagagatctgttcagttttcttagggaaaactaaaaatccaaggaaacggaactctacacctccctgctgcacccagaacctaatacagggctccacccctcccactccacagtgatgctccagtacctggggcctctgacctccagagaaaccgcagggcggcccgagaccagcccacccggcccctgttctcacggcccctctgaagagtatctttaaaaacagatttaatgtgttaaaaaaaaatagaatcaagtggtgtgcttcgccactgagatgattgtgctgtggctccggggccacatagcaccagggctcgatagcagacaggagtttcggccctcgtccagtgcatgtgactggtgcaggggcggaggcccagccccacgggggccagagcaggaacacagccacctgttccaacaggcgctgtgccttgtatgccccgtacatgtgcctgccctgagaggagcatgggccaggcctctcttccagctgtgcccccagggtgccagtgaggcagggcgacctctcaccaacagagctcctccaagccatgctggatttggattcctggaaccccctgtacccatgcggtgggccaccccagggggaggggaggagagatgggagactgtgtgtatgtcccctccctccaagtgcagcaggagaaaggtcactgggctggcctggtcacacaccgtcataggggcctgctggggtatgcccgatgccccccagcctccgggccatgctgatgagtgagcgcaactgcaccagcctcagtggccccacctctctggggtcctggttctccagccaccgcagagctgtttctagcccccgcacggcctccccggcagtcggcactgaggtccctccatagtcggtggcctcctcctcgtcctctccgccccccatggcagagggcagactggctggggccggaggcgctgcagggggcagggctgggcccacctcctccctgcagccctcgggcggacccccatcatcgtccaggtgcagccactccgcaacctcctccggagccaggcacttgtaggccagagccgccaggtgggtgaggtcgctgagcaccctgctgtgctcggcggcttcctcggcctgggccggctgcccagcactgtcctcgccgggccggggctcgaaggcagcccgcaggcccagcagccagcagcgctcaatgctgcccgcctgcaccaggtcccaggagaggccagccaggtagagcatgtccttgagcatgaagctgcgcatgaagtccagcggggagccgctggcgcaggacacagccagtcgcagcagctcgcgcttgtacagctgtttgaaggcggccaccacgccctgctccagcggtgcggggatatgtgcccggctgctgcctttggacaggaacagcacccgcacagcgccatccggtgtctgcagctcctccgggggaccgaggggctccggcctgcaccgcacgggggcatcctcgctgtccagggcgggcatactggcagctgggcttgggcagggcgggtgggccaccagcagcacggccttctgctgcaggcagcttcggcgcaggtagcgtttgacgcctgggacaaattcctcaaagaaccagccccgcagcagcgggcggctgagccaggcgtcggggctgtagcggtaggaggccgggaacttgtcctggttgtggtggcgcaggctgggcgggtccggcagccgcccgatgaccagcggcttcagcttgtggctgccggtcaggtttgcggccagcagcaccgttacgcggtcgccccgccagcgccggccacagccccccgccccggggtcccctgcgcccgggggcgcagcctgctccggaagcagcttccagtagaggccggtgacgctggcgctgtaaatctgctcgtccccgtagccgccctcggccgggggcggcggggccggggcgcggtcgggcagggggccggcgccggagggcagcgcgggctcctccttgacgggcgggccgggcgcggggctcggggctgggggcccggcctcgccgtagaagcgctggctggagatgccgtggcgcttctgccagcgccagaaccagccgtggctggccttgaaggtgcactcgggcccgtagatctggcgcgcgaaggcctcggcctgcgcctggatgagcgggccagacagcggcaccccgtgctggcgcagcgccaggaaccaggcgtacacggcgcggtcgatctcctcctcgttggccagccgcatcttcttgcgctgagtgcccacctcaccgcccagctgctccaggaaccagcgcagcttgggctcgtccttgagccagccgcgcagcgtcccgcccggcacgccgaagtcgcggcacacactggcctgccgctcgccgcccttgacgcgctcgatggcctgcagcttgtccttgatggagtaggccttgcggaaggccatcttcacggccacgcggggccgcggcccgggcgcggggggcggcggccgtgcagcggggacgggggctggggcgggcgcggggggcccgggcaggggacggcggccgcggcgcggtaccgggccggccggggggcccgcggggtacatggctgcggcgggggggacccgggccgcgcgggtcgcgggagccacacgcccagccgctcggggcggggcactc

SEQ ID NO: 19435 - RNA, 3343 nt, Homo sapiens
  source 1..3343: mol_type = other RNA
ttctgctgccggccaaggcggcggctggtggtggtttctggcttcgctgttccattcccttgtcttgaggtaccactactgggttttgcctgggtgcttgggactggcacagctccctcggggtggggagactgggataggatgccaagctggtactcttgccttccatcaatgtggggacagaaggagcaggttctcccgagagcaggttcatggggcttctggccagggtcagtcagaggtgaaaactgcccccctgtcccccaggccccccaacctctcccaccagcccagtttctacactcatgcctgttctgccagagggggaggccgcaccgtgtccctccaggttttgccagggtttctgtcctgtctgttgggagggggtcaggaggcccaggttgctcaagccagcccctcccctgctggcgtcatctgtttctctagcctgaccaggaaagtcctctccactcccacccctgccccaggagagcctcttcctgtctcagggtgcccaagaggcccaaggtgccactccagaaggctttccccttctgcctctcctgtgggcatgagggagctggtgcctctttagagaggagccagagacaaccttgtcccaacccagcctgatccagttcaccaaggcagttgctctaatccaggggtggtggtggggacaggtggccaggggctggtgccagacctttggctgtaattatcgttgccttgtcccaggtctcagccggttctcgctgagatggctacgtcagtgaggccagtcactcccggtgccgctgccttggcagagctggtttagaaccaccgtgaaggtcatcgaacggggccctccaccctgcaattggcctgcggccatccttgaggccatgtggtctttgcatgagcacccaggatggtgaggaacctccgcctgctgaggcagcccacccactgcagaaggtcggactccctgctggcccccagttagtcccacttgtggtcacttagaccttgccccctcttctgcctcgtagcccttcaggagcaagatggcagccggcatgtaccttctggatttccttctctgccaggggcctgctctagtgttttcagctgctcctccttgaatgccacctccacttcttccttttgtgacatgaacaggttgcttcatgtctctgatatggaatgagatgcccgtgttttgaggctattgggaggactgaccatctagcagcacattgtagacagccataggggggtgcccggcacacgagaatgcccccccgggacgggtctcactggctttgggggctgtcacccccgtgcaccgtcactagcacccccaacaccttttgggtgtctgtcctagggtgtctgcggtgtgtgccctgaaggaaggtaggcaagctggaggtggggagctatgtttttgttgttggttttggttttctttgagatggagtttctctcttgttgcccaagctagagtgcaatggcatgatctcagctcactgcaacctctgcctcccagattcaagtgattctcctgcctcagcctcccgagtagctgggatcacgagtgtgcgccaccatgcccggctaatttttgtatttttagtagaaacaggatttcaccatgttagccagactggtctcgaactcctgacatcaggtgatccgccctcggcctcccaaagtgttgggattacaggtgtgagccactgcgcccggcctggggagctgtttttttaagtgatgatgagggtagcaggcagaagatggctccgtggaaaattagatgagttcttgtcaaaagccgtgggttccctgagttagatccacccagcttctcacacctcacctggagtgagtgcgtttctgtggaggtgaggatctcagttttcaaatgtactgagaggcatagggtcctagaatgctatagatcatccgctcccgcctccttccttctatacgtggggaagctgagacccgagagagcaagcaacttctctgaggttacacagcaggacagggccccagccagcacccccactggtgccccacgctgtctctccatggaggcctgtctccagcttagaccagcaagatagccaggagcagccccgctgagggtactgcccgtgcagtgggctcagtacaggagccagggcccgagagccccctggaagccagctggctgtgctcggccagccccagcccacatttgtggatctgaagctgcttttatcagcatatcaccaccaggccggggccacaccaggctctttgagactacctggagtccttgtcaccacaggtacaggtcttgtgagtctagccagcctgagtgtaggactgaaccctctggtcagactgaatgggacattctctctggccaggtggagcaggcttgcacaaggacagtggtcccctcttggttccgggacctccgtgccatcctcacgccccagctttccaggttccctcattcttagagggacgacaatgccgacagtgtcccttacgggacagtttgcgcgtggttcaggagctgggctgcctttctcccctccctctctgtctacacttggtctggcgttttcagcctgactggcactgtgcccacacggcctaatgtagcccagcagagacactccttcaaagagggagcgggcagggagagctttttcgcttgtgccacacccagagacccagggagagattgcagggggcacttttccttgtgagcgagagacctggggctgtgctcaccagaacagggaggaggaaggttggactgaggctgaatttactggtgcaggaaaagtggggtttgttgctgagaagctctggccagcctcctccaggggctgcaaagtgggagagctgcagactcatgccgggtggaccccggcctccagcggggaaaagtgtcagttcccagcagcagcaggctgcggctgtggacagtgtcatagctttgcgcccagggcttccctagggggctgactggaagctgaatttgccagccaggcatggccagcctcacccagccccagggtctgacccaggggtactcacggtatcctgtcacacagtgagcagaagtaggaccgttggacgtggctgttctgcccccagagagctggagaggaaccccgggaccccctttgttttgcagttgatatcttgtcatttggagcgtaaacccgcgactgaaccttcatggcgcaggtgggggagctgaggggtcctgttctctaaagaggaggaggcgcattccagccggtccccaggtggtcttcccagcgggctatttaaagccaggccaaggagtgcc

SEQ ID NO: 19436 - RNA, 922 nt, Homo sapiens
  source 1..922: mol_type = other RNA
ttctgctgccggccaaggcggcggctggtggtggtttctggcttcgctgttccattcccttgtcttgaggtaccactactgggttttgcctgggtgcttgggactggcacagctccctcggggtggggagactgggataggatgccaagctggtactcttgccttccatcaatgtggggacagaaggagcaggttctcccgagagcaggttcatggggcttctggccagggtcagtcagaggtgaaaactgcccccctgtcccccaggccccccaacctctcccaccagcccagtttctacactcatgcctgttctgccagagggggaggccgcaccgtgtccctccaggttttgccagggtttctgtcctgtctgttgggagggggtcaggaggcccaggttgctcaagccagcccctcccctgctggcgtcatctgtttctctagcctgaccaggaaagtcctctccactcccacccctgccccaggagagcctcttcctgtctcagggtgcccaagaggcccaaggtgccactccagaaggctttccccttctgcctctcctgtgggcatgagggagctggtgcctctttagagaggagccagagacaaccttgtcccaacccagcctgatccagttcaccaaggcagttgctctaatccaggggtggtggtggggacaggtggccaggggctggtgccagacctttggctgtaattatcgttgccttgtcccaggtctcagccggttctcgctgagatggctacgtcagtgaggccagtcactcccggtgccgctgccttggcagagcttctggatttccttctctgccaggggcctgctctagtgttttcagctgctcctccttgaatgccacctccacttcttccttttgtgacatgaacaggttgcttcatgtct

SEQ ID NO: 19437 - RNA, 70 nt, Homo sapiens
  source 1..70: mol_type = other RNA
ttctggatatgaagacaatcaagaacaccaaatcttttcttgattgtcttcatatccagaactgggcaat

SEQ ID NO: 19438 - RNA, 46 nt, Homo sapiens
  source 1..46: mol_type = other RNA
ttgaactgttaagaaccactggacccagcgcgcgagtccccaacac

SEQ ID NO: 19439 - RNA, 41 nt, Homo sapiens
  source 1..41: mol_type = other RNA
ttgagaatgatgaatcattaggttccaattggaaattttat

SEQ ID NO: 19440 - RNA, 3506 nt, Homo sapiens
  source 1..3506: mol_type = other RNA
ttgaggagacatggtgggggccagcctgtgctgctaaacatagattttgctgatctgttggcttctcagtttatagcattcagccccctggctcctcagcagctccttctcttcggctgtgtctcgagctttcagctgcgagaagtgggcaggagaggcgatgagatcatattgttggtccagataccgcaggtagatgagcatgtgcagggcataggccaacaccagcagcaggatcagggacattgccaggccgatcagaaaagctggcgagaaggaggaggcgcagtcttgggctttggtaaatcgtccccccttgatggcaaaaccttggatctgcaggagaaaggaaggagctgaagtgatacatcccttctctcctaggatctacttcccagttgggctggcagttctggcccctaggtagccaaatttaatatactatcaccatatttgctgaataatttaaccacacaatttgacaaatgtgattgtgcttatggggacaatgcaactcaatcttaaaacaagactgacccagaaattctgggatgcatggatgtcataactaggaggctcatgaaattcaagactctgaaataaaaccttgatttcaaggctctgagataaaagttcttttaatctgatccttagaaatattccagttcatgtaaaaaccacaactgctgtggtgtctctaaaattcaaagcacactcaaaattttataagggtagtataagtttcacaaagattttaagtctccgttcctctgcctttgattctattgacaggaatgaggaagagtctttgaagggggatgtcatgatccttaatgaggtaaaacataaataataatcataaaagctaacacgtattgaaggtttttgtgcaccatatactaccttgtttagtaggcaaagagcctatgagtaagttactattttattcctactttatggatgaggaaactgaggcacagaaaaattaagtaacttgcccagagtcacataacagtaaatgctgtgatggtgtaattgaaacctgggcagtgggcgtcagactcatactccatagctcctggtgggttctgtctcttcctcctccctaccctctctctctctctctattggttttatcatacaggctttgtcccatttttggaagaggtggataccagcccctccttgcatcctacccattacgtttaatggcaaaaaccgcaatcacttttgcaccaaccaaatagaaagtaaagcttccattgtgtgcagatgaaatggtataattacttgaaaggaagagaggttcaaattgagaactggcactgatatctaatactgtcaaaatgaaacaggactatagagcaattactttaaagcaagagccatcgcttgtggaagacagctccctgtccagccggctttaaaagtatgaccctacacagcatttcctcattcagacacctactcagtttttaaagagtacatcagacaactgaactatccatgagtgctttactgaaaattcactttgatggcttaagtgagcactttggcattgtcccatgctaaaattattgaggccgcccatcactccatagacacaaggggccttgctcgcccaactcgattgaacccaaagcagatcctgaaggagactcttgtcctggcttcggggatccctgccccacacctcctggaaatcaataaaagtgacctcccacaggctcgacccatcatccgtgtcgctgggcagcaagagggcctggtcctgctgcaggctgcccacgcgttggcagcggtaggagtaaccagagggagcatatacgccagttgggttaaagactgcttggattgaattgttggaaatgatctcgactcggcgcaaactaaaccaactctggatggacaacttgttgtaattggtaaggatgaatcttatagcaagacttctggggtttccagcatcaccaagcttcaaagacaacctagcactttcttcactgcaatttgagttgtcagggtccacagttaccttctgaccaaatggctcgtctgtaaggtccagccaggtttgattcttaaatttaatcattattcttttggcccagaagagaatgcaaggaattccattgatggagacattaactgggccatgatggctgaatgcattccaaggttctttttctaaatgcccttctttgctcagattgtagttgagagcctgtgtgattggtattgttgtgaaattctggaatggtttcatatctccattattctgatcattcctcataaccacttctttatttgaagatgttggagaacttacattcttcctggcaaatatatggtccaaggttagtgaaagtcctataccttctctcctcaaacctttttctcccactctttctcttcactgatggccttgcatggcctacaggctccacatgttcctgtgtaactctcagaccccatctaatgccacactactcctcagtcactatgctccccttcttcactgatctttcagttcttagaaagcactagcccattctacatctgcacagagatgtcaccttaaactaccctatccagagtagccacccccatccccaagtcactatcacccatccagctatattttctctatagctctacagtatgtaaaaatcatctatttaattatttaatttacatctatctaactggtctgtcctctcacatttagaatataaactgtatcagagcagaaaccttcaccctcttaatttaaccgccatattcccggtacctacaacagcgtctggcacatagaaggcatttttaaacatccttgctgagtgaaccaatatcccagaaacctctcacagctagttcatcttacaggagaaacagtattaaagagttaattaaatggccaggcgcggtggctcacgcctgtaatcccagcacattgggaggccgaggcgggcggatcactcgaggtcaggagatcgacaccagcctggccaacatggtgaaaccccctctctactgaaaatacaaacatcagccaggcgtgatggtggaagcctgtaatcccagctactcaggaggctgaggtgggacaatcgcttgaacccgggaggcggaggttgtagtgagccaagatcgcaccactgcacaacagcctagaagacagagtgagaccctgtctcagaaaaaaataaaaataaaaataaataaatctataagtaaatgactcgccagtcaaaataaacggcaactttagggttaaaggcccaatctggctccaaagcttggggttttagttactacactacattgcttcactatattttacaatttactagctgcttataagtatgaattaaggctcagaagtctaattttccagactactcggaggactctcgccccactccactccacaaagattcagctcagcgactccttcctactctgacctagccccgcgtcccgctctcagtggcttgggcaagagc

SEQ ID NO: 19441 - RNA, 2272 nt, Homo sapiens
  source 1..2272: mol_type = other RNA
ttgaggagacatggtgggggccagcctgtgctgctaaacatagattttgctgatctgttggcttctcagtttatagcattcagccccctggctcctcagcagctccttctcttcggctgtgtctcgagctttcagctgcgagaagtgggcaggagaggcgatgagatcatattgttggtccagataccgcaggtagatgagcatgtgcagggcataggccaacaccagcagcaggatcagggacattgccaggccgatcagaaaagctggcgagaaggaggaggcgcagtcttgggctttggtaaatcgtccccccttgatggcaaaaccttggatctggaaatcaataaaagtgacctcccacaggctcgacccatcatccgtgtcgctgggcagcaagagggcctggtcctgctgcaggctgcccacgcgttggcagcggtaggagtaaccagagggagcatatacgccagttgggttaaagactgcttggattgaattgttggaaatgatctcgactcggcgcaaactaaaccaactctggatggacaacttgttgtaattggtaaggatgaatcttatagcaagacttctggggtttccagcatcaccaagcttcaaagacaaccatttggagttgagaccaagcctggaatcctttgctgttttcaaaacgagtttgagaacccttgctttccaaagtctcattttctacaagttattccgacaattagcaaaaaggttcagaagaaaactagcactttcttcactgcaatttgagttgtcagggtccacagttaccttctgaccaaatggctcgtctgtaaggtccagccaggtttgattcttaaatttaatcattattcttttggcccagaagagaatgcaaggaattccattgatggagacattaactgggccatgatggctgaatgcattccaaggttctttttctaaatgcccttctttgctcagattgtagttgagagcctgtgtgattggtattgttgtgaaattctggaatggtttcatatctccattattctgatcattcctcataaccacttctttatttgaagatgttggagaacttacattcttcctggcaaatatatggtccaaggttagtgaaagtcctataccttctctcctcaaacctttttctcccactctttctcttcactgatggccttgcatggcctacaggctccacatgttcctgtgtaactctcagaccccatctaatgccacactactcctcagtcactatgctccccttcttcactgatctttcagttcttagaaagcactagcccattctacatctgcacagagatgtcaccttaaactaccctatccagagtagccacccccatccccaagtcactatcacccatccagctatattttctctatagctctacagtatgtaaaaatcatctatttaattatttaatttacatctatctaactggtctgtcctctcacatttagaatataaactgtatcagagcagaaaccttcaccctcttaatttaaccgccatattcccggtacctacaacagcgtctggcacatagaaggcatttttaaacatccttgctgagtgaaccaatatcccagaaacctctcacagctagttcatcttacaggagaaacagtattaaagagttaattaaatggccaggcgcggtggctcacgcctgtaatcccagcacattgggaggccgaggcgggcggatcactcgaggtcaggagatcgacaccagcctggccaacatggtgaaaccccctctctactgaaaatacaaacatcagccaggcgtgatggtggaagcctgtaatcccagctactcaggaggctgaggtgggacaatcgcttgaacccgggaggcggaggttgtagtgagccaagatcgcaccactgcacaacagcctagaagacagagtgagaccctgtctcagaaaaaaataaaaataaaaataaataaatctataagtaaatgactcgccagtcaaaataaacggcaactttagggttaaaggcccaatctggctccaaagcttggggttttagttactacactacattgcttcactatattttacaatttactagctgcttataagtatgaattaaggctcagaagtctaattttccagactactcggaggactctcgccccactccactccacaaagattcagctcagcgactccttcctactctgacctagccccgcgtcccgctctcagtggcttgggcaagagc

SEQ ID NO: 19442 - RNA, 2220 nt, Homo sapiens
  source 1..2220: mol_type = other RNA
ttgaggagacatggtgggggccagcctgtgctgctaaacatagattttgctgatctgttggcttctcagtttatagcattcagccccctggctcctcagcagctccttctcttcggctgtgtctcgagctttcagctgcgagaagtgggcaggagaggcgatgagatcatattgttggtccagataccgcaggtagatgagcatgtgcagggcataggccaacaccagcagcaggatcagggacattgccaggccgatcagaaaagctggcgagaaggaggaggcgcagtcttgggctttggtaaatcgtccccccttgatggcaaaaccttggatctggaaatcaataaaagtgacctcccacaggctcgacccatcatccgtgtcgctgggcagcaagagggcctggtcctgctgcaggctgcccacgcgttggcagcggtaggagtaaccagagggagcatatacgccagttgggttaaagactgcttggattgaattgttggaaatgatctcgactcggcgcaaactaaaccaactctggatggacaacttgttgtaattggtaaggatgaatcttatagcaagacttctggggtttccagcatcaccaagcttcaaagacaaccatttggagttgagaccaagcctggaatcctttgctgttttcaaaacgagtttgagaacccttgctttccaaagtctcattttctacaagttattccgacaattagcaaaaaggttcagaagaaaactagcactttcttcactgcaatttgagttgtcagggtccacagttaccttctgaccaaatggctcgtctgtaaggtccagccaggtttgattcttaaatttaatcattattcttttggcccagaagagaatgcaaggaattccattgatggagacattaactgggccatgatggctgaatgcattccaaggttctttttctaaatgcccttctttgctcagattgtagttgagagcctgtgtgattggtattgttgtgaaattctggaatggtttcatatctccattattctgatcattcctcataaccacttctttatttgaagatgttggagaacttctctcctcaaacctttttctcccactctttctcttcactgatggccttgcatggcctacaggctccacatgttcctgtgtaactctcagaccccatctaatgccacactactcctcagtcactatgctccccttcttcactgatctttcagttcttagaaagcactagcccattctacatctgcacagagatgtcaccttaaactaccctatccagagtagccacccccatccccaagtcactatcacccatccagctatattttctctatagctctacagtatgtaaaaatcatctatttaattatttaatttacatctatctaactggtctgtcctctcacatttagaatataaactgtatcagagcagaaaccttcaccctcttaatttaaccgccatattcccggtacctacaacagcgtctggcacatagaaggcatttttaaacatccttgctgagtgaaccaatatcccagaaacctctcacagctagttcatcttacaggagaaacagtattaaagagttaattaaatggccaggcgcggtggctcacgcctgtaatcccagcacattgggaggccgaggcgggcggatcactcgaggtcaggagatcgacaccagcctggccaacatggtgaaaccccctctctactgaaaatacaaacatcagccaggcgtgatggtggaagcctgtaatcccagctactcaggaggctgaggtgggacaatcgcttgaacccgggaggcggaggttgtagtgagccaagatcgcaccactgcacaacagcctagaagacagagtgagaccctgtctcagaaaaaaataaaaataaaaataaataaatctataagtaaatgactcgccagtcaaaataaacggcaactttagggttaaaggcccaatctggctccaaagcttggggttttagttactacactacattgcttcactatattttacaatttactagctgcttataagtatgaattaaggctcagaagtctaattttccagactactcggaggactctcgccccactccactccacaaagattcagctcagcgactccttcctactctgacctagccccgcgtcccgctctcagtggcttgggcaagagc

SEQ ID NO: 19443 - RNA, 2298 nt, Homo sapiens
  source 1..2298: mol_type = other RNA
ttgaggagacatggtgggggccagcctgtgctgctaaacatagattttgctgatctgttggcttctcagtttatagcattcagccccctggctcctcagcagctccttctcttcggctgtgtctcgagctttcagctgcgagaagtgggcaggagaggcgatgagatcatattgttggtccagataccgcaggtagatgagcatgtgcagggcataggccaacaccagcagcaggatcagggacattgccaggccgatcagaaaagctggcgagaaggaggaggcgcagtcttgggctttggtaaatcgtccccccttgatggcaaaaccttggatctggaaatcaataaaagtgacctcccacaggctcgacccatcatccgtgtcgctgggcagcaagagggcctggtcctgctgcaggctgcccacgcgttggcagcggtaggagtaaccagagggagcatatacgccagttgggttaaagactgcttggattgaattgttggaaatgatctcgactcggcgcaaactaaaccaactctggatggacaacttgttgtaattggtaaggatgaatcttatagcaagacttctggggtttccagcatcaccaagcttcaaagacaaccatttggagttgagaccaagcctggaatcctttgctgttttcaaaacgagtttgagaacccttgctttccaaagtctcattttctacaagttattccgacaattagcaaaaaggttcagaagaaaactagcactttcttcactgcaatttgagttgtcagggtccacagttaccttctgaccaaatggctcgtctgtaaggtccagccaggtttgattcttaaatttaatcattattcttttggcccagaagagaatgcaaggaattccattgatggagacattaactgggccatgatggctgaatgcattccaaggttctttttctaaatgcccttctttgctcagattgtagttgagagctatcagggtgatgggattcataccgcaaactccagcattatgcactattctcacgtaacaaatctgcacatggaccctctgtgtgattggtattgttgtgaaattctggaatggtttcatatctccattattctgatcattcctcataaccacttctttatttgaagatgttggagaacttctctcctcaaacctttttctcccactctttctcttcactgatggccttgcatggcctacaggctccacatgttcctgtgtaactctcagaccccatctaatgccacactactcctcagtcactatgctccccttcttcactgatctttcagttcttagaaagcactagcccattctacatctgcacagagatgtcaccttaaactaccctatccagagtagccacccccatccccaagtcactatcacccatccagctatattttctctatagctctacagtatgtaaaaatcatctatttaattatttaatttacatctatctaactggtctgtcctctcacatttagaatataaactgtatcagagcagaaaccttcaccctcttaatttaaccgccatattcccggtacctacaacagcgtctggcacatagaaggcatttttaaacatccttgctgagtgaaccaatatcccagaaacctctcacagctagttcatcttacaggagaaacagtattaaagagttaattaaatggccaggcgcggtggctcacgcctgtaatcccagcacattgggaggccgaggcgggcggatcactcgaggtcaggagatcgacaccagcctggccaacatggtgaaaccccctctctactgaaaatacaaacatcagccaggcgtgatggtggaagcctgtaatcccagctactcaggaggctgaggtgggacaatcgcttgaacccgggaggcggaggttgtagtgagccaagatcgcaccactgcacaacagcctagaagacagagtgagaccctgtctcagaaaaaaataaaaataaaaataaataaatctataagtaaatgactcgccagtcaaaataaacggcaactttagggttaaaggcccaatctggctccaaagcttggggttttagttactacactacattgcttcactatattttacaatttactagctgcttataagtatgaattaaggctcagaagtctaattttccagactactcggaggactctcgccccactccactccacaaagattcagctcagcgactccttcctactctgacctagccccgcgtcccgctctcagtggcttgggcaagagc

SEQ ID NO: 19444 - RNA, 1180 nt, Homo sapiens
  source 1..1180: mol_type = other RNA
ttgaggagacatggtgggggccagcctgtgctgctaaacatagattttgctgatctgttggcttctcagtttatagcattcagccccctggctcctcagcagctccttctcttcggctgtgtctcgagctttcagctgcgagaagtgggcaggagaggcgatgagatcatattgttggtccagataccgcaggtagatgagcatgtgcagggcataggccaacaccagcagcaggatcagggacattgccaggccgatcagaaaagctggcgagaaggaggaggcgcagtcttgggctttggtaaatcgtccccccttgatggcaaaaccttggatctggaaatcaataaaagtgacctcccacaggctcgacccatcatccgtgtcgctgggcagcaagagggcctggtcctgctgcaggctgcccacgcgttggcagcggtaggagtaaccagagggagcatatacgccagttgggttaaagactgcttggattgaattgttggaaatgatctcgactcggcgcaaactaaaccaactctggatggacaacttgttgtaattggtaaggatgaatcttatagcaagacttctggggtttccagcatcaccaagcttcaaagacaaccatttggagttgagaccaagcctggaatcctttgctgttttcaaaacgagtttgagaacccttgctttccaaagtctcattttctacaagttattccgacaattagcaaaaaggttcagaagaaaactgccgggaaaatataacaattttttttttttgagatggagtctcactcactctgtcacccaagctggagagcaatggcgcgataacagcctagaagacagagtgagaccctgtctcagaaaaaaataaaaataaaaataaataaatctataagtaaatgactcgccagtcaaaataaacggcaactttagggttaaaggcccaatctggctccaaagcttggggttttagttactacactacattgcttcactatattttacaatttactagctgcttataagtatgaattaaggctcagaagtctaattttccagactactcggaggactctcgccccactccactccacaaagattcagctcagcgactccttcctactctgacctagccccgcgtcccgctctcagtggcttgggcaagagc

SEQ ID NO: 19445 - RNA, 1193 nt, Homo sapiens
  source 1..1193: mol_type = other RNA
ttgaggagacatggtgggggccagcctgtgctgctaaacatagattttgctgatctgttggcttctcagtttatagcattcagccccctggctcctcagcagctccttctcttcggctgtgtctcgagctttcagctgcgagaagtgggcaggagaggcgatgagatcatattgttggtccagataccgcaggtagatgagcatgtgcagggcataggccaacaccagcagcaggatcagggacattgccaggccgatcagaaaagctggcgagaaggaggaggcgcagtcttgggctttggtaaatcgtccccccttgatggcaaaaccttggatctggaaatcaataaaagtgacctcccacaggctcgacccatcatccgtgtcgctgggcagcaagagggcctggtcctgctgcaggctgcccacgcgttggcagcggtaggagtaaccagagggagcatatacgccagttgggttaaagactgcttggattgaattgttggaaatgatctcgactcggcgcaaactaaaccaactctggatggacaacttgttgtaattggtaaggatgaatcttatagcaagacttctggggtttccagcatcaccaagcttcaaagacaaccatttggagttgagaccaagcctggaatcctttgctgttttcaaaacgagtttgagaacccttgctttccaaagtctcattttctacaagttattccgacaattagcaaaaaggttcagaagaaaactgccgggaaaatataacaattttttttttttgagatggagtctcactcactctgtcacccaagctggagagcaatggcgcgatctcagctcaccacaacagcctagaagacagagtgagaccctgtctcagaaaaaaataaaaataaaaataaataaatctataagtaaatgactcgccagtcaaaataaacggcaactttagggttaaaggcccaatctggctccaaagcttggggttttagttactacactacattgcttcactatattttacaatttactagctgcttataagtatgaattaaggctcagaagtctaattttccagactactcggaggactctcgccccactccactccacaaagattcagctcagcgactccttcctactctgacctagccccgcgtcccgctctcagtggcttgggcaagagc

SEQ ID NO: 19446 - RNA, 2694 nt, Homo sapiens
  source 1..2694: mol_type = other RNA
ttgaggagacatggtgggggccagcctgtgctgctaaacatagattttgctgatctgttggcttctcagtttatagcattcagccccctggctcctcagcagctccttctcttcggctgtgtctcgagctttcagctgcgagaagtgggcaggagaggcgatgagatcatattgttggtccagataccgcaggtagatgagcatgtgcagggcataggccaacaccagcagcaggatcagggacattgccaggccgatcagaaaagctggcgagaaggaggaggcgcagtcttgggctttggtaaatcgtccccccttgatggcaaaaccttggatctggaaatcaataaaagtgacctcccacaggctcgacccatcatccgtgtcgctgggcagcaagagggcctggtcctgctgcaggctgcccacgcgttggcagcggtaggagtaaccagagggagcatatacgccagttgggttaaagactgcttggattgaattgttggaaatgatctcgactcggcgcaaactaaaccaactctggatggacaacttgttgtaattggtaaggatgaatcttatagcaagacttctggggtttccagcatcaccaagcttcaaagacaaccatttggagttgagaccaagcctggaatcctttgctgttttcaaaacgagtttgagaacccttgctttccaaagtctcattttctacaagttattccgacaattagcaaaaaggttcagaagaaaactgccgggaaaatataacaattttttttttttgagatggagtctcactcactctgtcacccaagctggagagcaatggcgcgatctcagctcaccacaacctccacctcccaggttcaagcaattctcctgtctcagcctcctgagtagctgggattacaggcacctgccaccacgcccggctaatttttgtattttagtagagacgaggtttcaccatgttggccaggcttgtctccaactcctgacctcaggtgatccactcccttggcctcccgaagtgctgggattacaggcgtgagccaccatgcccagccaacaatttttgaagttaacttctgacttgttcctttattttagacagtaaatacttcctcaaagatgtgtgtcagggtcctatacaaaggagcctactttttttttctagcactttcttcactgcaatttgagttgtcagggtccacagttaccttctgaccaaatggctcgtctgtaaggtccagccaggtttgattcttaaatttaatcattattcttttggcccagaagagaatgcaaggaattccattgatggagacattaactgggccatgatggctgaatgcattccaaggttctttttctaaatgcccttctttgctcagattgtagttgagagcctgtgtgattggtattgttgtgaaattctggaatggtttcatatctccattattctgatcattcctcataaccacttctttatttgaagatgttggagaacttacattcttcctggcaaatatatggtccaaggttagtgaaagtcctataccttctctcctcaaacctttttctcccactctttctcttcactgatggccttgcatggcctacaggctccacatgttcctgtgtaactctcagaccccatctaatgccacactactcctcagtcactatgctccccttcttcactgatctttcagttcttagaaagcactagcccattctacatctgcacagagatgtcaccttaaactaccctatccagagtagccacccccatccccaagtcactatcacccatccagctatattttctctatagctctacagtatgtaaaaatcatctatttaattatttaatttacatctatctaactggtctgtcctctcacatttagaatataaactgtatcagagcagaaaccttcaccctcttaatttaaccgccatattcccggtacctacaacagcgtctggcacatagaaggcatttttaaacatccttgctgagtgaaccaatatcccagaaacctctcacagctagttcatcttacaggagaaacagtattaaagagttaattaaatggccaggcgcggtggctcacgcctgtaatcccagcacattgggaggccgaggcgggcggatcactcgaggtcaggagatcgacaccagcctggccaacatggtgaaaccccctctctactgaaaatacaaacatcagccaggcgtgatggtggaagcctgtaatcccagctactcaggaggctgaggtgggacaatcgcttgaacccgggaggcggaggttgtagtgagccaagatcgcaccactgcacaacagcctagaagacagagtgagaccctgtctcagaaaaaaataaaaataaaaataaataaatctataagtaaatgactcgccagtcaaaataaacggcaactttagggttaaaggcccaatctggctccaaagcttggggttttagttactacactacattgcttcactatattttacaatttactagctgcttataagtatgaattaaggctcagaagtctaattttccagactactcggaggactctcgccccactccactccacaaagattcagctcagcgactccttcctactctgacctagccccgcgtcccgctctcagtggcttgggcaagagc

SEQ ID NO: 19447 - RNA, 2033 nt, Homo sapiens
  source 1..2033: mol_type = other RNA
ttgaggagacatggtgggggccagcctgtgctgctaaacatagattttgctgatctgttggcttctcagtttatagcattcagccccctggctcctcagcagctccttctcttcggctgtgtctcgagctttcagctgcgagaagtgggcaggagaggcgatgagatcatattgttggtccagataccgcaggtagatgagcatgtgcagggcataggccaacaccagcagcaggatcagggacattgccaggccgatcagaaaagctggcgagaaggaggaggcgcagtcttgggctttggtaaatcgtccccccttgatggcaaaaccttggatctggaaatcaataaaagtgacctcccacaggctcgacccatcatccgtgtcgctgggcagcaagagggcctggtcctgctgcaggctgcccacgcgttggcagcggtaggagtaaccagagggagcatatacgccagttgggttaaagactgcttggattgaattgttggaaatgatctcgactcggcgcaaactaaaccaactctggatggacaacttgttgtaattggtaaggatgaatcttatagcaagacttctggggtttccagcatcaccaagcttcaaagacaaccatttggagttgagaccaagcctggaatcctttgctgttttcaaaacgagtttgagaacccttgctttccaaagtctcattttctacaagttattccgacaattagcaaaaaggttcagaagaaaactgccgggaaaatataacaattttttttttttgagatggagtctcactcactctgtcacccaagctggagagcaatggcgcgatctcagctcaccacaacctccacctcccaggttcaagcaattctcctgtctcagcctcctgagtagctgggattacaggcacctgccaccacgcccggctaatttttgtattttagtagagacgaggtttcaccatgttggccaggcttgtctccaactcctgacctcaggtgatccactcccttggcctcccgaagtgctgggattacaggcgtgagccaccatgcccagccaacaatttttgaagttaacttctgacttgttcctttattttagacagtaaatacttcctcaaagatgtgtgtcagggtcctatacaaaggagcctactttttttttctagcactttcttcactgcaatttgagttgtcagggtccacagttaccttctgaccaaatggctcgtctgtaaggtccagccaggtttgattcttaaatttaatcattattcttttggcccagaagagaatgcaaggaattccattgatggagacattaactgggccatgatggctgaatgcattccaaggttctttttctaaatgcccttctttgctcagattgtagttgagagcctgtgtgattggtattgttgtgaaattctggaatggtttcatatctccattattctgatcattcctcataaccacttctttatttgaagatgttggagaacttacattcttcctggcaaatatatggtccaaggttagtgaaagtcctataccttctctcctcaaacctttttctcccactctttctcttcactgatggccttgcttcccaagtggcctcccagattcatgtctttttctcctctcaacagccagagtaaccccataaaaatataaatcttattttgctacctactcccaagctcaaaactttacaatggctttaaatcaccagaagagtagaaaaaggctttaccatggcctacaggctccacatgttcctgtgtaactctcagaccccatctaatgccacactactcctcagtcactatgctccccttcttcactgatctttcagttcttagaaagcactagcccattctacatctgcacagagatgtcaccttaaactaccctatccagagtagccacccccatccccaagtcactatcacccatccagctatattttctctatagctctacagtatgtaaaaatcatctatttaattatttaattta

SEQ ID NO: 19448 - RNA, 2845 nt, Homo sapiens
  source 1..2845: mol_type = other RNA
ttgaggagacatggtgggggccagcctgtgctgctaaacatagattttgctgatctgttggcttctcagtttatagcattcagccccctggctcctcagcagctccttctcttcggctgtgtctcgagctttcagctgcgagaagtgggcaggagaggcgatgagatcatattgttggtccagataccgcaggtagatgagcatgtgcagggcataggccaacaccagcagcaggatcagggacattgccaggccgatcagaaaagctggcgagaaggaggaggcgcagtcttgggctttggtaaatcgtccccccttgatggcaaaaccttggatctggaaatcaataaaagtgacctcccacaggctcgacccatcatccgtgtcgctgggcagcaagagggcctggtcctgctgcaggctgcccacgcgttggcagcggtaggagtaaccagagggagcatatacgccagttgggttaaagactgcttggattgaattgttggaaatgatctcgactcggcgcaaactaaaccaactctggatggacaacttgttgtaattggtaaggatgaatcttatagcaagacttctggggtttccagcatcaccaagcttcaaagacaaccatttggagttgagaccaagcctggaatcctttgctgttttcaaaacgagtttgagaacccttgctttccaaagtctcattttctacaagttattccgacaattagcaaaaaggttcagaagaaaactgccgggaaaatataacaattttttttttttgagatggagtctcactcactctgtcacccaagctggagagcaatggcgcgatctcagctcaccacaacctccacctcccaggttcaagcaattctcctgtctcagcctcctgagtagctgggattacaggcacctgccaccacgcccggctaatttttgtattttagtagagacgaggtttcaccatgttggccaggcttgtctccaactcctgacctcaggtgatccactcccttggcctcccgaagtgctgggattacaggcgtgagccaccatgcccagccaacaatttttgaagttaacttctgacttgttcctttattttagacagtaaatacttcctcaaagatgtgtgtcagggtcctatacaaaggagcctactttttttttctagcactttcttcactgcaatttgagttgtcagggtccacagttaccttctgaccaaatggctcgtctgtaaggtccagccaggtttgattcttaaatttaatcattattcttttggcccagaagagaatgcaaggaattccattgatggagacattaactgggccatgatggctgaatgcattccaaggttctttttctaaatgcccttctttgctcagattgtagttgagagcctgtgtgattggtattgttgtgaaattctggaatggtttcatatctccattattctgatcattcctcataaccacttctttatttgaagatgttggagaacttctctcctcaaacctttttctcccactctttctcttcactgatggccttgcatggcctacaggctccacatgttcctgtgtaactctcagaccccatctaatgccacactactcctcagtcactatgctccccttcttcactgatctttcagttcttagaaagcactagcccattctacatctgcacagagatgtcaccttaaactaccctatccagagtagccacccccatccccaagtcactatcacccatccagctatattttctctatagctctacagtatgtaaaaatcatctatttaattatttaatttacatctatctaactggtctgtcctctcacatttagaatataaactgtatcagagcagaaaccttcaccctcttaatttaaccgccatattcccggtacctacaacagcgtctggcacatagaaggcatttttaaacatccttgctgagtgaaccaatatcccagaaacctctcacagctagttcatcttacaggagaaacagtattaaagagttaattaaatggccaggcgcggtggctcacgcctgtaatcccagcacattgggaggccgaggcgggcggatcactcgaggtcaggagatcgacaccagcctggccaacatggtgaaaccccctctctactgaaaatacaaacatcagccaggcgtgatggtggaagcctgtaatcccagctactcaggaggctgaggtgggacaatcgcttgaacccgggaggcggaggttgtagtgagccaagatcgcaccactgcacaacagcctagaagacagagtgagaccctgtctcagaaaaaaataaaaataaaaataaataaatctataagtaaatgactcgccagtcaaaataaacggcaactttagggttaaaggcccaatctggctccaaagcttggggttttagttactacactacattgcttcactatattttacaatttactagctgcttataagtatgaattaaggctcagaagtctaattttccagactactcggaggactctcgccccactccactccacaaagattcagctcagcgactccttcctactctgacctagccccgcgtcccgctctcagtggcttgggcaagagcgcctgcgcggtgagcgggtcccataaaacgcattctgggattggtagtccatgttcctccggtctccagcattcaaaagaaaaagggggaaaaaaaaccatgcaaattagatatctctgaatttcttgcaaattaaataagacgcagattctggctcaggaaagtgatgcaaacgcgtcgttttcaaaggagagaccccagcc

SEQ ID NO: 19449 - RNA, 2772 nt, Homo sapiens
  source 1..2772: mol_type = other RNA
ttgaggagacatggtgggggccagcctgtgctgctaaacatagattttgctgatctgttggcttctcagtttatagcattcagccccctggctcctcagcagctccttctcttcggctgtgtctcgagctttcagctgcgagaagtgggcaggagaggcgatgagatcatattgttggtccagataccgcaggtagatgagcatgtgcagggcataggccaacaccagcagcaggatcagggacattgccaggccgatcagaaaagctggcgagaaggaggaggcgcagtcttgggctttggtaaatcgtccccccttgatggcaaaaccttggatctggaaatcaataaaagtgacctcccacaggctcgacccatcatccgtgtcgctgggcagcaagagggcctggtcctgctgcaggctgcccacgcgttggcagcggtaggagtaaccagagggagcatatacgccagttgggttaaagactgcttggattgaattgttggaaatgatctcgactcggcgcaaactaaaccaactctggatggacaacttgttgtaattggtaaggatgaatcttatagcaagacttctggggtttccagcatcaccaagcttcaaagacaaccatttggagttgagaccaagcctggaatcctttgctgttttcaaaacgagtttgagaacccttgctttccaaagtctcattttctacaagttattccgacaattagcaaaaaggttcagaagaaaactgccgggaaaatataacaattttttttttttgagatggagtctcactcactctgtcacccaagctggagagcaatggcgcgatctcagctcaccacaacctccacctcccaggttcaagcaattctcctgtctcagcctcctgagtagctgggattacaggcacctgccaccacgcccggctaatttttgtattttagtagagacgaggtttcaccatgttggccaggcttgtctccaactcctgacctcaggtgatccactcccttggcctcccgaagtgctgggattacaggcgtgagccaccatgcccagccaacaatttttgaagttaacttctgacttgttcctttattttagacagtaaatacttcctcaaagatgtgtgtcagggtcctatacaaaggagcctactttttttttctagcactttcttcactgcaatttgagttgtcagggtccacagttaccttctgaccaaatggctcgtctgtaaggtccagccaggtttgattcttaaatttaatcattattcttttggcccagaagagaatgcaaggaattccattgatggagacattaactgggccatgatggctgaatgcattccaaggttctttttctaaatgcccttctttgctcagattgtagttgagagctatcagggtgatgggattcataccgcaaactccagcattatgcactattctcacgtaacaaatctgcacatggaccctctgtgtgattggtattgttgtgaaattctggaatggtttcatatctccattattctgatcattcctcataaccacttctttatttgaagatgttggagaacttacattcttcctggcaaatatatggtccaaggttagtgaaagtcctataccttctctcctcaaacctttttctcccactctttctcttcactgatggccttgcatggcctacaggctccacatgttcctgtgtaactctcagaccccatctaatgccacactactcctcagtcactatgctccccttcttcactgatctttcagttcttagaaagcactagcccattctacatctgcacagagatgtcaccttaaactaccctatccagagtagccacccccatccccaagtcactatcacccatccagctatattttctctatagctctacagtatgtaaaaatcatctatttaattatttaatttacatctatctaactggtctgtcctctcacatttagaatataaactgtatcagagcagaaaccttcaccctcttaatttaaccgccatattcccggtacctacaacagcgtctggcacatagaaggcatttttaaacatccttgctgagtgaaccaatatcccagaaacctctcacagctagttcatcttacaggagaaacagtattaaagagttaattaaatggccaggcgcggtggctcacgcctgtaatcccagcacattgggaggccgaggcgggcggatcactcgaggtcaggagatcgacaccagcctggccaacatggtgaaaccccctctctactgaaaatacaaacatcagccaggcgtgatggtggaagcctgtaatcccagctactcaggaggctgaggtgggacaatcgcttgaacccgggaggcggaggttgtagtgagccaagatcgcaccactgcacaacagcctagaagacagagtgagaccctgtctcagaaaaaaataaaaataaaaataaataaatctataagtaaatgactcgccagtcaaaataaacggcaactttagggttaaaggcccaatctggctccaaagcttggggttttagttactacactacattgcttcactatattttacaatttactagctgcttataagtatgaattaaggctcagaagtctaattttccagactactcggaggactctcgccccactccactccacaaagattcagctcagcgactccttcctactctgacctagccccgcgtcccgctctcagtggcttgggcaagagc

SEQ ID NO: 19450 - RNA, 2556 nt, Homo sapiens
  source 1..2556: mol_type = other RNA
ttgaggagacatggtgggggccagcctgtgctgctaaacatagattttgctgatctgttggcttctcagtttatagcattcagccccctggctcctcagcagctccttctcttcggctgtgtctcgagctttcagctgcgagaagtgggcaggagaggcgatgagatcatattgttggtccagataccgcaggtagatgagcatgtgcagggcataggccaacaccagcagcaggatcagggacattgccaggccgatcagaaaagctggcgagaaggaggaggcgcagtcttgggctttggtaaatcgtccccccttgatggcaaaaccttggatctggaaatcaataaaagtgacctcccacaggctcgacccatcatccgtgtcgctgggcagcaagagggcctggtcctgctgcaggctgcccacgcgttggcagcggtaggagtaaccagagggagcatatacgccagttgggttaaagactgcttggattgaattgttggaaatgatctcgactcggcgcaaactaaaccaactctggatggacaacttgttgtaattggtaaggatgaatcttatagcaagacttctggggtttccagcatcaccaagcttcaaagacaaccatttggagttgagaccaagcctggaatcctttgctgttttcaaaacgagtttgagaacccttgctttccaaagtctcattttctacaagttattccgacaattagcaaaaaggttcagaagaaaactgccgggaaaatataacaattttttttttttgagatggagtctcactcactctgtcacccaagctggagagcaatggcgcgatctcagctcaccacaacctccacctcccaggttcaagcaattctcctgtctcagcctcctgagtagctgggattacaggcacctgccaccacgcccggctaatttttgtattttagtagagacgaggtttcaccatgttggccaggcttgtctccaactcctgacctcaggtgatccactcccttggcctcccgaagtgctgggattacaggcgtgagccaccatgcccagccaacaatttttgaagttaacttctgacttgttcctttattttagacagtaaatacttcctcaaagatgtgtgtcagggtcctatacaaaggagcctactttttttttctagcactttcttcactgcaatttgagttgtcagggtccacagttaccttctgaccaaatggctcgtctgtaaggtccagccaggtttgattcttaaatttaatcattattcttttggcccagaagagaatgcaaggaattccattgatggagacattaactgggccatgatggctgaatgcattccaaggttctttttctaaatgcccttctttgctcagattgtagttgagagctatcagggtgatgggattcataccgcaaactccagcattatgcactattctcacgtaacaaatctgcacatggaccctctgtgtgattggtattgttgtgaaattctggaatggtttcatatctccattattctgatcattcctcataaccacttctttatttgaagatgttggagaacttctctcctcaaacctttttctcccactctttctcttcactgatggccttgaacagcgtctggcacatagaaggcatttttaaacatccttgctgagtgaaccaatatcccagaaacctctcacagctagttcatcttacaggagaaacagtattaaagagttaattaaatggccaggcgcggtggctcacgcctgtaatcccagcacattgggaggccgaggcgggcggatcactcgaggtcaggagatcgacaccagcctggccaacatggtgaaaccccctctctactgaaaatacaaacatcagccaggcgtgatggtggaagcctgtaatcccagctactcaggaggctgaggtgggacaatcgcttgaacccgggaggcggaggttgtagtgagccaagatcgcaccactgcacaacagcctagaagacagagtgagaccctgtctcagaaaaaaataaaaataaaaataaataaatctataagtaaatgactcgccagtcaaaataaacggcaactttagggttaaaggcccaatctggctccaaagcttggggttttagttactacactacattgcttcactatattttacaatttactagctgcttataagtatgaattaaggctcagaagtctaattttccagactactcggaggactctcgccccactccactccacaaagattcagctcagcgactccttcctactctgacctagccccgcgtcccgctctcagtggcttgggcaagagcgcctgcgcggtgagcgggtcccataaaacgcattctgggattggtagtccatgttcctccggtctccagcattcaaaagaaaaagggggaaaaaaaaccatgcaaattagatatctctgaatttcttgcaaattaaataagacgcagattctggctcaggaaagtgatgcaaacgcgtcgttttcaaaggagagaccccagcc

SEQ ID NO: 19451 - RNA, 2720 nt, Homo sapiens
  source 1..2720: mol_type = other RNA
ttgaggagacatggtgggggccagcctgtgctgctaaacatagattttgctgatctgttggcttctcagtttatagcattcagccccctggctcctcagcagctccttctcttcggctgtgtctcgagctttcagctgcgagaagtgggcaggagaggcgatgagatcatattgttggtccagataccgcaggtagatgagcatgtgcagggcataggccaacaccagcagcaggatcagggacattgccaggccgatcagaaaagctggcgagaaggaggaggcgcagtcttgggctttggtaaatcgtccccccttgatggcaaaaccttggatctggaaatcaataaaagtgacctcccacaggctcgacccatcatccgtgtcgctgggcagcaagagggcctggtcctgctgcaggctgcccacgcgttggcagcggtaggagtaaccagagggagcatatacgccagttgggttaaagactgcttggattgaattgttggaaatgatctcgactcggcgcaaactaaaccaactctggatggacaacttgttgtaattggtaaggatgaatcttatagcaagacttctggggtttccagcatcaccaagcttcaaagacaaccatttggagttgagaccaagcctggaatcctttgctgttttcaaaacgagtttgagaacccttgctttccaaagtctcattttctacaagttattccgacaattagcaaaaaggttcagaagaaaactgccgggaaaatataacaattttttttttttgagatggagtctcactcactctgtcacccaagctggagagcaatggcgcgatctcagctcaccacaacctccacctcccaggttcaagcaattctcctgtctcagcctcctgagtagctgggattacaggcacctgccaccacgcccggctaatttttgtattttagtagagacgaggtttcaccatgttggccaggcttgtctccaactcctgacctcaggtgatccactcccttggcctcccgaagtgctgggattacaggcgtgagccaccatgcccagccaacaatttttgaagttaacttctgacttgttcctttattttagacagtaaatacttcctcaaagatgtgtgtcagggtcctatacaaaggagcctactttttttttctagcactttcttcactgcaatttgagttgtcagggtccacagttaccttctgaccaaatggctcgtctgtaaggtccagccaggtttgattcttaaatttaatcattattcttttggcccagaagagaatgcaaggaattccattgatggagacattaactgggccatgatggctgaatgcattccaaggttctttttctaaatgcccttctttgctcagattgtagttgagagctatcagggtgatgggattcataccgcaaactccagcattatgcactattctcacgtaacaaatctgcacatggaccctctgtgtgattggtattgttgtgaaattctggaatggtttcatatctccattattctgatcattcctcataaccacttctttatttgaagatgttggagaacttctctcctcaaacctttttctcccactctttctcttcactgatggccttgcatggcctacaggctccacatgttcctgtgtaactctcagaccccatctaatgccacactactcctcagtcactatgctccccttcttcactgatctttcagttcttagaaagcactagcccattctacatctgcacagagatgtcaccttaaactaccctatccagagtagccacccccatccccaagtcactatcacccatccagctatattttctctatagctctacagtatgtaaaaatcatctatttaattatttaatttacatctatctaactggtctgtcctctcacatttagaatataaactgtatcagagcagaaaccttcaccctcttaatttaaccgccatattcccggtacctacaacagcgtctggcacatagaaggcatttttaaacatccttgctgagtgaaccaatatcccagaaacctctcacagctagttcatcttacaggagaaacagtattaaagagttaattaaatggccaggcgcggtggctcacgcctgtaatcccagcacattgggaggccgaggcgggcggatcactcgaggtcaggagatcgacaccagcctggccaacatggtgaaaccccctctctactgaaaatacaaacatcagccaggcgtgatggtggaagcctgtaatcccagctactcaggaggctgaggtgggacaatcgcttgaacccgggaggcggaggttgtagtgagccaagatcgcaccactgcacaacagcctagaagacagagtgagaccctgtctcagaaaaaaataaaaataaaaataaataaatctataagtaaatgactcgccagtcaaaataaacggcaactttagggttaaaggcccaatctggctccaaagcttggggttttagttactacactacattgcttcactatattttacaatttactagctgcttataagtatgaattaaggctcagaagtctaattttccagactactcggaggactctcgccccactccactccacaaagattcagctcagcgactccttcctactctgacctagccccgcgtcccgctctcagtggcttgggcaagagc

SEQ ID NO: 19452 - RNA, 1099 nt, Homo sapiens
  source 1..1099: mol_type = other RNA
ttgaggagacatggtgggggccagcctgtgctgctaaacatagattttgctgatctgttggcttctcagtttatagcattcagccccctggctcctcagcagctccttctcttcggctgtgtctcgagctttcagctgcgagaagtgggcaggagaggcgatgagatcatattgttggtccagataccgcaggtagatgagcatgtgcagggcataggccaacaccagcagcaggatcagggacattgccaggccgatcagaaaagctggcgagaaggaggaggcgcagtcttgggctttggtaaatcgtccccccttgatggcaaaaccttggatctggaaatcaataaaagtgacctcccacaggctcgacccatcatccgtgtcgctgggcagcaagagggcctggtcctgctgcaggctgcccacgcgttggcagcggtaggagtaaccagagggagcatatacgccagttgggttaaagactgcttggattgaattgttggaaatgatctcgactcggcgcaaactaaaccaactctggatggacaacttgttgtaattggtaaggatgaatcttatagcaagacttctggggtttccagcatcaccaagcttcaaagacaaccatttggagttgagaccaagcctggaatcctttgctgttttcaaaacgagtttgagaacccttgctttccaaagtctcatttttctgtcacccaagctggagagcaatggcgcgatctcagctcaccacaacagcctagaagacagagtgagaccctgtctcagaaaaaaataaaaataaaaataaataaatctataagtaaatgactcgccagtcaaaataaacggcaactttagggttaaaggcccaatctggctccaaagcttggggttttagttactacactacattgcttcactatattttacaatttactagctgcttataagtatgaattaaggctcagaagtctaattttccagactactcggaggactctcgccccactccactccacaaagattcagctcagcgactccttcctactctgacctagccccgcgtcccgctctcagtggcttgggcaagagc

SEQ ID NO: 19453 - RNA, 2678 nt, Homo sapiens
  source 1..2678: mol_type = other RNA
ttgaggagacatggtgggggccagcctgtgctgctaaacatagattttgctgatctgttggcttctcagtttatagcattcagccccctggctcctcagcagctccttctcttcggctgtgtctcgagctttcagctgcgagaagtgggcaggagaggcgatgagatcatattgttggtccagataccgcaggtagatgagcatgtgcagggcataggccaacaccagcagcaggatcagggacattgccaggccgatcagaaaagctggcgagaaggaggaggcgcagtcttgggctttggtaaatcgtccccccttgatggcaaaaccttggatctggaaatcaataaaagtgacctcccacaggctcgacccatcatccgtgtcgctgggcagcaagagggcctggtcctgctgcaggctgcccacgcgttggcagcggtaggagtaaccagagggagcatatacgccagttgggttaaagactgcttggattgaattgttggaaatgatctcgactcggcgcaaactaaaccaactctggatggacaacttgttgtaattggtaaggatgaatcttatagcaagacttctggggtttccagcatcaccaagcttcaaagacaaccatttggagttgagaccaagcctggaatcctttgctgttttcaaaacgagtttgagaacccttgctttccaaagtctcatttttctgtcacccaagctggagagcaatggcgcgatctcagctcaccacaacctccacctcccaggttcaagcaattctcctgtctcagcctcctgagtagctgggattacaggcacctgccaccacgcccggctaatttttgtattttagtagagacgaggtttcaccatgttggccaggcttgtctccaactcctgacctcaggtgatccactcccttggcctcccgaagtgctgggattacaggcgtgagccaccatgcccagccaacaatttttgaagttaacttctgacttgttcctttattttagacagtaaatacttcctcaaagatgtgtgtcagggtcctatacaaaggagcctactttttttttctagcactttcttcactgcaatttgagttgtcagggtccacagttaccttctgaccaaatggctcgtctgtaaggtccagccaggtttgattcttaaatttaatcattattcttttggcccagaagagaatgcaaggaattccattgatggagacattaactgggccatgatggctgaatgcattccaaggttctttttctaaatgcccttctttgctcagattgtagttgagagctatcagggtgatgggattcataccgcaaactccagcattatgcactattctcacgtaacaaatctgcacatggaccctctgtgtgattggtattgttgtgaaattctggaatggtttcatatctccattattctgatcattcctcataaccacttctttatttgaagatgttggagaacttacattcttcctggcaaatatatggtccaaggttagtgaaagtcctataccttctctcctcaaacctttttctcccactctttctcttcactgatggccttgcatggcctacaggctccacatgttcctgtgtaactctcagaccccatctaatgccacactactcctcagtcactatgctccccttcttcactgatctttcagttcttagaaagcactagcccattctacatctgcacagagatgtcaccttaaactaccctatccagagtagccacccccatccccaagtcactatcacccatccagctatattttctctatagctctacagtatgtaaaaatcatctatttaattatttaatttacatctatctaactggtctgtcctctcacatttagaatataaactgtatcagagcagaaaccttcaccctcttaatttaaccgccatattcccggtacctacaacagcgtctggcacatagaaggcatttttaaacatccttgctgagtgaaccaatatcccagaaacctctcacagctagttcatcttacaggagaaacagtattaaagagttaattaaatggccaggcgcggtggctcacgcctgtaatcccagcacattgggaggccgaggcgggcggatcactcgaggtcaggagatcgacaccagcctggccaacatggtgaaaccccctctctactgaaaatacaaacatcagccaggcgtgatggtggaagcctgtaatcccagctactcaggaggctgaggtgggacaatcgcttgaacccgggaggcggaggttgtagtgagccaagatcgcaccactgcacaacagcctagaagacagagtgagaccctgtctcagaaaaaaataaaaataaaaataaataaatctataagtaaatgactcgccagtcaaaataaacggcaactttagggttaaaggcccaatctggctccaaagcttggggttttagttactacactacattgcttcactatattttacaatttactagctgcttataagtatgaattaaggctcagaagtctaattttccagactactcggaggactctcgccccactccactccacaaagattcagctcagcgactccttcctactctgacctagccccgcgtcccgctctcagtggcttgggcaagagc

SEQ ID NO: 19454 - RNA, 2952 nt, Homo sapiens
  source 1..2952: mol_type = other RNA
ttgaggagacatggtgggggccagcctgtgctgctaaacatagattttgctgatctgttggcttctcagtttatagcattcagccccctggctcctcagcagctccttctcttcggctgtgtctcgagctttcagctgcgagaagtgggcaggagaggcgatgagatcatattgttggtccagataccgcaggtagatgagcatgtgcagggcataggccaacaccagcagcaggatcagggacattgccaggccgatcagaaaagctggcgagaaggaggaggcgcagtcttgggctttggtaaatcgtccccccttgatggcaaaaccttggatctggaaatcaataaaagtgacctcccacaggctcgacccatcatccgtgtcgctgggcagcaagagggcctggtcctgctgcaggctgcccacgcgttggcagcggtaggagtaaccagagggagcatatacgccagttgggttaaagactgcttggattgaattgttggaaatgatctcgactcggcgcaaactaaaccaactctggatggacaacttgttgtaattggtaaggatgaatcttatagcaagacttctggggtttccagcatcaccaagcttcaaagacaaccatttggagttgagaccaagcctggaatcctttgctgttttcaaaacgagtttgagaacccttgctttccaaagtctcatttttctgtcacccaagctggagagcaatggcgcgatctcagctcaccacaacctccacctcccaggttcaagcaattctcctgtctcagcctcctgagtagctgggattacaggcacctgccaccacgcccggctaatttttgtattttagtagagacgaggtttcaccatgttggccaggcttgtctccaactcctgacctcaggtgatccactcccttggcctcccgaagtgctgggattacaggcgtgagccaccatgcccagccaacaatttttgaagttaacttctgacttgttcctttattttagacagtaaatacttcctcaaagatgtgtgtcagggtcctatacaaaggagcctactttttttttctagcactttcttcactgcaatttgagttgtcagggtccacagttaccttctgaccaaatggctcgtctgtaaggtccagccaggtttgattcttaaatttaatcattattcttttggcccagaagagaatgcaaggaattccattgatggagacattaactgggccatgatggctgaatgcattccaaggttctttttctaaatgcccttctttgctcagattgtagttgagagctatcagggtgatgggattcataccgcaaactccagcattatgcactattctcacgtaacaaatctgcacatggaccctctgtgtgattggtattgttgtgaaattctggaatggtttcatatctccattattctgatcattcctcataaccacttctttatttgaagatgttggagaacttctctcctcaaacctttttctcccactctttctcttcactgatggccttgccaagtgctgaggtcaaaaatcatagtgctgtaattaactcctctctcacatcctacagtcctgagcaaattctgttcattctaccaccaaacagtgtatctgacccaaccactttttactgtctccactgagggtccaagctatcaccatctctcatctgaactattgcaataccttcccaagtggcctcccagattcatgtctttttctcctctcaacagccagagtaaccccataaaaatataaatcttattttgctacctactcccaagctcaaaactttacaatggctttaaatcaccagaagagtagaaaaaggctttaccatggcctacaggctccacatgttcctgtgtaactctcagaccccatctaatgccacactactcctcagtcactatgctccccttcttcactgatctttcagttcttagaaagcactagcccattctacatctgcacagagatgtcaccttaaactaccctatccagagtagccacccccatccccaagtcactatcacccatccagctatattttctctatagctctacagtatgtaaaaatcatctatttaattatttaatttacatctatctaactggtctgtcctctcacatttagaatataaactgtatcagagcagaaaccttcaccctcttaatttaaccgccatattcccggtacctacaacagcgtctggcacatagaaggcatttttaaacatccttgctgagtgaaccaatatcccagaaacctctcacagctagttcatcttacaggagaaacagtattaaagagttaattaaatggccaggcgcggtggctcacgcctgtaatcccagcacattgggaggccgaggcgggcggatcactcgaggtcaggagatcgacaccagcctggccaacatggtgaaaccccctctctactgaaaatacaaacatcagccaggcgtgatggtggaagcctgtaatcccagctactcaggaggctgaggtgggacaatcgcttgaacccgggaggcggaggttgtagtgagccaagatcgcaccactgcacaacagcctagaagacagagtgagaccctgtctcagaaaaaaataaaaataaaaataaataaatctataagtaaatgactcgccagtcaaaataaacggcaactttagggttaaaggcccaatctggctccaaagcttggggttttagttactacactacattgcttcactatattttacaatttactagctgcttataagtatgaattaaggctcagaagtctaattttccagactactcggaggactctcgccccactccactccacaaagattcagctcagcgactccttcctactctgacctagccccgcgtcccgctctcagtggcttgggcaagagc

SEQ ID NO: 19455 - RNA, 2964 nt, Homo sapiens
  source 1..2964: mol_type = other RNA
ttgaggagacatggtgggggccagcctgtgctgctaaacatagattttgctgatctgttggcttctcagtttatagcattcagccccctggctcctcagcagctccttctcttcggctgtgtctcgagctttcagctgcgagaagtgggcaggagaggcgatgagatcatattgttggtccagataccgcaggtagatgagcatgtgcagggcataggccaacaccagcagcaggatcagggacattgccaggccgatcagaaaagctggcgagaaggaggaggcgcagtcttgggctttggtaaatcgtccccccttgatggcaaaaccttggatctggaaatcaataaaagtgacctcccacaggctcgacccatcatccgtgtcgctgggcagcaagagggcctggtcctgctgcaggctgcccacgcgttggcagcggtaggagtaaccagagggagcatatacgccagttgggttaaagactgcttggattgaattgttggaaatgatctcgactcggcgcaaactaaaccaactctggatggacaacttgttgtaattggtaaggatgaatcttatagcaagacttctggggtttccagcatcaccaagcttcaaagacaaccatttggagttgagaccaagcctggaatcctttgctgttttcaaaacgagtttgagaacccttgctttccaaagtctcatttttctgtcacccaagctggagagcaatggcgcgatctcagctcaccacaacctccacctcccaggttcaagcaattctcctgtctcagcctcctgagtagctgggattacaggcacctgccaccacgcccggctaatttttgtattttagtagagacgaggtttcaccatgttggccaggcttgtctccaactcctgacctcaggtgatccactcccttggcctcccgaagtgctgggattacaggcgtgagccaccatgcccagccaacaatttttgaagttaacttctgacttgttcctttattttagacagtaaatacttcctcaaagatgtgtgtcagggtcctatacaaaggagcctactttttttttctgaaatgacaaaaaaagttgaatgcagagttaacagaacgcaatagccctaggggcttcctcaaactgagagatcaacttacctagcactttcttcactgcaatttgagttgtcagggtccacagttaccttctgaccaaatggctcgtctgtaaggtccagccaggtttgattcttaaatttaatcattattcttttggcccagaagagaatgcaaggaattccattgatggagacattaactgggccatgatggctgaatgcattccaaggttctttttctaaatgcccttctttgctcagattgtagttgagagctatcagggtgatgggattcataccgcaaactccagcattatgcactattctcacgtaacaaatctgcacatggaccctctgtgtgattggtattgttgtgaaattctggaatggtttcatatctccattattctgatcattcctcataaccacttctttatttgaagatgttggagaacttacattcttcctggcaaatatatggtccaaggttagtgaaagtcctataccttctctcctcaaacctttttctcccactctttctcttcactgatggccttgcatggcctacaggctccacatgttcctgtgtaactctcagaccccatctaatgccacactactcctcagtcactatgctccccttcttcactgatctttcagttcttagaaagcactagcccattctacatctgcacagagatgtcaccttaaactaccctatccagagtagccacccccatccccaagtcactatcacccatccagctatattttctctatagctctacagtatgtaaaaatcatctatttaattatttaatttacatctatctaactggtctgtcctctcacatttagaatataaactgtatcagagcagaaaccttcaccctcttaatttaaccgccatattcccggtacctacaacagcgtctggcacatagaaggcatttttaaacatccttgctgagtgaaccaatatcccagaaacctctcacagctagttcatcttacaggagaaacagtattaaagagttaattaaatggccaggcgcggtggctcacgcctgtaatcccagcacattgggaggccgaggcgggcggatcactcgaggtcaggagatcgacaccagcctggccaacatggtgaaaccccctctctactgaaaatacaaacatcagccaggcgtgatggtggaagcctgtaatcccagctactcaggaggctgaggtgggacaatcgcttgaacccgggaggcggaggttgtagtgagccaagatcgcaccactgcacaacagcctagaagacagagtgagaccctgtctcagaaaaaaataaaaataaaaataaataaatctataagtaaatgactcgccagtcaaaataaacggcaactttagggttaaaggcccaatctggctccaaagcttggggttttagttactacactacattgcttcactatattttacaatttactagctgcttataagtatgaattaaggctcagaagtctaattttccagactactcggaggactctcgccccactccactccacaaagattcagctcagcgactccttcctactctgacctagccccgcgtcccgctctcagtggcttgggcaagagcgcctgcgcggtgagcgggtcccataaaacgcattctgggattggtagtccatgttcctccggtctccagcattcaaaagaaaaagggggaaaaaaaaccatgcaaattagatatctctgaatttcttgcaaattaaataagacgcagattctggctcaggaaagtgatgcaaacgcgtcgttttcaaaggagagaccccagcc

SEQ ID NO: 19456 - RNA, 1113 nt, Homo sapiens
  source 1..1113: mol_type = other RNA
ttgaggagacatggtgggggccagcctgtgctgctaaacatagattttgctgatctgttggcttctcagtttatagcattcagccccctggctcctcagcagctccttctcttcggctgtgtctcgagctttcagctgcgagaagtgggcaggagaggcgatgagatcatattgttggtccagataccgcaggtagatgagcatgtgcagggcataggccaacaccagcagcaggatcagggacattgccaggccgatcagaaaagctggcgagaaggaggaggcgcagtcttgggctttggtaaatcgtccccccttgatggcaaaaccttggatctggaaatcaataaaagtgacctcccacaggctcgacccatcatccgtgtcgctgggcagcaagagggcctggtcctgctgcaggctgcccacgcgttggcagcggtaggagtaaccagagggagcatatacgccagttgggttaaagactgcttggattgaattgttggaaatgatctcgactcggcgcaaactaaaccaactctggatggacaacttgttgtaattggtaaggatgaatcttatagcaagacttctggggtttccagcatcaccaagcttcaaagacaaccatttggagttgagaccaagcctggaatcctttgctgttttcaaaacgagtttgagaacccttgctttccaaagtctcatttttctgtcacccaagctggagagcaatggcgcgatctcagctcaccacaacctccactgcacaacagcctagaagacagagtgagaccctgtctcagaaaaaaataaaaataaaaataaataaatctataagtaaatgactcgccagtcaaaataaacggcaactttagggttaaaggcccaatctggctccaaagcttggggttttagttactacactacattgcttcactatattttacaatttactagctgcttataagtatgaattaaggctcagaagtctaattttccagactactcggaggactctcgccccactccactccacaaagattcagctcagcgactccttcctactctgacctagccccgcgtcccgctctcagtggcttgggcaagagc

SEQ ID NO: 19457 - RNA, 2678 nt, Homo sapiens
  source 1..2678: mol_type = other RNA
ttgaggagacatggtgggggccagcctgtgctgctaaacatagattttgctgatctgttggcttctcagtttatagcattcagccccctggctcctcagcagctccttctcttcggctgtgtctcgagctttcagctgcgagaagtgggcaggagaggcgatgagatcatattgttggtccagataccgcaggtagatgagcatgtgcagggcataggccaacaccagcagcaggatcagggacattgccaggccgatcagaaaagctggcgagaaggaggaggcgcagtcttgggctttggtaaatcgtccccccttgatggcaaaaccttggatctggaaatcaataaaagtgacctcccacaggctcgacccatcatccgtgtcgctgggcagcaagagggcctggtcctgctgcaggctgcccacgcgttggcagcggtaggagtaaccagagggagcatatacgccagttgggttaaagactgcttggattgaattgttggaaatgatctcgactcggcgcaaactaaaccaactctggatggacaacttgttgtaattggtaaggatgaatcttatagcaagacttctggggtttccagcatcaccaagcttcaaagacaacctaagaaaaggaaacaacgcagtcatttggagttgagaccaagcctggaatcctttgctgttttcaaaacgagtttgagaacccttgctttccaaagtctcatttttctgtcacccaagctggagagcaatggcgcgatctcagctcaccacaacctccacctcccaggttcaagcaattctcctgtctcagcctcctgagtagctgggattacaggcacctgccaccacgcccggctaatttttgtattttagtagagacgaggtttcaccatgttggccaggcttgtctccaactcctgacctcaggtgatccactcccttggcctcccgaagtgctgggattacaggcgtgagccaccatgcccagccaacaatttttgaagttaacttctgacttgttcctttattttagacagtaaatacttcctcaaagatgtgtgtcagggtcctatacaaaggagcctactttttttttctagcactttcttcactgcaatttgagttgtcagggtccacagttaccttctgaccaaatggctcgtctgtaaggtccagccaggtttgattcttaaatttaatcattattcttttggcccagaagagaatgcaaggaattccattgatggagacattaactgggccatgatggctgaatgcattccaaggttctttttctaaatgcccttctttgctcagattgtagttgagagccgcaaactccagcattatgcactattctcacgtaacaaatctgcacatggaccctctgtgtgattggtattgttgtgaaattctggaatggtttcatatctccattattctgatcattcctcataaccacttctttatttgaagatgttggagaacttacattcttcctggcaaatatatggtccaaggttagtgaaagtcctataccttctctcctcaaacctttttctcccactctttctcttcactgatggccttgcatggcctacaggctccacatgttcctgtgtaactctcagaccccatctaatgccacactactcctcagtcactatgctccccttcttcactgatctttcagttcttagaaagcactagcccattctacatctgcacagagatgtcaccttaaactaccctatccagagtagccacccccatccccaagtcactatcacccatccagctatattttctctatagctctacagtatgtaaaaatcatctatttaattatttaatttacatctatctaactggtctgtcctctcacatttagaatataaactgtatcagagcagaaaccttcaccctcttaatttaaccgccatattcccggtacctacaacagcgtctggcacatagaaggcatttttaaacatccttgctgagtgaaccaatatcccagaaacctctcacagctagttcatcttacaggagaaacagtattaaagagttaattaaatggccaggcgcggtggctcacgcctgtaatcccagcacattgggaggccgaggcgggcggatcactcgaggtcaggagatcgacaccagcctggccaacatggtgaaaccccctctctactgaaaatacaaacatcagccaggcgtgatggtggaagcctgtaatcccagctactcaggaggctgaggtgggacaatcgcttgaacccgggaggcggaggttgtagtgagccaagatcgcaccactgcacaacagcctagaagacagagtgagaccctgtctcagaaaaaaataaaaataaaaataaataaatctataagtaaatgactcgccagtcaaaataaacggcaactttagggttaaaggcccaatctggctccaaagcttggggttttagttactacactacattgcttcactatattttacaatttactagctgcttataagtatgaattaaggctcagaagtctaattttccagactactcggaggactctcgccccactccactccacaaagattcagctcagcgactccttcctactctgacctagccccgcgtcccgctctcagtggcttgggcaagagc

SEQ ID NO: 19458 - RNA, 2257 nt, Homo sapiens
  source 1..2257: mol_type = other RNA
ttgaggagacatggtgggggccagcctgtgctgctaaacatagattttgctgatctgttggcttctcagtttatagcattcagccccctggctcctcagcagctccttctcttcggctgtgtctcgagctttcagctgcgagaagtgggcaggagaggcgatgagatcatattgttggtccagataccgcaggtagatgagcatgtgcagggcataggccaacaccagcagcaggatcagggacattgccaggccgatcagaaaagctggcgagaaggaggaggcgcagtcttgggctttggtaaatcgtccccccttgatggcaaaaccttggatctggaaatcaataaaagtgacctcccacaggctcgacccatcatccgtgtcgctgggcagcaagagggcctggtcctgctgcaggctgcccacgcgttggcagcggtaggagtaaccagagggagcatatacgccagttgggttaaagactgcttggattgaattgttggaaatgatctcgactcggcgcaaactaaaccaactctggatggacaacttgttgtaattggtaaggatgaatcttatagcaagacttctggggtttccagcatcaccaagcttcaaagacaacctagcactttcttcactgcaatttgagttgtcagggtccacagttaccttctgaccaaatggctcgtctgtaaggtccagccaggtttgattcttaaatttaatcattattcttttggcccagaagagaatgcaaggaattccattgatggagacattaactgggccatgatggctgaatgcattccaaggttctttttctaaatgcccttctttgctcagattgtagttgagagcctgtgtgattggtattgttgtgaaattctggaatggtttcatatctccattattctgatcattcctcataaccacttctttatttgaagatgttggagaacttacattcttccatggcctacaggctccacatgttcctgtgtaactctcagaccccatctaatgccacactactcctcagtcactatgctccccttcttcactgatctttcagttcttagaaagcactagcccattctacatctgcacagagatgtcaccttaaactaccctatccagagtagccacccccatccccaagtcactatcacccatccagctatattttctctatagctctacagtatgtaaaaatcatctatttaattatttaatttacatctatctaactggtctgtcctctcacatttagaatataaactgtatcagagcagaaaccttcaccctcttaatttaaccgccatattcccggtacctacaacagcgtctggcacatagaaggcatttttaaacatccttgctgagtgaaccaatatcccagaaacctctcacagctagttcatcttacaggagaaacagtattaaagagttaattaaatggccaggcgcggtggctcacgcctgtaatcccagcacattgggaggccgaggcgggcggatcactcgaggtcaggagatcgacaccagcctggccaacatggtgaaaccccctctctactgaaaatacaaacatcagccaggcgtgatggtggaagcctgtaatcccagctactcaggaggctgaggtgggacaatcgcttgaacccgggaggcggaggttgtagtgagccaagatcgcaccactgcacaacagcctagaagacagagtgagaccctgtctcagaaaaaaataaaaataaaaataaataaatctataagtaaatgactcgccagtcaaaataaacggcaactttagggttaaaggcccaatctggctccaaagcttggggttttagttactacactacattgcttcactatattttacaatttactagctgcttataagtatgaattaaggctcagaagtctaattttccagactactcggaggactctcgccccactccactccacaaagattcagctcagcgactccttcctactctgacctagccccgcgtcccgctctcagtggcttgggcaagagcgcctgcgcggtgagcgggtcccataaaacgcattctgggattggtagtccatgttcctccggtctccagcattcaaaagaaaaagggggaaaaaaaaccatgcaaattagatatctctgaatttcttgcaaattaaataagacgcagattctggctcaggaaagtgatgcaaacgcgtcgttttcaaaggagagaccccagcc

SEQ ID NO: 19459 - RNA, 2203 nt, Homo sapiens
  source 1..2203: mol_type = other RNA
ttgaggagacatggtgggggccagcctgtgctgctaaacatagattttgctgatctgttggcttctcagtttatagcattcagccccctggctcctcagcagctccttctcttcggctgtgtctcgagctttcagctgcgagaagtgggcaggagaggcgatgagatcatattgttggtccagataccgcaggtagatgagcatgtgcagggcataggccaacaccagcagcaggatcagggacattgccaggccgatcagaaaagctggcgagaaggaggaggcgcagtcttgggctttggtaaatcgtccccccttgatggcaaaaccttggatctggaaatcaataaaagtgacctcccacaggctcgacccatcatccgtgtcgctgggcagcaagagggcctggtcctgctgcaggctgcccacgcgttggcagcggtaggagtaaccagagggagcatatacgccagttgggttaaagactgcttggattgaattgttggaaatgatctcgactcggcgcaaactaaaccaactctggatggacaacttgttgtaattggtaaggatgaatcttatagcaagacttctggggtttccagcatcaccaagcttcaaagacaacctagcactttcttcactgcaatttgagttgtcagggtccacagttaccttctgaccaaatggctcgtctgtaaggtccagccaggtttgattcttaaatttaatcattattcttttggcccagaagagaatgcaaggaattccattgatggagacattaactgggccatgatggctgaatgcattccaaggttctttttctaaatgcccttctttgctcagattgtagttgagagcctgtgtgattggtattgttgtgaaattctggaatggtttcatatctccattattctgatcattcctcataaccacttctttatttgaagatgttggagaacttacattcttcctggcaaatatatggtccaaggttagtgaaagtcctataccagtgagcaagctgacaccaggcaggttattttccctctagagccttgtttcctcatcttctctcctcaaacctttttctcccactctttctcttcactgatggccttgcatggcctacaggctccacatgttcctgtgtaactctcagaccccatctaatgccacactactcctcagtcactatgctccccttcttcactgatctttcagttcttagaaagcactagcccattctacatctgcacagagatgtcaccttaaactaccctatccagagtagccacccccatccccaagtcactatcacccatccagctatattttctctatagctctacagtatgtaaaaatcatctatttaattatttaatttacatctatctaactggtctgtcctctcacatttagaatataaactgtatcagagcagaaaccttcaccctcttaatttaaccgccatattcccggtacctacaacagcgtctggcacatagaaggcatttttaaacatccttgctgagtgaaccaatatcccagaaacctctcacagctagttcatcttacaggagaaacagtattaaagagttaattaaatggccaggcgcggtggctcacgcctgtaatcccagcacattgggaggccgaggcgggcggatcactcgaggtcaggagatcgacaccagcctggccaacatggtgaaaccccctctctactgaaaatacaaacatcagccaggcgtgatggtggaagcctgtaatcccagctactcaggaggctgaggtgggacaatcgcttgaacccgggaggcggaggttgtagtgagccaagatcgcaccactgcacaacagcctagaagacagagtgagaccctgtctcagaaaaaaataaaaataaaaataaataaatctataagtaaatgactcgccagtcaaaataaacggcaactttagggttaaaggcccaatctggctccaaagcttggggttttagttactacactacattgcttcactatattttacaatttactagctgcttataagtatgaattaaggctcagaagtctaattttccagactactcggaggactctcgccccactccactccacaaagattcagctcagcgactccttcctactctgacctagccccgcgtcccgctctcagtggcttgggcaagagc

SEQ ID NO: 19460 - RNA, 2146 nt, Homo sapiens
  source 1..2146: mol_type = other RNA
ttgaggagacatggtgggggccagcctgtgctgctaaacatagattttgctgatctgttggcttctcagtttatagcattcagccccctggctcctcagcagctccttctcttcggctgtgtctcgagctttcagctgcgagaagtgggcaggagaggcgatgagatcatattgttggtccagataccgcaggtagatgagcatgtgcagggcataggccaacaccagcagcaggatcagggacattgccaggccgatcagaaaagctggcgagaaggaggaggcgcagtcttgggctttggtaaatcgtccccccttgatggcaaaaccttggatctggaaatcaataaaagtgacctcccacaggctcgacccatcatccgtgtcgctgggcagcaagagggcctggtcctgctgcaggctgcccacgcgttggcagcggtaggagtaaccagagggagcatatacgccagttgggttaaagactgcttggattgaattgttggaaatgatctcgactcggcgcaaactaaaccaactctggatggacaacttgttgtaattggtaaggatgaatcttatagcaagacttctggggtttccagcatcaccaagcttcaaagacaacctagcactttcttcactgcaatttgagttgtcagggtccacagttaccttctgaccaaatggctcgtctgtaaggtccagccaggtttgattcttaaatttaatcattattcttttggcccagaagagaatgcaaggaattccattgatggagacattaactgggccatgatggctgaatgcattccaaggttctttttctaaatgcccttctttgctcagattgtagttgagagcctgtgtgattggtattgttgtgaaattctggaatggtttcatatctccattattctgatcattcctcataaccacttctttatttgaagatgttggagaacttacattcttcctggcaaatatatggtccaaggttagtgaaagtcctataccttctctcctcaaacctttttctcccactctttctcttcactgatggccttgcatggcctacaggctccacatgttcctgtgtaactctcagaccccatctaatgccacactactcctcagtcactatgctccccttcttcactgatctttcagttcttagaaagcactagcccattctacatctgcacagagatgtcaccttaaactaccctatccagagtagccacccccatccccaagtcactatcacccatccagctatattttctctatagctctacagtatgtaaaaatcatctatttaattatttaatttacatctatctaactggtctgtcctctcacatttagaatataaactgtatcagagcagaaaccttcaccctcttaatttaaccgccatattcccggtacctacaacagcgtctggcacatagaaggcatttttaaacatccttgctgagtgaaccaatatcccagaaacctctcacagctagttcatcttacaggagaaacagtattaaagagttaattaaatggccaggcgcggtggctcacgcctgtaatcccagcacattgggaggccgaggcgggcggatcactcgaggtcaggagatcgacaccagcctggccaacatggtgaaaccccctctctactgaaaatacaaacatcagccaggcgtgatggtggaagcctgtaatcccagctactcaggaggctgaggtgggacaatcgcttgaacccgggaggcggaggttgtagtgagccaagatcgcaccactgcacaacagcctagaagacagagtgagaccctgtctcagaaaaaaataaaaataaaaataaataaatctataagtaaatgactcgccagtcaaaataaacggcaactttagggttaaaggcccaatctggctccaaagcttggggttttagttactacactacattgcttcactatattttacaatttactagctgcttataagtatgaattaaggctcagaagtctaattttccagactactcggaggactctcgccccactccactccacaaagattcagctcagcgactccttcctactctgacctagccccgcgtcccgctctcagtggcttgggcaagagc

SEQ ID NO: 19461 - RNA, 2090 nt, Homo sapiens
  source 1..2090: mol_type = other RNA
ttgaggagacatggtgggggccagcctgtgctgctaaacatagattttgctgatctgttggcttctcagtttatagcattcagccccctggctcctcagcagctccttctcttcggctgtgtctcgagctttcagctgcgagaagtgggcaggagaggcgatgagatcatattgttggtccagataccgcaggtagatgagcatgtgcagggcataggccaacaccagcagcaggatcagggacattgccaggccgatcagaaaagctggcgagaaggaggaggcgcagtcttgggctttggtaaatcgtccccccttgatggcaaaaccttggatctggaaatcaataaaagtgacctcccacaggctcgacccatcatccgtgtcgctgggcagcaagagggcctggtcctgctgcaggctgcccacgcgttggcagcggtaggagtaaccagagggagcatatacgccagttgggttaaagactgcttggattgaattgttggaaatgatctcgactcggcgcaaactaaaccaactctggatggacaacttgttgtaattggtaaggatgaatcttatagcaagacttctggggtttccagcatcaccaagcttcaaagacaacctagcactttcttcactgcaatttgagttgtcagggtccacagttaccttctgaccaaatggctcgtctgtaaggtccagccaggtttgattcttaaatttaatcattattcttttggcccagaagagaatgcaaggaattccattgatggagacattaactgggccatgatggctgaatgcattccaaggttctttttctaaatgcccttctttgctcagattgtagttgagagcctgtgtgattggtattgttgtgaaattctggaatggtttcatatctccattattctgatcattcctcataaccacttctttatttgaagatgttggagaacttctctcctcaaacctttttctcccactctttctcttcactgatggccatggcctacaggctccacatgttcctgtgtaactctcagaccccatctaatgccacactactcctcagtcactatgctccccttcttcactgatctttcagttcttagaaagcactagcccattctacatctgcacagagatgtcaccttaaactaccctatccagagtagccacccccatccccaagtcactatcacccatccagctatattttctctatagctctacagtatgtaaaaatcatctatttaattatttaatttacatctatctaactggtctgtcctctcacatttagaatataaactgtatcagagcagaaaccttcaccctcttaatttaaccgccatattcccggtacctacaacagcgtctggcacatagaaggcatttttaaacatccttgctgagtgaaccaatatcccagaaacctctcacagctagttcatcttacaggagaaacagtattaaagagttaattaaatggccaggcgcggtggctcacgcctgtaatcccagcacattgggaggccgaggcgggcggatcactcgaggtcaggagatcgacaccagcctggccaacatggtgaaaccccctctctactgaaaatacaaacatcagccaggcgtgatggtggaagcctgtaatcccagctactcaggaggctgaggtgggacaatcgcttgaacccgggaggcggaggttgtagtgagccaagatcgcaccactgcacaacagcctagaagacagagtgagaccctgtctcagaaaaaaataaaaataaaaataaataaatctataagtaaatgactcgccagtcaaaataaacggcaactttagggttaaaggcccaatctggctccaaagcttggggttttagttactacactacattgcttcactatattttacaatttactagctgcttataagtatgaattaaggctcagaagtctaattttccagactactcggaggactctcgccccactccactccacaaagattcagctcagcgactccttcctactctgacctagccccgcgtcccgctctcagtggcttgggcaagagc

SEQ ID NO: 19462 - RNA, 1727 nt, Homo sapiens
  source 1..1727: mol_type = other RNA
ttgaggagacatggtgggggccagcctgtgctgctaaacatagattttgctgatctgttggcttctcagtttatagcattcagccccctggctcctcagcagctccttctcttcggctgtgtctcgagctttcagctgcgagaagtgggcaggagaggcgatgagatcatattgttggtccagataccgcaggtagatgagcatgtgcagggcataggccaacaccagcagcaggatcagggacattgccaggccgatcagaaaagctggcgagaaggaggaggcgcagtcttgggctttggtaaatcgtccccccttgatggcaaaaccttggatctggaaatcaataaaagtgacctcccacaggctcgacccatcatccgtgtcgctgggcagcaagagggcctggtcctgctgcaggctgcccacgcgttggcagcggtaggagtaaccagagggagcatatacgccagttgggttaaagactgcttggattgaattgttggaaatgatctcgactcggcgcaaactaaaccaactctggatggacaacttgttgtaattggtaaggatgaatcttatagcaagacttctggggtttccagcatcaccaagcttcaaagacaacctagcactttcttcactgcaatttgagttgtcagggtccacagttaccttctgaccaaatggctcgtctgtaaggtccagccaggtttgattcttaaatttaatcattattcttttggcccagaagagaatgcaaggaattccattgatggagacattaactgggccatgatggctgaatgcattccaaggttctttttctaaatgcccttctttgctcagattgtagttgagagcctgtgtgattggtattgttgtgaaattctggaatggtttcatatctccattattctgatcattcctcataaccacttctttatttgaagatgttggagaacttctctcctcaaacctttttctcccactctttctcttcactgatggccttgaacagcgtctggcacatagaaggcatttttaaacatccttgctgagtgaaccaatatcccagaaacctctcacagctagttcatcttacaggagaaacagtattaaagagttaattaaatggccaggcgcggtggctcacgcctgtaatcccagcacattgggaggccgaggcgggcggatcactcgaggtcaggagatcgacaccagcctggccaacatggtgaaaccccctctctactgaaaatacaaacatcagccaggcgtgatggtggaagcctgtaatcccagctactcaggaggctgaggtgggacaatcgcttgaacccgggaggcggaggttgtagtgagccaagatcgcaccactgcacaacagcctagaagacagagtgagaccctgtctcagaaaaaaataaaaataaaaataaataaatctataagtaaatgactcgccagtcaaaataaacggcaactttagggttaaaggcccaatctggctccaaagcttggggttttagttactacactacattgcttcactatattttacaatttactagctgcttataagtatgaattaaggctcagaagtctaattttccagactactcggaggactctcgccccactccactccacaaagattcagctcagcgactccttcctactctgacctagccccgcgtcccgctctcagtggcttgggcaagagc

SEQ ID NO: 19463 - RNA, 2094 nt, Homo sapiens
  source 1..2094: mol_type = other RNA
ttgaggagacatggtgggggccagcctgtgctgctaaacatagattttgctgatctgttggcttctcagtttatagcattcagccccctggctcctcagcagctccttctcttcggctgtgtctcgagctttcagctgcgagaagtgggcaggagaggcgatgagatcatattgttggtccagataccgcaggtagatgagcatgtgcagggcataggccaacaccagcagcaggatcagggacattgccaggccgatcagaaaagctggcgagaaggaggaggcgcagtcttgggctttggtaaatcgtccccccttgatggcaaaaccttggatctggaaatcaataaaagtgacctcccacaggctcgacccatcatccgtgtcgctgggcagcaagagggcctggtcctgctgcaggctgcccacgcgttggcagcggtaggagtaaccagagggagcatatacgccagttgggttaaagactgcttggattgaattgttggaaatgatctcgactcggcgcaaactaaaccaactctggatggacaacttgttgtaattggtaaggatgaatcttatagcaagacttctggggtttccagcatcaccaagcttcaaagacaacctagcactttcttcactgcaatttgagttgtcagggtccacagttaccttctgaccaaatggctcgtctgtaaggtccagccaggtttgattcttaaatttaatcattattcttttggcccagaagagaatgcaaggaattccattgatggagacattaactgggccatgatggctgaatgcattccaaggttctttttctaaatgcccttctttgctcagattgtagttgagagcctgtgtgattggtattgttgtgaaattctggaatggtttcatatctccattattctgatcattcctcataaccacttctttatttgaagatgttggagaacttctctcctcaaacctttttctcccactctttctcttcactgatggccttgcatggcctacaggctccacatgttcctgtgtaactctcagaccccatctaatgccacactactcctcagtcactatgctccccttcttcactgatctttcagttcttagaaagcactagcccattctacatctgcacagagatgtcaccttaaactaccctatccagagtagccacccccatccccaagtcactatcacccatccagctatattttctctatagctctacagtatgtaaaaatcatctatttaattatttaatttacatctatctaactggtctgtcctctcacatttagaatataaactgtatcagagcagaaaccttcaccctcttaatttaaccgccatattcccggtacctacaacagcgtctggcacatagaaggcatttttaaacatccttgctgagtgaaccaatatcccagaaacctctcacagctagttcatcttacaggagaaacagtattaaagagttaattaaatggccaggcgcggtggctcacgcctgtaatcccagcacattgggaggccgaggcgggcggatcactcgaggtcaggagatcgacaccagcctggccaacatggtgaaaccccctctctactgaaaatacaaacatcagccaggcgtgatggtggaagcctgtaatcccagctactcaggaggctgaggtgggacaatcgcttgaacccgggaggcggaggttgtagtgagccaagatcgcaccactgcacaacagcctagaagacagagtgagaccctgtctcagaaaaaaataaaaataaaaataaataaatctataagtaaatgactcgccagtcaaaataaacggcaactttagggttaaaggcccaatctggctccaaagcttggggttttagttactacactacattgcttcactatattttacaatttactagctgcttataagtatgaattaaggctcagaagtctaattttccagactactcggaggactctcgccccactccactccacaaagattcagctcagcgactccttcctactctgacctagccccgcgtcccgctctcagtggcttgggcaagagc

SEQ ID NO: 19464 - RNA, 2420 nt, Homo sapiens
  source 1..2420: mol_type = other RNA
ttgaggagacatggtgggggccagcctgtgctgctaaacatagattttgctgatctgttggcttctcagtttatagcattcagccccctggctcctcagcagctccttctcttcggctgtgtctcgagctttcagctgcgagaagtgggcaggagaggcgatgagatcatattgttggtccagataccgcaggtagatgagcatgtgcagggcataggccaacaccagcagcaggatcagggacattgccaggccgatcagaaaagctggcgagaaggaggaggcgcagtcttgggctttggtaaatcgtccccccttgatggcaaaaccttggatctggaaatcaataaaagtgacctcccacaggctcgacccatcatccgtgtcgctgggcagcaagagggcctggtcctgctgcaggctgcccacgcgttggcagcggtaggagtaaccagagggagcatatacgccagttgggttaaagactgcttggattgaattgttggaaatgatctcgactcggcgcaaactaaaccaactctggatggacaacttgttgtaattggtaaggatgaatcttatagcaagacttctggggtttccagcatcaccaagcttcaaagacaacctagcactttcttcactgcaatttgagttgtcagggtccacagttaccttctgaccaaatggctcgtctgtaaggtccagccaggtttgattcttaaatttaatcattattcttttggcccagaagagaatgcaaggaattccattgatggagacattaactgggccatgatggctgaatgcattccaaggttctttttctaaatgcccttctttgctcagattgtagttgagagcctgtgtgattggtattgttgtgaaattctggaatggtttcatatctccattattctgatcattcctcataaccacttctttatttgaagatgttggagaacttctctcctcaaacctttttctcccactctttctcttcactgatggccttgccaagtgctgaggtcaaaaatcatagtgctgtaattaactcctctctcacatcctacagtcctgagcaaattctgttcattctaccaccaaacagtgtatctgacccaaccactttttactgtctccactgagggtccaagctatcaccatctctcatctgaactattgcaataccttcccaagtggcctcccagattcatgtctttttctcctctcaacagccagagtaaccccataaaaatataaatcttattttgctacctactcccaagctcaaaactttacaatggctttaaatcaccagaagagtagaaaaaggctttaccatggcctacaggctccacatgttcctgtgtaactctcagaccccatctaatgccacactactcctcagtcactatgctccccttcttcactgatctttcagttcttagaaagcactagcccattctacatctgcacagagatgtcaccttaaactaccctatccagagtagccacccccatccccaagtcactatcacccatccagctatattttctctatagctctacagtatgtaaaaatcatctatttaattatttaatttacatctatctaactggtctgtcctctcacatttagaatataaactgtatcagagcagaaaccttcaccctcttaatttaaccgccatattcccggtacctacaacagcgtctggcacatagaaggcatttttaaacatccttgctgagtgaaccaatatcccagaaacctctcacagctagttcatcttacaggagaaacagtattaaagagttaattaaatggccaggcgcggtggctcacgcctgtaatcccagcacattgggaggccgaggcgggcggatcactcgaggtcaggagatcgacaccagcctggccaacatggtgaaaccccctctctactgaaaatacaaacatcagccaggcgtgatggtggaagcctgtaatcccagctactcaggaggctgaggtgggacaatcgcttgaacccgggaggcggaggttgtagtgagccaagatcgcaccactgcacaacagcctagaagacagagtgagaccctgtctcagaaaaaaataaaaataaaaataaataaatctataagtaaatgactcgccagtcaaaataaacggcaactttagggttaaaggcccaatctggctccaaagcttggggttttagttactacactacattgcttcactatattttacaatttactagctgcttataagtatgaattaaggctcagaagtctaattttccagactactcggaggactctcgccccactccactccacaaagattcagctcagcgactccttcctactctgacctagccccgcgtcccgctctcagtggcttgggcaagagc

SEQ ID NO: 19465 - RNA, 1627 nt, Homo sapiens
  source 1..1627: mol_type = other RNA
ttgaggagacatggtgggggccagcctgtgctgctaaacatagattttgctgatctgttggcttctcagtttatagcattcagccccctggctcctcagcagctccttctcttcggctgtgtctcgagctttcagctgcgagaagtgggcaggagaggcgatgagatcatattgttggtccagataccgcaggtagatgagcatgtgcagggcataggccaacaccagcagcaggatcagggacattgccaggccgatcagaaaagctggcgagaaggaggaggcgcagtcttgggctttggtaaatcgtccccccttgatggcaaaaccttggatctggaaatcaataaaagtgacctcccacaggctcgacccatcatccgtgtcgctgggcagcaagagggcctggtcctgctgcaggctgcccacgcgttggcagcggtaggagtaaccagagggagcatatacgccagttgggttaaagactgcttggattgaattgttggaaatgatctcgactcggcgcaaactaaaccaactctggatggacaacttgttgtaattggtaaggatgaatcttatagcaagacttctggggtttccagcatcaccaagcttcaaagacaacctagcactttcttcactgcaatttgagttgtcagggtccacagttaccttctgaccaaatggctcgtctgtaaggtccagccaggtttgattcttaaatttaatcattattcttttggcccagaagagaatgcaaggaattccattgatggagacattaactgggccatgatggctgaatgcattccaaggttctttttctaaatgcccttctttgctcagattgtagttgagagccttctctcctcaaacctttttctcccactctttctcttcactgatggccttgaacagcgtctggcacatagaaggcatttttaaacatccttgctgagtgaaccaatatcccagaaacctctcacagctagttcatcttacaggagaaacagtattaaagagttaattaaatggccaggcgcggtggctcacgcctgtaatcccagcacattgggaggccgaggcgggcggatcactcgaggtcaggagatcgacaccagcctggccaacatggtgaaaccccctctctactgaaaatacaaacatcagccaggcgtgatggtggaagcctgtaatcccagctactcaggaggctgaggtgggacaatcgcttgaacccgggaggcggaggttgtagtgagccaagatcgcaccactgcacaacagcctagaagacagagtgagaccctgtctcagaaaaaaataaaaataaaaataaataaatctataagtaaatgactcgccagtcaaaataaacggcaactttagggttaaaggcccaatctggctccaaagcttggggttttagttactacactacattgcttcactatattttacaatttactagctgcttataagtatgaattaaggctcagaagtctaattttccagactactcggaggactctcgccccactccactccacaaagattcagctcagcgactccttcctactctgacctagccccgcgtcccgctctcagtggcttgggcaagagc

SEQ ID NO: 19466 - RNA, 1994 nt, Homo sapiens
  source 1..1994: mol_type = other RNA
ttgaggagacatggtgggggccagcctgtgctgctaaacatagattttgctgatctgttggcttctcagtttatagcattcagccccctggctcctcagcagctccttctcttcggctgtgtctcgagctttcagctgcgagaagtgggcaggagaggcgatgagatcatattgttggtccagataccgcaggtagatgagcatgtgcagggcataggccaacaccagcagcaggatcagggacattgccaggccgatcagaaaagctggcgagaaggaggaggcgcagtcttgggctttggtaaatcgtccccccttgatggcaaaaccttggatctggaaatcaataaaagtgacctcccacaggctcgacccatcatccgtgtcgctgggcagcaagagggcctggtcctgctgcaggctgcccacgcgttggcagcggtaggagtaaccagagggagcatatacgccagttgggttaaagactgcttggattgaattgttggaaatgatctcgactcggcgcaaactaaaccaactctggatggacaacttgttgtaattggtaaggatgaatcttatagcaagacttctggggtttccagcatcaccaagcttcaaagacaacctagcactttcttcactgcaatttgagttgtcagggtccacagttaccttctgaccaaatggctcgtctgtaaggtccagccaggtttgattcttaaatttaatcattattcttttggcccagaagagaatgcaaggaattccattgatggagacattaactgggccatgatggctgaatgcattccaaggttctttttctaaatgcccttctttgctcagattgtagttgagagccttctctcctcaaacctttttctcccactctttctcttcactgatggccttgcatggcctacaggctccacatgttcctgtgtaactctcagaccccatctaatgccacactactcctcagtcactatgctccccttcttcactgatctttcagttcttagaaagcactagcccattctacatctgcacagagatgtcaccttaaactaccctatccagagtagccacccccatccccaagtcactatcacccatccagctatattttctctatagctctacagtatgtaaaaatcatctatttaattatttaatttacatctatctaactggtctgtcctctcacatttagaatataaactgtatcagagcagaaaccttcaccctcttaatttaaccgccatattcccggtacctacaacagcgtctggcacatagaaggcatttttaaacatccttgctgagtgaaccaatatcccagaaacctctcacagctagttcatcttacaggagaaacagtattaaagagttaattaaatggccaggcgcggtggctcacgcctgtaatcccagcacattgggaggccgaggcgggcggatcactcgaggtcaggagatcgacaccagcctggccaacatggtgaaaccccctctctactgaaaatacaaacatcagccaggcgtgatggtggaagcctgtaatcccagctactcaggaggctgaggtgggacaatcgcttgaacccgggaggcggaggttgtagtgagccaagatcgcaccactgcacaacagcctagaagacagagtgagaccctgtctcagaaaaaaataaaaataaaaataaataaatctataagtaaatgactcgccagtcaaaataaacggcaactttagggttaaaggcccaatctggctccaaagcttggggttttagttactacactacattgcttcactatattttacaatttactagctgcttataagtatgaattaaggctcagaagtctaattttccagactactcggaggactctcgccccactccactccacaaagattcagctcagcgactccttcctactctgacctagccccgcgtcccgctctcagtggcttgggcaagagc

SEQ ID NO: 19467 - RNA, 2335 nt, Homo sapiens
  source 1..2335: mol_type = other RNA
ttgaggagacatggtgggggccagcctgtgctgctaaacatagattttgctgatctgttggcttctcagtttatagcattcagccccctggctcctcagcagctccttctcttcggctgtgtctcgagctttcagctgcgagaagtgggcaggagaggcgatgagatcatattgttggtccagataccgcaggtagatgagcatgtgcagggcataggccaacaccagcagcaggatcagggacattgccaggccgatcagaaaagctggcgagaaggaggaggcgcagtcttgggctttggtaaatcgtccccccttgatggcaaaaccttggatctggaaatcaataaaagtgacctcccacaggctcgacccatcatccgtgtcgctgggcagcaagagggcctggtcctgctgcaggctgcccacgcgttggcagcggtaggagtaaccagagggagcatatacgccagttgggttaaagactgcttggattgaattgttggaaatgatctcgactcggcgcaaactaaaccaactctggatggacaacttgttgtaattggtaaggatgaatcttatagcaagacttctggggtttccagcatcaccaagcttcaaagacaacctagcactttcttcactgcaatttgagttgtcagggtccacagttaccttctgaccaaatggctcgtctgtaaggtccagccaggtttgattcttaaatttaatcattattcttttggcccagaagagaatgcaaggaattccattgatggagacattaactgggccatgatggctgaatgcattccaaggttctttttctaaatgcccttctttgctcagattgtagttgagagctatcagggtgatgggattcataccgcaaactccagcattatgcactattctcacgtaacaaatctgcacatggaccctctgtgtgattggtattgttgtgaaattctggaatggtttcatatctccattattctgatcattcctcataaccacttctttatttgaagatgttggagaacttacattcttccatggcctacaggctccacatgttcctgtgtaactctcagaccccatctaatgccacactactcctcagtcactatgctccccttcttcactgatctttcagttcttagaaagcactagcccattctacatctgcacagagatgtcaccttaaactaccctatccagagtagccacccccatccccaagtcactatcacccatccagctatattttctctatagctctacagtatgtaaaaatcatctatttaattatttaatttacatctatctaactggtctgtcctctcacatttagaatataaactgtatcagagcagaaaccttcaccctcttaatttaaccgccatattcccggtacctacaacagcgtctggcacatagaaggcatttttaaacatccttgctgagtgaaccaatatcccagaaacctctcacagctagttcatcttacaggagaaacagtattaaagagttaattaaatggccaggcgcggtggctcacgcctgtaatcccagcacattgggaggccgaggcgggcggatcactcgaggtcaggagatcgacaccagcctggccaacatggtgaaaccccctctctactgaaaatacaaacatcagccaggcgtgatggtggaagcctgtaatcccagctactcaggaggctgaggtgggacaatcgcttgaacccgggaggcggaggttgtagtgagccaagatcgcaccactgcacaacagcctagaagacagagtgagaccctgtctcagaaaaaaataaaaataaaaataaataaatctataagtaaatgactcgccagtcaaaataaacggcaactttagggttaaaggcccaatctggctccaaagcttggggttttagttactacactacattgcttcactatattttacaatttactagctgcttataagtatgaattaaggctcagaagtctaattttccagactactcggaggactctcgccccactccactccacaaagattcagctcagcgactccttcctactctgacctagccccgcgtcccgctctcagtggcttgggcaagagcgcctgcgcggtgagcgggtcccataaaacgcattctgggattggtagtccatgttcctccggtctccagcattcaaaagaaaaagggggaaaaaaaaccatgcaaattagatatctctgaatttcttgcaaattaaataagacgcagattctggctcaggaaagtgatgcaaacgcgtcgttttcaaaggagagaccccagcc

SEQ ID NO: 19468 - RNA, 1914 nt, Homo sapiens
  source 1..1914: mol_type = other RNA
ttgaggagacatggtgggggccagcctgtgctgctaaacatagattttgctgatctgttggcttctcagtttatagcattcagccccctggctcctcagcagctccttctcttcggctgtgtctcgagctttcagctgcgagaagtgggcaggagaggcgatgagatcatattgttggtccagataccgcaggtagatgagcatgtgcagggcataggccaacaccagcagcaggatcagggacattgccaggccgatcagaaaagctggcgagaaggaggaggcgcagtcttgggctttggtaaatcgtccccccttgatggcaaaaccttggatctggaaatcaataaaagtgacctcccacaggctcgacccatcatccgtgtcgctgggcagcaagagggcctggtcctgctgcaggctgcccacgcgttggcagcggtaggagtaaccagagggagcatatacgccagttgggttaaagactgcttggattgaattgttggaaatgatctcgactcggcgcaaactaaaccaactctggatggacaacttgttgtaattggtaaggatgaatcttatagcaagacttctggggtttccagcatcaccaagcttcaaagacaacctagcactttcttcactgcaatttgagttgtcagggtccacagttaccttctgaccaaatggctcgtctgtaaggtccagccaggtttgattcttaaatttaatcattattcttttggcccagaagagaatgcaaggaattccattgatggagacattaactgggccatgatggctgaatgcattccaaggttctttttctaaatgcccttctttgctcagattgtagttgagagctatcagggtgatgggattcataccgcaaactccagcattatgcactattctcacgtaacaaatctgcacatggaccctctgtgtgattggtattgttgtgaaattctggaatggtttcatatctccattattctgatcattcctcataaccacttctttatttgaagatgttggagaacttacattcttcctggcaaatatatggtccaaggttagtgaaagtcctataccagtgagcaagctgacaccaggcaggttattttccctctagagccttgtttcctcatcttctctcctcaaacctttttctcccactctttctcttcactgatggccttgaacagcgtctggcacatagaaggcatttttaaacatccttgctgagtgaaccaatatcccagaaacctctcacagctagttcatcttacaggagaaacagtattaaagagttaattaaatggccaggcgcggtggctcacgcctgtaatcccagcacattgggaggccgaggcgggcggatcactcgaggtcaggagatcgacaccagcctggccaacatggtgaaaccccctctctactgaaaatacaaacatcagccaggcgtgatggtggaagcctgtaatcccagctactcaggaggctgaggtgggacaatcgcttgaacccgggaggcggaggttgtagtgagccaagatcgcaccactgcacaacagcctagaagacagagtgagaccctgtctcagaaaaaaataaaaataaaaataaataaatctataagtaaatgactcgccagtcaaaataaacggcaactttagggttaaaggcccaatctggctccaaagcttggggttttagttactacactacattgcttcactatattttacaatttactagctgcttataagtatgaattaaggctcagaagtctaattttccagactactcggaggactctcgccccactccactccacaaagattcagctcagcgactccttcctactctgacctagccccgcgtcccgctctcagtggcttgggcaagagc

SEQ ID NO: 19469 - RNA, 2172 nt, Homo sapiens
  source 1..2172: mol_type = other RNA
ttgaggagacatggtgggggccagcctgtgctgctaaacatagattttgctgatctgttggcttctcagtttatagcattcagccccctggctcctcagcagctccttctcttcggctgtgtctcgagctttcagctgcgagaagtgggcaggagaggcgatgagatcatattgttggtccagataccgcaggtagatgagcatgtgcagggcataggccaacaccagcagcaggatcagggacattgccaggccgatcagaaaagctggcgagaaggaggaggcgcagtcttgggctttggtaaatcgtccccccttgatggcaaaaccttggatctggaaatcaataaaagtgacctcccacaggctcgacccatcatccgtgtcgctgggcagcaagagggcctggtcctgctgcaggctgcccacgcgttggcagcggtaggagtaaccagagggagcatatacgccagttgggttaaagactgcttggattgaattgttggaaatgatctcgactcggcgcaaactaaaccaactctggatggacaacttgttgtaattggtaaggatgaatcttatagcaagacttctggggtttccagcatcaccaagcttcaaagacaacctagcactttcttcactgcaatttgagttgtcagggtccacagttaccttctgaccaaatggctcgtctgtaaggtccagccaggtttgattcttaaatttaatcattattcttttggcccagaagagaatgcaaggaattccattgatggagacattaactgggccatgatggctgaatgcattccaaggttctttttctaaatgcccttctttgctcagattgtagttgagagctatcagggtgatgggattcataccgcaaactccagcattatgcactattctcacgtaacaaatctgcacatggaccctctgtgtgattggtattgttgtgaaattctggaatggtttcatatctccattattctgatcattcctcataaccacttctttatttgaagatgttggagaacttacattcttcctggcaaatatatggtccaaggttagtgaaagtcctataccatggcctacaggctccacatgttcctgtgtaactctcagaccccatctaatgccacactactcctcagtcactatgctccccttcttcactgatctttcagttcttagaaagcactagcccattctacatctgcacagagatgtcaccttaaactaccctatccagagtagccacccccatccccaagtcactatcacccatccagctatattttctctatagctctacagtatgtaaaaatcatctatttaattatttaatttacatctatctaactggtctgtcctctcacatttagaatataaactgtatcagagcagaaaccttcaccctcttaatttaaccgccatattcccggtacctacaacagcgtctggcacatagaaggcatttttaaacatccttgctgagtgaaccaatatcccagaaacctctcacagctagttcatcttacaggagaaacagtattaaagagttaattaaatggccaggcgcggtggctcacgcctgtaatcccagcacattgggaggccgaggcgggcggatcactcgaggtcaggagatcgacaccagcctggccaacatggtgaaaccccctctctactgaaaatacaaacatcagccaggcgtgatggtggaagcctgtaatcccagctactcaggaggctgaggtgggacaatcgcttgaacccgggaggcggaggttgtagtgagccaagatcgcaccactgcacaacagcctagaagacagagtgagaccctgtctcagaaaaaaataaaaataaaaataaataaatctataagtaaatgactcgccagtcaaaataaacggcaactttagggttaaaggcccaatctggctccaaagcttggggttttagttactacactacattgcttcactatattttacaatttactagctgcttataagtatgaattaaggctcagaagtctaattttccagactactcggaggactctcgccccactccactccacaaagattcagctcagcgactccttcctactctgacctagccccgcgtcccgctctcagtggcttgggcaagagc

SEQ ID NO: 19470 - RNA, 2373 nt, Homo sapiens
  source 1..2373: mol_type = other RNA
ttgaggagacatggtgggggccagcctgtgctgctaaacatagattttgctgatctgttggcttctcagtttatagcattcagccccctggctcctcagcagctccttctcttcggctgtgtctcgagctttcagctgcgagaagtgggcaggagaggcgatgagatcatattgttggtccagataccgcaggtagatgagcatgtgcagggcataggccaacaccagcagcaggatcagggacattgccaggccgatcagaaaagctggcgagaaggaggaggcgcagtcttgggctttggtaaatcgtccccccttgatggcaaaaccttggatctggaaatcaataaaagtgacctcccacaggctcgacccatcatccgtgtcgctgggcagcaagagggcctggtcctgctgcaggctgcccacgcgttggcagcggtaggagtaaccagagggagcatatacgccagttgggttaaagactgcttggattgaattgttggaaatgatctcgactcggcgcaaactaaaccaactctggatggacaacttgttgtaattggtaaggatgaatcttatagcaagacttctggggtttccagcatcaccaagcttcaaagacaacctagcactttcttcactgcaatttgagttgtcagggtccacagttaccttctgaccaaatggctcgtctgtaaggtccagccaggtttgattcttaaatttaatcattattcttttggcccagaagagaatgcaaggaattccattgatggagacattaactgggccatgatggctgaatgcattccaaggttctttttctaaatgcccttctttgctcagattgtagttgagagctatcagggtgatgggattcataccgcaaactccagcattatgcactattctcacgtaacaaatctgcacatggaccctctgtgtgattggtattgttgtgaaattctggaatggtttcatatctccattattctgatcattcctcataaccacttctttatttgaagatgttggagaacttacattcttcctggcaaatatatggtccaaggttagtgaaagtcctataccgcacagcaagtgacacaagcatcagtatatttggtcagctccccttcccctcggaataatgtaggtaggcccagatggatacttgcacacacagtgggctggagcccaggttggtgctcagtaaaatatacggaatgaatgaatgatccttctctcctcaaacctttttctcccactctttctcttcactgatggccttgcatggcctacaggctccacatgttcctgtgtaactctcagaccccatctaatgccacactactcctcagtcactatgctccccttcttcactgatctttcagttcttagaaagcactagcccattctacatctgcacagagatgtcaccttaaactaccctatccagagtagccacccccatccccaagtcactatcacccatccagctatattttctctatagctctacagtatgtaaaaatcatctatttaattatttaatttacatctatctaactggtctgtcctctcacatttagaatataaactgtatcagagcagaaaccttcaccctcttaatttaaccgccatattcccggtacctacaacagcgtctggcacatagaaggcatttttaaacatccttgctgagtgaaccaatatcccagaaacctctcacagctagttcatcttacaggagaaacagtattaaagagttaattaaatggccaggcgcggtggctcacgcctgtaatcccagcacattgggaggccgaggcgggcggatcactcgaggtcaggagatcgacaccagcctggccaacatggtgaaaccccctctctactgaaaatacaaacatcagccaggcgtgatggtggaagcctgtaatcccagctactcaggaggctgaggtgggacaatcgcttgaacccgggaggcggaggttgtagtgagccaagatcgcaccactgcacaacagcctagaagacagagtgagaccctgtctcagaaaaaaataaaaataaaaataaataaatctataagtaaatgactcgccagtcaaaataaacggcaactttagggttaaaggcccaatctggctccaaagcttggggttttagttactacactacattgcttcactatattttacaatttactagctgcttataagtatgaattaaggctcagaagtctaattttccagactactcggaggactctcgccccactccactccacaaagattcagctcagcgactccttcctactctgacctagccccgcgtcccgctctcagtggcttgggcaagagc

SEQ ID NO: 19471 - RNA, 2394 nt, Homo sapiens
  source 1..2394: mol_type = other RNA
ttgaggagacatggtgggggccagcctgtgctgctaaacatagattttgctgatctgttggcttctcagtttatagcattcagccccctggctcctcagcagctccttctcttcggctgtgtctcgagctttcagctgcgagaagtgggcaggagaggcgatgagatcatattgttggtccagataccgcaggtagatgagcatgtgcagggcataggccaacaccagcagcaggatcagggacattgccaggccgatcagaaaagctggcgagaaggaggaggcgcagtcttgggctttggtaaatcgtccccccttgatggcaaaaccttggatctggaaatcaataaaagtgacctcccacaggctcgacccatcatccgtgtcgctgggcagcaagagggcctggtcctgctgcaggctgcccacgcgttggcagcggtaggagtaaccagagggagcatatacgccagttgggttaaagactgcttggattgaattgttggaaatgatctcgactcggcgcaaactaaaccaactctggatggacaacttgttgtaattggtaaggatgaatcttatagcaagacttctggggtttccagcatcaccaagcttcaaagacaacctagcactttcttcactgcaatttgagttgtcagggtccacagttaccttctgaccaaatggctcgtctgtaaggtccagccaggtttgattcttaaatttaatcattattcttttggcccagaagagaatgcaaggaattccattgatggagacattaactgggccatgatggctgaatgcattccaaggttctttttctaaatgcccttctttgctcagattgtagttgagagctatcagggtgatgggattcataccgcaaactccagcattatgcactattctcacgtaacaaatctgcacatggaccctctgtgtgattggtattgttgtgaaattctggaatggtttcatatctccattattctgatcattcctcataaccacttctttatttgaagatgttggagaacttacattcttcctggcaaatatatggtccaaggttagtgaaagtcctatacctcaggtggtctgcccgcctcggccccgcagaatgctgggattacaggcgtgagccacgaccgcgccaggccatgaaagcctcttcttaactcagtgcttagctaaatagagtgcctattgttattccttccctgctggcctctcctttcacctcactcccctaaaaagccttctctcctcaaacctttttctcccactctttctcttcactgatggccttgcatggcctacaggctccacatgttcctgtgtaactctcagaccccatctaatgccacactactcctcagtcactatgctccccttcttcactgatctttcagttcttagaaagcactagcccattctacatctgcacagagatgtcaccttaaactaccctatccagagtagccacccccatccccaagtcactatcacccatccagctatattttctctatagctctacagtatgtaaaaatcatctatttaattatttaatttacatctatctaactggtctgtcctctcacatttagaatataaactgtatcagagcagaaaccttcaccctcttaatttaaccgccatattcccggtacctacaacagcgtctggcacatagaaggcatttttaaacatccttgctgagtgaaccaatatcccagaaacctctcacagctagttcatcttacaggagaaacagtattaaagagttaattaaatggccaggcgcggtggctcacgcctgtaatcccagcacattgggaggccgaggcgggcggatcactcgaggtcaggagatcgacaccagcctggccaacatggtgaaaccccctctctactgaaaatacaaacatcagccaggcgtgatggtggaagcctgtaatcccagctactcaggaggctgaggtgggacaatcgcttgaacccgggaggcggaggttgtagtgagccaagatcgcaccactgcacaacagcctagaagacagagtgagaccctgtctcagaaaaaaataaaaataaaaataaataaatctataagtaaatgactcgccagtcaaaataaacggcaactttagggttaaaggcccaatctggctccaaagcttggggttttagttactacactacattgcttcactatattttacaatttactagctgcttataagtatgaattaaggctcagaagtctaattttccagactactcggaggactctcgccccactccactccacaaagattcagctcagcgactccttcctactctgacctagccccgcgtcccgctctcagtggcttgggcaagagc

SEQ ID NO: 19472 - RNA, 1857 nt, Homo sapiens
  source 1..1857: mol_type = other RNA
ttgaggagacatggtgggggccagcctgtgctgctaaacatagattttgctgatctgttggcttctcagtttatagcattcagccccctggctcctcagcagctccttctcttcggctgtgtctcgagctttcagctgcgagaagtgggcaggagaggcgatgagatcatattgttggtccagataccgcaggtagatgagcatgtgcagggcataggccaacaccagcagcaggatcagggacattgccaggccgatcagaaaagctggcgagaaggaggaggcgcagtcttgggctttggtaaatcgtccccccttgatggcaaaaccttggatctggaaatcaataaaagtgacctcccacaggctcgacccatcatccgtgtcgctgggcagcaagagggcctggtcctgctgcaggctgcccacgcgttggcagcggtaggagtaaccagagggagcatatacgccagttgggttaaagactgcttggattgaattgttggaaatgatctcgactcggcgcaaactaaaccaactctggatggacaacttgttgtaattggtaaggatgaatcttatagcaagacttctggggtttccagcatcaccaagcttcaaagacaacctagcactttcttcactgcaatttgagttgtcagggtccacagttaccttctgaccaaatggctcgtctgtaaggtccagccaggtttgattcttaaatttaatcattattcttttggcccagaagagaatgcaaggaattccattgatggagacattaactgggccatgatggctgaatgcattccaaggttctttttctaaatgcccttctttgctcagattgtagttgagagctatcagggtgatgggattcataccgcaaactccagcattatgcactattctcacgtaacaaatctgcacatggaccctctgtgtgattggtattgttgtgaaattctggaatggtttcatatctccattattctgatcattcctcataaccacttctttatttgaagatgttggagaacttacattcttcctggcaaatatatggtccaaggttagtgaaagtcctataccttctctcctcaaacctttttctcccactctttctcttcactgatggccttgaacagcgtctggcacatagaaggcatttttaaacatccttgctgagtgaaccaatatcccagaaacctctcacagctagttcatcttacaggagaaacagtattaaagagttaattaaatggccaggcgcggtggctcacgcctgtaatcccagcacattgggaggccgaggcgggcggatcactcgaggtcaggagatcgacaccagcctggccaacatggtgaaaccccctctctactgaaaatacaaacatcagccaggcgtgatggtggaagcctgtaatcccagctactcaggaggctgaggtgggacaatcgcttgaacccgggaggcggaggttgtagtgagccaagatcgcaccactgcacaacagcctagaagacagagtgagaccctgtctcagaaaaaaataaaaataaaaataaataaatctataagtaaatgactcgccagtcaaaataaacggcaactttagggttaaaggcccaatctggctccaaagcttggggttttagttactacactacattgcttcactatattttacaatttactagctgcttataagtatgaattaaggctcagaagtctaattttccagactactcggaggactctcgccccactccactccacaaagattcagctcagcgactccttcctactctgacctagccccgcgtcccgctctcagtggcttgggcaagagc

SEQ ID NO: 19473 - RNA, 2224 nt, Homo sapiens
  source 1..2224: mol_type = other RNA
ttgaggagacatggtgggggccagcctgtgctgctaaacatagattttgctgatctgttggcttctcagtttatagcattcagccccctggctcctcagcagctccttctcttcggctgtgtctcgagctttcagctgcgagaagtgggcaggagaggcgatgagatcatattgttggtccagataccgcaggtagatgagcatgtgcagggcataggccaacaccagcagcaggatcagggacattgccaggccgatcagaaaagctggcgagaaggaggaggcgcagtcttgggctttggtaaatcgtccccccttgatggcaaaaccttggatctggaaatcaataaaagtgacctcccacaggctcgacccatcatccgtgtcgctgggcagcaagagggcctggtcctgctgcaggctgcccacgcgttggcagcggtaggagtaaccagagggagcatatacgccagttgggttaaagactgcttggattgaattgttggaaatgatctcgactcggcgcaaactaaaccaactctggatggacaacttgttgtaattggtaaggatgaatcttatagcaagacttctggggtttccagcatcaccaagcttcaaagacaacctagcactttcttcactgcaatttgagttgtcagggtccacagttaccttctgaccaaatggctcgtctgtaaggtccagccaggtttgattcttaaatttaatcattattcttttggcccagaagagaatgcaaggaattccattgatggagacattaactgggccatgatggctgaatgcattccaaggttctttttctaaatgcccttctttgctcagattgtagttgagagctatcagggtgatgggattcataccgcaaactccagcattatgcactattctcacgtaacaaatctgcacatggaccctctgtgtgattggtattgttgtgaaattctggaatggtttcatatctccattattctgatcattcctcataaccacttctttatttgaagatgttggagaacttacattcttcctggcaaatatatggtccaaggttagtgaaagtcctataccttctctcctcaaacctttttctcccactctttctcttcactgatggccttgcatggcctacaggctccacatgttcctgtgtaactctcagaccccatctaatgccacactactcctcagtcactatgctccccttcttcactgatctttcagttcttagaaagcactagcccattctacatctgcacagagatgtcaccttaaactaccctatccagagtagccacccccatccccaagtcactatcacccatccagctatattttctctatagctctacagtatgtaaaaatcatctatttaattatttaatttacatctatctaactggtctgtcctctcacatttagaatataaactgtatcagagcagaaaccttcaccctcttaatttaaccgccatattcccggtacctacaacagcgtctggcacatagaaggcatttttaaacatccttgctgagtgaaccaatatcccagaaacctctcacagctagttcatcttacaggagaaacagtattaaagagttaattaaatggccaggcgcggtggctcacgcctgtaatcccagcacattgggaggccgaggcgggcggatcactcgaggtcaggagatcgacaccagcctggccaacatggtgaaaccccctctctactgaaaatacaaacatcagccaggcgtgatggtggaagcctgtaatcccagctactcaggaggctgaggtgggacaatcgcttgaacccgggaggcggaggttgtagtgagccaagatcgcaccactgcacaacagcctagaagacagagtgagaccctgtctcagaaaaaaataaaaataaaaataaataaatctataagtaaatgactcgccagtcaaaataaacggcaactttagggttaaaggcccaatctggctccaaagcttggggttttagttactacactacattgcttcactatattttacaatttactagctgcttataagtatgaattaaggctcagaagtctaattttccagactactcggaggactctcgccccactccactccacaaagattcagctcagcgactccttcctactctgacctagccccgcgtcccgctctcagtggcttgggcaagagc

SEQ ID NO: 19474 - RNA, 1805 nt, Homo sapiens
  source 1..1805: mol_type = other RNA
ttgaggagacatggtgggggccagcctgtgctgctaaacatagattttgctgatctgttggcttctcagtttatagcattcagccccctggctcctcagcagctccttctcttcggctgtgtctcgagctttcagctgcgagaagtgggcaggagaggcgatgagatcatattgttggtccagataccgcaggtagatgagcatgtgcagggcataggccaacaccagcagcaggatcagggacattgccaggccgatcagaaaagctggcgagaaggaggaggcgcagtcttgggctttggtaaatcgtccccccttgatggcaaaaccttggatctggaaatcaataaaagtgacctcccacaggctcgacccatcatccgtgtcgctgggcagcaagagggcctggtcctgctgcaggctgcccacgcgttggcagcggtaggagtaaccagagggagcatatacgccagttgggttaaagactgcttggattgaattgttggaaatgatctcgactcggcgcaaactaaaccaactctggatggacaacttgttgtaattggtaaggatgaatcttatagcaagacttctggggtttccagcatcaccaagcttcaaagacaacctagcactttcttcactgcaatttgagttgtcagggtccacagttaccttctgaccaaatggctcgtctgtaaggtccagccaggtttgattcttaaatttaatcattattcttttggcccagaagagaatgcaaggaattccattgatggagacattaactgggccatgatggctgaatgcattccaaggttctttttctaaatgcccttctttgctcagattgtagttgagagctatcagggtgatgggattcataccgcaaactccagcattatgcactattctcacgtaacaaatctgcacatggaccctctgtgtgattggtattgttgtgaaattctggaatggtttcatatctccattattctgatcattcctcataaccacttctttatttgaagatgttggagaacttctctcctcaaacctttttctcccactctttctcttcactgatggccttgaacagcgtctggcacatagaaggcatttttaaacatccttgctgagtgaaccaatatcccagaaacctctcacagctagttcatcttacaggagaaacagtattaaagagttaattaaatggccaggcgcggtggctcacgcctgtaatcccagcacattgggaggccgaggcgggcggatcactcgaggtcaggagatcgacaccagcctggccaacatggtgaaaccccctctctactgaaaatacaaacatcagccaggcgtgatggtggaagcctgtaatcccagctactcaggaggctgaggtgggacaatcgcttgaacccgggaggcggaggttgtagtgagccaagatcgcaccactgcacaacagcctagaagacagagtgagaccctgtctcagaaaaaaataaaaataaaaataaataaatctataagtaaatgactcgccagtcaaaataaacggcaactttagggttaaaggcccaatctggctccaaagcttggggttttagttactacactacattgcttcactatattttacaatttactagctgcttataagtatgaattaaggctcagaagtctaattttccagactactcggaggactctcgccccactccactccacaaagattcagctcagcgactccttcctactctgacctagccccgcgtcccgctctcagtggcttgggcaagagc

SEQ ID NO: 19475 - RNA, 2172 nt, Homo sapiens
  source 1..2172: mol_type = other RNA
ttgaggagacatggtgggggccagcctgtgctgctaaacatagattttgctgatctgttggcttctcagtttatagcattcagccccctggctcctcagcagctccttctcttcggctgtgtctcgagctttcagctgcgagaagtgggcaggagaggcgatgagatcatattgttggtccagataccgcaggtagatgagcatgtgcagggcataggccaacaccagcagcaggatcagggacattgccaggccgatcagaaaagctggcgagaaggaggaggcgcagtcttgggctttggtaaatcgtccccccttgatggcaaaaccttggatctggaaatcaataaaagtgacctcccacaggctcgacccatcatccgtgtcgctgggcagcaagagggcctggtcctgctgcaggctgcccacgcgttggcagcggtaggagtaaccagagggagcatatacgccagttgggttaaagactgcttggattgaattgttggaaatgatctcgactcggcgcaaactaaaccaactctggatggacaacttgttgtaattggtaaggatgaatcttatagcaagacttctggggtttccagcatcaccaagcttcaaagacaacctagcactttcttcactgcaatttgagttgtcagggtccacagttaccttctgaccaaatggctcgtctgtaaggtccagccaggtttgattcttaaatttaatcattattcttttggcccagaagagaatgcaaggaattccattgatggagacattaactgggccatgatggctgaatgcattccaaggttctttttctaaatgcccttctttgctcagattgtagttgagagctatcagggtgatgggattcataccgcaaactccagcattatgcactattctcacgtaacaaatctgcacatggaccctctgtgtgattggtattgttgtgaaattctggaatggtttcatatctccattattctgatcattcctcataaccacttctttatttgaagatgttggagaacttctctcctcaaacctttttctcccactctttctcttcactgatggccttgcatggcctacaggctccacatgttcctgtgtaactctcagaccccatctaatgccacactactcctcagtcactatgctccccttcttcactgatctttcagttcttagaaagcactagcccattctacatctgcacagagatgtcaccttaaactaccctatccagagtagccacccccatccccaagtcactatcacccatccagctatattttctctatagctctacagtatgtaaaaatcatctatttaattatttaatttacatctatctaactggtctgtcctctcacatttagaatataaactgtatcagagcagaaaccttcaccctcttaatttaaccgccatattcccggtacctacaacagcgtctggcacatagaaggcatttttaaacatccttgctgagtgaaccaatatcccagaaacctctcacagctagttcatcttacaggagaaacagtattaaagagttaattaaatggccaggcgcggtggctcacgcctgtaatcccagcacattgggaggccgaggcgggcggatcactcgaggtcaggagatcgacaccagcctggccaacatggtgaaaccccctctctactgaaaatacaaacatcagccaggcgtgatggtggaagcctgtaatcccagctactcaggaggctgaggtgggacaatcgcttgaacccgggaggcggaggttgtagtgagccaagatcgcaccactgcacaacagcctagaagacagagtgagaccctgtctcagaaaaaaataaaaataaaaataaataaatctataagtaaatgactcgccagtcaaaataaacggcaactttagggttaaaggcccaatctggctccaaagcttggggttttagttactacactacattgcttcactatattttacaatttactagctgcttataagtatgaattaaggctcagaagtctaattttccagactactcggaggactctcgccccactccactccacaaagattcagctcagcgactccttcctactctgacctagccccgcgtcccgctctcagtggcttgggcaagagc

SEQ ID NO: 19476 - RNA, 2498 nt, Homo sapiens
  source 1..2498: mol_type = other RNA
ttgaggagacatggtgggggccagcctgtgctgctaaacatagattttgctgatctgttggcttctcagtttatagcattcagccccctggctcctcagcagctccttctcttcggctgtgtctcgagctttcagctgcgagaagtgggcaggagaggcgatgagatcatattgttggtccagataccgcaggtagatgagcatgtgcagggcataggccaacaccagcagcaggatcagggacattgccaggccgatcagaaaagctggcgagaaggaggaggcgcagtcttgggctttggtaaatcgtccccccttgatggcaaaaccttggatctggaaatcaataaaagtgacctcccacaggctcgacccatcatccgtgtcgctgggcagcaagagggcctggtcctgctgcaggctgcccacgcgttggcagcggtaggagtaaccagagggagcatatacgccagttgggttaaagactgcttggattgaattgttggaaatgatctcgactcggcgcaaactaaaccaactctggatggacaacttgttgtaattggtaaggatgaatcttatagcaagacttctggggtttccagcatcaccaagcttcaaagacaacctagcactttcttcactgcaatttgagttgtcagggtccacagttaccttctgaccaaatggctcgtctgtaaggtccagccaggtttgattcttaaatttaatcattattcttttggcccagaagagaatgcaaggaattccattgatggagacattaactgggccatgatggctgaatgcattccaaggttctttttctaaatgcccttctttgctcagattgtagttgagagctatcagggtgatgggattcataccgcaaactccagcattatgcactattctcacgtaacaaatctgcacatggaccctctgtgtgattggtattgttgtgaaattctggaatggtttcatatctccattattctgatcattcctcataaccacttctttatttgaagatgttggagaacttctctcctcaaacctttttctcccactctttctcttcactgatggccttgccaagtgctgaggtcaaaaatcatagtgctgtaattaactcctctctcacatcctacagtcctgagcaaattctgttcattctaccaccaaacagtgtatctgacccaaccactttttactgtctccactgagggtccaagctatcaccatctctcatctgaactattgcaataccttcccaagtggcctcccagattcatgtctttttctcctctcaacagccagagtaaccccataaaaatataaatcttattttgctacctactcccaagctcaaaactttacaatggctttaaatcaccagaagagtagaaaaaggctttaccatggcctacaggctccacatgttcctgtgtaactctcagaccccatctaatgccacactactcctcagtcactatgctccccttcttcactgatctttcagttcttagaaagcactagcccattctacatctgcacagagatgtcaccttaaactaccctatccagagtagccacccccatccccaagtcactatcacccatccagctatattttctctatagctctacagtatgtaaaaatcatctatttaattatttaatttacatctatctaactggtctgtcctctcacatttagaatataaactgtatcagagcagaaaccttcaccctcttaatttaaccgccatattcccggtacctacaacagcgtctggcacatagaaggcatttttaaacatccttgctgagtgaaccaatatcccagaaacctctcacagctagttcatcttacaggagaaacagtattaaagagttaattaaatggccaggcgcggtggctcacgcctgtaatcccagcacattgggaggccgaggcgggcggatcactcgaggtcaggagatcgacaccagcctggccaacatggtgaaaccccctctctactgaaaatacaaacatcagccaggcgtgatggtggaagcctgtaatcccagctactcaggaggctgaggtgggacaatcgcttgaacccgggaggcggaggttgtagtgagccaagatcgcaccactgcacaacagcctagaagacagagtgagaccctgtctcagaaaaaaataaaaataaaaataaataaatctataagtaaatgactcgccagtcaaaataaacggcaactttagggttaaaggcccaatctggctccaaagcttggggttttagttactacactacattgcttcactatattttacaatttactagctgcttataagtatgaattaaggctcagaagtctaattttccagactactcggaggactctcgccccactccactccacaaagattcagctcagcgactccttcctactctgacctagccccgcgtcccgctctcagtggcttgggcaagagc

SEQ ID NO: 19477 - RNA, 1853 nt, Homo sapiens
  source 1..1853: mol_type = other RNA
ttgaggagacatggtgggggccagcctgtgctgctaaacatagattttgctgatctgttggcttctcagtttatagcattcagccccctggctcctcagcagctccttctcttcggctgtgtctcgagctttcagctgcgagaagtgggcaggagaggcgatgagatcatattgttggtccagataccgcaggtagatgagcatgtgcagggcataggccaacaccagcagcaggatcagggacattgccaggccgatcagaaaagctggcgagaaggaggaggcgcagtcttgggctttggtaaatcgtccccccttgatggcaaaaccttggatcttatagcaagacttctggggtttccagcatcaccaagcttcaaagacaacctagcactttcttcactgcaatttgagttgtcagggtccacagttaccttctgaccaaatggctcgtctgtaaggtccagccaggtttgattcttaaatttaatcattattcttttggcccagaagagaatgcaaggaattccattgatggagacattaactgggccatgatggctgaatgcattccaaggttctttttctaaatgcccttctttgctcagattgtagttgagagcctgtgtgattggtattgttgtgaaattctggaatggtttcatatctccattattctgatcattcctcataaccacttctttatttgaagatgttggagaacttctctcctcaaacctttttctcccactctttctcttcactgatggccttgcatggcctacaggctccacatgttcctgtgtaactctcagaccccatctaatgccacactactcctcagtcactatgctccccttcttcactgatctttcagttcttagaaagcactagcccattctacatctgcacagagatgtcaccttaaactaccctatccagagtagccacccccatccccaagtcactatcacccatccagctatattttctctatagctctacagtatgtaaaaatcatctatttaattatttaatttacatctatctaactggtctgtcctctcacatttagaatataaactgtatcagagcagaaaccttcaccctcttaatttaaccgccatattcccggtacctacaacagcgtctggcacatagaaggcatttttaaacatccttgctgagtgaaccaatatcccagaaacctctcacagctagttcatcttacaggagaaacagtattaaagagttaattaaatggccaggcgcggtggctcacgcctgtaatcccagcacattgggaggccgaggcgggcggatcactcgaggtcaggagatcgacaccagcctggccaacatggtgaaaccccctctctactgaaaatacaaacatcagccaggcgtgatggtggaagcctgtaatcccagctactcaggaggctgaggtgggacaatcgcttgaacccgggaggcggaggttgtagtgagccaagatcgcaccactgcacaacagcctagaagacagagtgagaccctgtctcagaaaaaaataaaaataaaaataaataaatctataagtaaatgactcgccagtcaaaataaacggcaactttagggttaaaggcccaatctggctccaaagcttggggttttagttactacactacattgcttcactatattttacaatttactagctgcttataagtatgaattaaggctcagaagtctaattttccagactactcggaggactctcgccccactccactccacaaagattcagctcagcgactccttcctactctgacctagccccgcgtcccgctctcagtggcttgggcaagagc

SEQ ID NO: 19478 - RNA, 2094 nt, Homo sapiens
  source 1..2094: mol_type = other RNA
ttgaggagacatggtgggggccagcctgtgctgctaaacatagattttgctgatctgttggcttctcagtttatagcattcagccccctggctcctcagcagctccttctcttcggctgtgtctcgagctttcagctgcgagaagtgggcaggagaggcgatgagatcatattgttggtccagataccgcaggtagatgagcatgtgcagggcataggccaacaccagcagcaggatcagggacattgccaggccgatcagaaaagctggcgagaaggaggaggcgcagtcttgggctttggtaaatcgtccccccttgatggcaaaaccttggatcttatagcaagacttctggggtttccagcatcaccaagcttcaaagacaacctagcactttcttcactgcaatttgagttgtcagggtccacagttaccttctgaccaaatggctcgtctgtaaggtccagccaggtttgattcttaaatttaatcattattcttttggcccagaagagaatgcaaggaattccattgatggagacattaactgggccatgatggctgaatgcattccaaggttctttttctaaatgcccttctttgctcagattgtagttgagagctatcagggtgatgggattcataccgcaaactccagcattatgcactattctcacgtaacaaatctgcacatggaccctctgtgtgattggtattgttgtgaaattctggaatggtttcatatctccattattctgatcattcctcataaccacttctttatttgaagatgttggagaacttacattcttccatggcctacaggctccacatgttcctgtgtaactctcagaccccatctaatgccacactactcctcagtcactatgctccccttcttcactgatctttcagttcttagaaagcactagcccattctacatctgcacagagatgtcaccttaaactaccctatccagagtagccacccccatccccaagtcactatcacccatccagctatattttctctatagctctacagtatgtaaaaatcatctatttaattatttaatttacatctatctaactggtctgtcctctcacatttagaatataaactgtatcagagcagaaaccttcaccctcttaatttaaccgccatattcccggtacctacaacagcgtctggcacatagaaggcatttttaaacatccttgctgagtgaaccaatatcccagaaacctctcacagctagttcatcttacaggagaaacagtattaaagagttaattaaatggccaggcgcggtggctcacgcctgtaatcccagcacattgggaggccgaggcgggcggatcactcgaggtcaggagatcgacaccagcctggccaacatggtgaaaccccctctctactgaaaatacaaacatcagccaggcgtgatggtggaagcctgtaatcccagctactcaggaggctgaggtgggacaatcgcttgaacccgggaggcggaggttgtagtgagccaagatcgcaccactgcacaacagcctagaagacagagtgagaccctgtctcagaaaaaaataaaaataaaaataaataaatctataagtaaatgactcgccagtcaaaataaacggcaactttagggttaaaggcccaatctggctccaaagcttggggttttagttactacactacattgcttcactatattttacaatttactagctgcttataagtatgaattaaggctcagaagtctaattttccagactactcggaggactctcgccccactccactccacaaagattcagctcagcgactccttcctactctgacctagccccgcgtcccgctctcagtggcttgggcaagagcgcctgcgcggtgagcgggtcccataaaacgcattctgggattggtagtccatgttcctccggtctccagcattcaaaagaaaaagggggaaaaaaaaccatgcaaattagatatctctgaatttcttgcaaattaaataagacgcagattctggctcaggaaagtgatgcaaacgcgtcgttttcaaaggagagaccccagcc

SEQ ID NO: 19479 - RNA, 1637 nt, Homo sapiens
  source 1..1637: mol_type = other RNA
ttgcactctggccttctcccagggagttcctggaagatgctgagctggtgtcatccataccctcattctgggaggccaagctgctgaggttaaactccgcaggggtgatggtaatttctggatttgttgagttggaaggggagcctgttgagtgggaggtgagggcgcagtccccgttgggcaggtcactgaagctgagcgacagtggcattttctcctcggctgcctttccattttcaaagatgtcatcaggtagatttgaaaagaaggagtggtctttgaaggtgggcgtttccggggtaccctggctgtacatggacattctcctctgaagggctgctgccttgttcccagcgcctgaggatgcggtcatgtcctccacgtcaaatggataccaggtgatttccaggttcagtttgatggtaccaaggtcattgatgtcgacagccactacctgaggtcgggctgcaaacagctctttggtctcacaggtcacgctacctaccaggatgtgagttgctagccctttgagctccgtgaccttgatggagatgaacccaactatcaggggcagaaaaactgtttcttctccatcccagctctgcttgccatttacttctattttgcctttcagtttccaccgctgccggccatacttcatgaaaatttcatattgatctccaggacagaggcgtgcaaagccagccagacctttcatcttgatggagaattctcccagcagattctctagctccacttcaatggtgcacatattctctgtgtactccttgaagctccgattgatctctgtcagactctcccgggcagctttgctggcaggggatgttgcgaaggcttgcttcattttgctggcaccatcctggaggcgtcgctggatacaataagcttcatagagttcatctaccttacttatatgaaactccaggcgtctcatgtatctttcaattgttttaatttgcttgtctaggtcatacagtacacccaggcgagagtttcttttcatatcttttaactgagctgtcaacttgtccagctccgtctggtgaacctccagatattcatcaagtccatttttcaaggccctgtagacttcttccacccttttaggctgaggctctttggggggattgttgtttttgtggcctaaattgtgcattttcttcagtttggcctgaggcttcttgagagcggaggaattttcaatgaaggagttacacctggatcgcctttcctggaggccgctgaaacccgcaaaggactggcttctaatgatcccattgggccctccaggcgaaaaagactgggatcctaccaacatgatttccgggagtctggtcggtagtcatgatctgatttgtctgtcaacaagaatccaacagttcaggctcttgacacgtccctcttcagcctagggtgtgcagatgttatggaatcatcaccctcatagtcagccaagcacatcctcatttcagggtcccagaaactagcacctggcacagcctggaccatatgaccaccacctggtgagccgtttgctcccacacgtgaattctgttctgttcttgaaagcaggataggaacctacactgtgcatggcccttcttttttcctttttt

SEQ ID NO: 19480 - RNA, 1472 nt, Homo sapiens
  source 1..1472: mol_type = other RNA
ttgcactctggccttctcccagggagttcctggaagatgctgagctggtgtcatccataccctcattctgggaggccaagctgctgaggttaaactccgcaggggtgatggtaatttctggatttgttgagttggaaggggagcctgttgagtgggaggtgagggcgcagtccccgttgggcaggtcactgaagctgagcgacagtggcattttctcctcggctgcctttccattttcaaagatgtcatcaggtagatttgaaaagaaggagtggtctttgaaggtgggcgtttccggggtaccctggctgtacatggacattctcctctgaagggctgctgccttgttcccagcgcctgaggatgcggtcatgtcctccacgtcaaatggataccaggtgatttccaggttcagtttgatggtaccaaggtcattgatgtcgacagccactacctgaggtcgggctgcaaacagctctttggtctcacaggtcacgctacctaccaggatgtgagttgctagccctttgagctccgtgaccttgatggagatgaacccaactatcaggggcagaaaaactgtttcttctccatcccagctctgcttgccatttacttctattttgcctttcagtttccaccgctgccggccatacttcatgaaaatttcatattgatctccaggacagaggcgtgcaaagccagccagacctttcatcttgatggagaattctcccagcagattctctagctccacttcaatggtgcacatattctctgtgtactccttgaagctccgattgatctctgtcagactctcccgggcagctttgctggcaggggatgttgcgaaggcttgcttcattttgctggcaccatcctggaggcgtcgctggatacaataagcttcatagagttcatctaccttacttatatgaaactccaggcgtctcatgtatctttcaattgttttaatttgcttgtctaggtcatacagtacacccaggcgagagtttcttttcatatcttttaactgagctgtcaacttgtccagctccgtctggtgaacctccagatattcatcaagtccatttttcaaggccctgtagacttcttccacccttttaggctgaggctctttggggggattgttgtttttgtggcctaaattgtgcattttcttcagtttggcctgaggcttcttgagagcggaggaattttcaatgaaggagttacacctggatcgcctttcctggaggccgctgaaacccgcaaaggactggcttctaatgatcccattgggccctccaggcgaaaaagactgggatcctaccaacatgatttccgggagtctggtcggtagtccaccacctggtgagccgtttgctcccacacgtgaattctgttctgttcttgaaagcaggataggaacctacactgtgcatggcccttcttttttccttttttcaatt

SEQ ID NO: 19481 - RNA, 1685 nt, Homo sapiens
  source 1..1685: mol_type = other RNA
ttgcactctggccttctcccagggagttcctggaagatgctgagctggtgtcatccataccctcattctgggaggccaagctgctgaggttaaactccgcaggggtgatggtaatttctggatttgttgagttggaaggggagcctgttgagtgggaggtgagggcgcagtccccgttgggcaggtcactgaagctgagcgacagtggcattttctcctcggctgcctttccattttcaaagatgtcatcaggtagatttgaaaagaaggagtggtctttgaaggtgggcgtttccggggtaccctggctgtacatggacattctcctctgaagggctgctgccttgttcccagcgcctgaggatgcggtcatgtcctccacgtcaaatggataccaggtgatttccaggttcagtttgatggtaccaaggtcattgatgtcgacagccactacctgaggtcgggctgcaaacagctctttggtctcacaggtcacgctacctaccaggatgtgagttgctagccctttgagctccgtgaccttgatggagatgaacccaactatcaggggcagaaaaactgtttcttctccatcccagctctgcttgccatttacttctattttgcctttcagtttccaccgctgccggccatacttcatgaaaatttcatattgatctccaggacagaggcgtgcaaagccagccagacctttcatcttgatggagaattctcccagcagattctctagctccacttcaatggtgcacatattctctgtgtactccttgaagctccgattgatctctgtcagactctcccgggcagctttgctggcaggggatgttgcgaaggcttgcttcattttgctggcaccatcctggaggcgtcgctggatacaataagcttcatagagttcatctaccttacttatatgaaactccaggcgtctcatgtatctttcaattgttttaatttgcttgtctaggtcatacagtacacccaggcgagagtttcttttcatatcttttaactgagctgtcaacttgtccagctccgtctggtgaacctccagatattcatcaagtccatttttcaaggccctgtagacttcttccacccttttaggctgaggctctttggggggattgttgtttttgtggcctaaattgtgcattttcttcagtttggcctgaggcttcttgagagcggaggaattttcaatgaaggagttacacctggatcgcctttcctggaggccgctgaaacccgcaaaggactggcttctaatgatcccattgggccctccaggcgaaaaagactgggatcctaccaacatgatttccgggagtctggtcggtagtccattgtcttagcaggtgacttcaatccagagagggggacaggctagcaggaaaaagggtaaatagttactgcccagattgaagactccaaagtgggcagacaacaaatcggtatgtttgcagagtgtcgacaattgccctttaaagactcaaagaaagaaaagctaaaaaaaacaacagcagcagaactctctggtagtacatccagatgtaatggaaagaccaatttcactagaccttcctcaaagctacgcgaagcagctcagcaaggaaggcagtttgagcgagttacttccccagagagagaaggacaaacagcct

SEQ ID NO: 19482 - RNA, 1775 nt, Homo sapiens
  source 1..1775: mol_type = other RNA
ttgcactctggccttctcccagggagttcctggaagatgctgagctggtgtcatccataccctcattctgggaggccaagctgctgaggttaaactccgcaggggtgatggtaatttctggatttgttgagttggaaggggagcctgttgagtgggaggtgagggcgcagtccccgttgggcaggtcactgaagctgagcgacagtggcattttctcctcggctgcctttccattttcaaagatgtcatcaggtagatttgaaaagaaggagtggtctttgaaggtgggcgtttccggggtaccctggctgtacatggacattctcctctgaagggctgctgccttgttcccagcgcctgaggatgcggtcatgtcctccacgtcaaatggataccaggtgatttccaggttcagtttgatggtaccaaggtcattgatgtcgacagccactacctgaggtcgggctgcaaacagctctttggtctcacaggtcacgctacctaccaggatgtgagttgctagccctttgagctccgtgaccttgatggagatgaacccaactatcaggggcagaaaaactgtttcttctccatcccagctctgcttgccatttacttctattttgcctttcagtttccaccgctgccggccatacttcatgaaaatttcatattgatctccaggacagaggcgtgcaaagccagccagacctttcatcttgatggagaattctcccagcagattctctagctccacttcaatggtgcacatattctctgtgtactccttgaagctccgattgatctctgtcagactctcccgggcagctttgctggcaggggatgttgcgaaggcttgcttcattttgctggcaccatcctggaggcgtcgctggatacaataagcttcatagagttcatctaccttacttatatgaaactccaggcgtctcatgtatctttcaattgttttaatttgcttgtctaggtcatacagtacacccaggcgagagtttcttttcatatcttttaactgagctgtcaacttgtccagctccgtctggtgaacctccagatattcatcaagtccatttttcaaggccctgtagacttcttccacccttttaggctgaggctctttggggggattgttgtttttgtggcctaaattgtgcattttcttcagtttggcctgaggcttcttgagagcggaggaattttcaatgaaggagttacacctggatcgcctttcctggaggccgctgaaacccgcaaaggactggcttctaatgatcccattgggccctccaggcgaaaaagactgggatcctaccaacatgatttccgggagtctggtcggtagtccattgtcttagcaggtgacttcaatccagagagggggacaggctagcaggaaaaagggtaaatagttactgcccagattgaagactccaaagtgggcagacaacaaatcggtatgtttgcagagtgtcgacaattgccctttaaagactcaaagaaagaaaagctaaaaaaaacaacagcagcagaactctctggtagtacatccagatgtaatggaaagaccaatttcactagaccttcctcaaagctacgcgaagcagctcagcaaggaaggcagtttgagcgagttacttccccagagagagaaggacaaacagcctcctcccccatgttgctgcaggtttttaaatcccctccctccctctccaggagagagcagccctggagtttgtatgcattcttgcgaggta

SEQ ID NO: 19483 - RNA, 1596 nt, Homo sapiens
  source 1..1596: mol_type = other RNA
ttgcactctggccttctcccagggagttcctggaagatgctgagctggtgtcatccataccctcattctgggaggccaagctgctgaggttaaactccgcaggggtgatggtaatttctggatttgttgagttggaaggggagcctgttgagtgggaggtgagggcgcagtccccgttgggcaggtcactgaagctgagcgacagtggcattttctcctcggctgcctttccattttcaaagatgtcatcaggtagatttgaaaagaaggagtggtctttgaaggtgggcgtttccggggtaccctggctgtacatggacattctcctctgaagggctgctgccttgttcccagcgcctgaggatgcggtcatgtcctccacgtcaaatggataccaggtgatttccaggttcagtttgatggtaccaaggtcattgatgtcgacagccactacctgaggtcgggctgcaaacagctctttggtctcacaggtcacgctacctaccaggatgtgagttgctagccctttgagctccgtgaccttgatggagatgaacccaactatcaggggcagaaaaactgtttcttctccatcccagctctgcttgccatttacttctattttgcctttcagtttccaccgctgccggccatacttcatgaaaatttcatattgatctccaggacagaggcgtgcaaagccagccagacctttcatcttgatggagaattctcccagcagattctctagctccacttcaatggtgcacatattctctgtgtactccttgaagctccgattgatctctgtcagactctcccgggcagctttgctggcaggggatgttgcgaaggcttgcttcattttgctggcaccatcctggaggcgtcgctggatacaataagcttcatagagttcatctaccttacttatatgaaactccaggcgtctcatgtatctttcaattgttttaatttgcttgtctaggtcatacagtacacccaggcgagagtttcttttcatatcttttaactgagctgtcaacttgtccagctccgtctggtgaacctccagatattcatcaagtccatttttcaaggccctgtagacttcttccacccttttaggctgaggctctttggggggattgttgtttttgtggcctaaattgtgcattttcttcagtttggcctgaggcttcttgagagcggaggaattttcaatgaaggagttacacctggatcgcctttcctggaggccgctgaaacccgcaaaggactggcttctaatgatcccattgggccctccaggcgaaaaagactgggatcctaccaacatgatttccgggagtctggtcggtagtcctaacgacgacggctccttgtcatgtcaggggcacactcagggttctctggcatataaaagcctccgcaccaatgcaatgcccggagctgcccgcacctccggctttgcagacagcctgagctggctcacttgggtgaaggggaccccgggaggaagtcgggtggacgcgagctgtccccagcgccggctgccctgccgcgtccgctcgcagcagctgcggcgcgcggggt

SEQ ID NO: 19484 - RNA, 1718 nt, Homo sapiens
  source 1..1718: mol_type = other RNA
ttgcactctggccttctcccagggagttcctggaagatgctgagctggtgtcatccataccctcattctgggaggccaagctgctgaggttaaactccgcaggggtgatggtaatttctggatttgttgagttggaaggggagcctgttgagtgggaggtgagggcgcagtccccgttgggcaggtcactgaagctgagcgacagtggcattttctcctcggctgcctttccattttcaaagatgtcatcaggtagatttgaaaagaaggagtggtctttgaaggtgggcgtttccggggtaccctggctgtacatggacattctcctctgaagggctgctgccttgttcccagcgcctgaggatgcggtcatgtcctccacgtcaaatggataccaggtgatttccaggttcagtttgatggtaccaaggtcattgatgtcgacagccactacctgaggtcgggctgcaaacagctctttggtctcacaggtcacgctacctaccaggatgtgagttgctagccctttgagctccgtgaccttgatggagatgaacccaactatcaggggcagaaaaactgtttcttctccatcccagctctgcttgccatttacttctattttgcctttcagtttccaccgctgccggccatacttcatgaaaatttcatattgatctccaggacagaggcgtgcaaagccagccagacctttcatcttgatggagaattctcccagcagattctctagctccacttcaatggtgcacatattctctgtgtactccttgaagctccgattgatctctgtcagactctcccgggcagctttgctggcaggggatgttgcgaaggcttgcttcattttgctggcaccatcctggaggcgtcgctggatacaataagcttcatagagttcatctaccttacttatatgaaactccaggcgtctcatgtatctttcaattgttttaatttgcttgtctaggtcatacagtacacccaggcgagagtttcttttcatatcttttaactgagctgtcaacttgtccagctccgtctggtgaacctccagatattcatcaagtccatttttcaaggccctgtagacttcttccacccttttaggctgaggctctttggggggattgttgtttttgtggcctaaattgtgcattttcttcagtttggcctgaggcttcttgagagcggaggaattttcaatgaaggagttacacctggatcgcctttcctggaggccgctgaaacccgcaaaggactggcttctaatgatcccattgggccctccaggcgaaaaagactgggatcctaccaacatgatttccgggagtctggtcggtagtcctaacgacgacggctccttgtcatgtcaggggcacactcagggttctctggcatataaaagcctccgcaccaatgcaatgcccggagctgcccgcacctccggctttgcagacagcctgagctggctcacttgggtgaaggggaccccgggaggaagtcgggtggacgcgagctgtccccagcgccggctgccctgccgcgtccgctcgcagcagctgcggcgcgcggggtgaagttgcggggctggcgggcgcgagggtggcggagcgcggagctagagcggcggagcgggcggaggggcgggagccgtgaggagggggaggcgcggcgcgggggccggcggcgtcacttgt

SEQ ID NO: 19485 - RNA, 1509 nt, Homo sapiens
  source 1..1509: mol_type = other RNA
ttgcactctggccttctcccagggagttcctggaagatgctgagctggtgtcatccataccctcattctgggaggccaagctgctgaggttaaactccgcaggggtgatggtaatttctggatttgttgagttggaaggggagcctgttgagtgggaggtgagggcgcagtccccgttgggcaggtcactgaagctgagcgacagtggcattttctcctcggctgcctttccattttcaaagatgtcatcaggtagatttgaaaagaaggagtggtctttgaaggtgggcgtttccggggtaccctggctgtacatggacattctcctctgaagggctgctgccttgttcccagcgcctgaggatgcggtcatgtcctccacgtcaaatggataccaggtgatttccaggttcagtttgatggtaccaaggtcattgatgtcgacagccactacctgaggtcgggctgcaaacagctctttggtctcacaggtcacgctacctaccaggatgtgagttgctagccctttgagctccgtgaccttgatggagatgaacccaactatcaggggcagaaaaactgtttcttctccatcccagctctgcttgccatttacttctattttgcctttcagtttccaccgctgccggccatacttcatgaaaatttcatattgatctccaggacagaggcgtgcaaagccagccagacctttcatcttgatggagaattctcccagcagattctctagctccacttcaatggtgcacatattctctgtgtactccttgaagctccgattgatctctgtcagactctcccgggcagctttgctggcaggggatgttgcgaaggcttgcttcattttgctggcaccatcctggaggcgtcgctggatacaataagcttcatagagttcatctaccttacttatatgaaactccaggcgtctcatgtatctttcaattgttttaatttgcttgtctaggtcatacagtacacccaggcgagagtttcttttcatatcttttaactgagctgtcaacttgtccagctccgtctggtgaacctccagatattcatcaagtccatttttcaaggccctgtagacttcttccacccttttaggctgaggctctttggggggattgttgtttttgtggcctaaattgtgcattttcttcagtttggcctgaggcttcttgagagcggaggaattttcaatgaaggagttacacctggatcgcctttcctggaggccgctgaaacccgcaaaggactggcttctaatgatcccattgggccctccaggcgaaaaagactgggatcctaccaacatgatttccgggagtctggtcggtagtcctcataatccctactgcttggtcacagtgtagcatttccacagcagttctccttggcctggagagggtaacagcttctcctttatgttcaccattcaccccctgtactggatttttctccaccttgtcgcctcctctccaggtt

SEQ ID NO: 19486 - RNA, 1488 nt, Homo sapiens
  source 1..1488: mol_type = other RNA
ttgcactctggccttctcccagggagttcctggaagatgctgagctggtgtcatccataccctcattctgggaggccaagctgctgaggttaaactccgcaggggtgatggtaatttctggatttgttgagttggaaggggagcctgttgagtgggaggtgagggcgcagtccccgttgggcaggtcactgaagctgagcgacagtggcattttctcctcggctgcctttccattttcaaagatgtcatcaggtagatttgaaaagaaggagtggtctttgaaggtgggcgtttccggggtaccctggctgtacatggacattctcctctgaagggctgctgccttgttcccagcgcctgaggatgcggtcatgtcctccacgtcaaatggataccaggtgatttccaggttcagtttgatggtaccaaggtcattgatgtcgacagccactacctgaggtcgggctgcaaacagctctttggtctcacaggtcacgctacctaccaggatgtgagttgctagccctttgagctccgtgaccttgatggagatgaacccaactatcaggggcagaaaaactgtttcttctccatcccagctctgcttgccatttacttctattttgcctttcagtttccaccgctgccggccatacttcatgaaaatttcatattgatctccaggacagaggcgtgcaaagccagccagacctttcatcttgatggagaattctcccagcagattctctagctccacttcaatggtgcacatattctctgtgtactccttgaagctccgattgatctctgtcagactctcccgggcagctttgctggcaggggatgttgcgaaggcttgcttcattttgctggcaccatcctggaggcgtcgctggatacaataagcttcatagagttcatctaccttacttatatgaaactccaggcgtctcatgtatctttcaattgttttaatttgcttgtctaggtcatacagtacacccaggcgagagtttcttttcatatcttttaactgagctgtcaacttgtccagctccgtctggtgaacctccagatattcatcaagtccatttttcaaggccctgtagacttcttccacccttttaggctgaggctctttggggggattgttgtttttgtggcctaaattgtgcattttcttcagtttggcctgaggcttcttgagagcggaggaattttcaatgaaggagttacacctggatcgcctttcctggaggccgctgaaacccgcaaaggactggcttctaatgatcccattgggccctccaggcgaaaaagactgggatcctaccaacatgatttccgggagtctggtcggtagtccttcaccaaaaacatcatcctcttcatcgaccaggagctcctcagcatcaaaaaactgcatcttggagaggacaggcgcgagaagcagcaggcagcagccccggcagtctcagcagtcacact

SEQ ID NO: 19487 - RNA, 1726 nt, Homo sapiens
  source 1..1726: mol_type = other RNA
ttgcactctggccttctcccagggagttcctggaagatgctgagctggtgtcatccataccctcattctgggaggccaagctgctgaggttaaactccgcaggggtgatggtaatttctggatttgttgagttggaaggggagcctgttgagtgggaggtgagggcgcagtccccgttgggcaggtcactgaagctgagcgacagtggcattttctcctcggctgcctttccattttcaaagatgtcatcaggtagatttgaaaagaaggagtggtctttgaaggtgggcgtttccggggtaccctggctgtacatggacattctcctctgaagggctgctgccttgttcccagcgcctgaggatgcggtcatgtcctccacgtcaaatggataccaggtgatttccaggttcagtttgatggtaccaaggtcattgatgtcgacagccactacctgaggtcgggctgcaaacagctctttggtctcacaggtcacgctacctaccaggatgtgagttgctagccctttgagctccgtgaccttgatggagatgaacccaactatcaggggcagaaaaactgtttcttctccatcccagctctgcttgccatttacttctattttgcctttcagtttccaccgctgccggccatacttcatgaaaatttcatattgatctccaggacagaggcgtgcaaagccagccagacctttcatcttgatggagaattctcccagcagattctctagctccacttcaatggtgcacatattctctgtgtactccttgaagctccgattgatctctgtcagactctcccgggcagctttgctggcaggggatgttgcgaaggcttgcttcattttgctggcaccatcctggaggcgtcgctggatacaataagcttcatagagttcatctaccttacttatatgaaactccaggcgtctcatgtatctttcaattgttttaatttgcttgtctaggtcatacagtacacccaggcgagagtttcttttcatatcttttaactgagctgtcaacttgtccagctccgtctggtgaacctccagatattcatcaagtccatttttcaaggccctgtagacttcttccacccttttaggctgaggctctttggggggattgttgtttttgtggcctaaattgtgcattttcttcagtttggcctgaggcttcttgagagcggaggaattttcaatgaaggagttacacctggatcgcctttcctggaggccgctgaaacccgcaaaggactggcttctaatgatcccattgggccctccaggcgaaaaagactgggatcctaccaacatgatttccgggagtctggtcggtagtccttcaccaaaaacatcatcctcttcatcgaccaggagctcctcagcatcaaaaaactgcatcttggagaggacaggcgcgagaagcagcaggcagcagccccggcagtctcagcagtcacactgccgaccgaggtgatttcctttccttgggttgcccaagccctctggagggcagcttccgcatctgccctgaagaaagcagtttcattcatatgaataggcttcttgagccttgtgaagagtgaatcccaggtggggtaattctcaccactgaggagaaagaattttttgaagagggctgcagatccggttggatatgaatacagatatcactcaaagtctgaatgcaatgaattctat

SEQ ID NO: 19488 - RNA, 2306 nt, Homo sapiens
  source 1..2306: mol_type = other RNA
ttgcactctggccttctcccagggagttcctggaagatgctgagctggtgtcatccataccctcattctgggaggccaagctgctgaggttaaactccgcaggggtgatggtaatttctggatttgttgagttggaaggggagcctgttgagtgggaggtgagggcgcagtccccgttgggcaggtcactgaagctgagcgacagtggcattttctcctcggctgcctttccattttcaaagatgtcatcaggtagatttgaaaagaaggagtggtctttgaaggtgggcgtttccggggtaccctggctgtacatggacattctcctctgaagggctgctgccttgttcccagcgcctgaggatgcggtcatgtcctccacgtcaaatggataccaggtgatttccaggttcagtttgatggtaccaaggtcattgatgtcgacagccactacctgaggtcgggctgcaaacagctctttggtctcacaggtcacgctacctaccaggatgtgagttgctagccctttgagctccgtgaccttgatggagatgaacccaactatcaggggcagaaaaactgtttcttctccatcccagctctgcttgccatttacttctattttgcctttcagtttccaccgctgccggccatacttcatgaaaatttcatattgatctccaggacagaggcgtgcaaagccagccagacctttcatcttgatggagaattctcccagcagattctctagctccacttcaatggtgcacatattctctgtgtactccttgaagctccgattgatctctgtcagactctcccgggcagctttgctggcaggggatgttgcgaaggcttgcttcattttgctggcaccatcctggaggcgtcgctggatacaataagcttcatagagttcatctaccttacttatatgaaactccaggcgtctcatgtatctttcaattgttttaatttgcttgtctaggtcatacagtacacccaggcgagagtttcttttcatatcttttaactgagctgtcaacttgtccagctccgtctggtgaacctccagatattcatcaagtccatttttcaaggccctgtagacttcttccacccttttaggctgaggctctttggggggattgttgtttttgtggcctaaattgtgcattttcttcagtttggcctgaggcttcttgagagcggaggaattttcaatgaaggagttacacctggatcgcctttcctggaggccgctgaaacccgcaaaggactggcttctaatgatcccattgggccctccaggcgaaaaagactgggatcctaccaacatgatttccgggagtctggtcggtagtccttcaccaaaaacatcatcctcttcatcgaccaggagctcctcagcatcaaaaaactgcatcttggagaggacaggcgcgagaagcagcaggcagcagccccggcagtctcagcagtcacactgccgaccgaggtgatttcctttccttgggttgcccaagccctctggagggcagcttccgcatctgccctgaagaaagcagtttcattcatatgaataggcttcttgagccttgtgaagagtgaatcccaggtggggtaattctcaccactgaggagaaagaattttttgaagagggctgcagatccggttggatatgaatacagatatcactcaaagtctgaatgcaatgaattctatttcaaagcaacaactttcatatttccttaaagaggaaggtgggtgcttaactttcttgcttatgaatttgaacacaatgggttttgttgaaagagggagttcatatttctcatatcttggttttgcttcaattacaatttatggttgagctggcgcctccggatcctgtccctccatggcctgtttctgatccagtgtaatcgcgaaggtaacaccatggtcccaacagagcggcctaaaacctgctcatggcaaaggaacaaaagggtcttgcagctatcctggaagttaagtccagacgtataaaaatgaaaaagaaaacttaacccccccctttttgttcttttcttaaaaaaaaaaaaaagagtatttgaggcttccgttgacttcttttatcttgtaacttgccttgcctttccttcccttaacttccgactggcccgaaggcagctgctgtgctgggctgccctagcctcctgtgccatgttttatgcatgaagatgatggggcggtaatttattcaagcagagacgatcaccgggctcctgtgtctgccctcgcgtcagaggagccgtgcaat

SEQ ID NO: 19489 - RNA, 1550 nt, Homo sapiens
  source 1..1550: mol_type = other RNA
ttgcactctggccttctcccagggagttcctggaagatgctgagctggtgtcatccataccctcattctgggaggccaagctgctgaggttaaactccgcaggggtgatggtaatttctggatttgttgagttggaaggggagcctgttgagtgggaggtgagggcgcagtccccgttgggcaggtcactgaagctgagcgacagtggcattttctcctcggctgcctttccattttcaaagatgtcatcaggtagatttgaaaagaaggagtggtctttgaaggtgggcgtttccggggtaccctggctgtacatggacattctcctctgaagggctgctgccttgttcccagcgcctgaggatgcggtcatgtcctccacgtcaaatggataccaggtgatttccaggttcagtttgatggtaccaaggtcattgatgtcgacagccactacctgaggtcgggctgcaaacagctctttggtctcacaggtcacgctacctaccaggatgtgagttgctagccctttgagctccgtgaccttgatggagatgaacccaactatcaggggcagaaaaactgtttcttctccatcccagctctgcttgccatttacttctattttgcctttcagtttccaccgctgccggccatacttcatgaaaatttcatattgatctccaggacagaggcgtgcaaagccagccagacctttcatcttgatggagaattctcccagcagattctctagctccacttcaatggtgcacatattctctgtgtactccttgaagctccgattgatctctgtcagactctcccgggcagctttgctggcaggggatgttgcgaaggcttgcttcattttgctggcaccatcctggaggcgtcgctggatacaataagcttcatagagttcatctaccttacttatatgaaactccaggcgtctcatgtatctttcaattgttttaatttgcttgtctaggtcatacagtacacccaggcgagagtttcttttcatatcttttaactgagctgtcaacttgtccagctccgtctggtgaacctccagatattcatcaagtccatttttcaaggccctgtagacttcttccacccttttaggctgaggctctttggggggattgttgtttttgtggcctaaattgtgcattttcttcagtttggcctgaggcttcttgagagcggaggaattttcaatgaaggagttacacctggatcgcctttcctggaggccgctgaaacccgcaaaggactggcttctaatgatcccattgggccctccaggcgaaaaagactgggatcctaccaacatgatttccgggagtctggtcggtagtccttggcccgttcctccactccccagggcatccttcagttctgcttgcaaaaagtgcgcgtgcccctttcgctcagcaacttcccgaccgtaccctgtgggcttcagatgcccgaacccaccagggtggtggaagctgaggacgctccagtttcaacggctgcttagcattcaacgctcattcaag

SEQ ID NO: 19490 - RNA, 1552 nt, Homo sapiens
  source 1..1552: mol_type = other RNA
ttgcactctggccttctcccagggagttcctggaagatgctgagctggtgtcatccataccctcattctgggaggccaagctgctgaggttaaactccgcaggggtgatggtaatttctggatttgttgagttggaaggggagcctgttgagtgggaggtgagggcgcagtccccgttgggcaggtcactgaagctgagcgacagtggcattttctcctcggctgcctttccattttcaaagatgtcatcaggtagatttgaaaagaaggagtggtctttgaaggtgggcgtttccggggtaccctggctgtacatggacattctcctctgaagggctgctgccttgttcccagcgcctgaggatgcggtcatgtcctccacgtcaaatggataccaggtgatttccaggttcagtttgatggtaccaaggtcattgatgtcgacagccactacctgaggtcgggctgcaaacagctctttggtctcacaggtcacgctacctaccaggatgtgagttgctagccctttgagctccgtgaccttgatggagatgaacccaactatcaggggcagaaaaactgtttcttctccatcccagctctgcttgccatttacttctattttgcctttcagtttccaccgctgccggccatacttcatgaaaatttcatattgatctccaggacagaggcgtgcaaagccagccagacctttcatcttgatggagaattctcccagcagattctctagctccacttcaatggtgcacatattctctgtgtactccttgaagctccgattgatctctgtcagactctcccgggcagctttgctggcaggggatgttgcgaaggcttgcttcattttgctggcaccatcctggaggcgtcgctggatacaataagcttcatagagttcatctaccttacttatatgaaactccaggcgtctcatgtatctttcaattgttttaatttgcttgtctaggtcatacagtacacccaggcgagagtttcttttcatatcttttaactgagctgtcaacttgtccagctccgtctggtgaacctccagatattcatcaagtccatttttcaaggccctgtagacttcttccacccttttaggctgaggctctttggggggattgttgtttttgtggcctaaattgtgcattttcttcagtttggcctgaggcttcttgagagcggaggaattttcaatgaaggagttacacctggatcgcctttcctggaggccgctgaaacccgcaaaggactggcttctaatgatcccattgggccctccaggcgaaaaagactgggatcctaccaacatgatttccgggagtctggtcggtagtccttggcccgttcctccactccccagggcatccttcagttctgcttgcaaaaagtgcgcgtgcccctttcgctcagcaacttcccgaccgtaccctgtgggcttcagatgcccgaacccaccagggtggtggaagctgaggacgctccagtttcaacggctgcttagcattcaacgctcattcaagtc

SEQ ID NO: 19491 - RNA, 1683 nt, Homo sapiens
  source 1..1683: mol_type = other RNA
ttgcactctggccttctcccagggagttcctggaagatgctgagctggtgtcatccataccctcattctgggaggccaagctgctgaggttaaactccgcaggggtgatggtaatttctggatttgttgagttggaaggggagcctgttgagtgggaggtgagggcgcagtccccgttgggcaggtcactgaagctgagcgacagtggcattttctcctcggctgcctttccattttcaaagatgtcatcaggtagatttgaaaagaaggagtggtctttgaaggtgggcgtttccggggtaccctggctgtacatggacattctcctctgaagggctgctgccttgttcccagcgcctgaggatgcggtcatgtcctccacgtcaaatggataccaggtgatttccaggttcagtttgatggtaccaaggtcattgatgtcgacagccactacctgaggtcgggctgcaaacagctctttggtctcacaggtcacgctacctaccaggatgtgagttgctagccctttgagctccgtgaccttgatggagatgaacccaactatcaggggcagaaaaactgtttcttctccatcccagctctgcttgccatttacttctattttgcctttcagtttccaccgctgccggccatacttcatgaaaatttcatattgatctccaggacagaggcgtgcaaagccagccagacctttcatcttgatggagaattctcccagcagattctctagctccacttcaatggtgcacatattctctgtgtactccttgaagctccgattgatctctgtcagactctcccgggcagctttgctggcaggggatgttgcgaaggcttgcttcattttgctggcaccatcctggaggcgtcgctggatacaataagcttcatagagttcatctaccttacttatatgaaactccaggcgtctcatgtatctttcaattgttttaatttgcttgtctaggtcatacagtacacccaggcgagagtttcttttcatatcttttaactgagctgtcaacttgtccagctccgtctggtgaacctccagatattcatcaagtccatttttcaaggccctgtagacttcttccacccttttaggctgaggctctttggggggattgttgtttttgtggcctaaattgtgcattttcttcagtttggcctgaggcttcttgagagcggaggaattttcaatgaaggagttacacctggatcgcctttcctggaggccgctgaaacccgcaaaggactggcttctaatgatcccattgggccctccaggcgaaaaagactgggatcctaccaacatgatttccgggagtctggtcggtagtcggttgagctggcgcctccggatcctgtccctccatggcctgtttctgatccagtgtaatcgcgaaggtaacaccatggtcccaacagagcggcctaaaacctgctcatggcaaaggaacaaaagggtcttgcagctatcctggaagttaagtccagacgtataaaaatgaaaaagaaaacttaacccccccctttttgttcttttcttaaaaaaaaaaaaaagagtatttgaggcttccgttgacttcttttatcttgtaacttgccttgcctttccttcccttaacttccgactggcccgaaggcagctgctgtgct

SEQ ID NO: 19492 - RNA, 1797 nt, Homo sapiens
  source 1..1797: mol_type = other RNA
ttgcactctggccttctcccagggagttcctggaagatgctgagctggtgtcatccataccctcattctgggaggccaagctgctgaggttaaactccgcaggggtgatggtaatttctggatttgttgagttggaaggggagcctgttgagtgggaggtgagggcgcagtccccgttgggcaggtcactgaagctgagcgacagtggcattttctcctcggctgcctttccattttcaaagatgtcatcaggtagatttgaaaagaaggagtggtctttgaaggtgggcgtttccggggtaccctggctgtacatggacattctcctctgaagggctgctgccttgttcccagcgcctgaggatgcggtcatgtcctccacgtcaaatggataccaggtgatttccaggttcagtttgatggtaccaaggtcattgatgtcgacagccactacctgaggtcgggctgcaaacagctctttggtctcacaggtcacgctacctaccaggatgtgagttgctagccctttgagctccgtgaccttgatggagatgaacccaactatcaggggcagaaaaactgtttcttctccatcccagctctgcttgccatttacttctattttgcctttcagtttccaccgctgccggccatacttcatgaaaatttcatattgatctccaggacagaggcgtgcaaagccagccagacctttcatcttgatggagaattctcccagcagattctctagctccacttcaatggtgcacatattctctgtgtactccttgaagctccgattgatctctgtcagactctcccgggcagctttgctggcaggggatgttgcgaaggcttgcttcattttgctggcaccatcctggaggcgtcgctggatacaataagcttcatagagttcatctaccttacttatatgaaactccaggcgtctcatgtatctttcaattgttttaatttgcttgtctaggtcatacagtacacccaggcgagagtttcttttcatatcttttaactgagctgtcaacttgtccagctccgtctggtgaacctccagatattcatcaagtccatttttcaaggccctgtagacttcttccacccttttaggctgaggctctttggggggattgttgtttttgtggcctaaattgtgcattttcttcagtttggcctgaggcttcttgagagcggaggaattttcaatgaaggagttacacctggatcgcctttcctggaggccgctgaaacccgcaaaggactggcttctaatgatcccattgggccctccaggcgaaaaagactgggatcctaccaacatgatttccgggagtctggtcggtagtcggttgagctggcgcctccggatcctgtccctccatggcctgtttctgatccagtgtaatcgcgaaggtaacaccatggtcccaacagagcggcctaaaacctgctcatggcaaaggaacaaaagggtcttgcagctatcctggaagttaagtccagacgtataaaaatgaaaaagaaaacttaacccccccctttttgttcttttcttaaaaaaaaaaaaaagagtatttgaggcttccgttgacttcttttatcttgtaacttgccttgcctttccttcccttaacttccgactggcccgaaggcagctgctgtgctgggctgccctagcctcctgtgccatgttttatgcatgaagatgatggggcggtaatttattcaagcagagacgatcaccgggctcctgtgtctgccctcgcgtcagaggagccg

SEQ ID NO: 19493 - RNA, 1746 nt, Homo sapiens
  source 1..1746: mol_type = other RNA
ttgcactctggccttctcccagggagttcctggaagatgctgagctggtgtcatccataccctcattctgggaggccaagctgctgaggttaaactccgcaggggtgatggtaatttctggatttgttgagttggaaggggagcctgttgagtgggaggtgagggcgcagtccccgttgggcaggtcactgaagctgagcgacagtggcattttctcctcggctgcctttccattttcaaagatgtcatcaggtagatttgaatagagctctagcacggccttgggactcggcctgagggagggcaggtcactgaaggagcggctgcggtgcagcttggcaaagaaagtgtcttgcaaggcactcaagacagacagccgcctgggcttgtctggggaaggatgcagccacctaaagaaggagtggtctttgaaggtgggcgtttccggggtaccctggctgtacatggacattctcctctgaagggctgctgccttgttcccagcgcctgaggatgcggtcatgtcctccacgtcaaatggataccaggtgatttccaggttcagtttgatggtaccaaggtcattgatgtcgacagccactacctgaggtcgggctgcaaacagctctttggtctcacaggtcacgctacctaccaggatgtgagttgctagccctttgagctccgtgaccttgatggagatgaacccaactatcaggggcagaaaaactgtttcttctccatcccagctctgcttgccatttacttctattttgcctttcagtttccaccgctgccggccatacttcatgaaaatttcatattgatctccaggacagaggcgtgcaaagccagccagacctttcatcttgatggagaattctcccagcagattctctagctccacttcaatggtgcacatattctctgtgtactccttgaagctccgattgatctctgtcagactctcccgggcagctttgctggcaggggatgttgcgaaggcttgcttcattttgctggcaccatcctggaggcgtcgctggatacaataagcttcatagagttcatctaccttacttatatgaaactccaggcgtctcatgtatctttcaattgttttaatttgcttgtctaggtcatacagtacacccaggcgagagtttcttttcatatcttttaactgagctgtcaacttgtccagctccgtctggtgaacctccagatattcatcaagtccatttttcaaggccctgtagacttcttccacccttttaggctgaggctctttggggggattgttgtttttgtggcctaaattgtgcattttcttcagtttggcctgaggcttcttgagagcggaggaattttcaatgaaggagttacacctggatcgcctttcctggaggccgctgaaacccgcaaaggactggcttctaatgatcccattgggccctccaggcgaaaaagactgggatcctaccaacatgatttccgggagtctggtcggtagtcctaacgacgacggctccttgtcatgtcaggggcacactcagggttctctggcatataaaagcctccgcaccaatgcaatgcccggagctgcccgcacctccggctttgcagacagcctgagctggctcacttgggtgaaggggaccccgggaggaagtcgggtggacgcgagctgtccccagcgccggctgccctgccgcgtccgctcgcagcagctgcggcgcgcggggt

SEQ ID NO: 19494 - RNA, 1947 nt, Homo sapiens
  source 1..1947: mol_type = other RNA
ttgcactctggccttctcccagggagttcctggaagatgctgagctggtgtcatccataccctcattctgggaggccaagctgctgaggttaaactccgcaggggtgatggtaatttctggatttgttgagttggaaggggagcctgttgagtgggaggtgagggcgcagtccccgttgggcaggtcactgaagctgagcgacagtggcattttctcctcggctgcctttccattttcaaagatgtcatcaggtagatttgaatagagctctagcacggccttgggactcggcctgagggagggcaggtcactgaaggagcggctgcggtgcagcttggcaaagaaagtgtcttgcaaggcactcaagacagacagccgcctgggcttgtctggggaaggatgcagccacctaaagaaggagtggtctttgaaggtgggcgtttccggggtaccctggctgtacatggacattctcctctgaagggctgctgccttgttcccagcgcctgaggatgcggtcatgtcctccacgtcaaatggataccaggtgatttccaggttcagtttgatggtaccaaggtcattgatgtcgacagccactacctgaggtcgggctgcaaacagctctttggtctcacaggtcacgctacctaccaggatgtgagttgctagccctttgagctccgtgaccttgatggagatgaacccaactatcaggggcagaaaaactgtttcttctccatcccagctctgcttgccatttacttctattttgcctttcagtttccaccgctgccggccatacttcatgaaaatttcatattgatctccaggacagaggcgtgcaaagccagccagacctttcatcttgatggagaattctcccagcagattctctagctccacttcaatggtgcacatattctctgtgtactccttgaagctccgattgatctctgtcagactctcccgggcagctttgctggcaggggatgttgcgaaggcttgcttcattttgctggcaccatcctggaggcgtcgctggatacaataagcttcatagagttcatctaccttacttatatgaaactccaggcgtctcatgtatctttcaattgttttaatttgcttgtctaggtcatacagtacacccaggcgagagtttcttttcatatcttttaactgagctgtcaacttgtccagctccgtctggtgaacctccagatattcatcaagtccatttttcaaggccctgtagacttcttccacccttttaggctgaggctctttggggggattgttgtttttgtggcctaaattgtgcattttcttcagtttggcctgaggcttcttgagagcggaggaattttcaatgaaggagttacacctggatcgcctttcctggaggccgctgaaacccgcaaaggactggcttctaatgatcccattgggccctccaggcgaaaaagactgggatcctaccaacatgatttccgggagtctggtcggtagtcggttgagctggcgcctccggatcctgtccctccatggcctgtttctgatccagtgtaatcgcgaaggtaacaccatggtcccaacagagcggcctaaaacctgctcatggcaaaggaacaaaagggtcttgcagctatcctggaagttaagtccagacgtataaaaatgaaaaagaaaacttaacccccccctttttgttcttttcttaaaaaaaaaaaaaagagtatttgaggcttccgttgacttcttttatcttgtaacttgccttgcctttccttcccttaacttccgactggcccgaaggcagctgctgtgctgggctgccctagcctcctgtgccatgttttatgcatgaagatgatggggcggtaatttattcaagcagagacgatcaccgggctcctgtgtctgccctcgcgtcagaggagccg

SEQ ID NO: 19495 - RNA, 4975 nt, Homo sapiens
  source 1..4975: mol_type = other RNA
ttgcactctggccttctcccagggcgccaacgtcttgtcgtcgtccgcgctgtccaccagggccttgtcagcgggcatgtaccaggcagcgctgtgctctgccatcagcgagtccaggtcaatggtgctcatggcgctcttgaccgcctcggagcagcagctgcccagctcgctgtcgccattctgcgcccctgaggccccgacggcgcactcacccttcttgccacccttcagccccagaggctggtcctcggagatgctgaactgctgcctctgtagctggatctgcgcctgaaggatctccagggggtggatctcgtcgggtggcggggcgccgctgctgctcgtcggggtgcggacctgctccaggcccggagtgcccggatggcccgggcccccaccgccgccgtagctgtcaggggtcgaggtagagttagacatgatgcccaggccgagggcgggcgggggcgccttcggtccgtgttccccggcgcctaccccacggggagggagtttgggcgagccggtcaccaggggactcctgctcgctttaactagtgcctgggggttgtcagagctggacgacacctcgtcctcattggcgtagctcgtgctcacctcgtccgaggcgaactcacccacgtttggcgaactactgtccgacttggccccgccgtccagggacccaatgaggtccggctgatcccccaggagcaactcagcccccttcccccaggatggcgacgtgagcgccttttcgtggggcgtcggtgccccgcgcgtctcgcctgcggagcttcccccgacggctgcgcctgacgcttgctgctgccctgggctcaccccaggtgcgcccccgctgtccggagccgccgagtacttgtcaaagaaggtgccagggctcacgtgaccactgtccctttttctgcgaccccgtccccggccgccgcccccggagaccggcttgccgtcattccccgacgtggattccagggtgtagttgggggagaggctggtgccgtccccctgggctggagggttgggcggccccgaggctttggagccgctgctactggtcccggacgggcctccgggtcctggggccccaggagcagtccctcctgggaagtaatccgagcccgggttgccggccactgccgcgccgtcggtctcgttctggctcagtttcctcttgccctctggcgggttcttcttgttgaaggtcacgttgaggttgggggccccgaggctggcgatcatgttctggcaagcggtggagagcgcagccaggcagctctggccgaacaggttgtccttggagctgggcttgttgaaggagcccagcgagagcgcgcccaatttactggccgaggtgcgctggctgggctggaaatcaggctgcggcgggtaggcacccccgccaccgccgccaccagagctgccaccgccccctcccgcgctggggggcgagttcacgcctggaccgctgtgcggcgtggactgccggccggctgcaccaaacggaaagcccggctggcccccgagcgcagacgtagcaaagtccggcggcgggggccggcgctccgaagcagcgctggggagccccacgcccgccccgggcgactgcagctgacccaggcctcccagactgcccccgaactgcaggcccggtgaaggcagcgcgggcacgtggccctctccgggcatcctcatcggctcctgcagagggccccggaacagcacccccgagccaccaggcggaggagggggcgccaggctggggtcgtgcgggccacagtcagcgggcagacccgagccgcccatcctacggggcagcaggtctccgggcggcggatgcggacctgagaaccacgcgctctcttgcgccaagtgcggcgcctgctgctcgaaggtgcccagacgcccggcgcccgtgctgccgccttcgcgctcaaagttcggctgggccaagccgcccaccgggccgccatgcaccaggccgccctggcccacgtccccggggtggcctagctgagccaggttgggctggcgcagccgctgctgctgattccgcgacgccatctgcttaatcatgagggccgcgttttggcgctgctgctgctgctgctgttgctgttgctgttgctgctgctgctgctgctgttgctgctgctgctgctgctgctgctgctgttgcagggactggtggtccggggccggatgctgcaggggcggccccgaagggaagctgtcgggcacaggcggtgtgaactcgccgggtaggcctgggtaggcggaaggggagaggtgattatccagagcgccgttgtgcatgctgccgttccacgaagcgcagcggtccactcccgcgctgcccggaaagtcgaagcgcggcctcttggccacgttcatgtaggggggcgcgtcgaaatgctgcagccgctggttgggcgcctgctgcggaggaggatgctgcatgctgaaaacaggctcggaataagggtgcatgctccggttctccagccggtggatgggatactcgaattgcgcgtgctggctgggcagcatggggcctccgtcctgcaggccgccgctgggcgtgcccgcctcgccctgctggggccgagggagcgcaggcgggcacgaattttgtcggactagaagcccgggtggcggcggcggctgctgctgtggcggctgctgcgggggctgctgctgagggggtggcggggcctgctggggaggctgcattaacgggtgcctggagcccactgagggctccagacccacaggcatctttctggccccactgaacctctcaaagaacacaccatgctgctgctgctgctgctggggctgctgctgctgctggggctgctgctgcggtggctgggcgtgcattttggacaagcccaccatgcccgcagctctgggcatggccgaggcgcccgggaaagcgcccccaggaacctggcgacccgctgcataatgaggcagctgcccttcggagtcagagggcgaaaacatgtcaaaatgtcccgagggcgcctcgcccgggtaattgtattccagcgagtcgacggctccttggttcgtcaccctccgtggctccagactgtgggaatcggagccgctggaggacggcaggccgtggaaggaggcggctcggttagggctctggtccagcggcaggcatggggccggcacggcgtggctggaggcacctgaactgtggaagtccgggaggttccccggtcgctgcgggccgaagctctcaggcccctggctctccgccatgtgctcatagccctcggcgaagggcggctggctgcccaggcctccggctgcgccgccgtagccgagcaggcgacccccgtgcaggcacgaggccccggggtccgggccaccgaagttgcccccaaagtgggggtgatgctggtggggatgatgacttcccgggtggccgtggtgaggctgctggccgccaaagaagccgtgcacaggctgcgcttgcagcccccctgcgtgcaactccgagtggccgcgcgcgtggaagccgtagggctccatgttcatgcccaagatcgggggttcgcccagcgcgctcatagcaggatccacagggccagggggccccccagtgtggaaagccggggccttaaagtgggtgttcatgctcagtccggtctcgttaaagttcctctcgccctggccagcgttcctgctgttgacctggggctcgaattggtccagcccaaacatacttggcggggggcagagggggatcaatagggcatgacagccggctctccgcggcgcgcctccggccagctactcgttccagcccaggattgggcgctccgggacgctcagcaccgcgggggctcagcgcgcacctccaccccgcctgatgtgagggacggggggcggggtattagctcctctcctgaagctccgattctgcccggggagggcctctcacatcttgcgaggccgcggggcctctaggagccgtgttggggggcccatgccccgggcggttgtcacagccgcgggtgggtctgcggggaggggacgaagccgcggatgaacggagacaaaaagttaagtggggggaatggggagggaagggggttgggagagcagagcgatcaccttctcaagtccgattgggtctgctggggagccctcaggacgccgcccgcagcctcccggagtccgtggcagagctgctaagggcaggggagggagacccttcaaagccgcggctggcgccgggcaccgacagagcggtccctccccccgccccccggagtccccgcgccccgcagcccgagcctccaccgagcacgatccgctcgcacaatccccgtaggctccgggcgagcggctgctgcttcttcagcgggtcggaggactggaggctccgctcggcatcgccggtgccggcccccgagccgaggacgcagaggggctgcgaggcggcaggcgccgggggctggagccgagggtcggggaaaggcgcggctcctctgctcggcagcgggtgcgctgcgttcggcgcgcagcttcgcggccacgtccgccgcctgccgcttctgttctccgccgttgggtgtctgagttcgccggagtctccgcgcaccgttgcaggcgcgggagggcagcgagacgaggggttgggtcgctccaaggctccggttccctgcctccgcgctgaggtgcttcgcgagtccctctcggacctgagggaggggggcgtacgcgggtcggggggccacgccgggcgagcaggctaaggcgttcccgctgcgctctcagagcccggaatggggggaggggggcgcgggggcagctctggggggtctgcgcacccctctcccgactagcgggggggctctgcgtggggcgttccgagggtctcggctcccctctctgtgtctgcctctcgcccagcgccgggagaagcagcaac

SEQ ID NO: 19496 - RNA, 4584 nt, Homo sapiens
  source 1..4584: mol_type = other RNA
ttgccagggcaggaggtggaacccatgagccctgccttcagaagcccccacccaggcctcacagggatccttgaacccttggtcaccagctccaccccacccttgcccccagcgcagggccctagtggagccgcaggcactcgcagacacaccctgatcgccgcatctgggggctcctgccctagccagggaggggagagccaggctcctgcacaaggagccaaagcccagagagcgggtatgggtgacggcctcggccgctcctggagcaaagcacccctttgctcacttgcagacagcccccaactgaactctgctctctatgtcctgccacattagggtcacgaccctctgagccaatggaggaggagagggaaggaagatggggccagaggtgtgacggatccccccacaattgccactcaggagggaccagcctgccagggaggaggcgctagcctgggcccgggcaatgccccgctcacgtgcaaaggagccaccttacacctgcagtggtaacagcctggcctcgcttctgttgctgagaggtgaatgtggacagtggagagcatttgccagcagagacaggaaggccatggtggtctgggctaacacaggtggtgctggacaggccatgtgccctggctggacactttctctgccccgtgaccacacgcagcctcagccaagccctggaccccacccttggactcagcctgtgcccaatcctgctctacacctagccctggccctggggactctgatcgtagtgtgtgacctggaggcccaccctcagaatggggactgatgtcctgctgctccagggctgcatgcaccggccacagacccagggcggtcccaggggcattcttagccagcatggcactgcccacattcaagacacctcacacaaccactgcccagctccgcagccagcaacatctccctcagcgcccaggctgccaggtgggcacgccatgtcctgccccggcgcagtgcacagagatgcacaaggggaggggggctgctcccggtgctgtgcggccgcgtgttgctcgtggggtgaggacaggtttggtgcgtgggacctgtggtactgagcgacactccaatacctcatcagccatcagccctgggcccagtggctttgtcaggtcttggaggcccccagtctgtgaggtgagccctgcagagccacaggccctgggcacctgctcctcccaacacagggggtgctccacgggggccccttgcacatcccctgactccaggagtccaagggatacccaagcactaggccagaggcctccaggggccagagagagcagcctttgggaccgccctccccagacactcgcagagcagcacacacacctcaaaggaaactgcctgcccagtgccctcagggcacagggacccctgtgggagacccccctgcactgggtcaactcgctgcccccagccccacagccgtgaccagccctgcaggcctggccctgcccaaaccccaggcagtgccgctgcagagcggaaagcatggccggctcggggcaactgggcctgcagctgggatgcccccaccctgtcctcaggcttggcagccactttcctacttcctgcctctgcgcccacaagaggaagtctggccctgtcctaagcactctcgcttgggaattcaacacgtcagttgctgtcagcagcagggcaggccactcaaagcagctcacaggcaccaaagactcccgtgctgcaggggagcccagcggcctggggacctggagtggctgatccaccaggggtcacagaagtcgaggctgggtctcagtctagggcagggaaccacagggtgagcaaacctgagttcctgcagcctccagggctgaggacttgcagaaaaggactaagcacctgggccacaccagtgccacccctgccaggcccctccttctcagccccacaccacatgtctatccttgccatgaagcacccccaaaccaggtctgcctctgcccataggacccttggctgcaagaatctgcccttcaggagacaatgtggcctcaatgggggtggatccagccatccctggcctgcacaggcctgagaggacccagatcctcctccagccccaccccatcaggaggcccactgaccaggcccatcccccaagccccaccacaaggcctagtgcccaggcccatcgcccaaggcccacagcccaggccccttgtccaagcccagccacagggttggctgggtctacatgcgtctcccaaccagtccggcccactctgcccatgggtcccagcctcatgcaccgctgtgagcaggagcagctgaggatgccccagcgctccaagttctgccatggctgccactgggggcgtttgaggccagcccctgcctgtcctgtgaggctgggtccttctgtccactctgtggccctcaaggagctggtcctgcttccggggcttcgttcccaaagtccttccagcagctcccaggaaggggagggtccagcggggctctgcttcgaagggtgtgccaccatatgcggaggacggcgaaggagctcctggcacggtgtcttgaggaggagaggaggtgcggtgggaggaggcacggaggcggcaggaggaagcacggagccagcatcaccctcagagccagcgtcacccttggagccagtggcagctgcgggctgcagacgaggcttggcaggggctccgtggtctggccctcgccttggggaccgtgggcagaaaaggtctctgccaccatgcgctccacaggtgtgaggaggaggccgggggcggggccgccctccgccagcttcttgcgcacagcacctcgcaggtcccgccacttgtgcttgaggtcccccaggtcgcggcggcagtagcccagcgcgttcactgcctgcaggatgcggctccacacgcggtgctttcgggcaggtgtgccccgcagcgccccgaacagcagcgggtagtggcgccgcaccctctgcaccagcacctccgtctcctgggggctgaagttgggcttgcgtgtcttggtgcgggagtgggggcccggccgcaggggtgtggagcccggcccggcacccagcagcagggctgccgcggccggctcggggctgcagctctgctggcagatggctttgctgctgctggacccaacagcttctccttgctctgacaccatggaggccaagtccttgatgatctgattcacatccagcaagttgctctccatctgcaggatggcctcctcccgcagccggatggcctccaggtcctcttcagtgatgtccgggagcagcgcctgctcctggccctgccacatgttgtcactcccgttaaagaccttctcatcatcagccagctcggcaaacggggcctggggactctgctgtttactgcccctctgcgccatgggaagcagcgctctggacttttctgcaattttcttctgcaccactccatagcactgaatggcatctgagagctgggttttcagccggtccagctgaggacgctcctgctgcagacgctcctgcgggcaggagctgcgcagcagctcggccatctgcttcacggagctggcgctggctgcaatggtcttgttggtctcctgctgtgccgtgtgcaggctgtcccgaagctcctgcgtgtcactcggtgtccctaaggactgaaggctccgctccaaggaggtcacactggagttgattcggaagacgttggccgacatctcctggaacagctcctggaggttgcacggatcgacctgggtggctctgggcggctccagactgaagccctcggagggcagggcctggcaagagaaggtcttggccaccacctgctccacgggcgtgagagccagggcctggggcttgccggaaccagggctggggccatgggccgccttccggaggtcgcccagcttgcgccgcacgacggctcgtaggtcccgccacttgtgcttcaggtccacaacgtcgcggcgacagtagcccagcgcattcacggcctgcaggatgcggctccacacgcggtacctgcgagtgggctcggccttcagcagccccgtgccaaacagcagctggtggtgcttgctcaccttggacaccagcacctcggtctcctgcgggcagaagttgggcttcctcttcttggcccgggtagtgctgggccccgccatccggccatggggcccagcagccgagtccttcctcgggccaatggtgggtgatgaggtgggctccggcatccggctgccttcaggggcaaccccaggccctcgcttcctggcccttgggacaataggcgtgcctgctggccccagatcaccttccccgtccttccccacacagcggttctgcagcttgctctctggcgacgggcaggggaaatggcggattccatactcggtccaacatctagcgcactctaggggctgacagccttgtctcgaaggtcccccgaaagggccacggctccccaggccacctccacgggcgatggatccgtatgacatcttcttacagatggcagggccagcagcctccacactgag

SEQ ID NO: 19497 - RNA, 64 nt, Homo sapiens
  source 1..64: mol_type = other RNA
ttgccatgtctaagaagaaaactttggagaaaaattttcttcttagacatggcaacgtcaacag

SEQ ID NO: 19498 - RNA, 68 nt, Homo sapiens
  source 1..68: mol_type = other RNA
ttgccatgtctaagaagaaaatttttctccaaagttttcttcttagacatggcagcttcagcagtttc

SEQ ID NO: 19499 - RNA, 873 nt, Homo sapiens
  source 1..873: mol_type = other RNA
ttgcctgccctcttcctccagcaacctgaaaacttctcctgttgtgaggacacagtccacatcccgtgtctggtgctcctggttgaaaaagtcgggtctggaggcttccagctttttgtcatagcagggcatcactgtgacgtggtagatcttgtcaggggtcaagtgctgctgctgggcgaagaagtccttgaccagggagcccatgacctgctgcggggaccgggcggtgctgatgtgggggaggatgaagctgccgtgagtcttctcggcatagcagatccagcctgggcaggcagaggccagcaggggcagcgcctgtctgcagtcggcctgtcctcggaatcgccgcacaaactctcgctggctctccaggaggctgaagtgccttgagaaggcggtgtcgaagacgaagtgcacccctatttttttaaagaatgaggttaatttcctggcagtatctgtaggattcagctgaaaccgtgcagccagcgatgctctagactgtggtgagaccgaaactacaaccagcctctgctgactgggtgccgccatcttgttagcatctagaaccttcttcagctcctcgtggctctgctgggtgataagcacggtctctgcggaggtgatgcagccgctgcacgccaggcagtcgtttagcgagaccttggccttctccagcctccgggtcccgccgtcttggttaatttggaagtagctcccgtcatcttcaatgcgaatcttggccacgccacttcccgcccttttttccactttgacaggcttgatgcactcctgagacggcccgatgaagtcatccaggtccgtcagctgcagcgccccgctgaagggcgacgccatgacggccgcact

SEQ ID NO: 19500 - RNA, 955 nt, Homo sapiens
  source 1..955: mol_type = other RNA
ttgcctgccctcttcctccagcaacctgaaaacttctcctgttgtgaggacacagtccacatcccgtgtctggtgctcctggttgaaaaagtcgggtctggaggcttccagctttttgtcatagcagggcatcactgtgacgtggtagatcttgtcaggggtcaagtgctgctgctgggcgaagaagtccttgaccagggagcccatgacctgctgcggggaccgggcggtgctgatgtgggggaggatgaagctgccgtgagtcttctcggcatagcagatccagcctgggcaggcagaggccagcaggggcagcgcctgtctgcagtcggcctgtcctcggaatcgccgcacaaactctcgctggctctccaggaggctgaagtgccttgagaaggcggtgtcgaagacgaagtgcacccctatttttttaaagaatgaggttaatttcctggcagtatctgtaggattcagctgaaaccgtgcagccagcgatgctctagactgtggtgagaccgaaactacaaccagcctctgctgactgggtgccgccatcttgttagcatctagaaccttcttcagctcctcgtggctctgctgggtgataagcacggtctctgcggaggtgatgcagccgctgcacgccaggcagtcgtttagcgagaccttggccttctccagcctccgggtcccgccgtcttggttaatttggaagtagctcccgtcatcttcaatgcgaatcttggccacgccacttcccgcccttttttccactttgacaggcttgatgcactccttcacccttcacgtgaacagggggcgtgaccaccacagagaccagagttgcactgcccatcgagaggacgtgtgcttggatctgagacggcccgatgaagtcatccaggtccgtcagctgcagcgccccgctgaagggcgacgccatgacggccgcact

SEQ ID NO: 19501 - RNA, 1336 nt, Homo sapiens
  source 1..1336: mol_type = other RNA
ttgcctgccctcttcctccagcccttgacactgtttctcaggaagaaaacatccttcatgctggctactacctcatatgctctataacattgtggtgttcacagtttgaatttttcaaaatccagggtagaatttggcccccaaacctaaagctagtggacaagaggaaagtcaatcaatcagtaaatatttattattttctgtaactaaagtactgggctgtggtaggggagacaacaatcaaagacatagccttgtcttccagaagctcacaatctagttgggaattcaagaataccccttagaaaagttcattgacaatttacgaggtgctattagacagtaggagagaaaggcatacataccagggcccagggaagaagagctttgtgaatgaagaaggaaaaagtgtaagttgactttcaaaagtctctggaaacactggactttagctggtccaggaaatatagggaagaattggataggcaggaataaatggagaaagtgttcctacaggaaaagacatgtggaaaaggggagaggtaggcaagatcaaggagtgtttagaaggcaagactgagtatcaagaaagtgaatttctaagccctgcttactcagataagccattaggcttgtgtgagaatgctgatgtcctagataggagactctgggaggggaatatgaaggaagaaaataataatgaatcaaagagcacttccattcctggacactttatacattttcaagactattgcgcccccatcagcactctcatggtgtgtgtagacacagcccagggctgtatttccctgagatgccacacttttcccctggtgtcctcagatataatgcctcagttcctgcaaagtcacataaaataacttgtgagaacttggtgcttggtgagcatccttgtatccagctggcagtccattcgtcatatcccatctgccctggcctagagctggtaagcatgtgccgcacttggggtatttgacaaactgacactctaccacatggagtgtccaactcagcttgtcaaatacacggagcgtggcactgcaggaggccaggccaagagcttctgtggggaagtgagatcttcctgggagatgtgaccctggcaaagttgttggaaagtgttgctaagctttccagagcctcccacataggagctcaaaaggaccttgtctcagcccctggacctatggttggaggccagccaagcaagctgattaacagagtctgtcagtggagtggtgccttggtcatggaggggactctgattccccagtgctgagccaacctgcaggggccagatggaattgggctttct

SEQ ID NO: 19502 - RNA, 2277 nt, Homo sapiens
  source 1..2277: mol_type = other RNA
ttgcctgccctcttcctccagggctccaaaacagcccagcaggcagaggtcctcggccagcttctcaaagagcccattcctcctgaagaagtagccattgacagggtcccagtgcagcgctgcggacacagcacagagagtgtacaaaaccagctccagggtctgtctgggggatactgctccccatgcctgcagcgggggctcctggagggagccttccaggtcagagagcagagacagcagcccgttgaacccgctggagactctgaaggcagcacgacccttgggggtcaccaggatccggagcagagacttcaggagatccagtttcagctgcagctccccttgagtggatgagcatagagcacccacaatgatgctcatgtactcctcggcgttgatggctgagagctgctccaagatgctgagcgaggcctcccggtagcactcgtcatccaggaagatcttgatgaagggcaccatgccgtggtccttcaggacaactgcattcctcaccgagcctttcagaagtgtgactacaatcctcagcatcacacaggtgagttctctttctggatcctgaacaccaggagtggacactttgtttcctgacttcctcatgatcttggcttgcttccgaagctgtgccagtagcaggcccaggagccctgagtcccggaagatgtcggtgaagagggggtccccaccagcgatgctgaggatgctctgcagggccatgagggtgcaggatggcccagggctctccttgatcagatgctgtacctttcgcaggatctcatgaggcacgtagtgcagctcgaacaccagggcctctagaagctggaagaagtgttcctgcactggggccggcttcaggggcatgatctctacaaactgcgagatgggctgcagggtccactccagcaggaagaagtttcgagcattccaggcccacatggtcctgatgactgacaagacttgtatgcagaggacagagtcactggctttgtggaaaacattctgtaggacctggaaggcctgaagattcttaacagtcaccccagatgcctcatgatggaacttgaagccttcaagctgagggtaagtgatgctgtcaaacaccttcagctctgacctcccacaggttgtcagccacaccaccagcccaaggagctcctccagatgcgggtccacttcgctctgggtcagcccatcataccgaagtaacactttgagcagcagaggatagccctctgaattctcaaactccaggaacagagccgaggagacggggtaggagtccttcacgaatcccaagatcaggcttacagcctcgctcacttcaggggcagggagagtgtccgtgagcctggagaggttctggagggagagcctgacacagtctgtggcctgcaggtactggatgatgctgaggttctgggccttggagattgcccttagcacgcagaaggtgggttccttccagaagcagcagctgtgctcccgaaggcaggtcgtggcaatcagcagagactgcagctcacttcctgagaggagtccctccaggccctgagagtcactgcaaatattgagcaacatctgcacgaacatcttttgaacttgaagatcactctcaagaagctcatctttgtccagaggaaagacaaagaagaggtaaaggcactgtaggagcagggctggaagcccagactcagcaaccctgcccagcgtctccgagtctgtccccgtgagcacgtacactgacttcaggagcaagtagccatcctgatccacgtcccccttccaccacagcaactgtccagctgccaaccgagcttgctccgcaggcttccccacaagggccttctggagttgctgggcaagctggtcagacacgtcttcagccagcctttggagactgggaaagcagatgatccccacggagtgttcccaggcctttaggaatagggggagaagactcaacaggctcttctgacgctcaatggggctcttgtgagtcaactgctggtattccagaaacttcctttccagcatgtcccagagagctgtggggctggaggactgccctccatgtgggacatcaggctgcacagcagcaagctgcccttcatttttggaacctgggtcttcatttctgtcttcagcctttgaaagatcttctgcctccatgccgtggcaaagcagatcagaacccagtggagtaatgacagggccgggatagaccagctccctctgaggcccgttggaaatggccct

SEQ ID NO: 19503 - RNA, 2386 nt, Homo sapiens
  source 1..2386: mol_type = other RNA
ttgcctgccctcttcctccagggctccaaaacagcccagcaggcagaggtcctcggccagcttctcaaagagcccattcctcctgaagaagtagccattgacagggtcccagtgcagcgctgcggacacagcacagagagtgtacaaaaccagctccagggtctgtctgggggatactgctccccatgcctgcagcgggggctcctggagggagccttccaggtcagagagcagagacagcagcccgttgaacccgctggagactctgaaggcagcacgacccttgggggtcaccaggatccggagcagagacttcaggagatccagtttcagctgcagctccccttgagtggatgagcatagagcacccacaatgatgctcatgtactcctcggcgttgatggctgagagctgctccaagatgctgagcgaggcctcccggtagcactcgtcatccaggaagatcttgatgaagggcaccatgccgtggtccttcaggacaactgcattcctcaccgagcctttcagaagtgtgactacaatcctcagcatcacacaggtgagttctctttctggatcctgaacaccaggagtggacactttgtttcctgacttcctcatgatcttggcttgcttccgaagctgtgccagtagcaggcccaggagccctgagtcccggaagatgtcggtgaagagggggtccccaccagcgatgctgaggatgctctgcagggccatgagggtgcaggatggcccagggctctccttgatcagatgctgtacctttcgcaggatctcatgaggcacgtagtgcagctcgaacaccagggcctctagaagctggaagaagtgttcctgcactggggccggcttcaggggcatgatctctacaaactgcgagatgggctgcagggtccactccagcaggaagaagtttcgagcattccaggcccacatggtcctgatgactgacaagacttgtatgcagaggacagagtcactggctttgtggaaaacattctgtaggacctggaaggcctgaagattcttaacagtcaccccagatgcctcatgatggaacttgaagccttcaagctgagggtaagtgatgctgtcaaacaccttcagctctgacctcccacaggttgtcagccacaccaccagcccaaggagctcctccagatgcgggtccacttcgctctgggtcagcccatcataccgaagtaacactttgagcagcagaggatagccctctgaattctcaaactccaggaacagagccgaggagacggggtaggagtccttcacgaatcccaagatcaggcttacagcctcgctcacttcaggggcagggagagtgtccgtgagcctggagaggttctggagggagagcctgacacagtctgtggcctgcaggtactggatgatgctgaggttctgggccttggagattgcccttagcacgcagaaggtgggttccttccagaagcagcagctgtgctcccgaaggcaggtcgtggcaatcagcagagactgcagctcacttcctgagaggagtccctccaggccctgagagtcactgcaaatattgagcaacatctgcacgaacatcttttgaacttgaagatcactctcaagaagctcatctttgtccagaggaaagacaaagaagaggtaaaggcactgtaggagcagggctggaagcccagactcagcaaccctgcccagcgtctccgagtctgtccccgtgagcacgtacactgacttcaggagcaagtagccatcctgatccacgtcccccttccaccacagcaactgtccagctgccaaccgagcttgctccgcaggcttccccacaagggccttctggagttgctgggcaagctggtcagacacgtcttcagccagcctttggagactgggaaagcagatgatccccacggagtgttcccaggcctttaggaatagggggagaagactcaacaggctcttctgacgctcaatggggctcttgtgagtcaactgctggtattccagaaacttcctttccagcatgtcccagagagctgtggggctggaggactgccctccatgtgggacatcaggctgcacagcagcaagctgcccttcatttttggaacctgggtcttcatttctgtcttcagcctttgaaagatcttctgcctccatgccgtggcaaagcagatcgtcagaggtcgaggagtgctgctggagcccagcctgactcccaaacttcagcagtgacacacactcaggcagacccaggccctggagtggccctgaccacatgggccccccacgccacacacacttcctgctccccagctcacctcctctcccacattcacaaacccaaaccaggcac

SEQ ID NO: 19504 - RNA, 2388 nt, Homo sapiens
  source 1..2388: mol_type = other RNA
ttgcctgccctcttcctccagggctccaaaacagcccagcaggcagaggtcctcggccagcttctcaaagagcccattcctcctgaagaagtagccattgacagggtcccagtgcagcgctgcggacacagcacagagagtgtacaaaaccagctccagggtctgtctgggggatactgctccccatgcctgcagcgggggctcctggagggagccttccaggtcagagagcagagacagcagcccgttgaacccgctggagactctgaaggcagcacgacccttgggggtcaccaggatccggagcagagacttcaggagatccagtttcagctgcagctccccttgagtggatgagcatagagcacccacaatgatgctcatgtactcctcggcgttgatggctgagagctgctccaagatgctgagcgaggcctcccggtagcactcgtcatccaggaagatcttgatgaagggcaccatgccgtggtccttcaggacaactgcattcctcaccgagcctttcagaagtgtgactacaatcctcagcatcacacaggtgagttctctttctggatcctgaacaccaggagtggacactttgtttcctgacttcctcatgatcttggcttgcttccgaagctgtgccagtagcaggcccaggagccctgagtcccggaagatgtcggtgaagagggggtccccaccagcgatgctgaggatgctctgcagggccatgagggtgcaggatggcccagggctctccttgatcagatgctgtacctttcgcaggatctcatgaggcacgtagtgcagctcgaacaccagggcctctagaagctggaagaagtgttcctgcactggggccggcttcaggggcatgatctctacaaactgcgagatgggctgcagggtccactccagcaggaagaagtttcgagcattccaggcccacatggtcctgatgactgacaagacttgtatgcagaggacagagtcactggctttgtggaaaacattctgtaggacctggaaggcctgaagattcttaacagtcaccccagatgcctcatgatggaacttgaagccttcaagctgagggtaagtgatgctgtcaaacaccttcagctctgacctcccacaggttgtcagccacaccaccagcccaaggagctcctccagatgcgggtccacttcgctctgggtcagcccatcataccgaagtaacactttgagcagcagaggatagccctctgaattctcaaactccaggaacagagccgaggagacggggtaggagtccttcacgaatcccaagatcaggcttacagcctcgctcacttcaggggcagggagagtgtccgtgagcctggagaggttctggagggagagcctgacacagtctgtggcctgcaggtactggatgatgctgaggttctgggccttggagattgcccttagcacgcagaaggtgggttccttccagaagcagcagctgtgctcccgaaggcaggtcgtggcaatcagcagagactgcagctcacttcctgagaggagtccctccaggccctgagagtcactgcaaatattgagcaacatctgcacgaacatcttttgaacttgaagatcactctcaagaagctcatctttgtccagaggaaagacaaagaagaggtaaaggcactgtaggagcagggctggaagcccagactcagcaaccctgcccagcgtctccgagtctgtccccgtgagcacgtacactgacttcaggagcaagtagccatcctgatccacgtcccccttccaccacagcaactgtccagctgccaaccgagcttgctccgcaggcttccccacaagggccttctggagttgctgggcaagctggtcagacacgtcttcagccagcctttggagactgggaaagcagatgatccccacggagtgttcccaggcctttaggaatagggggagaagactcaacaggctcttctgacgctcaatggggctcttgtgagtcaactgctggtattccagaaacttcctttccagcatgtcccagagagctgtggggctggaggactgccctccatgtgggacatcaggctgcacagcagcaagctgcccttcatttttggaacctgggtcttcatttctgtcttcagcctttgaaagatcttctgcctccatgccgtggcaaagcagatcgtcagaggtcgaggagtgctgctggagcccagcctgactcccaaacttcagcagtgacacacactcaggcagacccaggccctggagtggccctgaccacatgggccccccacgccacacacacttcctgctccccagctcacctcctctcccacattcacaaacccaaaccaggcactg

SEQ ID NO: 19505 - RNA, 2414 nt, Homo sapiens
  source 1..2414: mol_type = other RNA
ttgcctgccctcttcctccagggctccaaaacagcccagcaggcagaggtcctcggccagcttctcaaagagcccattcctcctgaagaagtagccattgacagggtcccagtgcagcgctgcggacacagcacagagagtgtacaaaaccagctccagggtctgtctgggggatactgctccccatgcctgcagcgggggctcctggagggagccttccaggtcagagagcagagacagcagcccgttgaacccgctggagactctgaaggcagcacgacccttgggggtcaccaggatccggagcagagacttcaggagatccagtttcagctgcagctccccttgagtggatgagcatagagcacccacaatgatgctcatgtactcctcggcgttgatggctgagagctgctccaagatgctgagcgaggcctcccggtagcactcgtcatccaggaagatcttgatgaagggcaccatgccgtggtccttcaggacaactgcattcctcaccgagcctttcagaagtgtgactacaatcctcagcatcacacaggtgagttctctttctggatcctgaacaccaggagtggacactttgtttcctgacttcctcatgatcttggcttgcttccgaagctgtgccagtagcaggcccaggagccctgagtcccggaagatgtcggtgaagagggggtccccaccagcgatgctgaggatgctctgcagggccatgagggtgcaggatggcccagggctctccttgatcagatgctgtacctttcgcaggatctcatgaggcacgtagtgcagctcgaacaccagggcctctagaagctggaagaagtgttcctgcactggggccggcttcaggggcatgatctctacaaactgcgagatgggctgcagggtccactccagcaggaagaagtttcgagcattccaggcccacatggtcctgatgactgacaagacttgtatgcagaggacagagtcactggctttgtggaaaacattctgtaggacctggaaggcctgaagattcttaacagtcaccccagatgcctcatgatggaacttgaagccttcaagctgagggtaagtgatgctgtcaaacaccttcagctctgacctcccacaggttgtcagccacaccaccagcccaaggagctcctccagatgcgggtccacttcgctctgggtcagcccatcataccgaagtaacactttgagcagcagaggatagccctctgaattctcaaactccaggaacagagccgaggagacggggtaggagtccttcacgaatcccaagatcaggcttacagcctcgctcacttcaggggcagggagagtgtccgtgagcctggagaggttctggagggagagcctgacacagtctgtggcctgcaggtactggatgatgctgaggttctgggccttggagattgcccttagcacgcagaaggtgggttccttccagaagcagcagctgtgctcccgaaggcaggtcgtggcaatcagcagagactgcagctcacttcctgagaggagtccctccaggccctgagagtcactgcaaatattgagcaacatctgcacgaacatcttttgaacttgaagatcactctcaagaagctcatctttgtccagaggaaagacaaagaagaggtaaaggcactgtaggagcagggctggaagcccagactcagcaaccctgcccagcgtctccgagtctgtccccgtgagcacgtacactgacttcaggagcaagtagccatcctgatccacgtcccccttccaccacagcaactgtccagctgccaaccgagcttgctccgcaggcttccccacaagggccttctggagttgctgggcaagctggtcagacacgtcttcagccagcctttggagactgggaaagcagatgatccccacggagtgttcccaggcctttaggaatagggggagaagactcaacaggctcttctgacgctcaatggggctcttgtgagtcaactgctggtattccagaaacttcctttccagcatgtcccagagagctgtggggctggaggactgccctccatgtgggacatcaggctgcacagcagcaagctgcccttcatttttggaacctgggtcttcatttctgtcttcagcctttgaaagatcttctgcctccatgccgtggcaaagcagatcgtcagaggtcgaggagtgctgctggagcccagcctgactcccaaacttcagcagtgacacacactcaggcagacccaggccctggagtggccctgaccacatgggccccccacgccacacacacttcctgctccccagctcacctcctctcccacattcacaaacccaaaccaggcactgggtcacatgtgccccatagtcagcct

SEQ ID NO: 19506 - RNA, 2417 nt, Homo sapiens
  source 1..2417: mol_type = other RNA
ttgcctgccctcttcctccagggctccaaaacagcccagcaggcagaggtcctcggccagcttctcaaagagcccattcctcctgaagaagtagccattgacagggtcccagtgcagcgctgcggacacagcacagagagtgtacaaaaccagctccagggtctgtctgggggatactgctccccatgcctgcagcgggggctcctggagggagccttccaggtcagagagcagagacagcagcccgttgaacccgctggagactctgaaggcagcacgacccttgggggtcaccaggatccggagcagagacttcaggagatccagtttcagctgcagctccccttgagtggatgagcatagagcacccacaatgatgctcatgtactcctcggcgttgatggctgagagctgctccaagatgctgagcgaggcctcccggtagcactcgtcatccaggaagatcttgatgaagggcaccatgccgtggtccttcaggacaactgcattcctcaccgagcctttcagaagtgtgactacaatcctcagcatcacacaggtgagttctctttctggatcctgaacaccaggagtggacactttgtttcctgacttcctcatgatcttggcttgcttccgaagctgtgccagtagcaggcccaggagccctgagtcccggaagatgtcggtgaagagggggtccccaccagcgatgctgaggatgctctgcagggccatgagggtgcaggatggcccagggctctccttgatcagatgctgtacctttcgcaggatctcatgaggcacgtagtgcagctcgaacaccagggcctctagaagctggaagaagtgttcctgcactggggccggcttcaggggcatgatctctacaaactgcgagatgggctgcagggtccactccagcaggaagaagtttcgagcattccaggcccacatggtcctgatgactgacaagacttgtatgcagaggacagagtcactggctttgtggaaaacattctgtaggacctggaaggcctgaagattcttaacagtcaccccagatgcctcatgatggaacttgaagccttcaagctgagggtaagtgatgctgtcaaacaccttcagctctgacctcccacaggttgtcagccacaccaccagcccaaggagctcctccagatgcgggtccacttcgctctgggtcagcccatcataccgaagtaacactttgagcagcagaggatagccctctgaattctcaaactccaggaacagagccgaggagacggggtaggagtccttcacgaatcccaagatcaggcttacagcctcgctcacttcaggggcagggagagtgtccgtgagcctggagaggttctggagggagagcctgacacagtctgtggcctgcaggtactggatgatgctgaggttctgggccttggagattgcccttagcacgcagaaggtgggttccttccagaagcagcagctgtgctcccgaaggcaggtcgtggcaatcagcagagactgcagctcacttcctgagaggagtccctccaggccctgagagtcactgcaaatattgagcaacatctgcacgaacatcttttgaacttgaagatcactctcaagaagctcatctttgtccagaggaaagacaaagaagaggtaaaggcactgtaggagcagggctggaagcccagactcagcaaccctgcccagcgtctccgagtctgtccccgtgagcacgtacactgacttcaggagcaagtagccatcctgatccacgtcccccttccaccacagcaactgtccagctgccaaccgagcttgctccgcaggcttccccacaagggccttctggagttgctgggcaagctggtcagacacgtcttcagccagcctttggagactgggaaagcagatgatccccacggagtgttcccaggcctttaggaatagggggagaagactcaacaggctcttctgacgctcaatggggctcttgtgagtcaactgctggtattccagaaacttcctttccagcatgtcccagagagctgtggggctggaggactgccctccatgtgggacatcaggctgcacagcagcaagctgcccttcatttttggaacctgggtcttcatttctgtcttcagcctttgaaagatcttctgcctccatgccgtggcaaagcagatcgtcagaggtcgaggagtgctgctggagcccagcctgactcccaaacttcagcagtgacacacactcaggcagacccaggccctggagtggccctgaccacatgggccccccacgccacacacacttcctgctccccagctcacctcctctcccacattcacaaacccaaaccaggcactgggtcacatgtgccccatagtcagcctccc

SEQ ID NO: 19507 - RNA, 2418 nt, Homo sapiens
  source 1..2418: mol_type = other RNA
ttgcctgccctcttcctccagggctccaaaacagcccagcaggcagaggtcctcggccagcttctcaaagagcccattcctcctgaagaagtagccattgacagggtcccagtgcagcgctgcggacacagcacagagagtgtacaaaaccagctccagggtctgtctgggggatactgctccccatgcctgcagcgggggctcctggagggagccttccaggtcagagagcagagacagcagcccgttgaacccgctggagactctgaaggcagcacgacccttgggggtcaccaggatccggagcagagacttcaggagatccagtttcagctgcagctccccttgagtggatgagcatagagcacccacaatgatgctcatgtactcctcggcgttgatggctgagagctgctccaagatgctgagcgaggcctcccggtagcactcgtcatccaggaagatcttgatgaagggcaccatgccgtggtccttcaggacaactgcattcctcaccgagcctttcagaagtgtgactacaatcctcagcatcacacaggtgagttctctttctggatcctgaacaccaggagtggacactttgtttcctgacttcctcatgatcttggcttgcttccgaagctgtgccagtagcaggcccaggagccctgagtcccggaagatgtcggtgaagagggggtccccaccagcgatgctgaggatgctctgcagggccatgagggtgcaggatggcccagggctctccttgatcagatgctgtacctttcgcaggatctcatgaggcacgtagtgcagctcgaacaccagggcctctagaagctggaagaagtgttcctgcactggggccggcttcaggggcatgatctctacaaactgcgagatgggctgcagggtccactccagcaggaagaagtttcgagcattccaggcccacatggtcctgatgactgacaagacttgtatgcagaggacagagtcactggctttgtggaaaacattctgtaggacctggaaggcctgaagattcttaacagtcaccccagatgcctcatgatggaacttgaagccttcaagctgagggtaagtgatgctgtcaaacaccttcagctctgacctcccacaggttgtcagccacaccaccagcccaaggagctcctccagatgcgggtccacttcgctctgggtcagcccatcataccgaagtaacactttgagcagcagaggatagccctctgaattctcaaactccaggaacagagccgaggagacggggtaggagtccttcacgaatcccaagatcaggcttacagcctcgctcacttcaggggcagggagagtgtccgtgagcctggagaggttctggagggagagcctgacacagtctgtggcctgcaggtactggatgatgctgaggttctgggccttggagattgcccttagcacgcagaaggtgggttccttccagaagcagcagctgtgctcccgaaggcaggtcgtggcaatcagcagagactgcagctcacttcctgagaggagtccctccaggccctgagagtcactgcaaatattgagcaacatctgcacgaacatcttttgaacttgaagatcactctcaagaagctcatctttgtccagaggaaagacaaagaagaggtaaaggcactgtaggagcagggctggaagcccagactcagcaaccctgcccagcgtctccgagtctgtccccgtgagcacgtacactgacttcaggagcaagtagccatcctgatccacgtcccccttccaccacagcaactgtccagctgccaaccgagcttgctccgcaggcttccccacaagggccttctggagttgctgggcaagctggtcagacacgtcttcagccagcctttggagactgggaaagcagatgatccccacggagtgttcccaggcctttaggaatagggggagaagactcaacaggctcttctgacgctcaatggggctcttgtgagtcaactgctggtattccagaaacttcctttccagcatgtcccagagagctgtggggctggaggactgccctccatgtgggacatcaggctgcacagcagcaagctgcccttcatttttggaacctgggtcttcatttctgtcttcagcctttgaaagatcttctgcctccatgccgtggcaaagcagatcgtcagaggtcgaggagtgctgctggagcccagcctgactcccaaacttcagcagtgacacacactcaggcagacccaggccctggagtggccctgaccacatgggccccccacgccacacacacttcctgctccccagctcacctcctctcccacattcacaaacccaaaccaggcactgggtcacatgtgccccatagtcagcctccca

SEQ ID NO: 19508 - RNA, 2309 nt, Homo sapiens
  source 1..2309: mol_type = other RNA
ttgcctgccctcttcctccagggctccaaaacagcccagcaggcagaggtcctcggccagcttctcaaagagcccattcctcctgaagaagtagccattgacagggtcccagtgcagcgctgcggacacagcacagagagtgtacaaaaccagctccagggtctgtctgggggatactgctccccatgcctgcagcgggggctcctggagggagccttccaggtcagagagcagagacagcagcccgttgaacccgctggagactctgaaggcagcacgacccttgggggtcaccaggatccggagcagagacttcaggagatccagtttcagctgcagctccccttgagtggatgagcatagagcacccacaatgatgctcatgtactcctcggcgttgatggctgagagctgctccaagatgctgagcgaggcctcccggtagcactcgtcatccaggaagatcttgatgaagggcaccatgccgtggtccttcaggacaactgcattcctcaccgagcctttcagaagtgtgactacaatcctcagcatcacacaggtgagttctctttctggatcctgaacaccaggagtggacactttgtttcctgacttcctcatgatcttggcttgcttccgaagctgtgccagtagcaggcccaggagccctgagtcccggaagatgtcggtgaagagggggtccccaccagcgatgctgaggatgctctgcagggccatgagggtgcaggatggcccagggctctccttgatcagatgctgtacctttcgcaggatctcatgaggcacgtagtgcagctcgaacaccagggcctctagaagctggaagaagtgttcctgcactggggccggcttcaggggcatgatctctacaaactgcgagatgggctgcagggtccactccagcaggaagaagtttcgagcattccaggcccacatggtcctgatgactgacaagacttgtatgcagaggacagagtcactggctttgtggaaaacattctgtaggacctggaaggcctgaagattcttaacagtcaccccagatgcctcatgatggaacttgaagccttcaagctgagggtaagtgatgctgtcaaacaccttcagctctgacctcccacaggttgtcagccacaccaccagcccaaggagctcctccagatgcgggtccacttcgctctgggtcagcccatcataccgaagtaacactttgagcagcagaggatagccctctgaattctcaaactccaggaacagagccgaggagacggggtaggagtccttcacgaatcccaagatcaggcttacagcctcgctcacttcaggggcagggagagtgtccgtgagcctggagaggttctggagggagagcctgacacagtctgtggcctgcaggtactggatgatgctgaggttctgggccttggagattgcccttagcacgcagaaggtgggttccttccagaagcagcagctgtgctcccgaaggcaggtcgtggcaatcagcagagactgcagctcacttcctgagaggagtccctccaggccctgagagtcactgcaaatattgagcaacatctgcacgaacatcttttgaacttgaagatcactctcaagaagctcatctttgtccagaggaaagacaaagaagaggtaaaggcactgtaggagcagggctggaagcccagactcagcaaccctgcccagcgtctccgagtctgtccccgtgagcacgtacactgacttcaggagcaagtagccatcctgatccacgtcccccttccaccacagcaactgtccagctgccaaccgagcttgctccgcaggcttccccacaagggccttctggagttgctgggcaagctggtcagacacgtcttcagccagcctttggagactgggaaagcagatgatccccacggagtgttcccaggcctttaggaatagggggagaagactcaacaggctcttctgacgctcaatggggctcttgtgagtcaactgctggtattccagaaacttcctttccagcatgtcccagagagctgtggggctggaggactgccctccatgtgggacatcaggctgcacagcagcaagctgcccttcatttttggaacctgggtcttcatttctgtcttcagcctttgaaagatcttctgcctccatgccgtggcaaagcagatctaggggcactgtcccgcccttctgttcctgtcactcggatagggtaaaggtgtcctggcccacaggcccacaggtgtgtgaggcgtcagaggtcgaggagt

SEQ ID NO: 19509 - RNA, 2466 nt, Homo sapiens
  source 1..2466: mol_type = other RNA
ttgcctgccctcttcctccagggctccaaaacagcccagcaggcagaggtcctcggccagcttctcaaagagcccattcctcctgaagaagtagccattgacagggtcccagtgcagcgctgcggacacagcacagagagtgtacaaaaccagctccagggtctgtctgggggatactgctccccatgcctgcagcgggggctcctggagggagccttccaggtcagagagcagagacagcagcccgttgaacccgctggagactctgaaggcagcacgacccttgggggtcaccaggatccggagcagagacttcaggagatccagtttcagctgcagctccccttgagtggatgagcatagagcacccacaatgatgctcatgtactcctcggcgttgatggctgagagctgctccaagatgctgagcgaggcctcccggtagcactcgtcatccaggaagatcttgatgaagggcaccatgccgtggtccttcaggacaactgcattcctcaccgagcctttcagaagtgtgactacaatcctcagcatcacacaggtgagttctctttctggatcctgaacaccaggagtggacactttgtttcctgacttcctcatgatcttggcttgcttccgaagctgtgccagtagcaggcccaggagccctgagtcccggaagatgtcggtgaagagggggtccccaccagcgatgctgaggatgctctgcagggccatgagggtgcaggatggcccagggctctccttgatcagatgctgtacctttcgcaggatctcatgaggcacgtagtgcagctcgaacaccagggcctctagaagctggaagaagtgttcctgcactggggccggcttcaggggcatgatctctacaaactgcgagatgggctgcagggtccactccagcaggaagaagtttcgagcattccaggcccacatggtcctgatgactgacaagacttgtatgcagaggacagagtcactggctttgtggaaaacattctgtaggacctggaaggcctgaagattcttaacagtcaccccagatgcctcatgatggaacttgaagccttcaagctgagggtaagtgatgctgtcaaacaccttcagctctgacctcccacaggttgtcagccacaccaccagcccaaggagctcctccagatgcgggtccacttcgctctgggtcagcccatcataccgaagtaacactttgagcagcagaggatagccctctgaattctcaaactccaggaacagagccgaggagacggggtaggagtccttcacgaatcccaagatcaggcttacagcctcgctcacttcaggggcagggagagtgtccgtgagcctggagaggttctggagggagagcctgacacagtctgtggcctgcaggtactggatgatgctgaggttctgggccttggagattgcccttagcacgcagaaggtgggttccttccagaagcagcagctgtgctcccgaaggcaggtcgtggcaatcagcagagactgcagctcacttcctgagaggagtccctccaggccctgagagtcactgcaaatattgagcaacatctgcacgaacatcttttgaacttgaagatcactctcaagaagctcatctttgtccagaggaaagacaaagaagaggtaaaggcactgtaggagcagggctggaagcccagactcagcaaccctgcccagcgtctccgagtctgtccccgtgagcacgtacactgacttcaggagcaagtagccatcctgatccacgtcccccttccaccacagcaactgtccagctgccaaccgagcttgctccgcaggcttccccacaagggccttctggagttgctgggcaagctggtcagacacgtcttcagccagcctttggagactgggaaagcagatgatccccacggagtgttcccaggcctttaggaatagggggagaagactcaacaggctcttctgacgctcaatggggctcttgtgagtcaactgctggtattccagaaacttcctttccagcatgtcccagagagctgtggggctggaggactgccctccatgtgggacatcaggctgcacagcagcaagctgcccttcatttttggaacctgggtcttcatttctgtcttcagcctttgaaagatcttctgcctccatgccgtggcaaagcagatctaggggcactgtcccgcccttctgttcctgtcactcggatagggtaaaggtgtcctggcccacaggcccacaggtgtgtgaggctggaggggtggccgtcagcgcctgtagacatcagaaggcatgggccccctatccccagctgcagcccctcaggctcgggggaagaggacccggccccacatcgtcagtcctcagcgccgtttcactctgaatcactggagctgggtctctgctcatttcctggagaaagcagaa

SEQ ID NO: 19510 - RNA, 2336 nt, Homo sapiens
  source 1..2336: mol_type = other RNA
ttgcctgccctcttcctccagggctccaaaacagcccagcaggcagaggtcctcggccagcttctcaaagagcccattcctcctgaagaagtagccattgacagggtcccagtgcagcgctgcggacacagcacagagagtgtacaaaaccagctccagggtctgtctgggggatactgctccccatgcctgcagcgggggctcctggagggagccttccaggtcagagagcagagacagcagcccgttgaacccgctggagactctgaaggcagcacgacccttgggggtcaccaggatccggagcagagacttcaggagatccagtttcagctgcagctccccttgagtggatgagcatagagcacccacaatgatgctcatgtactcctcggcgttgatggctgagagctgctccaagatgctgagcgaggcctcccggtagcactcgtcatccaggaagatcttgatgaagggcaccatgccgtggtccttcaggacaactgcattcctcaccgagcctttcagaagtgtgactacaatcctcagcatcacacaggtgagttctctttctggatcctgaacaccaggagtggacactttgtttcctgacttcctcatgatcttggcttgcttccgaagctgtgccagtagcaggcccaggagccctgagtcccggaagatgtcggtgaagagggggtccccaccagcgatgctgaggatgctctgcagggccatgagggtgcaggatggcccagggctctccttgatcagatgctgtacctttcgcaggatctcatgaggcacgtagtgcagctcgaacaccagggcctctagaagctggaagaagtgttcctgcactggggccggcttcaggggcatgatctctacaaactgcgagatgggctgcagggtccactccagcaggaagaagtttcgagcattccaggcccacatggtcctgatgactgacaagacttgtatgcagaggacagagtcactggctttgtggaaaacattctgtaggacctggaaggcctgaagattcttaacagtcaccccagatgcctcatgatggaacttgaagccttcaagctgagggtaagtgatgctgtcaaacaccttcagctctgacctcccacaggttgtcagccacaccaccagcccaaggagctcctccagatgcgggtccacttcgctctgggtcagcccatcataccgaagtaacactttgagcagcagaggatagccctctgaattctcaaactccaggaacagagccgaggagacggggtaggagtccttcacgaatcccaagatcaggcttacagcctcgctcacttcaggggcagggagagtgtccgtgagcctggagaggttctggagggagagcctgacacagtctgtggcctgcaggtactggatgatgctgaggttctgggccttggagattgcccttagcacgcagaaggtgggttccttccagaagcagcagctgtgctcccgaaggcaggtcgtggcaatcagcagagactgcagctcacttcctgagaggagtccctccaggccctgagagtcactgcaaatattgagcaacatctgcacgaacatcttttgaacttgaagatcactctcaagaagctcatctttgtccagaggaaagacaaagaagaggtaaaggcactgtaggagcagggctggaagcccagactcagcaaccctgcccagcgtctccgagtctgtccccgtgagcacgtacactgacttcaggagcaagtagccatcctgatccacgtcccccttccaccacagcaactgtccagctgccaaccgagcttgctccgcaggcttccccacaagggccttctggagttgctgggcaagctggtcagacacgtcttcagccagcctttggagactgggaaagcagatgatccccacggagtgttcccaggcctttaggaatagggggagaagactcaacaggctcttctgacgctcaatggggctcttgtgagtcaactgctggtattccagaaacttcctttccagcatgtcccagagagctgtggggctggaggactgccctccatgtgggacatcaggctgcacagcagcaagctgcccttcatttttggaacctgggtcttcatttctgtcttcagcctttgaaagatcttctgcctccatgccgtggcaaagcagatctggaggggtggccgtcagcgcctgtagacatcagaaggcatgggccccctatccccagctgcagcccctcaggctcgggggaagaggacccggccccacatcgtcagtcctcagcgccgtttcactct

SEQ ID NO: 19511 - RNA, 2382 nt, Homo sapiens
  source 1..2382: mol_type = other RNA
ttgcctgccctcttcctccagggctccaaaacagcccagcaggcagaggtcctcggccagcttctcaaagagcccattcctcctgaagaagtagccattgacagggtcccagtgcagcgctgcggacacagcacagagagtgtacaaaaccagctccagggtctgtctgggggatactgctccccatgcctgcagcgggggctcctggagggagccttccaggtcagagagcagagacagcagcccgttgaacccgctggagactctgaaggcagcacgacccttgggggtcaccaggatccggagcagagacttcaggagatccagtttcagctgcagctccccttgagtggatgagcatagagcacccacaatgatgctcatgtactcctcggcgttgatggctgagagctgctccaagatgctgagcgaggcctcccggtagcactcgtcatccaggaagatcttgatgaagggcaccatgccgtggtccttcaggacaactgcattcctcaccgagcctttcagaagtgtgactacaatcctcagcatcacacaggtgagttctctttctggatcctgaacaccaggagtggacactttgtttcctgacttcctcatgatcttggcttgcttccgaagctgtgccagtagcaggcccaggagccctgagtcccggaagatgtcggtgaagagggggtccccaccagcgatgctgaggatgctctgcagggccatgagggtgcaggatggcccagggctctccttgatcagatgctgtacctttcgcaggatctcatgaggcacgtagtgcagctcgaacaccagggcctctagaagctggaagaagtgttcctgcactggggccggcttcaggggcatgatctctacaaactgcgagatgggctgcagggtccactccagcaggaagaagtttcgagcattccaggcccacatggtcctgatgactgacaagacttgtatgcagaggacagagtcactggctttgtggaaaacattctgtaggacctggaaggcctgaagattcttaacagtcaccccagatgcctcatgatggaacttgaagccttcaagctgagggtaagtgatgctgtcaaacaccttcagctctgacctcccacaggttgtcagccacaccaccagcccaaggagctcctccagatgcgggtccacttcgctctgggtcagcccatcataccgaagtaacactttgagcagcagaggatagccctctgaattctcaaactccaggaacagagccgaggagacggggtaggagtccttcacgaatcccaagatcaggcttacagcctcgctcacttcaggggcagggagagtgtccgtgagcctggagaggttctggagggagagcctgacacagtctgtggcctgcaggtactggatgatgctgaggttctgggccttggagattgcccttagcacgcagaaggtgggttccttccagaagcagcagctgtgctcccgaaggcaggtcgtggcaatcagcagagactgcagctcacttcctgagaggagtccctccaggccctgagagtcactgcaaatattgagcaacatctgcacgaacatcttttgaacttgaagatcactctcaagaagctcatctttgtccagaggaaagacaaagaagaggtaaaggcactgtaggagcagggctggaagcccagactcagcaaccctgcccagcgtctccgagtctgtccccgtgagcacgtacactgacttcaggagcaagtagccatcctgatccacgtcccccttccaccacagcaactgtccagctgccaaccgagcttgctccgcaggcttccccacaagggccttctggagttgctgggcaagctggtcagacacgtcttcagccagcctttggagactgggaaagcagatgatccccacggagtgttcccaggcctttaggaatagggggagaagactcaacaggctcttctgacgctcaatggggctcttgtgagtcaactgctggtattccagaaacttcctttccagcatgtcccagagagctgtggggctggaggactgccctccatgtgggacatcaggctgcacagcagcaagctgcccttcatttttggaacctgggtcttcatttctgtcttcagcctttgaaagatcttctgcctccatgccgtggcaaagcagatctggaggggtggccgtcagcgcctgtagacatcagaaggcatgggccccctatccccagctgcagcccctcaggctcgggggaagaggacccggccccacatcgtcagtcctcagcgccgtttcactctgaatcactggagctgggtctctgctcatttcctggagaaagcagaa

SEQ ID NO: 19512 - RNA, 188 nt, Homo sapiens
  source 1..188: mol_type = other RNA
ttgcctgccctcttcctccaggtccttggagcccagtgggcaatcccactcgggacccgatggatccagggagagcatctcgtgggtggagtggctgagagactggcggcggcagcggctcggcgggcgtggcgggcggactcggaccgggcgggatgcagcggcggcggcggtggcagtggcacagc

SEQ ID NO: 19513 - RNA, 757 nt, Homo sapiens
  source 1..757: mol_type = other RNA
ttgcctgccctcttcctccaggtccttggagcccagtgggcaatcccactcgggacccgatggatccagggagagctgagagggcagaagtggtaggtcttgggcagggtgggccagtgggcacattaagtcacccaagggtgtaagccccccactctcccagcctgggctatgttcagggctgacaccgtcccggggactaggagaggaaaggcttgtgttgggggcgaaggcttgttaatgggaacgcaaccgtgggagtgctttgtaaactgttctgtgtggtgcccctggggggagggcaggaagcaatgtcttgccagccagcccctcccgcccctgccatgctgggctccgccttagcttgcttcacagcagcagagttttctgcttgttttgttcatggaggcaaccccagcacctaaagcgtgcctggcacacagccacttctcagtaagtgtttgttgactgaagagtagatgaatgaacgaacccagccatcactctgaggtggcttatttctgtctcatgacccggcatggagtgtgctgacacctaaatgtgattccactgtcatccccacgtaggtcttgaagccctactgtgtgcccagccctgggctaaacattaggaggctagacagtatcccccctgcagatattttgagtcacggaaatgctttctttggatgaaacctaacgtccctcccctctctgaggctggcgcccccccaatatggggctgctgggaggcttcg

SEQ ID NO: 19514 - RNA, 1690 nt, Homo sapiens
  source 1..1690: mol_type = other RNA
ttgcctgccctcttcctccaggtccttggagcccagtgggcaatcccactcgggacccgatggatccagggagagctgagagggcagaagtggtaggtcttgggcagggtgggccagtgggcacattaagtcacccaagggtgtaagccccccactctcccagcctgggctatgttcagggctgacaccgtcccggggactaggagaggaaaggcttgtgttgggggcgaaggcttgttaatgggaacgcaaccgtgggagtgctttgtaaactgttctgtgtggtgcccctggggggagggcaggaagcaatgtcttgccagccagcccctcccgcccctgccatgctgggctccgccttagcttgcttcacagcagcagagttttctgcttgttttgttcatggaggcaaccccagcacctaaagcgtgcctggcacacagccacttctcagtaagtgtttgttgactgaagagtagatgaatgaacgaacccagccatcactctgaggtggcttatttctgtctcatgacccggcatggagtgtgctgacacctaaatgtgattccactgtcatccccacgtaggtcttgaagccctactgtgtgcccagccctgggctaaacattaggaggctagacagtatcccccctgcagatattttgagtcacggaaatgctttctttggatgaaacctaacgtccctcccctctctgaggctggcgcccccccaatatggggctgctgggaggcttcgtgtgaatggaattcttgttctttgcagtccccaggcctggacaggcctggcagctgagtctgtcctccaggggacaggctcggccaccttgagcaagtcgtgaggtctctttggaccttgttgcctggtgcctgccctctcccatcccctgggggctgatgaggctgggacgaagagaatctcttggttgttgggagatggtgtgctgtggcccagacggcagaggactgggcctcatgcctgggctcgaatcccagtttgccagggccagagcctctgtgccgtctcctagaaggtgagctccctgaggggccatggaatgaatgaatgtcacagggcactaagagtgcccacctcccaggatgcagccgcagggtgggggtgggggagctggtcgtgggtctaagctgtctgcagggggcaactcccaggcttaggtcctaggtgctgcctgctgtcctctgggcccactctctgcccagggacttgggccttgtgggggagggaccacagaagactcaccatctcgtgggtggagtggctgagagactgatggcagagacagagggacagagagacgaaggagtcagggcagccaagtccctgcctggccttccagcccctagactttgggagtggagaggtggccgacacctgtccctgcagagagaggccaaggcagccccacccccaccccgaaggtagggagggatttctgctgcccagaccgagtggctcctgccccagtgcggctcacaggtccttcctgccctggggtccgggcttggctctgcccctccagcgcgggggggagttgggggcaccgggtcccgggggtggggggcgtagcgtcgagggtcccgccgcggggagcgggcgcccggggtcctcgtccccgcgactcctgccccggccgcccccctccctggctct

SEQ ID NO: 19515 - RNA, 1392 nt, Homo sapiens
  source 1..1392: mol_type = other RNA
ttgcctgccctcttcctccaggtccttggagcccagtgggcaatcccactcgggacccgatggatccagggagagctgagagggcagaagtggtaggtcttgggcagggtgggccagtgggcacattaagtcacccaagggtgtaagccccccactctcccagcctgggctatgttcagggctgacaccgtcccggggactaggagaggaaaggcttgtgttgggggcgaaggcttgttaatgggaacgcaaccgtgggagtgctttgtaaactgttctgtgtggtgcccctggggggagggcaggaagcaatgtcttgccagccagcccctcccgcccctgccatgctgggctccgccttagcttgcttcacagcagcagagttttctgcttgttttgttcatggaggcaaccccagcacctaaagcgtgcctggcacacagccacttctcagtaagtgtttgttgactgaagagtagatgaatgaacgaacccagccatcactctgaggtggcttatttctgtctcatgacccggcatggagtgtgctgacacctaaatgtgattccactgtcatccccacgtaggtcttgaagccctactgtgtgcccagccctgggctaaacattaggaggctagacagtatcccccctgcagatattttgagtcacggaaatgctttctttggatgaaacctaacgtccctcccctctctgaggctggcgcccccccaatatggggctgctgggaggcttcgtgtgaatggaattcttgttctttgcagtccccaggcctggacaggcctggcagctgagtctgtcctccaggggacaggctcggccaccttgagcaagtcgtgaggtctctttggaccttgttgcctggtgcctgccctctcccatcccctgggggctgatgaggctgggacgaagagaatctcttggttgttgggagatggtgtgctgtggcccagacggcagaggactgggcctcatgcctgggctcgaatcccagtttgccagggccagagcctctgtgccgtctcctagaaggtgagctccctgaggggccatggaatgaatgaatgtcacagggcactaagagtgcccacctcccaggatgcagccgcagggtgggggtgggggagctggtcgtgggtctaagctgtctgcagggggcaactcccaggcttaggtcctaggtgctgcctgctgtcctctgggcccactctctgcccagggacttgggccttgtgggggagggaccacagaagactcaccatctcgtgggtggagtggctgagagactggcggcggcagcggctcggcgggcgtggcgggcggactcggaccgggcgggatgcagcggcggcggcggtggcagtggcacagc

SEQ ID NO: 19516 - RNA, 161 nt, Homo sapiens
  source 1..161: mol_type = other RNA
ttgcctgccctcttcctccaggtccttggagcccagtgggcaatcccactcgggacccgatggatccagggagagctggcggcggcagcggctcggcgggcgtggcgggcggactcggaccgggcgggatgcagcggcggcggcggtggcagtggcacagc

SEQ ID NO: 19517 - RNA, 1963 nt, Homo sapiens
  source 1..1963: mol_type = other RNA
ttgctctgctcccccgcccccagcctcagctgggcgtccagttctgggttgtccagcgacgccctctgggtgccagagtccagccctagctggggtcccagcagggttcagaaggggctctcagccaatctagggaggccaccagccaagggggtctccgcagatgaatcctggctgccaccacccctcccaaactgcagctccttgctgggagggccgtggccgggcgaagatgaggccctgtggttgctggtgttccgctcctcccatagcactttgcccaggcgccagcggtgccaacgccgccgcagctccgactgcacctccttgttgaggaagcagtagaggacagccaccagcaggccctggaaggagctgaggaagaggtcgaagaagagcttggcggagcgcagggtgccctgggcgtgctcgtccgtcacgaaggcgaagaccacttcgtggacgcccagcagagggatgagggtcagcgtggacttggccagccggaacttgtagtctgtgtggtgcatctgccgtgcccgcagcttggccacgagcagctgaacgatgcggacgaagatgaagaagttgatcaggatggccaggaagacggggaaccgcaggatccaccagaagcccatgttgtcattgctggtccagcactggacgttctcgaacagacacttgaccactgcccaggggacgacgaacagcatgggggcaccccagccgatgcccaggtagaggctgaagaagctcctctcggggagggtggccaggcccagcaggttgtgcaggtacaggccctccaccagcagccagcagtagttggccacgatgccatattgcatgaacaccgcggccacacggcagccagccaccgctccatcactgagccaggtgctgacactgaggtcgtcgccaattttctggctgtagcgggtcctgagcagcccatcaatgaccagcacggagctggctttcagcacgaaggacgcaaacagattcgcgtggatggcattgcgggtgcagtgcagcttgctgaggccccccaggatggccaaggcgaggagcagggcccccagggacaggctgtagcccactgtgtacatcacctggaagctgctgtacatcttggccacctccttctggacctcaatctcctcgccatccatctggcactgggaggcatcacgccaaggctgcccccggggtccacgcacccactgaccgtcgggcccgcatctcttgaacacgaagcggtgttgcacaggggcaggagatgttggccgtggtattggcgggggtgtccggccagcaggaatacttgtcgaaggttctgttgcacaccagctctgcccacggtggtgggggcctgaggaatgacagggccccttggcggggtcctcaaaggctgcataagcacccaggaaccttcccatgaagagaactcaggaagtgctgaggccaggcacaggctgaaaggctctgggtggggggctcacccgtgggagggggcagcaggctcaggttgtggtgacactggtcaccgtagagcttccacttctcaaacaggaagtccatcacctgagcggaggggacctgtggctggcaggccagcagcagcagcaacagcagcaggggtcgctgtggctggcaggggggcatgcctctgggcagctagctgcctcccacatctggcaggggctgcacagctggggcaatgcagtcctggtgggtgtgtacgctcctccgagggcagctgagtggcagagcagcagagcctggggcgtcctggccagtggggtgtcctcccctgaagctgcccctctgagcctcagggtccgcgcggcgctgctcgggggtcggcttggctccccgccgtcctctgggcgcgctcgggtcgggcgccggtgaccgctcgtcttcgcggcgctgccagatcggggtcggtgcaaacttt

SEQ ID NO: 19518 - RNA, 1884 nt, Homo sapiens
  source 1..1884: mol_type = other RNA
ttgctctgctcccccgcccccagcctcagctgggcgtccagttctgggttgtccagcgacgccctctgggtgccagagtccagccctagctggggtcccagcagggttcagaaggggctctcagccaatctagggaggccaccagccaagggggtctccgcagatgaatcctggctgccaccacccctcccaaactgcagctccttgctgggagggccgtggccgggcgaagatgaggccctgtggttgctggtgttccgctcctcccatagcactttgcccaggcgccagcggtgccaacgccgccgcagctccgactgcacctccttgttgaggaagcagtagaggacagccaccagcaggccctggaaggagctgaggaagaggtcgaagaagagcttggcggagcgcagggtgccctgggcgtgctcgtccgtcacgaaggcgaagaccacttcgtggacgcccagcagagggatgagggtcagcgtggacttggccagccggaacttgtagtctgtgtggtgcatctgccgtgcccgcagcttggccacgagcagctgaacgatgcggacgaagatgaagaagttgatcaggatggccaggaagacggggaaccgcaggatccaccagaagcccatgttgtcattgctggtccagcactggacgttctcgaacagacacttgaccactgcccaggggacgacgaacagcatgggggcaccccagccgatgcccaggtagaggctgaagaagctcctctcggggagggtggccaggcccagcaggttgtgcaggtacaggccctccaccagcagccagcagtagttggccacgatgccatattgcatgaacaccgcggccacacggcagccagccaccgctccatcactgagccaggtgctgacactgaggtcgtcgccaattttctggctgtagcgggtcctgagcagcccatcaatgaccagcacggagctggctttcagcacgaaggacgcaaacagattcgcgtggatggcattgcgggtgcagtgcagcttgctgaggccccccaggatggccaaggcgaggagcagggcccccagggacaggctgtagcccactgtgtacatcacctggaagctgctgtacatcttggccacctccttctggacctcaatctcctcgccatccatctggcactgggaggcatcacgccaaggctgcccccggggtccacgcacccactgaccgtcgggcccgcatctcttgaacacgaagcggtgttgcactttgtggtgccaaggcaggtaccaggggcaggagatgttggccgtggtattggcgggggtgtccggccagcaggaatacttgtcgaaggttctgttgcacaccagctccgtgggagggggcagcaggctcaggttgtggtgacactggtcaccgtagagcttccacttctcaaacaggaagtccatcacctgagcggaggggacctggcaggccagcagcagcagcaacagcagcaggggtcgctgtggctggcaggggggcatgcctctgggcagctagctgcctcccacatctggcaggggctgcacagctggggcaatgcagtcctggtgggtgtgtacgctcctccgagggcagctgagtggcagagcagcagagcctggggcgtcctggccagtggggtgtcctcccctgaagctgcccctctgagcctcagggtccgcgcggcgctgctcgggggtcggcttggctccccgccgtcctctgggcgcgctcgggtcgggcgccggtgaccgctcgtcttcgcggcgctgccagatcggggtcggtgcaaactttccggcggcgacgcagggcgagggcggcggcggagggcgggctcgggggcggccc

SEQ ID NO: 19519 - RNA, 1818 nt, Homo sapiens
  source 1..1818: mol_type = other RNA
ttgctctgctcccccgcccccagcctcagctgggcgtccagttctgggttgtccagcgacgccctctgggtgccagagtccagccctagctggggtcccagcagggttcagaaggggctctcagccaatctagggaggccaccagccaagggggtctccgcagatgaatcctggctgccaccacccctcccaaactgcagctccttgctgggagggccgtggccgggcgaagatgaggccctgtggttgctggtgttccgctcctcccatagcactttgcccaggcgccagcggtgccaacgccgccgcagctccgactgcacctccttgttgaggaagcagtagaggacagccaccagcaggccctggaaggagctgaggaagaggtcgaagaagagcttggcggagcgcagggtgccctgggcgtgctcgtccgtcacgaaggcgaagaccacttcgtggacgcccagcagagggatgagggtcagcgtggacttggccagccggaacttgtagtctgtgtggtgcatctgccgtgcccgcagcttggccacgagcagctgaacgatgcggacgaagatgaagaagttgatcaggatggccaggaagacggggaaccgcaggatccaccagaagcccatgttgtcattgctggtccagcactggacgttctcgaacagacacttgaccactgcccaggggacgacgaacagcatgggggcaccccagccgatgcccaggtagaggctgaagaagctcctctcggggagggtggccaggcccagcaggttgtgcaggtacaggccctccaccagcagccagcagtagttggccacgatgccatattgcatgaacaccgcggccacacggcagccagccaccgctccatcactgagccaggtgctgacactgaggtcgtcgccaattttctggctgtagcgggtcctgagcagcccatcaatgaccagcacggagctggctttcagcacgaaggacgcaaacagattcgcgtggatggcattgcgggtgcagtgcagcttgctgaggccccccaggatggccaaggcgaggagcagggcccccagggacaggctgtagcccactgtgtacatcacctggaagctgctgtacatcttggccacctccttctggacctcaatctcctcgccatccatctggcactgggaggcatcacgccaaggctgcccccggggtccacgcacccactgaccgtcgggcccgcatctcttgaacacgaagcggtgttgcactttgtggtgccaaggcaggtaccaggggcaggagatgttggccgtggtattggcgggggtgtccggccagcaggaatacttgtcgaaggttctgttgcacaccagctccgtgggagggggcagcaggctcaggttgtggtgacactggtcaccgtagagcttccacttctcaaacaggaagtccatcacctgagcggaggggacctgtggctggcaggccagcagcagcagcaacagcagcaggggtcgctgtggctggcaggggggcatgcctctgggcagctagctgcctcccacatctggcaggggctgcacagctggggcaatgcagtcctggtgggtgtgtacgctcctccgagggcagctgagtggcagagcagcagagcctggggcgtcctggccagtggggtgtcctcccctgaagctgcccctctgagcctcagggtccgcgcggcgctgctcgggggtcggcttggctccccgccgtcctctgggcgcgctcgggtcgggcgccggtgaccgctcgtcttcgcggcgctgccagatc

SEQ ID NO: 19520 - RNA, 1865 nt, Homo sapiens
  source 1..1865: mol_type = other RNA
ttgctctgctcccccgcccccagcctcagctgggcgtccagttctgggttgtccagcgacgccctctgggtgccagagtccagccctagctggggtcccagcagggttcagaaggggctctcagccaatctagggaggccaccagccaagggggtctccgcagatgaatcctggctgccaccacccctcccaaactgcagctccttgctgggagggccgtggccgggcgaagatgaggccctgtggttgctggtgttccgctcctcccatagcactttgcccaggcgccagcggtgccaacgccgccgcagctccgactgcacctccttgttgaggaagcagtagaggacagccaccagcaggccctggaaggagctgaggaagaggtcgaagaagagcttggcggagcgcagggtgccctgggcgtgctcgtccgtcacgaaggcgaagaccacttcgtggacgcccagcagagggatgagggtcagcgtggacttggccagccggaacttgtagtctgtgtggtgcatctgccgtgcccgcagcttggccacgagcagctgaacgatgcggacgaagatgaagaagttgatcaggatggccaggaagacggggaaccgcaggatccaccagaagcccatgttgtcattgctggtccagcactggacgttctcgaacagacacttgaccactgcccaggggacgacgaacagcatgggggcaccccagccgatgcccaggtagaggctgaagaagctcctctcggggagggtggccaggcccagcaggttgtgcaggtacaggccctccaccagcagccagcagtagttggccacgatgccatattgcatgaacaccgcggccacacggcagccagccaccgctccatcactgagccaggtgctgacactgaggtcgtcgccaattttctggctgtagcgggtcctgagcagcccatcaatgaccagcacggagctggctttcagcacgaaggacgcaaacagattcgcgtggatggcattgcgggtgcagtgcagcttgctgaggccccccaggatggccaaggcgaggagcagggcccccagggacaggctgtagcccactgtgtacatcacctggaagctgctgtacatcttggccacctccttctggacctcaatctcctcgccatccatctggcactgggaggcatcacgccaaggctgcccccggggtccacgcacccactgaccgtcgggcccgcatctcttgaacacgaagcggtgttgcactttgtggtgccaaggcaggtaccaggggcaggagatgttggccgtggtattggcgggggtgtccggccagcaggaatacttgtcgaaggttctgttgcacaccagctccgtgggagggggcagcaggctcaggttgtggtgacactggtcaccgtagagcttccacttctcaaacaggaagtccatcacctgagcggaggggacctgtggctggcaggccagcagcagcagcaacagcagcaggggtcgctgtggctggcaggggggcatgcctctgggcagctagctgcctcccacatctggcaggggctgcacagctggggcaatgcagtcctggtgggtgtgtacgctcctccgagggcagctgagtggcagagcagcagagcctggggcgtcctggccagtggggtgtcctcccctgaagctgcccctctgagcctcagggtcctggagctgggcccccaggatgggtggagcggccactggtccaggaaggcagcggggctcccagggcgtccgcaaggggcctctcagacgctttgaggagctccgggatgggagccgggatgtttttgtgaaaccagagaaggtagt

SEQ ID NO: 19521 - RNA, 1673 nt, Homo sapiens
  source 1..1673: mol_type = other RNA
ttgctctgctcccccgcccccagcctcagctgggcgtccagttctgggttgtccagcgacgccctctgggtgccagagtccagccctagctggggtcccagcagggttcagaaggggctctcagccaatctagggaggccaccagccaagggggtctccgcagatgaatcctggctgccaccacccctcccaaactgcagctccttgctgggagggccgtggccgggcgaagatgaggccctgtggttgctggtgttccgctcctcccatagcactttgcccaggcgccagcggtgccaacgccgccgcagctccgactgcacctccttgttgaggaagcagtagaggacagccaccagcaggccctggaaggagctgaggaagaggtcgaagaagagcttggcggagcgcagggtgccctgggcgtgctcgtccgtcacgaaggcgaagaccacttcgtggacgcccagcagagggatgagggtcagcgtggacttggccagccggaacttgtagtctgtgtggtgcatctgccgtgcccgcagcttggccacgagcagctgaacgatgcggacgaagatgaagaagttgatcaggatggccaggaagacggggaaccgcaggatccaccagaagcccatgttgtcattgctggtccagcactggacgttctcgaacagacacttgaccactgcccaggggacgacgaacagcatgggggcaccccagccgatgcccaggtagaggctgaagaagctcctctcggggagggtggccaggcccagcaggttgtgcaggtacaggccctccaccagcagccagcagtagttggccacgatgccatattgcatgaacaccgcggccacacggcagccagccaccgctccatcactgagccaggtgctgacactgaggtcgtcgccaattttctggctgtagcgggtcctgagcagcccatcaatgaccagcacggagctggctttcagcacgaaggacgcaaacagattcgcgtggatggcattgcgggtgcagtgcagcttgctgaggccccccaggatggccaaggcgaggagcagggcccccagggacaggctgtagcccactgtgtacatcacctggaagctgctgtacatcttggccacctccttctggacctcaatctcctcgccatccatctggcactgggaggcatcacgccaaggctgcccccggggtccacgcacccactgaccgtcgggcccgcatctcttgaacacgaagcggtgttgcactttgtggtgccaaggcaggtaccaggggcaggagatgttggccgtggtattggcgggggtgtccggccagcaggaatacttgtcgaaggttctgttgcacaccagctctgcccacggtggtgggggcctgaggaatgacagggccccttggcggggtcctcaaaggctgcataagcacccaggaaccttcccatgaagagaactcaggaagtgctgaggccaggcacaggctgaaaggctctgggtggggggctcacccgtgggagggggcagcaggctcaggttgtggtgacactggtcaccgtagagcttccacttctcaaacaggaagtccatcacctgagcggaggggacctggcaggccagcagcagcagcaacagcagcaggggtcgctgtggctg

SEQ ID NO: 19522 - RNA, 1175 nt, Homo sapiens
  source 1..1175: mol_type = other RNA
ttgctctgctcccccgcccccaggtggctggggcttctgttttctctttagtctgcaagttattgaaaaactgagtctatttatttcttcatttctgtatattcagtcatatagtaggagctcagaaaggtttctttttttttttttttattttaactccattctattgaactgaaaagataggtaccaaatccaagaaatgccaggctattctctctgattacgtctttctggttgagcacactgaatctacgtgggtttggggaggggtgtggagcgcccaaggatgacacacactgacctcccggctcacagaccacatgcatagcgtcattacatggagcgcctgttactggctgtgttatattaaaaacatccaagaaacaatatgatgaggcagtactagaggcagggagagaatgccctgtcaaagggtctgtaatgtgtaaagtgagtaaaactctatgaaaacccaggtctgtgagactcaaaatttccaccaagacctttatgctctacaacaggggcattgccactttggaaatatttgctttattctcaatccccatgagatatttagtattaaaaattaggaagaggccaggcgagatggctcatgcctgtaatgccagaactttgggagaccaagactggctgatcacctgaggtcaggagttcgaggccactctgttcaccatggcaaaaccccatctctactaaaaatacaaaaattttctgggcatggtggcaggcacctgtaatcccagctactctggaggctgagccaggaaaattgcttgaacccaggaggcagaggttgcagtgagctccaagctgggcgacagagggagattccgtctcaggcagtggctgcctctctccttccctctcaagccatagcatcttcagtggtcgctgccattgacccgcctgccttgattggagtcatcaaaatcgattcccctggagatgccattgtggatgacatcatcttccacttggagtcctcggtgcccagtgcagtggctggatcacaagctctcactaaaaatatgtgtttaactgggcaaaaaaaaaaaaaaaaaaaaaaaaaaaattttcatcctgagatttttgggaatctggaaaaacaggttctatttctgatttttttcacaactttttatatgaattta

SEQ ID NO: 19523 - RNA, 6017 nt, Homo sapiens
  source 1..6017: mol_type = other RNA
ttgctgacctgggtggtggtaaaacatgtacatgattatttattatacctcgatgtaaaatattttacagctcagctttttaggaaagagcccgatgaaaaaggaaaagaaaagttaaagagctgagtatggaggggatgtttcagcctggctcttgcgtaaggtgaccagctgtcccaatctgcctgggactgatggggtttcctggggcaagagactttcagtgctaaaacagggagagtcctgggcaaactaggacagctggtcacccaactcttgtggaagaggggaattgagatcgagtactgaatatctggcagagaggctggaatccttcagccccagagcccagggaccactccagtagatgcagagaggggcctgcccaggggtcagggcagtgggtatcactggtgacatcaagaatatcagggctggggaggcatctttgtttcctggtgccctcctcaaagttgctgacactttggggacgggaaggggtagaagtagggctgctccttttggagctggagggaatagacctggagacagagttgaggcagtcgggctgtccaggttctaagcatcacagcttctgcactgggctctgaggagattctcagccagaggatcccagcctcctcctccctcaaatgtcagtccaagcaaataccaaagcaacgcatcgattttgtggaagtcaattagagatgtggggagctatcggagacaagcactattgtaccttttcacctccacacttgtcacaagcagggactgtctcctccccactttgcttgccacgcctgccatggcttgagctggggtgaggagtggtctttatcttctttgggagatcctgactggttgcgcacttgctaagggcaggaagtctggagggctgcaggaatggtgccgttgataaacaggtggacttataatcatcatgcactgcaattgtagaacatagtctcctgccttttctcatttgtataattgtctgggtcaatattctcccaatattgggaggggctctgcagccctccagctgaggcctaaggtggattctgatggagagattgccagcagggctgggcaacttaggtgcacagaagagaaggcaggatactggaagcagcagccagggaggacaggctcagaagttctcatagtggtgcatgaagtgggctcggtcctgcctgttgacgagctgacaggccttctctacattcttggtcattcctggagggccgcagctgaacaccccgatcttgcgcacctgtgggtggacctcctgcagggagttgaagaagggctcgaaggggggacggccaaagtgggtgatggagcgcaggcccgtgaacagactccggttcagcactttctggaagtgccgctcgcagatgtatagcatggtggtcctgaggtcgaacttctcagccagctgggtgacataaatgtgcacagacaccaggtcctggtggtcgttctcctccacctcttggatgatgtcagccagccactcaaactgacgctgggtccgtgtcacccagatgaagtagatcttcttacacagcatttggctgcccaaggatgacttgaagaccaggtctttgaggatggaggcaaagggggtgaccccaatgccccctcccaccaacactgacacctcaaatttatgccactcctgatggccctctccaaacggtccatcaaggtacagctttgggtatccagcacagccattgccctttggggatgagtagatctccctgaggcgagtggtccagggccccactgcccggatgtgcaggctgagtgtgtcctcatggggcgcggaggtcagtgtgaaggggtggtactcggtggtccccagagccaggcaggcgatccgcacccactgtcctgacttgtactcaaagccttggggcctctggaattgcaggtaggtcactcctgagggcagcagctccgccttcaccacgctgatctccaccttcttccggctcaggctcaccagcttgtcacctccatagatgattgccgggaccaggaagtagatgtggaaagtgggcagctggatcagagcatagctgccatggatgatgagcagggcatagagcaggatgtagaggtggtgggtcagccagaagccccggaagctgcggcggcggaagtggtgggaggcgaagacatacatgatggccaggaccaggagcagaagcacacctgtcatacctgggacggtctggaagaaccaccaatagaacttctggggaagcttggacccatcattcacaaagacgttggggaatatgcaggccagcaggctgagtgggctgactgagaagatgtagacattgactgcgtggccagcactgtgcaaaatggccaggacaacagcagccatggcgatccagcggtggaagtccactgcggcatcaaaaggcacatagcggttgaggaaagtctctcgcaggaaggttatgaggttgcggcacatggtgagcaagatataagagaacatgaaggagacgctggccgccgtgcctcgtgacaggatgatgcccacgagggtggtctgtgcaatgtccgagggtggcgaggcaaagccatagtagtaagcacgatctgcaaacacgccaacacagatggccgagaagattgccacacacacgatgtgcctccggtagttctccacgaagcgcttgtactgctgcagcttttgggctaggaagcctcgctgcatcttctcttgcagcgcctctgtgtacagccggggagtgggcactgctgcctttttgccaaacctcttcttcagtccagggcctcccagctctggggcttctggggcagggggccccagtccctgggggtgggagcgctccccaggtgtccgagtgatgaacgagactcgacagctgatgttttgtttaaagatatctctaataccatttccacctccacctccacctttgacacagagctgcgtgaagcggagctcgctgtcatggtcccgcagcatgaagtgaaaatcctcccatgtcagctcctccttgtcctggaatcccgactcccggaacatagactccaccacctcggccagctgggccttggacaggcagttgttggagatctcgatgaaggatcgcatcatggtgaagaattcgtccttggagaggaagccattctcatccaggtcatacatggtaaacattagacgggacttatcctctggggagcctttcatgaagaccaccaggatgtccaggaactctcggaaggacaggtagccattgccatccttgtcagccagagagaacatggactccacaaacatgtcctggggcttgaggcccagggactcggcaaactcggccctgctcagctcgcaggtcagggcctcccgcaccttctgggaggagtccaggggcagggtccctgcgtcggcctggttgatgtccagcacctgagcaaaaaggtgtctgaagaagatctccaggatgcgttcccgctgctgctttgtcacagccttcctaaatagctccttctcgctcatctcagccacatggaggcccagagcccagcgcacgcagaagtcccatagctgctgcacaaaggcgccccgttcctcttcagaactaaacagcagcaccaggtcatactccttagggatcttgagcagcagggtgcggcatcctcggttgttggacaggatgaggttgacctgctgcagaggctgcagctggaccacacggagcacagtgagatgcctgttcaggacctgcagacacctgtctgacagcagctggatgatgatgggactgctcctctccttggggcctggccactccatcgctggcactccatctttggctgcttccttcttcacgctctctttgagtttcttttgtagcttcttgtgttctcggccccggaaataggccaccactccagagagaagcagactcactaagggaaggcagcagagagcaatgatggtgatggcaaaaccagggctgctgccttcaaagaagtcaagcacagtcaggggtgcacactggggcaggccgtcagttgtgagctgcttaggttgagggcagggtgcacctttatgccagacaaagacattgggctgcagggcactggggtcaatgttgataacagcgaccagcacgtcccgcagggtggtatttcggatgtcttcaatctccttcttggagaacagcccattcctggtgttctcaaaccagtagcggtcaccatcccgcagccgtacaaactggtcgaggacaatggcactgaacaggggtccagggtccccatggctctccaggagccccccaaggagcagctctagctgggataggtcctggttgtacagggcagctgtggcctccagcacctgggggtccacattagggttgagatcactccagttccttgggatgtccagcccaaaggccagcagggcctggctatagctgggcagccccatatctcggccacgttggatgctgctggccacatagtctgtacgggagaatttgccagggccaggccagtaatccctcagatcttcaaccactatgttgtcctccaactccgaaatctgggaggccattcccagcagcagctcattcacctcctgggtactgttcagattggggttctcccgaatccagtagttgttgcagaccctgagagcttgggagctttgaaaacccttgttcaggaccttccggaaatgacagctggcatttctcatgtagacaccagggggcaccatggtagagaagaactgctcagaggccaccacaaattccggggagatgctggggtctaggaaaggacggtatcctgtatactccgggagtgttttctgcaggaagctgggcagccactcatacacagcgatgttctggtaggtggcgatgaccctcttgcgtgcgtgctggaacagctcctcgtcctcccagtctgggtgctggcgggccagcctctgcgcccacaggttgtggtagcggaaccagagcaggcccagcgcctgcaggaagggttcccggttccctctctctgccccgaaggcgtacagcccccggggcccgttctgcccggtggcggggtcgggcgccgcccacatgagcagggggttctgcgagtctcgggggaaagcggggtcgggccccgacgccagctgtccccccgagaagctccgcagcgcgtcgctccaggagtgcgaggagccatagatggcgctgccgtccagccagcccgtcacctggttggccaggtcccgggggttgctgggactccgtccggtctcggggtcccagcggctcctctggaagggcagcaccacgtccccgcgctggtcggggtcgaacacggggtctccaggtgggatgcggatgttgaggaactcggcggggcaaccgggcgtttccacgctcaccacgtcggaaagaacatggtagccaaagaagacccccagtacggtgcggttgtggagcgacggcaggccggctatgccccgcgtggctgcgttgctgagccggcgcgggttgggcagctgcggctcctccagagcctgatacacaccgtcggcgtaattggctggtacgcggcgctgcaaccggcagccaacagcaccacgctcgtggtgcctcaggttgttaaaccagccgtcatagcgctgcacttcccagggcagtgagagtgcgtcctgactgcccgatggacccagggatccagtcagaagagctcccaggagcatcagtgcctctggtcttgcacggagcatgccaaccctgcagcctgtggtttagggtggtgttgggttcagatgtcttctttcctcttaaaatctttgcttctgtgctctacttcttgccttcaccctcactcttccagctccgccgatcctcagcctccccggctgcactctcacctttctctctgggtccttggtctcgccactgtgcaggtgtcggctcaggacagacctgcgccagtgt

SEQ ID NO: 19524 - RNA, 6017 nt, Homo sapiens
  source 1..6017: mol_type = other RNA
ttgctgacctgggtggtggtaaaacatgtacatgattatttattatacctcgatgtaaaatattttacagctcagctttttaggaaagagcccgatgaaaaaggaaaagaaaagttaaagagctgagtatggaggggatgtttcagcctggctcttgcgtaaggtgaccagctgtcccaatctgcctgggactgatggggtttcctggggcaagagactttcagtgctaaaacagggagagtcctgggcaaactaggacagctggtcacccaactcttgtggaagaggggaattgagatcgagtactgaatatctggcagagaggctggaatccttcagccccagagcccagggaccactccagtagatgcagagaggggcctgcccaggggtcagggcagtgggtatcactggtgacatcaagaatatcagggctggggaggcatctttgtttcctggtgccctcctcaaagttgctgacactttggggacgggaaggggtagaagtagggctgctccttttggagctggagggaatagacctggagacagagttgaggcagtcgggctgtccaggttctaagcatcacagcttctgcactgggctctgaggagattctcagccagaggatcccagcctcctcctccctcaaatgtcagtccaagcaaataccaaagcaacgcatcgattttgtggaagtcaattagagatgtggggagctatcggagacaagcactattgtaccttttcacctccacacttgtcacaagcagggactgtctcctccccactttgcttgccacgcctgccatggcttgagctggggtgaggagtggtctttatcttctttgggagatcctgactggttgcgcacttgctaagggcaggaagtctggagggctgcaggaatggtgccgttgataaacaggtggacttataatcatcatgcactgcaattgtagaacatagtctcctgccttttctcatttgtataattgtctgggtcaatattctcccaatattgggaggggctctgcagccctccagctgaggcctaaggtggattctgatggagagattgccagcagggctgggcaacttaggtgcacagaagagaaggcaggatactggaagcagcagccagggaggacaggctcagaagttctcatagtggtgcatgaagtgggctcggtcctgcctgttgacgagctgacaggccttctctacattcttggtcattcctggagggccgcagctgaacaccccgatcttgcgcacctgtgggtggacctcctgcagggagttgaagaagggctcgaaggggggacggccaaagtgggtgatggagcgcaggcccgtgaacagactccggttcagcactttctggaagtgccgctcgcagatgtatagcatggtggtcctgaggtcgaacttctcagccagctgggtgacataaatgtgcacagacaccaggtcctggtggtcgttctcctccacctcttggatgatgtcagccagccactcaaactgacgctgggtccgtgtcacccagatgaagtagatcttcttacacagcatttggctgcccaaggatgacttgaagaccaggtctttgaggatggaggcaaagggggtgaccccaatgccccctcccaccaacactgacacctcaaatttatgccactcctgatggccctctccaaacggtccatcaaggtacagctttgggtatccagcacagccattgccctttggggatgagtagatctccctgaggcgagtggtccagggccccactgcccggatgtgcaggctgagtgtgtcctcatggggcgcggaggtcagtgtgaaggggtggtactcggtggtccccagagccaggcaggcgatccgcacccactgtcctgacttgtactcaaagccttggggcctctggaattgcaggtaggtcactcctgagggcagcagctccgccttcaccacgctgatctccaccttcttccggctcaggctcaccagcttgtcacctccatagatgattgccgggaccaggaagtagatgtggaaagtgggcagctggatcagagcatagctgccatggatgatgagcagggcatagagcaggatgtagaggtggtgggtcagccagaagccccggaagctgcggcggcggaagtggtgggaggcgaagacatacatgatggccaggaccaggagcagaagcacacctgtcatacctgggacggtctggaagaaccaccaatagaacttctggggaagcttggacccatcattcacaaagacgttggggaatatgcaggccagcaggctgagtgggctgactgagaagatgtagacattgactgcgtggccagcactgtgcaaaatggccaggacaacagcagccatggcgatccagcggtggaagtccactgcggcatcaaaaggcacatagcggttgaggaaagtctctcgcaggaaggttatgaggttgcggcacatggtgagcaagatataagagaacatgaaggagacgctggccgccgtgcctcgtgacaggatgatgcccacgagggtggtctgtgcaatgtccgagggtggcgaggcaaagccatagtagtaagcacgatctgcaaacacgccaacacagatggccgagaagattgccacacacacgatgtgcctccggtagttctccacgaagcgcttgtactgctgcagcttttgggctaggaagcctcgctgcatcttctcttgcagcgcctctgtgtacagccggggagtgggcactgctgcctttttgccaaacctcttcttcagtccagggcctcccagctctggggcttctggggcagggggccccagtccctgggggtgggagcgctccccaggtgtccgagtgatgaacgagactcgacagctgatgttttgtttaaagatatctctaataccatttccacctccacctccacctttgacacagagctgcgtgaagcggagctcgctgtcatggtcccgcagcatgaagtgaaaatcctcccatgtcagctcctccttgtcctggaatcccgactcccggaacatagactccaccacctcggccagctgggccttggacaggcagttgttggagatctcgatgaaggatcgcatcatggtgaagaattcgtccttggagaggaagccattctcatccaggtcatacatggtaaacattagacgggacttatcctctggggagcctttcatgaagaccaccaggatgtccaggaactctcggaaggacaggtagccattgccatccttgtcagccagagagaacatggactccacaaacatgtcctggggcttgaggcccagggactcggcaaactcggccctgctcagctcgcaggtcagggcctcccgcaccttctgggaggagtccaggggcagggtccctgcgtcggcctggttgatgtccagcacctgagcaaaaaggtgtctgaagaagatctccaggatgcgttcccgctgctgctttgtcacagccttcctaaatagctccttctcgctcatctcagccacatggaggcccagagcccagcgcacgcagaagtcccatagctgctgcacaaaggcgccccgttcctcttcagaactaaacagcagcaccaggtcatactccttagggatcttgagcagcagggtgcggcatcctcggttgttggacaggatgaggttgacctgctgcagaggctgcagctggaccacacggagcacagtgagatgcctgttcaggacctgcagacacctgtctgacagcagctggatgatgatgggactgctcctctccttggggcctggccactccatcgctggcactccatctttggctgcttccttcttcacgctctctttgagtttcttttgtagcttcttgtgttctcggccccggaaataggccaccactccagagagaagcagactcactaagggaaggcagcagagagcaatgatggtgatggcaaaaccagggctgctgccttcaaagaagtcaagcacagtcaggggtgcacactggggcaggccgtcagttgtgagctgcttaggttgagggcagggtgcacctttatgccagacaaagacattgggctgcagggcactggggtcaatgttgataacagcgaccagcacgtcccgcagggtggtatttcggatgtcttcaatctccttcttggagaacagcccattcctggtgttctcaaaccagtagcggtcaccatcccgcagccgtacaaactggtcgaggacaatggcactgaacaggggtccagggtccccatggctctccaggagccccccaaggagcagctctagctgggataggtcctggttgtacagggcagctgtggcctccagcacctgggggtccacattagggttgagatcactccagttccttgggatgtccagcccaaaggccagcagggcctggctatagctgggcagccccatatctcggccacgttggatgctgctggccacatagtctgtacgggagaatttgccagggccaggccagtaatccctcagatcttcaaccactatgttgtcctccaactccgaaatctgggaggccattcccagcagcagctcattcacctcctgggtactgttcagattggggttctcccgaatccagtagttgttgcagaccctgagagcttgggagctttgaaaacccttgttcaggaccttccggaaatgacagctggcatttctcatgtagacaccagggggcaccatggtagagaagaactgctcagaggccaccacaaattccggggagatgctggggtctaggaaaggacggtatcctgtatactccgggagtgttttctgcaggaagctgggcagccactcatacacagcgatgttctggtaggtggcgatgaccctcttgcgtgcgtgctggaacagctcctcgtcctcccagtctgggtgctggcgggccagcctctgcgcccacaggttgtggtagcggaaccagagcaggcccagcgcctgcaggaagggttcccggttccctctctctgccccgaaggcgtacagcccccggggcccgttctgcccggtggcggggtcgggcgccgcccacatgagcagggggttctgcgagtctcgggggaaagcggggtcgggccccgacgccagctgtccccccgagaagctccgcagcgcgtcgctccaggagtgcgaggagccatagatggcgctgccgtccagccagcccgtcacctggttggccaggtcccgggggttgctgggactccgtccggtctcggggtcccagcggctcctctggaagggcagcaccacgtccccgcgctggtcggggtcgaacacggggtctccaggtgggatgcggatgttgaggaactcggcggggcaaccgggcgtttccacgctcaccacgtcggaaagaacatggtagccaaagaagacccccagtacggtgcggttgtggagcgacggcaggccggctatgccccgcgtggctgcgttgctgagccggcgcgggttgggcagctgcggctcctccagagcctgatacacaccgtcggcgtaattggctggtacgcggcgctgcaaccggcagccaacagcaccacgctcgtggtgcctcaggttgttaaaccagccgtcatagcgctgcacttcccagggcagtgagagtgcgtcctgattgcccgatggacccagggatccagtcagaagagctcccaggagcatcagtgcctctggtcttgcacggagcatgccaaccctgcagcctgtggtttagggtggtgttgggttcagatgtcttctttcctcttaaaatctttgcttctgtgctctacttcttgccttcaccctcactcttccagctccgccgatcctcagcctccccggctgcactctcacctttctctctgggtccttggtctcgccactgtgcaggtgtcggctcaggacagacctgcgccagtgt

SEQ ID NO: 19525 - RNA, 877 nt, Homo sapiens
  source 1..877: mol_type = other RNA
ttgctgacctgggtggtggtataggcgtctccattgcggtatctggtgacctggcgggtgcggcggacatagtggtagctgatggccttccaccagatgcagggcgtggcttgctgcatgcggcccacacgttcccgcacactgctcacatcaacacggtgctgcagctcatggcgggcttggcagtgccaacactccaccaggtagacggcgtacaacatgagcaggaaggccagggggatgtagacatagccgttggagcaggggctgtcatggtacatgaggctgttgccctggtaggcgctgctgaaggtgaggcgcgtcactgtggtgacgtggcaccaggccactgcccccaggcagccgtacatgagcagcgagagcaggaggcacttccagtgggactcacggcagagggacttggtgaaagagggctggatgggacgctgctcctctcgggcggggccctcgtccgccgccgccgctgccgccgccgccgtgagctcctccgagaccccggggccgccaccgccgccgccgccgccggcggcgctctctcccgcggccgagccagggggggacatggcgtagagggggcgcgtcgagctcaggacctcccggggggctgccaggggccgggggcatcctgcgcgggccctggggagaggacgggagggggcggggccctcgctgctccccaccccccgccgggggagggggcccggaaagggcaccgggagtaaggggctgggggctgagggtgggaggcaggctggggggccgggccggggggggccggggccgggggcgggtgtcaccttgaggccctcgcggcgccgctccgcctcccgcccgctcccgccgccgccttttgtct

SEQ ID NO: 19526 - RNA, 797 nt, Homo sapiens
  source 1..797: mol_type = other RNA
ttgctgacctgggtggtggtgaggccggtggcctcggccagctcccgcttctcacgcggcgatgggtagggattgtgcgcgtaccactcccgcaggacacccctcgacttctccttgaagcagtagctggtctcctcgccgtcccagatggtgcgcggcagtggaaattttcggcgcacccgatatttgcccacggcgcccaggggtcggccgcgcagcttctcggcctccacgtaatgcgccttcagccacagttgctgcagtttggggtggttgtgaggcgagaactggtggctctccaggatcttgtagagctcacggaagttgccgcggtggaaggcgaccaccgccttggccttgagtacgctctcgttcttgtgcaggtggtcgcaggcgggcagtgaccacaggaacctgcccaggcgctccaggtttccgccttgctgcagaacctcgcacacgcacgccacttgctcctgcgtaaagccaaacgacggcagcatcgacatggctggggcctgccggggcgcacggcccaggcgcacgcggcagggagcagagccgagaggcagggggcggcggccgcagggaggggggcgcggctgttcctaacctcctccttaggctttgcaaaggcgaaaaccggagtcggaacttggcggtgggcggccaaggaagagaaggcggaggagtaggggaggttctggacacggaacggccggcgcactcagtagcctttaaggccttgctgcctccgacctcccgcccggtggatgctgctagttgccggggaactt

SEQ ID NO: 19527 - RNA, 4583 nt, Homo sapiens
  source 1..4583: mol_type = other RNA
ttgctgacctgggtggtggtggcagcaggagggtctgggacacagggaggcttgagttgaactaaacaggttgaaagggaccaggggaattgttggcgcaacccacacttcatgcaaggcacatgtgctctcctgcgggtctgcagggaaccggcccagagagccccgcggcaggccctggaacacccgcctctgacctgagaaggggcagcaagggagcaagtgccggacattctgctggggtgacaaatggaaaatcggcaacagggttccgattttctttgccacaggggacccgcctgttgaaagctcgcttcaaaatagaaacggcagcatctcaacacacttcttgcacttcagcatcaaactcaccttggggagaagagggcagtgggtttgcagtggggacagaggggcatgggaagaggggtgattccgggggggagtgagcaggcggcggctggcctctcccacggtgatgctctttcctctgtgcctggcagctacttgtcctctgtgcactccggcatgcctgcctctagcagggcagcccggaactgcgtcaggacaccccggatgctcttgatgaaacccttggaaagtgggaagagggggaagccgatgtcagggtagccactcttctcaggtaagaagctccggtagctctttctccgcttctttggtttcacactgggtggcaccgatgcgtctggtgcggtctccgaagtctggtctgtgtggtccctgctagctgaggccaggccctgggcaccgccctctgagtctgagccctgggaggcctctcctggggctggccctccatcctcaggttcttgttggccggagtctgacagctcggctacagctgggggctctggcgagctgctggccttgggcaccccgttgggcagtgcctgggccttctccagcagggcatgggtttccagccaggactcgatacggttcaccagccgccagccaccagtgctaaagtgttgcctgatctcctgctcaaagacctcggggggccgccgcaccagctgggtcatggactgcaccacgcggatcagcgccatctcattgtaacagcgactgttttcatagccttcctgcaggcctcggtcactgtcgaagccggcttcgttgtagtatggttcatttaccaggatcagaccttggatggagatgagcacctggagaaggctggacttgcttgtccacctctctgtcccctttccaatccaggtgcccaggaggctgacacacaccttcccattgtcatacaggttggggttcaggcggccactgcattgggagaggtagcagaagtgggggggcacggctgggtagatgttggggagctggatgtcaaacaagtagaggccatcctcgtagggggttcgagtggggcccttgatgagagctgagaagaggtccattctatcttcaaaagtcttgaccatgatgccctcaggcagtgaggtagccagcagcgccatctccttccgcactgtgctgaagaacttcttggcttctggaggctggaactcaattttcttaaaagaatgatttgagggtgcaaactccagtacggagaagacctcgcccttggcgctggtgaaggtgacgccaggcttgccgccacactgctggcacagcaccggggtttcgctgggccactcagccttcacaggtgactgcccctcgggcttgtcctccttgcgctctacgtcgggcactgcttccatcttctcctcctctacaatggccacattgtccagggtcttcttgaggttttcctgtagcttcttgatgtcatccagaaacttcttctcccgagttggcttctcaggctccacagtcggagaggtgggcgagcccgtcagcagctgctccacagtcatgttcttgaggctctccaggatcttgatggcctctttcaactcccggaagctcttgggtggcccgtccttgccagccttctccatcagcccggccatgggggcagccatggccacagccccctggacggcagctgtggctgcctcttcactgatcaccactcccttgtcctcaggggccaccggctgctccaggggtgggatggggggctcctctatcttggggtgctcgtcctccaccagcccattgtccgtctcccagctgtcactatcatcttcccattcatccgaggatgccccgctggtgctgccttctaccgaatcgtagtctgactcctcaatctcagactctatgttgtacaagtgctggggcaggatgatggtctttgagttgtcagcccacaccacctccaccttgctgctgacgtccacacgggccacctggcccaccgatggctcatcctccttgtgaggagccccatcctcagtattgccgatgcggatgacgatgtcagttgtacggaacctaaagtcagggtggtcagcaatgtcgtaaacactcacatcttcctcttctccaatcagctccacgtcgtccccactcggcctcagcttgaaccacttcaccatgcaggtacggccgatgtggtccccagactgtaccacaccgtagacagcagggtctggacagctctggactcgcttatctaccacgaagtctccagggcagaactcgttgttgtccaggtggtgcacagggaagaggtcgttggagcggatgttgcattccacggagccatcctgccacatcacgtcggctgaggtcatcgtggtcaccacctccactgccaccctgtcccctggcttgaagtctcgagtgattttattcttcttcctcttgtgtttgcgctttaagttcttgatggacaaggggatgctctttttgcgactcgtgccgctgccgctctgggaggaagtggtggagctggcagaggaggtcaccgaactggtgtcgtccgtgtcatcagcagcctcatcatctgcgtcctgctctgccgagtgcagcctgtcatctctgccttcttttagcaggaatgggggcagctgctctcctgcctcgtggggctcctctgcaccctcgtcctgcatctccactggactggcagagccatcgggcgtctcctcagggctggcagactccgcttcgctcttggttttggattcccccttcttgtctgggtcttccatggaatggtcccgggaacactgggtgtctggggagcatgacatgatccgcacaacctgcttcttcaacaggcgcttcaccttcttggccatagagccctccccctgggcgcagtttttttctggacattcccaggcaatcttggctggctctaccttggctgggaagacatacagacagcgctccccaagctgccgctgagcatggtcaaagcatccgagacgcttcaccctgcctaggttttcctgggtgatgacagagggtggggggctgacgctgtccgtgccccctggacagaaactcttggtaatccatgtaactttcaactctacaacctgcacctcttccaccaccactcggaacttgctcttggtgctgagcacgggcttgacacctgacagccactggacgctggagaagatcttggcagggccaatgagcacctggcctgggtagaagccataggaatcatcgaagaagagacccgagtcgctgacgtgcgggcagacgtcgtagagcttggcgccatcttccgtgttcatggagcacctggcgccgttggatagcttcaggatgatctggttcttcaagtcgtagaccttccccagccagcagtcataggcaatgtagtccccatacatgaagggccagatgtgctgcaggtccttgctgttgacgggatagatgatgcagttggtgccgatgagcttgacggcacagtcgatgttgacgtcgatcaccgtgccacactgactgtcggtggatcgcatgtgccggaccacatctcggggcaccacagaacggtcctctagtttcagctgcagaattgggcagaaactcctcccagtctccatgatggtgctgtttccgctggtatttgagtcctggctcactgcatttagaggagctgcttgctgctgttgtgccttggtctccttcacatgctgcttgacgccctccgggtaccactggacgcgcacgtagccgcggcgcagggggctggcccggccctcctcgtggcccgcgcccccggcctcggagcaccccgagctcccgcggccctcctcctcgccctccgagtccgagtcctcgccgtggatgaggcgcaccagcccgaagtgcacggagccacggtaacggcccgacaccaggtcgtgagaaaacagcaggcgctgcgagccggcttctgggccggagtccgaggacggcccggaggccgagtccgaggcgggcgccggcgccgggacgggggctgcggctggggccgggactgcctccggggctggagccggggcctgggctggagcgggagctgcgggcgtgggggctgcgggatccgccataactgctctgcgcgagtctcgggcggcggcggcgacagcggcggcgaacgaggcgcggggaggcgggaccagcgggcgccgggggcggggcca

SEQ ID NO: 19528 - RNA, 4393 nt, Homo sapiens
  source 1..4393: mol_type = other RNA
ttgctgacctgggtggtggtggcagcaggagggtctgggacacagggaggcttgagttgaactaaacaggttgaaagggaccaggggaattgttggcgcaacccacacttcatgcaaggcacatgtgctctcctgcgggtctgcagggaaccggcccagagagccccgcggcaggccctggaacacccgcctctgacctgagaaggggcagcaagggagcaagtgccggacattctgctggggtgacaaatggaaaatcggcaacagggttccgattttctttgccacaggggacccgcctgttgaaagctcgcttcaaaatagaaacggcagcatctcaacacacttcttgcacttcagcatcaaactcaccttggggagaagagggcagtgggtttgcagtggggacagaggggcatgggaagaggggtgattccgggggggagtgagcaggcggcggctggcctctcccacggtgatgctctttcctctgtgcctggcagctacttgtcctctgtgcactccggcatgcctgcctctagcagggcagcccggaactgcgtcaggacaccccggatgctcttgatgaaacccttggaaagtgggaagagggggaagccgatgtcagggtagccactcttctcaggtaagaagctccggtagctctttctccgcttctttggtttcacactgggtggcaccgatgcgtctggtgcggtctccgaagtctggtctgtgtggtccctgctagctgaggccaggccctgggcaccgccctctgagtctgagccctgggaggcctctcctggggctggccctccatcctcaggttcttgttggccggagtctgacagctcggctacagctgggggctctggcgagctgctggccttgggcaccccgttgggcagtgcctgggccttctccagcagggcatgggtttccagccaggactcgatacggttcaccagccgccagccaccagtgctaaagtgttgcctgatctcctgctcaaagacctcggggggccgccgcaccagctgggtcatggactgcaccacgcggatcagcgccatctcattgtaacagcgactgttttcatagccttcctgcaggcctcggtcactgtcgaagccggcttcgttgtagtatggttcatttaccaggatcagaccttggatggagatgagcacctggagaaggctggacttgcttgtccacctctctgtcccctttccaatccaggtgcccaggaggctgacacacaccttcccattgtcatacaggttggggttcaggcggccactgcattgggagaggtagcagaagtgggggggcacggctgggtagatgttggggagctggatgtcaaacaagtagaggccatcctcgtagggggttcgagtggggcccttgatgagagctgagaagaggtccattctatcttcaaaagtcttgaccatgatgccctcaggcagtgaggtagccagcagcgccatctccttccgcactgtgctgaagaacttcttggcttctggaggctggaactcaattttcttaaaagaatgatttgagggtgcaaactccagtacggagaagacctcgcccttggcgctggtgaaggtgacgccaggcttgccgccacactgctggcacagcaccggggtttcgctgggccactcagccttcacaggtgactgcccctcgggcttgtcctccttgcgctctacgtcgggcactgcttccatcttctcctcctctacaatggccacattgtccagggtcttcttgaggttttcctgtagcttcttgatgtcatccagaaacttcttctcccgagttggcttctcaggctccacagtcggagaggtgggcgagcccgtcagcagctgctccacagtcatgttcttgaggctctccaggatcttgatggcctctttcaactcccggaagctcttgggtggcccgtccttgccagccttctccatcagcccggccatgggggcagccatggccacagccccctggacggcagctgtggctgcctcttcactgatcaccactcccttgtcctcaggggccaccggctgctccaggggtgggatggggggctcctctatcttggggtgctcgtcctccaccagcccattgtccgtctcccagctgtcactatcatcttcccattcatccgaggatgccccgctggtgctgccttctaccgaatcgtagtctgactcctcaatctcagactctatgttgtacaagtgctggggcaggatgatggtctttgagttgtcagcccacaccacctccaccttgctgctgacgtccacacgggccacctggcccaccgatggctcatcctccttgtgaggagccccatcctcagtattgccgatgcggatgacgatgtcagttgtacggaacctaaagtcagggtggtcagcaatgtcgtaaacactcacatcttcctcttctccaatcagctccacgtcgtccccactcggcctcagcttgaaccacttcaccatgcaggtacggccgatgtggtccccagactgtaccacaccgtagacagcagggtctggacagctctggactcgcttatctaccacgaagtctccagggcagaactcgttgttgtccaggtggtgcacagggaagaggtcgttggagcggatgttgcattccacggagccatcctgccacatcacgtcggctgaggtcatcgtggtcaccacctccactgccaccctgtcccctggcttgaagtctcgagtgattttattcttcttcctcttgtgtttgcgctttaagttcttgatggacaaggggatgctctttttgcgactcgtgccgctgccgctctgggaggaagtggtggagctggcagaggaggtcaccgaactggtgtcgtccgtgtcatcagcagcctcatcatctgcgtcctgctctgccgagtgcagcctgtcatctctgccttcttttagcaggaatgggggcagctgctctcctgcctcgtggggctcctctgcaccctcgtcctgcatctccactggactggcagagccatcgggcgtctcctcagggctggcagactccgcttcgctcttggttttggattcccccttcttgtctgggtcttccatggaatggtcccgggaacactgggtgtctggggagcatgacatgatccgcacaacctgcttcttcaacaggcgcttcaccttcttggccatagagccctccccctgggcgcagtttttttctggacattcccaggcaatcttggctggctctaccttggctgggaagacatacagacagcgctccccaagctgccgctgagcatggtcaaagcatccgagacgcttcaccctgcctaggttttcctgggtgatgacagagggtggggggctgacgctgtccgtgccccctggacagaaactcttggtaatccatgtaactttcaactctacaacctgcacctcttccaccaccactcggaacttgctcttggtgctgagcacgggcttgacacctgacagccactggacgctggagaagatcttggcagggccaatgagcacctggcctgggtagaagccataggaatcatcgaagaagagacccgagtcgctgacgtgcgggcagacgtcgtagagcttggcgccatcttccgtgttcatggagcacctggcgccgttggatagcttcaggatgatctggttcttcaagtcgtagaccttccccagccagcagtcataggcaatgtagtccccatacatgaagggccagatgtgctgcaggtccttgctgttgacgggatagatgatgcagttggtgccgatgagcttgacggcacagtcgatgttgacgtcgatcaccgtgccacactgactgtcggtggatcgcatgtgccggaccacatctcggggcaccacagaacggtcctctagtttcagcttggtctccttcacatgctgcttgacgccctccgggtaccactggacgcgcacgtagccgcggcgcagggggctggcccggccctcctcgtggcccgcgcccccggcctcggagcaccccgagctcccgcggccctcctcctcgccctccgagtccgagtcctcgccgtggatgaggcgcaccagcccgaagtgcacggagccacggtaacggcccgacaccaggtcgtgagaaaacagcaggcgctgcgagccggcttctgggccggagtccgaggacggcccggaggccgagtccgaggcgggcgccggcgccgggacgggggctgcggctggggccgggactgcctccggggctggagccggggcctgggctggagcgggagctgcgggcgtgggggctgcgggatccgccataactgctctgc

SEQ ID NO: 19529 - RNA, 4356 nt, Homo sapiens
  source 1..4356: mol_type = other RNA
ttgctgacctgggtggtggtggcagcaggagggtctgggacacagggaggcttgagttgaactaaacaggttgaaagggaccaggggaattgttggcgcaacccacacttcatgcaaggcacatgtgctctcctgcgggtctgcagggaaccggcccagagagccccgcggcaggccctggaacacccgcctctgacctgagaaggggcagcaagggagcaagtgccggacattctgctggggtgacaaatggaaaatcggcaacagggttccgattttctttgccacaggggacccgcctgttgaaagctcgcttcaaaatagaaacggcagcatctcaacacacttcttgcacttcagcatcaaactcaccttggggagaagagggcagtgggtttgcagtggggacagaggggcatgggaagaggggtgattccgggggggagtgagcaggcggcggctggcctctcccacggtgatgctctttcctctgtgcctggcagctacttgtcctctgtgcactccggcatgcctgcctctagcagggcagcccggaactgcgtcaggacaccccggatgctcttgatgaaacccttggaaagtgggaagagggggaagccgatgtcagggtagccactcttctcaggtaagaagctccggtagctctttctccgcttctttggtttcacactgggtggcaccgatgcgtctggtgcggtctccgaagtctggtctgtgtggtccctgctagctgaggccaggccctgggcaccgccctctgagtctgagccctgggaggcctctcctggggctggccctccatcctcaggttcttgttggccggagtctgacagctcggctacagctgggggctctggcgagctgctggccttgggcaccccgttgggcagtgcctgggccttctccagcagggcatgggtttccagccaggactcgatacggttcaccagccgccagccaccagtgctaaagtgttgcctgatctcctgctcaaagacctcggggggccgccgcaccagctgggtcatggactgcaccacgcggatcagcgccatctcattgtaacagcgactgttttcatagccttcctgcaggcctcggtcactgtcgaagccggcttcgttgtagtatggttcatttaccaggatcagaccttggatggagatgagcacctggagaaggctggacttgcttgtccacctctctgtcccctttccaatccaggtgcccaggaggctgacacacaccttcccattgtcatacaggttggggttcaggcggccactgcattgggagaggtagcagaagtgggggggcacggctgggtagatgttggggagctggatgtcaaacaagtagaggccatcctcgtagggggttcgagtggggcccttgatgagagctgagaagaggtccattctatcttcaaaagtcttgaccatgatgccctcaggcagtgaggtagccagcagcgccatctccttccgcactgtgctgaagaacttcttggcttctggaggctggaactcaattttcttaaaagaatgatttgagggtgcaaactccagtacggagaagacctcgcccttggcgctggtgaaggtgacgccaggcttgccgccacactgctggcacagcaccggggtttcgctgggccactcagccttcacaggtgactgcccctcgggcttgtcctccttgcgctctacgtcgggcactgcttccatcttctcctcctctacaatggccacattgtccagggtcttcttgaggttttcctgtagcttcttgatgtcatccagaaacttcttctcccgagttggcttctcaggctccacagtcggagaggtgggcgagcccgtcagcagctgctccacagtcatgttcttgaggctctccaggatcttgatggcctctttcaactcccggaagctcttgggtggcccgtccttgccagccttctccatcagcccggccatgggggcagccatggccacagccccctggacggcagctgtggctgcctcttcactgatcaccactcccttgtcctcaggggccaccggctgctccaggggtgggatggggggctcctctatcttggggtgctcgtcctccaccagcccattgtccgtctcccagctgtcactatcatcttcccattcatccgaggatgccccgctggtgctgccttctaccgaatcgtagtctgactcctcaatctcagactctatgttgtacaagtgctggggcaggatgatggtctttgagttgtcagcccacaccacctccaccttgctgctgacgtccacacgggccacctggcccaccgatggctcatcctccttgtgaggagccccatcctcagtattgccgatgcggatgacgatgtcagttgtacggaacctaaagtcagggtggtcagcaatgtcgtaaacactcacatcttcctcttctccaatcagctccacgtcgtccccactcggcctcagcttgaaccacttcaccatgcaggtacggccgatgtggtccccagactgtaccacaccgtagacagcagggtctggacagctctggactcgcttatctaccacgaagtctccagggcagaactcgttgttgtccaggtggtgcacagggaagaggtcgttggagcggatgttgcattccacggagccatcctgccacatcacgtcggctgaggtcatcgtggtcaccacctccactgccaccctgtcccctggcttgaagtctcgagtgattttattcttcttcctcttgtgtttgcgctttaagttcttgatggacaaggggatgctctttttgcgactcgtgccgctgccgctctgggaggaagtggtggagctggcagaggaggtcaccgaactggtgtcgtccgtgtcatcagcagcctcatcatctgcgtcctgctctgccgagtgcagcctgtcatctctgccttcttttagcaggaatgggggcagctgctctcctgcctcgtggggctcctctgcaccctcgtcctgcatctccactggactggcagagccatcgggcgtctcctcagggctggcagactccgcttcgctcttggttttggattcccccttcttgtctgggtcttccatggaatggtcccgggaacactgggtgtctggggagcatgacatgatccgcacaacctgcttcttcaacaggcgcttcaccttggctgggaagacatacagacagcgctccccaagctgccgctgagcatggtcaaagcatccgagacgcttcaccctgcctaggttttcctgggtgatgacagagggtggggggctgacgctgtccgtgccccctggacagaaactcttggtaatccatgtaactttcaactctacaacctgcacctcttccaccaccactcggaacttgctcttggtgctgagcacgggcttgacacctgacagccactggacgctggagaagatcttggcagggccaatgagcacctggcctgggtagaagccataggaatcatcgaagaagagacccgagtcgctgacgtgcgggcagacgtcgtagagcttggcgccatcttccgtgttcatggagcacctggcgccgttggatagcttcaggatgatctggttcttcaagtcgtagaccttccccagccagcagtcataggcaatgtagtccccatacatgaagggccagatgtgctgcaggtccttgctgttgacgggatagatgatgcagttggtgccgatgagcttgacggcacagtcgatgttgacgtcgatcaccgtgccacactgactgtcggtggatcgcatgtgccggaccacatctcggggcaccacagaacggtcctctagtttcagcttggtctccttcacatgctgcttgacgccctccgggtaccactggacgcgcacgtagccgcggcgcagggggctggcccggccctcctcgtggcccgcgcccccggcctcggagcaccccgagctcccgcggccctcctcctcgccctccgagtccgagtcctcgccgtggatgaggcgcaccagcccgaagtgcacggagccacggtaacggcccgacaccaggtcgtgagaaaacagcaggcgctgcgagccggcttctgggccggagtccgaggacggcccggaggccgagtccgaggcgggcgccggcgccgggacgggggctgcggctggggccgggactgcctccggggctggagccggggcctgggctggagcgggagctgcgggcgtgggggctgcgggatccgccataactgctctgcgcgagtctcgggcggcggcggcgacagcggcggcgaac

SEQ ID NO: 19530 - RNA, 4586 nt, Homo sapiens
  source 1..4586: mol_type = other RNA
ttgctgacctgggtggtggtggcagcaggagggtctgggacacagggaggcttgagttgaactaaacaggttgaaagggaccaggggaattgttggcgcaacccacacttcatgcaaggcacatgtgctctcctgcgggtctgcagggaaccggcccagagagccccgcggcaggccctggaacacccgcctctgacctgagaaggggcagcaagggagcaagtgccggacattctgctggggtgacaaatggaaaatcggcaacagggttccgattttctttgccacaggggacccgcctgttgaaagctcgcttcaaaatagaaacggcagcatctcaacacacttcttgcacttcagcatcaaactcaccttggggagaagagggcagtgggtttgcagtggggacagaggggcatgggaagaggggtgattccgggggggagtgagcaggcggcggctggcctctcccacggtgatgctctttcctctgtgcctggcagctacttgtcctctgtgcactccggcatgcctgcctctagcagggcagcccggaactgcgtcaggacaccccggatgctcttgatgaaacccttggaaagtgggaagagggggaagccgatgtcagggtagccactcttctcaggtaagaagctccggtagctctttctccgcttctttggtttcacactgggtggcaccgatgcgtctggtgcggtctccgaagtctggtctgtgtggtccctgctagctgaggccaggccctgggcaccgccctctgagtctgagccctgggaggcctctcctggggctggccctccatcctcaggttcttgttggccggagtctgacagctcggctacagctgggggctctggcgagctgctggccttgggcaccccgttgggcagtgcctgggccttctccagcagggcatgggtttccagccaggactcgatacggttcaccagccgccagccaccagtgctaaagtgttgcctgatctcctgctcaaagacctcggggggccgccgcaccagctgggtcatggactgcaccacgcggatcagcgccatctcattgtaacagcgactgttttcatagccttcctgcaggcctcggtcactgtcgaagccggcttcgttgtagtatggttcatttaccaggatcagaccttggatggagatgagcacctggagaaggctggacttgcttgtccacctctctgtcccctttccaatccaggtgcccaggaggctgacacacaccttcccattgtcatacaggttggggttcaggcggccactgcattgggagaggtagcagaagtgggggggcacggctgggtagatgttggggagctggatgtcaaacaagtagaggccatcctcgtagggggttcgagtggggcccttgatgagagctgagaagaggtccattctatcttcaaaagtcttgaccatgatgccctcaggcagtgaggtagccagcagcgccatctccttccgcactgtgctgaagaacttcttggcttctggaggctggaactcaattttcttaaaagaatgatttgagggtgcaaactccagtacggagaagacctcgcccttggcgctggtgaaggtgacgccaggcttgccgccacactgctggcacagcaccggggtttcgctgggccactcagccttcacaggtgactgcccctcgggcttgtcctccttgcgctctacgtcgggcactgcttccatcttctcctcctctacaatggccacattgtccagggtcttcttgaggttttcctgtagcttcttgatgtcatccagaaacttcttctcccgagttggcttctcaggctccacagtcggagaggtgggcgagcccgtcagcagctgctccacagtcatgttcttgaggctctccaggatcttgatggcctctttcaactcccggaagctcttgggtggcccgtccttgccagccttctccatcagcccggccatgggggcagccatggccacagccccctggacggcagctgtggctgcctcttcactgatcaccactcccttgtcctcaggggccaccggctgctccaggggtgggatggggggctcctctatcttggggtgctcgtcctccaccagcccattgtccgtctcccagctgtcactatcatcttcccattcatccgaggatgccccgctggtgctgccttctaccgaatcgtagtctgactcctcaatctcagactctatgttgtacaagtgctggggcaggatgatggtctttgagttgtcagcccacaccacctccaccttgctgctgacgtccacacgggccacctggcccaccgatggctgctcatcctccttgtgaggagccccatcctcagtattgccgatgcggatgacgatgtcagttgtacggaacctaaagtcagggtggtcagcaatgtcgtaaacactcacatcttcctcttctccaatcagctccacgtcgtccccactcggcctcagcttgaaccacttcaccatgcaggtacggccgatgtggtccccagactgtaccacaccgtagacagcagggtctggacagctctggactcgcttatctaccacgaagtctccagggcagaactcgttgttgtccaggtggtgcacagggaagaggtcgttggagcggatgttgcattccacggagccatcctgccacatcacgtcggctgaggtcatcgtggtcaccacctccactgccaccctgtcccctggcttgaagtctcgagtgattttattcttcttcctcttgtgtttgcgctttaagttcttgatggacaaggggatgctctttttgcgactcgtgccgctgccgctctgggaggaagtggtggagctggcagaggaggtcaccgaactggtgtcgtccgtgtcatcagcagcctcatcatctgcgtcctgctctgccgagtgcagcctgtcatctctgccttcttttagcaggaatgggggcagctgctctcctgcctcgtggggctcctctgcaccctcgtcctgcatctccactggactggcagagccatcgggcgtctcctcagggctggcagactccgcttcgctcttggttttggattcccccttcttgtctgggtcttccatggaatggtcccgggaacactgggtgtctggggagcatgacatgatccgcacaacctgcttcttcaacaggcgcttcaccttcttggccatagagccctccccctgggcgcagtttttttctggacattcccaggcaatcttggctggctctaccttggctgggaagacatacagacagcgctccccaagctgccgctgagcatggtcaaagcatccgagacgcttcaccctgcctaggttttcctgggtgatgacagagggtggggggctgacgctgtccgtgccccctggacagaaactcttggtaatccatgtaactttcaactctacaacctgcacctcttccaccaccactcggaacttgctcttggtgctgagcacgggcttgacacctgacagccactggacgctggagaagatcttggcagggccaatgagcacctggcctgggtagaagccataggaatcatcgaagaagagacccgagtcgctgacgtgcgggcagacgtcgtagagcttggcgccatcttccgtgttcatggagcacctggcgccgttggatagcttcaggatgatctggttcttcaagtcgtagaccttccccagccagcagtcataggcaatgtagtccccatacatgaagggccagatgtgctgcaggtccttgctgttgacgggatagatgatgcagttggtgccgatgagcttgacggcacagtcgatgttgacgtcgatcaccgtgccacactgactgtcggtggatcgcatgtgccggaccacatctcggggcaccacagaacggtcctctagtttcagctgcagaattgggcagaaactcctcccagtctccatgatggtgctgtttccgctggtatttgagtcctggctcactgcatttagaggagctgcttgctgctgttgtgccttggtctccttcacatgctgcttgacgccctccgggtaccactggacgcgcacgtagccgcggcgcagggggctggcccggccctcctcgtggcccgcgcccccggcctcggagcaccccgagctcccgcggccctcctcctcgccctccgagtccgagtcctcgccgtggatgaggcgcaccagcccgaagtgcacggagccacggtaacggcccgacaccaggtcgtgagaaaacagcaggcgctgcgagccggcttctgggccggagtccgaggacggcccggaggccgagtccgaggcgggcgccggcgccgggacgggggctgcggctggggccgggactgcctccggggctggagccggggcctgggctggagcgggagctgcgggcgtgggggctgcgggatccgccataactgctctgcgcgagtctcgggcggcggcggcgacagcggcggcgaacgaggcgcggggaggcgggaccagcgggcgccgggggcggggcca

SEQ ID NO: 19531 - RNA, 4434 nt, Homo sapiens
  source 1..4434: mol_type = other RNA
ttgctgacctgggtggtggtggcagcaggagggtctgggacacagggaggcttgagttgaactaaacaggttgaaagggaccaggggaattgttggcgcaacccacacttcatgcaaggcacatgtgctctcctgcgggtctgcagggaaccggcccagagagccccgcggcaggccctggaacacccgcctctgacctgagaaggggcagcaagggagcaagtgccggacattctgctggggtgacaaatggaaaatcggcaacagggttccgattttctttgccacaggggacccgcctgttgaaagctcgcttcaaaatagaaacggcagcatctcaacacacttcttgcacttcagcatcaaactcaccttggggagaagagggcagtgggtttgcagtggggacagaggggcatgggaagaggggtgattccgggggggagtgagcaggcggcggctggcctctcccacggtgatgctctttcctctgtgcctggcagctacttgtcctctgtgcactccggcatgcctgcctctagcagggcagcccggaactgcgtcaggacaccccggatgctcttgatgaaacccttggaaagtgggaagagggggaagccgatgtcagggtagccactcttctcaggtaagaagctccggtagctctttctccgcttctttggtttcacactgggtggcaccgatgcgtctggtgcggtctccgaagtctggtctgtgtggtccctgctagctgaggccaggccctgggcaccgccctctgagtctgagccctgggaggcctctcctggggctggccctccatcctcaggttcttgttggccggagtctgacagctcggctacagctgggggctctggcgagctgctggccttgggcaccccgttgggcagtgcctgggccttctccagcagggcatgggtttccagccaggactcgatacggttcaccagccgccagccaccagtgctaaagtgttgcctgatctcctgctcaaagacctcggggggccgccgcaccagctgggtcatggactgcaccacgcggatcagcgccatctcattgtaacagcgactgttttcatagccttcctgcaggcctcggtcactgtcgaagccggcttcgttgtagtatggttcatttaccaggatcagaccttggatggagatgagcacctggagaaggctggacttgcttgtccacctctctgtcccctttccaatccaggtgcccaggaggctgacacacaccttcccattgtcatacaggttggggttcaggcggccactgcattgggagaggtagcagaagtgggggggcacggctgggtagatgttggggagctggatgtcaaacaagtagaggccatcctcgtagggggttcgagtggggcccttgatgagagctgagaagaggtccattctatcttcaaaagtcttgaccatgatgccctcaggcagtgaggtagccagcagcgccatctccttccgcactgtgctgaagaacttcttggcttctggaggctggaactcaattttcttaaaagaatgatttgagggtgcaaactccagtacggagaagacctcgcccttggcgctggtgaaggtgacgccaggcttgccgccacactgctggcacagcaccggggtttcgctgggccactcagccttcacaggtgactgcccctcgggcttgtcctccttgcgctctacgtcgggcactgcttccatcttctcctcctctacaatggccacattgtccagggtcttcttgaggttttcctgtagcttcttgatgtcatccagaaacttcttctcccgagttggcttctcaggctccacagtcggagaggtgggcgagcccgtcagcagctgctccacagtcatgttcttgaggctctccaggatcttgatggcctctttcaactcccggaagctcttgggtggcccgtccttgccagccttctccatcagcccggccatgggggcagccatggccacagccccctggacggcagctgtggctgcctcttcactgatcaccactcccttgtcctcaggggccaccggctgctccaggggtgggatggggggctcctctatcttggggtgctcgtcctccaccagcccattgtccgtctcccagctgtcactatcatcttcccattcatccgaggatgccccgctggtgctgccttctaccgaatcgtagtctgactcctcaatctcagactctatgttgtacaagtgctggggcaggatgatggtctttgagttgtcagcccacaccacctccaccttgctgctgacgtccacacgggccacctggcccaccgatggctgctcatcctccttgtgaggagccccatcctcagtattgccgatgcggatgacgatgtcagttgtacggaacctaaagtcagggtggtcagcaatgtcgtaaacactcacatcttcctcttctccaatcagctccacgtcgtccccactcggcctcagcttgaaccacttcaccatgcaggtacggccgatgtggtccccagactgtaccacaccgtagacagcagggtctggacagctctggactcgcttatctaccacgaagtctccagggcagaactcgttgttgtccaggtggtgcacagggaagaggtcgttggagcggatgttgcattccacggagccatcctgccacatcacgtcggctgaggtcatcgtggtcaccacctccactgccaccctgtcccctggcttgaagtctcgagtgattttattcttcttcctcttgtgtttgcgctttaagttcttgatggacaaggggatgctctttttgcgactcgtgccgctgccgctctgggaggaagtggtggagctggcagaggaggtcaccgaactggtgtcgtccgtgtcatcagcagcctcatcatctgcgtcctgctctgccgagtgcagcctgtcatctctgccttcttttagcaggaatgggggcagctgctctcctgcctcgtggggctcctctgcaccctcgtcctgcatctccactggactggcagagccatcgggcgtctcctcagggctggcagactccgcttcgctcttggttttggattcccccttcttgtctgggtcttccatggaatggtcccgggaacactgggtgtctggggagcatgacatgatccgcacaacctgcttcttcaacaggcgcttcaccttcttggccatagagccctccccctgggcgcagtttttttctggacattcccaggcaatcttggctggctctaccttggctgggaagacatacagacagcgctccccaagctgccgctgagcatggtcaaagcatccgagacgcttcaccctgcctaggttttcctgggtgatgacagagggtggggggctgacgctgtccgtgccccctggacagaaactcttggtaatccatgtaactttcaactctacaacctgcacctcttccaccaccactcggaacttgctcttggtgctgagcacgggcttgacacctgacagccactggacgctggagaagatcttggcagggccaatgagcacctggcctgggtagaagccataggaatcatcgaagaagagacccgagtcgctgacgtgcgggcagacgtcgtagagcttggcgccatcttccgtgttcatggagcacctggcgccgttggatagcttcaggatgatctggttcttcaagtcgtagaccttccccagccagcagtcataggcaatgtagtccccatacatgaagggccagatgtgctgcaggtccttgctgttgacgggatagatgatgcagttggtgccgatgagcttgacggcacagtcgatgttgacgtcgatcaccgtgccacactgactgtcggtggatcgcatgtgccggaccacatctcggggcaccacagaacggtcctctagtttcagcttggtctccttcacatgctgcttgacgccctccgggtaccactggacgcgcacgtagccgcggcgcagggggctggcccggccctcctcgtggcccgcgcccccggcctcggagcaccccgagctcccgcggccctcctcctcgccctccgagtccgagtcctcgccgtggatgaggcgcaccagcccgaagtgcacggagccacggtaacggcccgacaccaggtcgtgagaaaacagcaggcgctgcgagccggcttctgggccggagtccgaggacggcccggaggccgagtccgaggcgggcgccggcgccgggacgggggctgcggctggggccgggactgcctccggggctggagccggggcctgggctggagcgggagctgcgggcgtgggggctgcgggatccgccataactgctctgcgcgagtctcgggcggcggcggcgacagcggcggcgaac

SEQ ID NO: 19532 - RNA, 4511 nt, Homo sapiens
  source 1..4511: mol_type = other RNA
ttgctgacctgggtggtggtggcagcaggagggtctgggacacagggaggcttgagttgaactaaacaggttgaaagggaccaggggaattgttggcgcaacccacacttcatgcaaggcacatgtgctctcctgcgggtctgcagggaaccggcccagagagccccgcggcaggccctggaacacccgcctctgacctgagaaggggcagcaagggagcaagtgccggacattctgctggggtgacaaatggaaaatcggcaacagggttccgattttctttgccacaggggacccgcctgttgaaagctcgcttcaaaatagaaacggcagcatctcaacacacttcttgcacttcagcatcaaactcaccttggggagaagagggcagtgggtttgcagtggggacagaggggcatgggaagaggggtgattccgggggggagtgagcaggcggcggctggcctctcccacggtgatgctctttcctctgtgcctggcagctacttgtcctctgtgcactccggcatgcctgcctctagcagggcagcccggaactgcgtcaggacaccccggatgctcttgatgaaacccttggaaagtgggaagagggggaagccgatgtcagggtagccactcttctcaggtaagaagctccggtagctctttctccgcttctttggtttcacactgggtggcaccgatgcgtctggtgcggtctccgaagtctggtctgtgtggtccctgctagctgaggccaggccctgggcaccgccctctgagtctgagccctgggaggcctctcctggggctggccctccatcctcaggttcttgttggccggagtctgacagctcggctacagctgggggctctggcgagctgctggccttgggcaccccgttgggcagtgcctgggccttctccagcagggcatgggtttccagccaggactcgatacggttcaccagccgccagccaccagtgctaaagtgttgcctgatctcctgctcaaagacctcggggggccgccgcaccagctgggtcatggactgcaccacgcggatcagcgccatctcattgtaacagcgactgttttcatagccttcctgcaggcctcggtcactgtcgaagccggcttcgttgtagtatggttcatttaccaggatcagaccttggatggagatgagcacctggagaaggctggacttgcttgtccacctctctgtcccctttccaatccaggtgcccaggaggctgacacacaccttcccattgtcatacaggttggggttcaggcggccactgcattgggagaggtagcagaagtgggggggcacggctgggtagatgttggggagctggatgtcaaacaagtagaggccatcctcgtagggggttcgagtggggcccttgatgagagctgagaagaggtccattctatcttcaaaagtcttgaccatgatgccctcaggcagtgaggtagccagcagcgccatctccttccgcactgtgctgaagaacttcttggcttctggaggctggaactcaattttcttaaaagaatgatttgagggtgcaaactccagtacggagaagacctcgcccttggcgctggtgaaggtgacgccaggcttgccgccacactgctggcacagcaccggggtttcgctgggccactcagccttcacaggtgactgcccctcgggcttgtcctccttgcgctctacgtcgggcactgcttccatcttctcctcctctacaatggccacattgtccagggtcttcttgaggttttcctgtagcttcttgatgtcatccagaaacttcttctcccgagttggcttctcaggctccacagtcggagaggtgggcgagcccgtcagcagctgctccacagtcatgttcttgaggctctccaggatcttgatggcctctttcaactcccggaagctcttgggtggcccgtccttgccagccttctccatcagcccggccatgggggcagccatggccacagccccctggacggcagctgtggctgcctcttcactgatcaccactcccttgtcctcaggggccaccggctgctccaggggtgggatggggggctcctctatcttggggtgctcgtcctccaccagcccattgtccgtctcccagctgtcactatcatcttcccattcatccgaggatgccccgctggtgctgccttctaccgaatcgtagtctgactcctcaatctcagactctatgttgtacaagtgctggggcaggatgatggtctttgagttgtcagcccacaccacctccaccttgctgctgacgtccacacgggccacctggcccaccgatggctgctcatcctccttgtgaggagccccatcctcagtattgccgatgcggatgacgatgtcagttgtacggaacctaaagtcagggtggtcagcaatgtcgtaaacactcacatcttcctcttctccaatcagctccacgtcgtccccactcggcctcagcttgaaccacttcaccatgcaggtacggccgatgtggtccccagactgtaccacaccgtagacagcagggtctggacagctctggactcgcttatctaccacgaagtctccagggcagaactcgttgttgtccaggtggtgcacagggaagaggtcgttggagcggatgttgcattccacggagccatcctgccacatcacgtcggctgaggtcatcgtggtcaccacctccactgccaccctgtcccctggcttgaagtctcgagtgattttattcttcttcctcttgtgtttgcgctttaagttcttgatggacaaggggatgctctttttgcgactcgtgccgctgccgctctgggaggaagtggtggagctggcagaggaggtcaccgaactggtgtcgtccgtgtcatcagcagcctcatcatctgcgtcctgctctgccgagtgcagcctgtcatctctgccttcttttagcaggaatgggggcagctgctctcctgcctcgtggggctcctctgcaccctcgtcctgcatctccactggactggcagagccatcgggcgtctcctcagggctggcagactccgcttcgctcttggttttggattcccccttcttgtctgggtcttccatggaatggtcccgggaacactgggtgtctggggagcatgacatgatccgcacaacctgcttcttcaacaggcgcttcaccttggctgggaagacatacagacagcgctccccaagctgccgctgagcatggtcaaagcatccgagacgcttcaccctgcctaggttttcctgggtgatgacagagggtggggggctgacgctgtccgtgccccctggacagaaactcttggtaatccatgtaactttcaactctacaacctgcacctcttccaccaccactcggaacttgctcttggtgctgagcacgggcttgacacctgacagccactggacgctggagaagatcttggcagggccaatgagcacctggcctgggtagaagccataggaatcatcgaagaagagacccgagtcgctgacgtgcgggcagacgtcgtagagcttggcgccatcttccgtgttcatggagcacctggcgccgttggatagcttcaggatgatctggttcttcaagtcgtagaccttccccagccagcagtcataggcaatgtagtccccatacatgaagggccagatgtgctgcaggtccttgctgttgacgggatagatgatgcagttggtgccgatgagcttgacggcacagtcgatgttgacgtcgatcaccgtgccacactgactgtcggtggatcgcatgtgccggaccacatctcggggcaccacagaacggtcctctagtttcagctgcagaattgggcagaaactcctcccagtctccatgatggtgctgtttccgctggtatttgagtcctggctcactgcatttagaggagctgcttgctgctgttgtgccttggtctccttcacatgctgcttgacgccctccgggtaccactggacgcgcacgtagccgcggcgcagggggctggcccggccctcctcgtggcccgcgcccccggcctcggagcaccccgagctcccgcggccctcctcctcgccctccgagtccgagtcctcgccgtggatgaggcgcaccagcccgaagtgcacggagccacggtaacggcccgacaccaggtcgtgagaaaacagcaggcgctgcgagccggcttctgggccggagtccgaggacggcccggaggccgagtccgaggcgggcgccggcgccgggacgggggctgcggctggggccgggactgcctccggggctggagccggggcctgggctggagcgggagctgcgggcgtgggggctgcgggatccgccataactgctctgcgcgagtctcgggcggcggcggcgacagcggcggcgaacgaggcgcggggaggcgggaccagcgggcgccgggggcggggcca

SEQ ID NO: 19533 - RNA, 2594 nt, Homo sapiens
  source 1..2594: mol_type = other RNA
ttggactttttcagatttggggatacagaaggatgcaaaatgaggcaacctagccacccaactggcccagtggtcaaggggggaaatgaggtggccgctagtcagcgctggagccatttctcgacggtgctttctgtttgtttgtttgtttttgttttgagatggagtctctctctgtcgcccaggctggagtgcagtggcgtgatctcggctcactgcaacctcaacggtgcttttttctgatcatagctgagctcaaatgctgaccccagtggcctgtctctaagcactgtggctccaggaaggaaaggcctggagagacctagaccaaggcctcagtagggagggagagaatttactctttgcaaaacgtatggagtccttgttatttaccaaatatcatgttacagaccagggataaaaacaacaataatgaatttcagtgaatctaaaacacaatccattgtaaggcacatcattattctatctcccaagacaggaaaaaaaatctttagatttcatagatatcaaatgggccaacaaaaatgtatcttggaataaacaaaatatgctaatgataacagtaagatatgtaggacatactacgtacaggtgctgttcttagcatttcatatctatcattttacccacacagtgaatctgtgagatggaagctattatcattccattttacagacacctacactgagactcaggcaggccagttgtcctgcccatgtacacacagctcctaagtggtagagtcaggatttgaacccagaccccgcagcctggctccatgctctcaacagctttgcagaaactaaagttggaatggaagactgctcattccaaatctgtcctattgtccagcatcctatggcccattccagaaagttcagtgggtgtcaattagcttggctgtagtgaccactcttaagtgtaccgttaccttttattttaatttgagaaattaaataaaatacatccacagcagtttacaactctgccatgatgtcattttgtcagatggcaaatttcaggagagggtcaaactcaaaaaaccctatgtcgttacctggatttatcgagaggacatcaaatcacttaattctatcacggcccacacccatgaattcactaagtaattatcacacacctgtcaggatccagacagttgctgaggaccaagatccagacgagactgacagagcttctattccccggcaccctccgtgaacttgggcacccaaaactaagggatctgaaacctgagaggaaatggaagcagactgtgaggccctgcagcgccgtctcttggatggtttattcttctctggcaggttttcccctaggtattcatggcatccaggggcatttcacctcagcaaagtgatgacgctgccactcaggttcccatggaaaccaaactgggacaggaggaacaaaaggctcctcaaggtcagtggtgcaaaggacattagagacaaagacagagacagcaaatcagcccaaagaacagacataaaccggcgcttcctccctcccatcaccacagctcggggctttgtcaccccagcacacctgggccctgcacctcagacgctgcgtgtgagcttctggggagagaagtgtgggcctccagggaggtgtaggcgctcctggctcctggcagactcctggcccaggcctggcctgtgtctgcttccggagccatgcgctgcctgtgctgggatgaatgcatggcccctgcatccttaccccctcctcagagcccacaagcttccgagtgcgtcatcttcattattggccacaggaaacgacttcttggagtaagtgactggtgctccgaggcccatctggacaaaagcaggatccggggtggacgcagaagagcaggcccggagccctgcaccccagccttccctccccatgcgctccacatgcgtcctttgttcagcctctccatttagctctcactttctggatgcagccaggcaccaccttccttccaaaagccttgtttctcagaaaacctttctgcctcctagaaacccaggattccgaggaggaggagggctggccttcctcttgggactattgatcagggctgtcagttcccagctctgtccaatgctctgaactggggacagtccgcatgcagctctgaggacccagatgctgtcactgggtcctggtgagtctgaaaacttgggatgtcggcaccacggtgagagcagagtctgcccggggctgtggcaggcaaaagaccgtctcggttttcactgcagggacttacccagccaggtgtgtgtgtctgagccctgccattcggaggcatcaccgagaggttctggtctcccctgcccaggccctgcctcctggccccactgcaggaagcttgagcagatctgaagctcgcctcagaggaagatcccatccaggggaggccctgtctgcagaaagcagagaacttggcttctcctcatttgttgttagggccagtccctaagggactgcctcctaggagtcggagggtccgtggaaatggtctcctcctgcacatctgtgctgctgtgactgggtgcaggtct

SEQ ID NO: 19534 - RNA, 5299 nt, Homo sapiens
  source 1..5299: mol_type = other RNA
ttggactttttcagatttggggatacagaaggatgcaaaatgaggcaacctagccacccaactggcccagtggtcaaggggggaaatgaggtggccgctagtcagcgctggagccatttctcgacggtgctttctgtttgtttgtttgtttttgttttgagatggagtctctctctgtcgcccaggctggagtgcagtggcgtgatctcggctcactgcaacctcaacggtgcttttttctgatcatagctgagctcaaatgctgaccccagtggcctgtctctaagcactgtggctccaggaaggaaaggcctggagagacctagaccaaggcctgtcaggatccagacagttgctgaggaccaagatccagacgagactgacagagcttctattccccggcaccctccgtgaacttgggcacccaaaactaagggatctgaaacccagccaggtgtgtgtgtctgagccctgccattcggaggcatcaccgagaggttctggtctcccctgcccaggccctgcctcctggccccactgcaggaagcttgagcagatctgaagctcgcctcagaggaagatcccatccaggggaggccctgtctgcagaaagcagagaacttggcttctcctcatttgttgttagggccagtccctaagggactaaaaacaaacaaaacaggctatgaacagaagcagtggtggcagcgctgggccagcaatgatgatttctactgttagggtttcagttgtacttggatctgggagggggaagccgatgcacccagagaccctagggctgggctgtaaccacacacctgaggagatgctttgggaaactcaaactgaagccatttgtgctgaatttggggaaagggggtgggatgatggagttaggagcgttgtcgttaactggtcattaattagatattaactaggcattaactagactttcggggaagcaacaaggcctctgtgtccacggttgtaaggtgtgggctaccctgatgaggggtgctccagctgtattcatgattcacattcattcattacatgcctgatctctatctcagaggcccggccttctgttagtaagctctcagattcagggaaaggagtctcagagaactccacatccgtgtggagtcagacggatcagagcagaacacagagctgccttctctgtcctgctctctctcccactcacctgctcagaggttgccagccgggccctgtctccctctctgccctcctgggtatcacggtccctcaacccagggaagctggtgccctcacttgtctcccatagtcctgtgtcatctgggcttctgtggcccctctcagctttcaggaccatccagtcttccccgtccctgttctttctctcgcaagtccccggtggcccagggtctagggagaagctgcattctgagctactgcccacatcgcttccccagggcggcgggagctctggaatggcaggccccgtccttgacagcctatccatgacctccaggggcagctcacagcagcgccacctgcatcacccacagaatggagggagacagcggctctccacacaaaggcactgagaaaaaagaataccctgaaagccacacaggtctcagggcagcagggagtgggagcactcatcacaggccagaagcccagcaagtagcatcagacacctcaggttaaagagaacgtagagattgtcgcttcccaccctccccattctagtcaattcggaccagtttggtacatgctggccatgtgcggtgaccacgctaagtactgtgcgtgtaccatttctcggaatacttcctgcaaccttatgaagttctcgcccaatttaacaagcactaaccaaactcagaaggcatttacccaatgctgcacgttacgaaaatgtaaaagaacgaacacggcttcaataccaggattgagcccaaaggtcacgttctttccctgcggctcccttccccatctggttctggggaagacactctgcacgcagcccccaggagaccacaggccctggactcccaaatcccagcagcaatgcaaagccacccccagaagagctgcccaggacaagtgatcctgcggcccattgctcactccccgcagaggcaggggcagctgactgctgtcccagatggacatagaaggtcaccatgtggcctgctggggtctgcaggatagaaggcgtgaggtgaagagtttgagctggtgcctacacctccgtcttccagccactgaaaacaggattctccagagttcacacctatgcatctggttcaatgctgggcattttgtcaggccacaagccagcagccatgcagcggatgcacctgtagatgatgcactgccttactgtccagacagaacaaaagggatcccctttccaacccgaaactgtcggattctctaagaggtccgtcacaacccatcttaatgcaagagggactgtggctcttctggaaacacgatgcctcggtgccatgaaatgacagctgcttcttttgaagaactgggctattcccatgtaaagctggctgcaatggatgatgtttctgactcatactctggctttaaaatcaaagtgtttgttagaaagcagctttgttttccttctatttcctgtttgaaaagtgaagcgttaacacgaaggagggtcccagcggagttcatgccgggactcaggttgcacacggccagtggtcccgggatatccagggagccactcagaggggacacttccagctgccatgcaaactcatcatgcacccagcccccccttgctccagctctgaccatagtgccctcaacacagggccctgggcagctaccctcaaacacctggatgccaagcatgagagggaaccaacttgccctccctggtctattatcacaaagaaccttggagcccctgcacaggaacccactccttagagggcacaaggggccaagttttgtttgagacaatgagctggcattggaagggagagatgacagctatcctctgtcctgcttccagggcagggcagagcaagctgcttttggccccgtctctgaggcagacatgagcacacttgtctcaggcagaagcagccttagatggtgttatggtttgaacgtgtttcccccgcaaaatccaggtgttgccaatgtgctagcattaagaggtggggccttaagaggggattaggccatgaatggaatcaggtgtcctgatgtaggtgctgtgtggagggagtacattcactcgttgcccttccaccttcagccatgtgaggacggcagcctttgtcccttctggaggacgcagcagcaaggcaccatcatgaaagcagagactggagccatcaccaggcacagaacctgctggcacctggctccagagctgtgggaagatacatttctgtcctttgtgaatcgcccactctccggggttgtgtgagagcagcacaaaatggactgggacagctggaatgtcagtttgcaacagtccccacccacacactcaaggcatgccacggcggccacgctgggtgcctttccgcaggtgcccaggcatcaggagcactggcccagtctcgaggggcgttcatgtcagggaggtgcccccgctagtgtcagcttcagcgccgccagcatcaggaagttcatctcgacaagcccgggcaagagaggaggcggtgagatcacctcctacccatccagagatcccccgactttggagtagtctgaaggacttgagactcctgaagtgagaggggacagagctaggagaagggagggcagccagaagggcaggggtgcagggggcgggatgaggagagccaggctggcattagcaagagcttcttcatgtccttttggcccaagggggccgtgttctctgaggaaatgggacttgctccagggaagaggaagagctcagcatccactttccctctgccgaacagctcctggggaaagcccaccactgtcttcttgccccgctctgtgccctcacacaagcgattctctccacctgcgacgtgtttcctctccctcccctggccagtgtccatgggttctctgagacggaacaggaagtattttaaggaagacctccctaacctcctcccagctgggtggatccctccctctgggcccccacacatctcagtttcaaaagaccattcacattgtagtctaaattagtggatccctggtgtgtgatgtgtgcagttataatgggttgcctcagcccccaacgcacctttcattgccttcttctgtgataatgcccctgggccctgtacccatttctcccttgccagctggcatgatgtttagccctgtgcagaggcaggggcctctccccggttccgacatttctttctctgcttgccccggctgctggggggacatgagggacacttggccctgttctctcttcagcaataattagtcccagcccaggttcctggcctgctgctccctgaggagggtttgccagtgccagcccgtgcttccttgtaccaggacttggtctgctgggacccagtggaaagcccacggctgccgcccccacccaccttcccctgcttgccagccacagtcaccagctgtagacttgtgtggctgtgctgcggaagcagatctgggtggaggagggccccacgcacagacgtgaatatgaagggaccctctagaggttgtggcaaacacaggtgccccgccccatgccctgtctgcagtcacagcccttcctacatggagggtgctatcatcaatcttctggggggctgtggacactctgcatccccatacctgtggcagtcctggcacacggtaagctctcagtaagtgtggtgagtcactgctgaaggaactaacaaataaacctcccaccaccaaccacaggtagctggggcagaactagggaactgctgaaaggaggctggtgaaccctgccatgacatgcccgctgtgcccaggacccaggctcccacagctcgcgtccttcctctatcccagatccattcaaagtgaagtggcctccatacaggcttccctaggggccctgctcagtgtccatgaggccaccatgccgccgttcaccaggggacgtgagaaaggggctggcctgtggaccaggactgacccaggtctgagccccagctcagcggtcggctagctgtgcgagcttgcgcagtagctccccaagtgtggctcaggacgcacagcatcggcgtcagcatcgcccaggaacctgcctcctaggagtcggagggtccgtggaaat

SEQ ID NO: 19535 - RNA, 741 nt, Homo sapiens
  source 1..741: mol_type = other RNA
ttggactttttcagatttggggatacagaaggatgcaaaatgaggcaacctagccacccaactggcccagtggtcaaggggggaaatgaggtggccgctagtcagcgctggagccatttctcgacggtgctttctgtttgtttgtttgtttttgttttgagatggagtctctctctgtcgcccaggctggagtgcagtggcgtgatctcggctcactgcaacctcaacggtgcttttttctgatcatagctgagctcaaatgctgaccccagtggcctgtctctaagcactgtggctccaggaaggaaaggcctggagagacctagaccaaggcctgtcaggatccagacagttgctgaggaccaagatccagacgagactgacagagcttctattccccggcaccctccgtgaacttgggcacccaaaactaagggatctgaaacccagccaggtgtgtgtgtctgagccctgccattcggaggcatcaccgagaggttctggtctcccctgcccaggccctgcctcctggccccactgcaggaagcttgagcagatctgaagctcgcctcagaggaagatcccatccaggggaggccctgtctgcagaaagcagagaacttggcttctcctcatttgttgttagggccagtccctaagggactgcctcctaggagtcggagggtccgtggaaatggtctcctcctgcacatctgtgctgctgtgactgggtgcaggtct

SEQ ID NO: 19536 - RNA, 2034 nt, Homo sapiens
  source 1..2034: mol_type = other RNA
ttggactttttcagatttggggatacagaaggatgcaaaatgaggcaacctagccacccaactggcccagtggtcaaggggggaaatgaggtggccgctagtcagcgctggagccatttctcgacggtgctttctgtttgtttgtttgtttttgttttgagatggagtctctctctgtcgcccaggctggagtgcagtggcgtgatctcggctcactgcaacctcaacggtgcttttttctgatcatagctgagctcaaatgctgaccccagtggcctgtctctaagcactgtggctccaggaaggaaaggcctggagagacctagaccaaggcctgtcaggatccagacagttgctgaggaccaagatccagacgagactgacagagcttctattccccggcaccctccgtgaacttgggcacccaaaactaagggatctgaaacccagccaggtgtgtgtgtctgagccctgccattcggaggcatcaccgagaggttctggtctcccctgcccaggccctgcctcctggccccactgcaggaagcttgagcagatctgaagctcgcctcagaggaagatcccatccaggggaggccctgtctgcctcctaggagtcggagggtccgtggaaatggtctcctcctgcacatctgtgctgctgtgactgggtgcaggtctgagcagaggctttcggagtgagctgagcaggcgagcccgagcacggcctctcagggagcgagcccataggctggggagccgtccctggagatgcccctgggctccttgcggggcatggctgagttcctgcctgtccttggcaggcccgcagtggtggggtggctcaggcagttacccttttcacaaccagtgctgctgggggtgaaggcaacgggtgggtgagcacggacagtgtgagccacgtggccgggagctgggccagctcgctgtatgtgcacatcgtttccatgtgtgcagcagaaattggcgtctctgcacaaagctgattttagtctttctcaccttttcttgctcagcttaaaataggcctctcttcagggacaaggtggccttataccaagccaaagtgctgagggcgcagggagacccgcgagacagggccccctgaagtcctggcggtttctagccagcctcttgaaattgacttgaaggtgtttaccttgcagattattttttccaacttcccacactctgcttcccgcactctgtccttcctcaaggctggcacgctcatcagttgacttcatctctccctaatggcaaggcctgacccagaaagaaatgcaactcagatcccggctcaaatgaggctgggaaagctgatgcctgtaagaccgacaaagacggtgcaaggtgaggtgaacgccgctgtgtctgggtgccgggctcccttgtcgagttgaccctgagtctgcatcagctcaaacgcagttcccggttccccactgagattcccactcccgcctggaggggagacgtgcctgccttttgaatgaagcgttgcacactagacatagtatcacaggcagaattgtcatttttagcctttttacatgttgccaactttcagacatactattccgttttatccctccaaattcctcaaaagctgcttctattttggagctctttcttgccagtgctgggtaatttctccctagccatgtttttattgtagagaatggaaacctgatgtgatgaacactctgagtagaaatccctgggggctcgcagttaaccggataagacatctcaccctgagaaacggtcccaatttccttttaaaaattcattgtctctctgagatacatacatatttccttgtctcattccagaatcaaaagttctaatgttgcaaagaataatttttgtccaaatatgttttcttcctggtgttccagagagtctgggatagcaagaggtgtggagctttggtcctcgggtgactctgattccatcgttcctccagcaaccagggagcaatcactgctgggcagggaacacctgcttcct

SEQ ID NO: 19537 - RNA, 591 nt, Homo sapiens
  source 1..591: mol_type = other RNA
ttggactttttcagatttggggatacagaaggatgcaaaatgaggcaacctagccacccaactggcccagtggtcaaggggggaaatgaggtggccgctagtcagcgctggagccatttctcgacggtgctttctgtttgtttgtttgtttttgttttgagatggagtctctctctgtcgcccaggctggagtgcagtggcgtgatctcggctcactgcaacctcaacggtgcttttttctgatcatagctgagctcaaatgctgaccccagtggcctgtctctaagcactgtggctccaggaaggaaaggcctggagagacctgtcaggatccagacagttgctgaggaccaagatccagacgagactgacagagcttctattccccggcaccctccgtgaacttgggcacccaaaactaagggatctgaaacccagccaggtgtgtgtgtctgagccctgccattcggaggcatcaccgagaggttctggtctcccctgcccaggccctgcctcctggccccactgcaggaagcttgagcagatctgaagctcgcctcagaggaagatcccatccaggggaggccctgt

SEQ ID NO: 19538 - RNA, 2028 nt, Homo sapiens
  source 1..2028: mol_type = other RNA
ttggactttttcagatttggggatacagaaggatgcaaaatgaggcaacctagccacccaactggcccagtggtcaaggggggaaatgaggtggccgctagtcagcgctggagccatttctcgacggtgctttctgtttgtttgtttgtttttgttttgagatggagtctctctctgtcgcccaggctggagtgcagtggcgtgatctcggctcactgcaacctcaacggtgcttttttctgatcatagctgagctcaaatgctgaccccagtggcctgtctctaagcactgtggctccaggaaggaaaggcctggagagacctgtcaggatccagacagttgctgaggaccaagatccagacgagactgacagagcttctattccccggcaccctccgtgaacttgggcacccaaaactaagggatctgaaacccagccaggtgtgtgtgtctgagccctgccattcggaggcatcaccgagaggttctggtctcccctgcccaggccctgcctcctggccccactgcaggaagcttgagcagatctgaagctcgcctcagaggaagatcccatccaggggaggccctgtctgcctcctaggagtcggagggtccgtggaaatggtctcctcctgcacatctgtgctgctgtgactgggtgcaggtctgagcagaggctttcggagtgagctgagcaggcgagcccgagcacggcctctcagggagcgagcccataggctggggagccgtccctggagatgcccctgggctccttgcggggcatggctgagttcctgcctgtccttggcaggcccgcagtggtggggtggctcaggcagttacccttttcacaaccagtgctgctgggggtgaaggcaacgggtgggtgagcacggacagtgtgagccacgtggccgggagctgggccagctcgctgtatgtgcacatcgtttccatgtgtgcagcagaaattggcgtctctgcacaaagctgattttagtctttctcaccttttcttgctcagcttaaaataggcctctcttcagggacaaggtggccttataccaagccaaagtgctgagggcgcagggagacccgcgagacagggccccctgaagtcctggcggtttctagccagcctcttgaaattgacttgaaggtgtttaccttgcagattattttttccaacttcccacactctgcttcccgcactctgtccttcctcaaggctggcacgctcatcagttgacttcatctctccctaatggcaaggcctgacccagaaagaaatgcaactcagatcccggctcaaatgaggctgggaaagctgatgcctgtaagaccgacaaagacggtgcaaggtgaggtgaacgccgctgtgtctgggtgccgggctcccttgtcgagttgaccctgagtctgcatcagctcaaacgcagttcccggttccccactgagattcccactcccgcctggaggggagacgtgcctgccttttgaatgaagcgttgcacactagacatagtatcacaggcagaattgtcatttttagcctttttacatgttgccaactttcagacatactattccgttttatccctccaaattcctcaaaagctgcttctattttggagctctttcttgccagtgctgggtaatttctccctagccatgtttttattgtagagaatggaaacctgatgtgatgaacactctgagtagaaatccctgggggctcgcagttaaccggataagacatctcaccctgagaaacggtcccaatttccttttaaaaattcattgtctctctgagatacatacatatttccttgtctcattccagaatcaaaagttctaatgttgcaaagaataatttttgtccaaatatgttttcttcctggtgttccagagagtctgggatagcaagaggtgtggagctttggtcctcgggtgactctgattccatcgttcctccagcaaccagggagcaatcactgctgggcagggaacacctgcttcctccctgg

SEQ ID NO: 19539 - RNA, 645 nt, Homo sapiens
  source 1..645: mol_type = other RNA
ttggagggtgtggaagacatcagctgagtggacgcggtcctgggcctggctttcatgggtgcgtggcagcgcctcaattccgtaaagagtcaggtagccggctctgagcaggaagctgtaggagaagtcgaggagacccatctcgtgccagccactgcctgcttctgtagcatcgcccaacagcactgcatggaggttggtatacatggcttctgtgagtgcctggagctctctgtggagaagagtcagtttcatcctggccttttcatcactggggctgtaatgtggaagctgcacatcaaaaatcctctccatgaggaagatggcataggcatggaagtcgagcctggtgcgaggctcccacaccaccgcgtcgtaggagtgtgggtccaggagaacggtgacatacctgcccccaaccagtatagtaaagatgtcaccgtgcttctccttcatcctcgtgaggaagctggcagcatcttttccaaagtccaaggcataccccaaccaggggatgctgcccaggtccaggggaggctcaccaggtcgccgcgtgcggcggcggctcagtagcagcagcagcaacagtgcggccaggaggccgaggagcgcggcccaagccatcgcggggctggcggggctggc

SEQ ID NO: 19540 - RNA, 196 nt, Homo sapiens
  source 1..196: mol_type = other RNA
ttggccaccacacctaccccttgtccaacctccctcaaatcccaagaaacatattcacatctgatcattcaaagccagactgtatgctatctgcaagtgtttcttatattttccttccatcctccaggcaaaccaagaccctggggaggcagagaagccctccttttgtctcccatttcttcagctatataagtaa

SEQ ID NO: 19541 - RNA, 1167 nt, Homo sapiens
  source 1..1167: mol_type = other RNA
ttggccatggggctgcgcggggccagcaggtccacgtccacgctggcgcgcttcaggctgcccagcgaggtcttctcgcgggccacgggccggggcgcgccctccagccgccctgggggccccagctcgtcggtgctcaccgacttattctgctgataaaccgagtcgtggccccgctgcgtcagggcccgcagcgcgtccttggcgggggccggggccgcgggcttctctgcaggtggggcctggaagttgcccaccgcgtggcaggccaggtaggcagcgatgcccgccccgatgaggaagccggcatacacgtccacagggtggctgcggtactgcgtgatctgcgtgagcccgcatacgcccgcggcgatggcaaaggcgaagaccaggatgggcttcagcagcttggtggtgtccgagatgaccgagttgaagtacatcgacacatagaccgcggcgaaggctgacagcgtggcgtgctgggacgggaaggtcttccgtgcagacaggatggcgtggatgtcgtggccggagcagatgtcctgcgtgatgtaggggttgacctcgcaggacgtgcccaggagagtgtagttgggcttgcagacggtgaggaagaagggagtgtggtaacccgtggccagctggatcacgtccgtcaccagggctgtggcacacaggccgaacacgtggacacccacaaaccgcaccgtacgccgcaggaaggagttgaagttgcagccgccggcgttgatgctgccctccgccccggcgggccccccggcacggccccacagccgggactgcagacagtacaacatgccctcggccaccatgatcgaggcggcaggggccgcgaaggccaagctgagcagcatcagcagcgggatgagctcctcgttggtctccacgtagggcatggagagagtgcggtcatagcactggaagcccaccttggccggcttgaagaggtcggtcagctccaggaagtacaaggatacgatggaagaagccactatgggcagctccacgaagtagaagcagggcagaagcgtcatgctgtccttcgggatcttgttcttctccttggtggagatcatggtgccgcgggcgccgcaggccgtggctggcgcggccggcgcccagcacaaagcgcgtctcctccgt

SEQ ID NO: 19542 - RNA, 1251 nt, Homo sapiens
  source 1..1251: mol_type = other RNA
ttggccatggggctgcgcggggccagcaggtccacgtccacgctggcgcgcttcaggctgcccagcgaggtcttctcgcgggccacgggccggggcgcgccctccagccgccctgggggccccagctcgtcggtgctcaccgacttattctgctgataaaccgagtcgtggccccgctgcgtcagggcccgcagcgcgtccttggcgggggccggggccgcgggcttctctgcaggtggggcctggaagttgcccaccgcgtggcaggccaggtaggcagcgatgcccgccccgatgaggaagccggcatacacgtccacagggtggctgcggtactgcgtgatctgcgtgagcccgcatacgcccgcggcgatggcaaaggcgaagaccaggatgggcttcagcagcttggtggtgtccgagatgaccgagttgaagtacatctggggcatgggggttggggtcagggagggctccccacgggtcagcaagagggcctgggaagggcagtgaggggccggactcaccgacacatagaccgcggcgaaggctgacagcgtggcgtgctgggacgggaaggtcttccgtgcagacaggatggcgtggatgtcgtggccggagcagatgtcctgcgtgatgtaggggttgacctcgcaggacgtgcccaggagagtgtagttgggcttgcagacggtgaggaagaagggagtgtggtaacccgtggccagctggatcacgtccgtcaccagggctgtggcacacaggccgaacacgtggacacccacaaaccgcaccgtacgccgcaggaaggagttgaagttgcagccgccggcgttgatgctgccctccgccccggcgggccccccggcacggccccacagccgggactgcagacagtacaacatgccctcggccaccatgatcgaggcggcaggggccgcgaaggccaagctgagcagcatcagcagcgggatgagctcctcgttggtctccacgtagggcatggagagagtgcggtcatagcactggaagcccaccttggccggcttgaagaggtcggtcagctccaggaagtacaaggatacgatggaagaagccactatgggcagctccacgaagtagaagcagggcagaagcgtcatgctgtccttcgggatcttgttcttctccttggtggagatcatggtgccgcgggcgccgcaggccgtggctggcgcggccggcgcccagcacaaagcgcgtctcctccgt

SEQ ID NO: 19543 - RNA, 1840 nt, Homo sapiens
  source 1..1840: mol_type = other RNA
ttggccatggggctgcgcggggccagcaggtccacgtccacgctggcgcgcttcaggctgcccagcgaggtcttctcgcgggccacgggccggggcgcgccctccagccgccctgggggccccagctcgtcggtgctcaccgacttattctgctgataaaccgagtcgtggccccgctgcgtcagggcccgcagcgcgtccttggcgggggccggggccgcgggcttctctgcaggtggggcctggaagttgcccaccgcgtggcaggccaggtaggcagcgatgcccgccccgatgaggaagccggcatacacgtccacagggtggctgcggtactgcgtgatctgcgtgagcccgcatacgcccgcggcgatggcaaaggcgaagaccaggatgggcttcagcagcttggtggtgtccgagatgaccgagttgaagtacatctggggcatgggggttggggtcagggagggctccccacgggtcagcaagagggcctgggaagggcagtgaggggccggactcaccgacacatagaccgcggcgaaggctgacagcgtggcgtgctgggacgggaaggtcttccgtgcagacaggatggcgtggatgtcgtggccggagcagatgtcctgcgtgatgtaggggttgacctcgcaggacgtgcccaggagagtgtagttgggcttgcagacggtgaggaagaagggagtgtggtaacccgtggccagctggatcacgtccgtcaccagggctgtggcacacaggccgaacacgtggacacccacaaaccgcaccgtacgccgcaggaaggagttgaagttgcagccgccggcgttgatgctgccctccgccccggcgggccccccggcacggccccacagccgggactgcagacagtacaacatgccctcggccaccatgatcgaggcggcaggggccgcgaaggccaagctgagcagcatcagcagcgggatgagctcctcgttggtctccacgtagggcatggagagagtgcggtcatagcactggaagcccaccttggccggcttgaagaggtcggtcagctccaggaagtacaaggatacgatggaagaagccactatgggcagctccacgaagtagaagcagggcagaagcgtcatgctgtccttcgggatcttgttcttctccttggtggagatcatggtgccgcgggcgccgcaggccgtggctttggatggactcggaggcagcccagcttcctgggacaggactgcacggactgcctggggaggggtctttggccccccggttcctgcaggggggctcggggaggccctgtgagcagttggtcacaggtgggtcccattcgatgcgatcctgttcctccccaacagccctggagaagggggacgttgcctgctgtggctgcggctgttttcctggcctgtgagaggcggggccagagtggccgttgggaatctgggtgttgcaaggtgaccacaaacagctctctgggggaggaggaggaaaatgcaattgattttcaggagccttctgaggtcaggagtgggagagtgtgcagggggaccctcctggcagcttgggggtccaacagaagatctgggggagtctcagggtcttctccccctaggatcaccagtggtggagatggggcaggcctggccatggagggcacgttgcttggctgaggggcctgggcttgagtgtggggcctgggcttgagtgatgggagagttccgagcaggccggaggggttgagcgtaccagacgctgctcaaaacttttatttaaaaatgattattattattattactattattttgagatggactcttgc

SEQ ID NO: 19544 - RNA, 3480 nt, Homo sapiens
  source 1..3480: mol_type = other RNA
ttggctggtctctgctccgcagacaggcgttcaggaggcccctgaagaagtgggcagtgatgtcctgtgtcagggcacctccgtgggagcagaagtttctcatctcagagttgaccaagtggaagaactgctcgcatctggcagtgatgggctgttctgcctggaagctgctgccgcagaggacagacgaaggcaggcggaggaggatccgtttgtacattagcagctccctctgtctctgaaggctggcagccacgctccacccgcttgtcagagcctggagccgtctgcggaaaatctcaaagaggaagtgctcctgggaaggggtgtggccgagaggcactatgaggtcttgctgcagctccaggtcagctaccatctcctgcaatctggaaataatatcctcatttcctgtgcggccaccaaagaccaaatcagaattttctgagtggtcataactccttgagctttggtggaaatccatcagtgcgttgacaagaatggtacacgcagcctgcaggtctccgtcacagccccctgaagccgaggactcagggagaaagtgctcatggatcgcccactggtggaagtcctgccgttcagtatctgaaagagcatcagcttcaggttgaatttccagctccaggtgtaaccagtcttggtaagttaagtgaacatcttcctctttcaacacctctcggaaggttctgtgtgtccagagagagagggcagctctctgccagtctgcagaaggaaggtgcaagggtctccaggaaaggctggctacgtcctcctcagaaagaggctgtcgggcctctgagaacaatctgaacatgaggaactgaaactttttaataaggcctggagataagcagctgcacaaagtatctcgtgactgggaagaaaacttgcagagagagtaagaaattgctgctgtacaaaatttcaggcagaagaacaaggaatccctcgtcctacaggtcaggaggctgtcaaagagcgcagggacaggaaggccagcaccaggtgcaggaggacccacatccacctctgggagcgcagacctggactcacccaggtgcacggccagggcagccaaccccagcacatgtggggcactcaggctcgggccctggtgacggagcagctggcagagccgggtgagcactgcagggagcacacgtccacacatggtcctcacgaagagggcagcccagggaccctgcctctccgggggagcgacactggaggcagccatcaggttctgacagaaagacgtcagcaggaggtccacagccatgtgttcccgtggctccagtctcggcgtgttgatgctgagctgaatctttgatatctcaacgctgctgtcatcctcattgtggcccaggacagccctcagtctttcagaaatcactgccacctgtgccgatataacatcacgctggctggggtctgtcatggaggctctcagctctcccagtgcagctgtgagctgtcccaggggctcctcagcagagttgggttctgccctcactcccagggctgcatcttctggcttctcttcagcagcagagcaggcctggcagtaggtggagtacagagatggggggattttatctgctctcttcagagactctataaacgccacacgggagtcagggactttggggagcactcgaggtgtgagcagggcggggaggaagtgggacacgtagtaaggcctcctgaatatgctggcctccatgacggtgactgggatgttccccgtatgctcaaacaccatgatggccttttcaacatcctgaagagcttggctgtggggctcagtaatgtccccagctgatgacaaatcctcgtagagtcccatgttttctatagaaaccttgaggtcggccagccgtgtcttggccaatgagatgtagtctgtgaggagggagcggtacttgccgggaaccaggggtgggtggagaatgtgcacctgcaggtaccggggagactcaaaaggcacgagttctgacaagaacgtaaacaggaagaccagggccttcttgctgcagccatggtagcctcgtgtgctcccaaaggaggccttgaaccagtctgcatatgacaggaacgcagaggggccctccagtgctgcctggcgcacaaccaggaacgcagtgaccatgctgtccagctggcagctctcgaatgcctgggccatcaaacgcgccacccagtcttcaagcagctgctgcgcttctggaaagcagacaaccagggcagacacaaaggagagcactctctgccagtgaacctcctgcgtttccagaacttcttgcaaatggccaaccaactcctctgcactcagcatcacaaagagcctgcggtacagtgaggtgagcagagggtgtgtccgcgcaaagctccactctctctgcatctgaacagcatcagatgctttcagcacagggctgtgagtgagtatctgagtcagggtatgactgaagaacctcttcagaggatctgtggaaattacactgccaagcgtgtgtccactgaacactccgaaccagcacctcacgatcttgtgagtggaggactcctcctgtactccagcagccaaagcgtcaagtgcaaaaatcagcattctctgcagtacatcaaccgtgacctgcggcattttttcaggctccacagttcttctcagatctgagtttttctgaaatcccctcaaaacaaacatttgaacaaaatcagaaagcatggccctggcgacgtcagcatgctggcaggatgcttccatctgttcacaaaggcagcacagattcctgaagagccacgatcccacagcatgcatgtcgggatggctttccagcagctcttgcaggctcacaatgccttgtacgtgaagatgccacaccgcttcaagcaacaaagaactctgtattttccataattcttgacagaaggaaagacgggagaacatactgtgtgccaataaatactgagcaaactctaacagggaagacagcttctttctctgctccacagtcagcagcacagggtgactggtctccgctggagccgtgcagatctgtcccacgctagaggcaaccatcccggctgagagaatacccacgggaacccccagccttgaggcttgatcctgcaaagcagagcctataaatgaactagaatgattagcataggcctcagaactgtcacagtcaatcactttgctgagagacaattttttacacagtggaccttctacctcaagcaaaagggcattcaggtcctgatggcttcgcaggaggcgcacagctgattcctttaatttctgtgccctttcaggattatatttttccctcttgacccttcccgccagcagctcggcccaggccctccggcggccccctgggtcctggcccgaggcggagttcgggacccacgagtcggacatggccttggcgcctacagccccggcggcggctc

SEQ ID NO: 19545 - RNA, 3818 nt, Homo sapiens
  source 1..3818: mol_type = other RNA
ttgggacatacttatgctaaaaaaaaattacagtctaccctcaattgaaattcagcttgtgtcctgtattttatgtggcaatccctgagctgacctgctgggtccatagagggcagcctggctcatcctgaaggcttgaggtgtccccgtaagctgtgcagagctctgatttcctgataaagtcaccatttctggtactgcaggggtgacaatgtgttctacaagaaattttaaattcatttcaaaaattatctaacaaaattaatctaagaaatcccacaatacctgcatgaccacagataaccaagtaatcccattacaatgacatggcgtccttgttcagcaggcgtttctttttgtgtttctcattaaatgatcagcaagtgaggtgacttttaaaaaacaattacaaagctttttcccccaattttcaaatctagctagatgaatttagtttgtatttttaaatgttaaaaagcaagttcagatcagttcatccatttcttcaaaccatgactgtaaagaaaaccggcagaaattaagccacagaaatgtgttaaagtacattgcagatgggacttgaacccacagtccaggaaacttgggtttgaggtaaaacctcgtcttagcatatcttgtaccttgctctcatgctgtatctactttcatttgcgtgttcaaattacagtgttctagtacactctgaaagtgttaattttcatgctacagtggttgctttccacacagcgacctgaggttttggttgagtacagttaacgtggttgtaaaaacgtctgattaaactctcctgacaaccgaccttgcaacaaaagtcatacaaagacagtgtgttttcagcttttacgctgtgtaaacttacaagtgagaccttttctgaaactattttttttgattaacaaatgttttgaaaaagagtttttagaaacttcataaaattaatcttctagaaaccataaggcatttttgtttacttgagaagaccagaggttgatggtgcaggtccctccagtggcccgaggatctcagtgttctgggctattgactctgcactttccctcgccttaccctgttggtggcaagacagctgctggagcaccaggcgtcaagtccttctgcctgcactctggcagaaaagacaagtcagaggaagacatatttcccacagaattaaaatgacatggcagaagatctttcccgtaagcccagtaatgagcctggcctccgcccttcacccggtgctccgtattttgagtctacttgtaatcagatttggagcttccgagggctgcagattcagcctcaactccctgctctcagattctctttgatcccagcttcatgagaatgtttgttttatttttgaatgtactatgatttgaatagctcactttctttcttaacatttttaatatcgtgaaatataacataaaaataggcacaaggcaaaaacatgctcctcaattgtttatcaagaaatgtgaccacacccaggtcagtacacagaacggccagaactcccaaaggcctgcgctttgtatgcccttccctgcgttgcaaagttcactatgctacgggctgcagtgcaatcacagcttcgcctttctgcagaggcttagctcaacatcactaagtacaacggtgttgccttccttttgaatgttacagacatgtaacatcatgcagtctacagtcctttgcagtctctcggttttacttgtgaggttcagctgctgctacctgtagccatggttcctttggtgtcactgctgtacaccgtcttattctgccgcatcaatgtaccgaagttcatgtatctattctctgtgtgggtggccaggaggcctgtgttgctgtctcgccctgggagggtggctcctccagtgtgggatgtgttgtaggtgtaacatacacaccgatttcaaagactctggtttacaaacaccgttcttttttgtctgaaaacttccaagttctcctgaaagcctaggctttgggaagaccaattcttgatatgcagctacttctgtgtgaagagtgagaagagaaggaggcggtggcagggagaggaaaaccccgtgtgtgtgcacattccaaaacacccacagccacaaacggcagatccgatgttttatggtacctttttactaaatggttgtgtttctttccttcgttctactggcccaagtcctaggtgcttaccaccatcagctgatgaggagggctcattggatgctgccgagatttgaaacaagagtcttccaaaccaaggtttcaactgtgaagtcgtttcttgcttaaagggccagtggaatctccttaaaaaggaatggaacatcttagcactctgtatcttttggctgagacgtatgcttcaaaataagtgttttcctgtaaacgggtccttactaagtgttggggtgagtgaatatgtgctcttgaaatgtgttatggtggaacgaaagcttcagtcacctgcagacatttccccggcggagataagcttcttccagtctgggcctggagtttcccttactccatcggaaaggaacccagactggtgataatgacaagttggcagtgtggctttcatgcaccagggccagtgatggaaatactctcttacccgaggctcgcagaatgctataaacttggggatggaggggccacaatgctggagggaaaagcataaagcagcccggagacaagaaacagactcgccaatcaaatgctgtgccttttccctcggtcccaggatggctgccctcatgattctggtgtagtccctgtcatccagcgccactgtgccgggctggcaatgccagtgctccatattagacagaaggacaaagaaagcttttaatttagtatcagagtaatgaaaacgccttcttccgcggatactgtaacactggcagggttttaagtaaatggaatcagatatttaaaaaggatttgccgaaaggaattaggaaagaatgcttcaaaaacattttaaatgctgcttagtagaggctcagtgttcacctaaatcaaagatgttttccccatatatttattttaataatttaaaatatgtctacatgtactaattacctatatttatctatctgaattttttcttcaatgaccaatatacaatgagtggtatatactgcatgtgtactgttttaaagacatactgtatatttaggaaaaggggtttcacatttctgccactttgtggatccctctgcttggctatctttttaaatttataggccttatttcccattaagactggaacaccttccaaaatattttctttttttagacatctataataagatgaaataacagtagtggcaaattcactgcgctcttgaagcatctgttggagctctctctttgtgggggtaaaccagccgccaaacagatcacctgcacggaaagtcctttgctcattttgtggatctgagttgctgccaacttttccgggtgttcatgttcagaaggagaagcaagatggccctgttaaaaagtcctacatggcatttgtcaaggatgttctgctcaggagagagactgaggcttccggtgagaaaaccctgcaggctggggaagtgcacctcgagctgaccccttgttcagggagctgatgaaggcacatgccatgggaatgagaaagccactccttaagcatcagtaacagaaggtgccatgtggataatacaggggctgaaaaatcataagattatttgggtgtccccacccaaatctcatctcgaattcccacatgttgtgggaggaatctggtggga

SEQ ID NO: 19546 - RNA, 2165 nt, Homo sapiens
  source 1..2165: mol_type = other RNA
ttgggagggaagacagctggagacggcaagaagtcagctgaacagctgagatgggcgaacaaggagccaccgtttactgcagctctgctcccacacgctgccgaacacgcctctgggctttccagatggtttctcctgttgattctgtgctgaaagccctgccccttggagaaatacctggaggatccaagtggcttccattcagagaaggacaaattcaagaagctatgctatgacctcatgagtggggcagtggagtcaggaaagcatgcgatgttaactcacacgcccagccgctgctctcatccagtgtctcatggcttcgagggaaataatagcaacagcaagccacgttaagacagagtcttgctgcttctttgagtgacactgggaagcttgattctgactacacagcatcccctgcatattcctctccactcagtctgctgcctccttggtgctccttggtcttcctctgaacatggtacctcattacacgggccttggccttcccacagtgtggtggtcttaggcggtcatgcttcttacacaagcctgcttggtaacagaactaacctcaggttcatccaagtaacaggctgttctggtgctcacccaggtaatagggctgttcttaggttcatccaggtaacagctgttcttgtgctcacctgggtaacagggatgccctgctaatgccagggaggaaagccagactcttgggtagaaagaatctgatagcagcctggctctctttgcctctgttaagcatcactgtgttcaatctccatttttagaactccacattaaaaggtcaagtgccttctaaagtatttattttctctccagtgtttgtgccctgattgaaatgacagcaccatgctgcttccctcgcacccacatcaagcttgatccacttggcacaggttattttttacccgaatggccaaagaagcctgaaattcacagcatttggggttctgttttttcttaatctggctgtaaccctgactcctagagccacaaaaacacgtggccactcagaaaaagcacaggtgtccttcctcccatggccagattggtggaatgcacctgccaagtcttcacccccatgggctttacctctgaacatatgatcttgctaaagtaaacccagctctgcccacctgtaggaccccaccatcccagaggtggccttccggagccctgcctgagggcttgcagaaagctcacggcgtggatgtctggattgctggcaggccttctccctgatctggctgtgtcttgtcgcctcttgctctgggcttcctggccagtcactgtgtcacagaactccatgaacttctctcccgctgtagctctccagaacagcccaaggcgtggccacacttcaccttggattccccacaacagagaatatcaggctccagtgttccaggtccagcttcccaggggctcctgggaaccaggcaagaaatcacaactctgaggagaaagccaaaccctgtttatcaaagatccctgtgtccttgtctattggccaggccccaggactggtgtcccctctccagagtccaggcctcctttctccaggggcctcatttccagagcaggcagggtacaggcactgttggattcacccgcacagctctgagagtgggcttggcccatttgcggaaccccgaaccagggatgccaaggttctgtgcactccaggctgctcaaccccaaactccagaagcaggtgaaaagagaatgtggctggaacgctcttctagcaaggtcctcgagttcttggaccagaaagacaaaacccttctcccatgggaaaaacagacttctaaccctagagcacacaaaaccaactcgcaccattaagcccagccattcacattctttttcgcaactctccaccttcccaagggcaaagcaaagccttctttccaagacaagtcccatctctcaccccaaaagaagagcaggggtagttgacggtgaaaactcataacagataagtgaagaacttcgtcctcacatcagccctgggggcagaattcccggcccagcacagagcccatccgggtaggagggacagcggcctgcgtgacgtggttgtcagagacagcctcgtgcttccatatcgccacccgcagagcacaacagtt

SEQ ID NO: 19547 - RNA, 4313 nt, Homo sapiens
  source 1..4313: mol_type = other RNA
ttgggagggaagacagctggagatttgaacaggagaggagggaaaagaaaagaaaagctttgaagtcagcctggcagccccaggatccctatttcccaggtgttagcaccccgagcttccaatcaacaaacaatggaggctgatcagtgggaaaaagatgggggatggctatgcctgttaaagggttaaataccagggactatctattccccaggcctaaagagagagacacacacagaccccttcaactcaaatataaacaaaataaaacaaaaacaaccccccatccaaacttgaccagttacgtgcaactagaatcagagttctcggccggggcatgggatggggggtggggatgcaaagggaagcagaaaagacattcctgaagaagtcgcagccttatctgtcctcagcagctctggaggcagccaggaccacagcctccggggcaggcagggaatccaggaagaatgagcttcagggtacgggagcaggggtctgaggggcctcccccggcttgttcgaaggggtctaaaccaaaagcaactcagtggagagaaggttgaggacccggttgtcttaacaagccccaaagaaacagccaccccggtgtcggcctcggaggttccagctacagtggcagctgcacagcttctgccccagctaagagcactggaatctgctctggcctcatggggtgggggcgccggccaggcctggactctgtaggggaggtggtcagctttgattgtccagatacaaaacacagactggtattgaattcagcctgatcccgatgtgggccctgctcccggctccagcgagggcaactccctgaaacgttctggccacaaatccattaaaaatggtcctccagagaaaaacactctgctaaagtctaaaatgaaaatagagagagagcagagagaggagagagaaatgctggatgtgggaagacagcaatctctaaaacggagaaataatttttaaggacaagaaaaagaacagcaaaatgacacgaaggcacgccagcaggttctgttaaaatgaccatactcttttcggatcctgggaatgtccacgttcaaataaacaagcgcctgatcgcgagccgagcactttcttgctgccgataaagcgaacgtttacactgtgagaaaggcgagattgatttacgaatctgaacgcgccagttttatggctgatcacaaatccgtcagcgctcaactcacgctgagaaacttcccaactccgttttccaaccagaccccctccccagctgccgcttcccagggagacccactgccagcgctggggccgccttcaagggctctggcagaactgggcaaccccctctgcccaggacaggcgggtggaagtaggagggagaatggggagggccgagggaactggggagaaagagggaaagaagtcaaaaggttgggaggactggagtggcactaggattgtctggagtgaaggaaatgggagatctggcagttccccttagtgaaccccaggcttccctgactatggtctctctccttttccctttggtgggccctaatcctcacattgcagaaagcagtttgtaaagtcctcggcgactaggtctttgtcacttgagcctgtagaaggcccacaactggctatctgcccttacaggtaatgaatacacatctccctgagccccatatatttttagtccaggagcagcctagctagctttgtgctcatcctctgtctttcctgaggcctccagcccctctacttatgccacccagggacaaaggagagagtatcaaccactccagttatttcttgcctgagatagagtccccaaatgtcaagaaacaatttacaaaatgcaaaccaacaacccacatatcccagcaaggttctgtctctcctagtcttaactgaagggtaacatttcatcttcccagccagcgtctgtctgtatctgtctctctttctctttctctttgtctctgtctctccctaagagggtggctgctggtgtggatttttaagatacagcaaacagaatacagtttttggaaaggctctatgttcagggctcactgtttggcaaatccttcacctatttcttaaaagtttctggaaactttggctaacctgggacagcaggccctggaaagtactcagaatagcctgcactgatcctcctcccatttcccttgctcctctggtgggtgaggcactccaagggcttttttcattattgaggagattgagaattaggggaaagaggtaaaggtagttatagaaatagcttcctcaacaaatgaacttcagaaaatgggttgacaggctgtggatttggatgtcagccctcagggagatgacagcctctgaagcaatgttcagggcggataagccctttctctcctcgcagcccaggagtttattcccctggccctctgaagccttgtggattaggcccctccaacctctcatatcttctccctttgtctttcttccctcagttccctccaggtgaaatagtaaagagatgaactggacctgggagtggttgcggggaggatggctggagcctggactgctgaaggtgctgtgtacagagagacagattagcaccctactttcgtcccccaactggacccttgggctaaaaatctttacgtttttttcccccagtgggcagtaatagaaaaataatccaaaatttccaaaatagcaaagatgggtttggggcctagagggggatggagaagatgggacatatgatgggccaaggacccctccctgcagaggtgtgactctccctcctgggcaggaggcaaatgccaacacaatgtccagtctcagcgaggtcaaggggcttccgaggtcattttgtggttctaatactgagctaatcgcctagaaaacgtggcctctccatgaactctctctcctgccagcctcccgcctccaaaccctaagtgaggcctcagggaaaaagggccaacacattcaggtcggctgcagagcccactgactccctcagcctaagaaacagggctgcagaggagagaacagagacctcaaattaggagagcaaagggaaaccaaaccaaaccaaaccaacattgctcctccaggaagaaggctggggggacagagcagaagagaaatatttctgcatcagtccaccttgtctgtgaactgagcagtttcctgctccagagagtagcacatatttgtctagaatcccaagctagacacaagaagaaaaaaaagaacatatccacttatacccgctccaaagctggaacattccatccaagcactggatttgatttttccaagaggcagcagtgacaacgtctcactggtaaacaggcataggggacaccagtacccagtgtagacaagcagagtcacaggaacacaccgaccacatgtggacctcactagacacacccatgcacacatgctggggctcgctgtgcctgcctgcattttccaaaaccagaaaagcgcttctgaactgcctcacaaaacaaccgtcttctctggggtttttcatgggccctgacacctcagtcccaaccagttcaaacactctccaggtgtcgaggcccctctttctctccctctgacccaagcatcagtcatcataaaagggagcaaacctgctgaagcatccaccataaaaacccagccaagaaagttaaaaaagaaaaaggaagaggcgagagagtgtttcttctttcagttgtgaaaagagctcataaaacgatcaaaacacgccagcccgggcccgggctttgttacctttgcgcctctcgcctcctctcgcccgaactctgcagatcccattcatgacgaagggcttcttccaaactgagagaaaaaagttttcaactttatggttccaaattttttcccccttgcagatccgggagagacggctaacacttttttcccccaacagccggtccaaggagatttgcgggaggctccccagccccgccggccgccgagccgcccgcggacgcgccgggcaacagctgagctctctcctgtccactattgtgtgtccggaaaaccggaccgcggcggcggacacagccacgggctccctcagaagccggaacgtgacttttttttttggtgtgtttttgttttggaagcgcaagttttcgtgttaatctcatactttggcagtctttgttaaacagctaggcgcgtcacgaggctctcaaacattttaataatttttagacgccgtgacctgcggttcacctctctcccagcctcccccacgagcaggcagttactat

SEQ ID NO: 19548 - RNA, 4494 nt, Homo sapiens
  source 1..4494: mol_type = other RNA
ttgggagggaagacagctggagatttgaacaggagaggagggaaaagaaaagaaaagctttgaagtcagcctggcagccccaggatccctatttcccaggtgttagcaccccgagcttccaatcaacaaacaatggaggctgatcagtgggaaaaagatgggggatggctatgcctgttaaagggttaaataccagggactatctattccccaggcctaaagagagagacacacacagaccccttcaactcaaatataaacaaaataaaacaaaaacaaccccccatccaaacttgaccagttacgtgcaactagaatcagagttctcggccggggcatgggatggggggtggggatgcaaagggaagcagaaaagacattcctgaagaagtcgcagccttatctgtcctcagcagctctggaggcagccaggaccacagcctccggggcaggcagggaatccaggaagaatgagcttcagggtacgggagcaggggtctgaggggcctcccccggcttgttcgaaggggtctaaaccaaaagcaactcagtggagagaaggttgaggacccggttgtcttaacaagccccaaagaaacagccaccccggtgtcggcctcggaggttccagctacagtggcagctgcacagcttctgccccagctaagagcactggaatctgctctggcctcatggggtgggggcgccggccaggcctggactctgtaggggaggtggtcagctttgattgtccagatacaaaacacagactggtattgaattcagcctgatcccgatgtgggccctgctcccggctccagcgagggcaactccctgaaacgttctggccacaaatccattaaaaatggtcctccagagaaaaacactctgctaaagtctaaaatgaaaatagagagagagcagagagaggagagagaaatgctggatgtgggaagacagcaatctctaaaacggagaaataatttttaaggacaagaaaaagaacagcaaaatgacacgaaggcacgccagcaggttctgttaaaatgaccatactcttttcggatcctgggaatgtccacgttcaaataaacaagcgcctgatcgcgagccgagcactttcttgctgccgataaagcgaacgtttacactgtgagaaaggcgagattgatttacgaatctgaacgcgccagttttatggctgatcacaaatccgtcagcgctcaactcacgctgagaaacttcccaactccgttttccaaccagaccccctccccagctgccgcttcccagggagacccactgccagcgctggggccgccttcaagggctctggcagaactgggcaaccccctctgcccaggacaggcgggtggaagtaggagggagaatggggagggccgagggaactggggagaaagagggaaagaagtcaaaaggttgggaggactggagtggcactaggattgtctggagtgaaggaaatgggagatctggcagttccccttagtgaaccccaggcttccctgactatggtctctctccttttccctttggtgggccctaatcctcacattgcagaaagcagtttgtaaagtcctcggcgactaggtctttgtcacttgagcctgtagaaggcccacaactggctatctgcccttacaggtaatgaatacacatctccctgagccccatatatttttagtccaggagcagcctagctagctttgtgctcatcctctgtctttcctgaggcctccagcccctctacttatgccacccagggacaaaggagagagtatcaaccactccagttatttcttgcctgagatagagtccccaaatgtcaagaaacaatttacaaaatgcaaaccaacaacccacatatcccagcaaggttctgtctctcctagtcttaactgaagggtaacatttcatcttcccagccagcgtctgtctgtatctgtctctctttctctttctctttgtctctgtctctccctaagagggtggctgctggtgtggatttttaagatacagcaaacagaatacagtttttggaaaggctctatgttcagggctcactgtttggcaaatccttcacctatttcttaaaagtttctggaaactttggctaacctgggacagcaggccctggaaagtactcagaatagcctgcactgatcctcctcccatttcccttgctcctctggtgggtgaggcactccaagggcttttttcattattgaggagattgagaattaggggaaagaggtaaaggtagttatagaaatagcttcctcaacaaatgaacttcagaaaatgggttgacaggctgtggatttggatgtcagccctcagggagatgacagcctctgaagcaatgttcagggcggataagccctttctctcctcgcagcccaggagtttattcccctggccctctgaagccttgtggattaggcccctccaacctctcatatcttctccctttgtctttcttccctcagttccctccaggtgaaatagtaaagagatgaactggacctgggagtggttgcggggaggatggctggagcctggactgctgaaggtgctgtgtacagagagacagattagcaccctactttcgtcccccaactggacccttgggctaaaaatctttacgtttttttcccccagtgggcagtaatagaaaaataatccaaaatttccaaaatagcaaagatgggtttggggcctagagggggatggagaagatgggacatatgatgggccaaggacccctccctgcagaggtgtgactctccctcctgggcaggaggcaaatgccaacacaatgtccagtctcagcgaggtcaaggggcttccgaggtcattttgtggttctaatactgagctaatcgcctagaaaacgtggcctctccatgaactctctctcctgccagcctcccgcctccaaaccctaagtgaggcctcagggaaaaagggccaacacattcaggtcggctgcagagcccactgactccctcagcctaagaaacagggctgcagaggagagaacagagacctcaaattaggagagcaaagggaaaccaaaccaaaccaaaccaacattgctcctccaggaagaaggctggggggacagagcagaagagaaatatttctgcatcagtccaccttgtctgtgaactgagcagtttcctgctccagagagtagcacatatttgtctagaatcccaagctagacacaagaagaaaaaaaagaacatatccacttatacccgctccaaagctggaacattccatccaagcactggatttgatttttccaagaggcagcagtgacaacgtctcactggtaaacaggcataggggacaccagtacccagtgtagacaagcagagtcacaggaacacaccgaccacatgtggacctcactagacacacccatgcacacatgctggggctcgctgtgcctgcctgcattttccaaaaccagaaaagcgcttctgaactgcctcacaaaacaaccgtcttctctggggtttttcatgggccctgacacctcagtcccaaccagttcaaacactctccaggtgtcgaggcccctctttctctccctctgacccaagcatcagtcatcataaaagggagcaaacctgctgaagcatccaccataaaaacccagccaagaaagttaaaaaagaaaaaggaagaggcgagagagtgtttcttctttcagttgtgaaaagagctcataaaacgatcaaaacacgccagcccgggcccgggctttgttacctttgcgcctctcgcctcctctcgcccgaactctgcagatcccattcatgacgaagggcttcttccaaactgagagaaaaaagttttcaactttatggttccaaattttttcccccttgcagatccgggagagacggctaacacttttttcccccaacagccggtccaaggagatttgctgttgaataataacaaaggagagaggatacgtatttaaagaaaagaagtgattaatggttttctgtataattctcacatttttcttagctcttgtctacacagaatggctgtgaactttaagctccatagaaatcttttttttttaaattctattcataccttccaaagagcagctttgatttggttctttagagacattccttaggggggcatatgctttttaagaactattttccccctcaactggggctgcggcatccccttgcagctaaaccaccacaccgcaatccgaccgaaataaagctcgcccctctcatcctccaggtccacgatgatttttttacgagtctcccagcagcatttaaacggacagttcagcagctcttttgcggctggggacaccggcctgtcggttccccctgccctacccagcctccaactaccggagctgcaagctggaggaatgcaaaataaataacaataaaacgcgcgggtgggattggttctttt

SEQ ID NO: 19549 - RNA, 3371 nt, Homo sapiens
  source 1..3371: mol_type = other RNA
ttgggcccaggagtaaacaggattaaggggcgtggatgtgggtgggtgggggaagagagctttctcaggatcggcaaccaatcccagaatctccagtcgcaggagcatgtatgtgaaggtttatttgcagggatccaccgtttgtaaaatagtacacgcttaataaaattaattttgaggtcaatcttaactgacagatctcttctttcttactggcgagtatttgtaaaataagaaaaacaggaggaaaagagaacaaacaagagagatgtgggatgacggagtaaggaaaggagtcacggagaggagagacaatgtctgtggctgttccctcagcgtctgggagaagagcccaagaatcccattgaactgagggggaggaaaggccctcctgcggcctaccgcaaggaaacgatcgcggcagacccgggactagcgccaaagggcttggaagggcggcgttaagaaaaatgggccgtacctacaacttctttcgcagccctcgctggcccgggagcggcccaggagcccagtgaccgttgcgtaagccacgcgccacccaggtgggcagggtggtgacgcgaaagcccggatagacttccgcgcaggggcggggcggggcgaggaggcggcagcgcgtttaagtgacgtcttggctgtccgcgccggcagaggcgagggttctggggtttctgggactgtctggtgtgttttctgtctattgaaccctttcctttcgacgtctcttctgaatattgactcatcgggttgtagaaatccagggacagagttgacatcactgggcattttagccaaaaagcagtgctcgggactgcatgtgccagaagtaaacttgtcaaaactcagattgtgtttcccctaaagtcagcttaaagtgcaatggtagaagagcacggtctctccccaagacggcctgagcttaaactgcagcgctgtcacttgctagctatgggacctaggcaaatacatcgtctccctgaggttgtcttctcatctgtaaaggacgctgtggtggtggtgtgagaataaatgagacatggcaagtgtctggaacaaagacgctgtgtacaaagtaaacacttaatatactgttatcagtataaaacctttgtgagttttttttttttttccgcatgaaatcttatgtggaaagttgtatgtgaaagaaatgaaagcggagctgcgttgatggtgggcccagaagctttggcctttcagtcccaaagtttccagtaatagaatccgcgcttcctctaaacttgcacagaagtctctccttgaacttcttcatctttattttgatgttcaactttctgcagaagcctggggcccagtaaaccaataagcagacttccaattggggctgtgatgaggatggacaaaaatgccactgtcaacacatccattccatagtcttctaattgtttctctccatgtgaccttgctgtgtccaaagccacagatcctattgcagcctacagtttctggtctgagagatgcaatagatacctctgctccaattagtccaaaaagaaggggctgaaaaatgtcccaggcaactgcaattatcttttcaacctctgccttttcgctggtccatcccatgcctgcaaggaaagccatgaccaacgtgcacagtcctcctgatccagggaaaccaaaatgcacactgctgaacacagctagcacagacaaccccaacacaaggaatgttctcttacacacaagtttgtcctggtcacggcttggaaagtactgaatgaaaaatccaagaacagatccagttgccacaccaattaccacctccaaaactcctctgaggacattaaagacagtagagcctgtggaaaaggctatgcccaagcatgtgttgaagccagtgatggccagaatgtcatcgaagctgccagctgccatgagcaaggttgggacacccttctcaacaccatagcctcctccctgcaaaaggagcattgaaggcaccacaacagctggagatacagcacctaaaacaaaacccagtataaatccccattgccatggtaaacccagcaggtaatgggcaagaagagcagatgtgcacgcctccacaatacagggacccatggacagtcttacacaaacgccctttaacttcttcagggcctttgaatccagaccaaggccagcacgaaccagaatgatagacagggctatgcttctcaaagaggaagaccacttgtgcttgatctgcacattatcgttgatgactgggatatttctgatgagaaaccctgcaagcagcatgccaagaagagaaggcagtggaggcaatgtaggtaacttaataagccccaaaagtttaccaccaatgatggcacaatagaataggattataattccaaataggtttcctccaggaagacattcactgccagtaattgaccaaactacagcccacagaagaacaatgatggtaacatttgttatgaccctgtccagtaaaccatgtggagggcaagccagcatttgtctcagtctttgtacgtgatttgcttcagttggtgtttcttgtagctttttttcactgcttttcaaaagaatacttccttctgttggttcatttgcatctatacctttgagcttcataactgtctcctcctgtgcttcttgatgcatggagggcgtgtaattcattcctgtggatggttctgaatcttcatatgtaattcttttatcttcatcccccattatttataattaagaagatgacacagggaagaggaacgagatctggcagtctccggcgaagtcgaccaggctccgtctgaacgattaggaaaggggctgtgggggaggcggcggagcccggtctagccaccgcgctctggggttcccgattcgcgcatcttcccaggctgagccgggaggctgcgttgactgcagataaacggtctcagggcgcggcaccgcgtgtagtcggccccgcctttcgcacgaacccgctgggcgacaccgcgcagggaggtccgacccgtcggcgccggtacaggctccggagtaagcatgggttggtccggggcccgcagcggcagccccgtgtgccctccgccgggtttcaggtccggcggcgcgggtgcagagccgcgtgcgatgcctggtgcgcgtggcttcccccggaaaggtggcgccaggccgaccatgggcccacgtcccggggcctcggagcggcaccgcgcggtctttcagctgcttatcctccctgggcgggtccgcaggcttctggggccaggaccagcgagctcccgggaaagcttcccggaaagcttacccagagagcgcggacccaggcgccgagtcttcccggagat

SEQ ID NO: 19550 - RNA, 3200 nt, Homo sapiens
  source 1..3200: mol_type = other RNA
ttgggcccaggagtaaacaggattaaggggcgtggatgtgggtgggtgggggaagagagctttctcaggatcggcaaccaatcccagaatctccagtcgcaggagcatgtatgtgaaggtttatttgcagggatccaccgtttgtaaaatagtacacgcttaataaaattaattttgaggtcaatcttaactgacagatctcttctttcttactggcgagtatttgtaaaataagaaaaacaggaggaaaagagaacaaacaagagagatgtgggatgacggagtaaggaaaggagtcacggagaggagagacaatgtctgtggctgttccctcagcgtctgggagaagagcccaagaatcccattgaactgagggggaggaaaggccctcctgcggcctaccgcaaggaaacgatcgcggcagacccgggactagcgccaaagggcttggaagggcggcgttaagaaaaatgggccgtacctacaacttctttcgcagccctcgctggcccgggagcggcccaggagcccagtgaccgttgcgtaagccacgcgccacccaggtgggcagggtggtgacgcgaaagcccggatagacttccgcgcaggggcggggcggggcgaggaggcggcagcgcgtttaagtgacgtcttggctgtccgcgccggcagaggcgagggttctggggtttctgggactgtctggtgtgttttctgtctattgaaccctttcctttcgacgtctcttctgaatattgactcatcgggttgtagaaatccagggacagagttgacatcactgggcattttagccaaaaagcagtgctcgggactgcatgtgccagaagtaaacttgtcaaaactcagattgtgtttcccctaaagtcagcttaaagtgcaatggtagaagagcacggtctctccccaagacggcctgagcttaaactgcagcgctgtcacttgctagctatgggacctaggcaaatacatcgtctccctgaggttgtcttctcatctgtaaaggacgctgtggtggtggtgtgagaataaatgagacatggcaagtgtctggaacaaagacgctgtgtacaaagtaaacacttaatatactgttatcagtataaaacctttgtgagttttttttttttttccgcatgaaatcttatgtggaaagttgtatgtgaaagaaatgaaagcggagctgcgttgatggtgggcccagaagctttggcctttcagtcccaaagtttccagtaatagaatccgcgcttcctctaaacttgcacagaagtctctccttgaacttcttcatctttattttgatgttcaactttctgcagaagcctggggcccagtaaaccaataagcagacttccaattggggctgtgatgaggatggacaaaaatgccactgtcaacacatccattccatagtcttctaattgtttctctccatgtgaccttgctgtgtccaaagccacagatcctattgcagcctacagtttctggtctgagagatgcaatagatacctctgctccaattagtccaaaaagaaggggctgaaaaatgtcccaggcaactgcaattatcttttcaacctctgccttttcgctggtccatcccatgcctgcaaggaaagccatgaccaacgtgcacagtcctcctgatccagggaaaccaaaatgcacactgctgaacacagctagcacagacaaccccaacacaaggaatgttctcttacacacaagtttgtcctggtcacggcttggaaagtactgaatgaaaaatccaagaacagatccagttgccacaccaattaccacctccaaaactcctctgaggacattaaagacagtagagcctgtggaaaaggctatgcccaagcatgtgttgaagccagtgatggccagaatgtcatcgaagctgccagctgccatgagcaaggttgggacacccttctcaacaccatagcctcctccctgcaaaaggagcattgaaggcaccacaacagctggagatacagcacctaaaacaaaacccagtataaatccccattgccatggtaaacccagcaggtaatgggcaagaagagcagatgtgcacgcctccacaatacagggacccatggacagtcttacacaaacgccctttaacttcttcagggcctttgaatccagaccaaggccagcacgaaccagaatgatagacagggctatgcttctcaaagaggaagaccacttgtgcttgatctgcacattatcgttgatgactgggatatttctgatgagaaaccctgcaagcagcatgccatttgttatgaccctgtccagtaaaccatgtggagggcaagccagcatttgtctcagtctttgtacgtgatttgcttcagttggtgtttcttgtagctttttttcactgcttttcaaaagaatacttccttctgttggttcatttgcatctatacctttgagcttcataactgtctcctcctgtgcttcttgatgcatggagggcgtgtaattcattcctgtggatggttctgaatcttcatatgtaattcttttatcttcatcccccattatttataattaagaagatgacacagggaagaggaacgagatctggcagtctccggcgaagtcgaccaggctccgtctgaacgattaggaaaggggctgtgggggaggcggcggagcccggtctagccaccgcgctctggggttcccgattcgcgcatcttcccaggctgagccgggaggctgcgttgactgcagataaacggtctcagggcgcggcaccgcgtgtagtcggccccgcctttcgcacgaacccgctgggcgacaccgcgcagggaggtccgacccgtcggcgccggtacaggctccggagtaagcatgggttggtccggggcccgcagcggcagccccgtgtgccctccgccgggtttcaggtccggcggcgcgggtgcagagccgcgtgcgatgcctggtgcgcgtggcttcccccggaaaggtggcgccaggccgaccatgggcccacgtcccggggcctcggagcggcaccgcgcggtctttcagctgcttatcctccctgggcgggtccgcaggcttctggggccaggaccagcgagctcccgggaaagcttcccggaaagcttacccagagagcgcggacccaggcgccgagtcttcccggagat

SEQ ID NO: 19551 - RNA, 3508 nt, Homo sapiens
  source 1..3508: mol_type = other RNA
ttgggcccaggagtaaacaggattaaggggcgtggatgtgggtgggtgggggaagagagctttctcaggatcggcaaccaatcccagaatctccagtcgcaggagcatgtatgtgaaggtttatttgcagggatccaccgtttgtaaaatagtacacgcttaataaaattaattttgaggtcaatcttaactgacagatctcttctttcttactggcgagtatttgtaaaataagaaaaacaggaggaaaagagaacaaacaagagagatgtgggatgacggagtaaggaaaggagtcacggagaggagagacaatgtctgtggctgttccctcagcgtctgggagaagagcccaagaatcccattgaactgagggggaggaaaggccctcctgcggcctaccgcaaggaaacgatcgcggcagacccgggactagcgccaaagggcttggaagggcggcgttaagaaaaatgggccgtacctacaacttctttcgcagccctcgctggcccgggagcggcccaggagcccagtgaccgttgcgtaagccacgcgccacccaggtgggcagggtggtgacgcgaaagcccggatagacttccgcgcaggggcggggcggggcgaggaggcggcagcgcgtttaagtgacgtcttggctgtccgcgccggcagaggcgagggttctggggtttctgggactgtctggtgtgttttctgtctattgaaccctttcctttcgacgtctcttctgaatattgactcatcgggttgtagaaatccagggacagagttgacatcactgggcattttagccaaaaagcagtgctcgggactgcatgtgccagaagtaaacttgtcaaaactcagattgtgtttcccctaaagtcagcttaaagtgcaatggtagaagagcacggtctctccccaagacggcctgagcttaaactgcagcgctgtcacttgctagctatgggacctaggcaaatacatcgtctccctgaggttgtcttctcatctgtaaaggacgctgtggtggtggtgtgagaataaatgagacatggcaagtgtctggaacaaagacgctgtgtacaaagtaaacacttaatatactgttatcagtataaaacctttgtgagttttttttttttttccgcatgaaatcttatgtggaaagttgtatgtgaaagaaatgaaagcggagctgcgttgatggtgggcccagaagctttggcctttcagtcccaaagtttccagtaatagaatccgcgcttcctctaaacttgcacagaagtctctccttgaacttcttcatctttattttgatgttcaactttctgcagaagcctggggcccagtaaaccaataagcagacttccaattggggctgtgatgaggatggacaaaaatgccactgtcaacacatccattccatagtcttctaattgtttctctccatgtgaccttgctgtgtccaaagccacagatcctattgcagcctgaactgtggcctttggaagccatgcaaaagaaataaatatcttttcttttaagttaaaaccagcaaaacacaccatcagaaatgtagtcaaaattcgtatcaatactgcaatgcctacggtggcaacacaaaggcctacagtttctggtctgagagatgcaatagatacctctgctccaattagtccaaaaagaaggggctgaaaaatgtcccaggcaactgcaattatcttttcaacctctgccttttcgctggtccatcccatgcctgcaaggaaagccatgaccaacgtgcacagtcctcctgatccagggaaaccaaaatgcacactgctgaacacagctagcacagacaaccccaacacaaggaatgttctcttacacacaagtttgtcctggtcacggcttggaaagtactgaatgaaaaatccaagaacagatccagttgccacaccaattaccacctccaaaactcctctgaggacattaaagacagtagagcctgtggaaaaggctatgcccaagcatgtgttgaagccagtgatggccagaatgtcatcgaagctgccagctgccatgagcaaggttgggacacccttctcaacaccatagcctcctccctgcaaaaggagcattgaaggcaccacaacagctggagatacagcacctaaaacaaaacccagtataaatccccattgccatggtaaacccagcaggtaatgggcaagaagagcagatgtgcacgcctccacaatacagggacccatggacagtcttacacaaacgccctttaacttcttcagggcctttgaatccagaccaaggccagcacgaaccagaatgatagacagggctatgcttctcaaagaggaagaccacttgtgcttgatctgcacattatcgttgatgactgggatatttctgatgagaaaccctgcaagcagcatgccaagaagagaaggcagtggaggcaatgtaggtaacttaataagccccaaaagtttaccaccaatgatggcacaatagaataggattataattccaaataggtttcctccaggaagacattcactgccagtaattgaccaaactacagcccacagaagaacaatgatggtaacatttgttatgaccctgtccagtaaaccatgtggagggcaagccagcatttgtctcagtctttgtacgtgatttgcttcagttggtgtttcttgtagctttttttcactgcttttcaaaagaatacttccttctgttggttcatttgcatctatacctttgagcttcataactgtctcctcctgtgcttcttgatgcatggagggcgtgtaattcattcctgtggatggttctgaatcttcatatgtaattcttttatcttcatcccccattatttataattaagaagatgacacagggaagaggaacgagatctggcagtctccggcgaagtcgaccaggctccgtctgaacgattaggaaaggggctgtgggggaggcggcggagcccggtctagccaccgcgctctggggttcccgattcgcgcatcttcccaggctgagccgggaggctgcgttgactgcagataaacggtctcagggcgcggcaccgcgtgtagtcggccccgcctttcgcacgaacccgctgggcgacaccgcgcagggaggtccgacccgtcggcgccggtacaggctccggagtaagcatgggttggtccggggcccgcagcggcagccccgtgtgccctccgccgggtttcaggtccggcggcgcgggtgcagagccgcgtgcgatgcctggtgcgcgtggcttcccccggaaaggtggcgccaggccgaccatgggcccacgtcccggggcctcggagcggcaccgcgcggtctttcagctgcttatcctccctgggcgggtccgcaggcttctggggccaggaccagcgagctcccgggaaagcttcccggaaagcttacccagagagcgcggacccaggcgccgagtcttcccggagat

SEQ ID NO: 19552 - RNA, 3102 nt, Homo sapiens
  source 1..3102: mol_type = other RNA
ttgggcccaggagtaaacaggattaaggggcgtggatgtgggtgggtgggggaagagagctttctcaggatcggcaaccaatcccagaatctccagtcgcaggagcatgtatgtgaaggtttatttgcagggatccaccgtttgtaaaatagtacacgcttaataaaattaattttgaggtcaatcttaactgacagatctcttctttcttactggcgagtatttgtaaaataagaaaaacaggaggaaaagagaacaaacaagagagatgtgggatgacggagtaaggaaaggagtcacggagaggagagacaatgtctgtggctgttccctcagcgtctgggagaagagcccaagaatcccattgaactgagggggaggaaaggccctcctgcggcctaccgcaaggaaacgatcgcggcagacccgggactagcgccaaagggcttggaagggcggcgttaagaaaaatgggccgtacctacaacttctttcgcagccctcgctggcccgggagcggcccaggagcccagtgaccgttgcgtaagccacgcgccacccaggtgggcagggtggtgacgcgaaagcccggatagacttccgcgcaggggcggggcggggcgaggaggcggcagcgcgtttaagtgacgtcttggctgtccgcgccggcagaggcgagggttctggggtttctgggactgtctggtgtgttttctgtctattgaaccctttcctttcgacgtctcttctgaatattgactcatcgggttgtagaaatccagggacagagttgacatcactgggcattttagccaaaaagcagtgctcgggactgcatgtgccagaagtaaacttgtcaaaactcagattgtgtttcccctaaagtcagcttaaagtgcaatggtagaagagcacggtctctccccaagacggcctgagcttaaactgcagcgctgtcacttgctagctatgggacctaggcaaatacatcgtctccctgaggttgtcttctcatctgtaaaggacgctgtggtggtggtgtgagaataaatgagacatggcaagtgtctggaacaaagacgctgtgtacaaagtaaacacttaatatactgttatcagtataaaacctttgtgagttttttttttttttccgcatgaaatcttatgtggaaagttgtatgtgaaagaaatgaaagcggagctgcgttgatggtgggcccagaagctttggcctttcagtcccaaagtttccagtaatagaatccgcgcttcctctaaacttgcacagaagtctctccttgaacttcttcatctttattttgatgttcaactttctgcagaagcctggggcccagtaaaccaataagcagacttccaattggggctgtgatgaggatggacaaaaatgccactgtcaacacatccattccatagtcttctaattgtttctctccatgtgaccttgctgtgtccaaagccacagatcctattgcagcctgaactgtggcctttggaagccatgcaaaagaaataaatatcttttcttttaagttaaaaccagcaaaacacaccatcagaaatgtagtcaaaattcgtatcaatactgcaatgcctacggtggcaacacaaaggcctacagtttctggtctgagagatgcaatagatacctctgctccaattagtccaaaaagaaggggctgaaaaatgtcccaggcaactgcaattatcttttcaacctctgccttttcgctggtccatcccatgcctgcaaggaaagccatgaccaacgtgcacagtcctcctgatccagggaaaccaaaatgcacactgctgaacacagctagcacagacaaccccaacacaaggaatgttctcttacacacaagtttgtcctggtcacggcttggaaagtactgaatgaaaaatccaagaacagatccagttgccacaccaattaccacctccaaaactcctctgaggacattaaagacagtagagcctgtggaaaaggctatgcccaagcatgtgttgaagccagtgatggccagaatgtcatcgaagctgccagctgccatgagcaaggttgggacacccttctcaacaccatagcctcctccctgcaaaaggagcattgaaggcaccacaacagctggagatacagcacctaaaacaaaacccagtataaatccccattgccatggtaaacccagcaggtaatgggcaagaagagcagatgtgcacgcctccacaatacagggacccatggacagtcttacacaaacgccctttaacttcttcagggcctttgaatccagaccaaggccagcacgaaccagaatgatagacagggctatgcttctcaaagaggaagaccacttgtgcttgatctgcacattatcgttgatgactgggatatttctgatgagaaaccctgcaagcagcatgccaagaagagaaggcagtggaggcaatgtaggtaacttaataagccccaaaagtttaccaccaatgatggcacaatagaataggattataattccaaataggtttcctccaggaagacattcactgccagtaattgaccaaactacagcccacagaagaacaatgatggtaacatttgttatgaccctgtccagtaaaccatgtggagggcaagccagcatttgtctcagtctttgtacgtgatttgcttcagttggtgtttcttgtagctttttttcactgcttttcaaaagaatacttccttctgttggttcatttgcatctatacctttgagcttcataactgtctcctcctgtgcttcttgatgcatggagggcgtgtaattcattcctgtggatggttctgaatcttcatatgtaattcttttatcttcatcccccattatttataattaagaagatgacacagggaagaggaacgagatctgtttttcactcctgtaagcaagtgccaatcttaatcaccgcttttcaagcaagggagattatcctcaaatttctccaccagtcagaaaccattcattcttgtctctcaggtcctcttttgtgatgaacctattggataggttccatccaatacccttcttcagatcatct

SEQ ID NO: 19553 - RNA, 3337 nt, Homo sapiens
  source 1..3337: mol_type = other RNA
ttgggcccaggagtaaacaggattaaggggcgtggatgtgggtgggtgggggaagagagctttctcaggatcggcaaccaatcccagaatctccagtcgcaggagcatgtatgtgaaggtttatttgcagggatccaccgtttgtaaaatagtacacgcttaataaaattaattttgaggtcaatcttaactgacagatctcttctttcttactggcgagtatttgtaaaataagaaaaacaggaggaaaagagaacaaacaagagagatgtgggatgacggagtaaggaaaggagtcacggagaggagagacaatgtctgtggctgttccctcagcgtctgggagaagagcccaagaatcccattgaactgagggggaggaaaggccctcctgcggcctaccgcaaggaaacgatcgcggcagacccgggactagcgccaaagggcttggaagggcggcgttaagaaaaatgggccgtacctacaacttctttcgcagccctcgctggcccgggagcggcccaggagcccagtgaccgttgcgtaagccacgcgccacccaggtgggcagggtggtgacgcgaaagcccggatagacttccgcgcaggggcggggcggggcgaggaggcggcagcgcgtttaagtgacgtcttggctgtccgcgccggcagaggcgagggttctggggtttctgggactgtctggtgtgttttctgtctattgaaccctttcctttcgacgtctcttctgaatattgactcatcgggttgtagaaatccagggacagagttgacatcactgggcattttagccaaaaagcagtgctcgggactgcatgtgccagaagtaaacttgtcaaaactcagattgtgtttcccctaaagtcagcttaaagtgcaatggtagaagagcacggtctctccccaagacggcctgagcttaaactgcagcgctgtcacttgctagctatgggacctaggcaaatacatcgtctccctgaggttgtcttctcatctgtaaaggacgctgtggtggtggtgtgagaataaatgagacatggcaagtgtctggaacaaagacgctgtgtacaaagtaaacacttaatatactgttatcagtataaaacctttgtgagttttttttttttttccgcatgaaatcttatgtggaaagttgtatgtgaaagaaatgaaagcggagctgcgttgatggtgggcccagaagctttggcctttcagtcccaaagtttccagtaatagaatccgcgcttcctctaaacttgcacagaagtctctccttgaacttcttcatctttattttgatgttcaactttctgcagaagcctggggcccagtaaaccaataagcagacttccaattggggctgtgatgaggatggacaaaaatgccactgtcaacacatccattccatagtcttctaattgtttctctccatgtgaccttgctgtgtccaaagccacagatcctattgcagcctgaactgtggcctttggaagccatgcaaaagaaataaatatcttttcttttaagttaaaaccagcaaaacacaccatcagaaatgtagtcaaaattcgtatcaatactgcaatgcctacggtggcaacacaaaggcctacagtttctggtctgagagatgcaatagatacctctgctccaattagtccaaaaagaaggggctgaaaaatgtcccaggcaactgcaattatcttttcaacctctgccttttcgctggtccatcccatgcctgcaaggaaagccatgaccaacgtgcacagtcctcctgatccagggaaaccaaaatgcacactgctgaacacagctagcacagacaaccccaacacaaggaatgttctcttacacacaagtttgtcctggtcacggcttggaaagtactgaatgaaaaatccaagaacagatccagttgccacaccaattaccacctccaaaactcctctgaggacattaaagacagtagagcctgtggaaaaggctatgcccaagcatgtgttgaagccagtgatggccagaatgtcatcgaagctgccagctgccatgagcaaggttgggacacccttctcaacaccatagcctcctccctgcaaaaggagcattgaaggcaccacaacagctggagatacagcacctaaaacaaaacccagtataaatccccattgccatggtaaacccagcaggtaatgggcaagaagagcagatgtgcacgcctccacaatacagggacccatggacagtcttacacaaacgccctttaacttcttcagggcctttgaatccagaccaaggccagcacgaaccagaatgatagacagggctatgcttctcaaagaggaagaccacttgtgcttgatctgcacattatcgttgatgactgggatatttctgatgagaaaccctgcaagcagcatgccatttgttatgaccctgtccagtaaaccatgtggagggcaagccagcatttgtctcagtctttgtacgtgatttgcttcagttggtgtttcttgtagctttttttcactgcttttcaaaagaatacttccttctgttggttcatttgcatctatacctttgagcttcataactgtctcctcctgtgcttcttgatgcatggagggcgtgtaattcattcctgtggatggttctgaatcttcatatgtaattcttttatcttcatcccccattatttataattaagaagatgacacagggaagaggaacgagatctggcagtctccggcgaagtcgaccaggctccgtctgaacgattaggaaaggggctgtgggggaggcggcggagcccggtctagccaccgcgctctggggttcccgattcgcgcatcttcccaggctgagccgggaggctgcgttgactgcagataaacggtctcagggcgcggcaccgcgtgtagtcggccccgcctttcgcacgaacccgctgggcgacaccgcgcagggaggtccgacccgtcggcgccggtacaggctccggagtaagcatgggttggtccggggcccgcagcggcagccccgtgtgccctccgccgggtttcaggtccggcggcgcgggtgcagagccgcgtgcgatgcctggtgcgcgtggcttcccccggaaaggtggcgccaggccgaccatgggcccacgtcccggggcctcggagcggcaccgcgcggtctttcagctgcttatcctccctgggcgggtccgcaggcttctggggccaggaccagcgagctcccgggaaagcttcccggaaagcttacccagagagcgcggacccaggcgccgagtcttcccggagat

SEQ ID NO: 19554 - RNA, 9408 nt, Homo sapiens
  source 1..9408: mol_type = other RNA
ttgggctgggctgggttgggagcgcctggagtctggagcggggccgacgccgtggtcaccacctgctgctgaatgagtttctgctgaaccacctgggcagtcgcggtcactgcagggatcatctgcacctgctgcccggccgccgtcgcctgcgtgagcgccacagtctgtggagaagcctgctgggaagcagaggcaacttgctggatgctggccacgggtgtttgctgttgaacaacttgaggaagttttgcaacctggatctgggtctgcacttgctgggccccggccagtttctgggcctgggagatgggtgtggtaagaaactgggtcttaagggccggctgcgcggcgtaggcaaccttctgctgcgcgccaggggtggtgatctgctgtgcggtgatcttctgctggacggctgccgggccctgtgcagcctggggctggatggccttctgctgctggacggcctgctgcttcagcttcagcagctgctgcatgtgcacgggctgggccaccacggtctgtcctgctgccttctgtggctgaccgatcgccacgctgatccccgcgacgttcatgggcagggtggtgactcccggtgaggagaccacagctgccgggacggacaccaccggaggcttcgccaaggccacctgggctggctggggtgcctgggtctgcatctgcccttgcgcctgcagctgagaagtgggaacccgggtgagccgggccacctggaggttggccacggtggtgcccgtcagcagggcaccaggccttggggccgtgaccgtcgtgagctgggggctctgctgctgcggcggctgcgaggtctgcacttgcacttgggctgttggctgcgggggcgcagactgggcctgtggcggtgggggctgcgggggcatctgcagtttctgcttctgcattttgatgaggtgttccggcgtcagcttgcccacagctttgatctgtgctggggactgggcctggccctggatctgtggaacttgcacctgagaggtcgtcgtcgtctgttgctgctgctgctgttgctgctgctgctgctgctgctgctgctgctgctgctgctgctgttgttgctgctgctgctgctgctgcctgagaagctggaaatgtgcaggtgtgatggtttttccagggagctgaactcctgtggcttgggacacttggggcaccaaagaccgtgccggggtctgcactggggtcaggttggtagtgaccacggccgaggctgtcacagaagtgaccgctcgaacaccctgagtcgttgccatggacaccaggtcaggggtcgccgtggctggggagccgactgcccgtggcgggggctgggtgtgcaccacctgggcgggagcagagcctcccggcgtagtcaaggccccaggagccactggcgacgccaggcgcttgttgatggactggaaggtggcagctgggacccctgcgatggtgttcacgatcacatttccactcacggcaccagtgggcatgctcgtcccagtaactgatgttttaatggttcctgccagtacggctgcactgccccccgtcgtgattgcgggctgcgccttcgctggggcctgcacaggctgtggctgggtctggggctgtggctggggttggggctggacagctggtggccctgctggcggctggctgcccgctgcctgtggttgtggcagcggtggcggtggctgctgcgggggtggtgggggctgcggctggggcgggggtggctgggccacggccggctgctgtgccttctgctgatcagccagagcctttttctcttttgcgattcgctctgcacggagagatgccacctggatgggaggcagcggcttgtcatagttgattccactttctgccaacacagacgcgtgcttggggttcttctgaaagggattcatgccaagcagaggtttgattgggggactcctcttgccagcagtcattttcattaagtcaaagtggctcgtgtacagctgggtgtgtgtggcattctcatcctgggcatagatctggctcgtacggagaggacggttgtttttactcttcccctcctctcgtggaatgatgacattctcgtagcgattccggcactgtttggaagagcggtagattcggctacaggagttaacaacgtcactgacaagatcccaattaggtgtgtgagcaggtgacacgattgtgaggttcaaaggcagctccagtaactgctttacagcctgcagcagcgcccagtcctcactgatgagccactcggggttgtcttgaccaggctcagctgtgggtttggcaaaagttggcaggggcttggcgaatggcacctgctgcttcagcagaatattcttcttctgctccttgccctctctgcgaattttcagaagtcctggtgttgcgcggtcaaacagggaccgaggagggacgaccgcctccccgtgacgctgcttcttcttcctgcctgcagctgaggggtctgttttgtgtcgcttccgctccttcctcacgtacacagggggcagcttagcctctgggatgggagtggcttcatacatgagacacatgaccgagtcgaggtagatgtcgctgtcgtcctgcggcggggtgggtggggtccagagcggcatgacttctgtctgcccatcgacatcttcgtagacatactccatgctgtaggcatcctctcgcgtgtaggtcaggagctccgcctcctcctgctccagccgcagccgggcctccctctcctgcagggtcttcaggttccagaactcccatgccctcactgcagtcatcactgcgtcctcactgtttctctccttttcttgctcaatagaagtatggaataattccaggtaatttaaagcatatttttcaattggtgtaagctgctccatgaagtcagctagctcctctaattgggatggttcttcatcacacggcatgttctcagagtctgatgacagagcatcagtgtgtggtcccagcaccccctcctgtgcggacttctgggcatcctcctccagatactcaatactcttgagggcctctatgaaaggtcttgcaattttgggtgcaatggtttccgtgacagaaggttcctgagaaagcaccacaaactcctcagctttgaccgggaagccagcatcatccatgggagaataaacttcaaacagctcctggatggttcgctgagttaagaaagccatggagtagtcatttccctgagcagccacttctcggatcagatctttagttccatttttcaacaatttctcttcaatggaattgccactcacaagcctgtatatgtggatgtctttgcatctcccgatcctatcgcaccactcctgagctttggcatccatcactggattcaggtcattgtcataaaacacgacggtgtccgcctctacaaggtttatacctgtggtacggctgtgagtggagagaatggcacaaaaaatccgcctgtctctgttgaaactcctcatcagttcctgccgttgctcactgctggcattttcatcgattcttacataggtgaggtaatggaagttcaagaacatctctaaaatgtccaacataagaatcatctgtgataaaatcagcacccgacgtccttcagatttcaatttctgaagcaagatagctaaagcttccaacttccctgagtcgaactgcaccagcctcagctcagggaactgcagcaggcgtggagccgtggtctgccgcagctgctggaagtacggcgcagcgtgctctctcaggccctgcctcaagatcctcattctgtggctgtacaggggtggcggccgcggcacccgtagggacgggggtgctgccaccaccggaggaatcacaaaggccaccctgtcaataacatcctgcagagactctccacaccgacaaagcgtcaacatcagctcacttggactttctgaggatgaagtgtaactgtgcgctggcccggcctccttcccacgacggccatccagggacccacgccactgtacccttccatggctaggcagggcacaaatccttagcaagtctctgccatagactggagcttgagaacagcgccgctcgttgactaaataaatctgatccaggcgctctttcaagagtctggtcttttcctcctgggtcggccctccaatgggagaagctggtttggaggccgttccgggttctcctacagccaaggcattcaccgccacgcggcccggaacgccaacttgtggggtcaagggtgcagggctgggaccgccggccgggggcttgcttcccagggcgccgtgcacagcgcccgcctgagacacggtctgcatcaccacagggccaggggctcgaaggtagggctgcccgggggcggacacgatctggaggacgctgccttgcagctgcagcggctggcccgctgtgagctgccggagctggctgtgtgacagggtgaacttgctgccctggaactgcagtgtcaccggcgtctctggctgagccacgcggctctgtggtcctgtgatggatgccagctgagctattttcactacctctccactgggcaagcgggcctgggcctgcgaggggagcaccagcctctgaggcagcgcgctctgcccggccgcgtgcgagggggcctggggctggggcgggggctggcctggggtggaggcctgtgctgtggtctgggcccgcagtttcgcaggatgggccgggctagcggctgtgctggaggccgaggcgggctggtgtcgtggagcactggcggaagcctgagaggtctgaaacggggctgctgctgcttttgcctccggattggcagagaacgtggcgatgggcggccgtcctcgaagcgggccctgtggagcagcagaggccgtggtgggggctgccgtccggggcgggtgagtgctggggaaagccacggtgcgaccctcgggcttctggccatactgcacaggctgaaacaacctgctggccttcagctttgctgctgctggtcgggctgctggggctgctgaagtggagatttcctccatgagtttccgcggtatctttttcttagacagcaactctgcctcgtgacgagtgattttattttctaagccgatgagatcaaacatagaaagatctgcttccttccagaaatctctctccagtgccttcaggattagagatgcggacggatactccagtggccccgccacgtaggaagagcctgggtgccggggctcgacgagcccagggtggttgcagatgcgctgcagccgcacaaggatgctcaggacgttgacaaagtgcccgctcttcaaggcctcctgagtgccaggttgcaggataacgtcctcgtataaggctttttgtcggttagaaaggcgacacttcaaaacatgctcatatttctttgttagttgcttttccacatctctcttagttctcctcaaaataaatggctgtgtcaccctgtgtaaccttatgaccactttatggtagtaatcctggctctcttcactgggggccctcagaggggagctcaggtagggcctggagatccctgggaccaggaagtgcaccatggtccagagctccaggaaggtattgtgcagcggcgagtcgatcagaagcagacgttgttggctctgcagggtgaaaaccgcttcccagtgcctctcggtcatgcccttcacgcgctgcatctcatcaatgaccaggcacttccagcgcactcgtgtgaaggcggtgaggccccggaagaactgagtgtaggacgtgatgcagacgtggaagctgttgggttcggcccactcctgtctctttgctttgagttctctgtggctgccaatatatgagaggattttgagtccgggacaccaacgtttcaattcaagctcccacttgagtatgttacaacttctcacaacaacaagatgggggccccaattaccttcgttacaagctaggtgggcaaaaaaagcaatgatctgcactgttttacccagcccagcttcatctgccaatatgccattgagattcttcctgtaaagtttggccagccagtccaggccaatcttctgataatctctgagagccccatacaacaaagatggagcattaaacttgaccgaggttgtgacccgagcactgcccttcggcaggatggcttcagccaccgcagtgacgtccgcaatgtccttggcgtttggcttcccgatattcatcctctcggcagctttgaactgatccatgatgaaaagcgagtcgatgagaaccaagtccttgcgactctccctgtcgcctggacagtcatctgcatcttcctctccgcttgtgtcctccccatcaggcttcggccggggccactgagaactcggcaggaaggcgccttcgtacagcttcatcaggtccaggaggggcagctcagcttccttggctaaattagaaagttctgtttggtggtccacaacgccttcatttgcttcctcctcttcaattgtttcctcttcatcgtccacttcgtcatcagtcaaagatatgctagcttttctttttcttccagacattcctgaatccagagaactttcctgtaatgcgtcaaatcctttaggtctcaattctttccctctcctggaaactttctgtaaatttaaggccttcttccttttttcttctaattctactcgtagttttatttccacaacctgttcaatattcgaccaaaagcactctatctcccgggccgtggaggcggctatccgcctcagtctgctctgctcttccttcttccccctttcttcacggagctgcttctcctcgtgatggcgcaccacagttctaacgagcttcttcgcagcagccaccttccacctcctctcctgggcaaagtctgtggccatccactgcatctcctccagcagatagtcccagtgggacttggggcgtggggcctcctgcagctttggcagacgcctctgggaccacagacctgctttcctcagctccgcaatgcgctgatgcacctggttctccagagttatttgttctgtcagcgtatcctgagaactgtcttgggacgaggtggcattctgagcaggactctgtggtttggtgggggcagatgccaccacccctggggtccgggaagtgactggagatagtgccttattggtggctgaggaaggtctatttactggagaggatcgagcaggggagggtcctgggccggagccactcacaggcgcgagggacgaggtagaagaggtgggcagaggccgtgggcagggcggggcagggtccacagggagccttgtcgatgctaccatctgtggcagggaggaaagctgagaggcctgcacctgcacctttccaggtgtgggaacgtggagggccagctgtgcaggctgcgagggagggatggggagttggctgctgggcggtgcagggatgggaacattgggctgctgagtcttcaccgggatttggagctgtgtctgggcctctaccacttgcggctgctgtgcaaactgcagcgcagaggagagggctgcagtgggaacaccggctgggggcagcctcccgggcagctgcggcagtggggtgtgcaagctggcagcgttctgcacgggaggccccgtggaggggtcatactgctgctgactctgcctctgtccagcgagctgcgcggcctgcggcgtggggggcattcctccttgtgcggtcggcattagttgctggagaggaacgcctgcgtccgcccctgggtgctggaaaactaccccttggtgacccacttcaaggcgaggcctcttagactgctctgccatacctgtggagggcatcgcctgctgcctcttaaacaggtccgtctctactgtgcttccggcccctgctaccaggctccctgcgagggcttgctgctcgtcattgataacctcagatttttcttcctcctcttcctcctcctcctcctcttcttcaatgtccaaatcattctgcctaagatatgcttgtaatggggcataatgtttcttcttgaaagctaagaaatccatcatgttcccttgaaagtgttgcaagaaaaacagttcaatcaaatactccttgaagacctccttcagagcctgcatctcctggtaatgatagtccaggcactgcttcctcatctgtgccatctccggagaggctgggggaatctcctctaacttcttgggaaccttcttcattcccgtgttccccacagacgtgagtgggaggctggaaaggcctgggggcacggcagtcctggaagggctggtgggcgggggtggggacgtcatcccaaaccccgctgcgcccccagccccggggagcagcacgccgggtgtcctctcgaagcccaggggccggggcagcggcggcccctgcagcacctgctgctgctgaaccagctggccctggatgatgctgctgatctgcggtggcaagttagccgtggtgatgtggcttgggctggccaggggctgcaggccggccccacccgcggctgcagggctctggggtcccaggtggtggatggtgccccctgactgtgtgtggggctgggagggtctccgctctcggactgtgatgggcgtacccgggtgctggagctgaacctgggctccctgggcgatctgggtgagccctgacccatcctgaaacacaaagtgtccaccactggaggggctcaagctgatctgcctcaccagcacgctggcatccacgaagccccctgtagggctgctgctgcagaggcccagcccagggccaggggcacctgcacgcacattctgcaaggcctgccccggccccggactgggctgcgtgggactctgggtctggacctgctgggacaagggggacgtgacctgaatgtatgatggagacccatgctcaaaccgccgaggctgagcgctgaactggaagcctggagaggtggggctggggagcggcagtggggccagtgtgatctgctggtttcccccgacgacagggcccacgctctgcagggtgatgttcacgttctgcccggttgcagggctcctattcatcagctgctgtatttgataactgggagactggggtgccgacgggcttgctgagggagcgaagggagctgcgggggacgggggtgggttggggtgggccggctgctcctcaccctcgctgccagggcaggccctggacctctgcagctgatgctggacgttctgggggccagtgccatggtgcatgatcacctcccttctgtatccaatgtgtcgttctccctgggcctcagggctgcgctccggccgcgtcaggagggcgggaggatggaagccgcgccgcagccgctcagtgcatccggggccccggcgggag

SEQ ID NO: 19555 - RNA, 2944 nt, Homo sapiens
  source 1..2944: mol_type = other RNA
ttgggctgggctgggttgggccgggttgggctgggttgggctaggccgtgctgctgctggagcaaggcgtgctctgcgtgctgccgatgctgtgggcagcactgctgttttccgaggctggcggggaggtggggacttgctgccttcctgctgtctcccctgtgtgagaatagatgtaccacaaggcccccgtcaggagtgctccgatcacaaaggctgcaaacgcaatgcccatcacggttagggtgtccagaccatggaaaattggtggagaaattggatttggttccttcatgcttggacctttttctttagattctgcttcatggtggatcacagcaaggggcttagtgaacgtcttcttattctgcatcatggcccagattatcgaggcgtccagcgaggtgcaggcttcgtcaggaggcacacacttaggcaacttctgggggtgcttctccatcttcgtacacagcgtcagctcacactgtagaaagagcagtgaggtgttgaagacaggcttgaagacaaagctgaatcgcttcttatccatgtcagcttgcgggataggaaagtgcactctcttgggactgtagaatttcacagattcatctttaggacaaatattctcaataatggtgtaatgagacatcctatcagggttcgaatatggagagataaagcacgtttggatggcaaatcccagttcttgttcagccttagtaacagatacctcaacataaacgtgtccattctctggcacagagaagacgccctgggagggcaccaaaaagaggtcagtgttgtatagctccatgttgaaggtgatgtttccgtggggctgttcctggaagctgctggggttcctcacctgctgaaggctgcaattaaacaccacgatttcaggtcgggtgaacagggaagcatctccttcatccatatctcccggaaatccattatcacctgactccagatcttcataaccatctggccaaccactactgtccccaagggctggaacctgtatcacaatggagttatagtagaccacaccatcaagggctgaccaccggggccgagtaccgcagccattcagaggagactccaaaacaaagtgtgtgccattcatcttggccttgcaggtaggatccaacagggtgacgtccatccccgagtagccactggcctgaaaagaatctttttctacagccacgatcatcttctcattgtcacatttgacagacagggcaatatccacgctcccttgcacctcttctggctctctgagaccaggaaacagttgtatgctgggaatgacagggtcctttggccgagggagcccatcttctccctcttcattccagactctcctggaaatatctgggaaaggaaacggaaggcctccattttggccttcccctccccggatgggcgggttctgcagggcaggcagggcaccagggtccagcaggatccgtagctcaggaggaatagtgtggacttcctcatctcccatctcctcattattttcaagccgaagatgaaatctattagccacaggagccattgtgtatgaagttattggactatagccattgtccaaagcccacttcaccagattcccttgggttgaaggaatgtcatctcttattgatttggtcattgtcatagatctttcactctcttttccaaagccaatactgttaggagcaataattttcaggcttcccttaacatcaaaagatttgatcacccagttgacagactttttgcacttcaagatcaggatgagatttttgaccacttcaagatcctcttgagaaggtcttatatcaattgttatatccacctggaaagcactgtaggggttagagttgggggtgattagctcgatgatgtgtacttcctcattctggggctggctggacatcacacacccttctgctgctttgggttgaaggtactcagcaaggtaattgagtgagagaaaattcttccctatgttgcactttggagggaacacttgatcttcccccactttaatataaatgtttcttgctatcttgagttcggtgaatgaagtaactgctccatactcttttcgggcccaatttaacagatgttcatttccatgggggaagttcctttcttctgtttctgctgtcaaggagaagtttgctgatgaaaactggaccacagaaccctcagacaccaaaaacagtctggagaccccagtggcaagtctctctgtcttcagatgccacaccagggggtgtggggagttgagcaggaacacaacagacttgtggtggatgtggactgaggagatgggattcaggtgaagtgtgacctctctctgtagctggccaggcccctggcctgcagtgcggagattcaggacatgcacctcctgtggcagcccagttgtgcctctgctggcacagcctgacaaaacagtgaagctctccatcaaggcctggacaggatgggaggcactgacaggtgacagttcacacagtgcaccaggctctggacctgcagtggctaaacaggagctcatcagggcaaagatggcaatcacataatgggaagtcatttttatttctccaacagtgcgtctcgtccagtcacttcagcctgctcagagcacagacaatctttgcaaatcagaagtagtcttaaagtccctccttgcaattttcaaactgccaccaaagatctacacacaaggattctctgccgtccctctgatgttgtgtccttgctttgactcaatgttgccagagctctgcttccttgtgtgtgctggcatccatctgcagatagcttcttcctgcacagcctgatgttaagaccatgcgcagcttcaggctcatgcggttctttcagtttgaaggcccaaggaaaaaaagctcctttctttcttagtagctacaaatcttaaaga

SEQ ID NO: 19556 - RNA, 2980 nt, Homo sapiens
  source 1..2980: mol_type = other RNA
ttgggctgggctgggttgggccgggttgggctgggttgggctaggccgtgctgctgctggagcaaggcgtgctctgcgtgctgccgatgctgtgggcagcactgctgttttccgaggctggcggggaggtggggacttgctgccttcctgctgtctcccctgtgtgagaatagatgtaccacaaggcccccgtcaggagtgctccgatcacaaaggctgcaaacgcaatgcccatcacggttagggtgtccagaccatggaaaattggtggagaaattggatttggttccttcatgcttggacctttttctttagattctgcttcatggtggatcacagcaaggggcttagtgaacgtcttcttattctgcatcatggcccagattatcgaggcgtccagcgaggtgcaggcttcgtcaggaggcacacacttaggcaacttctgggggtgcttctccatcttcgtacacagcgtcagctcacactgtagaaagagcagtgaggtgttgaagacaggcttgaagacaaagctgaatcgcttcttatccatgtcagcttgcgggataggaaagtgcactctcttgggactgtagaatttcacagattcatctttaggacaaatattctcaataatggtgtaatgagacatcctatcagggttcgaatatggagagataaagcacgtttggatggcaaatcccagttcttgttcagccttagtaacagatacctcaacataaacgtgtccattctctggcacagagaagacgccctgggagggcaccaaaaagaggtcagtgttgtatagctccatgttgaaggtgatgtttccgtggggctgttcctggaagctgctggggttcctcacctgctgaaggctgcaattaaacaccacgatttcaggtcgggtgaacagggaagcatctccttcatccatatctcccggaaatccattatcacctgactccagatcttcataaccatctggccaaccactactgtccccaagggctggaacctgtatcacaatggagttatagtagaccacaccatcaagggctgaccaccggggccgagtaccgcagccattcagaggagactccaaaacaaagtgtgtgccattcatcttggccttgcaggtaggatccaacagggtgacgtccatccccgagtagccactggcctgaaaagaatctttttctacagccacgatcatcttctcattgtcacatttgacagacagggcaatatccacgctcccttgcacctcttctggctctctgagaccaggaaacagttgtatgctgggaatgacagggtcctttggccgagggagcccatcttctccctcttcattccagactctcctggaaatatctgggaaaggaaacggaaggcctccattttggccttcccctccccggatgggcgggttctgcagggcaggcagggcaccagggtccagcaggatccgtagctcaggaggaatagtgtggacttcctcatctcccatctcctcattattttcaagccgaagatgaaatctattagccacaggagccattgtgtatgaagttattggactatagccattgtccaaagcccacttcaccagattcccttgggttgaaggaatgtcatctcttattgatttggtcattgtcatagatctttcactctcttttccaaagccaatactgttaggagcaataattttcaggcttcccttaacatcaaaagatttgatcacccagttgacagactttttgcacttcaagatcaggatgagatttttgaccacttcaagatcctcttgagaaggtcttatatcaattgttatatccacctggaaagcactgtaggggttagagttgggggtgattagctcgatgatgtgtacttcctcattctggggctggctggacatcacacacccttctgctgctttgggttgaaggtactcagcaaggtaattgagtgagagaaaattcttccctatgttgcactttggagggaacacttgatcttcccccactttaatataaatgtttcttgctatcttgagttcggtgaatgaagtaactgctccatactcttttcgggcccaatttaacagatgttcatttccatgggggaagttcctttcttctgtttctgctgtcaaggagaagtttgctgatgaaaactggaccacagaaccctcagacaccaaaaacagtctggagaccccagtggcaagtctctctgtcttcagatgccacaccagggggtgtggggagttgagcaggaacacaacagacttgtggtggatgtggactgaggagatgggattcaggtgaagtgtgacctctctctgtagctggccaggcccctggcctgcagtgcggagattcaggacatgcacctcctgtggcagcccagttgtgcctctgctggcacagcctgacaaaacagtgaagctctccatcaaggcctggacaggatgggaggcactgacaggtgacagttcacacagtgcaccaggctctggacctgcagtggctaaacaggagctcatcagggcaaagatggcaatcacataatgggaagtcatttttatttctccaacagtgcgtctcgtccagtcacttcagcctgctcagagcacagacaatctttgcaaatcagaagtagtcttaaagtccctccttgcaattttcaaactgcctcggaggcggtgtgtccagcggagatccacccgcagcaagttggaggaaagcggcggcaagtttccccgcccagcgctcggcggcggcgagctccggcagctgctgcgccgcggcaaaactacgccatccggacccgctggggactctcacctcctgcagggagctccgggaatcgcgcagggaaagtggccggggcgcgagagccgccgactgccctccttcactcgctgggaagaggaaagtgccgctcggcgtccccgaaaccctcgatt

SEQ ID NO: 19557 - RNA, 2830 nt, Homo sapiens
  source 1..2830: mol_type = other RNA
ttgggctgggctgggttgggccgggttgggctgggttgggctaggccgtgctgctgctggagcaaggcgtgctctgcgtgctgccgatgctgtgggcagcactgctgttttccgaggctggcggggaggtggggacttgctgccttcctgctgtctcccctgtgtgagaatagatgtaccacaaggcccccgtcaggagtgctccgatcacaaaggctgcaaacgcaatgcccatcacggttagggtgtccagaccatggaaaattggtggagaaattggatttggttccttcatgcttggacctttttctttagattctgcttcatggtggatcacagcaaggggcttagtgaacgtcttcttattctgcatcatggcccagattatcgaggcgtccagcgaggtgcaggcttcgtcaggaggcacacacttaggcaacttctgggggtgcttctccatcttcgtacacagcgtcagctcacactgtagaaagagcagtgaggtgttgaagacaggcttgaagacaaagctgaatcgcttcttatccatgtcagcttgcgggataggaaagtgcactctcttgggactgtagaatttcacagattcatctttaggacaaatattctcaataatggtgtaatgagacatcctatcagggttcgaatatggagagataaagcacgtttggatggcaaatcccagttcttgttcagccttagtaacagatacctcaacataaacgtgtccattctctggcacagagaagacgccctgggagggcaccaaaaagaggtcagtgttgtatagctccatgttgaaggtgatgtttccgtggggctgttcctggaagctgctggggttcctcacctgctgaaggctgcaattaaacaccacgatttcaggtcgggtgaacagggaagcatctccttcatccatatctcccggaaatccattatcacctgactccagatcttcataaccatctggccaaccactactgtccccaagggctggaacctgtatcacaatggagttatagtagaccacaccatcaagggctgaccaccggggccgagtaccgcagccattcagaggagactccaaaacaaagtgtgtgccattcatcttggccttgcaggtaggatccaacagggtgacgtccatccccgagtagccactggcctgaaaagaatctttttctacagccacgatcatcttctcattgtcacatttgacagacagggcaatatccacgctcccttgcacctcttctggctctctgagaccaggaaacagttgtatgctgggaatgacagggtcctttggccgagggagcccatcttctccctcttcattccagactctcctggaaatatctgggaaaggaaacggaaggcctccattttggccttcccctccccggatgggcgggttctgcagggcaggcagggcaccagggtccagcaggatccgtagctcaggaggaatagtgtggacttcctcatctcccatctcctctgcattattttcaagccgaagatgaaatctattagccacaggagccattgtgtatgaagttattggactatagccattgtccaaagcccacttcaccagattcccttgggttgaaggaatgtcatctcttattgatttggtcattgtcatagatctttcactctcttttccaaagccaatactgttaggagcaataattttcaggcttcccttaacatcaaaagatttgatcacccagttgacagactttttgcacttcaagatcaggatgagatttttgaccacttcaagatcctcttgagaaggtcttatatcaattgttatatccacctggaaagcactgtaggggttagagttgggggtgattagctcgatgatgtgtacttcctcattctggggctggctggacatcacacacccttctgctgctttgggttgaaggtactcagcaaggtaattgagtgagagaaaattcttccctatgttgcactttggagggaacacttgatcttcccccactttaatataaatgtttcttgctatcttgagttcggtgaatgaagtaactgctccatactcttttcgggcccaatttaacagatgttcatttccatgggggaagttcctttcttctgtttctgctgtcaaggagaagtttgctgatgaaaactggaccacagaaccctcagacaccaaaaacagtctggagaccccagtggcaagtctctctgtcttcagatgccacaccagggggtgtggggagttgagcaggaacacaacagacttgtggtggatgtggactgaggagatgggattcaggtgaagtgtgacctctctctgtagctggccaggcccctggcctgcagtgcggagattcaggacatgcacctcctgtggcagcccagttgtgcctctgctggcacagcctgacaaaacagtgaagctctccatcaaggcctggacaggatgggaggcactgacaggtgacagttcacacagtgcaccaggctctggacctgcagtggctaaacaggagctcatcagggcaaagatggcaatcacataatgggaagtcatttttatttctccaacagtgcgtctcgtccagtcacttcagcctgctcagagcacagacaatctttgcaaatcagaagtagtcttaaagtccctccttgcaattttcaaactgcctcctgcagggagctccgggaatcgcgcagggaaagtggccggggcgcgagagccgccgactgccctccttcactcgctgggaagaggaaagtgccgctcggcgtccccgaaaccctcgat

SEQ ID NO: 19558 - RNA, 2983 nt, Homo sapiens
  source 1..2983: mol_type = other RNA
ttgggctgggctgggttgggccgggttgggctgggttgggctaggccgtgctgctgctggagcaaggcgtgctctgcgtgctgccgatgctgtgggcagcactgctgttttccgaggctggcggggaggtggggacttgctgccttcctgctgtctcccctgtgtgagaatagatgtaccacaaggcccccgtcaggagtgctccgatcacaaaggctgcaaacgcaatgcccatcacggttagggtgtccagaccatggaaaattggtggagaaattggatttggttccttcatgcttggacctttttctttagattctgcttcatggtggatcacagcaaggggcttagtgaacgtcttcttattctgcatcatggcccagattatcgaggcgtccagcgaggtgcaggcttcgtcaggaggcacacacttaggcaacttctgggggtgcttctccatcttcgtacacagcgtcagctcacactgtagaaagagcagtgaggtgttgaagacaggcttgaagacaaagctgaatcgcttcttatccatgtcagcttgcgggataggaaagtgcactctcttgggactgtagaatttcacagattcatctttaggacaaatattctcaataatggtgtaatgagacatcctatcagggttcgaatatggagagataaagcacgtttggatggcaaatcccagttcttgttcagccttagtaacagatacctcaacataaacgtgtccattctctggcacagagaagacgccctgggagggcaccaaaaagaggtcagtgttgtatagctccatgttgaaggtgatgtttccgtggggctgttcctggaagctgctggggttcctcacctgctgaaggctgcaattaaacaccacgatttcaggtcgggtgaacagggaagcatctccttcatccatatctcccggaaatccattatcacctgactccagatcttcataaccatctggccaaccactactgtccccaagggctggaacctgtatcacaatggagttatagtagaccacaccatcaagggctgaccaccggggccgagtaccgcagccattcagaggagactccaaaacaaagtgtgtgccattcatcttggccttgcaggtaggatccaacagggtgacgtccatccccgagtagccactggcctgaaaagaatctttttctacagccacgatcatcttctcattgtcacatttgacagacagggcaatatccacgctcccttgcacctcttctggctctctgagaccaggaaacagttgtatgctgggaatgacagggtcctttggccgagggagcccatcttctccctcttcattccagactctcctggaaatatctgggaaaggaaacggaaggcctccattttggccttcccctccccggatgggcgggttctgcagggcaggcagggcaccagggtccagcaggatccgtagctcaggaggaatagtgtggacttcctcatctcccatctcctctgcattattttcaagccgaagatgaaatctattagccacaggagccattgtgtatgaagttattggactatagccattgtccaaagcccacttcaccagattcccttgggttgaaggaatgtcatctcttattgatttggtcattgtcatagatctttcactctcttttccaaagccaatactgttaggagcaataattttcaggcttcccttaacatcaaaagatttgatcacccagttgacagactttttgcacttcaagatcaggatgagatttttgaccacttcaagatcctcttgagaaggtcttatatcaattgttatatccacctggaaagcactgtaggggttagagttgggggtgattagctcgatgatgtgtacttcctcattctggggctggctggacatcacacacccttctgctgctttgggttgaaggtactcagcaaggtaattgagtgagagaaaattcttccctatgttgcactttggagggaacacttgatcttcccccactttaatataaatgtttcttgctatcttgagttcggtgaatgaagtaactgctccatactcttttcgggcccaatttaacagatgttcatttccatgggggaagttcctttcttctgtttctgctgtcaaggagaagtttgctgatgaaaactggaccacagaaccctcagacaccaaaaacagtctggagaccccagtggcaagtctctctgtcttcagatgccacaccagggggtgtggggagttgagcaggaacacaacagacttgtggtggatgtggactgaggagatgggattcaggtgaagtgtgacctctctctgtagctggccaggcccctggcctgcagtgcggagattcaggacatgcacctcctgtggcagcccagttgtgcctctgctggcacagcctgacaaaacagtgaagctctccatcaaggcctggacaggatgggaggcactgacaggtgacagttcacacagtgcaccaggctctggacctgcagtggctaaacaggagctcatcagggcaaagatggcaatcacataatgggaagtcatttttatttctccaacagtgcgtctcgtccagtcacttcagcctgctcagagcacagacaatctttgcaaatcagaagtagtcttaaagtccctccttgcaattttcaaactgcctcggaggcggtgtgtccagcggagatccacccgcagcaagttggaggaaagcggcggcaagtttccccgcccagcgctcggcggcggcgagctccggcagctgctgcgccgcggcaaaactacgccatccggacccgctggggactctcacctcctgcagggagctccgggaatcgcgcagggaaagtggccggggcgcgagagccgccgactgccctccttcactcgctgggaagaggaaagtgccgctcggcgtccccgaaaccctcgatt

SEQ ID NO: 19559 - RNA, 3080 nt, Homo sapiens
  source 1..3080: mol_type = other RNA
ttgggctgggctgggttgggccgggttgggctgggttgggctaggccgtgctgctgctggagcaaggcgtgctctgcgtgctgccgatgctgtgggcagcactgctgttttccgaggctggcggggaggtggggacttgctgccttcctgctgtctcccctgtgtgagaatagatgtaccacaaggcccccgtcaggagtgctccgatcacaaaggctgcaaacgcaatgcccatcacggttagggtgtccagaccatggaaaattggtggagaaattggatttggttccttcatgcttggacctttttctttagattctgcttcatggtggatcacagcaaggggcttagtgaacgtcttcttattctgcatcatggcccagattatcgaggcgtccagcgaggtgcaggcttcgtcaggaggcacacacttaggcaacttctgggggtgcttctccatcttcgtacacagcgtcagctcacactgtagaaagagcagtgaggtgttgaagacaggcttgaagacaaagctgaatcgcttcttatccatgtcagcttgcgggataggaaagtgcactctcttgggactgtagaatttcacagattcatctttaggacaaatattctcaataatggtgtaatgagacatcctatcagggttcgaatatggagagataaagcacgtttggatggcaaatcccagttcttgttcagccttagtaacagatacctcaacataaacgtgtccattctctggcacagagaagacgccctgggagggcaccaaaaagaggtcagtgttgtatagctccatgttgaaggtgatgtttccgtggggctgttcctggaagctgctggggttcctcacctgctgaaggctgcaattaaacaccacgatttcaggtcgggtgaacagggaagcatctccttcatccatatctcccggaaatccattatcacctgactccagatcttcataaccatctggccaaccactactgtccccaagggctggaacctgtatcacaatggagttatagtagaccacaccatcaagggctgaccaccggggccgagtaccgcagccattcagaggagactccaaaacaaagtgtgtgccattcatcttggccttgcaggtaggatccaacagggtgacgtccatccccgagtagccactggcctgaaaagaatctttttctacagccacgatcatcttctcattgtcacatttgacagacagggcaatatccacgctcccttgcacctcttctggctctctgagaccaggaaacagttgtatgctgggaatgacagggtcctttggccgagggagcccatcttctccctcttcattccagactctcctggaaatatctgggaaaggaaacggaaggcctccattttggccttcccctccccggatgggcgggttctgcagggcaggcagggcaccagggtccagcaggatccgtagctcaggaggaatagtgtggacttcctcatctcccatctcctctgcattattttcaagccgaagatgaaatctattagccacaggagccattgtgtatgaagttattggactatagccattgtccaaagcccacttcaccagattcccttgggttgaaggaatgtcatctcttattgatttggtcattgtcatagatctttcactctcttttccaaagccaatactgttaggagcaataattttcaggcttcccttaacatcaaaagatttgatcacccagttgacagactttttgcacttcaagatcaggatgagatttttgaccacttcaagatcctcttgagaaggtcttatatcaattgttatatccacctggaaagcactgtaggggttagagttgggggtgattagctcgatgatgtgtacttcctcattctggggctggctggacatcacacacccttctgctgctttgggttgaaggtactcagcaaggtaattgagtgagagaaaattcttccctatgttgcactttggagggaacacttgatcttcccccactttaatataaatgtttcttgctatcttgagttcggtgaatgaagtaactgctccatactcttttcgggcccaatttaacagatgttcatttccatgggggaagttcctttcttctgtttctgctgtcaaggagaagtttgctgatgaaaactggaccacagaaccctcagacaccaaaaacagtctggagaccccagtggcaagtctctctgtcttcagatgccacaccagggggtgtggggagttgagcaggaacacaacagacttgtggtggatgtggactgaggagatgggattcaggtgaagtgtgacctctctctgtagctggccaggcccctggcctgcagtgcggagattcaggacatgcacctcctgtggcagcccagttgtgcctctgctggcacagcctgacaaaacagtgaagctctccatcaaggcctggacaggatgggaggcactgacaggtgacagttcacacagtgcaccaggctctggacctgtaatcctagtactcaggaggctgaggcagaagaatcgcttgaacccgggaggcggaggttgcagtgagccaagatcgcgccattgcactccagcctgcagtggctaaacaggagctcatcagggcaaagatggcaatcacataatgggaagtcatttttatttctccaacagtgcgtctcgtccagtcacttcagcctgctcagagcacagacaatctttgcaaatcagaagtagtcttaaagtccctccttgcaattttcaaactgcctcggaggcggtgtgtccagcggagatccacccgcagcaagttggaggaaagcggcggcaagtttccccgcccagcgctcggcggcggcgagctccggcagctgctgcgccgcggcaaaactacgccatccggacccgctggggactctcacctcctgcagggagctccgggaatcgcgcagggaaagtggccggggcgcgagagccgccgactgccctccttcactcgctgggaagaggaaagtgccgctcggcgtccccgaaaccctcgatt

SEQ ID NO: 19560 - RNA, 2458 nt, Homo sapiens
  source 1..2458: mol_type = other RNA
ttgggctgggctgggttgggctgattggaggaaaggtcttgagacccaactgcatgttacctctgaagaataaatattctaagaaaaagggaaaaccatgaggcaagctgctgcagtcagtcaacgcagctgacaggcctggcatggcccacaacctgaccccatccacacaggaaacagctgtgcgggtctggatagaggagaggtcaagggcttggactggggaccctgagctgccaaggtgtggggactccttgcagtcctggtgcagcaatggcaggaaggccagcaggggccctagttgagcaggttgccctgctcctgggcctgggtcaggctgtccttgcggtgcaggtggtgaacccccatcctcttggggctgcgctgggggcgactggagctggggagtggccaggccctgccctcggtgtgggaagtgcctggcccctcctctgtgcccctgttaatgggcagcaggctctggcgctcttcctcaggactgataggcaggttcagctcttcttcctccctgggaaagccagagtcaggttctgtgggtagcaaaagctcactctcttcgggtcgggcagaaggtgcctggaccacctcatctctgtcagcggggctatgggcaaaatggcgctgcagctcagggagggcatcgcgtccaaaggctgtgcgctgggccacagcagcaggtggtggagtacggtccacaaatgcccgctgccagctgaccagcaggtcctcttcagagctggcagagctagctggggcactgagtgttaggggtgctgggctgggctggtggtggggtgaggcctgggctgaggcaggggtgctgggcactgggctggggcgggcccgctcactcccctcctctaccaggctcagggaaatggcctggcgggtagcgtaagtgcagttgggcagggggctgttgcgggggatccgaaccttatcctcagagaactctattaccctgcggccaggatacagtgggtgtggtggagacggggttgggtaggggttcagcttctcaaaggctggcaggggcagctcttcctccggggagcccctggcagtacccagagagtggcactccccattgggttgtggggtggggctgccaggggccgggggactggctggatcacctgggacaccctcactcatgtccacatgcacaaagacatcctcagccaaggggcgcccggcgctgcctgactgggctgaattgagcagtagagactccggcttctctaacactcgggcaatgactgaggtaggcaccacagcccctggggctaggctgggagcaggacctgggctggcggcctcttgaccactgtgcaaatgtttccgaaccatgtcctgtagctcacagggcagatcggcaaacttgtggtttcggaagtgggacttgttgcacttgaggagctgtacagccaggttgcagtccagccggtaccgctcattgagctcttccagcttgttgatggtgttcttggcatccagcagcttgttggtcagctccacaatctcccagtccagcgtcttcctatccatctcagccttcttgatcagtgtgtgcagcttgtcctccaactcctggttggtccgctgggaagccgtgtagctgttctgcagcctgcggaacttatccttaaatttgtccagctcctcgcggctctggcccagctccagctccaggcagtcctgcccaatttccagctcacgttccagggcctcagtgcgtctggtggcggaggccaggcgccggcgaagctcttcattctcctcctgtaagagcttcatcctttctgcatcagtcaggggttcctcctgctcaagccgggatccaggaatttccaaacgcagctcccgatgctctggtggtgccttacggtagggtttcttagcaggggcggcactagtcattctgggaggtgacggctcctccgccgtctgtttgtcggcagctctctctgttccgctgtccgggagttagccctcggctctccgcatcccacggcccctccacttcctttagccacagctcagggttagtgtcttctccccaaccagccagctctcctggttagtgcagttagcgacagactcatggcagatgccctccaggcactccatataaacagacagcttggtttgtgagcagcccaactccggagcaaaaaagcaaaagtagacacacagcgagaatgaattcaggagtcagtgacagcaggtacccgctctggggttggactggggcaagtcgctatctcttcttctttccaagtaggcactgtaatttcttccagtccctggggcacctgaatcttcagctgaaattggggcagatgctgctaacagctgtggaaaggctgatctaagctttccgccgctgccagctgcgttcaggccgccatcttgccgcggggcaggccgggtagtg

SEQ ID NO: 19561 - RNA, 2327 nt, Homo sapiens
  source 1..2327: mol_type = other RNA
ttgggctgggctgggttgggctgattggaggaaaggtcttgagacccaactgcatgttacctctgaagaataaatattctaagaaaaagggaaaaccatgaggcaagctgctgcagtcagtcaacgcagctgacaggcctggcatggcccacaacctgaccccatccacacaggaaacagctgtgcgggtctggatagaggagaggtcaagggcttggactggggaccctgagctgccaaggtgtggggactccttgcagtcctggtgcagcaatggcaggaaggccagcaggggccctagttgagcaggttgccctgctcctgggcctgggtcaggctgtccttgcggtgcaggtggtgaacccccatcctcttggggctgcgctgggggcgactggagctggggagtggccaggccctgccctcggtgtgggaagtgcctggcccctcctctgtgcccctgttaatgggcagcaggctctggcgctcttcctcaggactgataggcaggttcagctcttcttcctccctgggaaagccagagtcaggttctgtgggtagcaaaagctcactctcttcgggtcgggcagaaggtgcctggaccacctcatctctgtcagcggggctatgggcaaaatggcgctgcagctcagggagggcatcgcgtccaaaggctgtgcgctgggccacagcagcaggtggtggagtacggtccacaaatgcccgctgccagctgaccagcaggtcctcttcagagctggcagagctagctggggcactgagtgttaggggtgctgggctgggctggtggtggggtgaggcctgggctgaggcaggggtgctgggcactgggctggggcgggcccgctcactcccctcctctaccaggctcagggaaatggcctggcgggtagcgtaagtgcagttgggcagggggctgttgcgggggatccgaaccttatcctcagagaactctattaccctgcggccaggatacagtgggtgtggtggagacggggttgggtaggggttcagcttctcaaaggctggcaggggcagctcttcctccggggagcccctggcagtacccagagagtggcactccccattgggttgtggggtggggctgccaggggccgggggactggctggatcacctgggacaccctcactcatgtccacatgcacaaagacatcctcagccaaggggcgcccggcgctgcctgactgggctgaattgagcagtagagactccggcttctctaacactcgggcaatgactgaggtaggcaccacagcccctggggctaggctgggagcaggacctgggctggcggcctcttgaccactgtgcaaatgtttccgaaccatgtcctgtagctcacagggcagatcggcaaacttgtggtttcggaagtgggacttgttgcacttgaggagctgtacagccaggttgcagtccagccggtaccgctcattgagctcttccagcttgttgatggtgttcttggcatccagcagcttgttggtcagctccacaatctcccagtccagcgtcttcctatccatctcagccttcttgatcagtgtgtgcagcttgtcctccaactcctggttggtccgctgggaagccgtgtagctgttctgcagcctgcggaacttatccttaaatttgtccagctcctcgcggctctggcccagctccagctccaggcagtcctgcccaatttccagctcacgttccagggcctcagtgcgtctggtggcggaggccaggcgccggcgaagctcttcattctcctcctgtaagagcttcatcctttctgcatcagtcaggggttcctcctgctcaagccgggatccaggaatttccaaacgcagctcccgatgctctggtggtgccttacggtagggtttcttagcaggggcggcactagtcattctgggaggtgacggctcctccgccgtctgtttgtcggcagctctctctgttccgctgtccgggagttagccctcggctctccgcatcccacggcccctccacttcctttagccacagctccaaaaaagcaaaagtagacacacagcgagaatgaattcaggagtcagtgacagcaggtacccgctctggggttggactggggcaagtcgctatctcttcttctttccaagtaggcactgtaatttcttccagtccctggggcacctgaatcttcagctgaaattggggcagatgctgctaacagctgtggaaaggctgatctaagctttccgccgctgccagctgcgttcaggccgccatcttgccgcggggcaggccgggtagt

SEQ ID NO: 19562 - RNA, 2267 nt, Homo sapiens
  source 1..2267: mol_type = other RNA
ttgggctgggctgggttgggctgattggaggaaaggtcttgagacccaactgcatgttacctctgaagaataaatattctaagaaaaagggaaaaccatgaggcaagctgctgcagtcagtcaacgcagctgacaggcctggcatggcccacaacctgaccccatccacacaggaaacagctgtgcgggtctggatagaggagaggtcaagggcttggactggggaccctgagctgccaaggtgtggggactccttgcagtcctggtgcagcaatggcaggaaggccagcaggggccctagttgagcaggttgccctgctcctgggcctgggtcaggctgtccttgcggtgcaggtggtgaacccccatcctcttggggctgcgctgggggcgactggagctggggagtggccaggccctgccctcggtgtgggaagtgcctggcccctcctctgtgcccctgttaatgggcagcaggctctggcgctcttcctcaggactgataggcaggttcagctcttcttcctccctgggaaagccagagtcaggttctgtgggtagcaaaagctcactctcttcgggtcgggcagaaggtgcctggaccacctcatctctgtcagcggggctatgggcaaaatggcgctgcagctcagggagggcatcgcgtccaaaggctgtgcgctgggccacagcagcaggtggtggagtacggtccacaaatgcccgctgccagctgaccagcaggtcctcttcagagctggcagagctagctggggcactgagtgttaggggtgctgggctgggctggtggtggggtgaggcctgggctgaggcaggggtgctgggcactgggctggggcgggcccgctcactcccctcctctaccaggctcagggaaatggcctggcgggtagcgtaagtgcagttgggcagggggctgttgcgggggatccgaaccttatcctcagagaactctattaccctgcggccaggatacagtgggtgtggtggagacggggttgggtaggggttcagcttctcaaaggctggcaggggcagctcttcctccggggagcccctggcagtacccagagagtggcactccccattgggttgtggggtggggctgccaggggccgggggactggctggatcacctgggacaccctcactcatgtccacatgcacaaagacatcctcagccaaggggcgcccggcgctgcctgactgggctgaattgagcagtagagactccggcttctctaacactcgggcaatgactgaggtaggcaccacagcccctggggctaggctgggagcaggacctgggctggcggcctcttgaccactgtgcaaatgtttccgaaccatgtcctgtagctcacagggcagatcggcaaacttgtggtttcggaagtgggacttgttgcacttgaggagctgtacagccaggttgcagtccagccggtaccgctcattgagctcttccagcttgttgatggtgttcttggcatccagcagcttgttggtcagctccacaatctcccagtccagcgtcttcctatccatctcagccttcttgatcagtgtgtgcagcttgtcctccaactcctggttggtccgctgggaagccgtgtagctgttctgcagcctgcggaacttatccttaaatttgtccagctcctcgcggctctggcccagctccagctccaggcagtcctgcccaatttccagctcacgttccagggcctcagtgcgtctggtggcggaggccaggcgccggcgaagctcttcattctcctcctgtaagagcttcatcctttctgcatcagtcaggggttcctcctgctcaagccgggatccaggaatttccaaacgcagctcccgatgctctggtggtgccttacggtagggtttcttagcaggggcggcactagtcattctgggaggtgacggctcctccgccgtctgtttgtcggcagctctctctgttccgctgtccgggagttagccctcggctctccgcatcccacggcccctccacttcctttagccacagctcccgctctggggttggactggggcaagtcgctatctcttcttctttccaagtaggcactgtaatttcttccagtccctggggcacctgaatcttcagctgaaattggggcagatgctgctaacagctgtggaaaggctgatctaagctttccgccgctgccagctgcgttcaggccgccatcttgccgcggggcaggccgggtagt

SEQ ID NO: 19563 - RNA, 2217 nt, Homo sapiens
  source 1..2217: mol_type = other RNA
ttgggctgggctgggttgggctgattggaggaaaggtcttgagacccaactgcatgttacctctgaagaataaatattctaagaaaaagggaaaaccatgaggcaagctgctgcagtcagtcaacgcagctgacaggcctggcatggcccacaacctgaccccatccacacaggaaacagctgtgcgggtctggatagaggagaggtcaagggcttggactggggaccctgagctgccaaggtgtggggactccttgcagtcctggtgcagcaatggcaggaaggccagcaggggccctagttgagcaggttgccctgctcctgggcctgggtcaggctgtccttgcggtgcaggtggtgaacccccatcctcttggggctgcgctgggggcgactggagctggggagtggccaggccctgccctcggtgtgggaagtgcctggcccctcctctgtgcccctgttaatgggcagcaggctctggcgctcttcctcaggactgataggcaggttcagctcttcttcctccctgggaaagccagagtcaggttctgtgggtagcaaaagctcactctcttcgggtcgggcagaaggtgcctggaccacctcatctctgtcagcggggctatgggcaaaatggcgctgcagctcagggagggcatcgcgtccaaaggctgtgcgctgggccacagcagcaggtggtggagtacggtccacaaatgcccgctgccagctgaccagcaggtcctcttcagagctggcagagctagctggggcactgagtgttaggggtgctgggctgggctggtggtggggtgaggcctgggctgaggcaggggtgctgggcactgggctggggcgggcccgctcactcccctcctctaccaggctcagggaaatggcctggcgggtagcgtaagtgcagttgggcagggggctgttgcgggggatccgaaccttatcctcagagaactctattaccctgcggccaggatacagtgggtgtggtggagacggggttgggtaggggttcagcttctcaaaggctggcaggggcagctcttcctccggggagcccctggcagtacccagagagtggcactccccattgggttgtggggtggggctgccaggggccgggggactggctggatcacctgggacaccctcactcatgtccacatgcacaaagacatcctcagccaaggggcgcccggcgctgcctgactgggctgaattgagcagtagagactccggcttctctaacactcgggcaatgactgaggtaggcaccacagcccctggggctaggctgggagcaggacctgggctggcggcctcttgaccactgtgcaaatgtttccgaaccatgtcctgtagctcacagggcagatcggcaaacttgtggtttcggaagtgggacttgttgcacttgaggagctgtacagccaggttgcagtccagccggtaccgctcattgagctcttccagcttgttgatggtgttcttggcatccagcagcttgttggtcagctccacaatctcccagtccagcgtcttcctatccatctcagccttcttgatcagtgtgtgcagcttgtcctccaactcctggttggtccgctgggaagccgtgtagctgttctgcagcctgcggaacttatccttaaatttgtccagctcctcgcggctctggcccagctccagctccaggcagtcctgcccaatttccagctcacgttccagggcctcagtgcgtctggtggcggaggccaggcgccggcgaagctcttcattctcctcctgtaagagcttcatcctttctgcatcagtcaggggttcctcctgctcaagccgggatccaggaatttccaaacgcagctcccgatgctctggtggtgccttacggtagggtttcttagcaggggcggcactagtcattctgggaggtgacggctcctccgccgtctgtttgtcggcagctctctctgttccgctgtccgggagttagccctcggctctccgcatcccacggcccctccacttcctttagccacagctcccgctctggggttggactggggcaagtcgctatctcttcttctttccaagtaggcactgtaatttcttccagtccctggggcacctgaatcttcagtttccgccgctgccagctgcgttcaggccgccatcttgccgcggggcaggccgggtagt

SEQ ID NO: 19564 - RNA, 2121 nt, Homo sapiens
  source 1..2121: mol_type = other RNA
ttgggctgggctgggttgggctgattggaggaaaggtcttgagacccaactgcatgttacctctgaagaataaatattctaagaaaaagggaaaaccatgaggcaagctgctgcagtcagtcaacgcagctgacaggcctggcatggcccacaacctgaccccatccacacaggaaacagctgtgcgggtctggatagaggagaggtcaagggcttggactggggaccctgagctgccaaggtgtggggactccttgcagtcctggtgcagcaatggcaggaaggccagcaggggccctagttgagcaggttgccctgctcctgggcctgggtcaggctgtccttgcggtgcaggtggtgaacccccatcctcttggggctgcgctgggggcgactggagctggggagtggccaggccctgccctcggtgtgggaagtgcctggcccctcctctgtgcccctgttaatgggcagcaggctctggcgctcttcctcaggactgataggcaggttcagctcttcttcctccctgggaaagccagagtcaggttctgtgggtagcaaaagctcactctcttcgggtcgggcagaaggtgcctggaccacctcatctctgtcagcggggctatgggcaaaatggcgctgcagctcagggagggcatcgcgtccaaaggctgtgcgctgggccacagcagcaggtggtggagtacggtccacaaatgcccgctgccagctgaccagcaggtcctcttcagagctggcagagctagctggggcactgagtgttaggggtgctgggctgggctggtggtggggtgaggcctgggctgaggcaggggtgctgggcactgggctggggcgggcccgctcactcccctcctctaccaggctcagggaaatggcctggcgggtagcgtaagtgcagttgggcagggggctgttgcgggggatccgaaccttatcctcagagaactctattaccctgcggccaggatacagtgggtgtggtggagacggggttgggtaggggttcagcttctcaaaggctggcaggggcagctcttcctccggggagcccctggcagtacccagagagtggcactccccattgggttgtggggtggggctgccaggggccgggggactggctggatcacctgggacaccctcactcatgtccacatgcacaaagacatcctcagccaaggggcgcccggcgctgcctgactgggctgaattgagcagtagagactccggcttctctaacactcgggcaatgactgaggtaggcaccacagcccctggggctaggctgggagcaggacctgggctggcggcctcttgaccactgtgcaaatgtttccgaaccatgtcctgtagctcacagggcagatcggcaaacttgtggtttcggaagtgggacttgttgcacttgaggagctgtacagccaggttgcagtccagccggtaccgctcattgagctcttccagcttgttgatggtgttcttggcatccagcagcttgttggtcagctccacaatctcccagtccagcgtcttcctatccatctcagccttcttgatcagtgtgtgcagcttgtcctccaactcctggttggtccgctgggaagccgtgtagctgttctgcagcctgcggaacttatccttaaatttgtccagctcctcgcggctctggcccagctccagctccaggcagtcctgcccaatttccagctcacgttccagggcctcagtgcgtctggtggcggaggccaggcgccggcgaagctcttcattctcctcctgtaagagcttcatcctttctgcatcagtcaggggttcctcctgctcaagccgggatccaggaatttccaaacgcagctcccgatgctctggtggtgccttacggtagggtttcttagcaggggcggcactagtcattctgggaggtgacggctcctccgccgtctgtttgtcggcagctctctctgttccgctgtccgggagttagccctcggctctccgcatcccacggcccctccacttcctttagccacagctctttccgccgctgccagctgcgttcaggccgccatcttgccgcggggcaggccgggtagt

SEQ ID NO: 19565 - RNA, 2460 nt, Homo sapiens
  source 1..2460: mol_type = other RNA
ttgggctgggctgggttgggctgattggaggaaaggtcttgagacccaactgcatgttacctctgaagaataaatattctaagaaaaagggaaaaccatgaggcaagctgctgcagtcagtcaacgcagctgacaggcctggcatggcccacaacctgaccccatccacacaggaaacagctgtgcgggtctggatagaggagaggtcaagggcttggactggggaccctgagctgccaaggtgtggggactccttgcagtcctggtgcagcaatggcaggaaggccagcaggggccctagttgagcaggttgccctgctcctgggcctgggtcaggctgtccttgcggtgcaggtggtgaacccccatcctcttggggctgcgctgggggcgactggagctggggagtggccaggccctgccctcggtgtgggaagtgcctggcccctcctctgtgcccctgttaatgggcagcaggctctggcgctcttcctcaggactgataggcaggttcagctcttcttcctccctgggaaagccagagtcaggttctgtgggtagcaaaagctcactctcttcgggtcgggcagaaggtgcctggaccacctcatctctgtcagcggggctatgggcaaaatggcgctgcagctcagggagggcatcgcgtccaaaggctgtgcgctgggccacagcagcaggtggtggagtacggtccacaaatgcccgctgccagctgaccagcaggtcctcttcagagctggcagagctagctggggcactgagtgttaggggtgctgggctgggctggtggtggggtgaggcctgggctgaggcaggggtgctgggcactgggctggggcgggcccgctcactcccctcctctaccaggctcagggaaatggcctggcgggtagcgtaagtgcagttgggcagggggctgttgcgggggatccgaaccttatcctcagagaactctattaccctgcggccaggatacagtgggtgtggtggagacggggttgggtaggggttcagcttctcaaaggctggcaggggcagctcttcctccggggagcccctggcagtacccagagagtggcactccccattgggttgtggggtggggctgccaggggccgggggactggctggatcacctgggacaccctcactcatgtccacatgcacaaagacatcctcagccaaggggcgcccggcgctgcctgactgggctgaattgagcagtagagactccggcttctctaacactcgggcaatgactgaggtaggcaccacagcccctggggctaggctgggagcaggacctgggctggcggcctcttgaccactgtgcaaatgtttccgaaccatgtcctgtagctcacagggcagatcggcaaacttgtggtttcggaagtgggacttgttgcacttgaggagctgtacagccaggttgcagtccagccggtaccgctcattgagctcttccagcttgttgatggtgttcttggcatccagcagcttgttggtcagctccacaatctcccagtccagcgtcttcctatccatctcagccttcttgatcagtgtgtgcagcttgtcctccaactcctggttggtccgctgggaagccgtgtagctgttctgcagcctgcggaacttatccttaaatttgtccagctcctcgcggctctggcccagctccagctccaggcagtcctgcccaatttccagctcacgttccagggcctcagtgcgtctggtggcggaggccaggcgccggcgaagctcttcattctcctcctgtaagagcttcatcctttctgcatcagtcaggggttcctcctgctcaagccgggatccaggaatttccaaacgcagctcccgatgctctggtggtgccttacggtagggtttcttagcaggggcggcactagtcattctgggaggtgacggctcctccgcctgcgtctgtttgtcggcagctctctctgttccgctgtccgggagttagccctcggctctccgcatcccacggcccctccacttcctttagccacagctcagggttagtgtcttctccccaaccagccagctctcctggttagtgcagttagcgacagactcatggcagatgccctccaggcactccatataaacagacagcttggtttgtgagcagcccaactccggagcaaaaaagcaaaagtagacacacagcgagaatgaattcaggagtcagtgacagcaggtacccgctctggggttggactggggcaagtcgctatctcttcttctttccaagtaggcactgtaatttcttccagtccctggggcacctgaatcttcagctgaaattggggcagatgctgctaacagctgtggaaaggctgatctaagctttccgccgctgccagctgcgttcaggccgccatcttgccgcggggcaggccgggtagt

SEQ ID NO: 19566 - RNA, 2434 nt, Homo sapiens
  source 1..2434: mol_type = other RNA
ttgggctgggctgggttgggctgattggaggaaaggtcttgagacccaactgcatgttacctctgaagaataaatattctaagaaaaagggaaaaccatgaggcaagctgctgcagtcagtcaacgcagctgacaggcctggcatggcccacaacctgaccccatccacacaggaaacagctgtgcgggtctggatagaggagaggtcaagggcttggactggggaccctgagctgccaaggtgtggggactccttgcagtcctggtgcagcaatggcaggaaggccagcaggggccctagttgagcaggttgccctgctcctgggcctgggtcaggctgtccttgcggtgcaggtggtgaacccccatcctcttggggctgcgctgggggcgactggagctggggagtggccaggccctgccctcggtgtgggaagtgcctggcccctcctctgtgcccctgttaatgggcagcaggctctggcgctcttcctcaggactgataggcaggttcagctcttcttcctccctgggaaagccagagtcaggttctgtgggtagcaaaagctcactctcttcgggtcgggcagaaggtgcctggaccacctcatctctgtcagcggggctatgggcaaaatggcgctgcagctcagggagggcatcgcgtccaaaggctgtgcgctgggccacagcagcaggtggtggagtacggtccacaaatgcccgctgccagctgaccagcaggtcctcttcagagctggcagagctagctggggcactgagtgttaggggtgctgggctgggctggtggtggggtgaggcctgggctgaggcaggggtgctgggcactgggctggggcgggcccgctcactcccctcctctaccaggctcagggaaatggcctggcgggtagcgtaagtgcagttgggcagggggctgttgcgggggatccgaaccttatcctcagagaactctattaccctgcggccaggatacagtgggtgtggtggagacggggttgggtaggggttcagcttctcaaaggctggcaggggcagctcttcctccggggagcccctggcagtacccagagagtggcactccccattgggttgtggggtggggctgccaggggccgggggactggctggatcacctgggacaccctcactcatgtccacatgcacaaagacatcctcagccaaggggcgcccggcgctgcctgactgggctgaattgagcagtagagactccggcttctctaacactcgggcaatgactgaggtaggcaccacagcccctggggctaggctgggagcaggacctgggctggcggcctcttgaccactgtgcaaatgtttccgaaccatgtcctgtagctcacagggcagatcggcaaacttgtggtttcggaagtgggacttgttgcacttgaggagctgtacagccaggttgcagtccagccggtaccgctcattgagctcttccagcttgttgatggtgttcttggcatccagcagcttgttggtcagctccacaatctcccagtccagcgtcttcctatccatctcagccttcttgatcagtgtgtgcagcttgtcctccaactcctggttggtccgctgggaagccgtgtagctgttctgcagcctgcggaacttatccttaaatttgtccagctcctcgcggctctggcccagctccagctccaggcagtcctgcccaatttccagctcacgttccagggcctcagtgcgtctggtggcggaggccaggcgccggcgaagctcttcattctcctcctgtaagagcttcatcctttctgcatcagtcaggggttcctcctgctcaagccgggatccaggaatttccaaacgcagctcccgatgctctggtggtgccttacggtagggtttcttagcaggggcggcactagtcattctgggaggtgacggctcctccgcctgcgtctgtttgtcggcagctctctctgttccgctgtccgggagttagccctcggctctccgcatcccacggcccctccacttcctttagccacagctcagggttagtgtcttctccccaaccagccagctctcctggttagtgcagttagcgacagactcatggcagatgccctccaggcactccatataaacagacagcttggtttgtgagcagcccaactccggagccgctctggggttggactggggcaagtcgctatctcttcttctttccaagtaggcactgtaatttcttccagtccctggggcacctgaatcttcagctgaaattggggcagatgctgctaacagctgtggaaaggctgatctaagctttccgccgctgccagctgcgttcaggccgccatcttgccgcggggcaggccgggtagtggccagggccgcgggaatccccacgcacttggcg

SEQ ID NO: 19567 - RNA, 2330 nt, Homo sapiens
  source 1..2330: mol_type = other RNA
ttgggctgggctgggttgggctgattggaggaaaggtcttgagacccaactgcatgttacctctgaagaataaatattctaagaaaaagggaaaaccatgaggcaagctgctgcagtcagtcaacgcagctgacaggcctggcatggcccacaacctgaccccatccacacaggaaacagctgtgcgggtctggatagaggagaggtcaagggcttggactggggaccctgagctgccaaggtgtggggactccttgcagtcctggtgcagcaatggcaggaaggccagcaggggccctagttgagcaggttgccctgctcctgggcctgggtcaggctgtccttgcggtgcaggtggtgaacccccatcctcttggggctgcgctgggggcgactggagctggggagtggccaggccctgccctcggtgtgggaagtgcctggcccctcctctgtgcccctgttaatgggcagcaggctctggcgctcttcctcaggactgataggcaggttcagctcttcttcctccctgggaaagccagagtcaggttctgtgggtagcaaaagctcactctcttcgggtcgggcagaaggtgcctggaccacctcatctctgtcagcggggctatgggcaaaatggcgctgcagctcagggagggcatcgcgtccaaaggctgtgcgctgggccacagcagcaggtggtggagtacggtccacaaatgcccgctgccagctgaccagcaggtcctcttcagagctggcagagctagctggggcactgagtgttaggggtgctgggctgggctggtggtggggtgaggcctgggctgaggcaggggtgctgggcactgggctggggcgggcccgctcactcccctcctctaccaggctcagggaaatggcctggcgggtagcgtaagtgcagttgggcagggggctgttgcgggggatccgaaccttatcctcagagaactctattaccctgcggccaggatacagtgggtgtggtggagacggggttgggtaggggttcagcttctcaaaggctggcaggggcagctcttcctccggggagcccctggcagtacccagagagtggcactccccattgggttgtggggtggggctgccaggggccgggggactggctggatcacctgggacaccctcactcatgtccacatgcacaaagacatcctcagccaaggggcgcccggcgctgcctgactgggctgaattgagcagtagagactccggcttctctaacactcgggcaatgactgaggtaggcaccacagcccctggggctaggctgggagcaggacctgggctggcggcctcttgaccactgtgcaaatgtttccgaaccatgtcctgtagctcacagggcagatcggcaaacttgtggtttcggaagtgggacttgttgcacttgaggagctgtacagccaggttgcagtccagccggtaccgctcattgagctcttccagcttgttgatggtgttcttggcatccagcagcttgttggtcagctccacaatctcccagtccagcgtcttcctatccatctcagccttcttgatcagtgtgtgcagcttgtcctccaactcctggttggtccgctgggaagccgtgtagctgttctgcagcctgcggaacttatccttaaatttgtccagctcctcgcggctctggcccagctccagctccaggcagtcctgcccaatttccagctcacgttccagggcctcagtgcgtctggtggcggaggccaggcgccggcgaagctcttcattctcctcctgtaagagcttcatcctttctgcatcagtcaggggttcctcctgctcaagccgggatccaggaatttccaaacgcagctcccgatgctctggtggtgccttacggtagggtttcttagcaggggcggcactagtcattctgggaggtgacggctcctccgcctgcgtctgtttgtcggcagctctctctgttccgctgtccgggagttagccctcggctctccgcatcccacggcccctccacttcctttagccacagctccaaaaaagcaaaagtagacacacagcgagaatgaattcaggagtcagtgacagcaggtacccgctctggggttggactggggcaagtcgctatctcttcttctttccaagtaggcactgtaatttcttccagtccctggggcacctgaatcttcagctgaaattggggcagatgctgctaacagctgtggaaaggctgatctaagctttccgccgctgccagctgcgttcaggccgccatcttgccgcggggcaggccgggtagt

SEQ ID NO: 19568 - RNA, 2270 nt, Homo sapiens
  source 1..2270: mol_type = other RNA
ttgggctgggctgggttgggctgattggaggaaaggtcttgagacccaactgcatgttacctctgaagaataaatattctaagaaaaagggaaaaccatgaggcaagctgctgcagtcagtcaacgcagctgacaggcctggcatggcccacaacctgaccccatccacacaggaaacagctgtgcgggtctggatagaggagaggtcaagggcttggactggggaccctgagctgccaaggtgtggggactccttgcagtcctggtgcagcaatggcaggaaggccagcaggggccctagttgagcaggttgccctgctcctgggcctgggtcaggctgtccttgcggtgcaggtggtgaacccccatcctcttggggctgcgctgggggcgactggagctggggagtggccaggccctgccctcggtgtgggaagtgcctggcccctcctctgtgcccctgttaatgggcagcaggctctggcgctcttcctcaggactgataggcaggttcagctcttcttcctccctgggaaagccagagtcaggttctgtgggtagcaaaagctcactctcttcgggtcgggcagaaggtgcctggaccacctcatctctgtcagcggggctatgggcaaaatggcgctgcagctcagggagggcatcgcgtccaaaggctgtgcgctgggccacagcagcaggtggtggagtacggtccacaaatgcccgctgccagctgaccagcaggtcctcttcagagctggcagagctagctggggcactgagtgttaggggtgctgggctgggctggtggtggggtgaggcctgggctgaggcaggggtgctgggcactgggctggggcgggcccgctcactcccctcctctaccaggctcagggaaatggcctggcgggtagcgtaagtgcagttgggcagggggctgttgcgggggatccgaaccttatcctcagagaactctattaccctgcggccaggatacagtgggtgtggtggagacggggttgggtaggggttcagcttctcaaaggctggcaggggcagctcttcctccggggagcccctggcagtacccagagagtggcactccccattgggttgtggggtggggctgccaggggccgggggactggctggatcacctgggacaccctcactcatgtccacatgcacaaagacatcctcagccaaggggcgcccggcgctgcctgactgggctgaattgagcagtagagactccggcttctctaacactcgggcaatgactgaggtaggcaccacagcccctggggctaggctgggagcaggacctgggctggcggcctcttgaccactgtgcaaatgtttccgaaccatgtcctgtagctcacagggcagatcggcaaacttgtggtttcggaagtgggacttgttgcacttgaggagctgtacagccaggttgcagtccagccggtaccgctcattgagctcttccagcttgttgatggtgttcttggcatccagcagcttgttggtcagctccacaatctcccagtccagcgtcttcctatccatctcagccttcttgatcagtgtgtgcagcttgtcctccaactcctggttggtccgctgggaagccgtgtagctgttctgcagcctgcggaacttatccttaaatttgtccagctcctcgcggctctggcccagctccagctccaggcagtcctgcccaatttccagctcacgttccagggcctcagtgcgtctggtggcggaggccaggcgccggcgaagctcttcattctcctcctgtaagagcttcatcctttctgcatcagtcaggggttcctcctgctcaagccgggatccaggaatttccaaacgcagctcccgatgctctggtggtgccttacggtagggtttcttagcaggggcggcactagtcattctgggaggtgacggctcctccgcctgcgtctgtttgtcggcagctctctctgttccgctgtccgggagttagccctcggctctccgcatcccacggcccctccacttcctttagccacagctcccgctctggggttggactggggcaagtcgctatctcttcttctttccaagtaggcactgtaatttcttccagtccctggggcacctgaatcttcagctgaaattggggcagatgctgctaacagctgtggaaaggctgatctaagctttccgccgctgccagctgcgttcaggccgccatcttgccgcggggcaggccgggtagt

SEQ ID NO: 19569 - RNA, 2125 nt, Homo sapiens
  source 1..2125: mol_type = other RNA
ttgggctgggctgggttgggctgattggaggaaaggtcttgagacccaactgcatgttacctctgaagaataaatattctaagaaaaagggaaaaccatgaggcaagctgctgcagtcagtcaacgcagctgacaggcctggcatggcccacaacctgaccccatccacacaggaaacagctgtgcgggtctggatagaggagaggtcaagggcttggactggggaccctgagctgccaaggtgtggggactccttgcagtcctggtgcagcaatggcaggaaggccagcaggggccctagttgagcaggttgccctgctcctgggcctgggtcaggctgtccttgcggtgcaggtggtgaacccccatcctcttggggctgcgctgggggcgactggagctggggagtggccaggccctgccctcggtgtgggaagtgcctggcccctcctctgtgcccctgttaatgggcagcaggctctggcgctcttcctcaggactgataggcaggttcagctcttcttcctccctgggaaagccagagtcaggttctgtgggtagcaaaagctcactctcttcgggtcgggcagaaggtgcctggaccacctcatctctgtcagcggggctatgggcaaaatggcgctgcagctcagggagggcatcgcgtccaaaggctgtgcgctgggccacagcagcaggtggtggagtacggtccacaaatgcccgctgccagctgaccagcaggtcctcttcagagctggcagagctagctggggcactgagtgttaggggtgctgggctgggctggtggtggggtgaggcctgggctgaggcaggggtgctgggcactgggctggggcgggcccgctcactcccctcctctaccaggctcagggaaatggcctggcgggtagcgtaagtgcagttgggcagggggctgttgcgggggatccgaaccttatcctcagagaactctattaccctgcggccaggatacagtgggtgtggtggagacggggttgggtaggggttcagcttctcaaaggctggcaggggcagctcttcctccggggagcccctggcagtacccagagagtggcactccccattgggttgtggggtggggctgccaggggccgggggactggctggatcacctgggacaccctcactcatgtccacatgcacaaagacatcctcagccaaggggcgcccggcgctgcctgactgggctgaattgagcagtagagactccggcttctctaacactcgggcaatgactgaggtaggcaccacagcccctggggctaggctgggagcaggacctgggctggcggcctcttgaccactgtgcaaatgtttccgaaccatgtcctgtagctcacagggcagatcggcaaacttgtggtttcggaagtgggacttgttgcacttgaggagctgtacagccaggttgcagtccagccggtaccgctcattgagctcttccagcttgttgatggtgttcttggcatccagcagcttgttggtcagctccacaatctcccagtccagcgtcttcctatccatctcagccttcttgatcagtgtgtgcagcttgtcctccaactcctggttggtccgctgggaagccgtgtagctgttctgcagcctgcggaacttatccttaaatttgtccagctcctcgcggctctggcccagctccagctccaggcagtcctgcccaatttccagctcacgttccagggcctcagtgcgtctggtggcggaggccaggcgccggcgaagctcttcattctcctcctgtaagagcttcatcctttctgcatcagtcaggggttcctcctgctcaagccgggatccaggaatttccaaacgcagctcccgatgctctggtggtgccttacggtagggtttcttagcaggggcggcactagtcattctgggaggtgacggctcctccgcctgcgtctgtttgtcggcagctctctctgttccgctgtccgggagttagccctcggctctccgcatcccacggcccctccacttcctttagccacagctctttccgccgctgccagctgcgttcaggccgccatcttgccgcggggcaggccgggtagtg

SEQ ID NO: 19570 - RNA, 2322 nt, Homo sapiens
  source 1..2322: mol_type = other RNA
ttgggctgggctgggttgggctgattggaggaaaggtcttgagacccaactgcatgttacctctgaagaataaatattctaagaaaaagggaaaaccatgaggcaagctgctgcagtcagtcaacgcagctgacaggcctggcatggcccacaacctgaccccatccacacaggaaacagctgtgcgggtctggatagaggagaggtcaagggcttggactggggaccctgagctgccaaggtgtggggactccttgcagtcctggtgcagcaatggcaggaaggccagcaggggccctagttgagcaggttgccctgctcctgggcctgggtcaggctgtccttgcggtgcaggtggtgaacccccatcctcttggggctgcgctgggggcgactggagctggggagtggccaggccctgccctcggtgtgggaagtgcctggcccctcctctgtgcccctgttaatgggcagcaggctctggcgctcttcctcaggactgataggcaggttcagctcttcttcctccctgggaaagccagagtcaggttctgtgggtagcaaaagctcactctcttcgggtcgggcagaaggtgcctggaccacctcatctctgtcagcggggctatgggcaaaatggcgctgcagctcagggagggcatcgcgtccaaaggctgtgcgctgggccacagcagcaggtggtggagtacggtccacaaatgcccgctgccagctgaccagcaggtcctcttcagagctggcagagctagctggggcactgagtgttaggggtgctgggctgggctggtggtggggtgaggcctgggctgaggcaggggtgctgggcactgggctggggcgggcccgctcactcccctcctctaccaggctcagggaaatggcctggcgggtagcgtaagtgcagttgggcagggggctgttgcgggggatccgaaccttatcctcagagaactctattaccctgcggccaggatacagtgggtgtggtggagacggggttgggtaggggttcagcttctcaaaggctggcaggggcagctcttcctccggggagcccctggcagtacccagagagtggcactccccattgggttgtggggtggggctgccaggggccgggggactggctggatcacctgggacaccctcactcatgtccacatgcacaaagacatcctcagccaaggggcgcccggcgctgcctgactgggctgaattgagcagtagagactccggcttctctaacactcgggcaatgactgaggtaggcaccacagcccctggggctaggctgggagcaggacctgggctggcggcctcttgaccactgtgcaaatgtttccgaaccatgtcctgtagctcacagggcagatcggcaaacttgtggtttcggaagtgggacttgttgcacttgaggagctgtacagccaggttgcagtccagccggtaccgctcattgagctcttccagcttgttgatggtgttcttggcatccagcagcttgttggtcagctccacaatctcccagtccagcgtcttcctatccatctcagccttcttgatcagtgtgtgcagcttgtcctccaactcctggttggtccgctgggaagccgtgtagctgttctgcagcctgcggaacttatccttaaatttgtccagctcctcgcggctctggcccagctccagctccaggcagtcctgcccaatttccagctcacgttccagggcctcagtgcgtctggtggcggaggccaggcgccggcgaagctcttcattctcctcctgtaagagcttcatcctttctgcatcagtcaggggttcctcctgctcaagccgggatccaggaatttccaaacgcagctcccgatgctctggtggtgccttacggtagggtttcttagcaggggcggcactagtcattctgggaggtgacggctcctccgcctgctgagaagcaagaaggaggcaggctcagagatgtggccagaaggactctggacgtctgtttgtcggcagctctctctgttccgctgtccgggagttagccctcggctctccgcatcccacggcccctccacttcctttagccacagctcccgctctggggttggactggggcaagtcgctatctcttcttctttccaagtaggcactgtaatttcttccagtccctggggcacctgaatcttcagctgaaattggggcagatgctgctaacagctgtggaaaggctgatctaagctttccgccgctgccagctgcgttcaggccgccatcttgccgcggggcaggccgggtagt

SEQ ID NO: 19571 - RNA, 2306 nt, Homo sapiens
  source 1..2306: mol_type = other RNA
ttgggctgggctgggttgggctgattggaggaaaggtcttgagacccaactgcatgttacctctgaagaataaatattctaagaaaaagggaaaaccatgaggcaagctgctgcagtcagtcaacgcagctgacaggcctggcatggcccacaacctgaccccatccacacaggaaacagctgtgcgggtctggatagaggagaggtcaagggcttggactggggaccctgagctgccaaggtgtggggactccttgcagtcctggtgcagcaatggcaggaaggccagcaggggccctagttgagcaggttgccctgctcctgggcctgggtcaggctgtccttgcggtgcaggtggtgaacccccatcctcttggggctgcgctgggggcgactggagctggggagtggccaggccctgccctcggtgtgggaagtgcctggcccctcctctgtgcccctgttaatgggcagcaggctctggcgctcttcctcaggactgataggcaggttcagctcttcttcctccctgggaaagccagagtcaggttctgtgggtagcaaaagctcactctcttcgggtcgggcagaaggtgcctggaccacctcatctctgtcagcggggctatgggcaaaatggcgctgcagctcagggagggcatcgcgtccaaaggctgtgcgctgggccacagcagcaggtggtggagtacggtccacaaatgcccgctgccagctgaccagcaggtcctcttcagagctggcagagctagctggggcactgagtgttaggggtgctgggctgggctggtggtggggtgaggcctgggctgaggcaggggtgctgggcactgggctggggcgggcccgctcactcccctcctctaccaggctcagggaaatggcctggcgggtagcgtaagtgcagttgggcagggggctgttgcgggggatccgaaccttatcctcagagaactctattaccctgcggccaggatacagtgggtgtggtggagacggggttgggtaggggttcagcttctcaaaggctggcaggggcagctcttcctccggggagcccctggcagtacccagagagtggcactccccattgggttgtggggtggggctgccaggggccgggggactggctggatcacctgggacaccctcactcatgtccacatgcacaaagacatcctcagccaaggggcgcccggcgctgcctgactgggctgaattgagcagtagagactccggcttctctaacactcgggcaatgactgaggtaggcaccacagcccctggggctaggctgggagcaggacctgggctggcggcctcttgaccactgtgcaaatgtttccgaaccatgtcctgtagctcacagggcagatcggcaaacttgtggtttcggaagtgggacttgttgcacttgaggagctgtacagccaggttgcagtccagccggtaccgctcattgagctcttccagcttgttgatggtgttcttggcatccagcagcttgttggtcagctccacaatctcccagtccagcgtcttcctatccatctcagccttcttgatcagtgtgtgcagcttgtcctccaactcctggttggtccgctgggaagccgtgtagctgttctgcagcctgcggaacttatccttaaatttgtccagctcctcgcggctctggcccagctccagctccaggcagtcctgcccaatttccagctcacgttccagggcctcagtgcgtctggtggcggaggccaggcgccggcgaagctcttcattctcctcctgtaagagcttcatcctttctgcatcagtcaggggttcctctgccggtcaggctgtgataccagtcttgctgacctcctgctcaagccgggatccaggaatttccaaacgcagctcccgatgctctggtggtgccttacggtagggtttcttagcaggggcggcactagtcattctgggaggtgacggctcctccgcctgcgtctgtttgtcggcagctctctctgttccgctgtccgggagttagccctcggctctccgcatcccacggcccctccacttcctttagccacagctcccgctctggggttggactggggcaagtcgctatctcttcttctttccaagtaggcactgtaatttcttccagtccctggggcacctgaatcttcagctgaaattggggcagatgctgctaacagctgtggaaaggctgatctaagctttccgccgctgccagctgcgttcaggccgccatcttgccgcggggcaggccgggtagt

SEQ ID NO: 19572 - RNA, 2488 nt, Homo sapiens
  source 1..2488: mol_type = other RNA
ttgggctgggctgggttgggctgattggaggaaaggtcttgagacccaactgcatgttacctctgaagaataaatattctaagaaaaagggaaaaccatgaggcaagctgctgcagtcagtcaacgcagctgacaggcctggcatggcccacaacctgaccccatccacacaggaaacagctgtgcgggtctggatagaggagaggtcaagggcttggactggggaccctgagctgccaaggtgtggggactccttgcagtcctggtgcagcaatggcaggaaggccagcaggggccctagttgagcaggttgccctgctcctgggcctgggtcaggctgtccttgcggtgcaggtggtgaacccccatcctcttggggctgcgctgggggcgactggagctggggagtggccaggccctgccctcggtgtgggaagtgcctggcccctcctctgtgcccctgttaatgggcagcaggctctggcgctcttcctcaggactgataggcaggttcagctcttcttcctccctgggaaagccagagtcaggttctgtgggtagcaaaagctcactctcttcgggtcgggcagaaggtgcctggaccacctcatctctgtcagcggggctatgggcaaaatggcgctgcagctcagggagggcatcgcgtccaaaggctgtgcgctgggccacagcagcaggtggtggagtacggtccacaaatgcccgctgccagctgaccagcaggtcctcttcagagctggcagagctagctggggcactgagtgttaggggtgctgggctgggctggtggtggggtgaggcctgggctgaggcaggggtgctgggcactgggctggggcgggcccgctcactcccctcctctaccaggctcagggaaatggcctggcgggtagcgtaagtgcagttgggcagggggctgttgcgggggatccgaaccttatcctcagagaactctattaccctgcggccaggatacagtgggtgtggtggagacggggttgggtaggggttcagcttctcaaaggctggcaggggcagctcttcctccggggagcccctggcagtacccagagagtggcactccccattgggttgtggggtggggctgccaggggccgggggactggctggatcacctgggacaccctcactcatgtccacatgcacaaagacatcctcagccaaggggcgcccggcgctgcctgactgggctgaattgagcagtagagactccggcttctctaacactcgggcaatgactgaggtaggcaccacagcccctggggctaggctgggagcaggacctgggctggcggcctcttgaccactgtgcaaatgtttccgaaccatgtcctgtagctcacagggcagatcggcaaacttgtggtttcggaagtgggacttgttgcacttgaggagctgtacagccaggttgcagtccagccggtaccgctcattgagctcttccagcttgttgatggtgttcttggcatccagcagcttgttggtcagctccacaatctcccagtccagcgtcttcctatccatctcagccttcttgattgcaaaaatccagctgtggctaagagaggccagtgtgtgcagcttgtcctccaactcctggttggtccgctgggaagccgtgtagctgttctgcagcctgcggaacttatccttaaatttgtccagctcctcgcggctctggcccagctccagctccaggcagtcctgcccaatttccagctcacgttccagggcctcagtgcgtctggtggcggaggccaggcgccggcgaagctcttcattctcctcctgtaagagcttcatcctttctgcatcagtcaggggttcctcctgctcaagccgggatccaggaatttccaaacgcagctcccgatgctctggtggtgccttacggtagggtttcttagcaggggcggcactagtcattctgggaggtgacggctcctccgccgtctgtttgtcggcagctctctctgttccgctgtccgggagttagccctcggctctccgcatcccacggcccctccacttcctttagccacagctcagggttagtgtcttctccccaaccagccagctctcctggttagtgcagttagcgacagactcatggcagatgccctccaggcactccatataaacagacagcttggtttgtgagcagcccaactccggagcaaaaaagcaaaagtagacacacagcgagaatgaattcaggagtcagtgacagcaggtacccgctctggggttggactggggcaagtcgctatctcttcttctttccaagtaggcactgtaatttcttccagtccctggggcacctgaatcttcagctgaaattggggcagatgctgctaacagctgtggaaaggctgatctaagctttccgccgctgccagctgcgttcaggccgccatcttgccgcggggcaggccgggtagtg

SEQ ID NO: 19573 - RNA, 2268 nt, Homo sapiens
  source 1..2268: mol_type = other RNA
ttgggctgggctgggttgggctgattggaggaaaggtcttgagacccaactgcatgttacctctgaagaataaatattctaagaaaaagggaaaaccatgaggcaagctgctgcagtcagtcaacgcagctgacaggcctggcatggcccacaacctgaccccatccacacaggaaacagctgtgcgggtctggatagaggagaggtcaagggcttggactggggaccctgagctgccaaggtgtggggactccttgcagtcctggtgcagcaatggcaggaaggccagcaggggccctagttgagcaggttgccctgctcctgggcctgggtcaggctgtccttgcggtgcaggtggtgaacccccatcctcttggggctgcgctgggggcgactggagctggggagtggccaggccctgccctcggtgtgggaagtgcctggcccctcctctgtgcccctgttaatgggcagcaggctctggcgctcttcctcaggactgataggcaggttcagctcttcttcctccctgggaaagccagagtcaggttctgtgggtagcaaaagctcactctcttcgggtcgggcagaaggtgcctggaccacctcatctctgtcagcggggctatgggcaaaatggcgctgcagctcagggagggcatcgcgtccaaaggctgtgcgctgggccacagcagcaggtggtggagtacggtccacaaatgcccgctgccagctgaccagcaggtcctcttcagagctggcagagctagctggggcactgagtgttaggggtgctgggctgggctggtggtggggtgaggcctgggctgaggcaggggtgctgggcactgggctggggcgggcccgctcactcccctcctctaccaggctcagggaaatggcctggcgggtagcgtaagtgcagttgggcagggggctgttgcgggggatccgaaccttatcctcagagaactctattaccctgcggccaggatacagtgggtgtggtggagacggggttgggtaggggttcagcttctcaaaggctggcaggggcagctcttcctccggggagcccctggcagtacccagagagtggcactccccattgggttgtggggtggggctgccaggggccgggggactggctggatcacctgggacaccctcactcatgtccacatgcacaaagacatcctcagccaaggggcgcccggcgctgcctgactgggctgaattgagcagtagagactccggcttctctaacactcgggcaatgactgaggtaggcaccacagcccctggggctaggctgggagcaggacctgggctggcggcctcttgaccactgtgcaaatgtttccgaaccatgtcctgtagctcacagggcagatcggcaaacttgtggtttcggaagtgggacttgttgcacttgaggagctgtacagccaggttgcagtccagccggtaccgctcattgagctcttccagcttgttgatggtgttcttggcatccagcagcttgttggtcagctccacaatctcccagtccagcgtcttcctatccatctcagccttcttgattgcaaaaatccagctgtggctaagagaggccagtgtgtgcagcttgtcctccaactcctggttggtccgctgggaagccgtgtagctgttctgcagcctgcggaacttatccttaaatttgtccagctcctcgcggctctggcccagctccagctccaggcagtcctgcccaatttccagctcacgttccagggcctcagtgcgtctggtggcggaggccaggcgccggcgaagctcttcattctcctcctgtaagagcttcatcctttctgcatcagtcaggggttcctcctgctcaagccgggatccaggaatttccaaacgcagctcccgatgctctggtggtgccttacggtagggtttcttagcaggggcggcactagtcattctgggaggtgacggctcctccgccgtctgtttgtcggcagctctctctgttccgctgtccgggagttagccctcggctctccgcatcccacggcccctccacttcctttagccacagctcagggttagtgtcttctccccaaccagccagctctcctggttagtgcagttagcgacagactcatggcagatgccctccaggcactccatataaacagacagcttggtttgtgagcagcccaactccggagcaccagaccctcaggggctttctcccatccggaaaccatgccagat

SEQ ID NO: 19574 - RNA, 2387 nt, Homo sapiens
  source 1..2387: mol_type = other RNA
ttgggctgggctgggttgggctgattggaggaaaggtcttgagacccaactgcatgttacctctgaagaataaatattctaagaaaaagggaaaaccatgaggcaagctgctgcagtcagtcaacgcagctgacaggcctggcatggcccacaacctgaccccatccacacaggaaacagctgtgcgggtctggatagaggagaggtcaagggcttggactggggaccctgagctgccaaggtgtggggactccttgcagtcctggtgcagcaatggcaggaaggccagcaggggccctagttgagcaggttgccctgctcctgggcctgggtcaggctgtccttgcggtgcaggtggtgaacccccatcctcttggggctgcgctgggggcgactggagctggggagtggccaggccctgccctcggtgtgggaagtgcctggcccctcctctgtgcccctgttaatgggcagcaggctctggcgctcttcctcaggactgataggcaggttcagctcttcttcctccctgggaaagccagagtcaggttctgtgggtagcaaaagctcactctcttcgggtcgggcagaaggtgcctggaccacctcatctctgtcagcggggctatgggcaaaatggcgctgcagctcagggagggcatcgcgtccaaaggctgtgcgctgggccacagcagcaggtggtggagtacggtccacaaatgcccgctgccagctgaccagcaggtcctcttcagagctggcagagctagctggggcactgagtgttaggggtgctgggctgggctggtggtggggtgaggcctgggctgaggcaggggtgctgggcactgggctggggcgggcccgctcactcccctcctctaccaggctcagggaaatggcctggcgggtagcgtaagtgcagttgggcagggggctgttgcgggggatccgaaccttatcctcagagaactctattaccctgcggccaggatacagtgggtgtggtggagacggggttgggtaggggttcagcttctcaaaggctggcaggggcagctcttcctccggggagcccctggcagtacccagagagtggcactccccattgggttgtggggtggggctgccaggggccgggggactggctggatcacctgggacaccctcactcatgtccacatgcacaaagacatcctcagccaaggggcgcccggcgctgcctgactgggctgaattgagcagtagagactccggcttctctaacactcgggcaatgactgaggtaggcaccacagcccctggggctaggctgggagcaggacctgggctggcggcctcttgaccactgtgcaaatgtttccgaaccatgtcctgtagctcacagggcagatcggcaaacttgtggtttcggaagtgggacttgttgcacttgaggagctgtacagccaggttgcagtccagccggtaccgctcattgagctcttccagcttgttgatggtgttcttggcatccagcagcttgttggtcagctccacaatctcccagtccagcgtcttcctatccatctcagccttcttgattgcaaaaatccagctgtggctaagagaggccagtgtgtgcagcttgtcctccaactcctggttggtccgctgggaagccgtgtagctgttctgcagcctgcggaacttatccttaaatttgtccagctcctcgcggctctggcccagctccagctccaggcagtcctgcccaatttccagctcacgttccagggcctcagtgcgtctggtggcggaggccaggcgccggcgaagctcttcattctcctcctgtaagagcttcatcctttctgcatcagtcaggggttcctcctgctcaagccgggatccaggaatttccaaacgcagctcccgatgctctggtggtgccttacggtagggtttcttagcaggggcggcactagtcattctgggaggtgacggctcctccgccgtctgtttgtcggcagctctctctgttccgctgtccgggagttagccctcggctctccgcatcccacggcccctccacttcctttagccacagctccaaaaaagcaaaagtagacacacagcgagaatgaattcaggagtcagtgacagcaggtacccgctctggggttggactggggcaagtcgctatctcttcttctttccaagtaggcactgtaatttcttccagtccctggggcacctgaatcttcagctgaaattggggcagatgctgctaacagctgtggaaaggctgatctaagctttccgccgctgccagctgcgttcaggccgccatcttgccgcggggcaggccgggtagtggccagggccgcgggaatccccacgcactt

SEQ ID NO: 19575 - RNA, 2138 nt, Homo sapiens
  source 1..2138: mol_type = other RNA
ttgggctgggctgggttgggctgattggaggaaaggtcttgagacccaactgcatgttacctctgaagaataaatattctaagaaaaagggaaaaccatgaggcaagctgctgcagtcagtcaacgcagctgacaggcctggcatggcccacaacctgaccccatccacacaggaaacagctgtgcgggtctggatagaggagaggtcaagggcttggactggggaccctgagctgccaaggtgtggggactccttgcagtcctggtgcagcaatggcaggaaggccagcaggggccctagttgagcaggttgccctgctcctgggcctgggtcaggctgtccttgcggtgcaggtggtgaacccccatcctcttggggctgcgctgggggcgactggagctggggagtggccaggccctgccctcggtgtgggaagtgcctggcccctcctctgtgcccctgttaatgggcagcaggctctggcgctcttcctcaggactgataggcaggttcagctcttcttcctccctgggaaagccagagtcaggttctgtgggtagcaaaagctcactctcttcgggtcgggcagaaggtgcctggaccacctcatctctgtcagcggggctatgggcaaaatggcgctgcagctcagggagggcatcgcgtccaaaggctgtgcgctgggccacagcagcaggtggtggagtacggtccacaaatgcccgctgccagctgaccagcaggtcctcttcagagctggcagagctagctggggcactgagtgttaggggtgctgggctgggctggtggtggggtgaggcctgggctgaggcaggggtgctgggcactgggctggggcgggcccgctcactcccctcctctaccaggctcagggaaatggcctggcgggtagcgtaagtgcagttgggcagggggctgttgcgggggatccgaaccttatcctcagagaactctattaccctgcggccaggatacagtgggtgtggtggagacggggttgggtaggggttcagcttctcaaaggctggcaggggcagctcttcctccggggagcccctggcagtacccagagagtggcactccccattgggttgtggggtggggctgccaggggccgggggactggctggatcacctgggacaccctcactcatgtccacatgcacaaagacatcctcagccaaggggcgcccggcgctgcctgactgggctgaattgagcagtagagactccggcttctctaacactcgggcaatgactgaggtaggcaccacagcccctggggctaggctgggagcaggacctgggctggcggcctcttgaccactgtgcaaatgtttccgaaccatgtcctgtagctcacagggcagatcggcaaacttgtggtttcggaagtgggacttgttgcacttgaggagctgtacagccaggttgcagtccagccggtaccgctcattgagctcttccagcttgttgatggtgttcttggcatccagcagcttgttggtcagctccacaatctcccagtccagcgtcttcctatccatctcagccttcttgattgcaaaaatccagctgtggctaagagaggccagtgtgtgcagcttgtcctccaactcctggttggtccgctgggaagccgtgtagctgttctgcagcctgcggaacttatccttaaatttgtccagctcctcgcggctctggcccagctccagctccaggcagtcctgcccaatttccagctcacgttccagggcctcagtgcgtctggtggcggaggccaggcgccggcgaagctcttcattctcctcctgtaagagcttcatcctttctgcatcagtcaggggttcctcctgctcaagccgggatccaggaatttccaaacgcagctcccgatgctctggtggtgccttacggtagggtttcttagcaggggcggcactagtcattctgggaggtgacggctcctccgccgtctgtttgtcggcagctctctctgttccgctgtccgggagttagccctcggctctccgcatcccacggcccctccacttcctttagccacagctccaccagaccctcaggggctttctcccatccggaaaccatgccagat

SEQ ID NO: 19576 - RNA, 2297 nt, Homo sapiens
  source 1..2297: mol_type = other RNA
ttgggctgggctgggttgggctgattggaggaaaggtcttgagacccaactgcatgttacctctgaagaataaatattctaagaaaaagggaaaaccatgaggcaagctgctgcagtcagtcaacgcagctgacaggcctggcatggcccacaacctgaccccatccacacaggaaacagctgtgcgggtctggatagaggagaggtcaagggcttggactggggaccctgagctgccaaggtgtggggactccttgcagtcctggtgcagcaatggcaggaaggccagcaggggccctagttgagcaggttgccctgctcctgggcctgggtcaggctgtccttgcggtgcaggtggtgaacccccatcctcttggggctgcgctgggggcgactggagctggggagtggccaggccctgccctcggtgtgggaagtgcctggcccctcctctgtgcccctgttaatgggcagcaggctctggcgctcttcctcaggactgataggcaggttcagctcttcttcctccctgggaaagccagagtcaggttctgtgggtagcaaaagctcactctcttcgggtcgggcagaaggtgcctggaccacctcatctctgtcagcggggctatgggcaaaatggcgctgcagctcagggagggcatcgcgtccaaaggctgtgcgctgggccacagcagcaggtggtggagtacggtccacaaatgcccgctgccagctgaccagcaggtcctcttcagagctggcagagctagctggggcactgagtgttaggggtgctgggctgggctggtggtggggtgaggcctgggctgaggcaggggtgctgggcactgggctggggcgggcccgctcactcccctcctctaccaggctcagggaaatggcctggcgggtagcgtaagtgcagttgggcagggggctgttgcgggggatccgaaccttatcctcagagaactctattaccctgcggccaggatacagtgggtgtggtggagacggggttgggtaggggttcagcttctcaaaggctggcaggggcagctcttcctccggggagcccctggcagtacccagagagtggcactccccattgggttgtggggtggggctgccaggggccgggggactggctggatcacctgggacaccctcactcatgtccacatgcacaaagacatcctcagccaaggggcgcccggcgctgcctgactgggctgaattgagcagtagagactccggcttctctaacactcgggcaatgactgaggtaggcaccacagcccctggggctaggctgggagcaggacctgggctggcggcctcttgaccactgtgcaaatgtttccgaaccatgtcctgtagctcacagggcagatcggcaaacttgtggtttcggaagtgggacttgttgcacttgaggagctgtacagccaggttgcagtccagccggtaccgctcattgagctcttccagcttgttgatggtgttcttggcatccagcagcttgttggtcagctccacaatctcccagtccagcgtcttcctatccatctcagccttcttgattgcaaaaatccagctgtggctaagagaggccagtgtgtgcagcttgtcctccaactcctggttggtccgctgggaagccgtgtagctgttctgcagcctgcggaacttatccttaaatttgtccagctcctcgcggctctggcccagctccagctccaggcagtcctgcccaatttccagctcacgttccagggcctcagtgcgtctggtggcggaggccaggcgccggcgaagctcttcattctcctcctgtaagagcttcatcctttctgcatcagtcaggggttcctcctgctcaagccgggatccaggaatttccaaacgcagctcccgatgctctggtggtgccttacggtagggtttcttagcaggggcggcactagtcattctgggaggtgacggctcctccgccgtctgtttgtcggcagctctctctgttccgctgtccgggagttagccctcggctctccgcatcccacggcccctccacttcctttagccacagctcccgctctggggttggactggggcaagtcgctatctcttcttctttccaagtaggcactgtaatttcttccagtccctggggcacctgaatcttcagctgaaattggggcagatgctgctaacagctgtggaaaggctgatctaagctttccgccgctgccagctgcgttcaggccgccatcttgccgcggggcaggccgggtagt

SEQ ID NO: 19577 - RNA, 2247 nt, Homo sapiens
  source 1..2247: mol_type = other RNA
ttgggctgggctgggttgggctgattggaggaaaggtcttgagacccaactgcatgttacctctgaagaataaatattctaagaaaaagggaaaaccatgaggcaagctgctgcagtcagtcaacgcagctgacaggcctggcatggcccacaacctgaccccatccacacaggaaacagctgtgcgggtctggatagaggagaggtcaagggcttggactggggaccctgagctgccaaggtgtggggactccttgcagtcctggtgcagcaatggcaggaaggccagcaggggccctagttgagcaggttgccctgctcctgggcctgggtcaggctgtccttgcggtgcaggtggtgaacccccatcctcttggggctgcgctgggggcgactggagctggggagtggccaggccctgccctcggtgtgggaagtgcctggcccctcctctgtgcccctgttaatgggcagcaggctctggcgctcttcctcaggactgataggcaggttcagctcttcttcctccctgggaaagccagagtcaggttctgtgggtagcaaaagctcactctcttcgggtcgggcagaaggtgcctggaccacctcatctctgtcagcggggctatgggcaaaatggcgctgcagctcagggagggcatcgcgtccaaaggctgtgcgctgggccacagcagcaggtggtggagtacggtccacaaatgcccgctgccagctgaccagcaggtcctcttcagagctggcagagctagctggggcactgagtgttaggggtgctgggctgggctggtggtggggtgaggcctgggctgaggcaggggtgctgggcactgggctggggcgggcccgctcactcccctcctctaccaggctcagggaaatggcctggcgggtagcgtaagtgcagttgggcagggggctgttgcgggggatccgaaccttatcctcagagaactctattaccctgcggccaggatacagtgggtgtggtggagacggggttgggtaggggttcagcttctcaaaggctggcaggggcagctcttcctccggggagcccctggcagtacccagagagtggcactccccattgggttgtggggtggggctgccaggggccgggggactggctggatcacctgggacaccctcactcatgtccacatgcacaaagacatcctcagccaaggggcgcccggcgctgcctgactgggctgaattgagcagtagagactccggcttctctaacactcgggcaatgactgaggtaggcaccacagcccctggggctaggctgggagcaggacctgggctggcggcctcttgaccactgtgcaaatgtttccgaaccatgtcctgtagctcacagggcagatcggcaaacttgtggtttcggaagtgggacttgttgcacttgaggagctgtacagccaggttgcagtccagccggtaccgctcattgagctcttccagcttgttgatggtgttcttggcatccagcagcttgttggtcagctccacaatctcccagtccagcgtcttcctatccatctcagccttcttgattgcaaaaatccagctgtggctaagagaggccagtgtgtgcagcttgtcctccaactcctggttggtccgctgggaagccgtgtagctgttctgcagcctgcggaacttatccttaaatttgtccagctcctcgcggctctggcccagctccagctccaggcagtcctgcccaatttccagctcacgttccagggcctcagtgcgtctggtggcggaggccaggcgccggcgaagctcttcattctcctcctgtaagagcttcatcctttctgcatcagtcaggggttcctcctgctcaagccgggatccaggaatttccaaacgcagctcccgatgctctggtggtgccttacggtagggtttcttagcaggggcggcactagtcattctgggaggtgacggctcctccgccgtctgtttgtcggcagctctctctgttccgctgtccgggagttagccctcggctctccgcatcccacggcccctccacttcctttagccacagctcccgctctggggttggactggggcaagtcgctatctcttcttctttccaagtaggcactgtaatttcttccagtccctggggcacctgaatcttcagtttccgccgctgccagctgcgttcaggccgccatcttgccgcggggcaggccgggtagt

SEQ ID NO: 19578 - RNA, 2172 nt, Homo sapiens
  source 1..2172: mol_type = other RNA
ttgggctgggctgggttgggctgattggaggaaaggtcttgagacccaactgcatgttacctctgaagaataaatattctaagaaaaagggaaaaccatgaggcaagctgctgcagtcagtcaacgcagctgacaggcctggcatggcccacaacctgaccccatccacacaggaaacagctgtgcgggtctggatagaggagaggtcaagggcttggactggggaccctgagctgccaaggtgtggggactccttgcagtcctggtgcagcaatggcaggaaggccagcaggggccctagttgagcaggttgccctgctcctgggcctgggtcaggctgtccttgcggtgcaggtggtgaacccccatcctcttggggctgcgctgggggcgactggagctggggagtggccaggccctgccctcggtgtgggaagtgcctggcccctcctctgtgcccctgttaatgggcagcaggctctggcgctcttcctcaggactgataggcaggttcagctcttcttcctccctgggaaagccagagtcaggttctgtgggtagcaaaagctcactctcttcgggtcgggcagaaggtgcctggaccacctcatctctgtcagcggggctatgggcaaaatggcgctgcagctcagggagggcatcgcgtccaaaggctgtgcgctgggccacagcagcaggtggtggagtacggtccacaaatgcccgctgccagctgaccagcaggtcctcttcagagctggcagagctagctggggcactgagtgttaggggtgctgggctgggctggtggtggggtgaggcctgggctgaggcaggggtgctgggcactgggctggggcgggcccgctcactcccctcctctaccaggctcagggaaatggcctggcgggtagcgtaagtgcagttgggcagggggctgttgcgggggatccgaaccttatcctcagagaactctattaccctgcggccaggatacagtgggtgtggtggagacggggttgggtaggggttcagcttctcaaaggctggcaggggcagctcttcctccggggagcccctggcagtacccagagagtggcactccccattgggttgtggggtggggctgccaggggccgggggactggctggatcacctgggacaccctcactcatgtccacatgcacaaagacatcctcagccaaggggcgcccggcgctgcctgactgggctgaattgagcagtagagactccggcttctctaacactcgggcaatgactgaggtaggcaccacagcccctggggctaggctgggagcaggacctgggctggcggcctcttgaccactgtgcaaatgtttccgaaccatgtcctgtagctcacagggcagatcggcaaacttgtggtttcggaagtgggacttgttgcacttgaggagctgtacagccaggttgcagtccagccggtaccgctcattgagctcttccagcttgttgatggtgttcttggcatccagcagcttgttggtcagctccacaatctcccagtccagcgtcttcctatccatctcagccttcttgattgcaaaaatccagctgtggctaagagaggccagtgtgtgcagcttgtcctccaactcctggttggtccgctgggaagccgtgtagctgttctgcagcctgcggaacttatccttaaatttgtccagctcctcgcggctctggcccagctccagctccaggcagtcctgcccaatttccagctcacgttccagggcctcagtgcgtctggtggcggaggccaggcgccggcgaagctcttcattctcctcctgtaagagcttcatcctttctgcatcagtcaggggttcctcctgctcaagccgggatccaggaatttccaaacgcagctcccgatgctctggtggtgccttacggtagggtttcttagcaggggcggcactagtcattctgggaggtgacggctcctccgccgtctgtttgtcggcagctctctctgttccgctgtccgggagttagccctcggctctccgcatcccacggcccctccacttcctttagccacagctctttccgccgctgccagctgcgttcaggccgccatcttgccgcggggcaggccgggtagtggccagggccgcgggaatccc

SEQ ID NO: 19579 - RNA, 2490 nt, Homo sapiens
  source 1..2490: mol_type = other RNA
ttgggctgggctgggttgggctgattggaggaaaggtcttgagacccaactgcatgttacctctgaagaataaatattctaagaaaaagggaaaaccatgaggcaagctgctgcagtcagtcaacgcagctgacaggcctggcatggcccacaacctgaccccatccacacaggaaacagctgtgcgggtctggatagaggagaggtcaagggcttggactggggaccctgagctgccaaggtgtggggactccttgcagtcctggtgcagcaatggcaggaaggccagcaggggccctagttgagcaggttgccctgctcctgggcctgggtcaggctgtccttgcggtgcaggtggtgaacccccatcctcttggggctgcgctgggggcgactggagctggggagtggccaggccctgccctcggtgtgggaagtgcctggcccctcctctgtgcccctgttaatgggcagcaggctctggcgctcttcctcaggactgataggcaggttcagctcttcttcctccctgggaaagccagagtcaggttctgtgggtagcaaaagctcactctcttcgggtcgggcagaaggtgcctggaccacctcatctctgtcagcggggctatgggcaaaatggcgctgcagctcagggagggcatcgcgtccaaaggctgtgcgctgggccacagcagcaggtggtggagtacggtccacaaatgcccgctgccagctgaccagcaggtcctcttcagagctggcagagctagctggggcactgagtgttaggggtgctgggctgggctggtggtggggtgaggcctgggctgaggcaggggtgctgggcactgggctggggcgggcccgctcactcccctcctctaccaggctcagggaaatggcctggcgggtagcgtaagtgcagttgggcagggggctgttgcgggggatccgaaccttatcctcagagaactctattaccctgcggccaggatacagtgggtgtggtggagacggggttgggtaggggttcagcttctcaaaggctggcaggggcagctcttcctccggggagcccctggcagtacccagagagtggcactccccattgggttgtggggtggggctgccaggggccgggggactggctggatcacctgggacaccctcactcatgtccacatgcacaaagacatcctcagccaaggggcgcccggcgctgcctgactgggctgaattgagcagtagagactccggcttctctaacactcgggcaatgactgaggtaggcaccacagcccctggggctaggctgggagcaggacctgggctggcggcctcttgaccactgtgcaaatgtttccgaaccatgtcctgtagctcacagggcagatcggcaaacttgtggtttcggaagtgggacttgttgcacttgaggagctgtacagccaggttgcagtccagccggtaccgctcattgagctcttccagcttgttgatggtgttcttggcatccagcagcttgttggtcagctccacaatctcccagtccagcgtcttcctatccatctcagccttcttgattgcaaaaatccagctgtggctaagagaggccagtgtgtgcagcttgtcctccaactcctggttggtccgctgggaagccgtgtagctgttctgcagcctgcggaacttatccttaaatttgtccagctcctcgcggctctggcccagctccagctccaggcagtcctgcccaatttccagctcacgttccagggcctcagtgcgtctggtggcggaggccaggcgccggcgaagctcttcattctcctcctgtaagagcttcatcctttctgcatcagtcaggggttcctcctgctcaagccgggatccaggaatttccaaacgcagctcccgatgctctggtggtgccttacggtagggtttcttagcaggggcggcactagtcattctgggaggtgacggctcctccgcctgcgtctgtttgtcggcagctctctctgttccgctgtccgggagttagccctcggctctccgcatcccacggcccctccacttcctttagccacagctcagggttagtgtcttctccccaaccagccagctctcctggttagtgcagttagcgacagactcatggcagatgccctccaggcactccatataaacagacagcttggtttgtgagcagcccaactccggagcaaaaaagcaaaagtagacacacagcgagaatgaattcaggagtcagtgacagcaggtacccgctctggggttggactggggcaagtcgctatctcttcttctttccaagtaggcactgtaatttcttccagtccctggggcacctgaatcttcagctgaaattggggcagatgctgctaacagctgtggaaaggctgatctaagctttccgccgctgccagctgcgttcaggccgccatcttgccgcggggcaggccgggtagt

SEQ ID NO: 19580 - RNA, 2271 nt, Homo sapiens
  source 1..2271: mol_type = other RNA
ttgggctgggctgggttgggctgattggaggaaaggtcttgagacccaactgcatgttacctctgaagaataaatattctaagaaaaagggaaaaccatgaggcaagctgctgcagtcagtcaacgcagctgacaggcctggcatggcccacaacctgaccccatccacacaggaaacagctgtgcgggtctggatagaggagaggtcaagggcttggactggggaccctgagctgccaaggtgtggggactccttgcagtcctggtgcagcaatggcaggaaggccagcaggggccctagttgagcaggttgccctgctcctgggcctgggtcaggctgtccttgcggtgcaggtggtgaacccccatcctcttggggctgcgctgggggcgactggagctggggagtggccaggccctgccctcggtgtgggaagtgcctggcccctcctctgtgcccctgttaatgggcagcaggctctggcgctcttcctcaggactgataggcaggttcagctcttcttcctccctgggaaagccagagtcaggttctgtgggtagcaaaagctcactctcttcgggtcgggcagaaggtgcctggaccacctcatctctgtcagcggggctatgggcaaaatggcgctgcagctcagggagggcatcgcgtccaaaggctgtgcgctgggccacagcagcaggtggtggagtacggtccacaaatgcccgctgccagctgaccagcaggtcctcttcagagctggcagagctagctggggcactgagtgttaggggtgctgggctgggctggtggtggggtgaggcctgggctgaggcaggggtgctgggcactgggctggggcgggcccgctcactcccctcctctaccaggctcagggaaatggcctggcgggtagcgtaagtgcagttgggcagggggctgttgcgggggatccgaaccttatcctcagagaactctattaccctgcggccaggatacagtgggtgtggtggagacggggttgggtaggggttcagcttctcaaaggctggcaggggcagctcttcctccggggagcccctggcagtacccagagagtggcactccccattgggttgtggggtggggctgccaggggccgggggactggctggatcacctgggacaccctcactcatgtccacatgcacaaagacatcctcagccaaggggcgcccggcgctgcctgactgggctgaattgagcagtagagactccggcttctctaacactcgggcaatgactgaggtaggcaccacagcccctggggctaggctgggagcaggacctgggctggcggcctcttgaccactgtgcaaatgtttccgaaccatgtcctgtagctcacagggcagatcggcaaacttgtggtttcggaagtgggacttgttgcacttgaggagctgtacagccaggttgcagtccagccggtaccgctcattgagctcttccagcttgttgatggtgttcttggcatccagcagcttgttggtcagctccacaatctcccagtccagcgtcttcctatccatctcagccttcttgattgcaaaaatccagctgtggctaagagaggccagtgtgtgcagcttgtcctccaactcctggttggtccgctgggaagccgtgtagctgttctgcagcctgcggaacttatccttaaatttgtccagctcctcgcggctctggcccagctccagctccaggcagtcctgcccaatttccagctcacgttccagggcctcagtgcgtctggtggcggaggccaggcgccggcgaagctcttcattctcctcctgtaagagcttcatcctttctgcatcagtcaggggttcctcctgctcaagccgggatccaggaatttccaaacgcagctcccgatgctctggtggtgccttacggtagggtttcttagcaggggcggcactagtcattctgggaggtgacggctcctccgcctgcgtctgtttgtcggcagctctctctgttccgctgtccgggagttagccctcggctctccgcatcccacggcccctccacttcctttagccacagctcagggttagtgtcttctccccaaccagccagctctcctggttagtgcagttagcgacagactcatggcagatgccctccaggcactccatataaacagacagcttggtttgtgagcagcccaactccggagcaccagaccctcaggggctttctcccatccggaaaccatgccagat

SEQ ID NO: 19581 - RNA, 2361 nt, Homo sapiens
  source 1..2361: mol_type = other RNA
ttgggctgggctgggttgggctgattggaggaaaggtcttgagacccaactgcatgttacctctgaagaataaatattctaagaaaaagggaaaaccatgaggcaagctgctgcagtcagtcaacgcagctgacaggcctggcatggcccacaacctgaccccatccacacaggaaacagctgtgcgggtctggatagaggagaggtcaagggcttggactggggaccctgagctgccaaggtgtggggactccttgcagtcctggtgcagcaatggcaggaaggccagcaggggccctagttgagcaggttgccctgctcctgggcctgggtcaggctgtccttgcggtgcaggtggtgaacccccatcctcttggggctgcgctgggggcgactggagctggggagtggccaggccctgccctcggtgtgggaagtgcctggcccctcctctgtgcccctgttaatgggcagcaggctctggcgctcttcctcaggactgataggcaggttcagctcttcttcctccctgggaaagccagagtcaggttctgtgggtagcaaaagctcactctcttcgggtcgggcagaaggtgcctggaccacctcatctctgtcagcggggctatgggcaaaatggcgctgcagctcagggagggcatcgcgtccaaaggctgtgcgctgggccacagcagcaggtggtggagtacggtccacaaatgcccgctgccagctgaccagcaggtcctcttcagagctggcagagctagctggggcactgagtgttaggggtgctgggctgggctggtggtggggtgaggcctgggctgaggcaggggtgctgggcactgggctggggcgggcccgctcactcccctcctctaccaggctcagggaaatggcctggcgggtagcgtaagtgcagttgggcagggggctgttgcgggggatccgaaccttatcctcagagaactctattaccctgcggccaggatacagtgggtgtggtggagacggggttgggtaggggttcagcttctcaaaggctggcaggggcagctcttcctccggggagcccctggcagtacccagagagtggcactccccattgggttgtggggtggggctgccaggggccgggggactggctggatcacctgggacaccctcactcatgtccacatgcacaaagacatcctcagccaaggggcgcccggcgctgcctgactgggctgaattgagcagtagagactccggcttctctaacactcgggcaatgactgaggtaggcaccacagcccctggggctaggctgggagcaggacctgggctggcggcctcttgaccactgtgcaaatgtttccgaaccatgtcctgtagctcacagggcagatcggcaaacttgtggtttcggaagtgggacttgttgcacttgaggagctgtacagccaggttgcagtccagccggtaccgctcattgagctcttccagcttgttgatggtgttcttggcatccagcagcttgttggtcagctccacaatctcccagtccagcgtcttcctatccatctcagccttcttgattgcaaaaatccagctgtggctaagagaggccagtgtgtgcagcttgtcctccaactcctggttggtccgctgggaagccgtgtagctgttctgcagcctgcggaacttatccttaaatttgtccagctcctcgcggctctggcccagctccagctccaggcagtcctgcccaatttccagctcacgttccagggcctcagtgcgtctggtggcggaggccaggcgccggcgaagctcttcattctcctcctgtaagagcttcatcctttctgcatcagtcaggggttcctcctgctcaagccgggatccaggaatttccaaacgcagctcccgatgctctggtggtgccttacggtagggtttcttagcaggggcggcactagtcattctgggaggtgacggctcctccgcctgcgtctgtttgtcggcagctctctctgttccgctgtccgggagttagccctcggctctccgcatcccacggcccctccacttcctttagccacagctccaaaaaagcaaaagtagacacacagcgagaatgaattcaggagtcagtgacagcaggtacccgctctggggttggactggggcaagtcgctatctcttcttctttccaagtaggcactgtaatttcttccagtccctggggcacctgaatcttcagctgaaattggggcagatgctgctaacagctgtggaaaggctgatctaagctttccgccgctgccagctgcgttcaggccgccatcttgccgcggggcaggccgggtagtg

SEQ ID NO: 19582 - RNA, 2141 nt, Homo sapiens
  source 1..2141: mol_type = other RNA
ttgggctgggctgggttgggctgattggaggaaaggtcttgagacccaactgcatgttacctctgaagaataaatattctaagaaaaagggaaaaccatgaggcaagctgctgcagtcagtcaacgcagctgacaggcctggcatggcccacaacctgaccccatccacacaggaaacagctgtgcgggtctggatagaggagaggtcaagggcttggactggggaccctgagctgccaaggtgtggggactccttgcagtcctggtgcagcaatggcaggaaggccagcaggggccctagttgagcaggttgccctgctcctgggcctgggtcaggctgtccttgcggtgcaggtggtgaacccccatcctcttggggctgcgctgggggcgactggagctggggagtggccaggccctgccctcggtgtgggaagtgcctggcccctcctctgtgcccctgttaatgggcagcaggctctggcgctcttcctcaggactgataggcaggttcagctcttcttcctccctgggaaagccagagtcaggttctgtgggtagcaaaagctcactctcttcgggtcgggcagaaggtgcctggaccacctcatctctgtcagcggggctatgggcaaaatggcgctgcagctcagggagggcatcgcgtccaaaggctgtgcgctgggccacagcagcaggtggtggagtacggtccacaaatgcccgctgccagctgaccagcaggtcctcttcagagctggcagagctagctggggcactgagtgttaggggtgctgggctgggctggtggtggggtgaggcctgggctgaggcaggggtgctgggcactgggctggggcgggcccgctcactcccctcctctaccaggctcagggaaatggcctggcgggtagcgtaagtgcagttgggcagggggctgttgcgggggatccgaaccttatcctcagagaactctattaccctgcggccaggatacagtgggtgtggtggagacggggttgggtaggggttcagcttctcaaaggctggcaggggcagctcttcctccggggagcccctggcagtacccagagagtggcactccccattgggttgtggggtggggctgccaggggccgggggactggctggatcacctgggacaccctcactcatgtccacatgcacaaagacatcctcagccaaggggcgcccggcgctgcctgactgggctgaattgagcagtagagactccggcttctctaacactcgggcaatgactgaggtaggcaccacagcccctggggctaggctgggagcaggacctgggctggcggcctcttgaccactgtgcaaatgtttccgaaccatgtcctgtagctcacagggcagatcggcaaacttgtggtttcggaagtgggacttgttgcacttgaggagctgtacagccaggttgcagtccagccggtaccgctcattgagctcttccagcttgttgatggtgttcttggcatccagcagcttgttggtcagctccacaatctcccagtccagcgtcttcctatccatctcagccttcttgattgcaaaaatccagctgtggctaagagaggccagtgtgtgcagcttgtcctccaactcctggttggtccgctgggaagccgtgtagctgttctgcagcctgcggaacttatccttaaatttgtccagctcctcgcggctctggcccagctccagctccaggcagtcctgcccaatttccagctcacgttccagggcctcagtgcgtctggtggcggaggccaggcgccggcgaagctcttcattctcctcctgtaagagcttcatcctttctgcatcagtcaggggttcctcctgctcaagccgggatccaggaatttccaaacgcagctcccgatgctctggtggtgccttacggtagggtttcttagcaggggcggcactagtcattctgggaggtgacggctcctccgcctgcgtctgtttgtcggcagctctctctgttccgctgtccgggagttagccctcggctctccgcatcccacggcccctccacttcctttagccacagctccaccagaccctcaggggctttctcccatccggaaaccatgccagat

SEQ ID NO: 19583 - RNA, 2300 nt, Homo sapiens
  source 1..2300: mol_type = other RNA
ttgggctgggctgggttgggctgattggaggaaaggtcttgagacccaactgcatgttacctctgaagaataaatattctaagaaaaagggaaaaccatgaggcaagctgctgcagtcagtcaacgcagctgacaggcctggcatggcccacaacctgaccccatccacacaggaaacagctgtgcgggtctggatagaggagaggtcaagggcttggactggggaccctgagctgccaaggtgtggggactccttgcagtcctggtgcagcaatggcaggaaggccagcaggggccctagttgagcaggttgccctgctcctgggcctgggtcaggctgtccttgcggtgcaggtggtgaacccccatcctcttggggctgcgctgggggcgactggagctggggagtggccaggccctgccctcggtgtgggaagtgcctggcccctcctctgtgcccctgttaatgggcagcaggctctggcgctcttcctcaggactgataggcaggttcagctcttcttcctccctgggaaagccagagtcaggttctgtgggtagcaaaagctcactctcttcgggtcgggcagaaggtgcctggaccacctcatctctgtcagcggggctatgggcaaaatggcgctgcagctcagggagggcatcgcgtccaaaggctgtgcgctgggccacagcagcaggtggtggagtacggtccacaaatgcccgctgccagctgaccagcaggtcctcttcagagctggcagagctagctggggcactgagtgttaggggtgctgggctgggctggtggtggggtgaggcctgggctgaggcaggggtgctgggcactgggctggggcgggcccgctcactcccctcctctaccaggctcagggaaatggcctggcgggtagcgtaagtgcagttgggcagggggctgttgcgggggatccgaaccttatcctcagagaactctattaccctgcggccaggatacagtgggtgtggtggagacggggttgggtaggggttcagcttctcaaaggctggcaggggcagctcttcctccggggagcccctggcagtacccagagagtggcactccccattgggttgtggggtggggctgccaggggccgggggactggctggatcacctgggacaccctcactcatgtccacatgcacaaagacatcctcagccaaggggcgcccggcgctgcctgactgggctgaattgagcagtagagactccggcttctctaacactcgggcaatgactgaggtaggcaccacagcccctggggctaggctgggagcaggacctgggctggcggcctcttgaccactgtgcaaatgtttccgaaccatgtcctgtagctcacagggcagatcggcaaacttgtggtttcggaagtgggacttgttgcacttgaggagctgtacagccaggttgcagtccagccggtaccgctcattgagctcttccagcttgttgatggtgttcttggcatccagcagcttgttggtcagctccacaatctcccagtccagcgtcttcctatccatctcagccttcttgattgcaaaaatccagctgtggctaagagaggccagtgtgtgcagcttgtcctccaactcctggttggtccgctgggaagccgtgtagctgttctgcagcctgcggaacttatccttaaatttgtccagctcctcgcggctctggcccagctccagctccaggcagtcctgcccaatttccagctcacgttccagggcctcagtgcgtctggtggcggaggccaggcgccggcgaagctcttcattctcctcctgtaagagcttcatcctttctgcatcagtcaggggttcctcctgctcaagccgggatccaggaatttccaaacgcagctcccgatgctctggtggtgccttacggtagggtttcttagcaggggcggcactagtcattctgggaggtgacggctcctccgcctgcgtctgtttgtcggcagctctctctgttccgctgtccgggagttagccctcggctctccgcatcccacggcccctccacttcctttagccacagctcccgctctggggttggactggggcaagtcgctatctcttcttctttccaagtaggcactgtaatttcttccagtccctggggcacctgaatcttcagctgaaattggggcagatgctgctaacagctgtggaaaggctgatctaagctttccgccgctgccagctgcgttcaggccgccatcttgccgcggggcaggccgggtagt

SEQ ID NO: 19584 - RNA, 2251 nt, Homo sapiens
  source 1..2251: mol_type = other RNA
ttgggctgggctgggttgggctgattggaggaaaggtcttgagacccaactgcatgttacctctgaagaataaatattctaagaaaaagggaaaaccatgaggcaagctgctgcagtcagtcaacgcagctgacaggcctggcatggcccacaacctgaccccatccacacaggaaacagctgtgcgggtctggatagaggagaggtcaagggcttggactggggaccctgagctgccaaggtgtggggactccttgcagtcctggtgcagcaatggcaggaaggccagcaggggccctagttgagcaggttgccctgctcctgggcctgggtcaggctgtccttgcggtgcaggtggtgaacccccatcctcttggggctgcgctgggggcgactggagctggggagtggccaggccctgccctcggtgtgggaagtgcctggcccctcctctgtgcccctgttaatgggcagcaggctctggcgctcttcctcaggactgataggcaggttcagctcttcttcctccctgggaaagccagagtcaggttctgtgggtagcaaaagctcactctcttcgggtcgggcagaaggtgcctggaccacctcatctctgtcagcggggctatgggcaaaatggcgctgcagctcagggagggcatcgcgtccaaaggctgtgcgctgggccacagcagcaggtggtggagtacggtccacaaatgcccgctgccagctgaccagcaggtcctcttcagagctggcagagctagctggggcactgagtgttaggggtgctgggctgggctggtggtggggtgaggcctgggctgaggcaggggtgctgggcactgggctggggcgggcccgctcactcccctcctctaccaggctcagggaaatggcctggcgggtagcgtaagtgcagttgggcagggggctgttgcgggggatccgaaccttatcctcagagaactctattaccctgcggccaggatacagtgggtgtggtggagacggggttgggtaggggttcagcttctcaaaggctggcaggggcagctcttcctccggggagcccctggcagtacccagagagtggcactccccattgggttgtggggtggggctgccaggggccgggggactggctggatcacctgggacaccctcactcatgtccacatgcacaaagacatcctcagccaaggggcgcccggcgctgcctgactgggctgaattgagcagtagagactccggcttctctaacactcgggcaatgactgaggtaggcaccacagcccctggggctaggctgggagcaggacctgggctggcggcctcttgaccactgtgcaaatgtttccgaaccatgtcctgtagctcacagggcagatcggcaaacttgtggtttcggaagtgggacttgttgcacttgaggagctgtacagccaggttgcagtccagccggtaccgctcattgagctcttccagcttgttgatggtgttcttggcatccagcagcttgttggtcagctccacaatctcccagtccagcgtcttcctatccatctcagccttcttgattgcaaaaatccagctgtggctaagagaggccagtgtgtgcagcttgtcctccaactcctggttggtccgctgggaagccgtgtagctgttctgcagcctgcggaacttatccttaaatttgtccagctcctcgcggctctggcccagctccagctccaggcagtcctgcccaatttccagctcacgttccagggcctcagtgcgtctggtggcggaggccaggcgccggcgaagctcttcattctcctcctgtaagagcttcatcctttctgcatcagtcaggggttcctcctgctcaagccgggatccaggaatttccaaacgcagctcccgatgctctggtggtgccttacggtagggtttcttagcaggggcggcactagtcattctgggaggtgacggctcctccgcctgcgtctgtttgtcggcagctctctctgttccgctgtccgggagttagccctcggctctccgcatcccacggcccctccacttcctttagccacagctcccgctctggggttggactggggcaagtcgctatctcttcttctttccaagtaggcactgtaatttcttccagtccctggggcacctgaatcttcagtttccgccgctgccagctgcgttcaggccgccatcttgccgcggggcaggccgggtagtg

SEQ ID NO: 19585 - RNA, 2154 nt, Homo sapiens
  source 1..2154: mol_type = other RNA
ttgggctgggctgggttgggctgattggaggaaaggtcttgagacccaactgcatgttacctctgaagaataaatattctaagaaaaagggaaaaccatgaggcaagctgctgcagtcagtcaacgcagctgacaggcctggcatggcccacaacctgaccccatccacacaggaaacagctgtgcgggtctggatagaggagaggtcaagggcttggactggggaccctgagctgccaaggtgtggggactccttgcagtcctggtgcagcaatggcaggaaggccagcaggggccctagttgagcaggttgccctgctcctgggcctgggtcaggctgtccttgcggtgcaggtggtgaacccccatcctcttggggctgcgctgggggcgactggagctggggagtggccaggccctgccctcggtgtgggaagtgcctggcccctcctctgtgcccctgttaatgggcagcaggctctggcgctcttcctcaggactgataggcaggttcagctcttcttcctccctgggaaagccagagtcaggttctgtgggtagcaaaagctcactctcttcgggtcgggcagaaggtgcctggaccacctcatctctgtcagcggggctatgggcaaaatggcgctgcagctcagggagggcatcgcgtccaaaggctgtgcgctgggccacagcagcaggtggtggagtacggtccacaaatgcccgctgccagctgaccagcaggtcctcttcagagctggcagagctagctggggcactgagtgttaggggtgctgggctgggctggtggtggggtgaggcctgggctgaggcaggggtgctgggcactgggctggggcgggcccgctcactcccctcctctaccaggctcagggaaatggcctggcgggtagcgtaagtgcagttgggcagggggctgttgcgggggatccgaaccttatcctcagagaactctattaccctgcggccaggatacagtgggtgtggtggagacggggttgggtaggggttcagcttctcaaaggctggcaggggcagctcttcctccggggagcccctggcagtacccagagagtggcactccccattgggttgtggggtggggctgccaggggccgggggactggctggatcacctgggacaccctcactcatgtccacatgcacaaagacatcctcagccaaggggcgcccggcgctgcctgactgggctgaattgagcagtagagactccggcttctctaacactcgggcaatgactgaggtaggcaccacagcccctggggctaggctgggagcaggacctgggctggcggcctcttgaccactgtgcaaatgtttccgaaccatgtcctgtagctcacagggcagatcggcaaacttgtggtttcggaagtgggacttgttgcacttgaggagctgtacagccaggttgcagtccagccggtaccgctcattgagctcttccagcttgttgatggtgttcttggcatccagcagcttgttggtcagctccacaatctcccagtccagcgtcttcctatccatctcagccttcttgattgcaaaaatccagctgtggctaagagaggccagtgtgtgcagcttgtcctccaactcctggttggtccgctgggaagccgtgtagctgttctgcagcctgcggaacttatccttaaatttgtccagctcctcgcggctctggcccagctccagctccaggcagtcctgcccaatttccagctcacgttccagggcctcagtgcgtctggtggcggaggccaggcgccggcgaagctcttcattctcctcctgtaagagcttcatcctttctgcatcagtcaggggttcctcctgctcaagccgggatccaggaatttccaaacgcagctcccgatgctctggtggtgccttacggtagggtttcttagcaggggcggcactagtcattctgggaggtgacggctcctccgcctgcgtctgtttgtcggcagctctctctgttccgctgtccgggagttagccctcggctctccgcatcccacggcccctccacttcctttagccacagctctttccgccgctgccagctgcgttcaggccgccatcttgccgcggggcaggccgggtagt

SEQ ID NO: 19586 - RNA, 2576 nt, Homo sapiens
  source 1..2576: mol_type = other RNA
ttgggctgggctgggttgggctgattggaggaaaggtcttgagacccaactgcatgttacctctgaagaataaatattctaagaaaaagggaaaaccatgaggcaagctgctgcagtcagtcaacgcagctgacaggcctggcatggcccacaacctgaccccatccacacaggaaacagctgtgcgggtctggatagaggagaggtcaagggcttggactggggaccctgagctgccaaggtgtggggactccttgcagtcctggtgcagcaatggcaggaaggccagcaggggccctagttgagcaggttgccctgctcctgggcctgggtcaggctgtccttgcggtgcaggtggtgaacccccatcctcttggggctgcgctgggggcgactggagctggggagtggccaggccctgccctcggtgtgggaagtgcctggcccctcctctgtgcccctgttaatgggcagcaggctctggcgctcttcctcaggactgataggcaggttcagctcttcttcctccctgggaaagccagagtcaggttctgtgggtagcaaaagctcactctcttcgggtcgggcagaaggtgcctggaccacctcatctctgtcagcggggctatgggcaaaatggcgctgcagctcagggagggcatcgcgtccaaaggctgtgcgctgggccacagcagcaggtggtggagtacggtccacaaatgcccgctgccagctgaccagcaggtcctcttcagagctggcagagctagctggggcactgagtgttaggggtgctgggctgggctggtggtggggtgaggcctgggctgaggcaggggtgctgggcactgggctggggcgggcccgctcactcccctcctctaccaggctcagggaaatggcctggcgggtagcgtaagtgcagttgggcagggggctgttgcgggggatccgaaccttatcctcagagaactctattaccctgcggccaggatacagtgggtgtggtggagacggggttgggtaggggttcagcttctcaaaggctggcaggggcagctcttcctccggggagcccctggcagtacccagagagtggcactccccattgggttgtggggtggggctgccaggggccgggggactggctggatcacctgggacaccctcactcatgtccacatgcacaaagacatcctcagccaaggggcgcccggcgctgcctgactgggctgaattgagcagtagagactccggcttctctaacactcgggcaatgactgaggtaggcaccacagcccctggggctaggctgggagcaggacctgggctggcggcctcttgaccactgtgcaaatgtttccgaaccatgtcctgtagctcacagggcagatcggcaaacttgtggtttcggaagtgggacttgttgcacttgaggagctgtacagccaggttgcagtccagccggtaccgctcattgagctcttccagcttgttgatggtgttcttggcatccagcagcttgttggtcagctccacaatctcccagtccagcgtcttcctatccatctcagccttcttgattgcaaaaatccagctgtggctaagagaggccagtgtgtgcagcttgtcctccaactcctggttggtccgctgggaagccgtgtagctgttctgcagcctgcggaacttatccttaaatttgtccagctcctcgcggctctggcccagctccagctccaggcagtcctgcccaatttccagctcacgttccagggcctcagtgcgtctggtggcggaggccaggcgccggcgaagctcttcattctcctcctgtaagagcttcatcctttctgcatcagtcaggggttcctcctgctcaagccgggatccaggaatttccaaacgcagctcccgatgctctggtggtgccttacggtagggtttcttagcaggggcggcactagtcattctgggaggtgacggctcctccgcctgctgagaagcaagaaggaggcaggctcagagatgtggccagaaggactctggacgtctgtttgtcggcagctctctctgttccgctgtccgggagttagccctcggctctccgcatcccacggcccctccacttcctttagccacagctcagggttagtgtcttctccccaaccagccagctctcctggttagtgcagttagcgacagactcatggcagatgccctccaggcactccatataaacagacagcttggtttgtgagcagcccaactccggagcaaaaaagcaaaagtagacacacagcgagaatgaattcaggagtcagtgacagcaggtacccgctctggggttggactggggcaagtcgctatctcttcttctttccaagtaggcactgtaatttcttccagtccctggggcacctgaatcttcagctgaaattggggcagatgctgctaacagctgtggaaaggctgatctaagctttccgccgctgccagctgcgttcaggccgccatcttgccgcggggcaggccgggtagtggccagggccgcgggaatccccacgcacttggcg

SEQ ID NO: 19587 - RNA, 2497 nt, Homo sapiens
  source 1..2497: mol_type = other RNA
ttgggctgggctgggttgggctgattggaggaaaggtcttgagacccaactgcatgttacctctgaagaataaatattctaagaaaaagggaaaaccatgaggcaagctgctgcagtcagtcaacgcagctgacaggcctggcatggcccacaacctgaccccatccacacaggaaacagctgtgcgggtctggatagaggagaggtcaagggcttggactggggaccctgagctgccaaggtgtggggactccttgcagtcctggtgcagcaatggcaggaaggccagcaggggccctagttgagcaggttgccctgctcctgggcctgggtcaggctgtccttgcggtgcaggtggtgaacccccatcctcttggggctgcgctgggggcgactggagctggggagtggccaggccctgccctcggtgtgggaagtgcctggcccctcctctgtgcccctgttaatgggcagcaggctctggcgctcttcctcaggactgataggcaggttcagctcttcttcctccctgggaaagccagagtcaggttctgtgggtagcaaaagctcactctcttcgggtcgggcagaaggtgcctggaccacctcatctctgtcagcggggctatgggcaaaatggcgctgcagctcagggagggcatcgcgtccaaaggctgtgcgctgggccacagcagcaggtggtggagtacggtccacaaatgcccgctgccagctgaccagcaggtcctcttcagagctggcagagctagctggggcactgagtgttaggggtgctgggctgggctggtggtggggtgaggcctgggctgaggcaggggtgctgggcactgggctggggcgggcccgctcactcccctcctctaccaggctcagggaaatggcctggcgggtagcgtaagtgcagttgggcagggggctgttgcgggggatccgaaccttatcctcagagaactctattaccctgcggccaggatacagtgggtgtggtggagacggggttgggtaggggttcagcttctcaaaggctggcaggggcagctcttcctccggggagcccctggcagtacccagagagtggcactccccattgggttgtggggtggggctgccaggggccgggggactggctggatcacctgggacaccctcactcatgtccacatgcacaaagacatcctcagccaaggggcgcccggcgctgcctgactgggctgaattgagcagtagagactccggcttctctaacactcgggcaatgactgaggtaggcaccacagcccctggggctaggctgggagcaggacctgggctggcggcctcttgaccactgtgcaaatgtttccgaaccatgtcctgtagctcacagggcagatcggcaaacttgtggtttcggaagtgggacttgttgcacttgaggagctgtacagccaggttgcagtccagccggtaccgctcattgagctcttccagcttgttgatggtgttcttggcatccagcagcttgttggtcagctccacaatctcccagtccagcgtcttcctatccatctcagccttcttgattgcaaaaatccagctgtggctaagagaggccagtgtgtgcagcttgtcctccaactcctggttggtccgctgggaagccgtgtagctgttctgcagcctgcggaacttatccttaaatttgtccagctcctcgcggctctggcccagctccagctccaggcagtcctgcccaatttccagctcacgttccagggcctcagtgcgtctggtggcggaggccaggcgccggcgaagctcttcattctcctcctgtaagagcttcatcctttctgcatcagtcaggggttcctcctgctcaagccgggatccaggaatttccaaacgcagctcccgatgctctggtggtgccttacggtagggtttcttagcaggggcggcactagtcattctgggaggtgacggctcctccgcctgctgagaagcaagaaggaggcaggctcagagatgtggccagaaggactctggacgtctgtttgtcggcagctctctctgttccgctgtccgggagttagccctcggctctccgcatcccacggcccctccacttcctttagccacagctcagggttagtgtcttctccccaaccagccagctctcctggttagtgcagttagcgacagactcatggcagatgccctccaggcactccatataaacagacagcttggtttgtgagcagcccaactccggagcaccagaccctcaggggctttctcccatccggaaaccatgccagatggaagccaagcactccccctgccaaccagggaggccagcttgctgacctcaggcaaaaagcctctctggttggtcaacagaaagagaggacggctgttggagaaggggctcagctcctctatctcgcctgttccccaaacactgctgccaggctgcaccaggactctgaaagct

SEQ ID NO: 19588 - RNA, 2522 nt, Homo sapiens
  source 1..2522: mol_type = other RNA
ttgggctgggctgggttgggctgattggaggaaaggtcttgagacccaactgcatgttacctctgaagaataaatattctaagaaaaagggaaaaccatgaggcaagctgctgcagtcagtcaacgcagctgacaggcctggcatggcccacaacctgaccccatccacacaggaaacagctgtgcgggtctggatagaggagaggtcaagggcttggactggggaccctgagctgccaaggtgtggggactccttgcagtcctggtgcagcaatggcaggaaggccagcaggggccctagttgagcaggttgccctgctcctgggcctgggtcaggctgtccttgcggtgcaggtggtgaacccccatcctcttggggctgcgctgggggcgactggagctggggagtggccaggccctgccctcggtgtgggaagtgcctggcccctcctctgtgcccctgttaatgggcagcaggctctggcgctcttcctcaggactgataggcaggttcagctcttcttcctccctgggaaagccagagtcaggttctgtgggtagcaaaagctcactctcttcgggtcgggcagaaggtgcctggaccacctcatctctgtcagcggggctatgggcaaaatggcgctgcagctcagggagggcatcgcgtccaaaggctgtgcgctgggccacagcagcaggtggtggagtacggtccacaaatgcccgctgccagctgaccagcaggtcctcttcagagctggcagagctagctggggcactgagtgttaggggtgctgggctgggctggtggtggggtgaggcctgggctgaggcaggggtgctgggcactgggctggggcgggcccgctcactcccctcctctaccaggctcagggaaatggcctggcgggtagcgtaagtgcagttgggcagggggctgttgcgggggatccgaaccttatcctcagagaactctattaccctgcggccaggatacagtgggtgtggtggagacggggttgggtaggggttcagcttctcaaaggctggcaggggcagctcttcctccggggagcccctggcagtacccagagagtggcactccccattgggttgtggggtggggctgccaggggccgggggactggctggatcacctgggacaccctcactcatgtccacatgcacaaagacatcctcagccaaggggcgcccggcgctgcctgactgggctgaattgagcagtagagactccggcttctctaacactcgggcaatgactgaggtaggcaccacagcccctggggctaggctgggagcaggacctgggctggcggcctcttgaccactgtgcaaatgtttccgaaccatgtcctgtagctcacagggcagatcggcaaacttgtggtttcggaagtgggacttgttgcacttgaggagctgtacagccaggttgcagtccagccggtaccgctcattgagctcttccagcttgttgatggtgttcttggcatccagcagcttgttggtcagctccacaatctcccagtccagcgtcttcctatccatctcagccttcttgattgcaaaaatccagctgtggctaagagaggccagtgtgtgcagcttgtcctccaactcctggttggtccgctgggaagccgtgtagctgttctgcagcctgcggaacttatccttaaatttgtccagctcctcgcggctctggcccagctccagctccaggcagtcctgcccaatttccagctcacgttccagggcctcagtgcgtctggtggcggaggccaggcgccggcgaagctcttcattctcctcctgtaagagcttcatcctttctgcatcagtcaggggttcctcctgctcaagccgggatccaggaatttccaaacgcagctcccgatgctctggtggtgccttacggtagggtttcttagcaggggcggcactagtcattctgggaggtgacggctcctccgcctgctgagaagcaagaaggaggcaggctcagagatgtggccagaaggactctggacgtctgtttgtcggcagctctctctgttccgctgtccgggagttagccctcggctctccgcatcccacggcccctccacttcctttagccacagctccaaaaaagcaaaagtagacacacagcgagaatgaattcaggagtcagtgacagcaggtacccgctctggggttggactggggcaagtcgctatctcttcttctttccaagtaggcactgtaatttcttccagtccctggggcacctgaatcttcagctgaaattggggcagatgctgctaacagctgtggaaaggctgatctaagcctagaagagggtcatttgactggctttagttccctccttagcagatctgcccggcatcctccagatctctcttcctcactatcccactctactagaaagatccctttcccctctggccggccagatacagtcgggcctctatcccacgctccaggcttctttattcgcg

SEQ ID NO: 19589 - RNA, 2412 nt, Homo sapiens
  source 1..2412: mol_type = other RNA
ttgggctgggctgggttgggctgattggaggaaaggtcttgagacccaactgcatgttacctctgaagaataaatattctaagaaaaagggaaaaccatgaggcaagctgctgcagtcagtcaacgcagctgacaggcctggcatggcccacaacctgaccccatccacacaggaaacagctgtgcgggtctggatagaggagaggtcaagggcttggactggggaccctgagctgccaaggtgtggggactccttgcagtcctggtgcagcaatggcaggaaggccagcaggggccctagttgagcaggttgccctgctcctgggcctgggtcaggctgtccttgcggtgcaggtggtgaacccccatcctcttggggctgcgctgggggcgactggagctggggagtggccaggccctgccctcggtgtgggaagtgcctggcccctcctctgtgcccctgttaatgggcagcaggctctggcgctcttcctcaggactgataggcaggttcagctcttcttcctccctgggaaagccagagtcaggttctgtgggtagcaaaagctcactctcttcgggtcgggcagaaggtgcctggaccacctcatctctgtcagcggggctatgggcaaaatggcgctgcagctcagggagggcatcgcgtccaaaggctgtgcgctgggccacagcagcaggtggtggagtacggtccacaaatgcccgctgccagctgaccagcaggtcctcttcagagctggcagagctagctggggcactgagtgttaggggtgctgggctgggctggtggtggggtgaggcctgggctgaggcaggggtgctgggcactgggctggggcgggcccgctcactcccctcctctaccaggctcagggaaatggcctggcgggtagcgtaagtgcagttgggcagggggctgttgcgggggatccgaaccttatcctcagagaactctattaccctgcggccaggatacagtgggtgtggtggagacggggttgggtaggggttcagcttctcaaaggctggcaggggcagctcttcctccggggagcccctggcagtacccagagagtggcactccccattgggttgtggggtggggctgccaggggccgggggactggctggatcacctgggacaccctcactcatgtccacatgcacaaagacatcctcagccaaggggcgcccggcgctgcctgactgggctgaattgagcagtagagactccggcttctctaacactcgggcaatgactgaggtaggcaccacagcccctggggctaggctgggagcaggacctgggctggcggcctcttgaccactgtgcaaatgtttccgaaccatgtcctgtagctcacagggcagatcggcaaacttgtggtttcggaagtgggacttgttgcacttgaggagctgtacagccaggttgcagtccagccggtaccgctcattgagctcttccagcttgttgatggtgttcttggcatccagcagcttgttggtcagctccacaatctcccagtccagcgtcttcctatccatctcagccttcttgattgcaaaaatccagctgtggctaagagaggccagtgtgtgcagcttgtcctccaactcctggttggtccgctgggaagccgtgtagctgttctgcagcctgcggaacttatccttaaatttgtccagctcctcgcggctctggcccagctccagctccaggcagtcctgcccaatttccagctcacgttccagggcctcagtgcgtctggtggcggaggccaggcgccggcgaagctcttcattctcctcctgtaagagcttcatcctttctgcatcagtcaggggttcctcctgctcaagccgggatccaggaatttccaaacgcagctcccgatgctctggtggtgccttacggtagggtttcttagcaggggcggcactagtcattctgggaggtgacggctcctccgcctgctgagaagcaagaaggaggcaggctcagagatgtggccagaaggactctggacgtctgtttgtcggcagctctctctgttccgctgtccgggagttagccctcggctctccgcatcccacggcccctccacttcctttagccacagctccaaaaaagcaaaagtagacacacagcgagaatgaattcaggagtcagtgacagcaggtacccgctctggggttggactggggcaagtcgctatctcttcttctttccaagtaggcactgtaatttcttccagtccctggggcacctgaatcttcagctgaaattggggcagatgctgctaacagctgtggaaaggctgatctaagctttccgccgctgccagctgcgttcaggccgccatcttgccgcggggcaggccgggtagt

SEQ ID NO: 19590 - RNA, 2193 nt, Homo sapiens
  source 1..2193: mol_type = other RNA
ttgggctgggctgggttgggctgattggaggaaaggtcttgagacccaactgcatgttacctctgaagaataaatattctaagaaaaagggaaaaccatgaggcaagctgctgcagtcagtcaacgcagctgacaggcctggcatggcccacaacctgaccccatccacacaggaaacagctgtgcgggtctggatagaggagaggtcaagggcttggactggggaccctgagctgccaaggtgtggggactccttgcagtcctggtgcagcaatggcaggaaggccagcaggggccctagttgagcaggttgccctgctcctgggcctgggtcaggctgtccttgcggtgcaggtggtgaacccccatcctcttggggctgcgctgggggcgactggagctggggagtggccaggccctgccctcggtgtgggaagtgcctggcccctcctctgtgcccctgttaatgggcagcaggctctggcgctcttcctcaggactgataggcaggttcagctcttcttcctccctgggaaagccagagtcaggttctgtgggtagcaaaagctcactctcttcgggtcgggcagaaggtgcctggaccacctcatctctgtcagcggggctatgggcaaaatggcgctgcagctcagggagggcatcgcgtccaaaggctgtgcgctgggccacagcagcaggtggtggagtacggtccacaaatgcccgctgccagctgaccagcaggtcctcttcagagctggcagagctagctggggcactgagtgttaggggtgctgggctgggctggtggtggggtgaggcctgggctgaggcaggggtgctgggcactgggctggggcgggcccgctcactcccctcctctaccaggctcagggaaatggcctggcgggtagcgtaagtgcagttgggcagggggctgttgcgggggatccgaaccttatcctcagagaactctattaccctgcggccaggatacagtgggtgtggtggagacggggttgggtaggggttcagcttctcaaaggctggcaggggcagctcttcctccggggagcccctggcagtacccagagagtggcactccccattgggttgtggggtggggctgccaggggccgggggactggctggatcacctgggacaccctcactcatgtccacatgcacaaagacatcctcagccaaggggcgcccggcgctgcctgactgggctgaattgagcagtagagactccggcttctctaacactcgggcaatgactgaggtaggcaccacagcccctggggctaggctgggagcaggacctgggctggcggcctcttgaccactgtgcaaatgtttccgaaccatgtcctgtagctcacagggcagatcggcaaacttgtggtttcggaagtgggacttgttgcacttgaggagctgtacagccaggttgcagtccagccggtaccgctcattgagctcttccagcttgttgatggtgttcttggcatccagcagcttgttggtcagctccacaatctcccagtccagcgtcttcctatccatctcagccttcttgattgcaaaaatccagctgtggctaagagaggccagtgtgtgcagcttgtcctccaactcctggttggtccgctgggaagccgtgtagctgttctgcagcctgcggaacttatccttaaatttgtccagctcctcgcggctctggcccagctccagctccaggcagtcctgcccaatttccagctcacgttccagggcctcagtgcgtctggtggcggaggccaggcgccggcgaagctcttcattctcctcctgtaagagcttcatcctttctgcatcagtcaggggttcctcctgctcaagccgggatccaggaatttccaaacgcagctcccgatgctctggtggtgccttacggtagggtttcttagcaggggcggcactagtcattctgggaggtgacggctcctccgcctgctgagaagcaagaaggaggcaggctcagagatgtggccagaaggactctggacgtctgtttgtcggcagctctctctgttccgctgtccgggagttagccctcggctctccgcatcccacggcccctccacttcctttagccacagctccaccagaccctcaggggctttctcccatccggaaaccatgccagat

SEQ ID NO: 19591 - RNA, 2399 nt, Homo sapiens
  source 1..2399: mol_type = other RNA
ttgggctgggctgggttgggctgattggaggaaaggtcttgagacccaactgcatgttacctctgaagaataaatattctaagaaaaagggaaaaccatgaggcaagctgctgcagtcagtcaacgcagctgacaggcctggcatggcccacaacctgaccccatccacacaggaaacagctgtgcgggtctggatagaggagaggtcaagggcttggactggggaccctgagctgccaaggtgtggggactccttgcagtcctggtgcagcaatggcaggaaggccagcaggggccctagttgagcaggttgccctgctcctgggcctgggtcaggctgtccttgcggtgcaggtggtgaacccccatcctcttggggctgcgctgggggcgactggagctggggagtggccaggccctgccctcggtgtgggaagtgcctggcccctcctctgtgcccctgttaatgggcagcaggctctggcgctcttcctcaggactgataggcaggttcagctcttcttcctccctgggaaagccagagtcaggttctgtgggtagcaaaagctcactctcttcgggtcgggcagaaggtgcctggaccacctcatctctgtcagcggggctatgggcaaaatggcgctgcagctcagggagggcatcgcgtccaaaggctgtgcgctgggccacagcagcaggtggtggagtacggtccacaaatgcccgctgccagctgaccagcaggtcctcttcagagctggcagagctagctggggcactgagtgttaggggtgctgggctgggctggtggtggggtgaggcctgggctgaggcaggggtgctgggcactgggctggggcgggcccgctcactcccctcctctaccaggctcagggaaatggcctggcgggtagcgtaagtgcagttgggcagggggctgttgcgggggatccgaaccttatcctcagagaactctattaccctgcggccaggatacagtgggtgtggtggagacggggttgggtaggggttcagcttctcaaaggctggcaggggcagctcttcctccggggagcccctggcagtacccagagagtggcactccccattgggttgtggggtggggctgccaggggccgggggactggctggatcacctgggacaccctcactcatgtccacatgcacaaagacatcctcagccaaggggcgcccggcgctgcctgactgggctgaattgagcagtagagactccggcttctctaacactcgggcaatgactgaggtaggcaccacagcccctggggctaggctgggagcaggacctgggctggcggcctcttgaccactgtgcaaatgtttccgaaccatgtcctgtagctcacagggcagatcggcaaacttgtggtttcggaagtgggacttgttgcacttgaggagctgtacagccaggttgcagtccagccggtaccgctcattgagctcttccagcttgttgatggtgttcttggcatccagcagcttgttggtcagctccacaatctcccagtccagcgtcttcctatccatctcagccttcttgattgcaaaaatccagctgtggctaagagaggccagtgtgtgcagcttgtcctccaactcctggttggtccgctgggaagccgtgtagctgttctgcagcctgcggaacttatccttaaatttgtccagctcctcgcggctctggcccagctccagctccaggcagtcctgcccaatttccagctcacgttccagggcctcagtgcgtctggtggcggaggccaggcgccggcgaagctcttcattctcctcctgtaagagcttcatcctttctgcatcagtcaggggttcctcctgctcaagccgggatccaggaatttccaaacgcagctcccgatgctctggtggtgccttacggtagggtttcttagcaggggcggcactagtcattctgggaggtgacggctcctccgcctgctgagaagcaagaaggaggcaggctcagagatgtggccagaaggactctggacgtctgtttgtcggcagctctctctgttccgctgtccgggagttagccctcggctctccgcatcccacggcccctccacttcctttagccacagctcccgctctggggttggactggggcaagtcgctatctcttcttctttccaagtaggcactgtaatttcttccagtccctggggcacctgaatcttcagctgaaattggggcagatgctgctaacagctgtggaaaggctgatctaagctttccgccgctgccagctgcgttcaggccgccatcttgccgcggggcaggccgggtagtggccagggccgcgggaatccccacgcacttggcgtgtcgcgtcatct

SEQ ID NO: 19592 - RNA, 2301 nt, Homo sapiens
  source 1..2301: mol_type = other RNA
ttgggctgggctgggttgggctgattggaggaaaggtcttgagacccaactgcatgttacctctgaagaataaatattctaagaaaaagggaaaaccatgaggcaagctgctgcagtcagtcaacgcagctgacaggcctggcatggcccacaacctgaccccatccacacaggaaacagctgtgcgggtctggatagaggagaggtcaagggcttggactggggaccctgagctgccaaggtgtggggactccttgcagtcctggtgcagcaatggcaggaaggccagcaggggccctagttgagcaggttgccctgctcctgggcctgggtcaggctgtccttgcggtgcaggtggtgaacccccatcctcttggggctgcgctgggggcgactggagctggggagtggccaggccctgccctcggtgtgggaagtgcctggcccctcctctgtgcccctgttaatgggcagcaggctctggcgctcttcctcaggactgataggcaggttcagctcttcttcctccctgggaaagccagagtcaggttctgtgggtagcaaaagctcactctcttcgggtcgggcagaaggtgcctggaccacctcatctctgtcagcggggctatgggcaaaatggcgctgcagctcagggagggcatcgcgtccaaaggctgtgcgctgggccacagcagcaggtggtggagtacggtccacaaatgcccgctgccagctgaccagcaggtcctcttcagagctggcagagctagctggggcactgagtgttaggggtgctgggctgggctggtggtggggtgaggcctgggctgaggcaggggtgctgggcactgggctggggcgggcccgctcactcccctcctctaccaggctcagggaaatggcctggcgggtagcgtaagtgcagttgggcagggggctgttgcgggggatccgaaccttatcctcagagaactctattaccctgcggccaggatacagtgggtgtggtggagacggggttgggtaggggttcagcttctcaaaggctggcaggggcagctcttcctccggggagcccctggcagtacccagagagtggcactccccattgggttgtggggtggggctgccaggggccgggggactggctggatcacctgggacaccctcactcatgtccacatgcacaaagacatcctcagccaaggggcgcccggcgctgcctgactgggctgaattgagcagtagagactccggcttctctaacactcgggcaatgactgaggtaggcaccacagcccctggggctaggctgggagcaggacctgggctggcggcctcttgaccactgtgcaaatgtttccgaaccatgtcctgtagctcacagggcagatcggcaaacttgtggtttcggaagtgggacttgttgcacttgaggagctgtacagccaggttgcagtccagccggtaccgctcattgagctcttccagcttgttgatggtgttcttggcatccagcagcttgttggtcagctccacaatctcccagtccagcgtcttcctatccatctcagccttcttgattgcaaaaatccagctgtggctaagagaggccagtgtgtgcagcttgtcctccaactcctggttggtccgctgggaagccgtgtagctgttctgcagcctgcggaacttatccttaaatttgtccagctcctcgcggctctggcccagctccagctccaggcagtcctgcccaatttccagctcacgttccagggcctcagtgcgtctggtggcggaggccaggcgccggcgaagctcttcattctcctcctgtaagagcttcatcctttctgcatcagtcaggggttcctcctgctcaagccgggatccaggaatttccaaacgcagctcccgatgctctggtggtgccttacggtagggtttcttagcaggggcggcactagtcattctgggaggtgacggctcctccgcctgctgagaagcaagaaggaggcaggctcagagatgtggccagaaggactctggacgtctgtttgtcggcagctctctctgttccgctgtccgggagttagccctcggctctccgcatcccacggcccctccacttcctttagccacagctcccgctctggggttggactggggcaagtcgctatctcttcttctttccaagtaggcactgtaatttcttccagtccctggggcacctgaatcttcagtttccgccgctgccagctgcgttcaggccgccatcttgccgcggggcaggccgggtag

SEQ ID NO: 19593 - RNA, 2207 nt, Homo sapiens
  source 1..2207: mol_type = other RNA
ttgggctgggctgggttgggctgattggaggaaaggtcttgagacccaactgcatgttacctctgaagaataaatattctaagaaaaagggaaaaccatgaggcaagctgctgcagtcagtcaacgcagctgacaggcctggcatggcccacaacctgaccccatccacacaggaaacagctgtgcgggtctggatagaggagaggtcaagggcttggactggggaccctgagctgccaaggtgtggggactccttgcagtcctggtgcagcaatggcaggaaggccagcaggggccctagttgagcaggttgccctgctcctgggcctgggtcaggctgtccttgcggtgcaggtggtgaacccccatcctcttggggctgcgctgggggcgactggagctggggagtggccaggccctgccctcggtgtgggaagtgcctggcccctcctctgtgcccctgttaatgggcagcaggctctggcgctcttcctcaggactgataggcaggttcagctcttcttcctccctgggaaagccagagtcaggttctgtgggtagcaaaagctcactctcttcgggtcgggcagaaggtgcctggaccacctcatctctgtcagcggggctatgggcaaaatggcgctgcagctcagggagggcatcgcgtccaaaggctgtgcgctgggccacagcagcaggtggtggagtacggtccacaaatgcccgctgccagctgaccagcaggtcctcttcagagctggcagagctagctggggcactgagtgttaggggtgctgggctgggctggtggtggggtgaggcctgggctgaggcaggggtgctgggcactgggctggggcgggcccgctcactcccctcctctaccaggctcagggaaatggcctggcgggtagcgtaagtgcagttgggcagggggctgttgcgggggatccgaaccttatcctcagagaactctattaccctgcggccaggatacagtgggtgtggtggagacggggttgggtaggggttcagcttctcaaaggctggcaggggcagctcttcctccggggagcccctggcagtacccagagagtggcactccccattgggttgtggggtggggctgccaggggccgggggactggctggatcacctgggacaccctcactcatgtccacatgcacaaagacatcctcagccaaggggcgcccggcgctgcctgactgggctgaattgagcagtagagactccggcttctctaacactcgggcaatgactgaggtaggcaccacagcccctggggctaggctgggagcaggacctgggctggcggcctcttgaccactgtgcaaatgtttccgaaccatgtcctgtagctcacagggcagatcggcaaacttgtggtttcggaagtgggacttgttgcacttgaggagctgtacagccaggttgcagtccagccggtaccgctcattgagctcttccagcttgttgatggtgttcttggcatccagcagcttgttggtcagctccacaatctcccagtccagcgtcttcctatccatctcagccttcttgattgcaaaaatccagctgtggctaagagaggccagtgtgtgcagcttgtcctccaactcctggttggtccgctgggaagccgtgtagctgttctgcagcctgcggaacttatccttaaatttgtccagctcctcgcggctctggcccagctccagctccaggcagtcctgcccaatttccagctcacgttccagggcctcagtgcgtctggtggcggaggccaggcgccggcgaagctcttcattctcctcctgtaagagcttcatcctttctgcatcagtcaggggttcctcctgctcaagccgggatccaggaatttccaaacgcagctcccgatgctctggtggtgccttacggtagggtttcttagcaggggcggcactagtcattctgggaggtgacggctcctccgcctgctgagaagcaagaaggaggcaggctcagagatgtggccagaaggactctggacgtctgtttgtcggcagctctctctgttccgctgtccgggagttagccctcggctctccgcatcccacggcccctccacttcctttagccacagctctttccgccgctgccagctgcgttcaggccgccatcttgccgcggggcaggccgggtagtg

SEQ ID NO: 19594 - RNA, 2333 nt, Homo sapiens
  source 1..2333: mol_type = other RNA
ttgggctgggctgggttgggctgattggaggaaaggtcttgagacccaactgcatgttacctctgaagaataaatattctaagaaaaagggaaaaccatgaggcaagctgctgcagtcagtcaacgcagctgacaggcctggcatggcccacaacctgaccccatccacacaggaaacagctgtgcgggtctggatagaggagaggtcaagggcttggactggggaccctgagctgccaaggtgtggggactccttgcagtcctggtgcagcaatggcaggaaggccagcaggggccctagttgagcaggttgccctgctcctgggcctgggtcaggctgtccttgcggtgcaggtggtgaacccccatcctcttggggctgcgctgggggcgactggagctggggagtggccaggccctgccctcggtgtgggaagtgcctggcccctcctctgtgcccctgttaatgggcagcaggctctggcgctcttcctcaggactgataggcaggttcagctcttcttcctccctgggaaagccagagtcaggttctgtgggtagcaaaagctcactctcttcgggtcgggcagaaggtgcctggaccacctcatctctgtcagcggggctatgggcaaaatggcgctgcagctcagggagggcatcgcgtccaaaggctgtgcgctgggccacagcagcaggtggtggagtacggtccacaaatgcccgctgccagctgaccagcaggtcctcttcagagctggcagagctagctggggcactgagtgttaggggtgctgggctgggctggtggtggggtgaggcctgggctgaggcaggggtgctgggcactgggctggggcgggcccgctcactcccctcctctaccaggctcagggaaatggcctggcgggtagcgtaagtgcagttgggcagggggctgttgcgggggatccgaaccttatcctcagagaactctattaccctgcggccaggatacagtgggtgtggtggagacggggttgggtaggggttcagcttctcaaaggctggcaggggcagctcttcctccggggagcccctggcagtacccagagagtggcactccccattgggttgtggggtggggctgccaggggccgggggactggctggatcacctgggacaccctcactcatgtccacatgcacaaagacatcctcagccaaggggcgcccggcgctgcctgactgggctgaattgagcagtagagactccggcttctctaacactcgggcaatgactgaggtaggcaccacagcccctggggctaggctgggagcaggacctgggctggcggcctcttgaccactgtgcaaatgtttccgaaccatgtcctgtagctcacagggcagatcggcaaacttgtggtttcggaagtgggacttgttgcacttgaggagctgtacagccaggttgcagtccagccggtaccgctcattgagctcttccagcttgttgatggtgttcttggcatccagcagcttgttggtcagctccacaatctcccagtccagcgtcttcctatccatctcagccttcttgattgcaaaaatccagctgtggctaagagaggccagtgtgtgcagcttgtcctccaactcctggttggtccgctgggaagccgtgtagctgttctgcagcctgcggaacttatccttaaatttgtccagctcctcgcggctctggcccagctccagctccaggcagtcctgcccaatttccagctcacgttccagggcctcagtgcgtctggtggcggaggccaggcgccggcgaagctcttcattctcctcctgtaagagcttcatcctttctgcatcagtcaggggttcctctgccggtcaggctgtgataccagtcttgctgacctcctgctcaagccgggatccaggaatttccaaacgcagctcccgatgctctggtggtgccttacggtagggtttcttagcaggggcggcactagtcattctgggaggtgacggctcctccgccgtctgtttgtcggcagctctctctgttccgctgtccgggagttagccctcggctctccgcatcccacggcccctccacttcctttagccacagctcccgctctggggttggactggggcaagtcgctatctcttcttctttccaagtaggcactgtaatttcttccagtccctggggcacctgaatcttcagctgaaattggggcagatgctgctaacagctgtggaaaggctgatctaagctttccgccgctgccagctgcgttcaggccgccatcttgccgcggggcaggccgggtagt

SEQ ID NO: 19595 - RNA, 2307 nt, Homo sapiens
  source 1..2307: mol_type = other RNA
ttgggctgggctgggttgggctgattggaggaaaggtcttgagacccaactgcatgttacctctgaagaataaatattctaagaaaaagggaaaaccatgaggcaagctgctgcagtcagtcaacgcagctgacaggcctggcatggcccacaacctgaccccatccacacaggaaacagctgtgcgggtctggatagaggagaggtcaagggcttggactggggaccctgagctgccaaggtgtggggactccttgcagtcctggtgcagcaatggcaggaaggccagcaggggccctagttgagcaggttgccctgctcctgggcctgggtcaggctgtccttgcggtgcaggtggtgaacccccatcctcttggggctgcgctgggggcgactggagctggggagtggccaggccctgccctcggtgtgggaagtgcctggcccctcctctgtgcccctgttaatgggcagcaggctctggcgctcttcctcaggactgataggcaggttcagctcttcttcctccctgggaaagccagagtcaggttctgtgggtagcaaaagctcactctcttcgggtcgggcagaaggtgcctggaccacctcatctctgtcagcggggctatgggcaaaatggcgctgcagctcagggagggcatcgcgtccaaaggctgtgcgctgggccacagcagcaggtggtggagtacggtccacaaatgcccgctgccagctgaccagcaggtcctcttcagagctggcagagctagctggggcactgagtgttaggggtgctgggctgggctggtggtggggtgaggcctgggctgaggcaggggtgctgggcactgggctggggcgggcccgctcactcccctcctctaccaggctcagggaaatggcctggcgggtagcgtaagtgcagttgggcagggggctgttgcgggggatccgaaccttatcctcagagaactctattaccctgcggccaggatacagtgggtgtggtggagacggggttgggtaggggttcagcttctcaaaggctggcaggggcagctcttcctccggggagcccctggcagtacccagagagtggcactccccattgggttgtggggtggggctgccaggggccgggggactggctggatcacctgggacaccctcactcatgtccacatgcacaaagacatcctcagccaaggggcgcccggcgctgcctgactgggctgaattgagcagtagagactccggcttctctaacactcgggcaatgactgaggtaggcaccacagcccctggggctaggctgggagcaggacctgggctggcggcctcttgaccactgtgcaaatgtttccgaaccatgtcctgtagctcacagggcagatcggcaaacttgtggtttcggaagtgggacttgttgcacttgaggagctgtacagccaggttgcagtccagccggtaccgctcattgagctcttccagcttgttgatggtgttcttggcatccagcagcttgttggtcagctccacaatctcccagtccagcgtcttcctatccatctcagccttcttgattgcaaaaatccagctgtggctaagagaggccagtgtgtgcagcttgtcctccaactcctggttggtccgctgggaagccgtgtagctgttctgcagcctgcggaacttatccttaaatttgtccagctcctcgcggctctggcccagctccagctccaggcagtcctgcccaatttccagctcacgttccagggcctcagtgcgtctggtggcggaggccaggcgccggcgaagctcttcattctcctcctgtaagagcttcatcctttctgcatcagtcaggggttcctctgccggtcaggctgtgataccagtcttgctgacctcctgctcaagccgggatccaggaatttccaaacgcagctcccgatgctctggtggtgccttacggtagggtttcttagcaggggcggcactagtcattctgggaggtgacggctcctccgccgtctgtttgtcggcagctctctctgttccgctgtccgggagttagccctcggctctccgcatcccacggcccctccacttcctttagccacagctcccgctctggggttggactggggcaagtcgctatctcttcttctttccaagtaggcactgtaatttcttccagtccctggggcacctgaatcttcagtttccgccgctgccagctgcgttcaggccgccatcttgccgcggggcaggccgggtagtggccagggccgcgggaatccccac

SEQ ID NO: 19596 - RNA, 2187 nt, Homo sapiens
  source 1..2187: mol_type = other RNA
ttgggctgggctgggttgggctgattggaggaaaggtcttgagacccaactgcatgttacctctgaagaataaatattctaagaaaaagggaaaaccatgaggcaagctgctgcagtcagtcaacgcagctgacaggcctggcatggcccacaacctgaccccatccacacaggaaacagctgtgcgggtctggatagaggagaggtcaagggcttggactggggaccctgagctgccaaggtgtggggactccttgcagtcctggtgcagcaatggcaggaaggccagcaggggccctagttgagcaggttgccctgctcctgggcctgggtcaggctgtccttgcggtgcaggtggtgaacccccatcctcttggggctgcgctgggggcgactggagctggggagtggccaggccctgccctcggtgtgggaagtgcctggcccctcctctgtgcccctgttaatgggcagcaggctctggcgctcttcctcaggactgataggcaggttcagctcttcttcctccctgggaaagccagagtcaggttctgtgggtagcaaaagctcactctcttcgggtcgggcagaaggtgcctggaccacctcatctctgtcagcggggctatgggcaaaatggcgctgcagctcagggagggcatcgcgtccaaaggctgtgcgctgggccacagcagcaggtggtggagtacggtccacaaatgcccgctgccagctgaccagcaggtcctcttcagagctggcagagctagctggggcactgagtgttaggggtgctgggctgggctggtggtggggtgaggcctgggctgaggcaggggtgctgggcactgggctggggcgggcccgctcactcccctcctctaccaggctcagggaaatggcctggcgggtagcgtaagtgcagttgggcagggggctgttgcgggggatccgaaccttatcctcagagaactctattaccctgcggccaggatacagtgggtgtggtggagacggggttgggtaggggttcagcttctcaaaggctggcaggggcagctcttcctccggggagcccctggcagtacccagagagtggcactccccattgggttgtggggtggggctgccaggggccgggggactggctggatcacctgggacaccctcactcatgtccacatgcacaaagacatcctcagccaaggggcgcccggcgctgcctgactgggctgaattgagcagtagagactccggcttctctaacactcgggcaatgactgaggtaggcaccacagcccctggggctaggctgggagcaggacctgggctggcggcctcttgaccactgtgcaaatgtttccgaaccatgtcctgtagctcacagggcagatcggcaaacttgtggtttcggaagtgggacttgttgcacttgaggagctgtacagccaggttgcagtccagccggtaccgctcattgagctcttccagcttgttgatggtgttcttggcatccagcagcttgttggtcagctccacaatctcccagtccagcgtcttcctatccatctcagccttcttgattgcaaaaatccagctgtggctaagagaggccagtgtgtgcagcttgtcctccaactcctggttggtccgctgggaagccgtgtagctgttctgcagcctgcggaacttatccttaaatttgtccagctcctcgcggctctggcccagctccagctccaggcagtcctgcccaatttccagctcacgttccagggcctcagtgcgtctggtggcggaggccaggcgccggcgaagctcttcattctcctcctgtaagagcttcatcctttctgcatcagtcaggggttcctctgccggtcaggctgtgataccagtcttgctgacctcctgctcaagccgggatccaggaatttccaaacgcagctcccgatgctctggtggtgccttacggtagggtttcttagcaggggcggcactagtcattctgggaggtgacggctcctccgccgtctgtttgtcggcagctctctctgttccgctgtccgggagttagccctcggctctccgcatcccacggcccctccacttcctttagccacagctctttccgccgctgccagctgcgttcaggccgccatcttgccgcggggcaggccgggtagt

SEQ ID NO: 19597 - RNA, 2336 nt, Homo sapiens
  source 1..2336: mol_type = other RNA
ttgggctgggctgggttgggctgattggaggaaaggtcttgagacccaactgcatgttacctctgaagaataaatattctaagaaaaagggaaaaccatgaggcaagctgctgcagtcagtcaacgcagctgacaggcctggcatggcccacaacctgaccccatccacacaggaaacagctgtgcgggtctggatagaggagaggtcaagggcttggactggggaccctgagctgccaaggtgtggggactccttgcagtcctggtgcagcaatggcaggaaggccagcaggggccctagttgagcaggttgccctgctcctgggcctgggtcaggctgtccttgcggtgcaggtggtgaacccccatcctcttggggctgcgctgggggcgactggagctggggagtggccaggccctgccctcggtgtgggaagtgcctggcccctcctctgtgcccctgttaatgggcagcaggctctggcgctcttcctcaggactgataggcaggttcagctcttcttcctccctgggaaagccagagtcaggttctgtgggtagcaaaagctcactctcttcgggtcgggcagaaggtgcctggaccacctcatctctgtcagcggggctatgggcaaaatggcgctgcagctcagggagggcatcgcgtccaaaggctgtgcgctgggccacagcagcaggtggtggagtacggtccacaaatgcccgctgccagctgaccagcaggtcctcttcagagctggcagagctagctggggcactgagtgttaggggtgctgggctgggctggtggtggggtgaggcctgggctgaggcaggggtgctgggcactgggctggggcgggcccgctcactcccctcctctaccaggctcagggaaatggcctggcgggtagcgtaagtgcagttgggcagggggctgttgcgggggatccgaaccttatcctcagagaactctattaccctgcggccaggatacagtgggtgtggtggagacggggttgggtaggggttcagcttctcaaaggctggcaggggcagctcttcctccggggagcccctggcagtacccagagagtggcactccccattgggttgtggggtggggctgccaggggccgggggactggctggatcacctgggacaccctcactcatgtccacatgcacaaagacatcctcagccaaggggcgcccggcgctgcctgactgggctgaattgagcagtagagactccggcttctctaacactcgggcaatgactgaggtaggcaccacagcccctggggctaggctgggagcaggacctgggctggcggcctcttgaccactgtgcaaatgtttccgaaccatgtcctgtagctcacagggcagatcggcaaacttgtggtttcggaagtgggacttgttgcacttgaggagctgtacagccaggttgcagtccagccggtaccgctcattgagctcttccagcttgttgatggtgttcttggcatccagcagcttgttggtcagctccacaatctcccagtccagcgtcttcctatccatctcagccttcttgattgcaaaaatccagctgtggctaagagaggccagtgtgtgcagcttgtcctccaactcctggttggtccgctgggaagccgtgtagctgttctgcagcctgcggaacttatccttaaatttgtccagctcctcgcggctctggcccagctccagctccaggcagtcctgcccaatttccagctcacgttccagggcctcagtgcgtctggtggcggaggccaggcgccggcgaagctcttcattctcctcctgtaagagcttcatcctttctgcatcagtcaggggttcctctgccggtcaggctgtgataccagtcttgctgacctcctgctcaagccgggatccaggaatttccaaacgcagctcccgatgctctggtggtgccttacggtagggtttcttagcaggggcggcactagtcattctgggaggtgacggctcctccgcctgcgtctgtttgtcggcagctctctctgttccgctgtccgggagttagccctcggctctccgcatcccacggcccctccacttcctttagccacagctcccgctctggggttggactggggcaagtcgctatctcttcttctttccaagtaggcactgtaatttcttccagtccctggggcacctgaatcttcagctgaaattggggcagatgctgctaacagctgtggaaaggctgatctaagctttccgccgctgccagctgcgttcaggccgccatcttgccgcggggcaggccgggtagt

SEQ ID NO: 19598 - RNA, 2388 nt, Homo sapiens
  source 1..2388: mol_type = other RNA
ttgggctgggctgggttgggctgattggaggaaaggtcttgagacccaactgcatgttacctctgaagaataaatattctaagaaaaagggaaaaccatgaggcaagctgctgcagtcagtcaacgcagctgacaggcctggcatggcccacaacctgaccccatccacacaggaaacagctgtgcgggtctggatagaggagaggtcaagggcttggactggggaccctgagctgccaaggtgtggggactccttgcagtcctggtgcagcaatggcaggaaggccagcaggggccctagttgagcaggttgccctgctcctgggcctgggtcaggctgtccttgcggtgcaggtggtgaacccccatcctcttggggctgcgctgggggcgactggagctggggagtggccaggccctgccctcggtgtgggaagtgcctggcccctcctctgtgcccctgttaatgggcagcaggctctggcgctcttcctcaggactgataggcaggttcagctcttcttcctccctgggaaagccagagtcaggttctgtgggtagcaaaagctcactctcttcgggtcgggcagaaggtgcctggaccacctcatctctgtcagcggggctatgggcaaaatggcgctgcagctcagggagggcatcgcgtccaaaggctgtgcgctgggccacagcagcaggtggtggagtacggtccacaaatgcccgctgccagctgaccagcaggtcctcttcagagctggcagagctagctggggcactgagtgttaggggtgctgggctgggctggtggtggggtgaggcctgggctgaggcaggggtgctgggcactgggctggggcgggcccgctcactcccctcctctaccaggctcagggaaatggcctggcgggtagcgtaagtgcagttgggcagggggctgttgcgggggatccgaaccttatcctcagagaactctattaccctgcggccaggatacagtgggtgtggtggagacggggttgggtaggggttcagcttctcaaaggctggcaggggcagctcttcctccggggagcccctggcagtacccagagagtggcactccccattgggttgtggggtggggctgccaggggccgggggactggctggatcacctgggacaccctcactcatgtccacatgcacaaagacatcctcagccaaggggcgcccggcgctgcctgactgggctgaattgagcagtagagactccggcttctctaacactcgggcaatgactgaggtaggcaccacagcccctggggctaggctgggagcaggacctgggctggcggcctcttgaccactgtgcaaatgtttccgaaccatgtcctgtagctcacagggcagatcggcaaacttgtggtttcggaagtgggacttgttgcacttgaggagctgtacagccaggttgcagtccagccggtaccgctcattgagctcttccagcttgttgatggtgttcttggcatccagcagcttgttggtcagctccacaatctcccagtccagcgtcttcctatccatctcagccttcttgattgcaaaaatccagctgtggctaagagaggccagtgtgtgcagcttgtcctccaactcctggttggtccgctgggaagccgtgtagctgttctgcagcctgcggaacttatccttaaatttgtccagctcctcgcggctctggcccagctccagctccaggcagtcctgcccaatttccagctcacgttccagggcctcagtgcgtctggtggcggaggccaggcgccggcgaagctcttcattctcctcctgtaagagcttcatcctttctgcatcagtcaggggttcctctgccggtcaggctgtgataccagtcttgctgacctcctgctcaagccgggatccaggaatttccaaacgcagctcccgatgctctggtggtgccttacggtagggtttcttagcaggggcggcactagtcattctgggaggtgacggctcctccgcctgctgagaagcaagaaggaggcaggctcagagatgtggccagaaggactctggacgtctgtttgtcggcagctctctctgttccgctgtccgggagttagccctcggctctccgcatcccacggcccctccacttcctttagccacagctcccgctctggggttggactggggcaagtcgctatctcttcttctttccaagtaggcactgtaatttcttccagtccctggggcacctgaatcttcagctgaaattggggcagatgctgctaacagctgtggaaaggctgatctaagctttccgccgctgccagctgcgttcaggccgccatcttgccgcggggcaggccgggtagt

SEQ ID NO: 19599 - RNA, 2347 nt, Homo sapiens
  source 1..2347: mol_type = other RNA
ttgggctgggctgggttgggctgattggaggaaaggtcttgagacccaactgcatgttacctctgaagaataaatattctaagaaaaagggaaaaccatgaggcaagctgctgcagtcagtcaacgcagctgacaggcctggcatggcccacaacctgaccccatccacacaggaaacagctgtgcgggtctggatagaggagaggtcaagggcttggactggggaccctgagctgccaaggtgtggggactccttgcagtcctggtgcagcaatggcaggaaggccagcaggggccctagttgagcaggttgccctgctcctgggcctgggtcaggctgtccttgcggtgcaggtggtgaacccccatcctcttggggctgcgctgggggcgactggagctggggagtggccaggccctgccctcggtgtgggaagtgcctggcccctcctctgtgcccctgttaatgggcagcaggctctggcgctcttcctcaggactgataggcaggttcagctcttcttcctccctgggaaagccagagtcaggttctgtgggtagcaaaagctcactctcttcgggtcgggcagaaggtgcctggaccacctcatctctgtcagcggggctatgggcaaaatggcgctgcagctcagggagggcatcgcgtccaaaggctgtgcgctgggccacagcagcaggtggtggagtacggtccacaaatgcccgctgccagctgaccagcaggtcctcttcagagctggcagagctagctggggcactgagtgttaggggtgctgggctgggctggtggtggggtgaggcctgggctgaggcaggggtgctgggcactgggctggggcgggcccgctcactcccctcctctaccaggctcagggaaatggcctggcgggtagcgtaagtgcagttgggcagggggctgttgcgggggatccgaaccttatcctcagagaactctattaccctgcggccaggatacagtgggtgtggtggagacggggttgggtaggggttcagcttctcaaaggctggcaggggcagctcttcctccggggagcccctggcagtacccagagagtggcactccccattgggttgtggggtggggctgccaggggccgggggactggctggatcacctgggacaccctcactcatgtccacatgcacaaagacatcctcagccaaggggcgcccggcgctgcctgactgggctgaattgagcagtagagactccggcttctctaacactcgggcaatgactgaggtaggcaccacagcccctggggctaggctgggagcaggacctgggctggcggcctcttgaccactgtgcaaatgtttccgaaccatgtcctgtagctcacagggcagctctgtgtactcagcactctgctatctcctgttcttacagcatgccagtgtgtataccctcacttcacagacacataggcatcggcaaacttgtggtttcggaagtgggacttgttgcacttgaggagctgtacagccaggttgcagtccagccggtaccgctcattgagctcttccagcttgttgatggtgttcttggcatccagcagcttgttggtcagctccacaatctcccagtccagcgtcttcctatccatctcagccttcttgatcagtgtgtgcagcttgtcctccaactcctggttggtccgctgggaagccgtgtagctgttctgcagcctgcggaacttatccttaaatttgtccagctcctcgcggctctggcccagctccagctccaggcagtcctgcccaatttccagctcacgttccagggcctcagtgcgtctggtggcggaggccaggcgccggcgaagctcttcattctcctcctgtaagagcttcatcctttctgcatcagtcaggggttcctcctgctcaagccgggatccaggaatttccaaacgcagctcccgatgctctggtggtgccttacggtagggtttcttagcaggggcggcactagtcattctgggaggtgacggctcctccgccgtctgtttgtcggcagctctctctgttccgctgtccgggagttagccctcggctctccgcatcccacggcccctccacttcctttagccacagctcccgctctggggttggactggggcaagtcgctatctcttcttctttccaagtaggcactgtaatttcttccagtccctggggcacctgaatcttcagctgaaattggggcagatgctgctaacagctgtggaaaggctgatctaagctttccgccgctgccagctgcgttcaggccgccatcttgccgcggggcaggccgggtagt

SEQ ID NO: 19600 - RNA, 4079 nt, Homo sapiens
  source 1..4079: mol_type = other RNA
ttgggctgggctgggttggggaccagccggcagttgtctggtccagggggcaccaggtctgggataccatcattgtcatcatcatcatcacactcgtcaccaattccatccttatcggtgtccagctgggcactgttaatgacggtggggcagttgtctgtgctgtcctggtgcccatctccatcactgcaggagaaaggacaggtgatgtggctcacagttcagcagggaacaggaaggatccatttttaggaaggagagtctgtgcttgaggttttttttaaaccagggttggctcttaaaatcaaacccactggggtcattcccttagataaggctgccctatgggcctcagagacaattttcccatccccaacctcttaaaacaagtgagtcatttcctactaaagaagataagggtctatttctatgatttatgaccagatgctcctatcagtcagtccctgggaactgctagatgatactcaactcagaggatgtgtgaggggaacaatgacaggcagtggaaccagacagcctcagtgtaaatcctggctcagccactgtgcccagcgtgtgacctcaggcatgacacctgacctctctatggctcagtgtcctcatctgtaaaatgagaatagtacctacctcatagagttgttatggagattaaatgatgaaaatcagaatgttgcatattaaatttcaatatatgaaaaagtgctgactcttaggaagccctacagtgttttccgttatattactcttcacaatccctggctagtggatccaatgaggattcagacctgaacgccatggggagaagggcaaagtgaacagggccacgccttctcgaggagagtgtgtaggccgggctcagtgctggtctaaaggacttctcagaactctccttctctgtccacctgactttctgggctgaggggccacctgaagatgagtctgccctgcctccaagaggtgtcctggagtctgagacctctcatggttactctggaaaagaatgagcactcctttagacctggtccacctgcggcctgtcctgggccaggagctgcccctgcacccttttggagagggaagccagggaccagaccatgctctagggccacacctaccacatggtacagggggacagaaagggtccagtgaaagtgaagtcagccttgacaagcagaaaatgatgtggctcaaacagcagaatccctgtgcatgcagcaggtctgctttataaaacacaagactgagctatttccattagcagccgttctatgtagccctgaacatttttatgcaaaaacaagcagttcctatcctcttctccaaggttcaactttgtgggaattaaaacatagcagaatgagtcatttgttttgggcaaatatctagaggctggtgggacaggatattttagaaattaatgtagatagtagtcagagtgcaagatgacctgcaccagggaacattcttgacgcacatcatttagggcagttgtcaggatacagtcccaccttcctctcggaagaggagagggacatctgatgtcaggctctgttgctgatgtgcctttccttgtactgtgataccaataataacacggcccctgttttctgcatgtcacccttgggccagcactgtgccgggagctttacctacattatcttgatttttcaccataacctgtgcgatgcatttatttatctcctctttgcagatgaagaagttgagatgtgaagagactgggaaatatgtttaagttcacttagctagtacagtcaggcctctgtatccgcggttccgtatccgcagattcaaccaacttgggttgcaggtgccgctagggctgagtgacacacgtctgtttttggtgatgttcttccagaatctgatcagttgatccagccttgagtcttaatgtgggactccatcgtgttgagctaggagggttcacaaaactcacttccacagaacaattccactgtcctgattggtgtcacaggagtccccaaccagatcattatccacatcagactggttagggttgctgacatcaggacaactgtcacaggcatcccccacaccatcaccatccttgtcccgttggtcacgattgggaaattttgggcagttgtccagaatgttttttattccatctccatccatgtcatcatcacaggcatctcctcttccatccccatcggtgtctttctggtcgttatttaagacactcaggcagttatcacaggcatccccaaagatatctttatcgctgttcctttggtccacattatgaatcaggacacagttatcctgctcattcaggatcccatctccgtcagcatcctcgtcacaagcgtcgccaatgccatctctgtctgcatcttcttggccagaatttggcacatatttgcagttgtcctttttacagttcctggcagagcatggcagttcttcgtcggggtaactgtcgatgtccacatcctttccacagatatagccatctccagcccaaccgactccacacacacatgtcacatccccctgcctctcttcaatgcactgggcattcacactgcaagggttcagctctgggtttctgcagtttctttccgctttgcatccccttatctgatcaccagtataccccggcttacaaggcccacagcggtaagatcccaaagtattaacgcagatcgagttgggaacgcacgctccatttcgacactcatcaatgtcagtgcagacctgcttgtttgacttggcaaaactgatcccaacaccctgcaccatgggccctgtgaagcccactgggcaggcgtcacatctgaagccaggagacaaatttatgcagtgcacgcccgggtagcagggatggtatttgcactcatcaacatcaatacaggtgatcccgtttcctgtgtagccctcggggcagggcccacactggaagccatctctactgtcggtacattggacacctcggaaacatgggttggagtcacaccgacgaggtgggcgtgttggcggtgcagggggagccgggggcaccaccgtgcttggggtcggagactgaaacttgagaggaccgcaagcctggcattcagctatggtgtttcgcaaaaatgatgtttccttaacctgctgtctcagaaggtccttcacctctcccaggagttggtttaattgtgtcatttgacccaagaactgccggttaaagtcccctgtgcctgtggcagccagtggctcactctgctgcaggaagcagtcttgcaggctggccacctggaacagtgagcctctcaccaccagcttcagctcttccaagaagtcctgtggcttcctctggaaagtcctcaattcaatggtctcaggtttctgggaggggccagcaaaggccctggggagattgtgaacggaatccacctggatgcagtccaggtagagctctagggagccggcccctcgctgcaaattgctcagcctcaggaggatcctgtgccgccttccgtctgccagctgcaggttgttgaaaaccaccaaatgcaccttcccatcgttcttcaggtaacggaggatggctttgtttaagcgtcccatcacagtaaattcaaaatatttactgttgtcagttgaagagtaaagaccgaagatggtggctgaacttttagtctgcagcttgaaggtggaaatcacatagagatcattcagggcggggtctgtcaggactggcagcagagcgcctgggtttagcctctgactggaagatgggagaaggtcaaagacctggggggtggcctgggcgcctgccgctagccaccgctgcaggaccaggtgcagcaggaggacggcggctccgcgcggggccagcatgttggctcttcctgctccccgcgaggccgggggcgacggcggcgttggccccgcctgggggtccccgggccgtgcgttgaacctcggtcggcgcccgggccggcgccgcaggtgacccgtgctcggcgtccgggctgccgtcgggggcgcgctcgcgtccccgccgtgcggtgctggggagctggctgctg

SEQ ID NO: 19601 - RNA, 2167 nt, Homo sapiens
  source 1..2167: mol_type = other RNA
ttgggctgggctgggttggggaccagccggcagttgtctggtccagggggcaccaggtctgggataccatcattgtcatcatcatcatcacactcgtcaccaattccatccttatcggtgtccagctgggcactgttaatgacggtggggcagttgtctgtgctgtcctggtgcccatctccatcactgtcctgattggtgtcacaggagtccccaaccagatcattatccacatcagactggttagggttgctgacatcaggacaactgtcacaggcatcccccacaccatcaccatccttgtcccgttggtcacgattgggaaattttgggcagttgtccagaatgttttttattccatctccatccatgtcatcatcacaggcatctcctcttccatccccatcggtgtctttctggtcgttatttaagacactcaggcagttatcacaggcatccccaaagatatctttatcgctgttcctttggtccacattatgaatcaggacacagttatcctgctcattcaggatcccatctccgtcagcatcctcgtcacaagcgtcgccaatgccatctctgtctgcatcttcttggccagaatttggcacatatttgcagttgtcctttttacagttcctggcagagcatggcagttcttcgtcggggtaactgtcgatgtccacatcctttccacagatatagccatctccagcccaaccgactccacacacacatgtcacatccccctgcctctcttcaatgcactgggcattcacactgcaagggttcagctctgggtttctgcagtttctttccgctttgcatccccttatctgatcaccagtataccccggcttacaaggcccacagcggtaagatcccaaagtattaacgcagatcgagttgggaacgcacgctccatttcgacactcatcaatgtcagtgcagacctgcttgtttgacttggcaaaactgatcccaacaccctgcaccatgggccctgtgaagcccactgggcaggcgtcacatctgaagccaggagacaaatttatgcagtgcacgcccgggtagcagggatggtatttgcactcatcaacatcaatacaggtgatcccgtttcctgtgtagccctcggggcagggcccacactggaagccatctctactgtcggtacattggacacctcggaaacatgggttggagtcacaccgacgaggtgggcgtgttggcggtgcagggggagccgggggcaccaccgtgcttggggtcggagactgaaacttgagaggaccgcaagcctggcattcagctatggtgtttcgcaaaaatgatgtttccttaacctgctgtctcagaaggtccttcacctctcccaggagttggtttaattgtgtcatttgacccaagaactgccggttaaagtcccctgtgcctgtggcagccagtggctcactctgctgcaggaagcagtcttgcaggctggccacctggaacagtgagcctctcaccaccagcttcagctcttccaagaagtcctgtggcttcctctggaaagtcctcaattcaatggtctcaggtttctgggaggggccagcaaaggccctggggagattgtgaacggaatccacctggatgcagtccaggtagagctctagggagccggcccctcgctgcaaattgctcagcctcaggaggatcctgtgccgccttccgtctgccagctgcaggttgttgaaaaccaccaaatgcaccttcccatcgttcttcaggtaacggaggatggctttgtttaagcgtcccatcacagtaaattcaaaatatttactgttgtcagttgaagagtaaagaccgaagatggtggctgaacttttagtctgcagcttgaaggtggaaatcacatagagatcattcagggcggggtctgtcaggactggcagcagagcgcctgggtttagcctctgactggaagatgggagaaggtcaaagaaactccacaggctctacaggaaacatggctgagggggtctcagaaaacttacgatcatggtggaaggcgaaggcaaagcaggcacgtcccacacagcctttaggccaagctgctcctaagagttcttcttaatccctccagtcgttgtttctctcatctctcaagagcccccaaatt

SEQ ID NO: 19602 - RNA, 2268 nt, Homo sapiens
  source 1..2268: mol_type = other RNA
ttgggctgggctgggttggggaccagccggcagttgtctggtccagggggcaccaggtctgggataccatcattgtcatcatcatcatcacactcgtcaccaattccatccttatcggtgtccagctgggcactgttaatgacggtggggcagttgtctgtgctgtcctggtgcccatctccatcactgtcctgattggtgtcacaggagtccccaaccagatcattatccacatcagactggttagggttgctgacatcaggacaactgtcacaggcatcccccacaccatcaccatccttgtcccgttggtcacgattgggaaattttgggcagttgtccagaatgttttttattccatctccatccatgtcatcatcacaggcatctcctcttccatccccatcggtgtctttctggtcgttatttaagacactcaggcagttatcacaggcatccccaaagatatctttatcgctgttcctttggtccacattatgaatcaggacacagttatcctgctcattcaggatcccatctccgtcagcatcctcgtcacaagcgtcgccaatgccatctctgtctgcatcttcttggccagaatttggcacatatttgcagttgtcctttttacagttcctggcagagcatggcagttcttcgtcggggtaactgtcgatgtccacatcctttccacagatatagccatctccagcccaaccgactccacacacacatgtcacatccccctgcctctcttcaatgcactgggcattcacactgcaagggttcagctctgggtttctgcagtttctttccgctttgcatccccttatctgatcaccagtataccccggcttacaaggcccacagcggtaagatcccaaagtattaacgcagatcgagttgggaacgcacgctccatttcgacactcatcaatgtcagtgcagacctgcttgtttgacttggcaaaactgatcccaacaccctgcaccatgggccctgtgaagcccactgggcaggcgtcacatctgaagccaggagacaaatttatgcagtgcacgcccgggtagcagggatggtatttgcactcatcaacatcaatacaggtgatcccgtttcctgtgtagccctcggggcagggcccacactggaagccatctctactgtcggtacattggacacctcggaaacatgggttggagtcacaccgacgaggtgggcgtgttggcggtgcagggggagccgggggcaccaccgtgcttggggtcggagactgaaacttgagaggaccgcaagcctggcattcagctatggtgtttcgcaaaaatgatgtttccttaacctgctgtctcagaaggtccttcacctctcccaggagttggtttaattgtgtcatttgacccaagaactgccggttaaagtcccctgtgcctgtggcagccagtggctcactctgctgcaggaagcagtcttgcaggctggccacctggaacagtgagcctctcaccaccagcttcagctcttccaagaagtcctgtggcttcctctggaaagtcctcaattcaatggtctcaggtttctgggaggggccagcaaaggccctggggagattgtgaacggaatccacctggatgcagtccaggtagagctctagggagccggcccctcgctgcaaattgctcagcctcaggaggatcctgtgccgccttccgtctgccagctgcaggttgttgaaaaccaccaaatgcaccttcccatcgttcttcaggtaacggaggatggctttgtttaagcgtcccatcacagtaaattcaaaatatttactgttgtcagttgaagagtaaagaccgaagatggtggctgaacttttagtctgcagcttgaaggtggaaatcacatagagatcattcagggcggggtctgtcaggactggcagcagagcgcctgggtttagcctctgactggaagatgggagaaggtcaaagacctggggggtggcctgggcgcctgccgctagccaccgctgcaggaccaggtgcagcaggaggacggcggctccgcgcggggccagcatgttggctcttcctgctccccgcgaggccgggggcgacggcggcgttggccccgcctgggggtccccgggccgtgcgttgaacctcggtcggcgcccgggccggcgccgcaggtgacccgtgctcggcgtccgggctgccgtcgggggcgcgctcgcgtccccgccgtgcggtgctggggagctggctgct

SEQ ID NO: 19603 - RNA, 2145 nt, Homo sapiens
  source 1..2145: mol_type = other RNA
ttgggctgggctgggttggggaccagccggcagttgtctggtccagggggcaccaggtctgggataccatcattgtcatcatcatcatcacactcgtcaccaattccatccttatcggtgtccagctgggcactgttaatgacggtggggcagttgtctgtgctgtcctggtgcccatctccatcactgtcctgattggtgtcacaggagtccccaaccagatcattatccacatcagactggttagggttgctgacatcaggacaactgtcacaggcatcccccacaccatcaccatccttgtcccgttggtcacgattgggaaattttgggcagttgtccagaatgttttttattccatctccatccatgtcatcatcacaggcatctcctcttccatccccatcggtgtctttctggtcgttatttaagacactcaggcagttatcacaggcatccccaaagatatctttatcgctgttcctttggtccacattatgaatcaggacacagttatcctgctcattcaggatcccatctccgtcagcatcctcgtcacaagcgtcgccaatgccatctctgtctgcatcttcttggccagaatttggcacatatttgcagttgtcctttttacagttcctggcagagcatggcagttcttcgtcggggtaactgtcgatgtccacatcctttccacagatatagccatctccagcccaaccgactccacacacacatgtcacatccccctgcctctcttcaatgcactgggcattcacactgcaagggttcagctctgggtttctgcagtttctttccgctttgcatccccttatctgatcaccagtataccccggcttacaaggcccacagcggtaagatcccaaagtattaacgcagatcgagttgggaacgcacgctccatttcgacactcatcaatgtcagtgcagacctgcttgtttgacttggcaaaactgatcccaacaccctgcaccatgggccctgtgaagcccactgggcaggcgtcacatctgaagccaggagacaaatttatgcagtgcacgcccgggtagcagggatggtatttgcactcatcaacatcaatacaggtgatcccgtttcctgtgtagccctcggggcagggcccacactggaagccatctctactgtcggtacattggacacctcggaaacatgggttggagtcacaccgacgaggtgggcgtgttggcggtgcagggggagccgggggcaccaccgtgcttggggtcggagactgaaacttgagaggaccgcaagcctggcattcagctatggtgtttcgcaaaaatgatgtttccttaacctgctgtctcagaaggtccttcacctctcccaggagttggtttaattgtgtcatttgacccaagaactgccggttaaagtcccctgtgcctgtggcagccagtggctcactctgctgcaggaagcagtcttgcaggctggccacctggaacagtgagcctctcaccaccagcttcagctcttccaagaagtcctgtggcttcctctggaaagtcctcaattcaatggtctcaggtttctgggaggggccagcaaaggccctggggagattgtgaacggaatccacctggatgcagtccaggtagagctctagggagccggcccctcgctgcaaattgctcagcctcaggaggatcctgtgccgccttccgtctgccagctgcaggttgttgaaaaccaccaaatgcaccttcccatcgttcttcaggtaacggaggatggctttgtttaagcgtcccatcacagtaaattcaaaatatttactgttgtcagttgaagagtaaagaccgaagatggtggctgaacttttagtctgcagcttgaaggtggaaatcacatagagatcattcagggcggggtctgtcaggactggcagcagagcgcctgggtttagcctctgactggaagatgggagaaggtcaaagactcagaaattaagacatcaagccaatccttgaaataaactttctttttgtcgttcaagcaaagtcagagcagaaaatgcaggtggcagggcaagtagagtaattctgcgtctttctcagggatgtcaagagcagactctgggcatacatcgctcc

SEQ ID NO: 19604 - RNA, 2115 nt, Homo sapiens
  source 1..2115: mol_type = other RNA
ttgggctgggctgggttggggaccagccggcagttgtctggtccagggggcaccaggtctgggataccatcattgtcatcatcatcatcacactcgtcaccaattccatccttatcggtgtccagctgggcactgttaatgacggtggggcagttgtctgtgctgtcctggtgcccatctccatcactgtcctgattggtgtcacaggagtccccaaccagatcattatccacatcagactggttagggttgctgacatcaggacaactgtcacaggcatcccccacaccatcaccatccttgtcccgttggtcacgattgggaaattttgggcagttgtccagaatgttttttattccatctccatccatgtcatcatcacaggcatctcctcttccatccccatcggtgtctttctggtcgttatttaagacactcaggcagttatcacaggcatccccaaagatatctttatcgctgttcctttggtccacattatgaatcaggacacagttatcctgctcattcaggatcccatctccgtcagcatcctcgtcacaagcgtcgccaatgccatctctgtctgcatcttcttggccagaatttggcacatatttgcagttgtcctttttacagttcctggcagagcatggcagttcttcgtcggggtaactgtcgatgtccacatcctttccacagatatagccatctccagcccaaccgactccacacacacatgtcacatccccctgcctctcttcaatgcactgggcattcacactgcaagggttcagctctgggtttctgcagtttctttccgctttgcatccccttatctgatcaccagtataccccggcttacaaggcccacagcggtaagatcccaaagtattaacgcagatcgagttgggaacgcacgctccatttcgacactcatcaatgtcagtgcagacctgcttgtttgacttggcaaaactgatcccaacaccctgcaccatgggccctgtgaagcccactgggcaggcgtcacatctgaagccaggagacaaatttatgcagtgcacgcccgggtagcagggatggtatttgcactcatcaacatcaatacaggtgatcccgtttcctgtgtagccctcggggcagggcccacactggaagccatctctactgtcggtacattggacacctcggaaacatgggttggagtcacaccgacgaggtgggcgtgttggcggtgcagggggagccgggggcaccaccgtgcttggggtcggagactgaaacttgagaggaccgcaagcctggcattcagctatggtgtttcgcaaaaatgatgtttccttaacctgctgtctcagaaggtccttcacctctcccaggagttggtttaattgtgtcatttgacccaagaactgccggttaaagtcccctgtgcctgtggcagccagtggctcactctgctgcaggaagcagtcttgcaggctggccacctggaacagtgagcctctcaccaccagcttcagctcttccaagaagtcctgtggcttcctctggaaagtcctcaattcaatggtctcaggtttctgggaggggccagcaaaggccctggggagattgtgaacggaatccacctggatgcagtccaggtagagctctagggagccggcccctcgctgcaaattgctcagcctcaggaggatcctgtgccgccttccgtctgccagctgcaggttgttgaaaaccaccaaatgcaccttcccatcgttcttcaggtaacggaggatggctttgtttaagcgtcccatcacagtaaattcaaaatatttactgttgtcagttgaagagtaaagaccgaagatggtggctgaacttttagtctgcagcttgaaggtggaaatcacatagagatcattcagggcggggtctgtcaggactggcagcagagcgcctgggtttagcctctgactggaagatgggagaaggtcaaagagatcatggtggaaggcgaaggcaaagcaggcacgtcccacacagcctttaggccaagctgctcctaagagttcttcttaatccctccagtcgttgtttctctcatctctcaagagcccccaaatt

SEQ ID NO: 19605 - RNA, 116 nt, Homo sapiens
  source 1..116: mol_type = other RNA
ttgggctgggctgggttgggtctcctcattccttccttagcagaagtttgtggttttatcccagagcgttggccaaggctgcaacccaaggaccagcaccggcaccggtctctgag

SEQ ID NO: 19606 - RNA, 720 nt, Homo sapiens
  source 1..720: mol_type = other RNA
ttgggctgggctgggttgggtctcctcattccttccttagcagaagtttgtggttttatcccagagcgttggccaaggctgcaaccctatcaaaaatgtccaggaagattggaaaataaaccaaaatagaacttgcataaatgaaagttataactgatgatacaaaaatctcatcagatgattaaatagcagatcagatgcagctgaagagataattatgaattattaggttggtgcaaaagtaattgtgattttagccattaaaagtaatggccaataccacaattaattttgcaccaaccgaatagaaaatggatccacaaaagtacctatttctgcataattttcaacacagaaaaaggagaggtaaaatatgaaagatgtttaggagagaggggagggaaagatgagaaggtctactatttaactaagacccacaggaaagaatagagacagcaaaggtgaggtaacattcaaagagataatggctgagaacttttcagaacttataagaaacatgaattcacacctaggcatattgtaataaacttgcagaagaccaaaaggtaagagaagacctcagaatctatcagagaaaagaaacaagttggctgcaaaagaatgacatttaaaatactagtaactgaggccaaggcaggtggaccatgtgaggtcaagagttcaagaccagcctagccaacatggtgaaaccccatctgt

SEQ ID NO: 19607 - RNA, 236 nt, Homo sapiens
  source 1..236: mol_type = other RNA
ttggggtggagggccaaggagcaattcctgaggttcagctgtgaggttttgtgtctctggtagttactggtgcccatgtctctcactacgaggagaaacctaatcaacataacatagaataagttggagtcctgagcttgttttcctgcaactaggcagtctcatcaatgcaggcagtcatcgtccaatcttctgggggcaaaatatccatatactctgcactcctcccagcccag

SEQ ID NO: 19608 - RNA, 226 nt, Homo sapiens
  source 1..226: mol_type = other RNA
ttggggtggagggccaaggagctctggcccttactcttgttggcagccatctcgctggtcttctgaggctgtgacacacagatgacccactgaagagcagggaccagtcccgccgcctccgccgtccgcacccggcccgcagctcttaaacgcgccccgccccctcccggggccggaccccagccgtcctccaccgatttgtcattgagctgccgggctcgctttc

SEQ ID NO: 19609 - RNA, 228 nt, Homo sapiens
  source 1..228: mol_type = other RNA
ttggggtggagggccaaggagctctggcccttactcttgttggcagccatctcgctggtcttctgaggctgtgacacacagatgacccactgaagagcagggaccagtcccgccgcctccgccgtccgcacccggcccgcagctcttaaacgcgccccgccccctcccggggccggaccccagccgtcctccaccgatttgtcattgagctgccgggctcgctttccc

SEQ ID NO: 19610 - RNA, 447 nt, Homo sapiens
  source 1..447: mol_type = other RNA
ttggggtggagggccaaggagctctggcccttactcttgttggcagccatctcgctggtcttctgaggctgtgacacacagatgacccactgaagagctgataagaacaccaaagttccaacgtttctcgttggaaatgagcacagagaggacactgctcacacaagcagtgtggacgcagcaagctccgcgccccgcaaccctgcaccgagcacggttaacctcacactcccacaggcggcaagaaccgggacggcgatgcccagtccaggcgcttccccttagaagccccttcgccgctggcccctatcagaaaggaaaggggaggaggctgggggagaaacaactttatgctcatttgcaagacaggaccaaaacaaaaccagcaaaccgaagccctttaggaacaccgcccagttcacggcgcgtgcaagttccgagggcagt

SEQ ID NO: 19611 - RNA, 229 nt, Homo sapiens
  source 1..229: mol_type = other RNA
ttggggtggagggccaaggagctctggcccttactcttgttggcagccatctcgctggtcttctgaggctgtgacacacagatgacccactgaagagctgcagggaccagtcccgccgcctccgccgtccgcacccggcccgcagctcttaaacgcgccccgccccctcccggggccggaccccagccgtcctccaccgatttgtcattgagctgccgggctcgctttc

SEQ ID NO: 19612 - RNA, 1007 nt, Homo sapiens
  source 1..1007: mol_type = other RNA
ttgggttttctcttcaatccagagtctctcaggataaattggctcaaaggtgttcatgagatgcccttttccaaacatgactatgcttctcacaacatcccagtgggattttttcacaggacaagcagagacattcaaatatttctccttcatcttgaggaaagctgcctggagggcctcttggtctctctccatgccctgactgtcttgtaacctttttggctttgtctttctcatcttcctgtgagccttctgtacaatcagaaacacaacatgctccttcttccctgtcctctccacttcttcattcatgtcaagaatgtccatgattacatcaatatcaaagaagtctttggccacagcctcaatgatacctggtacaatgtggcacagaccacttctatccgagtagtaatggagaaacattttcccatctgctcctctctccacacgaaacgatggtgcattcatctcctgataagagagtgccaggtaactgtggagggcatccaggttttcaataaactccatgagatttcctcccagtgtccgtagcatcctgtcatagccagacatcttcagaattgaaagtattctccaaagagtttcaggatggcttccatggagacacccagaatgttgcaggcctcttggatgagcttaatggtgatgacgtcatcatacattgtgtaggtcatgaaggcatcttgtacttctgcagaagttttcaatttttcccatgtttcttcaccaaatttctctatcacaagagattgcagacaggtgttgataaatccatacatgttcctgccgcagctgctcctggggccacagggattgagatgcagcaccaagcgcccgcccttcctgccagcccctagtcactcaggagagaatccacagcgtctccagaagcctgtcttgtagaaatctgggcagtccacagtgaaattaggagctcatcactagcctccaagcaaggagcacactgttgggtcctcagtcac

SEQ ID NO: 19613 - RNA, 3133 nt, Homo sapiens
  source 1..3133: mol_type = other RNA
ttgtggatctcaaggatgtgctgccccctcagcagtgcattccttctccctttagttagtgtctgagacacattagtagtgttccccttaggaggaactcagtcacctgatggatggattctccagttgtagagtgcagagtcattctagcacaccaacttctctatccttgggacccacttttccagactctgccacagtagttctggtatctctgcttccacttgatttaatgtgtaccatggcttatactaagtctctaggagccacccaggagtatatcagaatcatcacctttggcccatgccaggctagttaaactctgtggtagcgaagcttgcccttttgtcaataattctcacgtatctggtttcacatttcacccttcctggaccaggatccactcccagacacaatctccttgctcctgctgatgcacgctggccagtcctacagctccttcggaggataaacgctctcttcactttgccgccctgcccatgactgttcacttgcattgtcctgagcggtctctacacagtcttccttcttgtaagaggccctgtggttctggaagatgaggcgcatgtcttgtacaaacccctccacttgggggtaaccgtgctcattcagccttttcttgattttatccaaccacatgggctccttcaggccttgacacgcctctctaatataataatagtatggaatcttggcaaaaaaggagctctcagaacagcaatagactttcaagaggaggaactcacatttcaactgttcctcaggacacatctgcctctccaggacctcagattcctgacaacactgttggcttcccggagactccttcatcctgcagaagatgcaattccacggggtcctctcagcttccacaggcgggatgtgacagtcctcatggaagactcttgaacaagtgtcgcaacagaacagctcccctccgtcccggcacacctcacactcatccaggtttctcatacaagggtcaactgagctattgttttgagacttcagtattctcttttttttcctgtaacgtattcttggaggatcaggcagaaatccattctccatcagccatcgtaggggccacccgccacagcgcacactcagcctccagttctttgatcttgcatggcctcctttgatttcaaattccgtgggggtgaaccattttccatcctcagtctgtatacacttcaccaagattccttgctgcaatttcttcttatgtaaaattcccttcaccccaccacaggtcactggaagcaaaggagccttaaaatccacagtttcatctttgtgctttcttgaagctcttgatcggactcttttctgtgcagctctgtcactctgagtgaagcgggttccaggtttgcctctctttctccccctaatcttggaaaggtctttcagattcacgttcgccttcttttcactggagaccacctggccgtcggctttgctattatcattttgttggctgttttcctgccttctcattctcattctgctccagccatgccccctcttttttcttcttttcctcttgggttttcccaaagtggagttgtttgcaatatccacagtatccattgtgccacacgcttgatcactttccgtccttgcttctgggcttcctggcacctcttctgagaaacacatgacacaggaacacttctcattttcatatgctgattgctccgctcctggtacattatcatatagcaggctagaagcaagctcttctgattctccttcttcattcattgggtgattttctagttcactagacactgacccacgtcttgctagggagctagaggcttcctggcgctcttctccatcacacatttccgaacagtcatcactgccctcttctccttcacctggtagtagactgagctccttctctggttctccttcattagtgacttggggagtctttagatcaaaggtctctgcagataaacaagaaactgacccacatcttgctagggagctagaggcttcctggggctcttctccatcacacatttctgaacagtcatcactgccctcttctccttcacctggtagtagacagagccccttctctggttctccttcattagtgacttggggagtttttagatcaaaggtctctttgtctcttccctctggactctcttggtacttctccttgtcttggtttctttttctgggactgttcctgccttcctcctctccctgtttctcccctggtgctgtgctgtatgtccttgccgcatctatcatcccgttgctttctagaacttctgtatcataaggcagtaacttgggcatttcttctgattctccttcatctatttgtatagcaagtttacaggacactcccccacctggtagtaggctgggtgcatcttcagcatctcctccaccagcctttgggagagctaactgctcacaagactctgaagagaaacctggctcacaccttggcgaggagctcaaggcttcctgaggcactgctatatcatccatttcatgacaggcattgctgttctcttgtttaccatatggtagtaatctgggtctatcttctaaatcgtttacattattcatttggagaggtgagtgttcatagcatacattctggaagcttctgtaaatctcgtttaaatcaggataggccatcaggttaatcctgctgaacaatgcttccagatgtgaccagccaaatgtcttctccagttcactgagtacacaatacatcactcttgtcactgggaccaggtttctaaaagcttcttgaaaatgttcatacatctgctcggagatgaaggagcggtctcggaggcccataaggaaaggaaatggccttgttattgcacttgcaatctccaccttgttttctctgaagaacctgaaaatgggctcagggcaaacctgctcctgcaggttctgaccctctacgttctggatctctgcgaccatcctgaagttgagattgctgtctccacttgccatctgcccctgctggccctgctgggccatgagcttggcctaggatcacacccgattcgattttcactgccccgttccttcctgcagctctgaggtgaagctgccaact

SEQ ID NO: 19614 - RNA, 1887 nt, Homo sapiens
  source 1..1887: mol_type = other RNA
ttgtgggtgggcagaagtctgttttcttcatggttttctgacctttgcctctcccctcaggaaatgctgacttttaacccacacaagcgaatctctgcctttcgagctctgcagcactcttatctacataaggatgaaggtaatccggagtgagcaatggagtggctgccatggaaggaagaaaagctgccatttcccttctggacactgagagggcaatctttgcctttatctctgaggctatggagggtcctcctccatctttctacagagattactttgctgccttaatgacattcccctcccacctctccttttgaggcttctccttctccttcccatttctctacactaaggggtatgttccctcttgtccctttccctacctttatatttggggtccttttttatacaggaaaaacaaaacaaagaaataatggtcttttttttttttttaatgtttcttcctctgtttggctttgccattgtgcgatttggaaaaaccacttggaagaagggactttcctgcaaaaccttaaagactggttaaattacagggcctaggaagtcagtggagccccttgactgacaaagcttagaaaggaactgaaattgcttctttgaatatggattttaggcggggcgtggtggctcacgcctataatcccagcacgttgggaggccaacgcgggtggatcacctgaggtcaggagttcgagaccagcctgactaacatggtgaaaccctgtctctactaaaaatacaaaattagtcaggcgtggtggtgcacacctgtaatcccagctacttgggagactgaggcaggaggatcgcttgaacccgggaggcagaggttgcggtgagccgagatcatgccattgcactccagcctgggcaacagagcaagactctgtgtcaaaaaaaaaaaaagaatatagatttttaaatggcttttacttttatattcgctaaactttctcaaactggatcctgcttattacaggaaagagttcttggttgttttctccttggccctatccctgatttacccttagagccacaccagggtatgttgaggtgatccagtatatggacagaggaagggaaacagctaagaatgactccagcccccatcctatgcactcacagaagcttcccatatcctcttggagagagaggaagaaagtttttccttttattccttatagtctggctcccactaaaatatgtcaaggcataaagtcttgctattccatcaattttagaggatgtgacaaggggcctttcctttttctcaaaccaaaacggttacagaccctagatattccctaagggaggaagagaaagcttagagagagcagaagaaaagtcagaaggatccaaagtctcatagaaaggcactggggttggctctaggatccttctgattccgaaatctcattgctagccaaacaccaaggatctctgtaaagctaaagaagagtccaacaccccctaggattttcagggcttcgtctgaatgcttaagaaacttttctccacacatctggcatgtggggctctggctcttgcagattgcagtgcagaaatcataatcttgttgatacagggttgtgaggttgaataagccacaacaatcaaaacttctttccagttcatcccgagtcttgttgctcatgacccaccaagaagcattgatgacatctgtcatgtagaccacgttgagagcgcaaagcgcattcttggagcaggcaaagccgccacaaaccatctccccagctctggggacccaagtggtcccaaggacttggggggagggtattggggaccgtcttccaggaccccgacagcttctgtctctttaaatcgaggccagccaaacccaat

SEQ ID NO: 19615 - RNA, 2136 nt, Homo sapiens
  source 1..2136: mol_type = other RNA
ttgtgggtgggcagaagtctgttttcttcatggttttctgacctttgcctctcccctcaggaaatgctgacttttaacccacacaagcgaatctctgcctttcgagctctgcagcactcttatctacataaggatgaaggtaatccggagtgagcaatggagtggctgccatggaaggaagaaaagctgccatttcccttctggacactgagagggcaatctttgcctttatctctgaggctatggagggtcctcctccatctttctacagagattactttgctgccttaatgacattcccctcccacctctccttttgaggcttctccttctccttcccatttctctacactaaggggtatgttccctcttgtccctttccctacctttatatttggggtccttttttatacaggaaaaacaaaacaaagaaataatggtcttttttttttttttaatgtttcttcctctgtttggctttgccattgtgcgatttggaaaaaccacttggaagaagggactttcctgcaaaaccttaaagactggttaaattacagggcctaggaagtcagtggagccccttgactgacaaagcttagaaaggaactgaaattgcttctttgaatatggattttaggcggggcgtggtggctcacgcctataatcccagcacgttgggaggccaacgcgggtggatcacctgaggtcaggagttcgagaccagcctgactaacatggtgaaaccctgtctctactaaaaatacaaaattagtcaggcgtggtggtgcacacctgtaatcccagctacttgggagactgaggcaggaggatcgcttgaacccgggaggcagaggttgcggtgagccgagatcatgccattgcactccagcctgggcaacagagcaagactctgtgtcaaaaaaaaaaaaagaatatagatttttaaatggcttttacttttatattcgctaaactttctcaaactggatcctgcttattacaggaaagagttcttggttgttttctccttggccctatccctgatttacccttagagccacaccagggtatgttgaggtgatccagtatatggacagaggaagggaaacagctaagaatgactccagcccccatcctatgcactcacagaagcttcccatatcctcttggagagagaggaagaaagtttttccttttattccttatagtctggctcccactaaaatatgtcaaggcataaagtcttgctattccatcaattttagaggatgtgacaaggggcctttcctttttctcaaaccaaaacggttacagaccctagatattccctaagggaggaagagaaagcttagagagagcagaagaaaagtcagaaggatccaaagtctcatagaaaggcactggggttggctctaggatccttctgattccgaaatctcattgctagccaaacaccaaggatctctgtaaagctaaagaagagtccaacaccccctaggattttcagggcttcgtctgaatgcttaagaaacttttctccacacatctggcatgtggggctctggctcttgcagattgcagtgcagaaatcataatcttgttgatacagggttgtgaggttgaataagccacaacaatcaaaacttctttccagttcatcccgagtcttgttgctcatgacccaccaagaagcattgatgacatctgtctgtttgcttcggttaatagccagacatgagcaagagattacaaattggaagatgaagaccaaaccaaggatgatcatgtaaaagaacagcaggacttggtggtggttgacagcacccaccagtccagccactgcaataaggagaaggaagactcccacagcaatgactccgccgatgatgtggatgctggacaccagacccaggcccttgccccaagcagccactccaatgagcaacaagctcaccagcatgtagaccacgttgagagcgcaaagcgcattcttggagcaggcaaagccgccacaaaccatctccccagctctggggacccaagtggtcccaaggacttggggggagggtattggggaccgtcttccaggaccccgacagcttctgtctctttaaatcgaggccagccaaacccaat

SEQ ID NO: 19616 - RNA, 2150 nt, Homo sapiens
  source 1..2150: mol_type = other RNA
ttgtgggtgggcagaagtctgttttcttcatggttttctgacctttgcctctcccctcaggaaatgctgacttttaacccacacaagcgaatctctgcctttcgagctctgcagcactcttatctacataaggatgaaggtaatccggagtgagcaatggagtggctgccatggaaggaagaaaagctgccatttcccttctggacactgagagggcaatctttgcctttatctctgaggctatggagggtcctcctccatctttctacagagattactttgctgccttaatgacattcccctcccacctctccttttgaggcttctccttctccttcccatttctctacactaaggggtatgttccctcttgtccctttccctacctttatatttggggtccttttttatacaggaaaaacaaaacaaagaaataatggtcttttttttttttttaatgtttcttcctctgtttggctttgccattgtgcgatttggaaaaaccacttggaagaagggactttcctgcaaaaccttaaagactggttaaattacagggcctaggaagtcagtggagccccttgactgacaaagcttagaaaggaactgaaattgcttctttgaatatggattttaggcggggcgtggtggctcacgcctataatcccagcacgttgggaggccaacgcgggtggatcacctgaggtcaggagttcgagaccagcctgactaacatggtgaaaccctgtctctactaaaaatacaaaattagtcaggcgtggtggtgcacacctgtaatcccagctacttgggagactgaggcaggaggatcgcttgaacccgggaggcagaggttgcggtgagccgagatcatgccattgcactccagcctgggcaacagagcaagactctgtgtcaaaaaaaaaaaaagaatatagatttttaaatggcttttacttttatattcgctaaactttctcaaactggatcctgcttattacaggaaagagttcttggttgttttctccttggccctatccctgatttacccttagagccacaccagggtatgttgaggtgatccagtatatggacagaggaagggaaacagctaagaatgactccagcccccatcctatgcactcacagaagcttcccatatcctcttggagagagaggaagaaagtttttccttttattccttatagtctggctcccactaaaatatgtcaaggcataaagtcttgctattccatcaattttagaggatgtgacaaggggcctttcctttttctcaaaccaaaacggttacagaccctagatattccctaagggaggaagagaaagcttagagagagcagaagaaaagtcagaaggatccaaagtctcatagaaaggcactggggttggctctaggatccttctgattccgaaatctcattgctagccaaacaccaaggatctctgtaaagctaaagaagagtccaacaccccctaggattttcagggcttcgtctgaatgcttaagaaacttttctccacacatctggcatgtggggctctggctcttgcagattgcagtgcagaaatcataatcttgttgatacagggttgtgaggttgaataagccacaacaatcaaaacttctttccagttcatcccgagtcttgttgctcatgacccaccaagaagcattgatgacatctgtctgtttgcttcggttaatagccagacatgagcaagagattacaaattggaagatgaagaccaaaccaaggatgatcatgtaaaagaacagcaggacttggtggtggttgacagcacccaccagtccagccactgcaataaggagaaggaagactcccacagcaatgactccgccgatgatgtggatgctggacaccagacccaggcccttgccccaagcagccactccaatgagcaacaagctcaccagctccaaaacctcaccatgtagaccacgttgagagcgcaaagcgcattcttggagcaggcaaagccgccacaaaccatctccccagctctggggacccaagtggtcccaaggacttggggggagggtattggggaccgtcttccaggaccccgacagcttctgtctctttaaatcgaggccagccaaacccaat

SEQ ID NO: 19617 - RNA, 10359 nt, Homo sapiens
  source 1..10359: mol_type = other RNA
ttgttctcaaactggctgtcagaatacttttatgaagagtattaggaagaccttaatttagttctgggtgctaaaaaaatcacgtgtaaggatatagtgtcagaacactgaaatctaagtctacaaagaatatcatgttttggtttgcagtgaaccacagtaagttgtcagtgctgctctgtgcttaccacttaaatcatgataaggtgaacctccataggtaaaccatgtgagaattctgtcctttcatttattttgaaccaagaactattattggattttaactctcattctgagatttcttctccaggtgatggtaaataaagtaatacgcacatgcattatgatgaggatggagggagtggttcacagcacctcaccttcgggtcctcaggtagaactgcaagagtaagaagttaggctctgatctgacatgttctcagaaactatacggttgaccttcaaataatgcaggagttaggggcatagaccccctaagtagtcaaaaatccacatctaactttgactcctccaaaacttaactactcatggcctactgctgaccagaagtcttacggataacatagtcgattgacacatattttgtatatgtattatatactgtattcttacaataaagtaagctagagaagagaaaatgtttgttaagattataaggaagagaaaatatatttactattcattaagtggaagtggatcatcatgaaggtcttcatccttgtcatcttcatgttgaataggctgaggatgagaaggggttggtcttgctatcttgggtggcagaggtggaagaaaatccatgtataagtggacccacacagttcaaacccgtgttgttcaagggtcaactgtattctgactcagaatagcttaagaccctcagggtcatagaaaaataccatcataatctcttttatggtaggttggcaatataaattattaacaaactctaaaatattaccagtacctgaaaaaaaaaaattcagcagaaaactgtgaagtggaacatttagtcactgtttttcattcattttgaaatttttatatgtttacatatatctgttgtaaaaaataccaactttccaagtactaggaatgctgaccactaagcctgatctaaagtttatgttggggacctcaggtatacaggagtggaacagggacaggagtgaaagctttgactgaagacaaatgtgggcttatggcctatctctgtcactaatttaactatatgggcaaagtactaaacctgtgtcttcatctgtaacatagggattagacaccagtgataggagggtcttggtcagtagctaatcacagagctgcttccttaaaagccttgagtacttttgtttaaaagtttaggtctacttgaaagtctgtaaagtgctaatttttatcatcctgagagatctgtttctcccctttccagttaccagtggcattctcccaaaactgttagtatctatgttatagaaagatacttaaatgctatgataaattgtatgaaaaaaactttaaaattcagcaagcaattcttaatgaaagataaaactggccctctagtaccataattagtttagaattcagtcttttaaattatttgcaccttgagactctgtgaaatgaaaacatttaacagtaaactcttgtcccaagggagcaaagtgagagtaaatgctggtccatagtgatggggaaaaaggactgtgttcaccatgagtttttcaggatgcagcataaagcttatctaaatactacacagatcattatcttttaacccaaccaatcatatattcaaactaagggaaaaatatgtaagcttttcctttggaacctgagacaccaggagccttaaaccacaaataatctactgtagctatggacagggtagtcaaatttatttcaaaacaaaagctttgttgggctgcatcaaatgcaggagaaaaggaatacttaggggcatggttaaattaccagtgtgcgtaacagtgaggtatgcctcaaataagcctttaaaactttataaactgaactagaacatacccatgcagtaatattttttcagtgctactaatgaaaaaaaaaaattaaagcctgcactggaaatttacaatatggcagaatttgttacttttaccttttgaccctaatgtacagattttatgacagggtctgtgttaaaaatctaaacattttcacaagattttaaacatcactggaaagctgaatttagaggaaacaatatcagataaaagtacaatgcccgtgacagccaacattatgtaactgggctgtatgaggttgtttagaaggctagggttaaaaagatagatagacaaaaagatttttaaaaatcacccccaaagttgatgcgctgatttgaacataagtacaccagatactacagcaaggggatatacactgcaaaaaggtcatctatttacagaagagtgatttaaagacattatggttttctttacagatgtaagaacagcaactgttcactttttaaaaactctacatctcaaccctccactattattatagtccactgaattgcctgtatcaaaggcagttttttgtttgtttttttcccatttgactctccaaatgaacttccatcatttcttcatcatctgtgggctggctctcctgaaaagtctcagggaataagtcacaggagggcaggtttttgacctgctactaaaaattaaaccacaaaaactagagatccctctcctgcaccctgttcccctcactttgtgcagttcagtcatcactatccgacagggtctcgtactgtgctgagagcagtggggcaggctctcgctcccagatcctgttctgttggtgaggagctgcttggttcaccgcagagggagcacatgcaatcggtgttggtggagtactgctgagcatccgcatagtcagagggttataaggaaactgagttgagcctgttgaagagggcctgtcttcccaggcccaccctggcgtctgcctatggtaatccccttctgaatgtacagaggagactgaagagggccgttccgttcctaagtagccttgcccaggtataggagacttagatttcctgctgtttgacttgctgatcagctttggtttgcaaactcctcctgaatgaggtgatgggtccccttcctctcttcgtgtctcaccactggtcacaactgaggtgttggcagtaccaggcactactcccataggctgggacatgacaactccatgatcctcaactttgtcatcaaagcttcccatgagagccttcctgataatgtcttccagcccaagattactggcaggatcagcaaaagaatggcctctagagctaactgagcctgacgtagtaactgctggcagattaaagatctcagttcctggctgagcagctgccatatcagagtcacctccaccagaggagttcaacttacgaaaaatctcctgcttctttgatttaaccatgggtgatgtattttcaagcttggtgaagaatgaaggcaagtagcttatactccctggtgagcgggcatcattcctctgctctgcaggctctgcgcccctctgagacaagagcagcaagctgtcctgtttctcatgcacaaccggaacctggggtggggagatgggctcgtagggctccgaagagacgtgactcctctctggggattttccaggcctacttcccctggatttgtccacaagattttctggagagacccttgaacctggtctttgatgatggacagactgagcctgggattctgggctgtaacggtttgatgttttagtcctcacaggtgtagataccaaagcagaaggtgagttctggaatgtagaagtaggaggctgctggggagtctgcgaggaaacttgatttctagcaaaatcttgtgtgataatttgacagatgtgatcagcaagtgtgatcagccgatgggtcctgggcacttgccccattccctctgcctgtgaagaagggggcagctgttgttggggagatggtgattcctgctgtggtcgatagtgatgtaatggtccttcatattgtctggtaggatcattttccgcttgatttgccttaacaacctctggctgataggtctgcagtttctcctggggtggcgcaggtgagctggcaggacttatcacctcaatagcatcgctaggtgtttcatacctgtgagaagataagctactagaagagtctgaactttgagagccacgttccctcgcatccttgtccgaggcaatttgccgggtgatgatcacgtctatgaagttagctgcagtaatggtagtcttccctctggtccttagctcttcctcatatctggattttggaggaggccctttatctttcccagcctcagaataaactactgaagaatgaggctggggcttgccacttggaaaggctgaagaagtgtataaacactgaacagatctcttctccacctccagggttttctgctctagctgctgctgttcactaactgctgctgacctgcttctcaaattttcttctaacctggcagcttcatgcttactctcttttgttttggacacatccatctggggtgcagaagctgcagcatccacaagagcagccagggcatccgcagcagtgttgtaacgggaggctggcaggccttggcttattgaagggcccccagcaggcagtggcatgattcgtagctgagcagttggatccaaaggtgtgattacactggttccattggttccttggaaaacactgggtctctgttgcaacatggtctcctgagttcttactgaaggggaaggggagcgaacatatccatgactgccaggtcggccaggctgttctgagcctggccgcaggtagaggtcggaggaagctgcagcaatccgttcccgctcccgctccttctcccgctcccgttcccgttccctctcagcacttgcagcagctgcaaggtgtgttgggtgtcctggagacatggaagcagagttgtacggcctgggagggaaagtaatctgtgtaccaggaatataagtgattctgtccatgggaggagtgcttgttccccctggatgaggcactaaaattgttggaggcatattggtcaggtcaatgattcctctcgttgctgggtatgggagacccagtggctgctctcttggggagagtcctctggccacatctggacgcaagttcacttgcatctgttgtgaggtaatgtaatcatttaagattgtctgtcttgtgttctccattgcgtaaagctgatactgacttgggtaacctggagttggtgaaagctgtctctgaaacaggtaagcagccgctgcaggatccaaagccctgtgaaaaggcatggctggatccaagtgcgtgggcaggtggctccgataaacctcgcctgcagtgctgcctctgtgatggggatcaaacggactgtggctcacgacagggtccaccccaggcactggagacttcgctgggatactttccctctgggtaggggtcagtgtcgatttcctttcatgattggtagacttgttagaagaaattgtaacatcagaagttctgttcatcatgggtgagcctctggacatggtgttttgataactcacaggggtcctccgtgcactggtgtcatcataaatcccagggctcagttgtgctttgggagcttcatgcagtgtggacctaagaacggaggggccagagcttaccactgacgtgtgccgggaacgcacggtctcgcctgctttcacatcctcatattttccccgttctaccacttttatgttctctggcacaatttccagcggaggcattccacgggatagtttgctaggccccgtgattaaggatttgacattgtgtttgatggcagattgacctgagttgttgtcaaactttattggtgtgccctgggaaatggaaccctcaattatcggccgtgtgctctggaccacttctggagttttccgactttcctgagttaaaatatcttgccttggaatctcatgaatggaacgccccatttctttgatggtggtgatgccatcatatggttttcctttggtaatggcaccttcaaatgctcgtatgggaggactttcccttttaatttgtttgggatatttaaggccatcttcaaagctttcagttgttgctcttggtgtcccctgcattatggagccagacaatacagtcctttctttgaggtcagaatgaggactccccctgggtaatgctcggcatatcagcccctctaacggtgctgatacaggagactccctcattgacatcccttgctttatatttccttccactgattcatagcttctctttaaactgatttcatgagctgttcttggactcctagtcccttctcgggcattcttaatattatcatatgacaagatatgtccacttttgccttcataaataacatggcctttggatgcagcttcctctctgcctttctcaggactgctgtcttcaatgggcattctcgaaatggaccccttcaccaaagcctctgttggtatgccagtctggggcagagccggggtgccctgagtgatagagccccgtagggatggaatgctctccactgaaattttgctggttggagttccccgagttatacttccttcttgtatggctcctgcggtacctctgactacaccttcatgttgggccctgaccaacagaccctcaggttgtgagttttggcttcggggagaaaattcttcctgcttgatgtagggcaaagtagctgatttggcagattcctgttgccgtggcagtccaagagagatagatcccactgacggcttgggtgtttcttgagtgtaggaagcctgattatgagaagtcaaataagtgcctggtgttccctgtgagatggagcctcccattataaaagatggtttttctgaagccactgtggttttggatgacgggatgagagggggcggtggcctggttggtcgagttgtcggaagccgaacgccttcagggagattagttatcacttgatgtggagcaggctgaaggacttcccactctctgtttggactcttggatgtgccacatggacttgtagaacttctacattccaaatctatctgttcttgtctctgccgctgctcctccaggagtgctgactcatgcattgctttaatgtgtcgctggtagagagcatagccgctcactggggttccaattggtatgttacatggggtgcaggataccattggtgggataacagcagctcgatgctgaagctgtggcagatccagtggatttggttttaacggagatgagacgagtatagatccagtggggtttaacagtgaaggctttgagtccataggaaacattctctgcctctctggctctccatccacatcctcatcagcgctgcacgtggcactggaatcattgtctgactggggctcgggcctttgggcatttatttgctgagctaccaccaaatcttcatctctaggttccaccttctcactggctctatccaagtctctttctttggtattatcaccttcaactttagatgcatggttttctggcaccctcacttcaacgtccacagagtcagctttggtagcgggtgggggatcacaaacagaaccctcttcagcactgtgctcctgctgatctacatccatctgctctgctgtctcagcactgatgctgtcattcacctgggtctccacactttcatcttcagctggttttgtacttggaactgctaaggagggagatgtactgggtgcagtttccgtggtgggctcaagctcaaccgcaggttctgtgtttcctcgagaagtagcattttcaggactgtcctcgctgggcttgacagcttcaacttcgctgtcttctggattttcttcttcattggaggcttcaatatcttcatcctcctgagcagaaacagtggaagcgacactttcacattgagacacatctcgctcttcacgaggttttcgtgaagttttctgtttatgctgctgtaagaggttgtcaagattgtgtcgccttttatagttaaaatagaagtttttacattgagcttcacttttcgttcccaccattttagcaattgctgcccagttacgaccatgttctactagaccttttttagcaacttccatttcttcttctgtccatcgagaggtctccacaggctctgtagaaatgggttctggtggcggtggcagaggtggtgggggctcttcagtagccgctgcggctgcagcactggcagctgcagcttcgtttgtcatggacctggtgatccggcccttacggcggccctgactgttggcagtctttcgcccccggggtgtggcttgctctctttcctcagtttcttctgctgtaccatctatcttgtccttttccttggtattttctttggagtcttctttttcatctttttcctcttcatctttcttttcttcttcttttttttctgttttttctgctttatcctcttctttttcttctactttttcttcttgcgagggtcgagcaatttgctggtttctgcctctgcgtttcccataattccttctgacgagggctttataattctcatttttcttggttaaatagtaatacaaaacacaatcaggaacactcttcctctccaagtatgatgcaattagtccaaagttttttggatgctggataaacttgtccttaaagatctccttttcatggtcagtccaaacattcataaactgcctatctttatacactttcatagggtcctccataagcccattcatgttaatgaacttgactcgtctttgttctgcatcaaacatcataggtggaatcacagagagctgccgcatttgtttctcattattctcctgctcagagagcccatcaataatttcagaaatctcatgctcactcctagcaatggtggctgaaagaccagctcccctctgcccaactcgctgaaatctttcttgctgttctctttgttttcgaatttctggaaactgcttttcatagtattcccttgttttgctttctttagctttcctccgaggattattttctattctgtccacttttttctcccatgcctccatgagctgatcataacgctggcagattttttgttccctttgttttcttgcatgatttcttcttttaaaaaataaaatgagttttttcctcatcacctggtttgtcttgatgttctcatggtacaccttggtatctgatggctggttatacagtggcagttcaacttttgggccaagaccttcaaaaattttatgagcttcttctgcttttttccgattctcatcataaataatttggacaatactgcggtgtttctgctccacaggaggaggggacacgggcttctcaggctcaggaggtttagctgcctcttcttcaagctgttgttgtttctttttcagtttaaggatctgctgttctacttttgcaatttctcgatctacacgatccatactctgtattaactcttcctttgagagttttgaaggtgaagcattttgatcatctccacatggttgccccgaaattggagaggatggagcttcatgtttgcctccgaatgctggatccttcttagcatctgcagaagccctcagcccttctggcagcgggtgcactaaaggcaaaaccgcagcactgacacgctgaaaatgagaatcagaaacctgttccagacgtggtcgcttcgattccagtgaatcatgatccactggggatgggcctggatgaaacggttcataactagttctcctttcttgaggcctgtcagaacctgggtgaaattctgaaagcaaggaaggtcgccttcgaagctgttgctgctgctgttgctgcaaaagctgtgatgcctgactcacttcaagatgagaggaacgataatcagggactgcgaactcctgctggtggcgggtgttgggaaatgtatactggacagagtgaggaggataacgactttgttctgtgctgaatgctccttggttgggaggataacctgaacttgacattatcagtaaagaagtcctcaccagactgtgagatcaatgccaataaacaatcatgtttctaggaaaccaccgggagctggctaagcgtgggagccgacgtgcgccccggcctgaggagtgggacgcggccacggcgcgcggccctacaccgggacctcgttcggcgcggcgagtcggacgctcactccagccgccgccgccgccgcggctgctgcttcgccaccttggccgccatcttgactc

SEQ ID NO: 19618 - RNA, 1188 nt, Homo sapiens
  source 1..1188: mol_type = other RNA
ttgttctttggtctttcagccagggccaggactagggtgaggaaagtacggcacctgtggtggtcacgtcactctcaggtccaccagggccaagcccctatgaaggtggtcagtcctcaggctccccggggctcatctccatttttggaatccaattacaaaacattgatccgatcccactccagagaactgatttatgccccggttgttcccttgtgtgttatctctgtctcctccccactgtcatctccacaagatcaagagcttcatatgtcttattcatctctttcacaccaattcagtacgtggcacatgatgggggctcaaaaaaaatagtatgtccaccagcagaatcatgaggtgatcattaaaacccctccaggatggcactcaatagtccttgacatctgcacccagaaagtaagggcggcatagggtgcgggaagagcggggatcatccaggagaacttgtgggaaaaggacgatcagagctggattctgggagacagaggaacgccagcctagagaaggggaaaacctgtcttgagaaggcaggcaggcaggagccacagcggtggagagcttcaagtccctgcagctgctacaccttcaggctcccagccaagaccatttggtgaactatattaataatcacaatacaagaatcccttgtggactggaacaatttcccttccaaggcagtgacatgcctatcacttcactttattcttctgccatccccttgatacaaaggaggagaaaatatcttctgctatgtataaaattaataacaattgttcatttgtatagtactttcccatttcccgaacacattttcttatacaggaatgatagtatttattcccatgttgcagatgaggagactcagagaggtgaaatgacttgtccgaggtcagtcatagcgtatgtagcctggaaaactcaagccccgaactccaaatttttcaacaacctagtggtgttttttccagatgaggaaactaacagagagagagagagagagagagagaaagtgtatggctagcttatgagagctccccacccacacatccagggggttaaattatttgtagggtcaggatgaggcatgcggacagtgggaagggaaccatctcccttcccgacctgagcatggagatggagatcaccctgagtgaaaatgttcat

SEQ ID NO: 19619 - RNA, 70 nt, Homo sapiens
  source 1..70: mol_type = other RNA
tttagtgtgataatggcgtttgatagtttagacacaaacaccattgtcacactccacagctctgctaagg

SEQ ID NO: 19620 - RNA, 470 nt, Homo sapiens
  source 1..470: mol_type = other RNA
tttagtgtgataatggcgtttgatagtttagacacaaacaccattgtcacactccacagctctgctaaggaaactctgtagccacgaaggtgttaacttcacctccacattccaccattgtcactgataataggggaaccttgtcagctccacatattgtgaccagggctatcgctgaccatccacaagaggctctagaagtctcttagctctgctgggaagaaacagtgagaggtgaacaattcactgattaaaagggtccccggaggatgcgcttggagcgctctatcctgggcaagggcttggacccatttcacttctcagggctccatagcagtatctgagcatcctccacttctccatgggggctctgttggcttttggctttgaataatccccagtcagctccggtcctctcagtccaaggcccttcctgtggcaggcaggatggcgccttccacagcttctgt

SEQ ID NO: 19621 - RNA, 632 nt, Homo sapiens
  source 1..632: mol_type = other RNA
tttagtgtgataatggcgtttgatagtttagacacaaacaccattgtcacactccacagctctgctaaggaaactctgtagccacgaaggtgttaacttcacctccacattccaccattgtcactgataataggggaaccttgtcagctccacatattgtgacctaagcagagaaaagaagcatcacgggtacaagcatcttgagcaatgggaagagctgaacactctcaatgaaaggcttctgtgttctggaacagtagagtagtagaggggtccactgcctgtgttccactgccacccagcaaaccccttctgcaaaaacttccagggctatcgctgaccatccacaagaggctctagaagtctcttagctctgctgggaagaaacagtgagaggtgaacaattcactgattaaaagggtccccggaggatgcgcttggagcgctctatcctgggcaagggcttggacccatttcacttctcagggctccatagcagtatctgagcatcctccacttctccatgggggctctgttggcttttggctttgaataatccccagtcagctccggtcctctcagtccaaggcccttcctgtggcaggcaggatggcgccttccacagcttctgt

SEQ ID NO: 19622 - RNA, 1662 nt, Homo sapiens
  source 1..1662: mol_type = other RNA
tttcagataacagtattacatgtcaacggtgtggttatgacctttatttatataaaaaccaaatatttagtcaatttaccgtgtcttaatttaatctttgtacaccttccatttttaagtgcttaaatgagtactatattgcaataaaatgtagtgatataattaaccagccattaaaaatttacttctacagatacagtgtcaattgagtttatatattaggtacttgcatactttttatgattactatgaaaattagagcaattaaaattaatggtttctacaattaatctgagttctacaacctaaaattgccttcagtttactggcatccctggattagggttagacctgatattgtggctgacacagaaaggcaacaggaaattaacttcattattttcatattcataatatggcatatgagactcaccaggcaagcaaatccccagactggttaaaagtaaaaatttaaaagctgttagctatattttgtgcactgaatctttaatagcaaattgtctacaggctgcagttagagactttgctggaatatccatttctccttttagtccgtgccatttttgccacccctctaacccggggagagtagaagaggtgctgttgctgatgtgggtatggcttgaattcagttaaatatattaaaaagaaaacaattccttcttaaaccactttttcctctaggattgcaaggcacagttctactccagaagaatgaaatgtggttgagcacttcctcaaataggtttatgatttttataatgatcctttaaaatgatctatgaatgatttattagataaattctatacatacaaagtacagattcttcatttagcattgatttacttcttagttttcatctttctgaccatccaccgtcttttaaacctcttggcattttgttttttttggattccccaagcattattcaaaaactggacagcagctcttttcactggtaacctcttgttggcaagagacaggaacttatttacagtagtcctgttggttcctggcccatataatgaattatgtatgaaggcttgtgctgcttgttgccttgaatctctcagatcttggtcttttagccttacggccaagtagcttttattctggctgacagactgtactttttgtactttaactttcttggagtcatttcctttttcacagtcttcatttttcttttgcaaattaacttctttcacctttcctggcgatttcttgatgttagtctgtgaagctgtggttaacttctccaaaatagtgtctggaaggagttttcttttcttctgttcgatgaacagctcctcgcgtcgcttcctcttctccttcaggagcgttttatccctgcgcacggtctcccgcactcgccgctcctcttctctcgcttccgcctgggcgctggcgaaagtcagctcctccggggcctcatcgtcaaactcatcgtccccttcctcgtcttcctccaggggctcggcggccgcgccgctgctgggctgcccgagcaacagcccgtgctccgcctcctcctcctccgaggccagctggccctcgtccaccatcgcctccgccgacgccggggcgcgagacgctcgcggtcggagctgcaccatggcccacgcagcgctagaccgtct

SEQ ID NO: 19623 - RNA, 818 nt, Homo sapiens
  source 1..818: mol_type = other RNA
tttcagataacagtattacattattggattgttccgagcagggaatgaaattttgcgggtacagcacaagaccacgttacctagtagtaataaggatttaataaatgttagctttaaatgttagtgagatatttcaggttaactttagccctagggaggagggagaagggtcctgggaaataagtagacatgaatgcaggaaggggatgacagaaagcactgactgaagcagcctgtcgagaaatgtgtcatcaagacccatgtccagcagcttattcctattccaccttttccctaccatttgtgaagtacctatcagcctaaaagcaatgagctcacattaggtaaacatatggtgatggtggggaacatgtaattaaataagtaaatgaataatccctgtgaccttctcacctaagggcttgcagagtttcttcacttttgattcctggcttccaatgcctcccgtttctgatccaaatgtatcatcttctgccagaagatggtctatgggttatgctttcttcttaccgccggctgcgcggtctcggccgcggtggcggcggcgacggcggcgacccccgcctgggtcatgatcccaggaggggaaggcaggagtgtctgaccgtctgggcgaatctctccgtccgcggccaccgcctgctcctccggggctgggggagcgcgggcccaggccctcctctccccccgcccccgccgcctctttttgcggccaccgcagccgctgcgagcccgagccctcaaggccggagacccggcggcagcgcggcctcaactttcccagcccccctcccccc

SEQ ID NO: 19624 - RNA, 63 nt, Homo sapiens
  source 1..63: mol_type = other RNA
tttcccttcagagcctggctttcatagatgccaaagccaggctctgaagggaaagctgaatct

SEQ ID NO: 19625 - RNA, 638 nt, Homo sapiens
  source 1..638: mol_type = other RNA
tttcccttcagagcctggctttccacatattccaaaagctgagatggacaattaagaatcgccatactggagatcacctaggtaaatacacctgtgcagattcttttcatatcaagtacttcaggtgattcagaagaacaaagtttgaaaacaactccagagccataaggaaaatctagtgatgcctttgaaaagaaatgaaactaatcattgattgaacccactactgtgtttcagactgctttggaactttctgacaattttatagcaattatctcacatttagaaatctgcctgattgagaaattcaacataattctgaaaagagagagaaaaaaatataaatctacatatactcttcaatcgtaaaatcataatttataaggtacatttcagcaaacaaaatcaaagcagttcatgaaataatcttattaatactcaaaatgtcctttgagttgcatgctgaggagtagtagcttgtaaatagctatgaaaaaatcaccagaccttcccaaattctatttgcactggctctagccaagtttaacaaatgctaccctctcaccctaataacaacaagcacttccttctttacctttgcgatctgagctcactgcaacctccgtctcccgggttca

SEQ ID NO: 19626 - RNA, 3258 nt, Homo sapiens
  source 1..3258: mol_type = other RNA
tttccctttccatcctggcagaaaaccctcttaaatggcatcggtgattcacccaaagttccatggccttttacaggctggcatgaaaccagaactggaattctgggccgaggccctctgagcagactgcctcgggaggggaggtgctcccgggcaactgagactctgcacctgaacggcccgcagtcaaaggagggtgggagggacatgatggtgtaggccaccggcaggaggctgaggaagagcaccagcagcaggaggcccatgtagaagttgttggatcgggaggctttgaacacgcgttcatggggtacgttgctgctcatcaccgcccagcactggaagtacatggaggtcagcaggcgcagcacattaatgcccaccaggcctggagcatagaaggagcccatccagatcattccttggttgaagatcaaacccagcacatttccactaatatcaaactcagcatatgaaggctgggccaggccaggatgagggatacataggtcaacatcctacggagcctttcaccaggagctcaggtaagaggtaggtaccttacatgcacaccagtgactgcaggctgggccagtgaggtgttgtggaagagacatgtacagcacaggtgcctgagccagagattctgccagagcatagaaggacactacagagaggaaatgacacacatttaccaggtaggtggggaagagggctataagggaatacaagtcaaaggaggtttctcaaagcatcatccagaagacaggaccaatggttattgtgttcttggtgtgttccaggacttcctgaaatattcgcctccactgtcagatttcagcccccataatgagagttgaggctgctcagatgcaattccctatcaaccattggctcagtactggagtgtgtggtccactttcccctaggccaaatgcctccatttcctagaatagaaggtcacattgttcattacactgggaaaaagcagtttcccttatgaaggcaaataggacccttaaaggaaatacaaattaaacactttactactctacagagcagagaccgtcattaagcttccaaagaaatgaaatgcccaagaatgcatctggctataagtatcaaagaagatagttgaaattcctttgtgcggaatgtccatgaagtggtgacctacaaatccagcctccaagtcccagcaccagcagtagttcatgaaccgcacaaaacaagcccgtaggaagtcccccagcaggatggtgatgtacgttaccagcatgtcagacaccgtcagcctcatgaattcaatgcccacagctgtctcccagcaagaaccccggggcacatctgcagggtgcaggggtggtcgggggacactctcgttccaaccagaagagttgtaatagttaaacagagtccagtgagtgatgttctttattgtctcttcattagcaagcttgaggtggacgtcatccatcagggccaagagaaatgtgtagaggttccccaggaagagtgcaaagatgcgtcccagctgccacttcagtccagtgcgtgggtggtaattctccagggcagcgatggtttcaaacagagggggacaaaacattccaagcagggacatcacgatctctacctcattcctttcataccagctgacattctgcattttggagaattgctgagatcgcttaaccacaaagtaaatgaggtacccacttccacacaaacagcagatgatgagaaagttggccaggacacgaagaaatcttgtcagatggatattttcttctttgttactctcttgttcatccactattgattccttgaagctggtggtgatggatgcatatttgttatcagctgtctctgaattcccgatcaggtagtcccagctggtgaacatcttgaagctgaatgtgaagttgtcactctccccttcgcctgtgcttccttgggtattgctggccatcgatcgaatgacaataatcaggctgtagccgaacacgctgacccccaccataaagtaagccataggcagccggtacctcagccacccgatggtcctctggttgttgtagtagccatagaagagtgcagagtacttgatatagccctcaaaatcccaaaggacagaaaaatccatggccttttcttcctcagcccgaggcactgtctttctgggaatactcccatagggcatgcccatcagtacctctgggattatgactagaccaaatattaagccaaaaaggacaaggttaactccatacatccatcggagaaagatgaaatacgatgccactgaagaaccaaagtgactttcaatgtccttgatcttcatttcccaggggatacattgagtcttgaaattatcaaagtctctcttaaatttgacccatttcttggccatcagcatcttgtaggcatatagttgcttgcctttcccctttcccaaggcaccttcatacttctccacaaattcctgggcctccctgagctctgtcagcttcttcgccatgggccagggcttgctccgcatggtggcaatgagcttctttttttcttccacctgctccaggatctgggccagttcctcctcggacagggactccccaccagaggcactggaggccaaggaggatgacctgggtttcttctgccgcttcgacttctcctccctcctcggaatctccttttccctctttggggctgctgtccgctcctggaaggaggccctctcgtcgcgctttctcctgccctcgcaggtcctctctgcctcgccccgctcctgctcccccagctcttctctgtgtctcctgcgccctgtttgcttcctccggggagaccccgggcttgggctgcccccggcgcgctccttctggcttcgctgagctccgcgcctgcctggggtcccctcggctttgagagcccgcttgcttgaggatctccttcccagcctgtcacctgccggggcgggaaaatggacagttctggttccaacggcctcaggcccaggaaaatgtccccggccgtgagaaatcagacgtccaagatgattccgagagcttgtgagctctgcggggctcagaacaggacaccccaaagtatggcaccttggcatgttgagtattttaagctgaaggaaactaagaaaactgcagaagcaggaaggtcactctctggccttctccctcccgtctcccttgaagacctcctgtgacaggtgtcctgccctatacccaaggaaaggaaagt

SEQ ID NO: 19627 - RNA, 93 nt, Homo sapiens
  source 1..93: mol_type = other RNA
tttccctttccatcctggcagcagttccacattgctggggaggtctcagaatcatggtgggaggcgaaaggcacttcttacatggtggcagca

SEQ ID NO: 19628 - RNA, 220 nt, Homo sapiens
  source 1..220: mol_type = other RNA
tttccctttccatcctggcagccaatggggggagaggctatttttcagtgtttcccagagctcctctgagggtctgcttacacagttcctggacttgcactcagtaggcaaggtgataagaataggggttgtctttgtttactgtataccgcccacgcttggcacactgggagctctatccgcgcgccccttccgctttgcggcgcctacactggctcct

SEQ ID NO: 19629 - RNA, 52 nt, Homo sapiens
  source 1..52: mol_type = other RNA
tttccctttccatcctggcagccagaaggaagaaactctgaacacatccgaa

SEQ ID NO: 19630 - RNA, 53 nt, Homo sapiens
  source 1..53: mol_type = other RNA
tttccctttccatcctggcagccagaaggaagaaactctgaacacatccgaac

SEQ ID NO: 19631 - RNA, 67 nt, Homo sapiens
  source 1..67: mol_type = other RNA
tttccctttccatcctggcagcctatccgcgcgccccttccgctttgcggcgcctacactggctcct

SEQ ID NO: 19632 - RNA, 393 nt, Homo sapiens
  source 1..393: mol_type = other RNA
tttccctttccatcctggcagcctgaggcggagagaggccgcttcgcgcctggggctcccgaaagcggccagctgtcctcctgctccccctgagcggggagcgctgcgtctcctgcgggctgcgggagacccttccagactcccgggtgggaaaaccacactgagcgccccgggaggttgccagatacaatactgtatctggcacccctgcccgggtgcccccgcccagttggctggctggctggctagctgtctcccaggtgtgggtaaggaatctccttccatctctgtggcaccttcttcacgctggaggcagctgtttagttccacattgctggggaggtctcagaatcatggtgggaggcgaaaggcacttcttacatggtggcagca

SEQ ID NO: 19633 - RNA, 611 nt, Homo sapiens
  source 1..611: mol_type = other RNA
tttccctttccatcctggcagcctgaggcggagagaggccgcttcgcgcctggggctcccgaaagcggccagctgtcctcctgctccccctgagcggggagcgctgcgtctcctgcgggctgcgggagacccttccagactcccgggtgggaaaaccacactgagcgccccgggaggttgccagatacaatactgtatctggcacccctgcccgggtgcccccgcccagttggctggctggctggctagctgtctcccaggtgtgggtaaggaatctccttccatctctgtggcaccttcttcacgctggaggcagctgtttctgtgggaaagggctttcttatgttgagccaagatgctttttaggagttagaaatggagtcaatatatcttcaaaagcaccttggggcctgtttaactcaaggtcttgcagaagtggcaagagttcgcccagtggatccgatagaatatttagcattgtggatttacaagtataaggaaaatgtgaccatggaacaactggtaagtaggaatctccttagttccacattgctggggaggtctcagaatcatggtgggaggcgaaaggcacttcttacatggtggcagca

SEQ ID NO: 19634 - RNA, 42 nt, Homo sapiens
  source 1..42: mol_type = other RNA
tttccctttccatcctggcagctgcaaaggtctgcagcttca

SEQ ID NO: 19635 - RNA, 737 nt, Homo sapiens
  source 1..737: mol_type = other RNA
tttctatttctcagtggggctcttacctattactcatcaaccttgtaggcagaattgactgatgcagcctacacagtatttaattacataaatgggacaccacctatgtgcccaacatgggatttgataggaaggatttgaaggggttagagacagggagaccaaataggagtctgcccagccacccagctttcgggtaatgtgcgtctggtcttcagggccaacaatagagagaatgtgaaattaagttgatgatggaaatgaaagaaggaggaattgaaagcttctcaactaagaaaccagaagacaagcaacaagagagcatctcatgaaatcacacaacagggtaactgagtgggtatttcctgtgagcagttataaagttagattgtggacgggtacggtggctcatgccactttgggaggccgaggcgcgccgatcacctgaggtcgggagttggagaccagcctgaccaacatggagaaaccccttctctactgataatacaaaaaaattagccaggcgtggtgacgcatgcctgtaatcccagctactcaggaggctgaggcaggagaatcgcttgaactcaggaggcggaggttgcggtgagctgagatcaggccattgcactccagcctggtcaacaagagtgaaactccgtctcaaaaaaaaaaaaaagattcaagtccagattttgctaaagatgataatttgggggttttcagcatggactatg

SEQ ID NO: 19636 - RNA, 845 nt, Homo sapiens
  source 1..845: mol_type = other RNA
tttctctctccacttcctcagaaactttgacactagagaaggtcatcaccacaccatcatcctcactgtttctatctccagccctgtcttcctcactctcgccttgggagtcttccgcgtcatccccttcttccatgccactctcttcgtcttcctcctcctcactgctcccaaggtcatccattcccttggtaaatttctcaaagtcactgatactctggacactgaagcccggtgtttttgcagagtggcttctgctcttcttgctctccctgtgatcaccacactcctgttcctcagcagcacccaggtcgtcctcatcatattcctccagacccagtccctctgaatcttcatctccagacccttcctcatcagatatttcctcatcagacgatcctggcagagtctgctcccaatggtcttcattccatgcttttctagaggtggttttgccgcaataccttttgtccgtgtccaagagggaggctgatgccagttttctaatgctacccactactaggaaatcaccttccccatcttccccttcatcaaacctgtcaatcaccctggcagcagtggcttcctcggggtccgcttcagggtccgcctcgcttggtcgcgggttcaacaactgttccagttgcagcgccaggggctgcggccccgccatcgtcaccagctcccggtccactccgcttcgcgcacgtaaatgtgcggcccaacccccggccccgaagctccttccctgccggatcctctcgccttgatccgattccccgactccgccagagaccgcgcggaggccaccccacagctctggaccggccacttccgggaggcgc

SEQ ID NO: 19637 - RNA, 299 nt, Homo sapiens
  source 1..299: mol_type = other RNA
tttctctctccacttcctcagcgtcccgggcgtcctccccccgactgcagttgctgcaaatgtgtttgatctccttgcctagttgacagtggatcacaaaggacacgttgttgttgttgttgggggcgggctccttcaggggcttcatcctcagcaaataaaaagctttctttttgggtttctcggcgctcgcgcctggcaccgcgccctccctgcagcgcggcgaacggagcgcaaacctccccggcttcgctgagcgcgtgggctccgccatccggcccccgggcgcccggggccgg

SEQ ID NO: 19638 - RNA, 607 nt, Homo sapiens
  source 1..607: mol_type = other RNA
tttctctctccacttcctcagcgtcccgggcgtcctccccccgactgcagttgctgcaaatgtgtttgatctccttgcctagttgacagtggatcacaaaggacacgttgttgttgttgttgggggcgggctccttcaggggcttcatcctcagcaaataaaaagctttctttttgggtttctcggcgctcgcgcctggcaccgcgccctccctgcagcgcggcgaacggagcgcaaacctccccggcttcgctgagcgcgtgggctccgccatccggcccccgggcgcccggggccgggcgctgctccggcccccgcgcgctgccactcgcgcccctcggcctcgccagcatgcccccgccccgcccgcgccggccgctctatataagcaccgccgcggcggggcgggtcggggagggcgccgaaagggtcttgacctcgccgacctcgctgccccagccaatccggatcccgaagccggaggagggggtaggcagggcgctcctgggtcctacctgagaagctccactcccacctctctcggggtctcacgtgcacatcctcctctggcagccccacccctccggaaatctcagcaccagctact

SEQ ID NO: 19639 - RNA, 317 nt, Homo sapiens
  source 1..317: mol_type = other RNA
tttctctctccacttcctcagctgcccccaggttaaaggagatcctggcctctgcgaggtacggcgtgtcgctcttggagcgcactctccggatgggccgccggtctatatcatcctccgaggatgccgccattaatgtgggaggcaggagcagggtcgcccggcgagcttgagctccttgactgtagaagaatctttgagctgactcaacatccaagagtctgtgagcagactctacatccagaaaataatccattttgggataatccatccttgatgttccaaacacagagttttgagagaaaacactggaacac

SEQ ID NO: 19640 - RNA, 465 nt, Homo sapiens
  source 1..465: mol_type = other RNA
tttctctctccacttcctcagctgcccccaggttaaaggagatcctggcctctgcgaggtacggcgtgtcgctcttggagcgcactctccggatgggccgccggtctatatcatcctccgaggatgccgccattaatgtgggaggcaggagcagggtcgcccggcgagcttgagctccttgactgtagaagaatctttgagctgactcaacatccaagagtctgtgagcagactctacatccagaaaataatccattttgggataatccatccttgatgttccaaacacagagttttgagagaaaacactggaacaccagcctttccttgctttatattctctggaacatatactgttaaattcacatgctatcagttttcaaaaggtctatttgataaatagcgtcattaagtgtcagccgttgtgagtgttgatcctcagctcatcctgggactttcggattc

SEQ ID NO: 19641 - RNA, 600 nt, Homo sapiens
  source 1..600: mol_type = other RNA
tttctctctccacttcctcagctgcccccaggttaaaggagatcctggcctctgcgaggtacggcgtgtcgctcttggagcgcactctccggatgggccgccggtctatatcatcctccgaggatgccgccattaatgtgggaggcaggagcagggtcgcccggcgagcttgagctccttgactgtagaagaatctttgagctgactcaacatccaagagtctgtgagcagactctacatccagaaaataatccattttgggataatccatccttgatgttccaaacacagagttttgagagaaaacactggaacaccagcctttccttgctttatattctctggaacatatactgttaaattcacatgctatcagttttcaaaaggtctatttgataaatagcgtcattaagtgtcagccgttgtgagtgttgatcctcagctcatcctgggactttcggattcccctggagcagggaaaattgcctgggaatccgagcctccactcatagatgccgtgcgtttatgacacacactgacatatttgctgtacaaatgctttgaattccttcctttccggcgattcccttcagcacattt

SEQ ID NO: 19642 - RNA, 447 nt, Homo sapiens
  source 1..447: mol_type = other RNA
tttctctctccacttcctcagctgcccccaggttaaaggagatcctggcctctgcgaggtacggcgtgtcgctcttggagcgcactctccggatgggccgccggtctatatcatcctccgaggatgccgccattaatgtgggaggcaggagcagggtcgcccggcgagcttgagctccttgactgtagaagaatctttgagctgactcaacatccaagagtctgtgagcagactctacatccagaaaataatccattttgggataatccatccttgatgttccaaacacagagttttgagagaaaacactggaacaccggcacttgttgacccctttcaacaggacacggtagagtacaaaacaaagcagtgcgacgcttctgagcccgcaagcacaaatgaacagcttctaattttcccttcaatctcgcttcaagagcactgagc

SEQ ID NO: 19643 - RNA, 579 nt, Homo sapiens
  source 1..579: mol_type = other RNA
tttctctctccacttcctcagctgcccccaggttaaaggagatcctggcctctgcgaggtacggcgtgtcgctcttggagcgcactctccggatgggccgccggtctatatcatcctccgaggatgccgccattaatgtgggaggcaggagcagggtcgcccggcgagcttgagctccttgactgtagaagaatctttgagctgactcaacatccaagagtctgtgagcagactctacatccagaaaataatccattttgggataatccatccttgatgttccaaacacagagttttgagagaaaacactggaacaccggcacttgttgacccctttcaacaggacacggtagagtacaaaacaaagcagtgcgacgcttctgagcccgcaagcacaaatgaacagcttctaattttcccttcaatctcgcttcaagagcactgagcagagggaagtgatggatttgcccatttatactgtgatgaaatgcaacccttaagaagagatctgagtggagctgctctttagaacacattagactgctaatttaagaaaattgaaaggttttgttttactgt

SEQ ID NO: 19644 - RNA, 492 nt, Homo sapiens
  source 1..492: mol_type = other RNA
tttctctctccacttcctcagctgcccccaggttaaaggagatcctggcctctgcgaggtacggcgtgtcgctcttggagcgcactctccggatgggccgccggtctatatcatcctccgaggatgccgccattaatgtgggaggcaggagcagggtcgcccggcgagcttgagctccttgactgtagaagaatctttgagctgactcaacatccaagagtctgtgagcagactctacatccagaaaataatccattttgggataatccatccttgatgttccaaacacagagttttgagagaaaacactggaacaccttagcaacggaaggtgacgccagcctcagcctctgcaccctccccggcacttgttgacccctttcaacaggacacggtagagtacaaaacaaagcagtgcgacgcttctgagcccgcaagcacaaatgaacagcttctaattttcccttcaatctcgcttcaagagcactgagc

SEQ ID NO: 19645 - RNA, 603 nt, Homo sapiens
  source 1..603: mol_type = other RNA
tttctctctccacttcctcagctgcccccaggttaaaggagatcctggcctctgcgaggtacggcgtgtcgctcttggagcgcactctccggatgggccgccggtctatatcatcctccgaggatgccgccattaatgtgggaggcaggagcagggtcgcccggcgagcttgagctccttgactgtagaagaatctttgagctgactcaacatccaagagtctgtgagcagactctacatccagaaaataatccattttgggataatccatccttgatgttccaaacacagagttttgagagaaaacactggaacaccttagcaacggaaggtgacgccagcctcagcctctgcaccctccccggcacttgttgacccctttcaacaggacacggtagagtacaaaacaaagcagtgcgacgcttctgagcccgcaagcacaaatgaacagcttctaattttcccttcaatctcgcttcaagagcactgagcagagggaagtgatggatttgcccatttatactgtgatgaaatgcaacccttaagaagagatctgagtggagctgctctttagaacacattagactgctaatttaagaaaat

SEQ ID NO: 19646 - RNA, 635 nt, Homo sapiens
  source 1..635: mol_type = other RNA
tttctctctccacttcctcagctgcccccaggttaaaggagatcctggcctctgcgaggtacggcgtgtcgctcttggagcgcactctccggatgggccgccggtctatatcatcctccgaggatgccgccattaatgtgggaggcaggagcagggtcgcccggcgagcttgagctccttgactgtagaagaatctttgagctgactcaacatccaagagtctgtgagcagactctacatccagaaaataatccattttgggataatccatccttgatgttccaaacacagagttttgagagaaaacactggaacactgcaaaaaataaaaatcaaaggctatctgtcagcggtaaaacaagagccgttccagccagagtgtctttgatcttgctaaatattcccggtgaaagtaaacgattttgattgtttgattagaacagtgatgaataatgcatacagtccactggacttcctttatcagataaaatggccagagcacgttaccttagcaacggaaggtgacgccagcctcagcctctgcaccctccccggcacttgttgacccctttcaacaggacacggtagagtacaaaacaaagcagtgcgacgcttctgagcccgcaagcacaaat

SEQ ID NO: 19647 - RNA, 682 nt, Homo sapiens
  source 1..682: mol_type = other RNA
tttctctctccacttcctcagctgcccccaggttaaaggagatcctggcctctgcgaggtacggcgtgtcgctcttggagcgcactctccggatgggccgccggtctatatcatcctccgaggatgccgccattaatgtgggaggcaggagcagggtcgcccggcgagcttgagctccttgactgtagaagaatctttgagctgactcaacatccaagagtctgtgagcagactctacatccagaaaataatccattttgggataatccatccttgatgttccaaacacagagttttgagagaaaacactggaacactgcaaaaaataaaaatcaaaggctatctgtcagcggtaaaacaagagccgttccagccagagtgtctttgatcttgctaaatattcccggtgaaagtaaacgattttgattgtttgattagaacagtgatgaataatgcatacagtccactggacttcctttatcagataaaatggccagagcacgttaccttagcaacggaaggtgacgccagcctcagcctctgcaccctccccggcacttgttgacccctttcaacaggacacggtagagtacaaaacaaagcagtgcgacgcttctgagcccgcaagcacaaatgaacagcttctaattttcccttcaatctcgcttcaagagcactgagc

SEQ ID NO: 19648 - RNA, 82 nt, Homo sapiens
  source 1..82: mol_type = other RNA
tttctctctccacttcctcagcttaaaggctgcccaaagctctttgctcccacatgcatccgcctctctgggtctgtttcct

SEQ ID NO: 19649 - RNA, 482 nt, Homo sapiens
  source 1..482: mol_type = other RNA
tttctctctccacttcctcagcttaaaggctgcccaaagctctttgctcccacatgcatccgcctctctgggtctgtttcctggctttccaatagctgtgctttcttaaattgagcaacagtctcctcaagtgtcgggctctgaaaatacacatgctacacacgcccatgcagcctctcggtgccaggcagccccttcgccttccttcccggccgtgccaattccctggccgctgaccagctcccacgtgggatggaatggagaaggggagggtgtcaaccaaagtcgggggatggattcaactcaccgtggactaggtggccacccatctggcatgaagggtccattttatcccttttctaacctaaaaccgcctccacgatggtctctccagcctcactcagagcccagaacagttggcaggcacaccaacccctcctgggtgtgacctgcgggtactcagacgtctctaaagtggcagc

SEQ ID NO: 19650 - RNA, 752 nt, Homo sapiens
  source 1..752: mol_type = other RNA
tttctctctccacttcctcagcttaaaggctgcccaaagctctttgctcccacatgcatccgcctctctgggtctgtttcctggctttccaatagctgtgctttcttaaattgagcaacagtctcctcaagtgtcgggctctgaaaatacacatgctacacacgcccatgcagcctctcggtgccaggcagccccttcgccttccttcccggccgtgccaattccctggccgctgaccagctcccacgtgggatggaatggagaaggggagggtgtcaaccaaagtcgggggatggattcaactcaccgtggactaggtggccacccatctggcatgaagggtccattttatcccttttctaacctaaaaccgcctccacgatggtctctccagcctcactcagagcccagaacagttggcaggcacaccaacccctcctgggtgtgacctgcgggtactcagacgtctctaaagtggcagcctccagccggtggggcacagactgcctcttaccttcacagagccccagtccttagaagcccagctggcgtctccaaggagtcctgcgttttacttgacattggaggcaaccggttgcagaaacagggaacatttcaaaatgaaacagaaagtaacccggggatccaaaccagacccccgacctgcctcggccgtccccaatctctgggagtcttctgactcagcaagcctgtacagctgtttcagcctggagaggattcagaggaaatgc

SEQ ID NO: 19651 - RNA, 259 nt, Homo sapiens
  source 1..259: mol_type = other RNA
tttctctctccacttcctcagcttcacagagccccagtccttagaagcccagctggcgtctccaaggagtcctgcgttttacttgacattggaggcaaccggttgcagaaacagggaacatttcaaaatgaaacagaaagtaacccggggatccaaaccagacccccgacctgcctcggccgtccccaatctctgggagtcttctgactcagcaagcctgtacagctgtttcagcctggagaggattcagaggaaatgc

SEQ ID NO: 19652 - RNA, 282 nt, Homo sapiens
  source 1..282: mol_type = other RNA
tttctctctccacttcctcagcttcacagagccccagtccttagaagcccagctggcgtctccaaggagtcctgcgttttacttgacattggaggcaaccggttgcagaaacagggaacatttcaaaatgaaacagaaagtaacccggggatccaaaccagacccccgacctgcctcggccgtccccaatctctgggagtcttctgactcagcaagcctgtacagctgtttcagcctggagaggattcagaggaaatgcagcttggaagtctggaactcaca

SEQ ID NO: 19653 - RNA, 287 nt, Homo sapiens
  source 1..287: mol_type = other RNA
tttctctctccacttcctcagcttcacagagccccagtccttagaagcccagctggcgtctccaaggagtcctgcgttttacttgacattggaggcaaccggttgcagaaacagggaacatttcaaaatgaaacagaaagtaacccggggatccaaaccagacccccgacctgcctcggccgtccccaatctctgggagtcttctgactcagcaagcctgtacagctgtttcagcctggagaggattcagaggaaatgcagcttggaagtctggaactcacagcctg

SEQ ID NO: 19654 - RNA, 2879 nt, Homo sapiens
  source 1..2879: mol_type = other RNA
tttctgtcttttctggtccagcccatccagttcaggggcatcaagggggctgaggccccggtagccactgtagaccctgtgactatcactgacaccgtcactgggctccattgggcaaatgtagtccgtcgattcatcgaacttcttttttcttatgtttccgaagtgtgaaaatcctagtttccttggccggactttggctgtggtggtcagtggtgtgtaagctggtgaggccattttctctcgcttctcctgttcagcctccggaccaatcaaggcattgaacttggtggtcaggtggcgcctgaggagcgtcttttgtggggggatgttgagaagcatagccagggtgtccccagtgaagcgtggctccaggataatgaggcctccatggactccactccctcgaagattgggtgcatactctgccaggtccacagatcgtaaccactccatcaccctgtggttggaccactgtacaacttctgaaggagaaaggttactctcatcagctggccgccggtgcaggcagtgggggttgaacttgttgacatgcagcacgtgaatggcacatttgatgctgagatgatgtagttggctggtgacttttaagaagagtaaatcgttcacagttaggtattgcagcattcgtctgtcaactctagattcatgaaactggtctttgtactggggtaagccaatatcatcaagccaccttgtcacccaaatgtggtctagcagtgcagacttctcctcctgtttggtgttgatggctttcactgctaaaacaagcttcttcctgtggagtgggtgcttaattcctagctccttttccatgtcctgaggggtggctgtcaataaggtgtggccagaagatacccactgcctggcaaagatcacatactgagccaggccaaagtcctccagccatgcacacacacgctctgtgctccactgggcaaagggggcattggcgtcacttttctgtcccttggagtccctggtcctagagagtcttggccctgcggttgcccggagcccacctcgtcgaaactctgccatccccagcgtgtcagtgtagaaatttcctgactgagttcttcggatttttccccagaacttcttaatgcctttgggattccgtttaccatctggtgtcagaggagactgaggacctgattcagtgcccgatgatgtggatgagaggtcattgaccacagcagtgtcgtcccagccactttctgtgtctcctaatacgggggcactgacactccggccacgattcagcctcagcaggctgctccccgtggcgtcaggctggcagatggtgggaggagatttggcagcctctccattgggcgtggctcctgaaagcttcccaggtaaagtgggatatttgtgctccgccaagaaagggctgtccttgggttctaacaccgggaagggctggttcccatccatacacttatccacagattcacttctcaagtcttctagactacaagagagctttttctgagccctggtttccagtgatttctgtggcaatggaggtggccccactgtaggagagctacatcttggaggcatctcttgtttaaataattcttcagggtccttatttgtagcgttccacttgctgaaacctccctccggttcttcttcattgattgagagagttctctccgaaggcccttgagtgaccatcacaatctcctttaccttccggtactggtttaacagccccgtaagctcctctatccgacggtccttatcttcattggcaagcagcaaagtttccatccccattttcagacgttgaatttcttggtctctctctgtgtgactctcactgtggagagctgctgtccgggagagctggctgtgcagacgctcaatttctgcatctttcagggccacctgttcttgcagctgggcgacttcagccttagtggcctttagcttccattcatactgattcctttcattttccaactcttccactttgattttgaggtgcctgagctcttgcagtaactcctctgcttttctctgcttctcctcctgctctctctgctccttctccatgccaaccagcttgagcttcagctcagacacttcagtcatcagatcgagcttctgggtctcaagagatgtgcggcttagcagctcctgttgaagcatctcttcagcagcattgagtttcacctggtgtccttccagacacacttccaggtctcgaatcttttctccctgggcttctacttggtctgtgaggacactcacctgcaatatgagggactccttatccccttctagacgtgccaagcgttcctggtaggtttcattactagcagcactgtggtggtttacctgggacaagctctcttcaaaccattcctttatgtaggcagctgttgggccagggatctggctcaggagggctgctctctcctgaggaagctccagcatctccaaggccagcctcaagtcctcgatgagatggagcaccgggaaggggttcatgtaggaggccggggaagccagtccaggctcacaagtaccatcactaagatctgcacctgttttagtgcctgcaatgatcccgtccatttgctccagggcagcttccagcgcatgactagcatcagaagccatgactccttttgcctgcctggcctcctcctcttcttactgggtacggggccgaggctcctctccgggcggctcaggtgtgcgggccgctcccgtgtccctcccaccttcaaacatgagagcccagaagcgagcgacgggccactggcccaccgaccaactgccggaccaagcgcccgaccaaccagcggaccgaccgcagcggccggggccggcgcccacgt

SEQ ID NO: 19655 - RNA, 29 nt, Homo sapiens
  source 1..29: mol_type = other RNA
tttcttcttagacatggcaacgtcaacag

SEQ ID NO: 19656 - RNA, 960 nt, Homo sapiens
  source 1..960: mol_type = other RNA
tttcttcttagacatggcagctactgcatcttcatgtgtcacaaactctacatctgcttctcctgtggctctgccatcagctccaatatcaatatgaactcgtattggatttagtggtgagaagaaattagcaatgtcattttcagttgcacgaaaaggcaaccctctcatatgtacgaaatgaccaccatgaaaacctgaacttgcatcaccagctccaccatagccatgtcctcccatacctcttccatctctcattctgtcatcaaagccatcattcccatagccgtaattattatagccaccatagtcatcaaaacctccataaccaccatcatatccatcacctcctcgtcgcattctgtcatacatacttccacgcccagctccataataaccccctcttcctcctattggtctatcatatggtcccggtcgctgtcccagcaatcttcttggtggatcataaaatcctttgatttcactcctgctacttctgaagatctcaatatacctgtgccctattctttccttgtgtttccccagagcattttctgctatctcctttgaagcaaactgcacgaaggcctcccctgtgcttctcccctggtagtccatcgtcaatgttatcccatttggcacgatttccaacccttgaaagaactgaactatttcctctttgctgcaaccaaatggtagtccacgaagtcgtactgtcccatcactagcgtcatttggaccattatgtttcataacccaatccatctcaataccgtttgatttaaatgccccttttacttcagataccctgtcaggcgatagttacgccgactctggtgctcgcggggtccagttcaaagaagggagaagtcgtttgcctcgtgtagcgctcgccacaacggttctcccaaccgtctccagcggtgacaaccgcttagggagctgcgcagcacagctact

SEQ ID NO: 19657 - RNA, 941 nt, Homo sapiens
  source 1..941: mol_type = other RNA
tttcttcttagacatggcagctactgcatcttcatgtgtcacaaactctacatctgcttctcctgtggctctgccatcagctccaatatcaatatgaactcgtattggatttagtggtgagaagaaattagcaatgtcattttcagttgcacgaaaaggcaaccctctcatatgtacgaaatgaccaccatgaaaacctgaacttgcatcaccagctccaccatagccatgtcctcccatacctcttccatctctcattctgtcatcaaagccatcattcccatagccgtaattattatagccaccatagtcatcaaaacctccataaccaccatcatatccatcacctcctcgtcgcattctgtcatacatacttccacgcccagctccataataaccccctcttcctcctattggtctatcatatggtcccggtcgctgtcccagcaatcttcttggtggatcataaaatcctttgatttcactcctgctacttctgaagatctcaatatacctgtgccctattctttccttgtgtttccccagagcattttctgctatctcctttgaagcaaactgcacgaaggcctcccctgtgcttctcccctggtagtccatcgtcaatgttatcccatttggcacgatttccaacccttgaaagaactgaactatttcctctttgctgcaaccaaatggtagtccacgaagtcgtactgtcccatcactagcgtcatttggaccattatgtttcataacccaatccatctcaataccgtttgatttaaatgcctgtcaggcgatagttacgccgactctggtgctcgcggggtccagttcaaagaagggagaagtcgtttgcctcgtgtagcgctcgccacaacggttctcccaaccgtctccagcggtgacaaccgcttagggagctgcgcagcacagctact

SEQ ID NO: 19658 - RNA, 922 nt, Homo sapiens
  source 1..922: mol_type = other RNA
tttcttcttagacatggcagctactgcatcttcatgtgtcacaaactctacatctgcttctcctgtggctctgccatcagctccaatatcaatatgaactcgtattggatttagtggtgagaagaaattagcaatgtcattttcagttgcacgaaaaggcaaccctctcatatgtacgaaatgaccaccatgaaaacctgaacttgcatcaccagctccaccatagccatgtcctcccatacctcttccatctctcattctgtcatcaaagccatcattcccatagccgtaattattatagccaccatagtcatcaaaacctccataaccaccatcatatccatcacctcctcgtcgcattctgtcatacatacttccacgcccagctccataataaccccctcttcctcctattggtctatcatatggtcccggtcgctgtcccagcaatcttcttggtggatcataaaatcctttgatttcactcctgctacttctgaagatctcaatatacctgtgccctattctttccttgtgtttccccagagcattttctgctatctcctttgaagcaaactgcacgaaggcctcccctgtgcttctcccctggtagtccatcgtcaatgttatcccatttggcacgatttccaacccttgaaagaactgaactatttcctctttgctgcaaccaaatggtagtccacgaagtcgtactgtcccatcactagcgtcatttggaccattatgtttcataacccaatccatctcaataccgtttgatttaaatggccgactctggtgctcgcggggtccagttcaaagaagggagaagtcgtttgcctcgtgtagcgctcgccacaacggttctcccaaccgtctccagcggtgacaaccgcttagggagctgcgcagcacagctact

SEQ ID NO: 19659 - RNA, 1078 nt, Homo sapiens
  source 1..1078: mol_type = other RNA
tttcttcttagacatggcagctactgcatcttcatgtgtcacaaactctacatctgcttctcctgtggctctgccatcagctccaatatcaatatgaactcgtattggatttagtggtgagaagaaattagcaatgtcattttcagttgcacgaaaaggcaaccctctcatatgtacgaaatgaccaccatgaaaacctgaacttgcatcaccagctccaccatagccatgtcctcccatacctcttccatctctcattctgtcatcaaagccatcattcccatagccgtaattattatagccaccatagtcatcaaaacctccataaccaccatcatatccatcacctcctcgtcgcattctgtcatacatacttccacgcccagctccataataaccccctcttcctcctattggtctatcatatggtcccggtcgctgtcccagcaatcttcttggtggatcataaaatcctttgatttcactcctgctacttctgaagatctcaatatacctgtgccctattctttccttgtgtttccccagagcattttctgctatctcctttgaagcaaactgcacgaaggcctcccctgtgcttctcccctggtagtccatcgtcaatgttatcccatttggcacgatttccaacccttgaaagaactgaactatttcctctttgctgcaaccaaatggtagtccacgaagtcgtactgtcccatcactagcgtcatttggaccattatgtttcataacccaatccatctcaataccgtttgatttaaatgtcttttcgaagttccaaatctggaatataagggccggctaagcgtcctttattcctcccaggagactttccgtttatctagctgccctagagaccagaaagctagggagagtacgccccttccccctcccgtcagcagccaagcctggcttaaaacccttcgccaccgggcggcagaattacaaaggaggccgtctgcctcctttgtcctggatttgggagttgagcaccttcgtcgccattggctttcctcccccagctccagcctctctcatcttgggaatctgcgtc

SEQ ID NO: 19660 - RNA, 821 nt, Homo sapiens
  source 1..821: mol_type = other RNA
tttcttcttagacatggcagctactgcatcttcatgtgtcacaaactctacatctgcttctcctgtggctctgccatcagctccaatatcaatatgaactcgtattggatttagtggtgagaagaaattagcaatgtcattttcagttgcacgaaaaggcaaccctctcatatgtacgaaatgaccaccatgaaaacctgaacttgcatcaccagctccaccatagccatgtcctcccatacctcttccatctctcattctgtcatcaaagccatcattcccatagccgtaattattatagccaccatagtcatcaaaacctccataaccaccatcatatccatcacctcctcgtcgcattctgtcatacatacttccacgcccagctccataataaccccctcttcctcctattggtctatcatatggtcccggtcgctgtcccagcaatcttcttggtggatcataaaatcctttgatttcactcctgctacttctgaagatctcaatataccttgaaagaactgaactatttcctctttgctgcaaccaaatggtagtccacgaagtcgtactgtcccatcactagcgtcatttggaccattatgtttcataacccaatccatctcaataccgtttgatttaaatgccccttttacttcagataccctgtcaggcgatagttacgccgactctggtgctcgcggggtccagttcaaagaagggagaagtcgtttgcctcgtgtagcgctcgccacaacggttctcccaaccgtctccagcggtgacaaccgcttagggagctgcgcagcacagctact

SEQ ID NO: 19661 - RNA, 802 nt, Homo sapiens
  source 1..802: mol_type = other RNA
tttcttcttagacatggcagctactgcatcttcatgtgtcacaaactctacatctgcttctcctgtggctctgccatcagctccaatatcaatatgaactcgtattggatttagtggtgagaagaaattagcaatgtcattttcagttgcacgaaaaggcaaccctctcatatgtacgaaatgaccaccatgaaaacctgaacttgcatcaccagctccaccatagccatgtcctcccatacctcttccatctctcattctgtcatcaaagccatcattcccatagccgtaattattatagccaccatagtcatcaaaacctccataaccaccatcatatccatcacctcctcgtcgcattctgtcatacatacttccacgcccagctccataataaccccctcttcctcctattggtctatcatatggtcccggtcgctgtcccagcaatcttcttggtggatcataaaatcctttgatttcactcctgctacttctgaagatctcaatataccttgaaagaactgaactatttcctctttgctgcaaccaaatggtagtccacgaagtcgtactgtcccatcactagcgtcatttggaccattatgtttcataacccaatccatctcaataccgtttgatttaaatgcctgtcaggcgatagttacgccgactctggtgctcgcggggtccagttcaaagaagggagaagtcgtttgcctcgtgtagcgctcgccacaacggttctcccaaccgtctccagcggtgacaaccgcttagggagctgcgcagcacagctact

SEQ ID NO: 19662 - RNA, 811 nt, Homo sapiens
  source 1..811: mol_type = other RNA
tttcttcttagacatggcagctactgcatcttcatgtgtcacaaactctacatctgcttctcctgtggctctgccatcagctccaatatcaatatgaactcgtattggatttagtggtgagaagaaattagcaatgtcattttcagttgcacgaaaaggcaaccctctcatatgtacgaaatgaccaccatgaaaacctgaacttgcatcaccagctccaccatagccatgtcctcccatacctcttccatctctcattctgtcatcaaagccatcattcccatagccgtaattattatagccaccatagtcatcaaaacctccataaccaccatcatatccatcacctcctcgtcgcattctgtcatacatacttccacgcccagctccataataaccccctcttcctcctattggtctatcatatggtcccggtcgctgtcccagcaatcttcttggtggatcataaaatcctttgatttcactcctgctacttctgaagatctcaatataccttgaaagaactgaactatttcctctttgctgcaaccaaatggtagtccacgaagtcgtactgtcccatcactagcgtcatttggaccattatgtttcataacccaatccatctcaataccgtttgatttaaatgcgtttttcttgcttacgttagaaccatccagttttcagagcgtaccattctgccgcctcggggcgatggcaatggcagttctgccagtgtgtagaaggaaccgtgccgtagcgctctggagaagttctccggtgatctgcccccaccgtgaacaaattctgt

SEQ ID NO: 19663 - RNA, 783 nt, Homo sapiens
  source 1..783: mol_type = other RNA
tttcttcttagacatggcagctactgcatcttcatgtgtcacaaactctacatctgcttctcctgtggctctgccatcagctccaatatcaatatgaactcgtattggatttagtggtgagaagaaattagcaatgtcattttcagttgcacgaaaaggcaaccctctcatatgtacgaaatgaccaccatgaaaacctgaacttgcatcaccagctccaccatagccatgtcctcccatacctcttccatctctcattctgtcatcaaagccatcattcccatagccgtaattattatagccaccatagtcatcaaaacctccataaccaccatcatatccatcacctcctcgtcgcattctgtcatacatacttccacgcccagctccataataaccccctcttcctcctattggtctatcatatggtcccggtcgctgtcccagcaatcttcttggtggatcataaaatcctttgatttcactcctgctacttctgaagatctcaatataccttgaaagaactgaactatttcctctttgctgcaaccaaatggtagtccacgaagtcgtactgtcccatcactagcgtcatttggaccattatgtttcataacccaatccatctcaataccgtttgatttaaatggccgactctggtgctcgcggggtccagttcaaagaagggagaagtcgtttgcctcgtgtagcgctcgccacaacggttctcccaaccgtctccagcggtgacaaccgcttagggagctgcgcagcacagctact

SEQ ID NO: 19664 - RNA, 939 nt, Homo sapiens
  source 1..939: mol_type = other RNA
tttcttcttagacatggcagctactgcatcttcatgtgtcacaaactctacatctgcttctcctgtggctctgccatcagctccaatatcaatatgaactcgtattggatttagtggtgagaagaaattagcaatgtcattttcagttgcacgaaaaggcaaccctctcatatgtacgaaatgaccaccatgaaaacctgaacttgcatcaccagctccaccatagccatgtcctcccatacctcttccatctctcattctgtcatcaaagccatcattcccatagccgtaattattatagccaccatagtcatcaaaacctccataaccaccatcatatccatcacctcctcgtcgcattctgtcatacatacttccacgcccagctccataataaccccctcttcctcctattggtctatcatatggtcccggtcgctgtcccagcaatcttcttggtggatcataaaatcctttgatttcactcctgctacttctgaagatctcaatataccttgaaagaactgaactatttcctctttgctgcaaccaaatggtagtccacgaagtcgtactgtcccatcactagcgtcatttggaccattatgtttcataacccaatccatctcaataccgtttgatttaaatgtcttttcgaagttccaaatctggaatataagggccggctaagcgtcctttattcctcccaggagactttccgtttatctagctgccctagagaccagaaagctagggagagtacgccccttccccctcccgtcagcagccaagcctggcttaaaacccttcgccaccgggcggcagaattacaaaggaggccgtctgcctcctttgtcctggatttgggagttgagcaccttcgtcgccattggctttcctcccccagctccagcctctctcatcttgggaatctgcgtc

SEQ ID NO: 19665 - RNA, 942 nt, Homo sapiens
  source 1..942: mol_type = other RNA
tttcttcttagacatggcagctactgcatcttcatgtgtcacaaactctacatctgcttctcctgtggctctgccatcagctccaatatcaatatgaactcgtattggatttagtggtgagaagaaattagcaatgtcattttcagttgcacgaaaaggcaaccctctcatatgtacgaaatgaccaccatgaaaacctgaacttgcatcaccagctccaccatagccatgtcctcccatacctcttccatctctcattctgtcatcaaagccatcattcccatagccgtaattattatagccaccatagtcatcaaaacctccataacctcctcgtcgcattctgtcatacatacttccacgcccagctccataataaccccctcttcctcctattggtctatcatatggtcccggtcgctgtcccagcaatcttcttggtggatcataaaatcctttgatttcactcctgctacttctgaagatctcaatatacctgtgccctattctttccttgtgtttccccagagcattttctgctatctcctttgaagcaaactgcacgaaggcctcccctgtgcttctcccctggtagtccatcgtcaatgttatcccatttggcacgatttccaacccttgaaagaactgaactatttcctctttgctgcaaccaaatggtagtccacgaagtcgtactgtcccatcactagcgtcatttggaccattatgtttcataacccaatccatctcaataccgtttgatttaaatgccccttttacttcagataccctgtcaggcgatagttacgccgactctggtgctcgcggggtccagttcaaagaagggagaagtcgtttgcctcgtgtagcgctcgccacaacggttctcccaaccgtctccagcggtgacaaccgcttagggagctgcgcagcacagctact

SEQ ID NO: 19666 - RNA, 923 nt, Homo sapiens
  source 1..923: mol_type = other RNA
tttcttcttagacatggcagctactgcatcttcatgtgtcacaaactctacatctgcttctcctgtggctctgccatcagctccaatatcaatatgaactcgtattggatttagtggtgagaagaaattagcaatgtcattttcagttgcacgaaaaggcaaccctctcatatgtacgaaatgaccaccatgaaaacctgaacttgcatcaccagctccaccatagccatgtcctcccatacctcttccatctctcattctgtcatcaaagccatcattcccatagccgtaattattatagccaccatagtcatcaaaacctccataacctcctcgtcgcattctgtcatacatacttccacgcccagctccataataaccccctcttcctcctattggtctatcatatggtcccggtcgctgtcccagcaatcttcttggtggatcataaaatcctttgatttcactcctgctacttctgaagatctcaatatacctgtgccctattctttccttgtgtttccccagagcattttctgctatctcctttgaagcaaactgcacgaaggcctcccctgtgcttctcccctggtagtccatcgtcaatgttatcccatttggcacgatttccaacccttgaaagaactgaactatttcctctttgctgcaaccaaatggtagtccacgaagtcgtactgtcccatcactagcgtcatttggaccattatgtttcataacccaatccatctcaataccgtttgatttaaatgcctgtcaggcgatagttacgccgactctggtgctcgcggggtccagttcaaagaagggagaagtcgtttgcctcgtgtagcgctcgccacaacggttctcccaaccgtctccagcggtgacaaccgcttagggagctgcgcagcacagctact

SEQ ID NO: 19667 - RNA, 803 nt, Homo sapiens
  source 1..803: mol_type = other RNA
tttcttcttagacatggcagctactgcatcttcatgtgtcacaaactctacatctgcttctcctgtggctctgccatcagctccaatatcaatatgaactcgtattggatttagtggtgagaagaaattagcaatgtcattttcagttgcacgaaaaggcaaccctctcatatgtacgaaatgaccaccatgaaaacctgaacttgcatcaccagctccaccatagccatgtcctcccatacctcttccatctctcattctgtcatcaaagccatcattcccatagccgtaattattatagccaccatagtcatcaaaacctccataacctcctcgtcgcattctgtcatacatacttccacgcccagctccataataaccccctcttcctcctattggtctatcatatggtcccggtcgctgtcccagcaatcttcttggtggatcataaaatcctttgatttcactcctgctacttctgaagatctcaatataccttgaaagaactgaactatttcctctttgctgcaaccaaatggtagtccacgaagtcgtactgtcccatcactagcgtcatttggaccattatgtttcataacccaatccatctcaataccgtttgatttaaatgccccttttacttcagataccctgtcaggcgatagttacgccgactctggtgctcgcggggtccagttcaaagaagggagaagtcgtttgcctcgtgtagcgctcgccacaacggttctcccaaccgtctccagcggtgacaaccgcttagggagctgcgcagcacagctact

SEQ ID NO: 19668 - RNA, 617 nt, Homo sapiens
  source 1..617: mol_type = other RNA
tttcttcttagacatggcagctactgcatcttcatgtgtcacaaactctacatctgcttctcctgtggctctgccatcagctccaatatcaatatgaactcgtattggatttagtggtgagaagaaattagcaatgtcattttcagttgcacgaaaaggcaaccctctcatatgtacgaaatgaccaccatgaaaacctgaacttgcatcaccagctccaccatagccatgtcctcccatacctcttccatctctcattctgtcatcaaagccatcattcccatagccgtaattattatagccaccatagtcatcaaaacctccataaccttgaaagaactgaactatttcctctttgctgcaaccaaatggtagtccacgaagtcgtactgtcccatcactagcgtcatttggaccattatgtttcataacccaatccatctcaataccgtttgatttaaatgcctgtcaggcgatagttacgccgactctggtgctcgcggggtccagttcaaagaagggagaagtcgtttgcctcgtgtagcgctcgccacaacggttctcccaaccgtctccagcggtgacaaccgcttagggagctgcgcagcacagctact

SEQ ID NO: 19669 - RNA, 915 nt, Homo sapiens
  source 1..915: mol_type = other RNA
tttcttcttagacatggcagctactgcatcttcatgtgtcacaaactctacatctgcttctcctgtggctctgccatcagctccaatatcaatatgaactcgtattggatttagtggtgagaagaaattagcaatgtcattttcagttgcacgaaaaggcaaccctctcatatgtacgaaatgaccaccatgaaaacctgaacttgcatcaccagctccaccatagccatgtcctcccatacctcttccatctctcattctgtcatcaaagccatcattcccatagccgtaattattatagccaccatagtcatcaaaacctccataacttccacgcccagctccataataaccccctcttcctcctattggtctatcatatggtcccggtcgctgtcccagcaatcttcttggtggatcataaaatcctttgatttcactcctgctacttctgaagatctcaatatacctgtgccctattctttccttgtgtttccccagagcattttctgctatctcctttgaagcaaactgcacgaaggcctcccctgtgcttctcccctggtagtccatcgtcaatgttatcccatttggcacgatttccaacccttgaaagaactgaactatttcctctttgctgcaaccaaatggtagtccacgaagtcgtactgtcccatcactagcgtcatttggaccattatgtttcataacccaatccatctcaataccgtttgatttaaatgccccttttacttcagataccctgtcaggcgatagttacgccgactctggtgctcgcggggtccagttcaaagaagggagaagtcgtttgcctcgtgtagcgctcgccacaacggttctcccaaccgtctccagcggtgacaaccgcttagggagctgcgcagcacagctact

SEQ ID NO: 19670 - RNA, 896 nt, Homo sapiens
  source 1..896: mol_type = other RNA
tttcttcttagacatggcagctactgcatcttcatgtgtcacaaactctacatctgcttctcctgtggctctgccatcagctccaatatcaatatgaactcgtattggatttagtggtgagaagaaattagcaatgtcattttcagttgcacgaaaaggcaaccctctcatatgtacgaaatgaccaccatgaaaacctgaacttgcatcaccagctccaccatagccatgtcctcccatacctcttccatctctcattctgtcatcaaagccatcattcccatagccgtaattattatagccaccatagtcatcaaaacctccataacttccacgcccagctccataataaccccctcttcctcctattggtctatcatatggtcccggtcgctgtcccagcaatcttcttggtggatcataaaatcctttgatttcactcctgctacttctgaagatctcaatatacctgtgccctattctttccttgtgtttccccagagcattttctgctatctcctttgaagcaaactgcacgaaggcctcccctgtgcttctcccctggtagtccatcgtcaatgttatcccatttggcacgatttccaacccttgaaagaactgaactatttcctctttgctgcaaccaaatggtagtccacgaagtcgtactgtcccatcactagcgtcatttggaccattatgtttcataacccaatccatctcaataccgtttgatttaaatgcctgtcaggcgatagttacgccgactctggtgctcgcggggtccagttcaaagaagggagaagtcgtttgcctcgtgtagcgctcgccacaacggttctcccaaccgtctccagcggtgacaaccgcttagggagctgcgcagcacagctact

SEQ ID NO: 19671 - RNA, 905 nt, Homo sapiens
  source 1..905: mol_type = other RNA
tttcttcttagacatggcagctactgcatcttcatgtgtcacaaactctacatctgcttctcctgtggctctgccatcagctccaatatcaatatgaactcgtattggatttagtggtgagaagaaattagcaatgtcattttcagttgcacgaaaaggcaaccctctcatatgtacgaaatgaccaccatgaaaacctgaacttgcatcaccagctccaccatagccatgtcctcccatacctcttccatctctcattctgtcatcaaagccatcattcccatagccgtaattattatagccaccatagtcatcaaaacctccataacttccacgcccagctccataataaccccctcttcctcctattggtctatcatatggtcccggtcgctgtcccagcaatcttcttggtggatcataaaatcctttgatttcactcctgctacttctgaagatctcaatatacctgtgccctattctttccttgtgtttccccagagcattttctgctatctcctttgaagcaaactgcacgaaggcctcccctgtgcttctcccctggtagtccatcgtcaatgttatcccatttggcacgatttccaacccttgaaagaactgaactatttcctctttgctgcaaccaaatggtagtccacgaagtcgtactgtcccatcactagcgtcatttggaccattatgtttcataacccaatccatctcaataccgtttgatttaaatgcgtttttcttgcttacgttagaaccatccagttttcagagcgtaccattctgccgcctcggggcgatggcaatggcagttctgccagtgtgtagaaggaaccgtgccgtagcgctctggagaagttctccggtgatctgcccccaccgtgaacaaattctgt

SEQ ID NO: 19672 - RNA, 877 nt, Homo sapiens
  source 1..877: mol_type = other RNA
tttcttcttagacatggcagctactgcatcttcatgtgtcacaaactctacatctgcttctcctgtggctctgccatcagctccaatatcaatatgaactcgtattggatttagtggtgagaagaaattagcaatgtcattttcagttgcacgaaaaggcaaccctctcatatgtacgaaatgaccaccatgaaaacctgaacttgcatcaccagctccaccatagccatgtcctcccatacctcttccatctctcattctgtcatcaaagccatcattcccatagccgtaattattatagccaccatagtcatcaaaacctccataacttccacgcccagctccataataaccccctcttcctcctattggtctatcatatggtcccggtcgctgtcccagcaatcttcttggtggatcataaaatcctttgatttcactcctgctacttctgaagatctcaatatacctgtgccctattctttccttgtgtttccccagagcattttctgctatctcctttgaagcaaactgcacgaaggcctcccctgtgcttctcccctggtagtccatcgtcaatgttatcccatttggcacgatttccaacccttgaaagaactgaactatttcctctttgctgcaaccaaatggtagtccacgaagtcgtactgtcccatcactagcgtcatttggaccattatgtttcataacccaatccatctcaataccgtttgatttaaatggccgactctggtgctcgcggggtccagttcaaagaagggagaagtcgtttgcctcgtgtagcgctcgccacaacggttctcccaaccgtctccagcggtgacaaccgcttagggagctgcgcagcacagctact

SEQ ID NO: 19673 - RNA, 1033 nt, Homo sapiens
  source 1..1033: mol_type = other RNA
tttcttcttagacatggcagctactgcatcttcatgtgtcacaaactctacatctgcttctcctgtggctctgccatcagctccaatatcaatatgaactcgtattggatttagtggtgagaagaaattagcaatgtcattttcagttgcacgaaaaggcaaccctctcatatgtacgaaatgaccaccatgaaaacctgaacttgcatcaccagctccaccatagccatgtcctcccatacctcttccatctctcattctgtcatcaaagccatcattcccatagccgtaattattatagccaccatagtcatcaaaacctccataacttccacgcccagctccataataaccccctcttcctcctattggtctatcatatggtcccggtcgctgtcccagcaatcttcttggtggatcataaaatcctttgatttcactcctgctacttctgaagatctcaatatacctgtgccctattctttccttgtgtttccccagagcattttctgctatctcctttgaagcaaactgcacgaaggcctcccctgtgcttctcccctggtagtccatcgtcaatgttatcccatttggcacgatttccaacccttgaaagaactgaactatttcctctttgctgcaaccaaatggtagtccacgaagtcgtactgtcccatcactagcgtcatttggaccattatgtttcataacccaatccatctcaataccgtttgatttaaatgtcttttcgaagttccaaatctggaatataagggccggctaagcgtcctttattcctcccaggagactttccgtttatctagctgccctagagaccagaaagctagggagagtacgccccttccccctcccgtcagcagccaagcctggcttaaaacccttcgccaccgggcggcagaattacaaaggaggccgtctgcctcctttgtcctggatttgggagttgagcaccttcgtcgccattggctttcctcccccagctccagcctctctcatcttgggaatctgcgtc

SEQ ID NO: 19674 - RNA, 776 nt, Homo sapiens
  source 1..776: mol_type = other RNA
tttcttcttagacatggcagctactgcatcttcatgtgtcacaaactctacatctgcttctcctgtggctctgccatcagctccaatatcaatatgaactcgtattggatttagtggtgagaagaaattagcaatgtcattttcagttgcacgaaaaggcaaccctctcatatgtacgaaatgaccaccatgaaaacctgaacttgcatcaccagctccaccatagccatgtcctcccatacctcttccatctctcattctgtcatcaaagccatcattcccatagccgtaattattatagccaccatagtcatcaaaacctccataacttccacgcccagctccataataaccccctcttcctcctattggtctatcatatggtcccggtcgctgtcccagcaatcttcttggtggatcataaaatcctttgatttcactcctgctacttctgaagatctcaatataccttgaaagaactgaactatttcctctttgctgcaaccaaatggtagtccacgaagtcgtactgtcccatcactagcgtcatttggaccattatgtttcataacccaatccatctcaataccgtttgatttaaatgccccttttacttcagataccctgtcaggcgatagttacgccgactctggtgctcgcggggtccagttcaaagaagggagaagtcgtttgcctcgtgtagcgctcgccacaacggttctcccaaccgtctccagcggtgacaaccgcttagggagctgcgcagcacagctact

SEQ ID NO: 19675 - RNA, 757 nt, Homo sapiens
  source 1..757: mol_type = other RNA
tttcttcttagacatggcagctactgcatcttcatgtgtcacaaactctacatctgcttctcctgtggctctgccatcagctccaatatcaatatgaactcgtattggatttagtggtgagaagaaattagcaatgtcattttcagttgcacgaaaaggcaaccctctcatatgtacgaaatgaccaccatgaaaacctgaacttgcatcaccagctccaccatagccatgtcctcccatacctcttccatctctcattctgtcatcaaagccatcattcccatagccgtaattattatagccaccatagtcatcaaaacctccataacttccacgcccagctccataataaccccctcttcctcctattggtctatcatatggtcccggtcgctgtcccagcaatcttcttggtggatcataaaatcctttgatttcactcctgctacttctgaagatctcaatataccttgaaagaactgaactatttcctctttgctgcaaccaaatggtagtccacgaagtcgtactgtcccatcactagcgtcatttggaccattatgtttcataacccaatccatctcaataccgtttgatttaaatgcctgtcaggcgatagttacgccgactctggtgctcgcggggtccagttcaaagaagggagaagtcgtttgcctcgtgtagcgctcgccacaacggttctcccaaccgtctccagcggtgacaaccgcttagggagctgcgcagcacagctact

SEQ ID NO: 19676 - RNA, 738 nt, Homo sapiens
  source 1..738: mol_type = other RNA
tttcttcttagacatggcagctactgcatcttcatgtgtcacaaactctacatctgcttctcctgtggctctgccatcagctccaatatcaatatgaactcgtattggatttagtggtgagaagaaattagcaatgtcattttcagttgcacgaaaaggcaaccctctcatatgtacgaaatgaccaccatgaaaacctgaacttgcatcaccagctccaccatagccatgtcctcccatacctcttccatctctcattctgtcatcaaagccatcattcccatagccgtaattattatagccaccatagtcatcaaaacctccataacttccacgcccagctccataataaccccctcttcctcctattggtctatcatatggtcccggtcgctgtcccagcaatcttcttggtggatcataaaatcctttgatttcactcctgctacttctgaagatctcaatataccttgaaagaactgaactatttcctctttgctgcaaccaaatggtagtccacgaagtcgtactgtcccatcactagcgtcatttggaccattatgtttcataacccaatccatctcaataccgtttgatttaaatggccgactctggtgctcgcggggtccagttcaaagaagggagaagtcgtttgcctcgtgtagcgctcgccacaacggttctcccaaccgtctccagcggtgacaaccgcttagggagctgcgcagcacagctact

SEQ ID NO: 19677 - RNA, 33 nt, Homo sapiens
  source 1..33: mol_type = other RNA
tttcttcttagacatggcagcttcagcagtttc

SEQ ID NO: 19678 - RNA, 70 nt, Homo sapiens
  source 1..70: mol_type = other RNA
tttgaggctacagtgagatgtggcaggatcacatctcactgtagcctcaaaccgctgggctcaagtgttt

SEQ ID NO: 19679 - RNA, 29 nt, Homo sapiens
  source 1..29: mol_type = other RNA
tttggacagaaaacacgcaggtggcacac

SEQ ID NO: 19680 - RNA, 35 nt, Homo sapiens
  source 1..35: mol_type = other RNA
tttggagaggtgtactcccaaataaagggcaggga

SEQ ID NO: 19681 - RNA, 79 nt, Homo sapiens
  source 1..79: mol_type = other RNA
tttgggactgatcttgatgtctgccaaaaccttggcagacatcaagatcagtcccaaatatttcagtttattatagaca

SEQ ID NO: 19682 - RNA, 80 nt, Homo sapiens
  source 1..80: mol_type = other RNA
tttgggactgatcttgatgtctgccaaggttttggcagacatcaagatcagtcccaaatatttcagtttattataaacaa

SEQ ID NO: 19683 - RNA, 3906 nt, Homo sapiens
  source 1..3906: mol_type = other RNA
tttgtatggatatgtgtgtgtatatatatatatatatatacacacattagcaatttaagccttttaacatgccaattttttagatgctttattggttttttttcccctttactactacttcctgttttcccctttactactacaatttaagcctttaaaaatggcaattttttagatgcttgagatagtttgggggatccctagctcttatcatggcactctgttgagtttgtgaaatgcatcttcaaagaggttgtcaataatatgcaaatttttgaaaactagtgagattactaattattgatgaataaaaaatgagtacttttaatctgccaagttaaagctctagaattccttttctccagtaataactcgcagcatcactaccaatggaagggacctaaggaataccgtgtacactgatatacacgaagctgctcctcatttttttgtcagattacaaaagctgggctcatgtagttatggcctatggacctctttttaagttattttagcagaagtagatgatggtctacaccttgctcctcttttatattaactgtccctaagccactctgatgactattctaatcaaaatcagtatagctgtgctcactaagcatatcactgcttattattcaaataccttctgttttctatgtagcaaaacaaaaagttttataaatttcagataagctttctgtttttcttcagtgcaaacatcctgaaacagcacaaaatcattcagctagtctgaggataaagtcagtttatgtagtgcttaaagtagaatcccagatattctggaatggaaatagctcatgtgaaacttcagttcatttttgtccttaagggcaaatgatcatcttcagagagtgaagactttttaaaatctgaattcacagataaaatcattttagctttactttataggtactgctgaagttgtagcaggaactactagtccttcactgaggcatgtagccgccttgccgtacagtctgtggtaagtaacttttaggcatgccttcatcagtcgcagcctccatgccaactgtttcaaatctttctacttgtccctcagtacctggaccaaaagcatctgctgcagaaacttcctgaaacattttcatttgcccagatccacaggattgtgaaatatgatctgaaatctgctgtttaagtctaacaaaatcttcctcattgactgatgaaacttgctttgacctttcaaaatgtgaaatatctggactggattcatgctgactgcagttctgtttgaagtactgttgcctgggcaaaataccatcaccgccatctacatgatctactaattgtagatcttctggccgctcctctgaatctaacaagggctgggtagactcggatcttgagaagacttggactgacggaacttggtgtctgtagccactgtgtaccacggtagaatactggacagtgctcgaagtgttttgtgaagattcattttcatcactgctagaaatgcttggcctagaagatgacatgcatgaagaccccccaataccactgctgtgtccttcagtattaattttttcctttttgaacaggtccaatgatttcagatcttctggaaaaggctttttgtcatttgcttctatttccacaacacttacatcagtgaaattgccatctgaatacatttgatcttttgaattaaaattgtgccttggaggagtgtgaggtgaccactgggcaatatgactctttgaaggatctggaacattaggccagatgtgttttttaattaggtctcgcttattaaagcagaacagcactcccagaagagttgtcaataggaatgctaagcaaacaggcacgactatggcttcaatttctccttgagcaaactttggggtagtaaaagtgaattctggaccatccttcccaccttcatctgtgtatgctgccattcgtaccatgtacaatgtgtcactagtcaaagaggacaatgtatattctgtgtgggaagaatccacattcacagcagtttcatttccaatgatggttctataaaatatagtataatttctgataaatccattctgaacatcaacaggaagttggtcccactctaagacagcttcgtttttccctactttttttgtccgaacagtaggtcctttggaaggtgctcttaaataggtgcgatgcacggtaccatcttcttgttgccagtctgtgatacagggtgctttatctgataacacacaccactcaagtatatatttctttacagattcccttggagtagtccattccacccaaagcatgttatctttggggaatgctttaagatccattacagggtgagtagcttgaaagtcacaggcagggatagttaaaacagctgcatctgatttgccaacaagatttcttactgttagggttgctagatagcgatcatttgtgagatttactgtcagttttgtggcattaactgtgtaattttgtaaatgtgatttccatcttgtgagagtcacttcataatccaagatttttccattggcttcaaaaggaggcaatgtcttccacacgagttgtacagttctgtagccttgagtatgggatggatctattttataccagaaacttggtgctttagatggtctatcttcataggtgatcccacttgcttcttcactccagtcactccagtatcccttaccatcttccttcatacagcgaatcctaaacacatattctgtaaaaggtttaaggtcttggacagtgaatgaagatcgggtggatgctgtgtcttcaggaggaatctggctccaagttgaggcatctttggtcctatattgaatgttatattttagtattataacactcttaatacttgggttggtccatgtcaattttaagatactagacagttcctctgagttgatcactgataaattatgtggcggattgggcttcactttatatacaggatcaaaattgatatgatctgatgtaaccttcccaagggcattctctgcttctacccagacttcaatgttgacaaaatacacagtagaataatcaacagtgcatgaggtgggggtgtcacgttttgctttgcaatcagcaaacttgtgtgttgcccattcagattttaaagtgaagtttgtctccaagtgtgtttcccttccaccatcccactcacacctcattttcttcccctcgttcacaatgcaactcaaatttttaggtttttctggaggcaagcctgaaattattgtgattccataaacattctgttcaagctgtccgaatgtaagaatgttgcaagtgagctgaatatttaatgaagctatatctgtaaaggtgacactggatgctgttctgtttatgatagtatattgctccttaggaatagtaaaatggtttgttttccagacaatgtaattagcatttacatgaaaataatccatacatttttcctttagcacacaaactgcagtgaaattagaatgaagttgtacaactggagattcaggactgatataaccacatggatctagaagttcacctgtagattcagtggtgaggaaaataaacaaggcttgcactagccaagtctgcaacgtcaacatcttgcgcggatatttccaaatcacaaaattagtaagtgaaggagtagggatttgaagctaagtcttctacttctaaatgtcatgctttttccattgggtttcactcaggccgcgccgcctcgaccctccgcgtctccacagcgcacgaaccccttggcgccaggctgggccagacccgtcggcctggcaggcgcggcccccggttcagctgcgccggggcggcccagcgcgactccgcgggccttttggctgctcgccccggctccggaacactgtcagatcc

SEQ ID NO: 19684 - RNA, 3933 nt, Homo sapiens
  source 1..3933: mol_type = other RNA
tttgtatggatatgtgtgtgtatatatatatatatatatacacacattagcaatttaagccttttaacatgccaattttttagatgctttattggttttttttcccctttactactacttcctgttttcccctttactactacaatttaagcctttaaaaatggcaattttttagatgcttgagatagtttgggggatccctagctcttatcatggcactctgttgagtttgtgaaatgcatcttcaaagaggttgtcaataatatgcaaatttttgaaaactagtgagattactaattattgatgaataaaaaatgagtacttttaatctgccaagttaaagctctagaattccttttctccagtaataactcgcagcatcactaccaatggaagggacctaaggaataccgtgtacactgatatacacgaagctgctcctcatttttttgtcagattacaaaagctgggctcatgtagttatggcctatggacctctttttaagttattttagcagaagtagatgatggtctacaccttgctcctcttttatattaactgtccctaagccactctgatgactattctaatcaaaatcagtatagctgtgctcactaagcatatcactgcttattattcaaataccttctgttttctatgtagcaaaacaaaaagttttataaatttcagataagctttctgtttttcttcagtgcaaacatcctgaaacagcacaaaatcattcagctagtctgaggataaagtcagtttatgtagtgcttaaagtagaatcccagatattctggaatggaaatagctcatgtgaaacttcagttcatttttgtccttaagggcaaatgatcatcttcagagagtgaagactttttaaaatctgaattcacagataaaatcattttagctttactttataggtactgctgaagttgtagcaggaactactagtccttcactgaggcatgtagccgccttgccgtacagtctgtggtaagtaacttttaggcatgccttcatcagtcgcagcctccatgccaactgtttcaaatctttctacttgtccctcagtacctggaccaaaagcatctgctgcagaaacttcctgaaacattttcatttgcccagatccacaggattgtgaaatatgatctgaaatctgctgtttaagtctaacaaaatcttcctcattgactgatgaaacttgctttgacctttcaaaatgtgaaatatctggactggattcatgctgactgcagttctgtttgaagtactgttgcctgggcaaaataccatcaccgccatctacatgatctactaattgtagatcttctggccgctcctctgaatctaacaagggctgggtagactcggatcttgagaagacttggactgacggaacttggtgtctgtagccactgtgtaccacggtagaatactggacagtgctcgaagtgttttgtgaagattcattttcatcactgctagaaatgcttggcctagaagatgacatgcatgaagaccccccaataccactgctgtgtccttcagtattaattttttcctttttgaacaggtccaatgatttcagatcttctggaaaaggctttttgtcatttgcttctatttccacaacacttacatcagtgaaattgccatctgaatacatttgatcttttgaattaaaattgtgccttggaggagtgtgaggtgaccactgggcaatatgactctttgaaggatctggaacattaggccagatgtgttttttaattaggtctcgcttattaaagcagaacagcactcccagaagagttgtcaataggaatgctaagcaaacaggcacgactatggcttcaatttctccttgagcaaactttggggtagtaaaagtgaattctggaccatccttcccaccttcatctgtgtatgctgccattcgtaccatgtacaatgtgtcactagtcaaagaggacaatgtatattctgtgtgggaagaatccacattcacagcagtttcatttccaatgatggttctataaaatatagtataatttctgataaatccattctgaacatcaacaggaagttggtcccactctaagacagcttcgtttttccctactttttttgtccgaacagtaggtcctttggaaggtggagcttgtttaaggtatgcctttatggattcagggcttcctggtccatcagcatatactggagtaactgttatcaaatagcatttgctctctgctaagttccctcttaaataggtgcgatgcacggtaccatcttcttgttgccagtctgtgatacagggtgctttatctgataacacacaccactcaagtatatatttctttacagattcccttggagtagtccattccacccaaagcatgttatctttggggaatgctttaagatccattacagggtgagtagcttgaaagtcacaggcagggatagttaaaacagctgcatctgatttgccaacaagatttcttactgttagggttgctagatagcgatcatttgtgagatttactgtcagttttgtggcattaactgtgtaattttgtaaatgtgatttccatcttgtgagagtcacttcataatccaagatttttccattggcttcaaaaggaggcaatgtcttccacacgagttgtacagttctgtagccttgagtatgggatggatctattttataccagaaacttggtgctttagatggtccaaccaaaattccaggatcaaccgcttcccaggggcttatcaagtgtatcttcataggtgatcccacttgcttcttcactccagtcactccagtatcccttaccatcttccttcatacagcgaatcctaaacacatattctgtaaaaggtttaaggtcttggacagtgaatgaagatcgggtggatgctgtgtcttcaggaggaatctggctccaagttgaggcatctttggtcctatattgaatgttatattttagtattataacactcttaatacttgggttggtccatgtcaattttaagatactagacagttcctctgagttgatcactgataaattatgtggcggattgggcttcactttatatacaggatcaaaattgatatgatctgatgtaaccttcccaagggcattctctgcttctacccagacttcaatgttgacaaaatacacagtagaataatcaacagtgcatgaggtgggggtgtcacgttttgctttgcaatcagcaaacttgtgtgttgccagcctgaaattattgtgattccataaacattctgttcaagctgtccgaatgtaagaatgttgcaagtgagctgaatatttaatgaagctatatctgtaaaggtgacactggatgctgttctgtttatgatagtatattgctccttaggaatagtaaaatggtttgttttccagacaatgtaattagcatttacatgaaaataatccatacatttttcctttagcacacaaactgcagtgaaattagaatgaagttgtacaactggagattcaggactgatataaccacatggatctagaagttcacctgtagattcagtggtgaggaaaataaacaaggcttgcactagccaagtctgcaacgtcaacatcttgcgcggatatttccaaatcacaaaattagtaagtgaaggagtagggatttgaagctaagtcttctacttctaaatgtcatgctttttccattgggtttcactcaggccgcgccgcctcgaccctccgcgtctccacagcgcacgaaccccttggcgccaggctgggccagacccgtcggcctggcaggcgcggcccccggttcagctgcgccggggcggcccagcgcgactccgcgggccttttggctgctcgccccggctccggaacactgtcagatcc

SEQ ID NO: 19685 - RNA, 4054 nt, Homo sapiens
  source 1..4054: mol_type = other RNA
tttgtatggatatgtgtgtgtatatatatatatatatatacacacattagcaatttaagccttttaacatgccaattttttagatgctttattggttttttttcccctttactactacttcctgttttcccctttactactacaatttaagcctttaaaaatggcaattttttagatgcttgagatagtttgggggatccctagctcttatcatggcactctgttgagtttgtgaaatgcatcttcaaagaggttgtcaataatatgcaaatttttgaaaactagtgagattactaattattgatgaataaaaaatgagtacttttaatctgccaagttaaagctctagaattccttttctccagtaataactcgcagcatcactaccaatggaagggacctaaggaataccgtgtacactgatatacacgaagctgctcctcatttttttgtcagattacaaaagctgggctcatgtagttatggcctatggacctctttttaagttattttagcagaagtagatgatggtctacaccttgctcctcttttatattaactgtccctaagccactctgatgactattctaatcaaaatcagtatagctgtgctcactaagcatatcactgcttattattcaaataccttctgttttctatgtagcaaaacaaaaagttttataaatttcagataagctttctgtttttcttcagtgcaaacatcctgaaacagcacaaaatcattcagctagtctgaggataaagtcagtttatgtagtgcttaaagtagaatcccagatattctggaatggaaatagctcatgtgaaacttcagttcatttttgtccttaagggcaaatgatcatcttcagagagtgaagactttttaaaatctgaattcacagataaaatcattttagctttactttataggtactgctgaagttgtagcaggaactactagtccttcactgaggcatgtagccgccttgccgtacagtctgtggtaagtaacttttaggcatgccttcatcagtcgcagcctccatgccaactgtttcaaatctttctacttgtccctcagtacctggaccaaaagcatctgctgcagaaacttcctgaaacattttcatttgcccagatccacaggattgtgaaatatgatctgaaatctgctgtttaagtctaacaaaatcttcctcattgactgatgaaacttgctttgacctttcaaaatgtgaaatatctggactggattcatgctgactgcagttctgtttgaagtactgttgcctgggcaaaataccatcaccgccatctacatgatctactaattgtagatcttctggccgctcctctgaatctaacaagggctgggtagactcggatcttgagaagacttggactgacggaacttggtgtctgtagccactgtgtaccacggtagaatactggacagtgctcgaagtgttttgtgaagattcattttcatcactgctagaaatgcttggcctagaagatgacatgcatgaagaccccccaataccactgctgtgtccttcagtattaattttttcctttttgaacaggtccaatgatttcagatcttctggaaaaggctttttgtcatttgcttctatttccacaacacttacatcagtgaaattgccatctgaatacatttgatcttttgaattaaaattgtgccttggaggagtgtgaggtgaccactgggcaatatgactctttgaaggatctggaacattaggccagatgtgttttttaattaggtctcgcttattaaagcagaacagcactcccagaagagttgtcaataggaatgctaagcaaacaggcacgactatggcttcaatttctccttgagcaaactttggggtagtaaaagtgaattctggaccatccttcccaccttcatctgtgtatgctgccattcgtaccatgtacaatgtgtcactagtcaaagaggacaatgtatattctgtgtgggaagaatccacattcacagcagtttcatttccaatgatggttctataaaatatagtataatttctgataaatccattctgaacatcaacaggaagttggtcccactctaagacagcttcgtttttccctactttttttgtccgaacagtaggtcctttggaaggtggagcttgtttaaggtatgcctttatggattcagggcttcctggtccatcagcatatactggagtaactgttatcaaatagcatttgctctctgctaagttccctcttaaataggtgcgatgcacggtaccatcttcttgttgccagtctgtgatacagggtgctttatctgataacacacaccactcaagtatatatttctttacagattcccttggagtagtccattccacccaaagcatgttatctttggggaatgctttaagatccattacagggtgagtagcttgaaagtcacaggcagggatagttaaaacagctgcatctgatttgccaacaagatttcttactgttagggttgctagatagcgatcatttgtgagatttactgtcagttttgtggcattaactgtgtaattttgtaaatgtgatttccatcttgtgagagtcacttcataatccaagatttttccattggcttcaaaaggaggcaatgtcttccacacgagttgtacagttctgtagccttgagtatgggatggatctattttataccagaaacttggtgctttagatggtccaaccaaaattccaggatcaaccgcttcccaggggcttatcaagtgtatcttcataggtgatcccacttgcttcttcactccagtcactccagtatcccttaccatcttccttcatacagcgaatcctaaacacatattctgtaaaaggtttaaggtcttggacagtgaatgaagatcgggtggatgctgtgtcttcaggaggaatctggctccaagttgaggcatctttggtcctatattgaatgttatattttagtattataacactcttaatacttgggttggtccatgtcaattttaagatactagacagttcctctgagttgatcactgataaattatgtggcggattgggcttcactttatatacaggatcaaaattgatatgatctgatgtaaccttcccaagggcattctctgcttctacccagacttcaatgttgacaaaatacacagtagaataatcaacagtgcatgaggtgggggtgtcacgttttgctttgcaatcagcaaacttgtgtgttgcccattcagattttaaagtgaagtttgtctccaagtgtgtttcccttccaccatcccactcacacctcattttcttcccctcgttcacaatgcaactcaaatttttaggtttttctggaggcaagcctgaaattattgtgattccataaacattctgttcaagctgtccgaatgtaagaatgttgcaagtgagctgaatatttaatgaagctatatctgtaaaggtgacactggatgctgttctgtttatgatagtatattgctccttaggaatagtaaaatggtttgttttccagacaatgtaattagcatttacatgaaaataatccatacatttttcctttagcacacaaactgcagtgaaattagaatgaagttgtacaactggagattcaggactgatataaccacatggatctagaagttcacctgtagattcagtggtgaggaaaataaacaaggcttgcactagccaagtctgcaacgtcaacatcttgcgcggatatttccaaatcacaaaattagtaagtgaaggagtagggatttgaagctaagtcttctacttctaaatgtcatgctttttccattgggtttcactcaggccgcgccgcctcgaccctccgcgtctccacagcgcacgaaccccttggcgccaggctgggccagacccgtcggcctggcaggcgcggcccccggttcagctgcgccggggcggcccagcgcgactccgcgggccttttggctgctcgccccggctccggaacactgtcagatcc

SEQ ID NO: 19686 - RNA, 3887 nt, Homo sapiens
  source 1..3887: mol_type = other RNA
tttgtatggatatgtgtgtgtatatatatatatatatatacacacattagcaatttaagccttttaacatgccaattttttagatgctttattggttttttttcccctttactactacttcctgttttcccctttactactacaatttaagcctttaaaaatggcaattttttagatgcttgagatagtttgggggatccctagctcttatcatggcactctgttgagtttgtgaaatgcatcttcaaagaggttgtcaataatatgcaaatttttgaaaactagtgagattactaattattgatgaataaaaaatgagtacttttaatctgccaagttaaagctctagaattccttttctccagtaataactcgcagcatcactaccaatggaagggacctaaggaataccgtgtacactgatatacacgaagctgctcctcatttttttgtcagattacaaaagctgggctcatgtagttatggcctatggacctctttttaagttattttagcagaagtagatgatggtctacaccttgctcctcttttatattaactgtccctaagccactctgatgactattctaatcaaaatcagtatagctgtgctcactaagcatatcactgcttattattcaaataccttctgttttctatgtagcaaaacaaaaagttttataaatttcagataagctttctgtttttcttcagtgcaaacatcctgaaacagcacaaaatcattcagctagtctgaggataaagtcagtttatgtagtgcttaaagtagaatcccagatattctggaatggaaatagctcatgtgaaacttcagttcatttttgtccttaagggcaaatgatcatcttcagagagtgaagactttttaaaatctgaattcacagataaaatcattttagctttactttataggtactgctgaagttgtagcaggaactactagtccttcactgaggcatgtagccgccttgccgtacagtctgtggtaagtaacttttaggcatgccttcatcagtcgcagcctccatgccaactgtttcaaatctttctacttgtccctcagtacctggaccaaaagcatctgctgcagaaacttcctgaaacattttcatttgcccagatccacaggattgtgaaatatgatctgaaatctgctgtttaagtctaacaaaatcttcctcattgactgatgaaacttgctttgacctttcaaaatgtgaaatatctggactggattcatgctgactgcagttctgtttgaagtactgttgcctgggcaaaataccatcaccgccatctacatgatctactaattgtagatcttctggccgctcctctgaatctaacaagggctgggtagactcggatcttgagaagacttggactgacggaacttggtgtctgtagccactgtgtaccacggtagaatactggacagtgctcgaagtgttttgtgaagattcattttcatcactgctagaaatgcttggcctagaagatgacatgcatgaagaccccccaataccactgctgtgtccttcagtattaattttttcctttttgaacaggtccaatgatttcagatcttctggaaaaggctttttgtcatttgcttctatttccacaacacttacatcagtgaaattgccatctgaatacatttgatcttttgaattaaaattgtgccttggaggagtgtgaggtgaccactgggcaatatgactctttgaaggatctggaacattaggccagatgtgttttttaattaggtctcgcttattaaagcagaacagcactcccagaagagttgtcaataggaatgctaagcaaacaggcacgactatggcttcaatttctccttgagcaaactttggggtagtaaaagtgaattctggaccatccttcccaccttcatctgtgtatgctgccattcgtaccatgtacaatgtgtcactagtcaaagaggacaatgtatattctgtgtgggaagaatccacattcacagcagtttcatttccaatgatggttctataaaatatagtataatttctgataaatccattctgaacatcaacaggaagttggtcccactctaagacagcttcgtttttccctactttttttgtccgaacagtaggtcctttggaaggtggagcttgtttaaggtatgcctttatggattcagggcttcctggtccatcagcatatactggagtaactgttatcaaatagcatttgctctctgctaagttccctcttaaataggtgcgatgcacggtaccatcttcttgttgccagtctgtgatacagggtgctttatctgataacacacaccactcaagtatatatttctttacagattcccttggagtagtccattccacccaaagcatgttatctttggggaatgctttaagatccattacagggtgagtagcttgaaagtcacaggcagggatagttaaaacagctgcatctgatttgccaacaagatttcttactgttagggttgctagatagcgatcatttgtgagatttactgtcagttttgtggcattaactgtgtaattttgtaaatgtgatttccatcttgtgagagtcacttcataatccaagatttttccattggcttcaaaaggaggcaatgtcttccacacgagttgtacagttctgtagccttgagtatgggatggatctattttataccagaaacttggtgctttagatggtctatcttcataggtgatcccacttgcttcttcactccagtcactccagtatcccttaccatcttccttcatacagcgaatcctaaacacatattctgtaaaaggtttaaggtcttggacagtgaatgaagatcgggtggatgctgtgtcttcaggaggaatctggctccaagttgaggcatctttggtcctatattgaatgttatattttagtattataacactcttaatacttgggttggtccatgtcaattttaagatactagacagttcctctgagttgatcactgataaattatgtggcggattgggcttcactttatatacaggatcaaaattgatatgatctgatgtaaccttcccaagggcattctctgcttctacccagacttcaatgttgacaaaatacacagtagaataatcaacagtgcatgaggtgggggtgtcacgttttgctttgcaatcagcaaacttgtgtgttgccagcctgaaattattgtgattccataaacattctgttcaagctgtccgaatgtaagaatgttgcaagtgagctgaatatttaatgaagctatatctgtaaaggtgacactggatgctgttctgtttatgatagtatattgctccttaggaatagtaaaatggtttgttttccagacaatgtaattagcatttacatgaaaataatccatacatttttcctttagcacacaaactgcagtgaaattagaatgaagttgtacaactggagattcaggactgatataaccacatggatctagaagttcacctgtagattcagtggtgaggaaaataaacaaggcttgcactagccaagtctgcaacgtcaacatcttgcgcggatatttccaaatcacaaaattagtaagtgaaggagtagggatttgaagctaagtcttctacttctaaatgtcatgctttttccattgggtttcactcaggccgcgccgcctcgaccctccgcgtctccacagcgcacgaaccccttggcgccaggctgggccagacccgtcggcctggcaggcgcggcccccggttcagctgcgccggggcggcccagcgcgactccgcgggccttttggctgctcgccccggctccggaacactgtcagatcc

SEQ ID NO: 19687 - RNA, 4008 nt, Homo sapiens
  source 1..4008: mol_type = other RNA
tttgtatggatatgtgtgtgtatatatatatatatatatacacacattagcaatttaagccttttaacatgccaattttttagatgctttattggttttttttcccctttactactacttcctgttttcccctttactactacaatttaagcctttaaaaatggcaattttttagatgcttgagatagtttgggggatccctagctcttatcatggcactctgttgagtttgtgaaatgcatcttcaaagaggttgtcaataatatgcaaatttttgaaaactagtgagattactaattattgatgaataaaaaatgagtacttttaatctgccaagttaaagctctagaattccttttctccagtaataactcgcagcatcactaccaatggaagggacctaaggaataccgtgtacactgatatacacgaagctgctcctcatttttttgtcagattacaaaagctgggctcatgtagttatggcctatggacctctttttaagttattttagcagaagtagatgatggtctacaccttgctcctcttttatattaactgtccctaagccactctgatgactattctaatcaaaatcagtatagctgtgctcactaagcatatcactgcttattattcaaataccttctgttttctatgtagcaaaacaaaaagttttataaatttcagataagctttctgtttttcttcagtgcaaacatcctgaaacagcacaaaatcattcagctagtctgaggataaagtcagtttatgtagtgcttaaagtagaatcccagatattctggaatggaaatagctcatgtgaaacttcagttcatttttgtccttaagggcaaatgatcatcttcagagagtgaagactttttaaaatctgaattcacagataaaatcattttagctttactttataggtactgctgaagttgtagcaggaactactagtccttcactgaggcatgtagccgccttgccgtacagtctgtggtaagtaacttttaggcatgccttcatcagtcgcagcctccatgccaactgtttcaaatctttctacttgtccctcagtacctggaccaaaagcatctgctgcagaaacttcctgaaacattttcatttgcccagatccacaggattgtgaaatatgatctgaaatctgctgtttaagtctaacaaaatcttcctcattgactgatgaaacttgctttgacctttcaaaatgtgaaatatctggactggattcatgctgactgcagttctgtttgaagtactgttgcctgggcaaaataccatcaccgccatctacatgatctactaattgtagatcttctggccgctcctctgaatctaacaagggctgggtagactcggatcttgagaagacttggactgacggaacttggtgtctgtagccactgtgtaccacggtagaatactggacagtgctcgaagtgttttgtgaagattcattttcatcactgctagaaatgcttggcctagaagatgacatgcatgaagaccccccaataccactgctgtgtccttcagtattaattttttcctttttgaacaggtccaatgatttcagatcttctggaaaaggctttttgtcatttgcttctatttccacaacacttacatcagtgaaattgccatctgaatacatttgatcttttgaattaaaattgtgccttggaggagtgtgaggtgaccactgggcaatatgactctttgaaggatctggaacattaggccagatgtgttttttaattaggtctcgcttattaaagcagaacagcactcccagaagagttgtcaataggaatgctaagcaaacaggcacgactatggcttcaatttctccttgagcaaactttggggtagtaaaagtgaattctggaccatccttcccaccttcatctgtgtatgctgccattcgtaccatgtacaatgtgtcactagtcaaagaggacaatgtatattctgtgtgggaagaatccacattcacagcagtttcatttccaatgatggttctataaaatatagtataatttctgataaatccattctgaacatcaacaggaagttggtcccactctaagacagcttcgtttttccctactttttttgtccgaacagtaggtcctttggaaggtggagcttgtttaaggtatgcctttatggattcagggcttcctggtccatcagcatatactggagtaactgttatcaaatagcatttgctctctgctaagttccctcttaaataggtgcgatgcacggtaccatcttcttgttgccagtctgtgatacagggtgctttatctgataacacacaccactcaagtatatatttctttacagattcccttggagtagtccattccacccaaagcatgttatctttggggaatgctttaagatccattacagggtgagtagcttgaaagtcacaggcagggatagttaaaacagctgcatctgatttgccaacaagatttcttactgttagggttgctagatagcgatcatttgtgagatttactgtcagttttgtggcattaactgtgtaattttgtaaatgtgatttccatcttgtgagagtcacttcataatccaagatttttccattggcttcaaaaggaggcaatgtcttccacacgagttgtacagttctgtagccttgagtatgggatggatctattttataccagaaacttggtgctttagatggtctatcttcataggtgatcccacttgcttcttcactccagtcactccagtatcccttaccatcttccttcatacagcgaatcctaaacacatattctgtaaaaggtttaaggtcttggacagtgaatgaagatcgggtggatgctgtgtcttcaggaggaatctggctccaagttgaggcatctttggtcctatattgaatgttatattttagtattataacactcttaatacttgggttggtccatgtcaattttaagatactagacagttcctctgagttgatcactgataaattatgtggcggattgggcttcactttatatacaggatcaaaattgatatgatctgatgtaaccttcccaagggcattctctgcttctacccagacttcaatgttgacaaaatacacagtagaataatcaacagtgcatgaggtgggggtgtcacgttttgctttgcaatcagcaaacttgtgtgttgcccattcagattttaaagtgaagtttgtctccaagtgtgtttcccttccaccatcccactcacacctcattttcttcccctcgttcacaatgcaactcaaatttttaggtttttctggaggcaagcctgaaattattgtgattccataaacattctgttcaagctgtccgaatgtaagaatgttgcaagtgagctgaatatttaatgaagctatatctgtaaaggtgacactggatgctgttctgtttatgatagtatattgctccttaggaatagtaaaatggtttgttttccagacaatgtaattagcatttacatgaaaataatccatacatttttcctttagcacacaaactgcagtgaaattagaatgaagttgtacaactggagattcaggactgatataaccacatggatctagaagttcacctgtagattcagtggtgaggaaaataaacaaggcttgcactagccaagtctgcaacgtcaacatcttgcgcggatatttccaaatcacaaaattagtaagtgaaggagtagggatttgaagctaagtcttctacttctaaatgtcatgctttttccattgggtttcactcaggccgcgccgcctcgaccctccgcgtctccacagcgcacgaaccccttggcgccaggctgggccagacccgtcggcctggcaggcgcggcccccggttcagctgcgccggggcggcccagcgcgactccgcgggccttttggctgctcgccccggctccggaacactgtcagatcc

SEQ ID NO: 19688 - RNA, 3798 nt, Homo sapiens
  source 1..3798: mol_type = other RNA
tttgtatggatatgtgtgtgtatatatatatatatatatacacacattagcaatttaagccttttaacatgccaattttttagatgctttattggttttttttcccctttactactacttcctgttttcccctttactactacaatttaagcctttaaaaatggcaattttttagatgcttgagatagtttgggggatccctagctcttatcatggcactctgttgagtttgtgaaatgcatcttcaaagaggttgtcaataatatgcaaatttttgaaaactagtgagattactaattattgatgaataaaaaatgagtacttttaatctgccaagttaaagctctagaattccttttctccagtaataactcgcagcatcactaccaatggaagggacctaaggaataccgtgtacactgatatacacgaagctgctcctcatttttttgtcagattacaaaagctgggctcatgtagttatggcctatggacctctttttaagttattttagcagaagtagatgatggtctacaccttgctcctcttttatattaactgtccctaagccactctgatgactattctaatcaaaatcagtatagctgtgctcactaagcatatcactgcttattattcaaataccttctgttttctatgtagcaaaacaaaaagttttataaatttcagataagctttctgtttttcttcagtgcaaacatcctgaaacagcacaaaatcattcagctagtctgaggataaagtcagtttatgtagtgcttaaagtagaatcccagatattctggaatggaaatagctcatgtgaaacttcagttcatttttgtccttaagggcaaatgatcatcttcagagagtgaagactttttaaaatctgaattcacagataaaatcattttagctttactttataggtactgctgaagttgtagcaggaactactagtccttcactgaggcatgtagccgccttgccgtacagtctgtggtaagtaacttttaggcatgccttcatcagtcgcagcctccatgccaactgtttcaaatctttctacttgtccctcagtacctggaccaaaagcatctgctgcagaaacttcctgaaacattttcatttgcccagatccacaggattgtgaaatatgatctgaaatctgctgtttaagtctaacaaaatcttcctcattgactgatgaaacttgctttgacctttcaaaatgtgaaatatctggactggattcatgctgactgcagttctgtttgaagtactgttgcctgggcaaaataccatcaccgccatctacatgatctactaattgtagatcttctggccgctcctctgaatctaacaagggctgggtagactcggatcttgagaagacttggactgacggaacttggtgtctgtagccactgtgtaccacggtagaatactggacagtgctcgaagtgttttgtgaagattcattttcatcactgctagaaatgcttggcctagaagatgacatgcatgaagaccccccaataccactgctgtgtccttcagtattaattttttcctttttgaacaggtccaatgatttcagatcttctggaaaaggctttttgtcatttgcttctatttccacaacacttacatcagtgaaattgccatctgaatacatttgatcttttgaattaaaattgtgccttggaggagtgtgaggtgaccactgggcaatatgactctttgaaggatctggaacattaggccagatgtgttttttaattaggtctcgcttattaaagcagaacagcactcccagaagagttgtcaataggaatgctaagcaaacaggcacgactatggcttcaatttctccttgagcaaactttggggtagtaaaagtgaattctggaccatccttcccaccttcatctgtgtatgctgccattcgtaccatgtacaatgtgtcactagtcaaagaggacaatgtatattctgtgtgggaagaatccacattcacagcagtttcatttccaatgatggttctataaaatatagtataatttctgataaatccattctgaacatcaacaggaagttggtcccactctaagacagcttcgtttttccctactttttttgtccgaacagtaggtcctttggaaggtggagcttgtttaaggtatgcctttatggattcagggcttcctggtccatcagcatatactggagtaactgttatcaaatagcatttgctctctgctaagttccctcttaaataggtgcgatgcacggtaccatcttcttgttgccagtctgtgatacagggtgctttatctgataacacacaccactcaagtatatatttctttacagattcccttggagtagtccattccacccaaagcatgttatctttggggaatgctttaagatccattacagggtgagtagcttgaaagtcacaggcagggatagttaaaacagctgcatctgatttgccaacaagatttcttactgttagggttgctagatagcgatcatttgtgagatttactgtcagttttgtggcattaactgtgtaattttgtaaatgtgatttccatcttgtgagagtcacttcataatccaagatttttccattggcttcaaaaggaggcaatgtcttccacacgagttgtacagttctgtagccttgagtatgggatggatctattttataccagaaacttggtgctttagatggtctatcttcataggtgatcccacttgcttcttcactccagtcactccagtatcccttaccatcttccttcatacagcgaatcctaaacacatattctgtaaaaggtttaaggtcttggacagtgaatgaagatcgggtggatgctgtgtcttcaggaggaatctggctccaagttgaggcatctttggtcctatattgaatgttatattttagtattataacactcttaatacttgggttggtccatgtcaattttaagatactagacagttcctctgagttgatcactgataaattatgtggcggattgggcttcactttatatacaggatcaaaattgatatgatctgatgtaaccttcccaagggcattctctgcttctacccagacttcaatgttgacaaaatacacagtagaataatcaacagtgcatgaggtgggggtgtcacgttttgctttgcaatcagcaaacttgtgtgttgcccattcagattttaaagtgaagtttgtctccaagtgtgtttcccttccaccatcccactcacacctcattttcttcccctcgttcacaatgcaactcaaatttttaggtttttctggaggcaatttttcctttagcacacaaactgcagtgaaattagaatgaagttgtacaactggagattcaggactgatataaccacatggatctagaagttcacctgtagattcagtggtgaggaaaataaacaaggcttgcactagccaagtctgcaacgtcaacatcttgcgcggatatttccaaatcacaaaattagtaagtgaaggagtagggatttgaagctaagtcttctacttctaaatgtcatgctttttccattgggtttcactcaggccgcgccgcctcgaccctccgcgtctccacagcgcacgaaccccttggcgccaggctgggccagacccgtcggcctggcaggcgcggcccccggttcagctgcgccggggcggcccagcgcgactccgcgggccttttggctgctcgccccggctccggaacactgtcagatcc

SEQ ID NO: 19689 - RNA, 3804 nt, Homo sapiens
  source 1..3804: mol_type = other RNA
tttgtatggatatgtgtgtgtatatatatatatatatatacacacattagcaatttaagccttttaacatgccaattttttagatgctttattggttttttttcccctttactactacttcctgttttcccctttactactacaatttaagcctttaaaaatggcaattttttagatgcttgagatagtttgggggatccctagctcttatcatggcactctgttgagtttgtgaaatgcatcttcaaagaggttgtcaataatatgcaaatttttgaaaactagtgagattactaattattgatgaataaaaaatgagtacttttaatctgccaagttaaagctctagaattccttttctccagtaataactcgcagcatcactaccaatggaagggacctaaggaataccgtgtacactgatatacacgaagctgctcctcatttttttgtcagattacaaaagctgggctcatgtagttatggcctatggacctctttttaagttattttagcagaagtagatgatggtctacaccttgctcctcttttatattaactgtccctaagccactctgatgactattctaatcaaaatcagtatagctgtgctcactaagcatatcactgcttattattcaaataccttctgttttctatgtagcaaaacaaaaagttttataaatttcagataagctttctgtttttcttcagtgcaaacatcctgaaacagcacaaaatcattcagctagtctgaggataaagtcagtttatgtagtgcttaaagtagaatcccagatattctggaatggaaatagctcatgtgaaacttcagttcatttttgtccttaagggcaaatgatcatcttcagagagtgaagactttttaaaatctgaattcacagataaaatcattttagctttactttataggtactgctgaagttgtagcaggaactactagtccttcactgaggcatgtagccgccttgccgtacagtctgtggtaagtaacttttaggcatgccttcatcagtcgcagcctccatgccaactgtttcaaatctttctacttgtccctcagtacctggaccaaaagcatctgctgcagaaacttcctgaaacattttcatttgcccagatccacaggattgtgaaatatgatctgaaatctgctgtttaagtctaacaaaatcttcctcattgactgatgaaacttgctttgacctttcaaaatgtgaaatatctggactggattcatgctgactgcagttctgtttgaagtactgttgcctgggcaaaataccatcaccgccatctacatgatctactaattgtagatcttctggccgctcctctgaatctaacaagggctgggtagactcggatcttgagaagacttggactgacggaacttggtgtctgtagccactgtgtaccacggtagaatactggacagtgctcgaagtgttttgtgaagattcattttcatcactgctagaaatgcttggcctagaagatgacatgcatgaagaccccccaataccactgctgtgtccttcagtattaattttttcctttttgaacaggtccaatgatttcagatcttctggaaaaggctttttgtcatttgcttctatttccacaacacttacatcagtgaaattgccatctgaatacatttgatcttttgaattaaaattgtgccttggaggagtgtgaggtgaccactgggcaatatgactctttgaaggatctggaacattaggccagatgtgttttttaattaggtctcgcttattaaagcagaacagcactcccagaagagttgtcaataggaatgctaagcaaacaggcacgactatggcttcaatttctccttgagcaaactttggggtagtaaaagtgaattctggaccatccttcccaccttcatctgtgtatgctgccattcgtaccatgtacaatgtgtcactagtcaaagaggacaatgtatattctgtgtgggaagaatccacattcacagcagtttcatttccaatgatggttctataaaatatagtataatttctgataaatccattctgaacatcaacaggaagttggtcccactctaagacagcttcgtttttccctactttttttgtccgaacagtaggtcctttggaaggtggagcttgtttaaggtatgcctttatggattcagggcttcctggtccatcagcatatactggagtaactgttatcaaatagcatttgctctctgctaagttccctcttaaataggtgcgatgcacggtaccatcttcttgttgccagtctgtgatacagggtgctttatctgataacacacaccactcaagtatatatttctttacagattcccttggagtagtccattccacccaaagcatgttatctttggggaatgctttaagatccattacagggtgagtagcttgaaagtcacaggcagggatagttaaaacagctgcatctgatttgccaacaagatttcttactgttagggttgctagatagcgatcatttgtgagatttactgtcagttttgtggcattaactgtgtaattttgtaaatgtgatttccatcttgtgagagtcacttcataatccaagatttttccattggcttcaaaaggaggcaatgttatcttcataggtgatcccacttgcttcttcactccagtcactccagtatcccttaccatcttccttcatacagcgaatcctaaacacatattctgtaaaaggtttaaggtcttggacagtgaatgaagatcgggtggatgctgtgtcttcaggaggaatctggctccaagttgaggcatctttggtcctatattgaatgttatattttagtattataacactcttaatacttgggttggtccatgtcaattttaagatactagacagttcctctgagttgatcactgataaattatgtggcggattgggcttcactttatatacaggatcaaaattgatatgatctgatgtaaccttcccaagggcattctctgcttctacccagacttcaatgttgacaaaatacacagtagaataatcaacagtgcatgaggtgggggtgtcacgttttgctttgcaatcagcaaacttgtgtgttgccagcctgaaattattgtgattccataaacattctgttcaagctgtccgaatgtaagaatgttgcaagtgagctgaatatttaatgaagctatatctgtaaaggtgacactggatgctgttctgtttatgatagtatattgctccttaggaatagtaaaatggtttgttttccagacaatgtaattagcatttacatgaaaataatccatacatttttcctttagcacacaaactgcagtgaaattagaatgaagttgtacaactggagattcaggactgatataaccacatggatctagaagttcacctgtagattcagtggtgaggaaaataaacaaggcttgcactagccaagtctgcaacgtcaacatcttgcgcggatatttccaaatcacaaaattagtaagtgaaggagtagggatttgaagctaagtcttctacttctaaatgtcatgctttttccattgggtttcactcaggccgcgccgcctcgaccctccgcgtctccacagcgcacgaaccccttggcgccaggctgggccagacccgtcggcctggcaggcgcggcccccggttcagctgcgccggggcggcccagcgcgactccgcgggccttttggctgctcgccccggctccggaacactgtcagatcc

SEQ ID NO: 19690 - RNA, 3925 nt, Homo sapiens
  source 1..3925: mol_type = other RNA
tttgtatggatatgtgtgtgtatatatatatatatatatacacacattagcaatttaagccttttaacatgccaattttttagatgctttattggttttttttcccctttactactacttcctgttttcccctttactactacaatttaagcctttaaaaatggcaattttttagatgcttgagatagtttgggggatccctagctcttatcatggcactctgttgagtttgtgaaatgcatcttcaaagaggttgtcaataatatgcaaatttttgaaaactagtgagattactaattattgatgaataaaaaatgagtacttttaatctgccaagttaaagctctagaattccttttctccagtaataactcgcagcatcactaccaatggaagggacctaaggaataccgtgtacactgatatacacgaagctgctcctcatttttttgtcagattacaaaagctgggctcatgtagttatggcctatggacctctttttaagttattttagcagaagtagatgatggtctacaccttgctcctcttttatattaactgtccctaagccactctgatgactattctaatcaaaatcagtatagctgtgctcactaagcatatcactgcttattattcaaataccttctgttttctatgtagcaaaacaaaaagttttataaatttcagataagctttctgtttttcttcagtgcaaacatcctgaaacagcacaaaatcattcagctagtctgaggataaagtcagtttatgtagtgcttaaagtagaatcccagatattctggaatggaaatagctcatgtgaaacttcagttcatttttgtccttaagggcaaatgatcatcttcagagagtgaagactttttaaaatctgaattcacagataaaatcattttagctttactttataggtactgctgaagttgtagcaggaactactagtccttcactgaggcatgtagccgccttgccgtacagtctgtggtaagtaacttttaggcatgccttcatcagtcgcagcctccatgccaactgtttcaaatctttctacttgtccctcagtacctggaccaaaagcatctgctgcagaaacttcctgaaacattttcatttgcccagatccacaggattgtgaaatatgatctgaaatctgctgtttaagtctaacaaaatcttcctcattgactgatgaaacttgctttgacctttcaaaatgtgaaatatctggactggattcatgctgactgcagttctgtttgaagtactgttgcctgggcaaaataccatcaccgccatctacatgatctactaattgtagatcttctggccgctcctctgaatctaacaagggctgggtagactcggatcttgagaagacttggactgacggaacttggtgtctgtagccactgtgtaccacggtagaatactggacagtgctcgaagtgttttgtgaagattcattttcatcactgctagaaatgcttggcctagaagatgacatgcatgaagaccccccaataccactgctgtgtccttcagtattaattttttcctttttgaacaggtccaatgatttcagatcttctggaaaaggctttttgtcatttgcttctatttccacaacacttacatcagtgaaattgccatctgaatacatttgatcttttgaattaaaattgtgccttggaggagtgtgaggtgaccactgggcaatatgactctttgaaggatctggaacattaggccagatgtgttttttaattaggtctcgcttattaaagcagaacagcactcccagaagagttgtcaataggaatgctaagcaaacaggcacgactatggcttcaatttctccttgagcaaactttggggtagtaaaagtgaattctggaccatccttcccaccttcatctgtgtatgctgccattcgtaccatgtacaatgtgtcactagtcaaagaggacaatgtatattctgtgtgggaagaatccacattcacagcagtttcatttccaatgatggttctataaaatatagtataatttctgataaatccattctgaacatcaacaggaagttggtcccactctaagacagcttcgtttttccctactttttttgtccgaacagtaggtcctttggaaggtggagcttgtttaaggtatgcctttatggattcagggcttcctggtccatcagcatatactggagtaactgttatcaaatagcatttgctctctgctaagttccctcttaaataggtgcgatgcacggtaccatcttcttgttgccagtctgtgatacagggtgctttatctgataacacacaccactcaagtatatatttctttacagattcccttggagtagtccattccacccaaagcatgttatctttggggaatgctttaagatccattacagggtgagtagcttgaaagtcacaggcagggatagttaaaacagctgcatctgatttgccaacaagatttcttactgttagggttgctagatagcgatcatttgtgagatttactgtcagttttgtggcattaactgtgtaattttgtaaatgtgatttccatcttgtgagagtcacttcataatccaagatttttccattggcttcaaaaggaggcaatgttatcttcataggtgatcccacttgcttcttcactccagtcactccagtatcccttaccatcttccttcatacagcgaatcctaaacacatattctgtaaaaggtttaaggtcttggacagtgaatgaagatcgggtggatgctgtgtcttcaggaggaatctggctccaagttgaggcatctttggtcctatattgaatgttatattttagtattataacactcttaatacttgggttggtccatgtcaattttaagatactagacagttcctctgagttgatcactgataaattatgtggcggattgggcttcactttatatacaggatcaaaattgatatgatctgatgtaaccttcccaagggcattctctgcttctacccagacttcaatgttgacaaaatacacagtagaataatcaacagtgcatgaggtgggggtgtcacgttttgctttgcaatcagcaaacttgtgtgttgcccattcagattttaaagtgaagtttgtctccaagtgtgtttcccttccaccatcccactcacacctcattttcttcccctcgttcacaatgcaactcaaatttttaggtttttctggaggcaagcctgaaattattgtgattccataaacattctgttcaagctgtccgaatgtaagaatgttgcaagtgagctgaatatttaatgaagctatatctgtaaaggtgacactggatgctgttctgtttatgatagtatattgctccttaggaatagtaaaatggtttgttttccagacaatgtaattagcatttacatgaaaataatccatacatttttcctttagcacacaaactgcagtgaaattagaatgaagttgtacaactggagattcaggactgatataaccacatggatctagaagttcacctgtagattcagtggtgaggaaaataaacaaggcttgcactagccaagtctgcaacgtcaacatcttgcgcggatatttccaaatcacaaaattagtaagtgaaggagtagggatttgaagctaagtcttctacttctaaatgtcatgctttttccattgggtttcactcaggccgcgccgcctcgaccctccgcgtctccacagcgcacgaaccccttggcgccaggctgggccagacccgtcggcctggcaggcgcggcccccggttcagctgcgccggggcggcccagcgcgactccgcgggccttttggctgctcgccccggctccggaacactgtcagatcc

SEQ ID NO: 19691 - RNA, 3825 nt, Homo sapiens
  source 1..3825: mol_type = other RNA
tttgtatggatatgtgtgtgtatatatatatatatatatacacacattagcaatttaagccttttaacatgccaattttttagatgctttattggttttttttcccctttactactacttcctgttttcccctttactactacaatttaagcctttaaaaatggcaattttttagatgcttgagatagtttgggggatccctagctcttatcatggcactctgttgagtttgtgaaatgcatcttcaaagaggttgtcaataatatgcaaatttttgaaaactagtgagattactaattattgatgaataaaaaatgagtacttttaatctgccaagttaaagctctagaattccttttctccagtaataactcgcagcatcactaccaatggaagggacctaaggaataccgtgtacactgatatacacgaagctgctcctcatttttttgtcagattacaaaagctgggctcatgtagttatggcctatggacctctttttaagttattttagcagaagtagatgatggtctacaccttgctcctcttttatattaactgtccctaagccactctgatgactattctaatcaaaatcagtatagctgtgctcactaagcatatcactgcttattattcaaataccttctgttttctatgtagcaaaacaaaaagttttataaatttcagataagctttctgtttttcttcagtgcaaacatcctgaaacagcacaaaatcattcagctagtctgaggataaagtcagtttatgtagtgcttaaagtagaatcccagatattctggaatggaaatagctcatgtgaaacttcagttcatttttgtccttaagggcaaatgatcatcttcagagagtgaagactttttaaaatctgaattcacagataaaatcattttagctttactttataggtactgctgaagttgtagcaggaactactagtccttcactgaggcatgtagccgccttgccgtacagtctgtggtaagtaacttttaggcatgccttcatcagtcgcagcctccatgccaactgtttcaaatctttctacttgtccctcagtacctggaccaaaagcatctgctgcagaaacttcctgaaacattttcatttgcccagatccacaggattgtgaaatatgatctgaaatctgctgtttaagtctaacaaaatcttcctcattgactgatgaaacttgctttgacctttcaaaatgtgaaatatctggactggattcatgctgactgcagttctgtttgaagtactgttgcctgggcaaaataccatcaccgccatctacatgatctactaattgtagatcttctggccgctcctctgaatctaacaagggctgggtagactcggatcttgagaagacttggactgacggaacttggtgtctgtagccactgtgtaccacggtagaatactggacagtgctcgaagtgttttgtgaagattcattttcatcactgctagaaatgcttggcctagaagatgacatgcatgaagaccccccaataccactgctgtgtccttcagtattaattttttcctttttgaacaggtccaatgatttcagatcttctggaaaaggctttttgtcatttgcttctatttccacaacacttacatcagtgaaattgccatctgaatacatttgatcttttgaattaaaattgtgccttggaggagtgtgaggtgaccactgggcaatatgactctttgaaggatctggaacattaggccagatgtgttttttaattaggtctcgcttattaaagcagaacagcactcccagaagagttgtcaataggaatgctaagcaaacaggcacgactatggcttcaatttctccttgagcaaactttggggtagtaaaagtgaattctggaccatccttcccaccttcatctgtgtatgctgccattcgtaccatgtacaatgtgtcactagtcaaagaggacaatgtatattctgtgtgggaagaatccacattcacagcagtttcatttccaatgatggttctataaaatatagtataatttctgataaatccattctgaacatcaacaggaagttggtcccactctaagacagcttcgtttttccctactttttttgtccgaacagtaggtcctttggaaggtggagcttgtttaaggtatgcctttatggattcagggcttcctggtccatcagcatatactggagtaactgttatcaaatagcatttgctctctgctaagttcccttgaaagtcacaggcagggatagttaaaacagctgcatctgatttgccaacaagatttcttactgttagggttgctagatagcgatcatttgtgagatttactgtcagttttgtggcattaactgtgtaattttgtaaatgtgatttccatcttgtgagagtcacttcataatccaagatttttccattggcttcaaaaggaggcaatgtcttccacacgagttgtacagttctgtagccttgagtatgggatggatctattttataccagaaacttggtgctttagatggtctatcttcataggtgatcccacttgcttcttcactccagtcactccagtatcccttaccatcttccttcatacagcgaatcctaaacacatattctgtaaaaggtttaaggtcttggacagtgaatgaagatcgggtggatgctgtgtcttcaggaggaatctggctccaagttgaggcatctttggtcctatattgaatgttatattttagtattataacactcttaatacttgggttggtccatgtcaattttaagatactagacagttcctctgagttgatcactgataaattatgtggcggattgggcttcactttatatacaggatcaaaattgatatgatctgatgtaaccttcccaagggcattctctgcttctacccagacttcaatgttgacaaaatacacagtagaataatcaacagtgcatgaggtgggggtgtcacgttttgctttgcaatcagcaaacttgtgtgttgcccattcagattttaaagtgaagtttgtctccaagtgtgtttcccttccaccatcccactcacacctcattttcttcccctcgttcacaatgcaactcaaatttttaggtttttctggaggcaagcctgaaattattgtgattccataaacattctgttcaagctgtccgaatgtaagaatgttgcaagtgagctgaatatttaatgaagctatatctgtaaaggtgacactggatgctgttctgtttatgatagtatattgctccttaggaatagtaaaatggtttgttttccagacaatgtaattagcatttacatgaaaataatccatacatttttcctttagcacacaaactgcagtgaaattagaatgaagttgtacaactggagattcaggactgatataaccacatggatctagaagttcacctgtagattcagtggtgaggaaaataaacaaggcttgcactagccaagtctgcaacgtcaacatcttgcgcggatatttccaaatcacaaaattagtaagtgaaggagtagggatttgaagctaagtcttctacttctaaatgtcatgctttttccattgggtttcactcaggccgcgccgcctcgaccctccgcgtctccacagcgcacgaaccccttggcgccaggctgggccagacccgtcggcctggcaggcgcggcccccggttcagctgcgccggggcggcccagcgcgactccgcgggccttttggctgctcgccccggctccggaacactgtcagatcc

SEQ ID NO: 19692 - RNA, 4889 nt, Homo sapiens
  source 1..4889: mol_type = other RNA
tttgtatggatatgtgtgtgtatatatatatatatatatacacacattagcaatttaagccttttaacatgccaattttttagatgctttattggttttttttcccctttactactacttcctgttttcccctttactactacaatttaagcctttaaaaatggcaattttttagatgcttgagatagtttgggggatccctagctcttatcatggcactctgttgagtttgtgaaatgcatcttcaaagaggttgtcaataatatgcaaatttttgaaaactagtgagattactaattattgatgaataaaaaatgagtacttttaatctgccaagttaaagctctagaattccttttctccagtaataactcgcagcatcactaccaatggaagggacctaaggaataccgtgtacactgatatacacgaagctgctcctcatttttttgtcagattacaaaagctgggctcatgtagttatggcctatggacctctttttaagttattttagcagaagtagatgatggtctacaccttgctcctcttttatattaactgtccctaagccactctgatgactattctaatcaaaatcagtatagctgtgctcactaagcatatcactgcttattattcaaataccttctgttttctatgtagcaaaacaaaaagttttataaatttcagataagctttctgtttttcttcagtgcaaacatcctgaaacagcacaaaatcattcagctagtctgaggataaagtcagtttatgtagtgcttaaagtagaatcccagatattctggaatggaaatagctcatgtgaaacttcagttcatttttgtccttaagggcaaatgatcatcttcagagagtgaagactttttaaaatctgaattcacagataaaatcattttagctttactttataggtactgctgaagttgtagcaggaactactagtccttcactgaggcatgtagccgccttgccgtacagtctgtggtaagtaacttttaggcatgccttcatcagtcgcagcctccatgccaactgtttcaaatctttctacttgtccctcagtacctggaccaaaagcatctgctgcagaaacttcctgaaacattttcatttgcccagatccacaggattgtgaaatatgatctgaaatctgctgtttaagtctaacaaaatcttcctcattgactgatgaaacttgctttgacctttcaaaatgtgaaatatctggactggattcatgctgactgcagttctgtttgaagtactgttgcctgggcaaaataccatcaccgccatctacatgatctactaattgtagatcttctggccgctcctctgaatctaacaagggctgggtagactcggatcttgagaagacttggactgacggaacttggtgtctgtagccactgtgtaccacggtagaatactggacagtgctcgaagtgttttgtgaagattcattttcatcactgctagaaatgcttggcctagaagatgacatgcatgaagaccccccaataccactgctgtgtccttcagtattaattttttcctttttgaacaggtccaatgatttcagatcttctggaaaaggctttttgtcatttgcttctatttccacaacacttacatcagtgaaattgccatctgaatacatttgatcttttgaattaaaattgtgccttggaggagtgtgaggtgaccactgggcaatatgactctttgaaggatctggaacattaggccagatgtgttttttaattaggtctcgcttattaaagcagaacagcactcccagaagagttgtcaataggaatgctaagcaaacaggcacgactatggcttcaatttctccttgagcatttttcaaaaggaggatatagctggtacagggctaagaactttaggagctgctcaatgggcatgaggagtggcacgagtaggaataaactaaaaagtaaacaagcctaagatccctaaataccacacaaatcctcatctgcatttaaaagaggacttgttcatcaaattaatcactaattgggataattaacattggagattttttaaatgactgtcctgattaattttgaattttacttagtcttttacagtaaaaaatgtatgaaagtaatattgcagccatatactattcacttaattttatccttccaccacacatatccctttgtaagtaactaacatcctatgaagctcagtagaaatcaagaaatcagttaaatgcttgagaataaactatgggttggcaaatattaactcttaaatgctaagcatcatatatatatatatatgggtgtatgtatatatatttatgtgtgtatatattgatatatgtgtgtatatatatattgatatgggtatgtatgtgtgtatatatatataaaatgccaaatctaatttaggcagaaactttgctttattaaacatctgcttttatgttttcaagcctgtgcctttgctcatgctgctctctaagatgccaccttcttcctatttgtccacatactaactcaaggctcaagtattttcttcttcataaaacctttgaaggtaaaattatccactactggtatatttaaattcctactctatttactgtctacatagtccacaggttctcctttttctgatttacttatgcaaaatttcttcaactaagctgtaaggtcctcgttggcaagactcaagccatgtgaagaagccataatggatccatgagacaaactttggggtagtaaaagtgaattctggaccatccttcccaccttcatctgtgtatgctgccattcgtaccatgtacaatgtgtcactagtcaaagaggacaatgtatattctgtgtgggaagaatccacattcacagcagtttcatttccaatgatggttctataaaatatagtataatttctgataaatccattctgaacatcaacaggaagttggtcccactctaagacagcttcgtttttccctactttttttgtccgaacagtaggtcctttggaaggtggagcttgtttaaggtatgcctttatggattcagggcttcctggtccatcagcatatactggagtaactgttatcaaatagcatttgctctctgctaagttccctcttaaataggtgcgatgcacggtaccatcttcttgttgccagtctgtgatacagggtgctttatctgataacacacaccactcaagtatatatttctttacagattcccttggagtagtccattccacccaaagcatgttatctttggggaatgctttaagatccattacagggtgagtagcttgaaagtcacaggcagggatagttaaaacagctgcatctgatttgccaacaagatttcttactgttagggttgctagatagcgatcatttgtgagatttactgtcagttttgtggcattaactgtgtaattttgtaaatgtgatttccatcttgtgagagtcacttcataatccaagatttttccattggcttcaaaaggaggcaatgtcttccacacgagttgtacagttctgtagccttgagtatgggatggatctattttataccagaaacttggtgctttagatggtctatcttcataggtgatcccacttgcttcttcactccagtcactccagtatcccttaccatcttccttcatacagcgaatcctaaacacatattctgtaaaaggtttaaggtcttggacagtgaatgaagatcgggtggatgctgtgtcttcaggaggaatctggctccaagttgaggcatctttggtcctatattgaatgttatattttagtattataacactcttaatacttgggttggtccatgtcaattttaagatactagacagttcctctgagttgatcactgataaattatgtggcggattgggcttcactttatatacaggatcaaaattgatatgatctgatgtaaccttcccaagggcattctctgcttctacccagacttcaatgttgacaaaatacacagtagaataatcaacagtgcatgaggtgggggtgtcacgttttgctttgcaatcagcaaacttgtgtgttgcccattcagattttaaagtgaagtttgtctccaagtgtgtttcccttccaccatcccactcacacctcattttcttcccctcgttcacaatgcaactcaaatttttaggtttttctggaggcaagcctgaaattattgtgattccataaacattctgttcaagctgtccgaatgtaagaatgttgcaagtgagctgaatatttaatgaagctatatctgtaaaggtgacactggatgctgttctgtttatgatagtatattgctccttaggaatagtaaaatggtttgttttccagacaatgtaattagcatttacatgaaaataatccatacatttttcctttagcacacaaactgcagtgaaattagaatgaagttgtacaactggagattcaggactgatataaccacatggatctagaagttcacctgtagattcagtggtgaggaaaataaacaaggcttgcactagccaagtctgcaacgtcaacatcttgcgcggatatttccaaatcacaaaattagtaagtgaaggagtagggatttgaagctaagtcttctacttctaaatgtcatgctttttccattgggtttcactcaggccgcgccgcctcgaccctccgcgtctccacagcgcacgaaccccttggcgccaggctgggccagacccgtcggcctggcaggcgcggcccccggttcagctgcgccggggcggcccagcgcgactccgcgggccttttggctgctcgccccggctccggaacactgtcagatcc

SEQ ID NO: 19693 - RNA, 54 nt, Homo sapiens
  source 1..54: mol_type = other RNA
ttttaaggacactgagggatccagaacaaaggatccctcagtgtccttaaaaca

SEQ ID NO: 19694 - RNA, 146 nt, Homo sapiens
  source 1..146: mol_type = other RNA
ttttgcaatatgttcctgaataccaacgagacggagcttctttttgtatgtgtattatccatatatatgtcctttgaagccagcctcaagtccaggaagtcagccaagtcctgggttgtgataatcctcctgcagcctcatctggt

SEQ ID NO: 19695 - RNA, 5830 nt, Homo sapiens
  source 1..5830: mol_type = other RNA
ttttgcaccttttggagtgaaaaaaatgaggtttacactgtagtataacaaaatgcctttttgtaaaggccagaagaaatggctgtgctgtgctgcctgaagcagaaaaaccttcatgtaccaggtgaatgtaaagcctttctcctcccacacacaatggactcacccagtattaccctccactaccacttttgaccctcataacagcaccctggcgggggggcagattgatgttatcaccatttaccagatgaggaaactgaggcctgatgggcagtgatttgtgcactgcgacataggactcagtgaagagcctagccagctgacggtcagctgactggtgcactctttccctcaccttctctctcaagggcacagctacactctttctccaccattattaacactcacagggcacaggtagagcgtccccagacctgtgcaatattctacacgaaaacatttggaatgtgagcaatgtctgaacaggggcttgccaggcacatctgatcaccataaatgctcccacccctgcctgtcctcacttgtgctgcactatgcaagcaagcagcaggttctcagaaggccactgtcctgcatgtcacaatgagtggccaactccttcacagaacagcaaatagcagccctggctacaaggtgcagtgtgcaacccccatatgccaaggggcagctgctatcttccagcagagagagaacccccagctctgctccctacctatgccctgcttcctgtgcctcacacagccagccttgctggcctgctggctattgtctctgactctgagctgtgctgaccaccaagtgttactcctctccaagacttgactcccaggcatgggtgggagagttgaacctcaatgcaatctgctcccactctgaagctcgtctacccaccccatttgttacaattaaagatggttttctcatccctccagagactccagtttcagactctgtctccagagctggaatgtatagggcagaggtagaaagaggcaggagagttggagaacaagagcacctagaaaagaacagaggagctcaagctcatttaatcaaaatgcttaaatgttttaattccagcattctccagagttcacagaaaagagggatgcaagcccaaaaagcaaaagcaggagcttatggtcacatgcctccagctgcaggcagtggggcctctggtactgagagggaatgccacccgaatatgccccagctgtctccacccaggaaaaggaaagccaggtacacttctcatcacagtaagactagcctaacaggggaaaacagatttacatgtttcgttcattagcatattagggaaggggaaaccttttgggctctggccccgtggttgggaaacccttcctaagagcatggagccacactctggccttgatacagtagatgggacttaacacactctgatgctcaaggccttgcagcatctgataccagaaggcacctctaaagttttgttttcaacattatttcatctattcccagatctagtccagtgatgtcagctgcacaggtagcatttaactactgggaaaacaaaagtgctacaacaacagtgagtccatggtggagtgaggataactcctgggatttggaaccagtttgctggtatcaaggatcacacaagaggctataaacctccaaccctgaaccaagtcaaacctaagcctggggatttccctcggatgaaatcaccagaacttctttcctattttcagtctcttccttcagtgagctgaggattcttttagctagctggatttcagtcaaacaatgtttttgtggtcattacttgtactgtttttctagtgcatcttttcccttttgtttgcaaaagtcaatctcaccccatgtagatgttaactgatatccacacattcgacctggtgtggataacatctctggtagtgcctcggtggtcaggaagcattaccaggaaggactcatcttcaaggaccgtttctttactgcctgctgaatatggatcataggctcagatgcccaaagcacctggggtacaggtctacatggcaacccaatgccacataggaaaagaaaacagtccatttttaagccgttcttaccgactttttttttttttttttttgagacggagtcttgctttgtcaccaggctggagtgcagtggctcgatctcggctcactgcaacctccacctcccgggttcaagagattctcctgcctcagcctcctgagtagctggggctacaggcacaagccaccgtgcccagctaatttttgtatttttagtagagatggggtttcaccatgttagccaggatggtctcgatctcttgacctcgtgatctgcccacctcagcttcccaaagtgttattgacttttaaagcttttttgttcttctcatttaaaacattttacctcccctccttaacttcccattctatttcaccatctcttcaaaattgtctcccagaaaaactgaaaattcacctgctgggtatgcagaaaattatgcagatgtgaaatcagtgtagagacaactttggagtttatgtctgagtatgctgccaatataattttcatattcagactttttagagacagggtttcactctgtcatgcaggctggggtgcagtggtgtgattatagctcatggaagcctcaaactcctggactcaagggatcctcctgcctcagactcccaaagtgctgggattacaggcatgtgccatcacatccggctaatttttttttttgtagagatgaatcttactatgttgtccaggctggtctcaaactactggcctcaaccgagtctcctgctttggccttccaaagtgctgggaatacaggcatgagccatcatgcctggcccatatccaaatattttatgtttggtcaaaaatagaaaattctattataaaaaataaagttactatggcaacattttcccaacatagttcccagtatataaacttatttttcttaaaatgataacaaggtagctcaataacaatacaataccagtgataaccaaatataattgaatttttctaaaactacattcttacattccctatccactcaactcttgtaatggttttccacttttaaaaactatcaaaataggatttttaaaaatttatcaagaccacataatgcagttgaacactcaaagtgttccatgcaactgtggttgaactattcagattccagacttctaccaagaacaatccaaagagcaaactcccaaaatgacctcctgcgtggtacaaaacaagccaggctgaaatttcgggaaacctaagggatcttatccagaaccatattttggaaaactgtgatcaatcaattttttgacagtgaaagagagtaactttccagagtatgtgttaattatatctctatcaagctttaaaaagttaacagatacttaactcttgttcataaaaaatgaggccctcaagctaattaagatgactgggaaaggtgcagaggagtaattaattttggaggcgctctgggaacaggtacacagggtacagtagtcatcatcattaaaacaacaggcactcagctctactgaaaaggctgatgacagcagcccctcccaagcggatctgtaaagtgccactgaatccatgttcattcacctactccaggttgtggtcaattgtaagtaatcctgaaattctcatttctgctcatgctgacaaacttatcatctagaagtactggttattcaattaatttttaaaatattcggatataccctgcaaataaatataaaacatctctgtacccaaacagtcccaccactataaaaggttacatataaattaaataaactcagatttcttaaccattttctcagcttaagtttgccctcaccctaaatgaagtccaatttatatccaaaatataattaaatattccaaaggtatatcgaacctaagatattgaaaaaatgtaaacaaaatttatctagcttacatttatgaaccatatttttaggtttttaattcatcctgtactgaccctctgaaaaaaaaaactaatcaagttatgtttagactgaaagctgatttggattttaaagtggttccttggagacaactctcaatgactaaaaccagtgttattgaatcaagtggtttactgtatcattcaacttaaaagaccaaaatatttcctttctctcttccaataaagctctttctggatgagcccccagatccagctgtcctaggtaaacgtgctgaactggctggagatcctgcagtaatgcttggcacagaaccaaggctgggtatcaagcaacctcatgacttccactgcaactgtttaacatccccaattcctggtttttcagtccagttggctgaaaaggatggaaactggagtgtaaagtagagaagcagaaagagaaacatagattgatcctcaaaagaaaatcaaagaatccattcatcacagtgtcatcctcatactccacagtcagactgcttctcctgaagctgccttgttagtatctgatatgaagacagaaaagccactcctatgtggaaaaggatttgccagaggttcctcagcccgtgcaggtacatgttgcccaggcaaataaagagcagcataagcaccaccttcatagtcctggctggactgtagaacaggtacaaataacactggaaaatgcaggctacgaaaggaacaagaaaagccagaatgtttccaatttcctcatgggcaacctgtaaagaatgttctgcaaggtgaactcctcgaatgagattcagggcagcacacatgatgttgagaatgagggagaggatacccagggctgtcactggttccattcggaaattaggagcaggctccaagtgcatcggtgtgtgaccattcatcaccccatttgccacatctgtgtcctccagagtgagaaccgctggaggctgcaacttgagctcctcctgaattttttccaagctgcactccatctgagaggaacttacatagttaaaatgccacttcactttctgaatgatgctgtcaaactcaagaaaagcgtatggcctggaggctaggccaatgcaggtagtgtcataggaagctgtgaattcccaccacagggtctccaggaagcagaaggccatggctgctggacactggcaggagcagatagccatgcaggccacgtccccgaaagaagaaaaactgaattctgcacttgcttggctttaaacagtcctgtagctgtttgctgcaggtatattgtctcttcagttcgacctattcctgagactgtctttcttccgcttcctttaaaatgtctagtagtcttaatcaatgacagcctgtgatcactcttatttattcatgcatgagggatgcatattctattgggggaattagcctcagacttctccacatctattgagaaaacgtttttcttctttaattgtatactaaagtcacaaccttctgcagaacctcgacctggatactgggccagtcgcaaggctaaactcttgagccgtctcctccattccaaaaaatcttgggtgtggtaaaaatcagtagaggctgagaggggcagtccatcccttacccgtaccacgcaggcaaaaaagatcacggacatggtccacaagagaagtcatgaggacacctcgcccggacggcggccttcggaagtcggcgcctgccagctacccgccgcctcctcagcaatcttagccgaccgggagggctcggcccaggtcaccggcagcccaggcgcaggtaggccgtggtgcgcgtgcgcga

SEQ ID NO: 19696 - RNA, 5763 nt, Homo sapiens
  source 1..5763: mol_type = other RNA
ttttgcaccttttggagtgaaaaaaatgaggtttacactgtagtataacaaaatgcctttttgtaaaggccagaagaaatggctgtgctgtgctgcctgaagcagaaaaaccttcatgtaccaggtgaatgtaaagcctttctcctcccacacacaatggactcacccagtattaccctccactaccacttttgaccctcataacagcaccctggcgggggggcagattgatgttatcaccatttaccagatgaggaaactgaggcctgatgggcagtgatttgtgcactgcgacataggactcagtgaagagcctagccagctgacggtcagctgactggtgcactctttccctcaccttctctctcaagggcacagctacactctttctccaccattattaacactcacagggcacaggtagagcgtccccagacctgtgcaatattctacacgaaaacatttggaatgtgagcaatgtctgaacaggggcttgccaggcacatctgatcaccataaatgctcccacccctgcctgtcctcacttgtgctgcactatgcaagcaagcagcaggttctcagaaggccactgtcctgcatgtcacaatgagtggccaactccttcacagaacagcaaatagcagccctggctacaaggtgcagtgtgcaacccccatatgccaaggggcagctgctatcttccagcagagagagaacccccagctctgctccctacctatgccctgcttcctgtgcctcacacagccagccttgctggcctgctggctattgtctctgactctgagctgtgctgaccaccaagtgttactcctctccaagacttgactcccaggcatgggtgggagagttgaacctcaatgcaatctgctcccactctgaagctcgtctacccaccccatttgttacaattaaagatggttttctcatccctccagagactccagtttcagactctgtctccagagctggaatgtatagggcagaggtagaaagaggcaggagagttggagaacaagagcacctagaaaagaacagaggagctcaagctcatttaatcaaaatgcttaaatgttttaattccagcattctccagagttcacagaaaagagggatgcaagcccaaaaagcaaaagcaggagcttatggtcacatgcctccagctgcaggcagtggggcctctggtactgagagggaatgccacccgaatatgccccagctgtctccacccaggaaaaggaaagccaggtacacttctcatcacagtaagactagcctaacaggggaaaacagatttacatgtttcgttcattagcatattagggaaggggaaaccttttgggctctggccccgtggttgggaaacccttcctaagagcatggagccacactctggccttgatacagtagatgggacttaacacactctgatgctcaaggccttgcagcatctgataccagaaggcacctctaaagttttgttttcaacattatttcatctattcccagatctagtccagtgatgtcagctgcacaggtagcatttaactactgggaaaacaaaagtgctacaacaacagtgagtccatggtggagtgaggataactcctgggatttggaaccagtttgctggtatcaaggatcacacaagaggctataaacctccaaccctgaaccaagtcaaacctaagcctggggatttccctcggatgaaatcaccagaacttctttcctattttcagtctcttccttcagtgagctgaggattcttttagctagctggatttcagtcaaacaatgtttttgtggtcattacttgtactgtttttctagtgcatcttttcccttttgtttgcaaaagtcaatctcaccccatgtagatgttaactgatatccacacattcgacctggtgtggataacatctctggtagtgcctcggtggtcaggaagcattaccaggaaggactcatcttcaaggaccgtttctttactgcctgctgaatatggatcataggctcagatgcccaaagcacctggggtacaggtctacatggcaacccaatgccacataggaaaagaaaacagtccatttttaagccgttcttaccgactttttttttttttttttttgagacggagtcttgctttgtcaccaggctggagtgcagtggctcgatctcggctcactgcaacctccacctcccgggttcaagagattctcctgcctcagcctcctgagtagctggggctacaggcacaagccaccgtgcccagctaatttttgtatttttagtagagatggggtttcaccatgttagccaggatggtctcgatctcttgacctcgtgatctgcccacctcagcttcccaaagtgttattgacttttaaagcttttttgttcttctcatttaaaacattttacctcccctccttaacttcccattctatttcaccatctcttcaaaattgtctcccagaaaaactgaaaattcacctgctgggtatgcagaaaattatgcagatgtgaaatcagtgtagagacaactttggagtttatgtctgagtatgctgccaatataattttcatattcagactttttagagacagggtttcactctgtcatgcaggctggggtgcagtggtgtgattatagctcatggaagcctcaaactcctggactcaagggatcctcctgcctcagactcccaaagtgctgggattacaggcatgtgccatcacatccggctaatttttttttttgtagagatgaatcttactatgttgtccaggctggtctcaaactactggcctcaaccgagtctcctgctttggccttccaaagtgctgggaatacaggcatgagccatcatgcctggcccatatccaaatattttatgtttggtcaaaaatagaaaattctattataaaaaataaagttactatggcaacattttcccaacatagttcccagtatataaacttatttttcttaaaatgataacaaggtagctcaataacaatacaataccagtgataaccaaatataattgaatttttctaaaactacattcttacattccctatccactcaactcttgtaatggttttccacttttaaaaactatcaaaataggatttttaaaaatttatcaagaccacataatgcagttgaacactcaaagtgttccatgcaactgtggttgaactattcagattccagacttctaccaagaacaatccaaagagcaaactcccaaaatgacctcctgcgtggtacaaaacaagccaggctgaaatttcgggaaacctaagggatcttatccagaaccatattttggaaaactgtgatcaatcaattttttgacagtgaaagagagtaactttccagagtatgtgttaattatatctctatcaagctttaaaaagttaacagatacttaactcttgttcataaaaaatgaggccctcaagctaattaagatgactgggaaaggtgcagaggagtaattaattttggaggcgctctgggaacaggtacacagggtacagtagtcatcatcattaaaacaacaggcactcagctctactgaaaaggctgatgacagcagcccctcccaagcggatctgtaaagtgccactgaatccatgttcattcacctactccaggttgtggtcaattgtaagtaatcctgaaattctcatttctgctcatgctgacaaacttatcatctagaagtactggttattcaattaatttttaaaatattcggatataccctgcaaataaatataaaacatctctgtacccaaacagtcccaccactataaaaggttacatataaattaaataaactcagatttcttaaccattttctcagcttaagtttgccctcaccctaaatgaagtccaatttatatccaaaatataattaaatattccaaaggtatatcgaacctaagatattgaaaaaatgtaaacaaaatttatctagcttacatttatgaaccatatttttaggtttttaattcatcctgtactgaccctctgaaaaaaaaaactaatcaagttatgtttagactgaaagctgatttggattttaaagtggttccttggagacaactctcaatgactaaaaccagtgttattgaatcaagtggtttactgtatcattcaacttaaaagaccaaaatatttcctttctctcttccaataaagctctttctggatgagcccccagatccagctgtcctaggtaaacgtgctgaactggctggagatcctgcagtaatgcttggcacagaaccaaggctgggtatcaagcaacctcatgacttccactgcaactgtttaacatccccaattcctggtttttcagtccagttggctgaaaaggatggaaactggagtgtaaagtagagaagcagaaagagaaacatagattgatcctcaaaagaaaatcaaagaatccattcatcacagtgtcatcctcatactccacagtcagactgcttctcctgaagctgccttgttagtatctgatatgaagacagaaaagccactcctatgtggaaaaggatttgccagaggttcctcagcccgtgcaggtacatgttgcccaggcaaataaagagcagcataagcaccaccttcatagtcctggctggactgtagaacaggtacaaataacactggaaaatgcaggctacgaaaggaacaagaaaagccagaatgtttccaatttcctcatgggcaacctgtaaagaatgttctgcaaggtgaactcctcgaatgagattcagggcagcacacatgatgttgagaatgagggagaggatacccagggctgtcactggttccattcggaaattaggagcaggctccaagtgcatcggtgtgtgaccattcatcaccccatttgccacatctgtgtcctccagagtgagaaccgctggaggctgcaacttgagctcctcctgaattttttccaagctgcactccatctgagaggaacttacatagttaaaatgccacttcactttctgaatgatgctgtcaaactcaagaaaagcgtatggcctggaggctaggccaatgcaggtagtgtcataggaagctgtgaattcccaccacagggtctccaggaagcagaaggccatggctgctggacactggcaggagcagatagccatgcaggccacgtccccgaaagaagaaaaactgaattctgcacttgcttggctttaaacagtcctgtagctgtttgctgcaggtatattgtctcttcagttcgacctattcctgagactgtctttcttccgcttcctttaaaatgtctagtagtcttaatcaatgacagcctgtgatcactcttatttattcatgcatgagggatgcatattctattgggggaattagcctcagacttctccacattgtatactaaagtcacaaccttctgcagaacctcgacctggatactgggccagtcgcaaggctaaactcttgagccgtctcctccattccaaaaaatcttgggtgtggtaaaaatcagtagaggctgagaggggcagtccatcccttacccgtaccacgcaggcaaaaaagatcacggacatggtccacaagagaagtcatgaggacaccgcggcggtttgagatccaagcctgtaattctcacgtccggaggtgagaaggagccttcgtgatctaagctcgattcctgccggggtagcaaccggact

SEQ ID NO: 19697 - RNA, 5805 nt, Homo sapiens
  source 1..5805: mol_type = other RNA
ttttgcaccttttggagtgaaaaaaatgaggtttacactgtagtataacaaaatgcctttttgtaaaggccagaagaaatggctgtgctgtgctgcctgaagcagaaaaaccttcatgtaccaggtgaatgtaaagcctttctcctcccacacacaatggactcacccagtattaccctccactaccacttttgaccctcataacagcaccctggcgggggggcagattgatgttatcaccatttaccagatgaggaaactgaggcctgatgggcagtgatttgtgcactgcgacataggactcagtgaagagcctagccagctgacggtcagctgactggtgcactctttccctcaccttctctctcaagggcacagctacactctttctccaccattattaacactcacagggcacaggtagagcgtccccagacctgtgcaatattctacacgaaaacatttggaatgtgagcaatgtctgaacaggggcttgccaggcacatctgatcaccataaatgctcccacccctgcctgtcctcacttgtgctgcactatgcaagcaagcagcaggttctcagaaggccactgtcctgcatgtcacaatgagtggccaactccttcacagaacagcaaatagcagccctggctacaaggtgcagtgtgcaacccccatatgccaaggggcagctgctatcttccagcagagagagaacccccagctctgctccctacctatgccctgcttcctgtgcctcacacagccagccttgctggcctgctggctattgtctctgactctgagctgtgctgaccaccaagtgttactcctctccaagacttgactcccaggcatgggtgggagagttgaacctcaatgcaatctgctcccactctgaagctcgtctacccaccccatttgttacaattaaagatggttttctcatccctccagagactccagtttcagactctgtctccagagctggaatgtatagggcagaggtagaaagaggcaggagagttggagaacaagagcacctagaaaagaacagaggagctcaagctcatttaatcaaaatgcttaaatgttttaattccagcattctccagagttcacagaaaagagggatgcaagcccaaaaagcaaaagcaggagcttatggtcacatgcctccagctgcaggcagtggggcctctggtactgagagggaatgccacccgaatatgccccagctgtctccacccaggaaaaggaaagccaggtacacttctcatcacagtaagactagcctaacaggggaaaacagatttacatgtttcgttcattagcatattagggaaggggaaaccttttgggctctggccccgtggttgggaaacccttcctaagagcatggagccacactctggccttgatacagtagatgggacttaacacactctgatgctcaaggccttgcagcatctgataccagaaggcacctctaaagttttgttttcaacattatttcatctattcccagatctagtccagtgatgtcagctgcacaggtagcatttaactactgggaaaacaaaagtgctacaacaacagtgagtccatggtggagtgaggataactcctgggatttggaaccagtttgctggtatcaaggatcacacaagaggctataaacctccaaccctgaaccaagtcaaacctaagcctggggatttccctcggatgaaatcaccagaacttctttcctattttcagtctcttccttcagtgagctgaggattcttttagctagctggatttcagtcaaacaatgtttttgtggtcattacttgtactgtttttctagtgcatcttttcccttttgtttgcaaaagtcaatctcaccccatgtagatgttaactgatatccacacattcgacctggtgtggataacatctctggtagtgcctcggtggtcaggaagcattaccaggaaggactcatcttcaaggaccgtttctttactgcctgctgaatatggatcataggctcagatgcccaaagcacctggggtacaggtctacatggcaacccaatgccacataggaaaagaaaacagtccatttttaagccgttcttaccgactttttttttttttttttttgagacggagtcttgctttgtcaccaggctggagtgcagtggctcgatctcggctcactgcaacctccacctcccgggttcaagagattctcctgcctcagcctcctgagtagctggggctacaggcacaagccaccgtgcccagctaatttttgtatttttagtagagatggggtttcaccatgttagccaggatggtctcgatctcttgacctcgtgatctgcccacctcagcttcccaaagtgttattgacttttaaagcttttttgttcttctcatttaaaacattttacctcccctccttaacttcccattctatttcaccatctcttcaaaattgtctcccagaaaaactgaaaattcacctgctgggtatgcagaaaattatgcagatgtgaaatcagtgtagagacaactttggagtttatgtctgagtatgctgccaatataattttcatattcagactttttagagacagggtttcactctgtcatgcaggctggggtgcagtggtgtgattatagctcatggaagcctcaaactcctggactcaagggatcctcctgcctcagactcccaaagtgctgggattacaggcatgtgccatcacatccggctaatttttttttttgtagagatgaatcttactatgttgtccaggctggtctcaaactactggcctcaaccgagtctcctgctttggccttccaaagtgctgggaatacaggcatgagccatcatgcctggcccatatccaaatattttatgtttggtcaaaaatagaaaattctattataaaaaataaagttactatggcaacattttcccaacatagttcccagtatataaacttatttttcttaaaatgataacaaggtagctcaataacaatacaataccagtgataaccaaatataattgaatttttctaaaactacattcttacattccctatccactcaactcttgtaatggttttccacttttaaaaactatcaaaataggatttttaaaaatttatcaagaccacataatgcagttgaacactcaaagtgttccatgcaactgtggttgaactattcagattccagacttctaccaagaacaatccaaagagcaaactcccaaaatgacctcctgcgtggtacaaaacaagccaggctgaaatttcgggaaacctaagggatcttatccagaaccatattttggaaaactgtgatcaatcaattttttgacagtgaaagagagtaactttccagagtatgtgttaattatatctctatcaagctttaaaaagttaacagatacttaactcttgttcataaaaaatgaggccctcaagctaattaagatgactgggaaaggtgcagaggagtaattaattttggaggcgctctgggaacaggtacacagggtacagtagtcatcatcattaaaacaacaggcactcagctctactgaaaaggctgatgacagcagcccctcccaagcggatctgtaaagtgccactgaatccatgttcattcacctactccaggttgtggtcaattgtaagtaatcctgaaattctcatttctgctcatgctgacaaacttatcatctagaagtactggttattcaattaatttttaaaatattcggatataccctgcaaataaatataaaacatctctgtacccaaacagtcccaccactataaaaggttacatataaattaaataaactcagatttcttaaccattttctcagcttaagtttgccctcaccctaaatgaagtccaatttatatccaaaatataattaaatattccaaaggtatatcgaacctaagatattgaaaaaatgtaaacaaaatttatctagcttacatttatgaaccatatttttaggtttttaattcatcctgtactgaccctctgaaaaaaaaaactaatcaagttatgtttagactgaaagctgatttggattttaaagtggttccttggagacaactctcaatgactaaaaccagtgttattgaatcaagtggtttactgtatcattcaacttaaaagaccaaaatatttcctttctctcttccaataaagctctttctggatgagcccccagatccagctgtcctaggtaaacgtgctgaactggctggagatcctgcagtaatgcttggcacagaaccaaggctgggtatcaagcaacctcatgacttccactgcaactgtttaacatccccaattcctggtttttcagtccagttggctgaaaaggatggaaactggagtgtaaagtagagaagcagaaagagaaacatagattgatcctcaaaagaaaatcaaagaatccattcatcacagtgtcatcctcatactccacagtcagactgcttctcctgaagctgccttgttagtatctgatatgaagacagaaaagccactcctatgtggaaaaggatttgccagaggttcctcagcccgtgcaggtacatgttgcccaggcaaataaagagcagcataagcaccaccttcatagtcctggctggactgtagaacaggtacaaataacactggaaaatgcaggctacgaaaggaacaagaaaagccagaatgtttccaatttcctcatgggcaacctgtaaagaatgttctgcaaggtgaactcctcgaatgagattcagggcagcacacatgatgttgagaatgagggagaggatacccagggctgtcactggttccattcggaaattaggagcaggctccaagtgcatcggtgtgtgaccattcatcaccccatttgccacatctgtgtcctccagagtgagaaccgctggaggctgcaacttgagctcctcctgaattttttccaagctgcactccatctgagaggaacttacatagttaaaatgccacttcactttctgaatgatgctgtcaaactcaagaaaagcgtatggcctggaggctaggccaatgcaggtagtgtcataggaagctgtgaattcccaccacagggtctccaggaagcagaaggccatggctgctggacactggcaggagcagatagccatgcaggccacgtccccgaaagaagaaaaactgaattctgcacttgcttggctttaaacagtcctgtagctgtttgctgcaggtatattgtctcttcagttcgacctattcctgagactgtctttcttccgcttcctttaaaatgtctagtagtcttaatcaatgacagcctgtgatcactcttatttattcatgcatgagggatgcatattctattgggggaattagcctcagacttctccacattgtatactaaagtcacaaccttctgcagaacctcgacctggatactgggccagtcgcaaggctaaactcttgagccgtctcctccattccaaaaaatcttgggtgtggtaaaaatcagtagaggctgagaggggcagtccatcccttacccgtaccacgcaggcaaaaaagatcacggacatggtccacaagagaagtcatgaggacacctcgcccggacggcggccttcggaagtcggcgcctgccagctacccgccgcctcctcagcaatcttagccgaccgggagggctcggcccaggtcaccggcagcccaggcgcaggtaggccgtggtgcgcgtgcgcgagtct

SEQ ID NO: 19698 - RNA, 5694 nt, Homo sapiens
  source 1..5694: mol_type = other RNA
ttttgcaccttttggagtgaaaaaaatgaggtttacactgtagtataacaaaatgcctttttgtaaaggccagaagaaatggctgtgctgtgctgcctgaagcagaaaaaccttcatgtaccaggtgaatgtaaagcctttctcctcccacacacaatggactcacccagtattaccctccactaccacttttgaccctcataacagcaccctggcgggggggcagattgatgttatcaccatttaccagatgaggaaactgaggcctgatgggcagtgatttgtgcactgcgacataggactcagtgaagagcctagccagctgacggtcagctgactggtgcactctttccctcaccttctctctcaagggcacagctacactctttctccaccattattaacactcacagggcacaggtagagcgtccccagacctgtgcaatattctacacgaaaacatttggaatgtgagcaatgtctgaacaggggcttgccaggcacatctgatcaccataaatgctcccacccctgcctgtcctcacttgtgctgcactatgcaagcaagcagcaggttctcagaaggccactgtcctgcatgtcacaatgagtggccaactccttcacagaacagcaaatagcagccctggctacaaggtgcagtgtgcaacccccatatgccaaggggcagctgctatcttccagcagagagagaacccccagctctgctccctacctatgccctgcttcctgtgcctcacacagccagccttgctggcctgctggctattgtctctgactctgagctgtgctgaccaccaagtgttactcctctccaagacttgactcccaggcatgggtgggagagttgaacctcaatgcaatctgctcccactctgaagctcgtctacccaccccatttgttacaattaaagatggttttctcatccctccagagactccagtttcagactctgtctccagagctggaatgtatagggcagaggtagaaagaggcaggagagttggagaacaagagcacctagaaaagaacagaggagctcaagctcatttaatcaaaatgcttaaatgttttaattccagcattctccagagttcacagaaaagagggatgcaagcccaaaaagcaaaagcaggagcttatggtcacatgcctccagctgcaggcagtggggcctctggtactgagagggaatgccacccgaatatgccccagctgtctccacccaggaaaaggaaagccaggtacacttctcatcacagtaagactagcctaacaggggaaaacagatttacatgtttcgttcattagcatattagggaaggggaaaccttttgggctctggccccgtggttgggaaacccttcctaagagcatggagccacactctggccttgatacagtagatgggacttaacacactctgatgctcaaggccttgcagcatctgataccagaaggcacctctaaagttttgttttcaacattatttcatctattcccagatctagtccagtgatgtcagctgcacaggtagcatttaactactgggaaaacaaaagtgctacaacaacagtgagtccatggtggagtgaggataactcctgggatttggaaccagtttgctggtatcaaggatcacacaagaggctataaacctccaaccctgaaccaagtcaaacctaagcctggggatttccctcggatgaaatcaccagaacttctttcctattttcagtctcttccttcagtgagctgaggattcttttagctagctggatttcagtcaaacaatgtttttgtggtcattacttgtactgtttttctagtgcatcttttcccttttgtttgcaaaagtcaatctcaccccatgtagatgttaactgatatccacacattcgacctggtgtggataacatctctggtagtgcctcggtggtcaggaagcattaccaggaaggactcatcttcaaggaccgtttctttactgcctgctgaatatggatcataggctcagatgcccaaagcacctggggtacaggtctacatggcaacccaatgccacataggaaaagaaaacagtccatttttaagccgttcttaccgactttttttttttttttttttgagacggagtcttgctttgtcaccaggctggagtgcagtggctcgatctcggctcactgcaacctccacctcccgggttcaagagattctcctgcctcagcctcctgagtagctggggctacaggcacaagccaccgtgcccagctaatttttgtatttttagtagagatggggtttcaccatgttagccaggatggtctcgatctcttgacctcgtgatctgcccacctcagcttcccaaagtgttattgacttttaaagcttttttgttcttctcatttaaaacattttacctcccctccttaacttcccattctatttcaccatctcttcaaaattgtctcccagaaaaactgaaaattcacctgctgggtatgcagaaaattatgcagatgtgaaatcagtgtagagacaactttggagtttatgtctgagtatgctgccaatataattttcatattcagactttttagagacagggtttcactctgtcatgcaggctggggtgcagtggtgtgattatagctcatggaagcctcaaactcctggactcaagggatcctcctgcctcagactcccaaagtgctgggattacaggcatgtgccatcacatccggctaatttttttttttgtagagatgaatcttactatgttgtccaggctggtctcaaactactggcctcaaccgagtctcctgctttggccttccaaagtgctgggaatacaggcatgagccatcatgcctggcccatatccaaatattttatgtttggtcaaaaatagaaaattctattataaaaaataaagttactatggcaacattttcccaacatagttcccagtatataaacttatttttcttaaaatgataacaaggtagctcaataacaatacaataccagtgataaccaaatataattgaatttttctaaaactacattcttacattccctatccactcaactcttgtaatggttttccacttttaaaaactatcaaaataggatttttaaaaatttatcaagaccacataatgcagttgaacactcaaagtgttccatgcaactgtggttgaactattcagattccagacttctaccaagaacaatccaaagagcaaactcccaaaatgacctcctgcgtggtacaaaacaagccaggctgaaatttcgggaaacctaagggatcttatccagaaccatattttggaaaactgtgatcaatcaattttttgacagtgaaagagagtaactttccagagtatgtgttaattatatctctatcaagctttaaaaagttaacagatacttaactcttgttcataaaaaatgaggccctcaagctaattaagatgactgggaaaggtgcagaggagtaattaattttggaggcgctctgggaacaggtacacagggtacagtagtcatcatcattaaaacaacaggcactcagctctactgaaaaggctgatgacagcagcccctcccaagcggatctgtaaagtgccactgaatccatgttcattcacctactccaggttgtggtcaattgtaagtaatcctgaaattctcatttctgctcatgctgacaaacttatcatctagaagtactggttattcaattaatttttaaaatattcggatataccctgcaaataaatataaaacatctctgtacccaaacagtcccaccactataaaaggttacatataaattaaataaactcagatttcttaaccattttctcagcttaagtttgccctcaccctaaatgaagtccaatttatatccaaaatataattaaatattccaaaggtatatcgaacctaagatattgaaaaaatgtaaacaaaatttatctagcttacatttatgaaccatatttttaggtttttaattcatcctgtactgaccctctgaaaaaaaaaactaatcaagttatgtttagactgaaagctgatttggattttaaagtggttccttggagacaactctcaatgactaaaaccagtgttattgaatcaagtggtttactgtatcattcaacttaaaagaccaaaatatttcctttctctcttccaataaagctctttctggatgagcccccagatccagctgtcctaggtaaacgtgctgaactggctggagatcctgcagtaatgcttggcacagaaccaaggctgggtatcaagcaacctcatgacttccactgcaactgtttaacatccccaattcctggtttttcagtccagttggctgaaaaggatggaaactggagtgtaaagtagagaagcagaaagagaaacatagattgatcctcaaaagaaaatcaaagaatccattcatcacagtgtcatcctcatactccacagtcagactgcttctcctgaagctgccttgttagtatctgatatgaagacagaaaagccactcctatgtggaaaaggatttgccagaggttcctcagcccgtgcaggtacatgttgcccaggcaaataaagagcagcataagcaccaccttcatagtcctggctggactgtagaacaggtacaaataacactggaaaatgcaggctacgaaaggaacaagaaaagccagaatgtttccaatttcctcatgggcaacctgtaaagaatgttctgcaaggtgaactcctcgaatgagattcagggcagcacacatgatgttgagaatgagggagaggatacccagggctgtcactggttccattcggaaattaggagcaggctccaagtgcatcggtgtgtgaccattcatcaccccatttgccacatctgtgtcctccagagtgagaaccgctggaggctgcaacttgagctcctcctgaattttttccaagctgcactccatctgagaggaacttacatagttaaaatgccacttcactttctgaatgatgctgtcaaactcaagaaaagcgtatggcctggaggctaggccaatgcaggtagtgtcataggaagctgtgaattcccaccacagggtctccaggaagcagaaggccatggctgctggacactggcaggagcagatagccatgcaggccacgtccccgaaagaagaaaaactgaattctgcacttgcttggctttaaacagtcctgtagctgtttgctgcaggtatattgtctcttcagttcgacctattcctgagactgtctttcttccgcttcctttaaaatgtctagtagtcttaatcaatgacagcctgtgatcactcttatttattcatgcatgagggatgcatattctattgggggaattagcctcagacttctccacattgtatactaaagtcacaaccttctgcagaacctcgacctggatactgggccagtcgcaaggctaaactcttgagccgtctcctccattccaaaaaatcttgggtgtggtaaaaatcagtagaggctgagaggggcagtccatcccttacccgtaccacgcaggcaaaaaagatcacggacatggtccacaagagaagtcatgaggacaccttcagccacaggacttgagaactggttac

SEQ ID NO: 19699 - RNA, 5705 nt, Homo sapiens
  source 1..5705: mol_type = other RNA
ttttgcaccttttggagtgaaaaaaatgaggtttacactgtagtataacaaaatgcctttttgtaaaggccagaagaaatggctgtgctgtgctgcctgaagcagaaaaaccttcatgtaccaggtgaatgtaaagcctttctcctcccacacacaatggactcacccagtattaccctccactaccacttttgaccctcataacagcaccctggcgggggggcagattgatgttatcaccatttaccagatgaggaaactgaggcctgatgggcagtgatttgtgcactgcgacataggactcagtgaagagcctagccagctgacggtcagctgactggtgcactctttccctcaccttctctctcaagggcacagctacactctttctccaccattattaacactcacagggcacaggtagagcgtccccagacctgtgcaatattctacacgaaaacatttggaatgtgagcaatgtctgaacaggggcttgccaggcacatctgatcaccataaatgctcccacccctgcctgtcctcacttgtgctgcactatgcaagcaagcagcaggttctcagaaggccactgtcctgcatgtcacaatgagtggccaactccttcacagaacagcaaatagcagccctggctacaaggtgcagtgtgcaacccccatatgccaaggggcagctgctatcttccagcagagagagaacccccagctctgctccctacctatgccctgcttcctgtgcctcacacagccagccttgctggcctgctggctattgtctctgactctgagctgtgctgaccaccaagtgttactcctctccaagacttgactcccaggcatgggtgggagagttgaacctcaatgcaatctgctcccactctgaagctcgtctacccaccccatttgttacaattaaagatggttttctcatccctccagagactccagtttcagactctgtctccagagctggaatgtatagggcagaggtagaaagaggcaggagagttggagaacaagagcacctagaaaagaacagaggagctcaagctcatttaatcaaaatgcttaaatgttttaattccagcattctccagagttcacagaaaagagggatgcaagcccaaaaagcaaaagcaggagcttatggtcacatgcctccagctgcaggcagtggggcctctggtactgagagggaatgccacccgaatatgccccagctgtctccacccaggaaaaggaaagccaggtacacttctcatcacagtaagactagcctaacaggggaaaacagatttacatgtttcgttcattagcatattagggaaggggaaaccttttgggctctggccccgtggttgggaaacccttcctaagagcatggagccacactctggccttgatacagtagatgggacttaacacactctgatgctcaaggccttgcagcatctgataccagaaggcacctctaaagttttgttttcaacattatttcatctattcccagatctagtccagtgatgtcagctgcacaggtagcatttaactactgggaaaacaaaagtgctacaacaacagtgagtccatggtggagtgaggataactcctgggatttggaaccagtttgctggtatcaaggatcacacaagaggctataaacctccaaccctgaaccaagtcaaacctaagcctggggatttccctcggatgaaatcaccagaacttctttcctattttcagtctcttccttcagtgagctgaggattcttttagctagctggatttcagtcaaacaatgtttttgtggtcattacttgtactgtttttctagtgcatcttttcccttttgtttgcaaaagtcaatctcaccccatgtagatgttaactgatatccacacattcgacctggtgtggataacatctctggtagtgcctcggtggtcaggaagcattaccaggaaggactcatcttcaaggaccgtttctttactgcctgctgaatatggatcataggctcagatgcccaaagcacctggggtacaggtctacatggcaacccaatgccacataggaaaagaaaacagtccatttttaagccgttcttaccgactttttttttttttttttttgagacggagtcttgctttgtcaccaggctggagtgcagtggctcgatctcggctcactgcaacctccacctcccgggttcaagagattctcctgcctcagcctcctgagtagctggggctacaggcacaagccaccgtgcccagctaatttttgtatttttagtagagatggggtttcaccatgttagccaggatggtctcgatctcttgacctcgtgatctgcccacctcagcttcccaaagtgttattgacttttaaagcttttttgttcttctcatttaaaacattttacctcccctccttaacttcccattctatttcaccatctcttcaaaattgtctcccagaaaaactgaaaattcacctgctgggtatgcagaaaattatgcagatgtgaaatcagtgtagagacaactttggagtttatgtctgagtatgctgccaatataattttcatattcagactttttagagacagggtttcactctgtcatgcaggctggggtgcagtggtgtgattatagctcatggaagcctcaaactcctggactcaagggatcctcctgcctcagactcccaaagtgctgggattacaggcatgtgccatcacatccggctaatttttttttttgtagagatgaatcttactatgttgtccaggctggtctcaaactactggcctcaaccgagtctcctgctttggccttccaaagtgctgggaatacaggcatgagccatcatgcctggcccatatccaaatattttatgtttggtcaaaaatagaaaattctattataaaaaataaagttactatggcaacattttcccaacatagttcccagtatataaacttatttttcttaaaatgataacaaggtagctcaataacaatacaataccagtgataaccaaatataattgaatttttctaaaactacattcttacattccctatccactcaactcttgtaatggttttccacttttaaaaactatcaaaataggatttttaaaaatttatcaagaccacataatgcagttgaacactcaaagtgttccatgcaactgtggttgaactattcagattccagacttctaccaagaacaatccaaagagcaaactcccaaaatgacctcctgcgtggtacaaaacaagccaggctgaaatttcgggaaacctaagggatcttatccagaaccatattttggaaaactgtgatcaatcaattttttgacagtgaaagagagtaactttccagagtatgtgttaattatatctctatcaagctttaaaaagttaacagatacttaactcttgttcataaaaaatgaggccctcaagctaattaagatgactgggaaaggtgcagaggagtaattaattttggaggcgctctgggaacaggtacacagggtacagtagtcatcatcattaaaacaacaggcactcagctctactgaaaaggctgatgacagcagcccctcccaagcggatctgtaaagtgccactgaatccatgttcattcacctactccaggttgtggtcaattgtaagtaatcctgaaattctcatttctgctcatgctgacaaacttatcatctagaagtactggttattcaattaatttttaaaatattcggatataccctgcaaataaatataaaacatctctgtacccaaacagtcccaccactataaaaggttacatataaattaaataaactcagatttcttaaccattttctcagcttaagtttgccctcaccctaaatgaagtccaatttatatccaaaatataattaaatattccaaaggtatatcgaacctaagatattgaaaaaatgtaaacaaaatttatctagcttacatttatgaaccatatttttaggtttttaattcatcctgtactgaccctctgaaaaaaaaaactaatcaagttatgtttagactgaaagctgatttggattttaaagtggttccttggagacaactctcaatgactaaaaccagtgttattgaatcaagtggtttactgtatcattcaacttaaaagaccaaaatatttcctttctctcttccaataaagctctttctggatgagcccccagatccagctgtcctaggtaaacgtgctgaactggctggagatcctgcagtaatgcttggcacagaaccaaggctgggtatcaagcaacctcatgacttccactgcaactgtttaacatccccaattcctggtttttcagtccagttggctgaaaaggatggaaactggagtgtaaagtagagaagcagaaagagaaacatagattgatcctcaaaagaaaatcaaagaatccattcatcacagtgtcatcctcatactccacagtcagactgcttctcctgaagctgccttgttagtatctgatatgaagacagaaaagccactcctatgtggaaaaggatttgccagaggttcctcagcccgtgcaggtacatgttgcccaggcaaataaagagcagcataagcaccaccttcatagtcctggctggactgtagaacaggtacaaataacactggaaaatgcaggctacgaaaggaacaagaaaagccagaatgtttccaatttcctcatgggcaacctgtaaagaatgttctgcaaggtgaactcctcgaatgagattcagggcagcacacatgatgttgagaatgagggagaggatacccagggctgtcactggttccattcggaaattaggagcaggctccaagtgcatcggtgtgtgaccattcatcaccccatttgccacatctgtgtcctccagagtgagaaccgctggaggctgcaacttgagctcctcctgaattttttccaagctgcactccatctgagaggaacttacatagttaaaatgccacttcactttctgaatgatgctgtcaaactcaagaaaagcgtatggcctggaggctaggccaatgcaggtagtgtcataggaagctgtgaattcccaccacagggtctccaggaagcagaaggccatggctgctggacactggcaggagcagatagccatgcaggccacgtccccgaaagaagaaaaactgaattctgcacttgcttggctttaaacagtcctgtagctgtttgctgcaggtatattgtctcttcagttcgacctattcctgagactgtctttcttccgcttcctttaaaatgtctagtagttgtatactaaagtcacaaccttctgcagaacctcgacctggatactgggccagtcgcaaggctaaactcttgagccgtctcctccattccaaaaaatcttgggtgtggtaaaaatcagtagaggctgagaggggcagtccatcccttacccgtaccacgcaggcaaaaaagatcacggacatggtccacaagagaagtcatgaggacacctcgcccggacggcggccttcggaagtcggcgcctgccagctacccgccgcctcctcagcaatcttagccgaccgggagggctcggcccaggtcaccggcagcccaggcgcaggtaggccgtggtgcgcgtgc

SEQ ID NO: 19700 - RNA, 6350 nt, Homo sapiens
  source 1..6350: mol_type = other RNA
ttttgcaccttttggagtgaaaaaaatgaggtttacactgtagtataacaaaatgcctttttgtaaaggccagaagaaatggctgtgctgtgctgcctgaagcagaaaaaccttcatgtaccaggtgaatgtaaagcctttctcctcccacacacaatggactcacccagtattaccctccactaccacttttgaccctcataacagcaccctggcgggggggcagattgatgttatcaccatttaccagatgaggaaactgaggcctgatgggcagtgatttgtgcactgcgacataggactcagtgaagagcctagccagctgacggtcagctgactggtgcactctttccctcaccttctctctcaagggcacagctacactctttctccaccattattaacactcacagggcacaggtagagcgtccccagacctgtgcaatattctacacgaaaacatttggaatgtgagcaatgtctgaacaggggcttgccaggcacatctgatcaccataaatgctcccacccctgcctgtcctcacttgtgctgcactatgcaagcaagcagcaggttctcagaaggccactgtcctgcatgtcacaatgagtggccaactccttcacagaacagcaaatagcagccctggctacaaggtgcagtgtgcaacccccatatgccaaggggcagctgctatcttccagcagagagagaacccccagctctgctccctacctatgccctgcttcctgtgcctcacacagccagccttgctggcctgctggctattgtctctgactctgagctgtgctgaccaccaagtgttactcctctccaagacttgactcccaggcatgggtgggagagttgaacctcaatgcaatctgctcccactctgaagctcgtctacccaccccatttgttacaattaaagatggttttctcatccctccagagactccagtttcagactctgtctccagagctggaatgtatagggcagaggtagaaagaggcaggagagttggagaacaagagcacctagaaaagaacagaggagctcaagctcatttaatcaaaatgcttaaatgttttaattccagcattctccagagttcacagaaaagagggatgcaagcccaaaaagcaaaagcaggagcttatggtcacatgcctccagctgcaggcagtggggcctctggtactgagagggaatgccacccgaatatgccccagctgtctccacccaggaaaaggaaagccaggtacacttctcatcacagtaagactagcctaacaggggaaaacagatttacatgtttcgttcattagcatattagggaaggggaaaccttttgggctctggccccgtggttgggaaacccttcctaagagcatggagccacactctggccttgatacagtagatgggacttaacacactctgatgctcaaggccttgcagcatctgataccagaaggcacctctaaagttttgttttcaacattatttcatctattcccagatctagtccagtgatgtcagctgcacaggtagcatttaactactgggaaaacaaaagtgctacaacaacagtgagtccatggtggagtgaggataactcctgggatttggaaccagtttgctggtatcaaggatcacacaagaggctataaacctccaaccctgaaccaagtcaaacctaagcctggggatttccctcggatgaaatcaccagaacttctttcctattttcagtctcttccttcagtgagctgaggattcttttagctagctggatttcagtcaaacaatgtttttgtggtcattacttgtactgtttttctagtgcatcttttcccttttgtttgcaaaagtcaatctcaccccatgtagatgttaactgatatccacacattcgacctggtgtggataacatctctggtagtgcctcggtggtcaggaagcattaccaggaaggactcatcttcaaggaccgtttctttactgcctgctgaatatggatcataggctcagatgcccaaagcacctggggtacaggtctacatggcaacccaatgccacataggaaaagaaaacagtccatttttaagccgttcttaccgactttttttttttttttttttgagacggagtcttgctttgtcaccaggctggagtgcagtggctcgatctcggctcactgcaacctccacctcccgggttcaagagattctcctgcctcagcctcctgagtagctggggctacaggcacaagccaccgtgcccagctaatttttgtatttttagtagagatggggtttcaccatgttagccaggatggtctcgatctcttgacctcgtgatctgcccacctcagcttcccaaagtgttattgacttttaaagcttttttgttcttctcatttaaaacattttacctcccctccttaacttcccattctatttcaccatctcttcaaaattgtctcccagaaaaactgaaaattcacctgctgggtatgcagaaaattatgcagatgtgaaatcagtgtagagacaactttggagtttatgtctgagtatgctgccaatataattttcatattcagactttttagagacagggtttcactctgtcatgcaggctggggtgcagtggtgtgattatagctcatggaagcctcaaactcctggactcaagggatcctcctgcctcagactcccaaagtgctgggattacaggcatgtgccatcacatccggctaatttttttttttgtagagatgaatcttactatgttgtccaggctggtctcaaactactggcctcaaccgagtctcctgctttggccttccaaagtgctgggaatacaggcatgagccatcatgcctggcccatatccaaatattttatgtttggtcaaaaatagaaaattctattataaaaaataaagttactatggcaacattttcccaacatagttcccagtatataaacttatttttcttaaaatgataacaaggtagctcaataacaatacaataccagtgataaccaaatataattgaatttttctaaaactacattcttacattccctatccactcaactcttgtaatggttttccacttttaaaaactatcaaaataggatttttaaaaatttatcaagaccacataatgcagttgaacactcaaagtgttccatgcaactgtggttgaactattcagattccagacttctaccaagaacaatccaaagagcaaactcccaaaatgacctcctgcgtggtacaaaacaagccaggctgaaatttcgggaaacctaagggatcttatccagaaccatattttggaaaactgtgatcaatcaattttttgacagtgaaagagagtaactttccagagtatgtgttaattatatctctatcaagctttaaaaagttaacagatacttaactcttgttcataaaaaatgaggccctcaagctaattaagatgactgggaaaggtgcagaggagtaattaattttggaggcgctctgggaacaggtacacagggtacagtagtcatcatcattaaaacaacaggcactcagctctactgaaaaggctgatgacagcagcccctcccaagcggatctgtaaagtgccactgaatccatgttcattcacctactccaggttgtggtcaattgtaagtaatcctgaaattctcatttctgctcatgctgacaaacttatcatctagaagtactggttattcaattaatttttaaaatattcggatataccctgcaaataaatataaaacatctctgtacccaaacagtcccaccactataaaaggttacatataaattaaataaactcagatttcttaaccattttctcagcttaagtttgccctcaccctaaatgaagtccaatttatatccaaaatataattaaatattccaaaggtatatcgaacctaagatattgaaaaaatgtaaacaaaatttatctagcttacatttatgaaccatatttttaggtttttaattcatcctgtactgaccctctgaaaaaaaaaactaatcaagttatgtttagactgaaagctgatttggattttaaagtggttccttggagacaactctcaatgactaaaaccagtgttattgaatcaagtggtttactgtatcattcaacttaaaagaccaaaatatttcctttctctcttccaataaagctctttctggatgagcccccagatccagctgtcctaggtaaacgtgctgaactggctggagatcctgcagtaatgcttggcacagaaccaaggctgggtatcaagcaacctcatgacttccactgcaactgtttaacatccccaattcctggtttttcagtccagttggctgaaaaggatggaaactggagtgtaaagtagagaagcagaaagagaaacatagattgatcctcaaaagaaaatcaaagaatccattcatcacagtgtcatcctcatactccacagtcagactgcttctcctgaagctgccttgttagtatctgatatgaagacagaaaagccactcctatgtggaaaaggatttgccagaggttcctcagcccgtgcaggtacatgttgcccaggcaaataaagagcagcataagcaccaccttcatagtcctggctggactgtagaacaggtacaaataacactggaaaatgcaggctacgaaaggaacaagaaaagccagaatgtttccaatttcctcatgggcaacctgtaaagaatgttctgcaaggtgaactcctcgaatgagattcagggcagcacacatgatgttgagaatgagggagaggatacccagggctgtcactggttccattcggaaattaggagcaggctccaagtgcatcggtgtgtgaccattcatcaccccatttgccacatctgtgtcctccagagtgagaaccgctggaggctgcaacttgagctcctcctgaattttttccaagctgcactccatctgagaggaacttacatagttaaaatgccacttcactttctgaatgatgctgtcaaactcaagaaaagcgtatggcctggaggctaggccaatgcaggtagtgtcataggaagctgtgaattcccaccacagggtctccaggaagcagaaggccatggctgctggacactggcaggagcagatagccatgcaggccacgtccccgaaagaagaaaaatgtatactaaagtcacaaccttctgcagaacctcgacctggatactgggccagtcgcaaggctaaactcttgagccgtctcctccattccaaaaaatcttgggtgtggtaaaaatcagtagaggctgagaggggcagtccatcccttacccgtaccacgcaggcaaaaaagatcacggacatggtccacaagagaagtcatgaggacaccgcggcggtttgagatccaagcctgtaattctcacgtccggaggtgagaaggagccttcgtgatctaagctcgattcctgccggggtagcaaccggactgacgtctggaggcggggaggctccgcgtgacagagtgataacgcccggggcgtatgttctgcggtccgcgcggctgggcgggaggcccgagataggcaaaccaaagagcacaacctactgccagcctggatggggcgccaaagtccgacccagggggacacaccccaagctggggaccgaggcacccacagatggatgactggctggaaggagattaggtaggtagcagagtccgtccatttattcatttagcaagtattgagcacctgctatgtgccaggggttgtggacaaagcgaggaattcctgacacgaaaaactatgttaagagaggaggcagggtgagagcacccttcaaacaatcaaacacctgtataaatacaaactgctcttcagggaggagcaggggttttgggagaatttacagaagcttctaggctggtgttgggaatcacaggaggctaactaggcaaaggggagaggaagtgtgtttcagatggagagattagcatgtatataagaactctgtggaaggcagcagagctcctttgagggatgaaaagaaacccagaaagggggaaatggaaagttagtgcttaataggtacagaatttcagctggagaagatgaaacagttctggaaatggatagtagtgatgatcacacaacaatgtgaatgtaccaaatgccacagatctgcacacttaaaaatggttatgtacattttaccacaaaaagaaaagaaactcagagtttagagaataaaggagtggagtgagatccactagagcgaatagaaggggc

SEQ ID NO: 19701 - RNA, 5570 nt, Homo sapiens
  source 1..5570: mol_type = other RNA
ttttgcaccttttggagtgaaaaaaatgaggtttacactgtagtataacaaaatgcctttttgtaaaggccagaagaaatggctgtgctgtgctgcctgaagcagaaaaaccttcatgtaccaggtgaatgtaaagcctttctcctcccacacacaatggactcacccagtattaccctccactaccacttttgaccctcataacagcaccctggcgggggggcagattgatgttatcaccatttaccagatgaggaaactgaggcctgatgggcagtgatttgtgcactgcgacataggactcagtgaagagcctagccagctgacggtcagctgactggtgcactctttccctcaccttctctctcaagggcacagctacactctttctccaccattattaacactcacagggcacaggtagagcgtccccagacctgtgcaatattctacacgaaaacatttggaatgtgagcaatgtctgaacaggggcttgccaggcacatctgatcaccataaatgctcccacccctgcctgtcctcacttgtgctgcactatgcaagcaagcagcaggttctcagaaggccactgtcctgcatgtcacaatgagtggccaactccttcacagaacagcaaatagcagccctggctacaaggtgcagtgtgcaacccccatatgccaaggggcagctgctatcttccagcagagagagaacccccagctctgctccctacctatgccctgcttcctgtgcctcacacagccagccttgctggcctgctggctattgtctctgactctgagctgtgctgaccaccaagtgttactcctctccaagacttgactcccaggcatgggtgggagagttgaacctcaatgcaatctgctcccactctgaagctcgtctacccaccccatttgttacaattaaagatggttttctcatccctccagagactccagtttcagactctgtctccagagctggaatgtatagggcagaggtagaaagaggcaggagagttggagaacaagagcacctagaaaagaacagaggagctcaagctcatttaatcaaaatgcttaaatgttttaattccagcattctccagagttcacagaaaagagggatgcaagcccaaaaagcaaaagcaggagcttatggtcacatgcctccagctgcaggcagtggggcctctggtactgagagggaatgccacccgaatatgccccagctgtctccacccaggaaaaggaaagccaggtacacttctcatcacagtaagactagcctaacaggggaaaacagatttacatgtttcgttcattagcatattagggaaggggaaaccttttgggctctggccccgtggttgggaaacccttcctaagagcatggagccacactctggccttgatacagtagatgggacttaacacactctgatgctcaaggccttgcagcatctgataccagaaggcacctctaaagttttgttttcaacattatttcatctattcccagatctagtccagtgatgtcagctgcacaggtagcatttaactactgggaaaacaaaagtgctacaacaacagtgagtccatggtggagtgaggataactcctgggatttggaaccagtttgctggtatcaaggatcacacaagaggctataaacctccaaccctgaaccaagtcaaacctaagcctggggatttccctcggatgaaatcaccagaacttctttcctattttcagtctcttccttcagtgagctgaggattcttttagctagctggatttcagtcaaacaatgtttttgtggtcattacttgtactgtttttctagtgcatcttttcccttttgtttgcaaaagtcaatctcaccccatgtagatgttaactgatatccacacattcgacctggtgtggataacatctctggtagtgcctcggtggtcaggaagcattaccaggaaggactcatcttcaaggaccgtttctttactgcctgctgaatatggatcataggctcagatgcccaaagcacctggggtacaggtctacatggcaacccaatgccacataggaaaagaaaacagtccatttttaagccgttcttaccgactttttttttttttttttttgagacggagtcttgctttgtcaccaggctggagtgcagtggctcgatctcggctcactgcaacctccacctcccgggttcaagagattctcctgcctcagcctcctgagtagctggggctacaggcacaagccaccgtgcccagctaatttttgtatttttagtagagatggggtttcaccatgttagccaggatggtctcgatctcttgacctcgtgatctgcccacctcagcttcccaaagtgttattgacttttaaagcttttttgttcttctcatttaaaacattttacctcccctccttaacttcccattctatttcaccatctcttcaaaattgtctcccagaaaaactgaaaattcacctgctgggtatgcagaaaattatgcagatgtgaaatcagtgtagagacaactttggagtttatgtctgagtatgctgccaatataattttcatattcagactttttagagacagggtttcactctgtcatgcaggctggggtgcagtggtgtgattatagctcatggaagcctcaaactcctggactcaagggatcctcctgcctcagactcccaaagtgctgggattacaggcatgtgccatcacatccggctaatttttttttttgtagagatgaatcttactatgttgtccaggctggtctcaaactactggcctcaaccgagtctcctgctttggccttccaaagtgctgggaatacaggcatgagccatcatgcctggcccatatccaaatattttatgtttggtcaaaaatagaaaattctattataaaaaataaagttactatggcaacattttcccaacatagttcccagtatataaacttatttttcttaaaatgataacaaggtagctcaataacaatacaataccagtgataaccaaatataattgaatttttctaaaactacattcttacattccctatccactcaactcttgtaatggttttccacttttaaaaactatcaaaataggatttttaaaaatttatcaagaccacataatgcagttgaacactcaaagtgttccatgcaactgtggttgaactattcagattccagacttctaccaagaacaatccaaagagcaaactcccaaaatgacctcctgcgtggtacaaaacaagccaggctgaaatttcgggaaacctaagggatcttatccagaaccatattttggaaaactgtgatcaatcaattttttgacagtgaaagagagtaactttccagagtatgtgttaattatatctctatcaagctttaaaaagttaacagatacttaactcttgttcataaaaaatgaggccctcaagctaattaagatgactgggaaaggtgcagaggagtaattaattttggaggcgctctgggaacaggtacacagggtacagtagtcatcatcattaaaacaacaggcactcagctctactgaaaaggctgatgacagcagcccctcccaagcggatctgtaaagtgccactgaatccatgttcattcacctactccaggttgtggtcaattgtaagtaatcctgaaattctcatttctgctcatgctgacaaacttatcatctagaagtactggttattcaattaatttttaaaatattcggatataccctgcaaataaatataaaacatctctgtacccaaacagtcccaccactataaaaggttacatataaattaaataaactcagatttcttaaccattttctcagcttaagtttgccctcaccctaaatgaagtccaatttatatccaaaatataattaaatattccaaaggtatatcgaacctaagatattgaaaaaatgtaaacaaaatttatctagcttacatttatgaaccatatttttaggtttttaattcatcctgtactgaccctctgaaaaaaaaaactaatcaagttatgtttagactgaaagctgatttggattttaaagtggttccttggagacaactctcaatgactaaaaccagtgttattgaatcaagtggtttactgtatcattcaacttaaaagaccaaaatatttcctttctctcttccaataaagctctttctggatgagcccccagatccagctgtcctaggtaaacgtgctgaactggctggagatcctgcagtaatgcttggcacagaaccaaggctgggtatcaagcaacctcatgacttccactgcaactgtttaacatccccaattcctggtttttcagtccagttggctgaaaaggatggaaactggagtgtaaagtagagaagcagaaagagaaacatagattgatcctcaaaagaaaatcaaagaatccattcatcacagtgtcatcctcatactccacagtcagactgcttctcctgaagctgccttgttagtatctgatatgaagacagaaaagccactcctatgtggaaaaggatttgccagaggttcctcagcccgtgcaggtacatgttgcccaggcaaataaagagcagcataagcaccaccttcatagtcctggctggactgtagaacaggtacaaataacactggaaaatgcaggctacgaaaggaacaagaaaagccagaatgtttccaatttcctcatgggcaacctgtaaagaatgttctgcaaggtgaactcctcgaatgagattcagggcagcacacatgatgttgagaatgagggagaggatacccagggctgtcactggttccattcggaaattaggagcaggctccaagtgcatcggtgtgtgaccattcatcaccccatttgccacatctgtgtcctccagagtgagaaccgctggaggctgcaacttgagctcctcctgaattttttccaagctgcactccatctgagaggaacttacatagttaaaatgccacttcactttctgaatgatgctgtcaaactcaagaaaagcgtatggcctggaggctaggccaatgcaggtagtgtcataggaagctgtgaattcccaccacagggtctccaggaagcagaaggccatggctgctggacactggcaggagcagatagccatgcaggccacgtccccgaaagaagaaaaatgtatactaaagtcacaaccttctgcagaacctcgacctggatactgggccagtcgcaaggctaaactcttgagccgtctcctccattccaaaaaatcttgggtgtggtaaaaatcagtagaggctgagaggggcagtccatcccttacccgtaccacgcaggcaaaaaagatcacggacatggtccacaagagaagtcatgaggacacctcgcccggacggcggccttcggaagtcggcgcctgccagctacccgccgcctcctcagcaatcttagccgaccgggagggctcggcccaggtcaccggcagcccaggcgcaggtaggccgt

SEQ ID NO: 19702 - RNA, 7579 nt, Homo sapiens
  source 1..7579: mol_type = other RNA
ttttgcaccttttggagtgaaaaaaatgaggtttacactgtagtataacaaaatgcctttttgtaaaggccagaagaaatggctgtgctgtgctgcctgaagcagaaaaaccttcatgtaccaggtgaatgtaaagcctttctcctcccacacacaatggactcacccagtattaccctccactaccacttttgaccctcataacagcaccctggcgggggggcagattgatgttatcaccatttaccagatgaggaaactgaggcctgatgggcagtgatttgtgcactgcgacataggactcagtgaagagcctagccagctgacggtcagctgactggtgcactctttccctcaccttctctctcaagggcacagctacactctttctccaccattattaacactcacagggcacaggtagagcgtccccagacctgtgcaatattctacacgaaaacatttggaatgtgagcaatgtctgaacaggggcttgccaggcacatctgatcaccataaatgctcccacccctgcctgtcctcacttgtgctgcactatgcaagcaagcagcaggttctcagaaggccactgtcctgcatgtcacaatgagtggccaactccttcacagaacagcaaatagcagccctggctacaaggtgcagtgtgcaacccccatatgccaaggggcagctgctatcttccagcagagagagaacccccagctctgctccctacctatgccctgcttcctgtgcctcacacagccagccttgctggcctgctggctattgtctctgactctgagctgtgctgaccaccaagtgttactcctctccaagacttgactcccaggcatgggtgggagagttgaacctcaatgcaatctgctcccactctgaagctcgtctacccaccccatttgttacaattaaagatggttttctcatccctccagagactccagtttcagactctgtctccagagctggaatgtatagggcagaggtagaaagaggcaggagagttggagaacaagagcacctagaaaagaacagaggagctcaagctcatttaatcaaaatgcttaaatgttttaattccagcattctccagagttcacagaaaagagggatgcaagcccaaaaagcaaaagcaggagcttatggtcacatgcctccagctgcaggcagtggggcctctggtactgagagggaatgccacccgaatatgccccagctgtctccacccaggaaaaggaaagccaggtacacttctcatcacagtaagactagcctaacaggggaaaacagatttacatgtttcgttcattagcatattagggaaggggaaaccttttgggctctggccccgtggttgggaaacccttcctaagagcatggagccacactctggccttgatacagtagatgggacttaacacactctgatgctcaaggccttgcagcatctgataccagaaggcacctctaaagttttgttttcaacattatttcatctattcccagatctagtccagtgatgtcagctgcacaggtagcatttaactactgggaaaacaaaagtgctacaacaacagtgagtccatggtggagtgaggataactcctgggatttggaaccagtttgctggtatcaaggatcacacaagaggctataaacctccaaccctgaaccaagtcaaacctaagcctggggatttccctcggatgaaatcaccagaacttctttcctattttcagtctcttccttcagtgagctgaggattcttttagctagctggatttcagtcaaacaatgtttttgtggtcattacttgtactgtttttctagtgcatcttttcccttttgtttgcaaaagtcaatctcaccccatgtagatgttaactgatatccacacattcgacctggtgtggataacatctctggtagtgcctcggtggtcaggaagcattaccaggaaggactcatcttcaaggaccgtttctttactgcctgctgaatatggatcataggctcagatgcccaaagcacctggggtacaggtctacatggcaacccaatgccacataggaaaagaaaacagtccatttttaagccgttcttaccgactttttttttttttttttttgagacggagtcttgctttgtcaccaggctggagtgcagtggctcgatctcggctcactgcaacctccacctcccgggttcaagagattctcctgcctcagcctcctgagtagctggggctacaggcacaagccaccgtgcccagctaatttttgtatttttagtagagatggggtttcaccatgttagccaggatggtctcgatctcttgacctcgtgatctgcccacctcagcttcccaaagtgttattgacttttaaagcttttttgttcttctcatttaaaacattttacctcccctccttaacttcccattctatttcaccatctcttcaaaattgtctcccagaaaaactgaaaattcacctgctgggtatgcagaaaattatgcagatgtgaaatcagtgtagagacaactttggagtttatgtctgagtatgctgccaatataattttcatattcagactttttagagacagggtttcactctgtcatgcaggctggggtgcagtggtgtgattatagctcatggaagcctcaaactcctggactcaagggatcctcctgcctcagactcccaaagtgctgggattacaggcatgtgccatcacatccggctaatttttttttttgtagagatgaatcttactatgttgtccaggctggtctcaaactactggcctcaaccgagtctcctgctttggccttccaaagtgctgggaatacaggcatgagccatcatgcctggcccatatccaaatattttatgtttggtcaaaaatagaaaattctattataaaaaataaagttactatggcaacattttcccaacatagttcccagtatataaacttatttttcttaaaatgataacaaggtagctcaataacaatacaataccagtgataaccaaatataattgaatttttctaaaactacattcttacattccctatccactcaactcttgtaatggttttccacttttaaaaactatcaaaataggatttttaaaaatttatcaagaccacataatgcagttgaacactcaaagtgttccatgcaactgtggttgaactattcagattccagacttctaccaagaacaatccaaagagcaaactcccaaaatgacctcctgcgtggtacaaaacaagccaggctgaaatttcgggaaacctaagggatcttatccagaaccatattttggaaaactgtgatcaatcaattttttgacagtgaaagagagtaactttccagagtatgtgttaattatatctctatcaagctttaaaaagttaacagatacttaactcttgttcataaaaaatgaggccctcaagctaattaagatgactgggaaaggtgcagaggagtaattaattttggaggcgctctgggaacaggtacacagggtacagtagtcatcatcattaaaacaacaggcactcagctctactgaaaaggctgatgacagcagcccctcccaagcggatctgtaaagtgccactgaatccatgttcattcacctactccaggttgtggtcaattgtaagtaatcctgaaattctcatttctgctcatgctgacaaacttatcatctagaagtactggttattcaattaatttttaaaatattcggatataccctgcaaataaatataaaacatctctgtacccaaacagtcccaccactataaaaggttacatataaattaaataaactcagatttcttaaccattttctcagcttaagtttgccctcaccctaaatgaagtccaatttatatccaaaatataattaaatattccaaaggtatatcgaacctaagatattgaaaaaatgtaaacaaaatttatctagcttacatttatgaaccatatttttaggtttttaattcatcctgtactgaccctctgaaaaaaaaaactaatcaagttatgtttagactgaaagctgatttggattttaaagtggttccttggagacaactctcaatgactaaaaccagtgttattgaatcaagtggtttactgtatcattcaacttaaaagaccaaaatatttcctttctctcttccaataaagctctttctggatgagcccccagatccagctgtcctaggtaaacgtgctgaactggctggagatcctgcagtaatgcttggcacagaaccaaggctgggtatcaagcaacctcatgacttccactgcaactgtttaacatccccaattcctggtttttcagtccagttggctgaaaaggatggaaactggagtgtaaagtagagaagcagaaagagaaacatagattgatcctcaaaagaaaatcaaagaatccattcatcacagtgtcatcctcatactccacagtcagactgcttctcctgaagctgccttgttagtatctgatatgaagacagaaaagccactcctatgtggaaaaggatttgccagaggttcctcagcccgtgcaggtacatgttgcccaggcaaataaagagcagcataagcaccaccttcatagtcctggctggactgtagaacaggtacaaataacactggaaaatgcaggctacgaaaggaacaagaaaagccagaatgtttccaatttcctcatgggcaacctgtaaagaatgttctgcaaggtgaactcctcgaatgagattcagggcagcacacatgatgttgagaatgagggagaggatacccagggctgtcactggttccattcggaaattaggagcaggctccaagtgcatcggtgtgtgaccattcatcaccccatttgccacatctgtgtcctccagagtgagaaccgctggaggctgcaacttgagctcctcctgaattttttccaagctgcactccatctgagaggaacttacatagttaaaatgccacttcactttctgaatgatgctgtcaaactcaagaaaagcgtatggcctggaggctaggccaatgcaggtagtgtcataggaagctgtgaattcccaccacagggtctccaggaagcagaaggccatggctgctggacactggcaggagcagatagccatgcaggccacgtccccgaaagaagaaaaatgtatactaaagtcacaaccttctgcagaacctcgacctggatactgggccagtcgcaaggctaaactcttgagccgtctcctccattccaaaaaatcttgggtgtggtaaaaatcagtagaggctgagaggggcagtccatcccttacccgtaccacgcaggcaaaaaagatcacggacatggtccacaagagaagtcatgaggacacctcggtcgcgatgggggcgcaggaccggccgcagtgccacttcgacatcgagatcaaccgggagccgggtgagctggaaactggggagcgctgctggggccgaggcctgccttggcgaaggggaggggtctaccctcagcaaccctcccccggcctttttgggagcgggtaggaggcgcaggcaactttccgttttctcttgagagaaaatcagtgggagaggaaggtggcctgggcacacccctaactcgcagtccgggcctcttcctgccaaaccccacacaccccgctgcatctccggactgagtcctcgtagccagcctggcgccaagaaaaggaggtgcagttctttgaggactttttctctcccagtgtctccgtgaggcagacactcccgatccgatttccggttatcttgcttggtgctatgaagtttcaactagtaggaaatattgtgtgtttcctaatcacgatatatcactaatatgttaattttgcctctatttttccttaagaatctttagctagaatttcgtggttcctgggaaaatggcttagtgaagatcttttgtgataaaccagagcattttgtaccagcagaattgcagcatgcatgcacttagcattaatgtttgtctttagggaatccagacatttgttagtgtattttttttaaatgaaacatttccttctaaagcatagttatttcattctaagtagcagagcgtgcagggtttcaaactgttttcttagctttttttgttatccgtgacaaaagttttaattggagacatatatatatgtgttgtctttgtgcaacatcttgttctgcatattcttatgagagcctgctactgttctagggtctggagatagagcagcgcataaaacaaaggcctcttccttttatagtttatattctattggggggaagacggacaactaggaaaaaaataacagtgacttgtagttgggatactattttaataagttggtcagacaaggccattttgagaagatgagatttaagcaggtatcagaaggagatgaagtgagccgtatttaagaagagcattcgtggtagagggaaacagcacagccctgaggtgaggagtagtatacagtcaggcgccaaatgacatttctatctttaacaatggtcttatatataatacctttttttggtaactttttaatgtttagctgtgtttagatatacaaatacttcattgtgttaaagttgcctacggtattcagtggagtaacatcctgtacaggtttgtagcctaggagcaaatagactatatagcttaggtgtgtagtaggccgtaccatctaggtgtgtttaaatacattccatgatgttcacacaatgacgaaattgcctaattacacatttctcagaatccgtcctggttattaaacaatggaggactgtacttgcatgtttgagggacagcagggtgcccagtgtggctggagtagaagaggaaagagaatagtaagaaatggcctgtaggactgactcagtgaggtaggaagatattaaagggtttcgagcaaagggatgagataatcctggaaatttggttgccttctctctctttttaatgtttttagccttgattgatcttttttttttttttttttaaataagtgttactagaaagccttgatggaccttaatctttattttgtagtgaatccatgctttagataacagggttattttctattaagaattaaaaatagctcacgcctgtaatcccagcactttgggaggcagacgcgggtgtatcattttgaggtcaggagttcgagaccagcctggcctacatggcgaaaccccatctctacaaaaaataaaaaaattagctgggcatggtggctctcttagtttttgcctgtagtcccagctatttgggaggctgagactgaaggactgcttgagcctgggaagcagaggttgcagtgagtagagattataccactgcatgtcagcctgggtgacggagtgagaccctgtctcaaaaaaaaaaaaaaagaaaagaaaagaaaaatagtagattgctgaagagtagaagtatgaccaagcatggtggctcataccagtaatcccagtacttaggga

SEQ ID NO: 19703 - RNA, 5478 nt, Homo sapiens
  source 1..5478: mol_type = other RNA
ttttgcaccttttggagtgaaaaaaatgaggtttacactgtagtataacaaaatgcctttttgtaaaggccagaagaaatggctgtgctgtgctgcctgaagcagaaaaaccttcatgtaccaggtgaatgtaaagcctttctcctcccacacacaatggactcacccagtattaccctccactaccacttttgaccctcataacagcaccctggcgggggggcagattgatgttatcaccatttaccagatgaggaaactgaggcctgatgggcagtgatttgtgcactgcgacataggactcagtgaagagcctagccagctgacggtcagctgactggtgcactctttccctcaccttctctctcaagggcacagctacactctttctccaccattattaacactcacagggcacaggtagagcgtccccagacctgtgcaatattctacacgaaaacatttggaatgtgagcaatgtctgaacaggggcttgccaggcacatctgatcaccataaatgctcccacccctgcctgtcctcacttgtgctgcactatgcaagcaagcagcaggttctcagaaggccactgtcctgcatgtcacaatgagtggccaactccttcacagaacagcaaatagcagccctggctacaaggtgcagtgtgcaacccccatatgccaaggggcagctgctatcttccagcagagagagaacccccagctctgctccctacctatgccctgcttcctgtgcctcacacagccagccttgctggcctgctggctattgtctctgactctgagctgtgctgaccaccaagtgttactcctctccaagacttgactcccaggcatgggtgggagagttgaacctcaatgcaatctgctcccactctgaagctcgtctacccaccccatttgttacaattaaagatggttttctcatccctccagagactccagtttcagactctgtctccagagctggaatgtatagggcagaggtagaaagaggcaggagagttggagaacaagagcacctagaaaagaacagaggagctcaagctcatttaatcaaaatgcttaaatgttttaattccagcattctccagagttcacagaaaagagggatgcaagcccaaaaagcaaaagcaggagcttatggtcacatgcctccagctgcaggcagtggggcctctggtactgagagggaatgccacccgaatatgccccagctgtctccacccaggaaaaggaaagccaggtacacttctcatcacagtaagactagcctaacaggggaaaacagatttacatgtttcgttcattagcatattagggaaggggaaaccttttgggctctggccccgtggttgggaaacccttcctaagagcatggagccacactctggccttgatacagtagatgggacttaacacactctgatgctcaaggccttgcagcatctgataccagaaggcacctctaaagttttgttttcaacattatttcatctattcccagatctagtccagtgatgtcagctgcacaggtagcatttaactactgggaaaacaaaagtgctacaacaacagtgagtccatggtggagtgaggataactcctgggatttggaaccagtttgctggtatcaaggatcacacaagaggctataaacctccaaccctgaaccaagtcaaacctaagcctggggatttccctcggatgaaatcaccagaacttctttcctattttcagtctcttccttcagtgagctgaggattcttttagctagctggatttcagtcaaacaatgtttttgtggtcattacttgtactgtttttctagtgcatcttttcccttttgtttgcaaaagtcaatctcaccccatgtagatgttaactgatatccacacattcgacctggtgtggataacatctctggtagtgcctcggtggtcaggaagcattaccaggaaggactcatcttcaaggaccgtttctttactgcctgctgaatatggatcataggctcagatgcccaaagcacctggggtacaggtctacatggcaacccaatgccacataggaaaagaaaacagtccatttttaagccgttcttaccgactttttttttttttttttttgagacggagtcttgctttgtcaccaggctggagtgcagtggctcgatctcggctcactgcaacctccacctcccgggttcaagagattctcctgcctcagcctcctgagtagctggggctacaggcacaagccaccgtgcccagctaatttttgtatttttagtagagatggggtttcaccatgttagccaggatggtctcgatctcttgacctcgtgatctgcccacctcagcttcccaaagtgttattgacttttaaagcttttttgttcttctcatttaaaacattttacctcccctccttaacttcccattctatttcaccatctcttcaaaattgtctcccagaaaaactgaaaattcacctgctgggtatgcagaaaattatgcagatgtgaaatcagtgtagagacaactttggagtttatgtctgagtatgctgccaatataattttcatattcagactttttagagacagggtttcactctgtcatgcaggctggggtgcagtggtgtgattatagctcatggaagcctcaaactcctggactcaagggatcctcctgcctcagactcccaaagtgctgggattacaggcatgtgccatcacatccggctaatttttttttttgtagagatgaatcttactatgttgtccaggctggtctcaaactactggcctcaaccgagtctcctgctttggccttccaaagtgctgggaatacaggcatgagccatcatgcctggcccatatccaaatattttatgtttggtcaaaaatagaaaattctattataaaaaataaagttactatggcaacattttcccaacatagttcccagtatataaacttatttttcttaaaatgataacaaggtagctcaataacaatacaataccagtgataaccaaatataattgaatttttctaaaactacattcttacattccctatccactcaactcttgtaatggttttccacttttaaaaactatcaaaataggatttttaaaaatttatcaagaccacataatgcagttgaacactcaaagtgttccatgcaactgtggttgaactattcagattccagacttctaccaagaacaatccaaagagcaaactcccaaaatgacctcctgcgtggtacaaaacaagccaggctgaaatttcgggaaacctaagggatcttatccagaaccatattttggaaaactgtgatcaatcaattttttgacagtgaaagagagtaactttccagagtatgtgttaattatatctctatcaagctttaaaaagttaacagatacttaactcttgttcataaaaaatgaggccctcaagctaattaagatgactgggaaaggtgcagaggagtaattaattttggaggcgctctgggaacaggtacacagggtacagtagtcatcatcattaaaacaacaggcactcagctctactgaaaaggctgatgacagcagcccctcccaagcggatctgtaaagtgccactgaatccatgttcattcacctactccaggttgtggtcaattgtaagtaatcctgaaattctcatttctgctcatgctgacaaacttatcatctagaagtactggttattcaattaatttttaaaatattcggatataccctgcaaataaatataaaacatctctgtacccaaacagtcccaccactataaaaggttacatataaattaaataaactcagatttcttaaccattttctcagcttaagtttgccctcaccctaaatgaagtccaatttatatccaaaatataattaaatattccaaaggtatatcgaacctaagatattgaaaaaatgtaaacaaaatttatctagcttacatttatgaaccatatttttaggtttttaattcatcctgtactgaccctctgaaaaaaaaaactaatcaagttatgtttagactgaaagctgatttggattttaaagtggttccttggagacaactctcaatgactaaaaccagtgttattgaatcaagtggtttactgtatcattcaacttaaaagaccaaaatatttcctttctctcttccaataaagctctttctggatgagcccccagatccagctgtcctaggtaaacgtgctgaactggctggagatcctgcagtaatgcttggcacagaaccaaggctgggtatcaagcaacctcatgacttccactgcaactgtttaacatccccaattcctggtttttcagtccagttggctgaaaaggatggaaactggagtgtaaagtagagaagcagaaagagaaacatagattgatcctcaaaagaaaatcaaagaatccattcatcacagtgtcatcctcatactccacagtcagactgcttctcctgaagctgccttgttagtatctgatatgaagacagaaaagccactcctatgtggaaaaggatttgccagaggttcctcagcccgtgcaggtacatgttgcccaggcaaataaagagcagcataagcaccaccttcatagtcctggctggactgtagaacaggtacaaataacactggaaaatgcaggctacgaaaggaacaagaaaagccagaatgtttccaatttcctcatgggcaacctgtaaagaatgttctgcaaggtgaactcctcgaatgagattcagggcagcacacatgatgttgagaatgagggagaggatacccagggctgtcactggttccattcggaaattaggagcaggctccaagtgcatcggtgtgtgaccattcatcaccccatttgccacatctgtgtcctccagagtgagaaccgctggaggctgcaacttgagctcctcctgaattttttccaagctgcactccatctgagaggaacttacatagttaaaatgccacttcactttctgaatgatgctgtcaaactcaagaaaagcgtatggcctggaggctaggccaatgcaggtagtgtcataggaagctgtgaattcccaccacagggtctccaggaagcagaaggccatggctgctggacactggcaggagcagatagccatgcaggccacgtccccgaaagaagaaaaatgtatactaaagtcacaaccttctgcagaacctcgacctggatactgggccagtcgcaaggctaaactcttgagccgtctcctccattccaaaaaatcttgggtgtggtaaaaatcagtagaggctgagaggggcagtccatcccttacccgtaccacgcaggcaaaaaagatcacggacatggtccacaagagaagtcatgaggacaccttcagccacaggacttgagaactggttac

SEQ ID NO: 19704 - RNA, 1314 nt, Homo sapiens
  source 1..1314: mol_type = other RNA
ttttgtgtctcccattccccaggtgcaacccatctcatcatcttggctaccagcatttatcttcctttcagaggtatccatttcctcttcttcatctgagtcttctcctagcatcttcttctccaacaatatttgctgctgcttgcgcaattccttcaactgtgttactgttaactcggattctgcctctcggtcttcctctggtccctgcaggataaagagccgggtgctgcctccaaagcgaacaacatgcccaacgtggactcgacagtaggtgcgaggtgggatgcgagttttgttgagaaaagtgccatgggtgcttcccagatcgtagaggtagaagcccggcccgttgctgtcgcattctccgtcagggccggacgccctgtgctgcagcactgcgtggtaccgagacaccgaagggtgctccaggcacacgtcgcagccagacagcctcccgaaaaggcagtaactcgtccctttcaagctacgggtgccaaggatagtgccgcccttcagggtctctaagctgtagggggctgtggcagggccaccccatggaggctcttggtaggggggagcccgggctggaccgccaggggaagaaaccgctgtcggggggcgcgactgctcctcctgtagactcctaaaatcaccgcagtccggctgaggaggagggatgtcgggctccccagaattggagtcctgcaacgcagtgggcccttccttctgtacctcctcagggtttgaagaactgctggccggggccttactccgcgccgctggggacaccggcagagctggcttcttgaagtccccactgaggtcttgcgacgccagggtctctgactgagagagaatgtcagccatcctcaaccggtgcaacttcgaaatccgctccttcgaaacccacccttcggtctttacgttcctgtccacgtcccactctcccaagctcccagtggcgtctgtaggcggcgatggtgaagttgctccttcacgacctggagcgttgcgaagtggtgctaacatgagaaggtcataatatgagaaaaacaaaacggttatcgggatgctgtgcagaacggggacatatttagaggttacaacgggatcgtaatgacttcctgttgcatagcttgattgagaagaagcgcttccggcggtcttagatcactaatcaacaaaccagctttcggggtctgacgcgatccttgcctcaggcctctcgaggtccagacagccgcccagcccgctctgcgacgcagcagtgaatagtgtggtacctccttgtctcggttcaggtccagacct

SEQ ID NO: 19705 - RNA, 4880 nt, Homo sapiens
  source 1..4880: mol_type = other RNA
ttttttgctggaacatttctggaactgggcctcttccacctaacaggctctcattataccctaaaggccctctggaacccacctgagatgggtgctgcagacaggccccacatatacacagttctcaggggcagggcagtatctaggttcttctgtactgacccttcctatggtcctatggagccaaagatcgctttaggtgctgtatcagtaaaaggggcatctgttaagactccccagctagaattcatgctaaaatccccatactaacatcctcagagtagaagaggaggaagaatcagccacccttcctcaatacccagtgggaagaggggtgggtatacacatggttattgaggtcatgtttcatcagcacagcaaaaagaaccaggaaaaaacaaagaaaccaccacagacctgggggtggggagccacagagtgccgcaagtccaagtcggtatctggaaggaaggagtctactcagttcttcctgctctaacttgggttcaaacctcccacctacatcctcatctccagaacaagacacatggatgccagtcaccttaaaaactaggtttctatttctggttagattctagagcagtggaactcaggagtgatactataccctacccagtcccaccacagcctgcctccttcctcccacagagataacattgtacaaaactgtatttacaagaaaaccaattaaaaattaagggtgtgtgcaaaagtagacaggagagtcaagacatatcaatgcagggatggctttggggaatgggggactcaggttctacactggaacctggggtcatgtatcatgtaccaggtggggagaagtgtagcaaatctcagtgccaatttgaggggaagccagtcattccaggagaagagctgaggggaaagagctgttgactttcataatgcagtcttaattatccagtcaccctcctgccacatggcagaagccaggtggcagtgatggtggtgggggaaacaaaacacacagtctctggcaagccccaccgggaaaggagggctcagaaggcgtagcgggtccggatatcctcgagtttcttggacacttcgggtggggttcggtccagttcttcagagacgttcttttgtttgttgggttccatggaattgaactgctcacagaggtctccatcaatcacattcttcacagggaagtagtaggagcgaaagctgaggtggtcccgcccacagagagggggatgttcagaccgcaggtgcatttccacatgctggaagaagtcatggtcctcatgggacgtgaatggcacaaggatgccaattcctccagacaaggtggtatagacaagtgattctgagcctccagggatcagcgtggtcttctgcaaggacagcaccgtctccccgacatggtagttcatgatcacctctgccttctgggaggccccattgagcaagccacggtcccacagggctttgtttcctgtaggatcctcatctacttcatcattggtgttaggtgggagcctcaccacacatatgttgccaaacttgtctgccccagccacagtgtcatagtccaggaggctggctgtagtgacccatcgggggtaggtatcatcagcaaagatgataagctggttttcattacgcttgtagcgaacccagatgaaactttcttggacatcagatacaattaccctatgtccgatagtctggatcccagagatataattggcaatatgcttattctcacattttcggagtaacttcttctttcccaggtcatagacacgcaacagcttccccacaccaatcaacaccctcccctggaatggggcaatagcagcagggacctcttccacaggagtcttgtgcaaaaactccagtttttccccattgttcacaagcttgtaagtatagacgaagccccctgccacagatcgggggtttagtatcaggtccttggccacacccaccagcacataccagtcttcaccagtgttggaaaacctgcacacagccacactaaaagctgcctcattctgttccagctggacaaggtccagtgtgttcccttgaatgggattcatcactcggatcacagaggcccactgcccattgccagccttgggagctccaaagatggattcagggaggttttcattgaggaatgctgctgccatctctgcggccagctcccgctcatcctcccctgctgcttccaccatttcctctgccatctgctgctttctctgagctttcgtggcctcagtgtaggcattgtggtccgtttcaatgataataaggttgttactctcagggtggatgacaaatttcctgggtgtgtactgcagtgggaaggctacttgattgaagacagcaccgagcttctctaatgccaaaatccgtagggtgttggtggagatggccacaatgccctcgggacactgttccgaggcaaaacccgatgcaaattccagtgtctcgtaagacagtggggtgagatggaagcgagattggtaagaatagctcaaccatgagcggcttgacatggccaatactgcctcctggccttgcattcggactcggaagagcttcacaggacgggaccccaggtaccgagtgcgagtatcagacaaatccccagtgacagggtccaagacagtcctcagcagcacaccgttctgtagcccaatattcaggtataggaagccaatcgagcccctctcacccagctcatcctgcttctcagtcccacccatttccacgatacacaaggactcaggctgggctgggagagcctgcatgcttagaggttgcaaacagtctgagggatccagggagatgattctgacagtgttgtccacaagccccacagccaggaagcgagaccgctgctctccagggggtacattggccagactcatgcacaccacatctgctgacatctccttccgttctgtgtactcattcagctgtcctgaaggatccatctcgaaatagaccagctctcctcctgtcagggcaatcaccacttgtcgctggttcactgcacacttcacaattgttttctttccaggggtcttccactcattgactctcttgtctgctcgtatgtgccgaatgccatctggatagacctgcaccaaggcatcatctcctaataaggagcaggacaaggtcggggtggtccccaggaacccagagtcagtcacttcttctacagtttctccaatggacaacactagggtggcattcacgaaagacacaatgatgtaggcatcaaactcatcttcaatgtgtcgacgcactgtccagacagcgttggggttaccaggtagctcagaaacagccatttctgacacctcaagtccatgtcttaggactctcagagatgatcggggtcccctaccacaggccacatacaactgtggagtatcttcattggccagatcagctatctggcaaaacagaatgggagagaggctgtccaactcatcaaccagcacaaggtttttaagtggtcttggctgaaaaaagaatgtgtctccttcttccagaggcatggctgatgaaaactcaggttcttcatcatcatctccaagatgtgcaatttgatataagtaatggtttccaaattctgatgctacaaaaaggaaccctgttttaagcacacacatggcagcagcaacgggtacagtatcaaaatatttgagccggatctcagtaaccatatcttcatctgtctccaaagtgatcttaaagatatctccctgctcagtttgagccaaaaagaagaacatcgatttggttttatgggttgcagagcagacaaaaatcattcctctttcagggtcatccaggtcattccgcctcctgggaattggacagcggatatctggctggtcaccaaagttcttgtaagtaatatagttttcagagcagatcagtactccacttggaccatctgaccctcctggaactgtaataaggaagttgccgtgttcctccaaaggttcactgtattttcggaccacatgatttaaaccaaggtctagctcatagaaagtaagtgtctgctgggtattagctgctgcttcccctgttggatcattgtctgcttcctcataatccatttccagacaagcaaacattggattttcaaatccgacatctactccaactacatgatacactaaagtgtttgctttgtgggcttccaggggagatgaaatggtaagtcgggctgcagcatctctgttcaaaatatacaccaatttctgtttctcaatggcactaatcataacggctcgccctttgggatccacagctaagaactggccaggaacgatgcgacggcatccactcttgccaaaggtttcttggtgaatcttctcaaacatattcttagatggctggtattccaaaataacaattcgaccagagtcactgccaactacaatgtagtctttggtgccacctgtcagcctaaaggccatgagtgaccggataacaccgaatacttccacagtgagtagggtatgtactttgccagtgttggggtctgggcgaagcagctccaagatcttcccacgggaaacaacaatttcttgttgtttggttccagaaaagtttccatgaatggcaaagctgatgccagtggctctctgcaaggttaagttgtacagaaacatggctgcaggaaacctgagccacccagacctccaggccttggttacaccaacagtacggagtccaagaaagcctgcagcgagaaggatggtgtggatatccaacggatgctacctcccttcaaaacttaagccaccaccaactccaacatactggcgtccgccattagacctcaagacagggac

SEQ ID NO: 19706 - RNA, 12424 nt, Homo sapiens
  source 1..12424: mol_type = other RNA
ttttttgctggaacatttctggcctccttctaactgggaccaccactaaaccgactggtcccaactacccagagggcacctggtatacactgaatgcaatgtcctagccagtcagtgcccagcctggtggggacaaggtccccagggcaggctgggccggaaggcacggccatccctgcttatcctataggcaggcagagctgggacgggcaagcacaggctcagacttccccaaggtcactcggcaaagcctcactagcacagaggctctgtctacactccagcccacggccccttgccaggagcacactccctccgcagcaggaacacgctcctcagcgctgttcccgggagacctaaaaaggagcgactctgatcttgcagggactcagaaaacctggcaacgtctgccttccttctccagaagggctcatgcctcctgcctcgggggacagcgggcaacttgtcgtccagctccttggcccaagctcggcctgagttgtgcatcctggacttggaaacctagctcaactatttttagtccattctgtctgttcctgagctagtgtggggaaaggtgaggtggtgttctgttgcagactttactgttctaataaaaaggagggagcccagcgggagggatccagaccagtgggctctgggtgagcagctccgaagggctgttccctggctgctctgttctgagatgaaaccctgccaggaacacagagctgatatcccctcaatggctcactcaagtttacaggggaggtatggctggttttctgtagtgcaggaggggcccctgaagtctgtgatgcaggctaggctaggatccaatatgtaggggcactgggtgagcaccaatttccctggcaggctttgtcgggggctgtggcccatggtcccatgtagacagtcctaagccaggtgcttcaaaaagctgctctgtgtctatctggcagctcttggtgtggctggaactctacattcagtgctaattcctggctgttgccatgctgggaagaacaccatcaaacaggccggctgccggctgggaaccaccagagggagcctggacctgcgatcagagctgggactcactcactgtcctgggaacctggggtctggagtgtctggaggacacggcacctgctcagagccagggagcaaccctggcccacggaggcctccacgggcccttcctaaacttgggcccctcctaaacttgggccccagtgaccagtgtgcagacggctcctagacctccagacaaactgatgggtgccagtctttcaaggccatgctgtcggacgccactcactgcagacaactgggctggggcagagacctccccacactctggacagccctgcccgtccttaggtggctccttagtccacctctccagagcctcggcctcgattgggccctgcccctcacttgcccaccatgcagatggcacccaaagacagcccccacctggccccctgccactcgctctgtgccaggaaaagcacccccacctcctgtccataaggcagcaacgggagaacaaaggaaactttcaggaggctgccaattgacgccaggcccacctcggtctccctgtggggcttccatccccagccaggcccaggaagaggcggcgccaaggccctggactgctcagtggtgctggggcgggggcttggcagcctcatcccagctgttgggggatccgctgctttcttcccagaatgtaaaagtggcagcacacaggacgacaggagggccggctcttggacttggcatctcctgcttttgtgcagccgacatcagctgaagccccccaggcgcaagtggaggctccctccccactccagccatggcacaaaaacagcctgctcttgggtcaacggccctgccctctgggtagcccgagcacctgccccatccagaccctcagcctgtggccaagaagacatctcaaccaagaaggattcaaactgagggtgtgtgcctgggacagggggactaaaaagtggtcagcccctgagcaatccccacattcgcttttcacctcacagggctcaatactgcccaggagcccacgggacagctggggcagcccacctcccatcatgggtgccctggcggcttcacctcagtcccccacaacttcccgcgcaccctcaggtgggtcagcccccgccatggtcagcactggctcccttttctggcacaggagaaaaatgggcatccagggacaaaaccccttttaaggtgtctacgtattgaacaaccatgttcttgagccaaaaactgtccacaaagcatgcattgggaagcaggatctgccttggctctgcccagggagacctggggctgttttcatgttgccttgagctaaatgaccccacattgcactaggccccattgcacacaggcctgctccacagacagcccacagtggtacgcagcactgaccaccctggctgcagaggtcagggcctggtgggcgcagtgcagggtgggggccctcctctctggatgccctccaccccgaggcctcctgaacacctgctgcaaagagcctcgctgagcatgcactctctccccaccgggagggatgaaagcattccacggtgggagaaggcctagaaggcatcgtgcagtgacaccggagggtccctgagccaaacatgctgcagccaacagccaatgtggagaaaacccaaagagataccagcgtgcagagagaaaggcccacagggtgccagaacatgcccggtcaggtgggaagatccagaaggaccccagcttctgacaagcagaaccaacagaaccacgaccagaggtgccatctcagcatctgcacctgaccctcctccctggctccaaggccaacatcccttagaatgcactgggccaggtgtggtggctcccacctgtaatcccagcactttgggaggccaacgtgggtggactgcttgagcccaggaggtctagaccagcctaggcaacatggtgagaccctgtctctactaaaaatacaaaaaagtagctgggtgtggtggtgcagacctgtggtcccagctacttgggaggctgaggtgggaagattgcttgagtcagggaagcggaggttgcagtgagctgagatcttgccgctgcactccagtctgggtaacagagccagactttgtctcaaaaaaaaaaagggagactgctctggggcactgggtcatgtgagctccccacagcaactgctgaccacaagggggcatctgcaagctgggtgagaagtctatgccaaggggcccagctcacaggggttctaagcagggccttgcactccctaggggtctgtccacctgctgctcccagcctccactgctttattccctgtcctgcaccttgagtcagctcgggcctctggaggtgcctgctgcactgccctgctctatccctgggcacagccacctgggcacccgcagcccatcctctggcctggcctcaacccaccctgcctggggccgtttcatcttctctgaccttcacagaggccaggatccttctatatttcaaaatttaacacattttgttttcctggaactgtttctcttccaggaagtgggagtgccccacaccagggcagtgagctgaaagctctccccaggccctagggagcaaaggctgggctggctgcgccggctgccccccactagccgcaccttggcatccaccctgctcctcctctacttgcagcgcgacccccgacccctcggtgtcttccatacaccgacctcagcgtcttcctagcccatctgctcacactacccctgcctgcaaccctccctcctggcctccaagcctggcgcaatcccacagcttccgcccaagtcctcagcctctcagcgctcacagggctgcgcccacccctgcagtctttcccctggaggtgcttggtctcctcacagaccccacagctctcccttctcttttgggctgccctgggggtttacccatgagcagcagatgtgccagtggatggctcaacaagaagtccagcctccacagcccaggggcacagaggcaggaggggccagtcccagccacatcccaggagagtggcagagacttcggaggcctggagctgatccagacagggcttgagaggcgcccagggcagaggcccacctgggctctccccggccagcaacttcagagtgtgggggaactgggggagacattatggcccaaaaagactaagactaagacttgcctgatgggggctaagccgtgaaaacaagcaataccacaaaacacagcatgggggtggaagtggggcctgggtaggcgccatacctgacactaacaccctgcactgagtctcccaggtgccctcgcccccagtgacagccccagatcgagccgcacatgcaggagccggaagaggagcagcaagtgaggcacaaggccagcagggccgggaaccggctgcggagaaggaaccacagccggctgccataagaggacccagagacgcaggggtgggggggaaggcgcccactcctccccagattcaactcagcaactcaccagacaccaggccacccagacccccagaccaacagcccagatgacatggtggccgaaacagggcagcctgttaaacaggcgaacgggaagccctgggaaggccctggcattcctacatggcccttgtgtcctcgaattgcctgcccggagaatgatgacccacatggacctctgatggggtgggtggatggcagtggacgcctcccacaggcatggcctctggctcccaacaagcacaatgtatctttattgtacaagcaaaaagtcacgtgccccaaaccagcatatccaatccaattgttgaaaaagcttaattttcctgttaaaaagacaaaagcctaaaaatctcacagcttttggttcactggccgatcgtcctgagggttaaaaacaaactgcgtgctttgggatggccccaagcaggcagagccttccctggagatggagttcctgggcactaactgtgttccaggggatctgagcaaggctgggactgggttttggcttagtagcaattggaggaactgcgtcattgacttcatccctgcggtcatgggaggtcacaggaaaatacagcaagtaaagtgctcccactggctggaggaggaggaggagccggccaagcaggatgcatgctccaaagaagagctgcccaggtggccgtcactctcctatttggggttggagacagcagtgggtgaggagcaatgacaaaggggaccagacctgcccttccagtggggaggggctggggaggcccgaactggagcacgttctctcagcatttccacatgcagggcacagggcggtgggtgtgcagggtactgggtgctgggatttggccctggtacagaaaccacgccctccagtgacctttagaaccgtataggctcgctatgtgcatgtcttcacagtccagacacgcgtgacacacactgtgcatctggaggaggttggggttgtctttttgttgtcgctggaactggggacagcggacatgtatatttgccacaattgcaacagaaaaaaaaactacatccaacataaaaaaaaaaattaaataaatgaggtgacgaaaagaatgcaaagggctccagtccttctgggcagaggtgcccggggcggaaggcaggccagccgctgcacatgctttccgtgcccaggcaccagccatgagcatgcacacacgctgtgtggggcttgggggtaggcgctggcggccgccgctccaggggaccggctcatggggttccactttgatattaaataggtgacttcgatggggtgggggaggcatcctatgaaatgtatgaaaggtaatgaagacagggagggggtggggggagaaaaccaagggccaggaggtgataaaatacaaaagaacaaatacagacagatggacacagatacgggtccactgaggaatcgagcacgaggtttgctactagacttataggtcactctctcagacgttgggtggtaaaccgtccagccttggccacgcgctccgcctccatcactggctaagccggagcagatgtccgaagacagggaggcccggacggagcagggctgctgggtctgcactgccttcccgctcaggcccgtgctgtctgcagtgagccccacactggcttgggcagggtccttagcgggagggcctctgctggagtcagccaagtgacctgtgctggaggccacgaccttgagctgccgcaccaggggatttagcagcttgcctgccttcagcttgctcttgctggtttttctccggcggccagtggggggtgccgtgtggaagaagcccacgttggggggcagtggcttgcccaggcggcggtacagagcttcgatctcctgcttctgctggctctgcagctccgagatctccttcaggtgcttctcccgcagactctgcagctccttctttatgtcagcatcctcgagctccgaatcattgtcgctgctgatgtaggacgactgggaatggaaggaggtcacgctgatcgtggggaccttcatgcccaccctgctgggtgtctcggggcccagcgagccggcccgagaaggcctctgcaggaaggcggtggccttcttcacgaagtcgccagccacgctgccactcacgggcagggacgcctgcttctgcaccgggggtctcgcccgagggccctcgtccccagagtcgctggacacgggctcgcccacgccgacctcgatggaggaggccgtctgcgcccgccgcactgccagcttcacgtcggggctggagggggcctcgtccaggtagacgtcgggtggggcagagtatctcaggctgtggggggaggccagggtccactcgtcctgagtgctgaccaccgagaaacggcccacagtcttggctggtgagctgacatcctgctgctctggacgtttccgaggggaccccaaagctcgagcgccgagtgtctgggggtggctagcctggccccccactgtgcccatgtcactcggcgggggctctgccgagctttctccagcttctccaccatccctgtctgtgggctccacacgtgcaggtctcacaaaagcaggtacatcctgggggacgctggggaccacatgggagtctgaggccacctgccttccatctctgtcatagcctagcatactcctgggagacgactctgctgtcattgacgaggacgtgccctgctccatcacggcccctcgagtgggggccagttctgacttctccaccaagggctggggcagctggacacgccctgagaccgcctccttaggcactgggggcagggccaggtcccccccgcagacctctgagcggggctggtcccctctcaggggctccagggtgaagtctctgtcgcccacctccacaggggtcccagctgaggctgaggaggtgggcacgtgctcctggtagagcagagtccgcagcttctcgtccaggctcttgatggtgctgtccacaaagcccaccctggggggcggcccttccccatccgactccagggccgagggtggctgtggggggacggtgggccccaggggtgggcttgggagctgggaggtggccaggctgacggcccccactgcggcaggaagcaggggagcaggttgacccaaggcgggctgtggggtcccgctgtgggggctgggctcaggtgcaggaggtggcaggggctcccttggggcactggcgtccctggttgaggcagcctctggagctggagtgcaaggtgctaggcccaccacgaggggctgcacagcaagcggggcctcgtgagtctccgctagtggctgagacgtctcgagctcactggtcagcccctgaggtgtccctggaccccctgcctggctggcagttcctgacgctggctctggcatggtgctggtggctggagctgctccatcttggggcagagcagtcacaggaggggaggagggggccaaaggggctgggggtgccccaggagggttgctggggcccgcctggctcaggagctgctgactggctagaaagctgggttgttccttcgaggacagctggtctttatagggcgctgaatcttggctggcttctggcggcagggagcttagaggaagtgggggcgaagattcaggggcctcgggggcggggtgctcagccaccggacagatgatgaaccacctcttcccggtgtgcaggacgttctgctgatacacgggggcgttggcttgggattgtcggctctcctccccggtgcccaggccgcaggtgctgaggtgtggcgggctggtccctgggtcggagccacggtcggcgtctgtgtcctcgctgagcatgtcctctgccttgtccatgacatccttcatctgctcgatgaacgtttcccgctcggcctgcaggataaagtcatgctccaccatatacgtggcaatttcatcgggtgcgtccccgtccaagtcgaacttgaaggtcaccatcttgtggttgtgcgtctccagctggcactccaccatcttgtccccagtgttgcacacgttcaagatggtaagccggggccggctggccctctcctgccgggagcgcgcacgcgtggacctgcggtggtgttttcgggctgccctgccctccagcctgccccctccaaaggcgccttcacagctgtcactcagctcttttccagaagtgacatcagaacctccatagctctcacagctctgcgggaggccgggcggcttgtcctgtgaggcctgctcctcttggactggttccaccgtcagctggacagttgggcaagggctggcgatcccgggcccgccaggcagcggtgggtttgctggtggcagaagtgtggcagtctgggtgggcacactctgcacagaggcagacaccgtggccagggagctggggaactgaggcaggagctcaggggcggcaggcagcagcacttccggcagaggcggcgagaggaccgcagccggtggcacaggcacggtggggacctgagcggcgacgtccacagcatagggagctgggtggccaagcagaatctggctccctggtgtagcagctggagcagcttgttcaggaaggtggggctggaggggctcagggcgcacaggcagtgccggctgcgggggcagcacaggttgtgggggcagcatgggttgcgggggcagcacaggttgagggggccgtgtgggttgcgggggcaacacaggttgagggggcagcgtgggttgcgggggcagcacgggttgtgggggcagtgtgggttgtggaggcagtgccggctgtggaggggtggccctcatattctgcaccgtgtgatggggggaaggagggacgtcagtaggcgccatctgtgggaaggccgctgggtacacaggttggcctgggagctgggccacggcagaatgaatggacagggcagccacgcccggtggggctacggccagcagggggatagtggccggtgcatttggcacaatggtccggcagggcatggccaggggcgccccaggggggtggggcagcttcacagcctgcagaggcaaggctggggacgcaggggggagtggggcagcgaggctcggcaagatcacggctggagagaaatactgaggtggtggcacgggaggcacagtcgcggtcggcaggtctgggagggccggagggaggccgtcgattcccgccaggggcgtgatggggggcacaacaggaatcgggggcatctgcggagggacttgagcaagcggctgcaggggcgcctgtggcatctggaggggcttcagctgagcgggggcccccacctgggaggctggagccaggtacggtggcaggtgggggggaaccggctggagggggaccacgggctgtggggccaggacctgcggcaggggtgtcggctgggccagcggaggaggctgctggccggggggtgctggctggcctgggcccgtgggcatgggggtgctgggcggcggcagcacgggggcgaagctcatggccggatccgggaagtgctgctggagggacggagggcaggcgggggccgggacagagcccaccggcaagccaggtgcagccgtgggctgctggtaggcccccagcgagggcaggctctgcggcaggacgggcccctcgctcacaggggggctgcacacacactgggccggggacggcgctgcgtcggcaagggagccaagcatcacgctctgctggctgctctgcgagtctgagtacacggtagagccctggccgctgtcgaaggtgctgtccgaggccagggaggtggcgctggtcggcaacgtaggtggcaggaggtgctggtcggcctccggctcctcgggctctggtggcccgggctgcccagcctgtgcatggtaggtcacctggacctgcaggggcaccggcggacccctggccttgtccgggctgcccacatcctgctgctccttgggctgcagcgcgggccagatcctctcccgccgccactggatcaaggccacgcggtcacggatggacttggccacgatcttgacgtcactctcgtggaagaatccagactcaatcatctcttgggccacctcatccggcgtctccttctccaggtcgaaggtgaactctatggctccattgtccttgggctttcccttcagtttcttggggtcttccacccagagcctcagggcgatggtggacttcctgccgtggtcctcctccgcgagctccaccctcacgcctgtgtcctctgcgaagaaggcgtggctcagcaggtctttgatctcgtacctttcctccttgtttttgcagatacactccccaataatctccttgatttcaggatcgtgcactttctcaaagctggccggcttgataccacaggtgaccttgcggtagatctgggccgcattctggcactccgagtaggggtactccgaggtggccatctccagcatgcacatcccaaaggcatagacgtccacggactcatcgtagtgctcctcgtacatctcgggcgccatgaactcgggagtacctatcacacttttggcaaatgacgctcttttcagagtggccaggcccaagtcgccaatcttcacagacccagttggtccggtgatgaaaatattgtcacatttcaggtctcggtggatgatgggtggcgtccttgtgtgcaggaacagcaggcccttcaggatctgccggcaccagctgcggagaaccttgggcttcatcaccttgaaccgcttcaggtatgtcttcagcgtccctgaggtcatcagctccgtcaccagcacaatgcaccgcttgcccttggcgctggactcccagaagtcgtagaagcgcacgatgttggggtgctgcaggcctttcagcatctcagcctcttccttgaaccgctgccgctccagcttggtgagcttccggtcctgcagctcacaccaggccacctccacccaggtctccgtgtccagccccttgtagaccgtcttgaaggaaccgcggcccagctcgatgtcgaacttgaggaagcggccgtccagagaggtggccacggccttgaggtcgtcctcgtcgtcctcctcctcttcgggctcgtcccggcgagtgcgcccgggctcaggcttcgcctcggccgccccctcatcctccttcctcacggtcgccgccgcctcctccctggggccgccgtcgggggcaggcgcggtttcgacagcggctgcgatggggtccgggccgggctcctgcgtgcccacgggctcggggccggcgtccgcgggggctccgggggctcccggctgcgctaccagcgctgcgggcgcgggggcggcggggcgtccgcgggcgcgctccgcgatgaggcggcgcgtcttgcagagcagaagcacccggcgctgcaggggctgcgggggctgcgggcccggcgcctcggctgcctccaagcccggcggctcctcctggtccgactctaccacgctgcgccgcagaaagcgctggggccccggccgcgccgccttcgcccgaggctccgccatgcccgcgggccccgcgccgcgcccgggctccatcagcgtgccggggacgtctcggcggccgccatcgccgtccatctagggcgagcggacgccgtccatgcccgcggcccggcggccagggcgtgcgaggcgggagagatcacgcttcgaggacggggtccgagttccgggcgaggtccgcgctggggtgggggccgtggcgccgctccagctcctgcgcgctgctctctcgggccgggccactgcggggccgcgctcccgcgtgctcctgccggcttcgcgcggctccgctcccgcaccggctccg

SEQ ID NO: 19707 - RNA, 3802 nt, Homo sapiens
  source 1..3802: mol_type = other RNA
ttttttgctggaacatttctgggaacttgacgggattgcctcctagaaatgtcatggggccatccacagagagccgccgaccccgtcgtgcaggggtgctattccacatgtgagtgcccatgtgtaccttaagattgcctttagtcgtgaaagctcttccacaaatagtgcaagcaaagggtttctctccagtgtgagttctctcgtgaatctgcagggcactcgatgaggagaaggttttgccacatgtgttgcagtagtgctgcttgggagttctcctgggcagagcagggagcagaactggggatgtggcagaggaagacagaggcccagacgggacgtgactggtgggggtgtccttactgtcctgaggagaaacatgcacgaagccgttgacctctgtcttgatgagagatgacaacgagttggcgggaatcaccgctgagttctgattggggccaaggttggaactgggctcaaagagctgggatggcagatctcgcatctgatgtgtcaacatgtgctgcttcaaattaccctttgtggaaaagccacgattgcaaactgtgcaaataaatggtctctctttggtatgacttctatagtgaatgtccaaggcactctgacaagcaaatgttttgccacaaatgtcacaagcagtgtttttaaatttaccccggtctctaaaagggaagaggatccccaaagaatcttctttgatgattttctctgcgtgactagatgtcaaatccaaagccccaccattcactggggtgggagacaaaccattggcaaactcgcttgggaccgctctctgtggtttctcctcaatgctgggtgacttgtggaactcctgcgtgctgttggacggggacagagcctgcatggaagaggtagactctgagatggctgggctgccagcactttggctttccatgtcaccacccactgaggatgaatcattggtcaggacatccccctcgatggacccattctccactgacttcaggctggcctgtagctgctctgccaggccagcattgatcatcttcatctgattttccaaagcagcgatgctcgacatctcgaggggcaaaggcgaagaggataagctgtcttgggaggcgtctgcagacttaggtgtatcagggatgctgccctcaggacagtcttccatgttttcatcagagaagttgtctaggtcatcaaaatttttctcatcaaaggaacctgtgtcagactccatggactcagagtagctgtcggggactggggtgttggggatctggcctcccatatgcattcggatgtgctgctgcaggaccacagcgttcgtgaacttcttctggcagatggggcaggaatgctggactctgagcgggggcatagcacgatggacactgtagtgggttttaagattccctttcgtggtgaaagcccggccacagatcttacacttaaagggcctctccccagtgtgtgtcctgtagtgcattttcaaggcgctctggcagctgagaacccggtggcagatgatgcactcattggggtcagtggccttcttgtcaatgttttctaccagttgctgaagcttggacgtctctgatgcctgagctgagtccaggagtcccccaaaaggaaacttggccttgaactgctcggacatgagcggcaacaaagggttggtgaaggtggtggcactgcccgcggggccgcagtctgccgctggggagctcaggacgctactgctcgccgtcgggactgagttggtgaccatgccactctcttcgcttttgccaccagagggtggcagagtggacccttcggcttcctctgggagcccacctaggtttcttgtggctgactcagggcccccggagtcacttttgactgagcctggggggctggtggcagaatggctgatggggatgggggctggctcttccgtcttgatgaagggtatgaggcttgggagggttgggggcaacggcaggccgactgaagtggtcagagtaggcaggactggtttggtgtctagccagctggtgactggcttctctggagggatggacatgccatatgggatgccagtactcgtggggatattgtccaaatgctcaggcacaggataggggttcatctggatatgagggtatttctctttgtggcgctgaaagtggactttcagattccccttggtggagaacctgttcccgcagatgttgcacttgaatggcctctctccggtatgggaacgcaagtggatctgcaaggcactgtcactcccaaagaccttcgcgcagaacctgcacttgtgtttgaagaatgcctcatcggaagtacttttcgcttcaaaggcagtgacatttggtggcttgctttttctttgctgggccaaggcagacaaggagtttaaatcctctgcagttgttccgatgttgggcaaagggctggggaaaaccgagttagcggaggcttgctgaggtagaagtggattagacgcaggacttaataaactgcttattgcaaaagctggtgaggacgatgatgagaccgctgggttgctgacatgggaggccccagcacttgaagccactttttcagaggacggggtggtaactgccgctgccaatatgttcatattgggagaagagccgctgttggatggaatgatggtgttgccagaactgctctgaggtagctggattgggggtagctgtttcacaccactaatgctggcagattggctggcgaggctctgtgccaatccagctgctgctgccagctgctgagataaatgggaacttagcgtggacaaggggttggcagatgttcgtaaagtaccttgagaaggactagaagatgttggcaagtctgcattctgagaagccaacagcaatatttggtgacgaatctgttcgatcaattgcagctggtggatctgctgctgctgcagagctaggagttgttccatgagggctgggacggccagcttgcccccagaggccccgccgcacctcgcttcctgggagaactgggccaccgccaccttggtgctctggaggttctcgatgatgacgttgctgttgattacggagaagttgcccagtgttgtcaggtccccgagttgaggtagagaggttgtgatcgctgaggtacctgtggaggagctgccgccgccgccgctgctgctgctgctgctgctgctgctgcttggggcggtactgctgtggctgccgctggaagtgccgctgccgcttttgttagcaaccggggcctccacctccatggactcttccctgtcaagtccgttgtgttctgaaaggtcgctgcagtccacttgatctgttttgttaactgtgtcattcatttgttcatcaggattatcaggaggggggctgggggagaaggtttcgggtggggaggctggattttcatttacgattaaaactaattgatttttagtacagttcttcttgtggagcagaagatctgataattcaaagaactcggcacagcaccggccacagacgtgggcatccttgctcttagtagggcgactcggttgacccttttctgtgtctccagaaagattttggggggcagagggtgcaagtgttgtgggaagagatgcggagataaattttgcgagccagaccccgacactttccccgtccgtttgcaccgtctccggaacaactggcggccagcagcactctccaccccggccgcaaccccagcgggtcaggcgctggcgccccgacaccagtccccatcttcttgcagctctgaacctccaaag

SEQ ID NO: 19708 - RNA, 3690 nt, Homo sapiens
  source 1..3690: mol_type = other RNA
ttttttgctggaacatttctgggaacttgacgggattgcctcctagaaatgtcatggggccatccacagagagccgccgaccccgtcgtgcaggggtgctattccacatgtgagtgcccatgtgtaccttaagattgcctttagtcgtgaaagctcttccacaaatagtgcaagcaaagggtttctctccagtgtgagttctctcgtgaatctgcagggcactcgatgaggagaaggttttgccacatgtgttgcagtagtgctgcttgggagttctcctgggcagagcagggagcagaactggggatgtggcagaggaagacagaggcccagacgggacgtgactggtgggggtgtccttactgtcctgaggagaaacatgcacgaagccgttgacctctgtcttgatgagagatgacaacgagttggcgggaatcaccgctgagttctgattggggccaaggttggaactgggctcaaagagctgggatggcagatctcgcatctgatgtgtcaacatgtgctgcttcaaattaccctttgtggaaaagccacgattgcaaactgtgcaaataaatggtctctctttggtatgacttctatagtgaatgtccaaggcactctgacaagcaaatgttttgccacaaatgtcacaagcagtgtttttaaatttaccccggtctctaaaagggaagaggatccccaaagaatcttctttgatgattttctctgcgtgactagatgtcaaatccaaagccccaccattcactggggtgggagacaaaccattggcaaactcgcttgggaccgctctctgtggtttctcctcaatgctgggtgacttgtggaactcctgcgtgctgttggacggggacagagcctgcatggaagaggtagactctgagatggctgggctgccagcactttggctttccatgtcaccacccactgaggatgaatcattggtcaggacatccccctcgatggacccattctccactgacttcaggctggcctgtagctgctctgccaggccagcattgatcatcttcatctgattttccaaagcagcgatgctcgacatctcgaggggcaaaggcgaagaggataagctgtcttgggaggcgtctgcagacttaggtgtatcagggatgctgccctcaggacagtcttccatgttttcatcagagaagttgtctaggtcatcaaaatttttctcatcaaaggaacctgtgtcagactccatggactcagagtagctgtcggggactggggtgttggggatctggcctcccatatgcattcggatgtgctgctgcaggaccacagcgttcgtgaacttcttctggcagatggggcaggaatgctggactctgagcgggggcatagcacgatggacactgtagtgggttttaagattccctttcgtggtgaaagcccggccacagatcttacacttaaagggcctctccccagtgtgtgtcctgtagtgcattttcaaggcgctctggcagctgagaacccggtggcagatgatgcactcattggggtcagtggccttcttgtcaatgttttctaccagttgctgaagcttggacgtctctgatgcctgagctgagtccaggagtcccccaaaaggaaacttggccttgaactgctcggacatgagcggcaacaaagggttggtgaaggtggtggcactgcccgcggggccgcagtctgccgctggggagctcaggacgctactgctcgccgtcgggactgagttggtgaccatgccactctcttcgcttttgccaccagagggtggcagagtggacccttcggcttcctctgggagcccacctaggtttcttgtggctgactcagggcccccggagtcacttttgactgagcctggggggctggtggcagaatggctgatggggatgggggctggctcttccgtcttgatgaagggtatgaggcttgggagggttgggggcaacggcaggccgactgaagtggtcagagtaggcaggactggtttggtgtctagccagctggtgactggcttctctggagggatggacatgccatatgggatgccagtactcgtggggatattgtccaaatgctcaggcacaggataggggttcatctggatatgagggtatttctctttgtggcgctgaaagtggactttcagattccccttggtggagaacctgttcccgcagatgttgcacttgaatggcctctctccggtatgggaacgcaagtggatctgcaaggcactgtcactcccaaagaccttcgcgcagaacctgcacttgtgtttgaagaatgcctcatcggaagtacttttcgcttcaaaggcagtgacatttggtggcttgctttttctttgctgggccaaggcagacaaggagtttaaatcctctgcagttgttccgatgttgggcaaagggctggggaaaaccgagttagcggaggcttgctgaggtagaagtggattagacgcaggacttaataaactgcttattgcaaaagctggtgaggacgatgatgagaccgctgggttgctgacatgggaggccccagcacttgaagccactttttcagaggacggggtggtaactgccgctgccaatatgttcatattgggagaagagccgctgttggatggaatgatggtgttgccagaactgctctgaggtagctggattgggggtagctgtttcacaccactaatgctggcagattggctggcgaggctctgtgccaatccagctgctgctgccagctgctgagataaatgggaacttagcgtggacaaggggttggcagatgttcgtaaagtaccttgagaaggactagaagatgttggcaagtctgcattctgagaagccaacagcaatatttggtgacgaatctgttcgatcaattgcagctggtggatctgctgctgctgcagagctaggagttgttccatgagggctgggacggccagcttgcccccagaggccccgccgcacctcgcttcctgggagaactgggccaccgccaccttggtgctctggaggttctcgatgatgacgttgctgttgattacggagaagttgcccagtgttgtcaggtccccgagttgaggtagagaggttgtgatcgctgaggtacctgtggaggagctgccgccgccgccgctgctgctgctgctgctgctgctgctgcttggggcggtactgctgtggctgccgctggaagtgccgctgccgcttttgttagcaaccggggcctccacctccatggactcttccctgtcaagtccgttgtgttctgaaaggtcgctgcagtccacttgatctgttttgttaactgtgtcattcatttgttcatcaggattatcaggaggggggctgggggagaaggtttcgggtggggaggctggattttcatttacgattaaaactaattgatttttagtacagttcttcttgtggagcagaagatctgataattcaaagaactcggcacagcaccggccacagacgtgggcatccttgctcttagtagggcgactcggttgacccttttctgtgtctccatctcgccgggggagcgaggccacttcggggtcggattggaaatgttgaggcttcgcttgcttcctccgcgacatgctggctcaaacatcagctggggcagaat

SEQ ID NO: 19709 - RNA, 2710 nt, Homo sapiens
  source 1..2710: mol_type = other RNA
ttttttgctggaacatttctggtcttgaacgcatagaaggtgcagctcaaaatcaacaatccattgtatccaagtggagtgacaactcctaggttggtggtgttacagatcaggtagacttctcgaatgcttgggtagtcatgcattatgtcaggaggctccattataaagagggcaacgatgatgcccaactggatgcatatgagaatgaaagcaatcactagctgggcacaggcactcatgaatctgggctttttggtacagatcttcttcttgctgccagccaggatccttgcaatacggttggtctttgttacaagggctgagtagctcatggctggggagagaccaatgccaattctctgaaggtagcagtaaatctgtttgggcttcgcaatgaggcagaaggtacataagtagcccaggcagatgccagcaaggataatgtagcagagttccctgcttgaggacttgactactggtgtatcacggtaaatgatgaagactacagtaacaaacagggtggccaggaggccaaggcaggcaaacaccacagctgcaatgggttcagggtcaccccatcgaagatactgtactgggatcaagtcacaacctgtgagatcatcagtgggccaagaccccagttggcatgccttgcatgtgtactcatcaaagacatactcattctccttacaaggtgtacaggtccaacaacagctgacttctccctttcggatcaccttgatctggcctttctcacatggttcactgcacacagatctgatgatgttgcttttcttggaccatacttcatcatcatccatttttaattctccattgtcccaacttccaacgttgatataatcaaagtaatcttttcccatttccttgaaattcattatttcataccttcctggagagtctccattctcatcgaataggatcgtatctccagaaaccccagtaaaattggttttcatcagggactccaaaagtttccgtccatcaattggcttcatggcatcacagagtcctgcatagcctgggcagagggacatctgcatgttgtggagcccataggccatcgaatagatggcgttgatcacaaatcccattttggaatcctgaacatgatgtgttttcagagtcagagaactattgcaagtcttgttgtatttgctgttctcctgtggaaacccttccagtcggcactgaaaacgatgctgccaaaattcttgaaaccaagggtttcggtggtttgtttctggccggagcttcagataataatcatcaaaccacttgacatcgggagattggagcttgattgtgatgccaccaacagcttctcgctgatatccatctgtcacatcatacctgtcagcccagccatcactgcccagaagcagaaattctcccgctagacccaggcgcctcatggccatcagcagacctctcaccgtcatgccctcacagaagcaggccaccacccgggccttgggcaagtgacttgtgagcttcttcagcagcttatcaaagctctgctcccctgcattactgtagattttgtaagagtgggcgatgcaaatcccttccttcgctgacatatctttgaaggcttccatcccactttctccatagttgccttctgtgtgcacggctgatacataggtccagttgtacctcttcactatgtccaccatggcccttgcctgctgagcatctgaaggcacaaccctcatgaaatatttgaacagagtcttgtcactcagatccatgctggttgctgagtaagcaatctgaggtatgttgaaaagctggagcaaattctggacctgaatggctacagaactggagccaggcccaatgacccctactatgggcttcttggagcggaaggaagaggaggagccatccacacagcgtaccaagccttcttcctcttctgaagaaatgagggaatctcttatgaactcaatgctctgctctagggccacagccgaatgccagcaggagtcccttatctcacagcccagtgtgatgttgggcaagagtgtggggtctgaattgatcctttccagggtatgcagcatggcctccactctctgaatgccatactgttcacggaccgccccacacttcctctcatgaactttgtccacagtaggctggtgatgaacagaaaagagagctccaataatgatgtcacccggcatgtgagccaccaccctcctctcactggactgtgcactcccacggacatcttctttcaaaagtaagactgacaggatcaacagaaggaccattttaggaaaggagttcaagccaataaagatagcatggtggggaaaattcaggagggttctgatagctacgaacaagcgatgtcctacgttgagtcgcaaatcaagaaattagccagcaattcagatgtattttctaaaggaccattttgtccccatgtaccatttagttagatgatccatgtggtcatgatcttctaaaccaggtgcgcgccctgagccttgcgcccccaggcagccgctcctcgagggcttcctgcgctctcgtagcggccttggctgcagctggagcgctagtgtcggcgatggaggcagcggtgacagcaggcagaacggctgcggggcccgcggcggtggcgctcgctctctcgcgccagcgccgggagcacgtgccgcgctcgggcagacgc

SEQ ID NO: 19710 - RNA, 2682 nt, Homo sapiens
  source 1..2682: mol_type = other RNA
ttttttgctggaacatttctggtcttgaacgcatagaaggtgcagctcaaaatcaacaatccattgtatccaagtggagtgacaactcctaggttggtggtgttacagatcaggtagacttctcgaatgcttgggtagtcatgcattatgtcaggaggctccattataaagagggcaacgatgatgcccaactggatgcatatgagaatgaaagcaatcactagctgggcacaggcactcatgaatctgggctttttggtacagatcttcttcttgctgccagccaggatccttgcaatacggttggtctttgttacaagggctgagtagctcatggctggggagagaccaatgccaattctctgaaggtagcagtaaatctgtttgggcttcgcaatgaggcagaaggtacataagtagcccaggcagatgccagcaaggataatgtagcagagttccctgcttgaggacttgactactggtgtatcacggtaaatgatgaagactacagtaacaaacagggtggccaggaggccaaggcaggcaaacaccacagctgcaatgggttcagggtcaccccatcgaagatactgtactgggatcaagtcacaacctgtgagatcatcagtgggccaagaccccagttggcatgccttgcatgtgtactcatcaaagacatactcattctccttacaaggtgtacaggtccaacaacagctgacttctccctttcggatcaccttgatctggcctttctcacatggttcactgcacacagatctgatgatgttgcttttcttggaccatacttcatcatcatccatttttaattctccattgtcccaacttccaacgttgatataatcaaagtaatcttttcccatttccttgaaattcattatttcataccttcctggagagtctccattctcatcgaataggatcgtatctccagaaaccccagtaaaattggttttcatcagggactccaaaagtttccgtccatcaattggcttcatggcatcacagagtcctgcatagcctgggcagagggacatctgcatgttgtggagcccataggccatcgaatagatggcgttgatcacaaatcccattttggaatcctgaacatgatgtgttttcagagtcagagaactattgcaagtcttgttgtatttgctgttctcctgtggaaacccttccagtcggcactgaaaacgatgctgccaaaattcttgaaaccaagggtttcggtggtttgtttctggccggagcttcagataataatcatcaaaccacttgacatcgggagattggagcttgattgtgatgccaccaacagcttctcgctgatatccatctgtcacatcatacctgtcagcccagccatcactgcccagaagcagaaattctcccgctagacccaggcgcctcatggccatcagcagacctctcaccgtcatgccctcacagaagcaggccaccacccgggccttgggcaagtgacttgtgagcttcttcagcagcttatcaaagctctgctcccctgcattactgtagattttgtaagagtgggcgatgcaaatcccttccttcgctgacatatctttgaaggcttccatcccactttctccatagttgccttctgtgtgcacggctgatacataggtccagttgtacctcttcactatgtccaccatggcccttgcctgctgagcatctgaaggcacaaccctcatgaaatatttgaacagagtcttgtcactcagatccatgctggttgctgagtaagcaatctgaggtatgttgaaaagctggagcaaattctggacctgaatggctacagaactggagccaggcccaatgacccctactatgggcttcttggagcggaaggaagaggaggagccatccacacagcgtaccaagccttcttcctcttctgaagaaatgagggaatctcttatgaactcaatgctctgctctagggccacagccgaatgccagcaggagtcccttatctcacagcccagtgtgatgttgggcaagagtgtggggtctgaattgatcctttccagggtatgcagcatggcctccactctctgaatgccatactgttcacggaccgccccacacttcctctcatgaactttgtccacagtaggctggtgatgaacagaaaagagagctccaataatgatgtcacccggcatgtgagccaccaccctcctctcactggactgtgcactcccacggacatcttctttcaaaagtaagactgacaggatcaacagaaggaccattttaggaaaggagttcaagccaataaagatagcatggtggggaaaattcaggagggttctgatagctacgaacaagcgatgtcctacgttgagtcgcaaatcaagaaattagccagcaattcagatgtattttctaaaggaccattttgtccccatgtaccatttagttagatgatccatgtggtcatgatcttctaaacccccctgttggctgcgctgcgagcagtgagactcggtctagctagccccccgaaaagttgggccacggggatcagcagggcagagccggcctctccagtccccggcttcccccccaagatgatctcaagctcattccctccgctcagcgtgcgcagaacagccgagctgagggcggcgt

SEQ ID NO: 19711 - RNA, 2701 nt, Homo sapiens
  source 1..2701: mol_type = other RNA
ttttttgctggaacatttctggtcttgaacgcatagaaggtgcagctcaaaatcaacaatccattgtatccaagtggagtgacaactcctaggttggtggtgttacagatcaggtagacttctcgaatgcttgggtagtcatgcattatgtcaggaggctccattataaagagggcaacgatgatgcccaactggatgcatatgagaatgaaagcaatcactagctgggcacaggcactcatgaatctgggctttttggtacagatcttcttcttgctgccagccaggatccttgcaatacggttggtctttgttacaagggctgagtagctcatggctggggagagaccaatgccaattctctgaaggtagcagtaaatctgtttgggcttcgcaatgaggcagaaggtacataagtagcccaggcagatgccagcaaggataatgtagcagagttccctgcttgaggacttgactactggtgtatcacggtaaatgatgaagactacagtaacaaacagggtggccaggaggccaaggcaggcaaacaccacagctgcaatgggttcagggtcaccccatcgaagatactgtactgggatcaagtcacaacctgtgagatcatcagtgggccaagaccccagttggcatgccttgcatgtgtactcatcaaagacatactcattctccttacaaggtgtacaggtccaacaacagctgacttctccctttcggatcaccttgatctggcctttctcacatggttcactgcacacagatctgatgatgttgcttttcttggaccatacttcatcatcatccatttttaattctccattgtcccaacttccaacgttgatataatcaaagtaatcttttcccatttccttgaaattcattatttcataccttcctggagagtctccattctcatcgaataggatcgtatctccagaaaccccagtaaaattggttttcatcagggactccaaaagtttccgtccatcaattggcttcatggcatcacagagtcctgcatagcctgggcagagggacatctgcatgttgtggagcccataggccatcgaatagatggcgttgatcacaaatcccattttggaatcctgaacatgatgtgttttcagagtcagagaactattgcaagtcttgttgtatttgctgttctcctgtggaaacccttccagtcggcactgaaaacgatgctgccaaaattcttgaaaccaagggtttcggtggtttgtttctggccggagcttcagataataatcatcaaaccacttgacatcgggagattggagcttgattgtgatgccaccaacagcttctcgctgatatccatctgtcacatcatacctgtcagcccagccatcactgcccagaagcagaaattctcccgctagacccaggcgcctcatggccatcagcagacctctcaccgtcatgccctcacagaagcaggccaccacccgggccttgggcaagtgacttgtgagcttcttcagcagcttatcaaagctctgctcccctgcattactgtagattttgtaagagtgggcgatgcaaatcccttccttcgctgacatatctttgaaggcttccatcccactttctccatagttgccttctgtgtgcacggctgatacataggtccagttgtacctcttcactatgtccaccatggcccttgcctgctgagcatctgaaggcacaaccctcatgaaatatttgaacagagtcttgtcactcagatccatgctggttgctgagtaagcaatctgaggtatgttgaaaagctggagcaaattctggacctgaatggctacagaactggagccaggcccaatgacccctactatgggcttcttggagcggaaggaagaggaggagccatccacacagcgtaccaagccttcttcctcttctgaagaaatgagggaatctcttatgaactcaatgctctgctctagggccacagccgaatgccagcaggagtcccttatctcacagcccagtgtgatgttgggcaagagtgtggggtctgaattgatcctttccagggtatgcagcatggcctccactctctgaatgccatactgttcacggaccgccccacacttcctctcatgaactttgtccacagtaggctggtgatgaacagaaaagagagctccaataatgatgtcacccggcatgtgagccaccaccctcctctcactggactgtgcactcccacggacatcttctttcaaaagtaagactgacaggatcaacagaaggaccattttaggaaaggagttcaagccaataaagatagcatggtggggaaaattcaggagggttctgatagctacgaacaagcgatgtcctacgttgagtcgcaaatcaagaaattagccagcaattcagatgtattttctaaaggaccattttgtccccatgtaccatttagttagatgatccatgtggtcatgatcttctaaacccccctgttggctgcgctgcgagcagtgagactcggtctagctagccccccgaaaagttgggccacggggatcagcagggcagagccggcctctccagtccccggcttcccccccaagatgatctcaagctcattccctccgctcagcgtgcgcagaacagccgagctgagggcggcgtgtgcagcaatctccccgct

SEQ ID NO: 19712 - RNA, 3716 nt, Homo sapiens
  source 1..3716: mol_type = other RNA
ttttttgctggaacatttctggttgtgcttctgcctctcaccacgtgggattgtaatgaggggcagcattggggttgggaagggggctgggatccccttcacccctgggaaaacatgcaacaggcctttctggagggacccacggtacccagagaataggccctgccctctgtcctccctaatctgccattgaatccatgagttttcctgttccacaccatcccccgccctgcttgccactccttcattcactcctccttccttcatgcgcccacctcacgctgctctgaccacggctgcccctgccacggacctccggggactttccagctcagtcacatccagactcctcttccctgacaatggtcctgtccctgagcctttgcaaggctgttctccatgcaggaatgttcagggagcatccttcccacaccagggtgtccgctgcctcttcaggaagctgcctcaggccaccagtcctcgtggttctgtgctctctgccctctcaagctctccatcccctgtccttgcacttcatttatttttactggtgttcctcagccatttttctctatacagctccccccaccccccaggagaagagtagcctgagagattttaatgtgaccagtgtcttgaggacaccaaggcccagagctggcagggccttacaggcagagcaggccctggaacccaggcctcctgactcccaggctctgggcctgcggccatcatgccctgttctcttgcctgggctgcatcccttcagtcccctgcagcacccctgagcaggctcaggcctctgcacaggtgggcaggtaggcctggctcctgctcacagatccctgctcctcacctgcctcctccactcccagaacccagtcccttccttggccttttctccccgaggcttcttcctcctgctagagcaggaggagggaggccatcgagggcagctcagggaaggctgtcttcagggtgggggacggtgtctgtccattctaggaaatagcatcagcgctgttagtgcctgtcaccatggcgacccgagggcaggaacaatcaagggacgtgtgtgatgtgtgcagaggagcgggggtggctggagtttggtggggacacactgccctagaggtctctgagtgggagatgggggagggagtgccaagtccttttcctaccacctcacaccctagctcagggctcggggtctgtgggagcacaagggcaagacccggaggacaccctgctctaatcagaacacctttttcttgaggattggggtgggggagacggagagagattcacaggttgctaggagctcagacgtgatgccaggaggccttgcccaagctgggatacttgggaaacaactttcagcttcatgtgcaagtggaagaattaaaattaggactctgacacagttggagaggtcccccaaagggcatggcagcttctgctgcagtccccaggcagttgggggcctgtagaaacccacatggaggctgtgcaagagggaggcaaatgatggttgagggaatcattacttcctggagccagttgtgtgtgtcttaatttgagcttttttctccaacctgtcttgctcgttttctaaatgggagaaagatgaagccagcagggagtgcgtaatgtttgcatgcagcagggctttcgtgactgtgttttttgaaaaggccttgttaaggaaatgctgacgatgagtgaaacttgccaggtctggctgataacatgggtgagtgccctgatcctggaaggaggtctcagagagaagggacagcagggggcgagggatacccagaaggaagcttctgcatgtgtacgtggttcaggaaatcggcatgctcttgcccagacaatgttccttcccttattggtgtgttgactcacccatcattcgttccattctcactgggcatcttctatgtggcagggcctgtaccatgtgctggggcctttggagaccatcccattccttgtccagtctcataaaggcctgttactaaagcaccgtagatgctgagaggtccgatttgtgtagaaatcaatgggccaggagagagagagctgatgaagaatgctggtccgctgggggctcctttgcctcctccatctctccctgcatcatcaggcacagtagatctgggcacacaacctgcttagtagctgctgttgagtggacactgatgtgctaaagacatagacaatggtgacaggaaaggctatgaagtggttctgtcctggaaatgtgctccaggcagagattcccaaagtcatacgtgcacactcatggtccacccaccacaccctcacacacacatgtctacataccttaatatgcacatgcttacctatctcagacacatctccaacactgagggaggggccaacggagacgagcatggagacagccagtgcagaaggccattgagggcggtgggagtgggtatgggattgcagccctgaattcgagccccacctgtgcccttctgagtccctgatccatctcctcatatgtcatgtgaggaaggaaaatccaattttaaatcaaccaacacagaccctgagctctcagggtgatctgggcattgaggctctgaaggtgagtgaggcccaggctctaccctcaaggaactgggaaccagttgtattaattctctattgctgcagaacgattaaccctgaaacttagctacttaaaacaacgaaccattgttatctcacagttcctgtggcctgcaatctcggttcaacttagctgggtaccttgtggctcaggatctcacagagaaaactctttaggcaagagcatgtggatttcctgaatcacatacacatatagaaacttccttcttgggcatcccccaccccctgctgtcccttctctctgagacctccttctaggatcagggcactctcagagaagcagccagctgtcaccagggttgctgtcatctcaaggcttaactggggatggagaatctacttccaagctcattcaagaggcagttggcaggaagccgcagttgctggccaaaggctggaggcctccatttcttgctgcagagacctccatctaggccttctgagttctctcagcacatggcaactggtttcccccagagcaagtgatcagagaaagagaaagagaatgcaaaacaagccacagtgtcttttataacaatcagaagtgacatgccatcacttctgccagaggttcctgggtcacatgaaacaatgctgatacaacgtggactaactacccaagggtatgagcacaggaggtggggatccctaggggccatcttagaggctgtctactacacaagtcaagtctcagccgagtggaaagtagtattgttgtagctgttgttattgtaggccactgcggacagttagttggtcagctggcatcaaggactgggctcctgtctccattccaggattctgccgagccctcttgaaggtgcacagtggtagggaagagatgactgaaaggacatccagtgcctttaggagttgactggcaacgtgggctctatgaggacgaggggtgagtgtcctgctccaagggggcgggtgtgcccaggtccccatcctcaaggtccatgggattccttggtacctggggcacccatctgagctgggggtcctgtgagtcctgctggatgcatgtgtgcatctctctccctccccag

SEQ ID NO: 19713 - protein, 15 aa, Homo sapiens
CANIFPVFAPVTFRT

SEQ ID NO: 19714 - protein, 16 aa, Homo sapiens
PVFSLKHKCHHVTGSC

SEQ ID NO: 19715 - protein, 16 aa, Homo sapiens
LAPKPKPGGFQEQLRC

SEQ ID NO: 19716 - protein, 16 aa, Homo sapiens
CGMGHRAQPLRSDFKQ

SEQ ID NO: 19717 - RNA, 21 nt, synthetic construct
  source 1..21: mol_type = other RNA
  misc_feature 1..21: note = shRNA-1
ggagtcatctccactgcattt

SEQ ID NO: 19718 - RNA, 21 nt, synthetic construct
  source 1..21: mol_type = other RNA
  misc_feature 1..21: note = shRNA-2
gcgtctacttccttcgtcttg

SEQ ID NO: 19719 - RNA, 21 nt, synthetic construct
  source 1..21: mol_type = other RNA
  misc_feature 1..21: note = shRNA-3
gctaggtgcgtctgcttcatt

SEQ ID NO: 19720 - RNA, 21 nt, synthetic construct
  source 1..21: mol_type = other RNA
  misc_feature 1..21: note = ctrl-shRNA
cctaaggttaagtcgccctcg

SEQ ID NO: 19721 - DNA, 20 bp, synthetic construct
  source 1..20: mol_type = other DNA
  misc_feature 1..20: note = midRs0045 primers
atggcggcagcggctgtggt

SEQ ID NO: 19722 - DNA, 20 bp, synthetic construct
  source 1..20: mol_type = other DNA
  misc_feature 1..20: note = midRs0045 primers
aaactccaccaatccacagc

SEQ ID NO: 19723 - DNA, 20 bp, synthetic construct
  source 1..20: mol_type = other DNA
  misc_feature 1..20: note = midRs0045 primers
agtaaagcatcccttcatcg

SEQ ID NO: 19724 - DNA, 21 bp, synthetic construct
  source 1..21: mol_type = other DNA
  misc_feature 1..21: note = midRs0112 primers
atggcgagcacggtggtgaag

SEQ ID NO: 19725 - DNA, 20 bp, synthetic construct
  source 1..20: mol_type = other DNA
  misc_feature 1..20: note = midRs0112 primers
tggcaatgggcacagtgagt

SEQ ID NO: 19726 - DNA, 20 bp, synthetic construct
  source 1..20: mol_type = other DNA
  misc_feature 1..20: note = midRs0112 primers
gcgagcacggtggtgaagta

SEQ ID NO: 19727 - DNA, 20 bp, synthetic construct
  source 1..20: mol_type = other DNA
  misc_feature 1..20: note = midRs0188.1 primers
ggttgccacatccaagaaga

SEQ ID NO: 19728 - DNA, 20 bp, synthetic construct
  source 1..20: mol_type = other DNA
  misc_feature 1..20: note = midRs0188.1 primers
ccggaggtagtgaagtaagg

SEQ ID NO: 19729 - DNA, 20 bp, synthetic construct
  source 1..20: mol_type = other DNA
  misc_feature 1..20: note = midRs0188.1 primers
aggcatcaagtatcggaaga

SEQ ID NO: 19730 - DNA, 19 bp, synthetic construct
  source 1..19: mol_type = other DNA
  misc_feature 1..19: note = midRs0188.2 primers
agaccaccgacagcaagat

SEQ ID NO: 19731 - DNA, 21 bp, synthetic construct
  source 1..21: mol_type = other DNA
  misc_feature 1..21: note = midRs0188.2 primers
cgtgggtgttgagacggtagg

SEQ ID NO: 19732 - DNA, 20 bp, synthetic construct
  source 1..20: mol_type = other DNA
  misc_feature 1..20: note = midRs0188.2 primers
cggtccgaaggcatcaagta

SEQ ID NO: 19733 - DNA, 19 bp, synthetic construct
  source 1..19: mol_type = other DNA
  misc_feature 1..19: note = ssmidRs0323 primers
gcatcttccagatcccaat

SEQ ID NO: 19734 - DNA, 24 bp, synthetic construct
  source 1..24: mol_type = other DNA
  misc_feature 1..24: note = ssmidRs0323 primers
cgatgtagaagagccagggaagta

SEQ ID NO: 19735 - DNA, 21 bp, synthetic construct
  source 1..21: mol_type = other DNA
  misc_feature 1..21: note = ssmidRs0323 primers
tgggatgtaacagagcaagcg

SEQ ID NO: 19736 - DNA, 114 bp, synthetic construct
  source 1..114: mol_type = other DNA
  misc_feature 1..114: note = CSSD
aattcaaagaattaaccttaattgaaggggagggttcagtacttttgtgtagtacaaatatcagtacttttgtgtagtacaaaagggagggcttcaattaaggttaattctttg

SEQ ID NO: 19737 - DNA, 117 bp, synthetic construct
  source 1..117: mol_type = other DNA
  misc_feature 1..117: note = CSSD
gaattcaaagaattaaccttaattgaaggggagggttcaccactgcactcgctccagccatatggctcatgcctgtaatcccagcaagggagggcttcaattaaggttaattctttg

SEQ ID NO: 19738 - DNA, 118 bp, synthetic construct
  source 1..118: mol_type = other DNA
  misc_feature 1..118: note = CSSD
aattcaaagaattaaccttaattgaaggggagggttctggggcaggagggaggtcagcatgatatacctgtagtcccagctattcagaagggagggcttcaattaaggttaattcttt
